European Patent Specification EP 3 579 852 B1 - sequence listing, part 3

SEQ ID NO: 3 - DNA, 732877 bp, Lactobacillus buchneri
aaccaagtagaaatggtgttcaagggcagaaaattaatattagctagttttgagagaacgaagttctttcaaggaaaaatagtgtggtggcgatagccagaaggatacacctgttcccatgccgaacacagaagttaagcttctgcacgccaagagtagttgggggatcgccccctgcgagggtaggacgttgccacgcgattattccggcatagctcagttggtagagcacctgactgttaatcaggttgtcgacggttcgagcccgcctgccggagctttgtcgaaatgctaacttaattgttagcattttttgtacaatggatttgccgacttagctcagttggtagagcatcggtatcgtaaaccgagggtcacaggttcgactcctgcagtcggcataattatgcaaattagaagaaatattaaaatcaggaatgcctatttaacggcattcttgatttttttaatttataaaaacgtactagaaagtattaaaatataaataataacgggcaaataacggtcaaacgggcagaagaagtttaacctgatacagagtaaaataacaaaataaaaacggaaccttattaaaggttccgcttaattggtatagtttcatcatgagaggaaaggttatctaactcttcacgaatctgttgatcgttttttgctttatattcatccattaaataggaataaatctttgttgttgtggatacgtcagcatggcctaaacgcttagaaatgatgtaaatgtcaattcctcgagatagtaggtaagctacatgtgagtgtcgtaaagaatgaaagtgaaagccttgctttttaattcctaagtcttttagtatagaacgcaactttttattaacggcagaggatgatggaatggatttatattgattaacaaaaattagttctccattattgtgatccttcaagatctttaatgatttcagcaattcgtcattaactgcaatgattcgatttgaaccagccgtcttggtatctttgaatccaccgccttcggatgaattccaagatttagtaatgctaatcgttttaaaattaaaattaacgtcattccaagttaatgcttgaatttcccccaagcgagcaccagttaaaacggccgtcaggatcataaaagtggaggtaaagtgatagtttaagtgattctccaaataagcgatgagacgcttaatctcagccacgttgaggtattccacatgcttatcacgtgacttatcataaataagactgactcgctgggtgaaatctttatgaatcagatcgtcaagaatggcattttgaacggttgctctaatcagtgaattaactttataaacagtatcttttgcatgagaatgaccatagaagttaataaatgcttgatattgtgggcggtcaatactttttaaagtaacatcaccgaaataattatgtaatacgcgactagttattttatagcgattcttagtctgattttcaatcttaggctctttgtacgtgtgataaaaatagtcaaaatagtcagcaaacttaggatctttaggaacgagatccaaaccattgtggatatcgatttctaattgactcgcaaatagttttgcagctgatttagttctaaagccgctctttgttttctcgtgttcctggccattggcatcataatagtagtatcttacttggtatccatgaccatgtttacgtattgatggcattattaccctcctttggataatatactaacacatagtggggaatctacttaatagagcgatcatttattaattatcatggcatatagattacaaaaaaatgttaaagcctttacaacttctgttttcttttgcattcaaccttgattatgttatactatttacagcaagttagttgaggcatgtgtttgcatgcctaggcagcttgaaaaaacaatttttttgggaggaaattatacatgaaaaagtcattgaaaaagactctttttgctggtgtagctgcattatcatttgtagctgttgccggtgtatctagcacaaatgctagtgcaaaatcatatgccaaagttacatcaaacaaagctttgacaactgatgctactactcgtaacgttaactttaatggtactaacgctctttatacaaaggctggtactttgaagggtgccaagaccgttgcaactaagactactaccaaagcattagctaatgcacaaactggtaaggctaatctacgtgcttaccgtgttgctactactaaccgtggttcagtttactacaaggttgtatcattcgataaacaatatcgtggctggatttatggtggtaagagtgcctcagcatttgctggtggtgtagcttcatacgctactactaaggatgctactgctcctgcatcaactaacacttataagttgaactcaactagcacaactgctaatactactttgttcaaggctccagcatggactcaatataaagttggccgtgctaaggatgcaagtggtaaggtaattacttctactgacgcttataaaaatgcaacatttactgtaagcaaggctgttactacttcacgtgaaggtgaaacttggtatcaaatttcatcatcaaatgctaatcttaacggtgcttgggtaaaggcatctgacgttactcaaactaatccacaaagtgacacatcagtacgattcacatttactgatccttcaggaaatgttgtaaaaactttagattattctaaggcaaatgctaagtcgggtgagacccttggatcattaacaggaacaaatggtaattattcatggtcgttatccactgatgttgcaactgatcttcaaagcaagattgatgctactttgaatggtaccggctattcttacaatgtttcagcaaacacatctacactggctcaagcaaaagcaggctcaacagttacattgcctgtgactaagggtgatgttgtttatcaaacgcttaagccttatgtcgctaccaaagatgatgttacatcaactcatttattaactgcaaattccaaatcagctggtgcgttctttaagggctcatttaaggaaggcgatcaaaccattgacattagtcagcttgtgattactgatgataatgggaatgttcaatcgcacagtaattctttgcctgctgttaaaacttatattgatggtgtaacaacggacaaggatactgctcttgcaaaccttaataatgatgttaaagagtatgctgcaaacttctatttggctcctgctaatattagtacatctgatttattcagtggaactaagggatccgcatttagttctcaagatgttcttaattatttagcaaagcattctactttgaatactcttaagtcagctatttatccggtatttaatgctgacggtactgttaaggaatgggatcagttaaacttgaatgctacgagtgctaatagtggtactttcggctcttcacctgttcaagttgtttatacttacggtgatggtagtgctgtttcagatccattcagtgcaacaaataatggtagttcagtaaatccattacaataattaatttagcttttgttgatttataagcaaatccttttggatttgcttttttcttttgcattgattaaattaagcaaataattccatttgaacactagttcgataatggtcaaaattcagataatcataggagcatttgtattcaaaaagattgataccttacggtatcaacctgaaaaagtttactgtgtataattattgtttgctgcaaagattgtgtattagcctttctattcaaaatctagctcaacaacagattcttctagttgatccaatatctcattaactgaaataaagtgtcgccacttattaggatcatgcttagcaagtcccttaaaattactgctgatcttatcgtggatatttactagaaatttgtaatacatattagttgcttcacgatcgattctttcctgtggccaacgtttatccagagaacgttggttatttttttcggtcaaatattgcaggcatttgctagtaaacaaattctcgatattgctattctcttttaagtaatctcttaattcttcagtatccatgttagaatcctccttaaaattaattaattgactatttaggactcgaacctaagcaaaccacctggttagtcgaaacatatgttcttttaaaactttaaatgaagcccccacatttgggagctcataagatcactttaccgattacattaacttcatcacaatcaaacaccatgtcatcgtatgccttgttaattgattttaaggtaacggtattatcctcatttacataaaactttttacaagtaacaccaacatcacgaatgtggacgatcgcaatttcaccattctcaacctctggttgatagtgaatgaacacctgactacccttttgtagtaggggctccatagaatcaccatccacagtaactaattcatctgcacccgcggggaccttctcaccagcaatcatcttatggataagatgagtatcttgatcattgccgttgataggtgatccggcagcagttgaacgtccagaagggatttcaatcattggcttgtggtcaaacattgaagacattttttcattattctgttcgtctaattgatcactggcataattgtaaactttcttttggcgagaagggtggagctgattataaataggaagaattgcattttctttgtttactttttctctattgcgtgggacatcaaaccccattagccatccttcatttacatttagagctttggccaatatatataatttatcttgacgaggttcgcttttattattaatatattggcttaaatcggttttacttattcttattcccgttttttctgagaaaggccttgttttcgctatgatgtctacttgcttaatatttcgctcattcatcaattgtttcaaacgggcaccagtagaaattttgctagtcaacttttcatctccttaactacttgatgtcttaattatacttttgattgaacaaaagttcaatatgaaaattcaatttttttgaacttaaacttgacatacaactaaatgttaattattataataaatgtaagttcaattcttttgaactaaaaatttttgaaaggaggtttttctatgatttttgattactcaatgttattaggaaaaattgtttccaaatatggaactcaatataattttgcgattgcattaggtacttccgagaggactctatcacttaaactaaataataaaattccttggactcaaaaagaaattgaacattgtattagtttactagatatttctaggagagacattcctaaatatttttttgatttgaaagttcaattttcttgaactttttttagaatagaaggtgttacaaagacaaatttcagtttttatttagtccagatacgtacacacagccagcataggagatgatttaaatgaaaatcgaaaattggaacgatcatgagattcgttttgtggaagtagaaggtgagtggtgggcagtactatcagatattgcgcaagcattgtctctggatactcgaaaactgaatcaacgtcttgatgatgacgtactttcaaagtaccccatcttagattccttgaatcgaaagcagttgacttctgtagttagtgaatttggtatttacgatgcaatcttttcgagccgtaagccagaggccaaatcatttaaacgatgggtcttcaacgtcattaagcaattacgtgaatccgctggactcgagggcttcgaagtatttcgcatgatggacaaacaacaccagaaggatgccatgaaacgattgagagacggcttgaaacggccagtaagagttaactttatcaaagctaacaccgtggccaacaaagctgtttcgacaaaatatggttatccaaagatgataaagaaaggcgagatgactccagcaatgttagttgatcgggaaactgttttagacgacaccgtgaagctgatggaagttaacgatcgctataacctggggttgtctgtaagtaaggcgatttatgcaagtttagcgaaggcacagccagcatagaaaggaggtgagttaaatggaaaaaggcaaactgcatcagtactttgatagtaatattcagcctattttaaatatggcgataggagttctatttatgacaattggttacttacttggtcatatgtcctagaaagaagccaagtgatcgtcaatgaatagttgaaaggaggtgaataaagtgaaccaagacgcagaaaaaacaccccgagccatttgtggtagcaaggagtgcaataaggaaaaaatcgtgccaatgacaaaagaatcgcgtaaaagagcatttaatcttttatcaaaaattctttcagagctatacgaaccaaattgttagttcgttcattctcatactgctgaataaatttaaatattttgttcgtccagtcgtcgttgggattgccatttttgacatcctcacgtatccgctcaatgttctcttcatcatcaaacatgtcgtcaaacttgtttaaaaattcagcgcttgtcacaattttcacctcgattacttgaattaattaaattatacgtcagtaaataatagaaggaagtaataaaaaatggcaaaaccacgtttagttttagaaaagaaagcaccagaaccacgagtatcacgattgattagcattaacactgatttgtataaccagttaatggacattaagcacgaaactggattaactgtcacagcggtagttaataagtttatcgcttatggagtgaagaatgtagaaattgaagacaacaaaaacgacgattaattaatccacgtcagatcttatcaaaaggaagtgagaaagatgatcgataagaacaccagttttgaattaaaacaaattgatttattagatcaggcaaaaagcacaaatatttctctcatcttggagaatggaagtattcttctttcagaaataaaaaaagctcagcagctaagtgctgagctaggagatgtgctgaatcatatcaagcactttaatcccgagtttcggatgaagtgattgatacaatcttaaaatctgcgattgattagaataattcaagcatacgccaataaataccataggagaattaatcttgaagcacgattatatttatttttgccatgacaatcaaggaaataatgttccacttgcaacaggatcaacgagtgacttacaactagtcctttggttgaatcgacaagaaaaagaaaccatcattccaaaaaaatgggcttctaaagaattatttgttcgtgtcaatgaggagaactttatcgttaaaaaccgttcttaatcatctgacttttaatgatgtttgaaatcacttgtgctgagatgctttcaatcatggacatggaaaccgaagctagcttttcagtaacgctctttgtagttgaccaaactttgctgtctctaatagtgtctaagaatttgtggccgtcccaggtaagcatgccaaatgtaacattcttctcaataaacagcataatatctcgaacacagtcctggttaagtttcatcgttatcacctcgattaattgggataaatcaagtatacaactaagccaaaattggaagtgaattaaatggatcagaaacttcataatgcagtacgagaatatttattggaactattgagcgaaaaaaataaaagtccagaaatggctgcaaccattgctgaactttatagattgttacttgaataagacactcatgatgtctcttcggtcaatgctaaagattgtatcaccaataaatttgacttctccgttagcatcatttaaagaaaattgaatcatgagactttgtggtaattaccacagtgttcatagagttcacctcaattaattgggataaataaattatacaactaaaggaagtgacaaaatgtctcaagtcattagtgctaaagtatcaattcaaattcctgataattttgaattgataaataaggaagattaccaaaagttaaaacgggaatcaaccttcggacgaacttggaatttaaacgatcttcgtaaatggtgtgggaacaaatcaccacaatggttaaaagaaaatttcttggaaaatccaaaatattcacgggaaatgcaagccttaatggatgatagatatttagtccatcgtggaagtaaaggtagtccgtggctgtttaaagctaccaaaatgcagcagtttctggaggatcattggagtgaattcaattggtaaaaacattaaattcttggtaaatctaataatcgatcgtgacggcttaaggaattcttagttttaatatataaagcattgtcatgatcgtaatcataagtgatttcataggtaccattaccgagaatgtaaaagtagtgatcaccacgaataatattggctgctgtggcttgaataagttcaattttcccactggcctgttttattaaatcaatattttctggtgatgcttgctttcccttggaataagttcgtaatcgaatagcaacaatttgatgaatcatacgacttaacctccttaatgggttgaattcaaaattctacaaatattaaaaaggagtgatttaattaatggaatcattggaagtactagttttattgttcttagcagccctggtcattgaatacttcataccaactgggcgtcactaagaaaaaaagaagctcaatcttgtcatgataactcatatgtcactgaaaggtcatgaaaatatgaagcttccaaatgattactggattttattaattagcgacttttctccgctaaataatagttgaagacgtttttaacaatttctaatttggaatctgaaaaaccacttgacttaagatattcttttaaatgtttccaatctaaatttcccttaggaaacgatctatcagatcttatttctcttgctacatcaccaactggtaagctaacgtctttaaagcgcattaaccaattgtaaaaattcataaaaattcaccaccttaattatatgcactaaatagcccactaccgtaaatgggtggactataactactaatattataacacctggagggtcatcagaatgaaaacattaacaatacagaaccgtatcaaacgtttgaatatgattattggacgcacacccgtggaaaacgatcatagcttgttggcatatttctttgtcttagataaagaaaagcaacgactatctgaatatattttacatcacgaggtggaataatgactaaattttggaaagcagttggtgtaatggattcccaaatattagaaactggtgtctctcgtgccgacgttatgcgaaagctcagcataaagtatccgacttacgtcgtaactgggaccgacaaggattttatgaagaagcggaaagaacgagtcccaatttatcccgaaccaattagattaatctgtggcagaatcacaaaatctaaaagaaaagaaatagcgtcaatgaaggattcaattgatcaacgacactatttacattaaaagatggaggtaaatataaatggcaaatgaattatccctaccagaatacacgattgactatcggccaaccgttattacaattaataattttgatcaattaaaaacagctgtagaagcatatgccaataaatatcaaggaatggcagtaacagcttccacagaaaaagaagccaagtccagtcgagcagaacttcgaaaattgaagcaagctcttgatgataagcgtaaggaaattagaaaaaaatatgctgaaccatatcaacggtttgcagctcaaattaaagatttggaaatgaccctggatagttcgattaacccaattgacgctgggctaaaggaattggaagatcagcaacgccagcttcgcttaaaacatgttcaatctctgattgctgaaatggcacctaattaccatgtggaaccaggcgaggttgaaattgatccgacttggttaaataaaaccaccaccaagaagaaagtaaccgaaggaattgctgatgtgatgggttacattaaaaagcaacacgatgatttaaaaaccggtatcagtactattaccaaatatgctcaagcttatcacattgatccagctggttggatcgaccagttgaagcaaggccaagatgttaattatttgcttcaagcaattgataatcaggtcaaactaaataaacaaaaacagcagactctggaagcacaagcagcagaagcacaaacacatcaaattcagcagaaagatagaacgattgatactaacactggtgaagttgtttcacattcagtgtctttaaaaataacggcaacaattccacaaatgaaactgttgagggctttcatggatagtaacggaattcgttatcaaagagtgggtgcttaatcatgaagacgattgaagctaaagatttgcagcgaaccttgaattggcgagtcattctatatgctaaacccggaactgggaaaacaacttgtgttaaatatttacctggtaaaactagaatttttgatttggataactccgctaaagtattagctggcattagcaacgttacagtcgatgaaatagatcgaactcaccccgaagaagacatgaagcaatatcttgaacatgcttcagaattgattgttggttacgacaatttagttattgataatgtatcaagttttgaaaaagattggtttgtggaaaaggggaagggtagtcataacggcatctcaaatgaattgcaggattattcacagtggactaattatttttcgagagtaatgactgctatctacgcgttgccagttaatgtattaactacagcttgggagacgcaacgccaaattactactgaaaatggtcagcaatttaatcaatatgcacccgaaattcgtcaaagcgtgatggatggaatgttgggattatgtgatgtagtcggacggttgattattaatccgaagactaacggtcgtggcgttatgctgcaaggaaatgactcgatttatgccaaaaatcgtttggacaatcgaaccatgtgtgctgctaaggacttatttaggtttggcggtgaatagtattgccatttaaattattcgattatcaacaacgattggtagatgaagcccgtcaaaagcttgctgaaggcaatcaaggtgttttgatcgtttcaccaccaggaagtggtaagtcggttattattgcagaaattgccaggttaacagttgctaaaggtggacaagtaatgttttttgtccacagacaggaactcgtgaatcaaataacccaatcttttcagaaacaagacgttgatttaatgcactgcacaattatgactgtgggcaagattgttaaccgtctggggaaactacctaaaccaaacttaattatttgcgatgaatcgcaacatagtcgggcaaagtcctatttaaaaatatttgatttttatagagatgtaccaagactgggattcactggtagtccttggcgaatgaatggtaaaggatttgatgatatttattcagccatggttgaaggacaaaacgttacttggctaatacaacatcgtcaccttgccccatacaaatactattctattaagttagtggatgacagtaaactaaagaaatcaagtactggtgattacaccaataactcgattgacgatgccattgggaaaacaatctttggggatgtggtcaaaacatatcgtgaaaaggttcctggtcaacaggcaattgtatacgcccatgacattgaacatagtcaggcaaccgcagccgcgttttgtgccgctggaattaaagcagttcatgcagatgccaaaacgcccaaagccaaacgtgatcaaattatgcatgattttaaaaatggcaacattaaggttctatgtaacgtggatttgatctcggaggggtttgatgttccagattgctctgtagtcattatgttacggccaaccgagtcattggtattggacattcaacaatccatgcgatgcatgcgatataagcccaataaagcggccacaattattgatcatgtggctaactatacccgttttggtctgcctgatactccacgacaatggagccttgaaggacgacctaagaaaaaacggcagaataacacaaaatcaattccggtcaaaacttgtccaaattgttttgccgtggtaccgacacaatgccgtgtttgcccacaatgtggtaatgagattaaatatgacgctgacggaatggaaattgatgaaacggccagtattgaaaaaattggggaatttaaactgactactgattattcaaaaatccagacggcaagaaaaaagccggaagatgcacaaagttacaaagagttactagaaatcgctaaagcccgtggatataaagctggttgggcctatgtacaagctaaacgactaaaaatggttaactaatggaggaattttaaaaatggcatttatgcaagcaaattacaagaacaacgaacacaaagatttttcagctttaccaagtggaaattacgagatgattattaaatctgcccaggagaaggcaactaagaacggggcagaatcactgcaattagatttagtggttcgaaatgacttagatggggttactggattaaaaaataccaatgccaagtaccataaccgtcatgtctttatggacaattggaaacgcaaaactactaatcagtacgatttggatagtttccaatacattcttgaagctgttcaaattccagaaggaacaccattgaatacaattaatgattttactaaagcagttgctaacaagccagccaaagtgtatgtcaaaaaaacggttgatgattatggcggtgaaaagaaagacatcaatcaaattgccccttggaattttagcaagagcgattatccacaagtgcagcatgtatggaaagaccaaaaggacggtaaaaacccatttactggtaatcaaccagcatcagccccaacagataatccatttgacaattctggagattcaattgatatttcagacgatgatttaccattctaggagggtaaacagtggcatatgaaaaaattccaaatgaattacgggccttaaaacaatggggactgtttcagaaaatctggcaacctgagcgaaataagtacaccaaaataccccacaatgcgctcgatggtggagctggacgcacgaatgacccaagtacctggactgattatcaaacagccttaaaagcgcttaaaacgtatcaaatggatggtctcgcgttttactttgctaatggttatgtcggtttagacatcgatcatattggagacgaactggaaagatacgccgcacaggattatcaacaaaatgaagttcaagatgtgttaacgatgactaaatcctatgtggaaattagtttatctggtaaagggattcatgccatttttaagggcaagattcctggtgatcgacgccgtaaaggtaacgttgaaatgtatgagtccggacgtttcttcgcgttaactgggaaaaccattggtccatatagtgatcgaatcaacacaccacaaccgcaagtgatgaaacttatttataaacactatttcggtgaaaacaatgtggtaaagcttcccaatcaggcaccaatcaggccaaatgatttaagtgttgatgaaattattaaacgcgcggaactttcacggactggtaaacgtttcaagatgtttatgcacggtggttgggagggcttctatacttcccattcagaagctgatctagccttttcgaatgatttagccttttggaccggtcgcgactttaacaaaatggatgaaatatttcgaaagtctagcctcatgcgaccaaaatatgatgaaaaacatgggaaaaccacttatggggtttcactccttaacaaatccattaatgaaactcgggaaacctttaatccacaacaacatcccttgcataaatataatcttaaattcctacaatctaagcctaaaaagaaattaccacctagaagctgggatgacactgtgaatgctgatcgatttattgatgtttttggaaatttagttaaatattcctatgttgataagtcctggtatttctataatggcagttattgggaaatggacgatcagggaaaagcagctcaatttgttgatatgactgtggataatatgaagaatgagaagctgcatgttgctgccggagtggatcctgaaaaggctaaagtagcttgggaaaagtttttgaagaagtcgcgtagtcatgctgctaaacaagccatgataagcgaagtacaacatcgggttccggtattgcatgggcagtttgatcaagacaaaactttattgaacgcggttaatggttatattgatttaacttcaggtatcttaaaagaccacgatattaagaaaatgttcagtcatcagacaagcgtggaatacaccgacaaaattgattgtccagaatgggatgaatttttaaatcaaatttttgctggtgatcaggaattaatccattacattcaaaaagcggttggatactcggccacgggaagtatcaaggaacaagtgatgttcattctgtatggcaatggtcgtaatggtaaatcaattttcatcgatacgatttctgatattctgggaacttatactaagtcaatgcaagccgattcaattatggtacggcaaaacaaatcgggagccaactcggatattgctcggttggaaagcgcccgattagttacctcaagcgagcctaatgagggtgtgagattggacgagggattagttaaacaattaaccggtggcgataaagtaaccgcacggtacttatatggtaaggaatttgaattcaaaccacagtttaagctgtggttagccactaaccataaaccaatcattcgtggtactgatgacggaatttggcgacgattgatgttaattccatttaaggtaaaaattcccgatggccaagttgataaaaacctaaaggataaattaaaacgcgaatccgtgggaatccttaattggatcgttgagggttgcttattatggcaacgtgaaggcttgaatccaccaataagtgttactcgtgctagtcggcaatatcgtgaagaaatggatgttattagtttatttgtagatgattgctgtgaagtgggtgatagttaccaagcgcctgctggtgaactttttaagaaatatcaatcctgggcaaaagacaattcggaatactctatgagtaagcagaagtttagcagagaaatgaaacagaaatttgaaaccaagaaaagtggatccatattttatattggattgaaaattaaaggcgatccaagactgggctggattaaataaaaatgggaggataaaagctcttttgggaggataatgggaggatcattttcaagctaaaacccttgatacaactacatttatatactctttttatactatgggaggataaattaataaaagtatataagataaaagagtaaaaaaagatatatataaaggtttggtgaaaagatcctcccatacacccaaaaacaggctttgttcttacagccgcaatggatacagcgactgaatcatcctcccatttatcctcccatccgtcataattatttggaggcgtgtaaagattaaatcagaacatgaaattcaaacagaaattcttttggcattatctcgacatgattgtactgtttgccgtagtaacgctggaaaaattaaaactgatgatggcagacgaattatgttatttccgagaggttggccggacattaccggttttgaacatcacagtggaaaaatgattttgattgaagttaaaaacgaacgaggcaagttacgtgacgatcagaagcggtttgcaaaatttattaagcaatatccagtgttatatggtgtttgccgttctgtagatgacgcattaaaaataattggaggtaaataaaaatgacagtaaagattgttgataaggaattgttcaaaatgtaccaatgcgcaatggcagaaaatatttctgattggaagcgaatagctaaattcgccaaattcattgataaatatgctgatgatgaaactatttctaaccgtgatgatttagccagtgttatagatgcaattttaaatcatgaaacagtgaaattgtctgcaccaatgtatcgcttgaagatgaatggcatggttggtagcaatgggcaacagtatgtatctcggcgagtagatgatcgtggtgggtatttcatctgtggagttcgtaacccgcgcgttgatcgaggcgcaattacgcagcaatttacacgtgatgaagctgaatttttgaaggatttgttaaataattcaagcattcaaagtgtggaggagtgacgataatgaacagacaaattaaattccgtatttggagagcacccgatgagtatagcaaaacatcctggatggaatcatgggatagccttatgaactactctatgtctgatatctttcagctggataaccctgatgatgttcttgagcagtataccggcctgaaagacgtcaatggcaaggaaatttacgaaggtgacattctagcctggcattcaaacatttatagaaagcatgattgggtaggattagttctgtatcgcggagctggatttgcggtacaagagagcgataagtcctatagttcaccagaatggctggattgtgcttgccgtaaggatgctaatatcattgaagtcatcggaaatatccacaagaatccagaattagtggaggcagaaaaatgagaaagtttgaatatgtagcgttagcagaaaaaggaattattgaaagtacttttgaaattcaacctaatgcacatggcacctttacttttaccgcaattcaaaaatatcctcacaagaaagataagattgttcaaatgcgatttaacaagtttgggttgatcgctattatcggaatgttacgctaccttgatcttgaatctcaggaggatgactaatgaaacaaatacttgaaggcatttggaatgcccagcccagccagatttttacttggatagcaattgctgttggggtattggccgttgtttattgtttgattgtatttttaatttttaagtggatgaaataaaggaggccgaatgatggtaccaaaatttagagcgtggtatatgccgtttggtcctaaaggggcagcacaagaaatggtacatggaaaagctagtagtattttgacgtttgctgagatgtcaccagatgagtatattgttgagcagtttactggtttaaaagattcaaatggtgatgatatttatgaaaatgatttagtgttgcttgacccagacgacccaccttatcaagttattttcgatgaaggcaaatttgaactatctaatgattatttaaggttagtttatgatcttagtgaagaacatatgggctgcgaaattatcggtaacattcacgataatccggaattattggaggaagacaaatgaagatctattgttatttcgttccgaagtatacttttgtagctgagcatcgtgtttttaaggtaggcgaggaatacccagtttacatccgagaagattattttacgttggttgctgaaaatggcgagtttaacctaagcaaaaaagcccttgacgagaccgttaaaaattggaaggaccaagttaaagtcaaaatggaagcatacaaatgagtgaccgtccaattgtcgattagtttttgttggaggaatgaaattagaaccacaaggcttatgaaagcttgccaattagctgttaaatgtgcacaataagtatatgtaatattatttgattagaggaattttatatgacgtatgtgataacaaagcaagggaaagttcacaaactgaaagaatttcgcagcattcaagcagttttgaaagcagaaactggtttgccaatcaaaacctggatggttgaaaaatctgttcagcatcatcaaaccatctgtggatggacaatttctgaaataaacgcaaagaaatccgttaataattagtttctccttatcgtcaatgtctaactgtaagtaaaccaagtttaaaggcggtgaaaaaatgggaaatgaaaacttagtaaaagcgattgctaagagccggaattttgaaaacggcattaaccggattcattattcaattcattgttcaaaagacgatgcttttagtctattaattgagcaagtattaagacgaattcatttttggaattctaacaatgctaataccttgattaaggcattcagcgatcatagcaatccagattttaagaataagcaatgggcaattacctatgctgctaaagatgtggttgaagattattatggtcacaagacgttattggtagagaattttgataaatctgatgaacttggacaattggcgcctataaattgtaaaagttcagtgtcagttgagaattcattagtgaataaagttatttcattattcccgacggataaaaccaaactgtttgtaaaaagcctgcttaaatatggaaaaatagctacaatggatattttttcaatgaccgataaaaagtttgaacatgcattgtatgatcgtatagcttacgttaaatcaaatgcacaaatgtttacggaacagttaagtggtttcgatcatcaggatacgttagataagctaaaggtattaggtgattttgaatattgccttaataaatacgccgatccaatgacgttaaacagcgaagttcacaccttatttatcagcaatagcgacttgttcaatgatatattcgattacgcaactaaagtatatggaatgaaataccaaggcattgtttggaaatcgtttggtttaattaatgatcatcaattgaaactggatgaatacaaattaattgattcaatcattgatttacagcaggaattaagtaaacagttcgtaccgaaagaaggacaggtgagcttatatgaagctacatatctgtcatgaggttggctgtcaagcattgataccaatggggcaaaggtattgcagtgagcacgttacacagcaccagaagcccaaccatgcagtcagttctgcacgaaaccgagagtacaatatgtactatcgtgatcaaacagcgaatcagttttatcactcaaaggaatggaaaaagattcggcaatttgttgctgcacgagattattatttagatgcagtcactggtttgccggtctcaaacgataagattattgttgaccacatcgtccctagacgtgtactaccagttgataaatggttagacatggataacttatggtgcttgtcaccgactacgcataatacgaaaaccaagattgaacaatcactcaatcaaaaccaactcaaacactgcagcaaacgttggtggattaaagtattatctgaacgcacgaaataaacatccctgatgtaggaaactcctgccagcttggatggtaataatttcaggggtgggtaccgtttcttggatggtggggatcttcatcaacaaaactaaaaaaagatgtcttcgtgaaacgacaaagtgtttttcaggtggtatcatgtaggtaatcggaataaatatttctgatgaggtttacttattaaaaacaattttttcaacctcctctgggtgatatagatataaagaaaaaattgtttaaagcttactgtttgaatcttacaaaaaaatatacaatttaggtgaatgtttaaacacccccggggtggtgaaagcctaggggagcgcacgcccaggagtagcgcacgttaaaagttgtaaattcaaaacttttttatgggcttactataactgggtgcacgcaatttcacaaattgcttatatgaataaccctactataacgactatgtatatttccctcctaaaagttaatataattagacgttttttcacgattgtagggtgtatacgttcgaacagtgtgtttaatgatttttttgtgattcattagtctaaatgaatcagattgaaagagtccctattgggggctcttttttattgcttggaggtgaactaaaaaatgccaaaacaaatgaaactaactacagacaagcatgctcgcaaggatcagcgagttagaactcaaaaactaataacggaaacttctggaatggatttgattcaaaagagttgtccaaaatatctgtcaagttatgcgcgagcaatgtggacgaaacttgtaccaattttgcaagcatcaggatatgttaaacaggccgacaagggaacaattgaagcgttttgtattaactatcaattattgcggaaaggctatgactcaattaaaacagatggtgttgtcaccaaagtttctaaaactgtggtcaatcaacgaactggagaaacatatgaagacaacgcaggctggaaacgtaatccggcatcacaaattattgattctgctacggcaaaattaaacagcttagcacacgaattaggcttaacaccatctgcacgagcctcattactgcaactctcagatgacaacgatgaggaacccaatattaaagagatgttaaatgggggaagtgagttttagtggtacaggaatttgattttactcaaagaaatactaacttggataaaatatttcagcagcttgatgggaaaggctactttgatgaaatcaaaagtaaataccgtgatccggccactgtttattgctaccgggtattaactggtcaacagttagcctgcaaaacaattaaactagcagcgtttagacatttgaatgatttaaagcgatccacggaaggtaattttccgtattactatgatttggataaatgccgaaatatctgtaacttcgcacgcatgtgccctgatgtttctcaaaacaagccgataccactgatgatttggcaacaagcaatcttgtgcctttctcagggatggcgaacaaaggaagacaagcagaagcgatttgagcgatgtatggtttcagtggctcggactaatggtaagtcatatctattgaatatcttgatcctttacgcttacttggtcgaggccagtgaccagtttaacgccgatttatgttacttggcgccggttgataaacagtctaagaagtcttggcgttacattaaacagacttttaatagtttacagtcaatgcctggatttcgtaaattaatcaaggatcagaatattgcgattaatgatgatgttttgaaatccacgaagactcaaaatcagatattacgaatgacagctggtagtgcacaattagatgcctttcatttcctctttgctactgtggatgaatacggggatgaaaactttaattcagatgtgatttctaaggtcacttctggacaagttcaaaccagtaaccgacaaacattttttatcagtacggcatacagtaaccctaaagtcccgatgtatagtgatgttagacgactcactaaggtgatggaaaaagattctaaccgaacggaagattcaacgttggcattaatttggcagcaggatgatcaagatgaagttgagaaccccgaaacatgggtgaaaagtaatccattactagatttaccggctaagcatgataccctactgaaagggttaattagtgaacgtgattctaagctggaagacggtacgctaaatgatttcattaaccgtaacctcaatatgtggttgcagactgctaaagataaatatttgaaattagaggatatacaaaagtcagttgtttctgatttcgaaattgataatcaagattgctatgtgggttttgatttatcacatgcttcagatgatacggcttatagttttgttttcccacatttgaatggcgaacaaaagaaatatttcatcttgcagcattcatttgttccgttagcccgagcagataattccattattgtgaaagaaaaacaagatggaattaattactcaaacgcagaaaagttaggcttttgtgatatttcgcaaaattcttatggcttaattgatgaagattttgttgggcgctggttcctggactttgttaacgatcatcatttgagagtcaaagcgtttatttatgatccttatcaagctagcgcaattactgattggttggataataatatgccagaagtgccttttattactttaaagcaagggacggttagtttgagctcgcccacagtatttttgagaaatcagtttattgctggaaatattgaaatgttagctgatccgattttgcagacctgcttggctaacgctgtaacagtggctaatccatatggtattaaaattgatcgaacggcgttgacttcgaaaattgattgtgccgatgccactatcgatgccatgtctcaagcccttttttattttgaaaatcctaatcatggccttaaagaagataaaaagaatccatttaatggaatgagtaatgaggaggtcaacgaattctttaccagtgatcattttagtttttaatattttcaacacttgttgggtgatatatgtagtgaataaattattagggaggcagattagttgaatctgaaacaactatgggcaggtttaatcactaacctgtcttttatattatttttatttgggttaattgcatttgtgattgccgcaagcctaattaattttattgtaggttgggtagttgccgcgattgctttaatcgttttagcctatgtcatttcgtgaaaggaggcgttgaatgctgaacccctttaaaaattttatgtcaaaacaaacacaaacaattagtaccaccgggtattcaccatttatgttaaatggtacattgttatccactaacactgtggatgcagacggagcactgcaaaacagtgatatttatgcggtgattaatcgaattgcaggtgatgtggccagctgtgaatttaaaacagaccaatatagcaacatgctaaatcagcccagcacattattgagtgcttataatttttggcaagcagttagtgctcaaatgatgttaactggcaacgcctttgctctaattcagcgaaatggaaatggaagtccagcagggttgaccttaatcccgttttaccaggtcagcattactttagataatcaacaaaatgttctttattacacagttaattacggtgatgaccgagggcaggtgacatatttagctgccgacgttttacatttccgcttgtttgtttccggacaagttgccactgaattggttggtagcagtccgctaaacagtttagctaaagaaattaacatccagaactatagtaatcaattgtcactgagcagtttaaagaatgcaattgcgcctagttatacgattacggttccggcggccaaattggaaccggaagctaaagaaaatattagaaaatcgtttgagaatcagaattctggttcgaatgctggtcgaccaattgttttggatcaatctgctcagcttgattccttacagattaatccggatatagctaaattattaaataatgcaacatttagtcagacccagattgccaaagccttttgtgttccagatagttatttaaacggtcaaggcgatgaacaatcatcaattgagatgattcgttctctgtatcaaaatagtttgagcctatatattcggccaattgaatcagaattgtctttaaagttgggaatcgacattaaaatggatattaattcggctattgatgttgatcatcagcaattaattagtaatattactaaattaagtactggtcagtcaccagcattaacgccgcaacaagcgcaaacaattctgaaacaagcgggagtttttcctgatctaaaagtctcagcagtggaaggaggtgatgataatgacaacagtaccaattaaaggtgttgtatctagtgatgatgatgctgaagtatatgaattctttggctattcaacagttactccttccgcagttaaagatgcgttaaacactgcaaatggtcaaaatattgttgccgaaattaattcacctggtggcgatgtgtttgctggttctgagatatataccacacttaagaattataccggtaatgtggaagttgacattgttggattagcagcgagtgcggccagtgtcattgcaatggctggtgatacgattaaaatttcgccaacggctcaattaatgattcatcgggcttccactgtatctcaagggaatgcagatgatttatccagcgatttacaaggcttgaactcgactgatcaatcaattgcaaatgtttatgtgcaacgaacgggtttggatccgcaaacagtcatgcaaatgatggccaaggaaacttatatcaatgcaaaagatgccgttgaacagggatttgcagacgaaatgatgtttgacgatcaaccagccaaagttactaatatgctctcgccggttatgttgagtaatcaggcaattagtaaaattaaatcattgttaaccaaagtaaaagaaaagcctaaagaaactaatagccaaactagtgaccaattacgatcacataagttggctattttatttaagaaagaaggaaattaaattatggatttaaataagctgcacgatgcttggcttgaagctggtcaaaaagtaacggaccttcaagaaaagcgtaatcaaatggcagttgaactgaacgattctcctgaaaaatattcagatgaggatctaactaaaattgctgattcaattgataaagcaaagaagacccgagattttgctaaaggtgcatatgatgatgccctggcaactgctaaattagtaaagcctgataaaccagctgcaggtggtcaaaaagatgttacgccaaaagacaagcctaagtttattaatattgtcaagggagccttaaagggtgatccaaagtttttgaatttgatgtctagtggacttgatgtcaatggaaacggtgttggcttgacaattccaaaagatgtccaaacggccatcaacactttaaagcaaacctttacgtcgctggagccattagtaactgtggaaggagttagcgcaccatctggttcacgagttattgaaccacgtcagtcggtgaccccatttgccaacttggatgatgaaacagcccaaattgggaataatgatgatccggcatctttcaaaccattaacttataaaattcatcgctatgctggtatttctagcattacaaatactttgatgaatgatagtgatgccaacctcttagcatatttggaaaattggattgctaagaaggatgttattactcgaaacagtgaaattttaaaagcgttggctaaattgccaaccacgcaaaagaccacagttgatagctttgacgccattaaggatatttacaacaaggaattggatccactgatttggaatgaatctgcatttgttactaaccaatcaggctttgctgttctggataaagtcaaggataataacggacaatacgtcattcaacctaacccgcttaatccatcacaaaaaatgttggctggtaagacaattacagttattgccgatgcctttctgcccaatgatggaaacagtttcccactttacattggtgctttgacggaagctgttcgtctattcgaccttcagcagatgtctttgttggccaccaacattggcgccggttctttcgaaaatgacttgactaagattcgtgccattgatcgctttgacgtcgagttgtgggatactgaatcggtcatttatgcaccatttaccggattagcagatttaactcctgctgcaaagactagtgggactactagttcaactggcaagtaattgaaataagtcgccaatgaaataaacaatacagtgatgggcggctgttaggaggggtgtcatgtgacggttaatccgacagaattaatggatgagttgcatattgaccaaagtccgactgaattaacgactgttaccaatttgattaatgaggcaactgagattgtcaatcattcagtcagttcaactgaaacccaatatcaagcctcatcaatttacgacctagcaataaaaacactggcaactcaattatattatgatcgaggattatctaaggggatgtcggctggtttgttgatgatgctagatcaactccaaggaatggtttcaggaagtgatccggatggcacttaataaatttagtccggagcagtttaatcggcaggcccagtttggaacggctttaccaacaattaatcctaatactggtgcatcaggaacgcaatttaaaccacagttcgtgttatggtgcatgccttatacgcgaactaacacacagaacgtttcgcttttgggaacggattttgaagatactattcaaattgttattcgacacaatccgttaattgacaaaggtctgctagttcaatatcaagaccaactgtatcaaatcgttaatttgagtttagatgatagcaataaaattgtgacttatgacattttgactctacagattaatgagagggttggtaaaaaacatggttagtatggccgaacaattagacgattatttagcgaaaataaagcgattggtacccaaccgggcggaaagaactataatcactaaagccggtgccgatgttttacaaaagaaattggctaataaaactaagcagctacattacactaatcgaattgcctcagaaaaggatccacatttagctgatagtgtgctagttagtatgacaaacgttgatggtgatgtggatgggacttccacagttggttgggtaaagaaaaaagcggtgattgcccgctggttaaatgatggtactgtttatatcactggggatcactttgtagaaaaggcacgtgaagaagcccactctgatatattaaaagctgaatatattaaatggaaggagttggggcactgatggagttaccagttatgactgtttatcatttagttcagtctttgcactatggttggattgaccagctttattccatgaacattcctcctggggctgatacttctggaaagcagaccattgtattagttacttcagttactgaaccgttgggcggatttcgcaacgatcaatttagtaatttacaggctaacattcagattcaaatattttggaaaaaaaaaacacaagaaaatatttttaacaatgaagttgccctaatgaatgatttggaaaatcaggattggctggttagctcacatgagcctaccactgtggatccagacaccgatcaagttacggcaactttttcagttactaaaacaattatagtaaagaaagaaggactttaaatgtcaacacatggtattaaagatgtcacctttggtttggttgatgctaatggtaaattactgactagcgatgcaggagtaggaactaatggtatctatttagtcgatggtgacgaagaaggtgctacgacggccacagtttctggcttggaagccgagggtactgtcgcctatgctaatgatgaagcaaaacgagtttcaaatggtcaggcacaaccacaggtcgcattggaattcttggatattgattttgacgagttgcaaaaactcaaaggatatattcatgatgcggctaatggtggttggacacgtcaattgccaaagccccatgtagcaatgttgttacattttcgttcatacacgaatattgatatgtacgaaggctttgctaatggtcaactaattgaaactggtagttctcatgcaacggataataatgctgaaactgatgccaatacggcgttaacttaccaagcattaacaccagctgacaatacaatcttcaacggagaaccgtacaagatttggatgtctcaagatactggatttgataaagctaaaatgttggccgaagtctttggtggttattcagctactaccggtagtagcacgactggttcaaccactggatcgactacgggtagcacaactggctcaacgactggcggtacaacaccaggaaaataaattaaggcggggattgttccccgtatacataactaaataaaataaaggagttttgatcatgaaaattaatattactcgattaggtttacgcaaaaagtcagctgaagttaaaaccactgtgggtgttattgagaaagcccaaaatttacaaattcaattgttgaaatcagatgcagttgattttactaatgatgacccactagcagttttggaaacgcaaaagaaaatggttcaaggattattgcaatttatgattgatatttttaagctatccgacaaagaagttgaaaagattaaatccactttggattttacggattttcaaaatttcatggcctatgtattattccggtttcaaggtatgagtgatgaagattgggagactgttactaaacaacaaactgaggaatcagcagacccaaaagaaagcaattaagattagccaaattaattaatgacctaagcatatcccaacaagatatgcttttttttaaacaacaaatgatgaaacagggaatcttaccagatgaattaaatcgacaagattactttgaatttatggcagtcttaaatgctaaagataagaaaaaacaagtaacggatccggttgtcgagttattaaataaacgaaaggggactgactaatggctactattaatgatgtaatgagtacttcaattcgcttggatgcagtacaaccagcacggtcattaaagactttaaccaattacattaaagctaataccaatgcatggcgttctcaggaggtggccttaaaatcttctggagataaactagatgctttaaaaactaggtatcaaggaatatcagaagaaatcaaaggttataacttaaaaattgatgagttgaagcgtcgacagtcaggcctcgatcaaacgaccaatcaaggttcagaaaaatatgccaaatatgctaatcagattgctaaagcacaagagaagattgctggattaaatgatcaacagtctaaggcggaaaagcaatttgaataccttaattcaggactatctggattgcagcgtaactatcataaccttaatcaggtaactaattcttatgtggatgcgctaaaggctcaaggaaagattaaccaggctggtcaagtaaagcttaaaggccttaaggaaggattgaatagcttatctgatcagtacagattacaaaatagtgaactcagtaaaaactcacaggcttataaacaagcccagttggcctatgaaaaacaacaaaatgttgttaaccgcctcgccaatgatacccacaagaatgcggatgaatatgttcaagaaaaggaaaaacttaatcaattaaaaggtagcttggacattgctaacgaagcttttaacacccaacaagtacgagtcaacaaaacagccacttcactggccaatgtgcgttctgatgtggtcaagtacgatttacaagtcggtcacatgagtgatgcaatggtgcgattgggcgataaagctaacattgctaagaataaatttaaaaattcatttggatcaattaaaggtagtttactaggtgccagcgtagcgatggggacattgggagcagcagctttttctggcgctaaaaaagcaactgaacttcaaaatgtttataaagtaaaccggaacttgttagttacgggtggtgataagactaaagctgccattaagaccgtgacagaaatgcaaaaagatgggactaagtacgctctcaaatatggagttagtcaaaaagaaattgctgatcaataccaggatttaatcaagcgtggtcatacaggagctgagtcgttagcggttatgaaaactgagctacaggccagtgtggcttcaggtgacgactttaaagatgtggttaaagtatcaagccaggcgattgaagcatttggcatgaaaaccaataatacggcaaaaatgatgcacaacactaaacgtgtagttaatgcattagcttattctgctgacatgactgctactgacttccaaagtttaggcaaaggtatggagtatgtaggtgattcagctaataatgcgggctttagtatcgagcaaacttccgctgctttaggtgaattaagtaaccacggtttggaagctgataaagccggaacgggtctacgaaaaattattactagtttagcagcaccaactaattcagctatgggtgctttgaatgacattgggattaaatcaactaaaatattccaaactgccaatggtaatttcaaaacgttgcctgcaatttttaaaattattgaggaacatactaaaaaacttggtggagctgatacagcacgcatatttaaaaatatttttggtccaaccggcatgcaagcagctcaaatcttagctaaatataatggccaattggctgatttaaccaacaatgtttctaaagcaagcaaagctgggacttacgttcaaagattagctaacaaaaatgctcaaactgcccaaatgtctcagaaacgatttaagcaagcctgggatcaattatcaattatgtttgggtctaagttattgccgtatatgacaaaagcagctaatcaaatgaccaagctttttggtgaaaaaggatttcagaaagatattggtaaaacggctactttaactgcacatgtggcagaaggaattgccaatattggtatttttgctgttaagcattatgaaggcgtcaaacattttggtgaagcattagctgcaatttgggcagttggtaaagtttataaatattttaaaatatttagtgatattacctctgtctttggcggtcaaaagctaaaggtgaaccgattgacatcagcatatgatgatcaaactttagctattgaacgtaacactaaggctaaagaagctaatgtggatgccggaaatggtaccagtgcaattgatgatattgctgataactctggtggcgaaggtaaggttgccgaagataccgggagggtaggccgattcgctaaattagctgaaaagtttaaaggtgttagcaaattcggaaaggttgttgcaggctctgtaggtgtcttagacgtcttaaattctgcaactgatttaattggcatgaaaaagaagactgccggttcacacattggcgctgctactggttcactaggtggtacagtagctggtgcagcaatcgggacagctatttttcctggaattggtacagctgtcggagctggcttaggtggactagtgggcgaaggcgttggtcgtaagtttggtaaagctatccaaaaaggactatcggctcaaaaaattcatgtaccaaaactatctgccaaatcttctttcaagaaactttctgatgaagcgacaagctattataaaaaccgtgaagctcaggacaagaagaacttacaattactttataaaaacggggacattactaaaaaagagtacgaaaaacgcctgcaaattattaaagatgaaggatctaaagccaaccgattaactctgatgagtcaaaaggatcagcaggcaattgccaaatattatgcgcaatcacggcaacgactaacggaatcatggaatgaaaagattttaaaagctgagaataaatatggtaaaggatccgttcaagttgaaaaaatgcagaaggaaaagaaagaagcacttgagaaacaacatcttaagtttgctactcaagtgactgctaaagaagccaaactgcatacaaccttagctggtcagattaaactgtctactaataagattgctaaagattataaaacgctcactgaaaagagtaaaaaatattccaaagaaaaaatgattaaattggtggcaaacgctgatgaagaacaaaagtctgtcagcaaaaaagctaacgatgaatatcatagtgtctataacgctgcttggaagaaatataaaaatacagttaaagcagcggatgaagagtataagggaaatagttcagctgccaaagcccaacgtcaaaagattattgaagaagctcgtaaacaaagaattggtgttattaatcacgctgataagcaaaaaaatgattcaatcaccaaagcaaagcagcagtctgataaggtgtacgattatgcacataatcaaaatcgtaaagtaacggctcaggctgtttctcagtatgagaatattaagaaaaacaattccaaaactaaagataattacagtctttcctggcatggaatttggaagtcagttggtaattggattggcaaactggtaaatgggatgaataagaatgccatttcagcccagaacaaagtctttaaacaatacggtggttcacaaaccctagatcagattccaacggtagcctgggcaacaggtaccggattattgaaaaatggtttattaacccaaccggttttggctaagcttaatgatggtcacgattcaccagaaacacataataaagaaatcattgtccacgcagatgggcaattagaaccagttgaaggtaaagatactcaccggttcctagaagctggttccggcgttttaaatgctacagagtctaagatgttaatggctttaaatggcatgcagcactttgcgtcaggtactggtttatttggtggtatcgggaaactctttaaaggcatttggggttctttaaaacagaagttgtcggcactatcacacattgctaatcattctgatgcaactttcaaacaagtttttcaacctaattttggcgatataaagggaacagttggagagaactttgccaatatgtttggcaaacgcgacaagcaacagggttcggtttggtgggatactgcctggaatatgctacatggcatggtttccgaaggcggcggtcagactgattcagcatttttgaatgaagctaagaaattggcaaatcgtgcccatcaccgatattctgaaggctctaatgtccgcttaggaccgaattattatgattgttctggcttagtttatgagactttgaaacacatgggaattacagttcctggtggctcgactactgtccctgaatacaacttttctaagcctgtatcttggaagaatgcgaagactggtgatttagcgttcttcggtcgtggaggaagccaacacgttggtattgtggttgataatagtggctccgggcatatgttcagtgccgaaaatccaaaggacgggattaaatattctaccatcaagggattcggtgattttgttgggatccgaagagtacctggattaattgacaaagttaaaaagtcaactaaatctcataaacaaagctccggattacaagcactagtaaagtcacaattaaagaattctggagtttggggttgggtatcaaaaaacttaaaaccattatggcaaaaactgtttggtagtttaagtagttttggattaagtggcgacgtggcggctagagccaaaaccttagcaaaagcattgaaaaaactagatccacgcgcaaccaaggcaggaattgctgcaatccttggcaattgggaatttgagtcgggattaaatcctaatgcaagagattcatctggtggagcctccggtcttggacagtggttggatggtagattgaatcatttgaagtcatatgctcgacgtcatggtgaaaactggcaaaatgcggctacccaattaaagtttgcgttaagcgatgacagttctgattcttctgtatttaaacgaatcctggaaggccacggttcgatcgcttcgttagccagtcagttttctgaagattgggaacgtggcggttatacgggacagcatgttaatggtgcgaagaaagttgctaattatttaggatatgcgaatggtggcttagttgatcaagaacagttaattaaagtggccgaacgtaataaaccagaaaccatcattccgtgggatattaacaaacggggacgagcctatgaattgttagccgatactatggctcattttaagcaaacagatcagcataccaaccaatcaagcaattcggatggtcaggctgtcaaaagacttgaagcaaagtttgatacaatgattaaacttatgagtcaattggtagatggccaaaacaatccgattccggcagtagtgactgacaagcaagttgttcaggcagtcaataagcataacaaacgaacaacggctaagaataattggggaagaggcgtaacctttggctaacaatgataattatgatgtgaacacgtttgattttgcatttgatgaaaatggaaatgatggctttaattcacaagatgatttaggaatctttttgaatcatgtatcgaaaccgttagcacctagcattactgagtcatttcaagacgtccctaaacgttatggtggtgtttacttgggaacagattacggtgaaaaggaatttgacattccaattacctgtttctgtactactcgtgacgaatataatgagcgcattaaaacattgactaatgttttagttaatatcagcagtgatgctgatactgaatatccgttaaggtttaatgacgatccagatgtaacttattatggtcacttcacaagtattccaacaccgacatttattaacgagggtgttcaggattttcaaactacgttagtcttcatgttggcggatccacgtggatttctaccacaaaaagaaataaaaattacggacaatgatcagcaaattattcctgaaggaaatactgaagttgatccaattattcatattattccgaaaaccgatctttattatgtgggttatgaaacaaatgatgattatgtagcggttggatataacgttgatgatggtgatacggctacggatagtgatggtaacattacagtcatgggacaatcccaaactcaacaggttgacgacccatgtaactcattagcaacgtggattcaatgtagtgaaaatacgcaagcctttccaatttataagggtgagttagatggaaactcagcagccactggtacttcaattatggtggctaaagataaagatgatcattacgaatggggatctcgtgggaagcacaagaatttttacggaccagcggttatgcataatggtctaccgaaaattactccctattggaaagtttcggtgcgtttgcatcatgttaaacgaatgaaaaatgagcgggcaatgggaaaaattgaagcttatttattggataataacggtaatgtttgtggccggatggggattgaagattattcaatgggccgttacccacgggcgtttattcaattaggtaataattttgatagtagtaactctgatagttatttgacattgctatttgatgaaggtaatggacaacagaagcaaaacgaggctacaaaacatgttaaagtagcatacaccaaaacggtcaccgttaagaagaagacagccaaaaagaagaagacgactaaaaagaagaagtgatataaatgaatctacaattctttgcgcgaaagaaacgaaaaactcgtaagaaggctaagactaaaaagaaacgagttgtaaaagccaaaaagggtggcaagaaaagtagtagcaaagggggcaaaaagacatcagctcccaaagctacaacgaaaaagaaaaaggaaaaagaatatgtaactgaaacttcgtatatgaatagggatgcttactcgaatttttatggtgaatttattcttgaacgacagaagaaatcggatagttcggggaatgtttacgataactgggtagcagaaattaaccagtgggatcctaaaactggtgaaccatatagtgttaataatacctataaaactcatatgcataaggaaaaattggataagtccggtaagtttggcttcgccttggcaaatttaggcgttttctttggcaaacatgatattaaagaggacttggttaatccggtggtggcgtataagtcagattatgaagctttaaccaattatgaagaatggcgcagtgatggctctactgatccagatgatacgccacatattattgccaaggctggtcaagaaattattattgatacagccaataataaagttactattgatggaaagccggccgataaatacgtttcatggttatcgaccttccctaaattaactggtggagttccacaaactctacactttttcccggatcccaaaaatgctgatgtaacaattgaatatcgaccagcaattaagtagtcacgaaagcgactactttttttatacataaataaggaggttagagatttgtatattatcctggataaaaatttaaagcgagttgccacgttatcgactaattcagacgccaacccgttttggggtgaggtagttgaacgccaaattgccgatgataacagtaactcggatgatggcattactggcgttagcacttttaatagtacggatccgaatgctaactccaaaagctggaatgatacattaacaggactaaccatgttacaaagtgcccctgcggctcaatacttaacggttggtaatagtgttgctgtgtatgatgatgtgcataatcattggcgtatttatcgaatttatcaggttgatgaaactattgatgccactagtggggctcacttagtaacggtggatgctattaacctagcaatctataaacttaataagaccattccaccacaaaaagaaattaaagattgtaaattagatcaagccatgcagtggatcatggctgataccggttgggatttacaaaataattgctcttcaggattatttgccgatattagctttgatggtacggcttctagtcaagcagccttgcagacggttctatcaacttacgatgcggaagctgatgcttattgccatattgacactaatggtattgtgactgacctgattttagaattagctgatcaattaggtgaaaatgaggggaaatcaattacttatgggcaaaacatgttgtctgtccaacgagaaacggttgatactaatttagttaccaaactctatatcgttggagcaaataatgcttcaattgcctcggttaataacggcaagaattatattactgacgtttcagcaaactctctttataacaatgatagcaatacctggctagaagggaccatcacgagtgataccattactgaacctaaagcattacttgattggggattacgtgaattaagattgtacaatcatccacgaattaactatgccgtggaggtaactcaagattttcaagctaacttgggcgatactattaaggtgattgatttatccatgaacccaattttgacaacggaagcgcgagtcattcagcaaaccacttcggagagtgatccaagtcaaaataaagtcgtcttgggagagtttagcacagttaaagtaattacgccggcgtttatccgtaatatggaacagcgttggaatgaccatgttaagaaactatttgaagatgcccgagaaaataccaatgcagccacagttagtttgattacgccgttaggttcaacttggtataacacggatacttccaaacgggtgattgcaagactatttattgaaggtgagaatgtaacctcttatctgtcaccacaagcgtttaattggcaaaaaattaatatggatggcacccgtgatattggctgggaagctgaccatgcaaaagatggttatcaggttactatcgaaccaccatttgtcgggacactattagtcaccattgatgatacttatgtgaaagatgaggcagagatgtggattgataccagtagttcagctgatggttcctggaataagctttgggaaaccaaagatgctgccaacaaagattttaatggcgatcagcatattggggccttacaattttcatatttattgggtgatggttcagtgttgtctagttatcactacactaaagacaaaagccattctgattgtgagtttattaaatggaacaccgatggaacattgcaaagcatgatgtttgtaactggaggtggccattgtggttcttttggttatgatgaaggttccaacacaatttatacagaaataaaagatccaattgatgggaaatattatttggtaacaatggcataccaagcaaatacgagtgccagtaacataaccaagtggtgccaagtaacacaatattttcgagttgcagttgatttgaaaaataatctatggctgggaagcacgacgagtgggaaagtgtatgtttgtcagataagcgatttacagacaggaaacttcaaaccaatcattgaatttaaattgcaagattttaaatggaagccattaccagctggaaccactaataatggcgcttataacactcttcaggcaaatgggattagttatccatttgctttttttacggcgggtgatgctaacaatgctgatgacaaacatgttatgtgtattaacttaattacacagtcaatggtatttgatcatgtggtggaaccaatgcaggatattaagttaacagtgccgttggaaaatggcgggcatttggaacccgaaggtgtttatgaagatgttaataattctaggttaattgttggctttaacgtttctgaatatagggatgctgcacatactgtctctattgctcatagtgccctatatacagctccacttaaaatccgtgatgattctaaagacttagttgttgaatatcctgaacaagatgaaggtgaaaatgatgaagctgaacaaccagtaattgctggaaatgataatgcggatgattcagatgatagttctgatagtgatgaagatggggatgaatcaactggtgaaggaaccaaaattgaggatggtgataacaattgattattgcaacgggaactttaaatattgatgaaaatgctaagcttgcccaacaggcctctgacgatgccaaaaatgctgctaactctgcagctgatgaagcgggtaagattaaaacatcgttggatggaaaaattactgtttcatcgcaagagccttttgatgatgggaaaagtcatgatgaaggtgatatttggtacgtccaagacagtaaccatataactagtgaaatgtacacctatgatggatctgattgggttaagactaagatgtcccaaacagccttgtcagttggccagctttcagcgttatctgctgatttgggaactattgaagccggatatttaaactctgtggaaattgactcatcaatcattaaagccgccaaaattgatgcaacttcgacaattacaggggcatcaattgaagaagatggcagtaatggcaaaataacattagacacaaacggtttttgcgccattagcaatgggaaatatcttcaatttgtatctggaaatagtaatggatatactcaaatccgtggtggcttggatgttgattcaattaatgttggagcttcagttattgaaggacagacttttcaagcatatggcggtaataatactcatattggtagtgcagatgcttggacgtatttagcagaaggaattaaatgtggtccccaaggttatatttcatcagtttcaggaactgatatctattttcataatgaagctggatcgacaattgatattcatgctggtgacgtcatttcacatggaactaatttacttgatgaaattaatgggattaaaaagaaattgaagatgtaaggtgatctgatgaatgatattaacgcacaagatttaattaaccaattggttaatgagtacagtcaagatatggcagcaaaaaatcaacaaattgcgttattaaaaattgaaaataatcagcttagaaagaaggtgaaaactaatgagtaaggagctcgcattcacggatgataatgatgtggttaaatatttagatacaaccactgcttttaatctggcactcacggccgacggggtagcctttgatttaactaatgctaagtcaattttggtaaaaatagctaacgatgatggctatatcatgcaacaaactattgatttaaccactgtaactagtccgcttggtggaacactaagctttccaattaatcaggatattatgaacacattggttccggatgattatgatattgaagtttgggttactatgagtgatggtacgcaggctattttcccaagtgatgggacattagggttctcaattgaagagaacttaatgagtgatactggtgaggtgatcccgacaatcactttgaatgattttcagcaacaatttgatgatttaagcagtcaaatggcgaatgcggttcaaaatgttaagaaaggtgaccaaggtaaccctggtaatggtattaagtctgccaacaatcagtatcagttaagtgattcaccagttacagttcccacagggggctggtcagatactattttggcaacaactgatcaacttcctcatctgtggactaaaattatttttacctacgatgacgggacaactaaagaaactaattttgtttccagccgaggtgataccggtagtcaggggccaattggaccagtgggaccacaaggaaaacaaggaaatggtttggttgttagggggaaagctgataaagaggaaaatttacccacaacgggtaacaaccagggtgatggttacttagttggaacagacttatatatctggatagatggttcatggcaaaatatggggagtattacgcctgatttagctgattatgtaaaagtggctgatatgaacaatgctttaaacactaaagttaatgttactgacatgcgcaagcctgctagtgatgtagctgggattgaagaagttaacgccaaacaagataaaattggctacacgccggctgacgattctaaagtagcccacctatctggtgctaacaactttgataccgtcccaactgttaaaaataatccgttattacttgcaagcagtttaccatctgacctagcacgaacaggtcaagatcaggagtttacaggtaaaaataaatttgatacagcacccattgacaagacaactggtcatccgtatatcactaaagacggtgtgccagcagttcctgatactttggcggacaccactaaagatactaacttcaccagaaaacttcaaaagtctgggattgacgtggcaaccacaacggacgttaaaaatgctgttaataccgcaacggctaacatggtagataccacaaaaccagccaactttaccgcaggtttgcagaaaggaggtatcgatgtcgccacggcggctgacttaaaaagcgttgaagacagcgcttggcgtcagctagatataacagagactaacaacgttaactctgggaaatcattattactatgcaaaataaatgtatctacgaacgactgcttgatagcaggatacattaatatgtattattcctccagaattgccaatattacggccgttataccctctgattataagtttagaagtattggagatttacctaccaatctaaatgctggattatcaattgatgttaactctagcggacagttatctatcaattacaattctatacgaggtgggggtaagcctatctattggtcgatagccggtccagatgcaacagcattacaggcgactgttactccaatgtcttagaatagaaaggacgattacatgtttatttatgtaacgtataacaaagatggtttcatcacggcgtaccagaataccgaggcagatgggtttaccaaggtgttcattcttgattcatggattacccagtttgctcaatacccagataagtttagatatgatttaactaatcaaaaattgcttaatccaggtaacttaccgagtgtttcattgaaccaagtaagtacagatgtaacaactttacaaactcaattacaatctttgcaatcaacaggtacgcaaactgattcacaattgggagctttggtaagtaacatttcagtggttcaaggacaaattctcgtagaactacaaaatattcaaactcaattaaatgcttctgaaaaagcaactactgtaccagcagcaaatacaactaattcaccagcttaataaaaggaggtaatacaatgtttaatattgattggcacggaatgcttaaaattgaatatgataacggttggttatcttatgataaattgaaactgttcgttggttggaatgaattaacaaaagatcagtttactgatattactggtaagaattatgacacaggggtggaaaattcatcaactgcttcttaattgacggtcagttgagtacactcacatgtagacgttttttggaatgcaagtttaattaaattaaagtccgtcacttttttgaaacagtggtataatcattttcgtaggcattaacccctttggtgcctacgcattcgaatattcatctgagcatttatgaatgccccatgctcatacattcccctcaatgtatgtgatgtatacacgcccgtcataagatgggcgtgtttgtttttaataattagttgttacgactaaataatcgtgatacaatgcgtttgtggaattccattcctccaagaaggaatttcatgttcttcaatatgatatgaattgaggacgccctttaaagcggggcgttttcttttacacaaattttatggaggttgtcttatgtatacacaaatattaaatgttttaaattcctttaaagcaaccggattggttgcttttttaattgctgtaattccagcaacttacaaattggttaaaccgttgattgaagctaaaattaaaactgaaaagaatactcatatcaagcaagggatggaattaggcttgaaattagcgaatgctttcgttcctgtggtggcaagtatgcctgctttaagtaactcagatcgcaaaaaggcggttaaccaatttattgattccaatttaaaaaattccggctttaattttaaagcagaaacaattgaaggattagcagaacaagcttaccagtattataaacacactctaaagggagataatcacaaagcacctgttactccggcgcctaccaatgacgttacacccgacgttccagtcgatgacgatccggaagtatttaacgaaccccaatcatctgaacaaaagtaggaagtgacgaaaatgacaaaaaaggttgctgatttatcagtatttcaaggaagctccgagtcttatatgaagtcactgaaaagtcacggaattgataccacggtggttaaattgacggaaggcactggatacattaaccctaaagctagagaacaagtggctaacggattcaaagtatttggtactgtgagtgtttatcatttctttcatggtcatggttcatcagaagctaagtatttcttagcttgggtaaaaagctttgggttggataaatccacagtcttggccctagatgtggaagcacaagaccttccttggaagaccacagctgaagtaaatgcctttttaaaggagttaaaagccaacggatttaccaacgttattacttatggatccggttcatggtttgctgaaaagcgaattgatcgagcgaaacttattgataagcatatttgggtagcggcgtatggtgttagtcaaccgggaattgataatgcgaatgcctggcaatataccgataactatgatggattaaaggttgacgccagcttagattttgatggttcactgtccggaagtggggtagttattaaacctgctaaaccggaatattatcaaactccaggcctatacgaagcaacacaaagcgtaattcaccaatttaacgatgctgaattcaagtctaaacggcatactcgtctgattaaaggaagtcgattctatgctaccccaataaaatatggtgaaatttatcgcctttctacaccaaccggttactatacagcaaacaaagataaagttaaatttatttttgcagtaaaggctggtgataaataatggtgggagttcctgatgaaatcaatatgactaaaatgctcattggcattaaagaagatatttcttccattaaacaacagctgaatgatcaggctgatttgaatgctaaaacagataaagctttggctaagtctattgaaaatgaacatcgaattgataaccttacacatattaactatgcattaatttctttagtggcaacgggaattattgtaccgttgattatttatttaattgagagatttatgtgagataaatcccccttggataattattttttttggggggggaatacatatattggtatatattaattaatattattttgtgcttttgataatattatgcatatattagcttttggttattgaactatcatttttgaggacaaaatagctaataacgggcaaataacggccaattaaaattataaatgcctttatatcaacgtttgtaagggacacttgtgcctgcagtcggcataacatttcgtaaaaatagggaaaccaacgaatgacaatttgttgggttccctatttttgtattcctgcttgtaatatctccatgaaacaccatcataaagttcgcggacgatgtcagacgagaattggtatacaagaaatatcatagattggtatatgataataatattttgaaatagcccgacgtaacggtacccgattggataatcaggaaaaattgggcttgtggtatacgttgttttgcgttatgctgtactggtaaatacaaattgtttgggagtgaacaaaatgaaaaaagtattattaatttgcgagagtggaatttccagcaactttctcgctaaatcggctaggccctttattgaactgtatgatgcaaagattgaactgattccaactaacattgacaatgcggacacatatttgggtgatccaattgacttagtgctcgttgctcctcaagccagttatcacaaaaaagaacttgaattgtttgaccgcgcaacgcaaattaaaacaattcctgacgagatttatggttgggcaaacggtgagaaactcgttaagttcatcatggcccaattatctccgattggggccgcttaagatgactgatgagcagttaaacgggatcgccatgaaaatgctgacttattctggcaaagcaaagagcatcttatcggacttgatggatcatctcaactcatcaagtcatgatagtgatattgatgcccaattaaacgaagctcatcagtggttggtccaggcacatcagcaacaaaatttggtgattgccgaagctgagacagttggatactcattgctcttcacacatgcgcaagatacccttatgaatacagaaacaattgaatttgtgattagaaagtctatcgctgcatttacaaatcattcataagttcaatccggcatccggttattaatttgatactacttacgaaataggtcttgcctaattttgctgtgtatataacttgtcgtgacctccgattctgttgaattaaaattcaatctggcctataatggtctgtatgatttattcttgtaatgaacttcaggagtaatttaaaatcaaaaatctaatctgattaacttgttttgttaataagattagatttattttttggagggtatcacatgcaacaacaagatcaaacagaccaggaacgtcgcgcagatgcctctttctttggccagcctcggggactctcaaccctgttcttcacggaaatgtgggaacggttcagttactacggaatgcgtgccattcttctttactacatgtattatagtgtaactaaaggcggcctggggtttgataagccattagctgcgtctgttatgtcgatttatggctcgttagtctacttaacctcggttatcggtggctttgtgagtgaccgaatcctgggtagtcgccggaccgtgttctatggcggtgttctgattatgtttgggcacatcgcgctgtcgttgccaatgggtgcgccggcattattcacctcaattgtcctgatcacgattgggactggattattgaagccaaacatttctgaaatggtcggtgggttatataccgagtatgatacacggcgcgattccggattcacaattttcgtattcggaattaatttgggatcattcattgcgccgctgctggttagttggctcggattcaacgtcaacttccaccttggcttctcactggctgctattgggatgttctttggattactgcaatatattcgcggtggcaaaaaacatttgcctagtgccagcctgtatccaagcgatccattagaacccaacgatgccaagaaattgactatccgggttggtttgggagtggttgtcttcggcttgatcctgttgctcatgcaggtcatgggggcattatcactcagctcatttattaccttgctgagtatcattgccgtggccacgccaattatttactttgttgtcattatttcaagcaaaaaaatctcttccaccgaacgctcaagagttgttgcctatattccactgtttatcgcagctgcgatcttctgggcaattgaagagcagggatccgttgttttggcactatttgccggaacccaaacgaataataatgttggcggtattttcaatatttcgccaggttggtttcaatcgttgaacccactgttcattatgctgtacacgccattctttgcttggatgtggattaaacttggcaaaaagcagccgagctcaccatccaaattttcactgggattaggtattgccggattatcctatctgtttatggtgattccagttgccttatttggcgcacaagcaaaagtgagtccactatggctgctcggaagctgggccattgtggaaattgctgaactgttaatttcaccaattggactctctgttacgaccaaactggcaccaaaagcctttgaatctcagatgatgagtatgtggttcttagccgattcagctggtcaagcggtcaactcacaaattgttaaatactatacaccggacaatgaaattaattacttcttgatcgttggtctggttgcaattgtcgccggagttttgttggcattcctggttaaaccaattaagcggttaatggaaggtgtcaattagattcaagaacgaccgaatgtgttatcctaatttggatagcacatttttattttggggagaaaacgtgatggtaaagattgccgtaaccagtgataatcacttagatttgaataaggtgacactggccgatacaattaaacagcaggcaacttttttgcaagaccaaggggtagacgattacctgattgccggcgatctattcaatgattttcagaagtcggtggattacgttcagcagctgtcagcagccgttgatccaatccgagtttttttcatcgccggcaatcacgacatgatcaaaggtgtcagttatgatgaattggaaaatggccagtggccggggtatctgaacaatcaattctttgacgtccctcaaaccgactaccgaattattggcatgaacggctggtatgactacacttttgcagtgaatgaagataaaactgaagatgaatttcatcgttggaaaatggcttactggatagacgggctgatttcgcagcctatgagcgatcctgaacgggagcagatagtcctttcggaattgacccaacagctccagaacgcgcaatcagcgggcaagaaagtgattttgatgactcactttgttcccaaccaacacttcattcattatacgaatgattttcgcttctggaatatggccaatgccatgatgggcagtctgcattttcaaaaattgattgagaactatcaggttgaacgggtcgttttcgggcatattcatcaacgactggtgcctattaggcttaaggcgacgacatactataatgcagcggtgggataccacaaccatcgtcacaatgagtggcagacgaatgatttcatatctgaatgggcaaagcagttgaaaatgttccaaattttttgatgattgcgcttgacggaatcactaaaattttgtattattatattcgttggtttgatagcaacactcttttggaggggtagcgaagtctggctaaacgcggcggactgtaaatccgctccttcgggttcggtggttcgaatccactcccctccattttatttttgggctatagccaagtggtaaggcaacgggttttgatcccgtgatgcgctggttcgaacccagctagcccaattactaaacgtctgtgacgaaaggaactcgtcgcgggcgtttttttgtattttcaacgatcgaccattttgatattgcaaaattttgcattttccgctattgtcagtgttagaagaattggaatagtccgattgtaaattcaggaggtagcttatgaaaattggttttattggcgttggggcaatggctcaagcgatcattcaaggactgctgaaagcagaatttgttcctgctcaagacattttggtacacagtgctcaccaagatcattacgaaaaatatgcggctcaatatggcctgaccccgaaagaatcgaacacggcggttgttgacggcagtgatctggtggttttggcagtggtaccagccgttgtcaccgatgtggtggcggaaatccgtggtgcactgtcagccaagaagacgttgatctcaattgtttcaggggtttcgctggatcgattagaagagttgaccgattacaacctgccaattcttcgcagtctgccaaatatcaactctgaattcggtcaggggatgaccgctgttgcggctaacgagaacttaaccggggatcgaaaagcccaagccatctcgctatatcaagcaactggaagtgtgttggagcttaaagaaagccaattttcggtattcagcgccatttccggtagtgcggtagcgtacgttgacttctttatcgatagtctcagccgggccggggtcaagtatggcttcaccaaagaaatggccacccaaattgctgcccaaacaactctcggctctgcgcactcattgatggcatccaagaagtcgccagctgaaatgattgataaagtcagttcgccaggtggtgatactatcgccggcattctggcgatggaagaggctggattcctaccttctgtcatcaagggaattgacgcgacgattgccaagtcaaccggtaaccattagtcgacttgtggagcagatatgtcaacagtattaattcatgcaaagatctatacaggtaaacgaattattcaagacggctacatcagatttggtcaaacaattctcaacgttggcccaataactaattttgaacagcagccaagtgatcggatcatcgatgcttctcaacgcacaattgtccctggcttcattgatgtgcatacccatggtggttatggtgcagattccatgaatttggatcctcaagttattagccggatcgtcaacctgatggcccacgagggggttaccggcgtttttctgactaccatgactcaaagtgccgatgccattgctaagagcatgcagacgattaaaatggcggctgaaaccaacccgcgaattttaggtattcatcttgaaggaccgtttatttcacccaagtaccacggcgcccagccaacggaaaagattcaaaagcttgacgttgataaaattaccaggtggaatactctctcgggtgggctggtcaaaattttgacctacgctccggaaatgcgcgttgacccaacagccgtcagttattgtcgagaacacgggattcaaatggcagttggccactctgatgcaacctatcagttgcttaatcaagctctgcccccgcacgttacccatttatttaacgcccagcgaggtctccatcagcgagaaattggtgtggtggggtatgcgatgctttctcaagccaaagtggagttgatttgtgatgggttccatgtggtgcctgaagcggtacaaattgcttatcaaaccattggccccgatcggctggaactgattactgattccatggaagccaaagggcagccagatggcatgtatcagcttggcggccaaccggtcaatgtttttcggggaagggcaaccttggctaatggccatttagcaggatcggttctcaagtttgcggacgcttttaaaaatatgattcaatttaccgattgttcaattgcttcagccgtcaaaatgacctcgaccaatcaggcggaggaatttcacctgaaaggcaaaggattcattgagaatgggtatgatgccgatctaaatttgtttgacaatcacctagaccttatggcaacgtatagttatggcaaattagtgaataaaaactaagggagttggtatcagtgggtttaccaatttatattcaaattcataatgagattaaacgaaacattgaagcaaataggtggaaaattggtgatcgcattccctctgagcgtgagttatcgaccgactttggtgtgagtcggatgacgttgcgtcaagccattcaaaccttggtggacgaaggtattttagagcgtcgagtcggttcgggaacgtttgtggccaatcagaaagtgcaggagaaaatgtctggggttaccggcttcaccgatctgatgctggctcaggggaaaaagccttccagcaaaacaatttcgtatcacacgatggaaccgtctttgagcgagatggaaaaattacacatcagtcaggaacaagcggttttacggatggaacgaatccgttatggcgacgacattccgatttgctttgaagtcgccacggtgcctgaaaatattgtcgagggcttggaaaaatccgaagtaaccagttcgctttatcgaaccctggagcaaaagaagaacctgcaaatcggcaaggcccagcagacggtgtcggcgatgctggcatcggagcggattgctgaatatctgaacatcaaacgaggcgatgccattttgagactcagacagattacttcacttcaagacggtcgcccgttcgagtatgtccgcacccaatatgtgggcgatcggtttgaattttatttggaaaaagagtagtgggcgacgagacccgggagatgcgttttctaagggtactgggatttaaataccggttttgagggatttgaatcccagtacccttagaagtgagcatctgggtcgtcggagccgtcctcagaagtgactaaaccacaaggtgacataatatctccgagtaacgagataggcggccgccatataccaagtgccccttagaagtgagcatctgggtcgtcggagccgtcccccaagcggacaaatccagcaacacaaaaacttttcacacaaaaaccaggccatcacatttgttggcctggttttatcgtcctatgattgttttttctgatttttcttctttggccgatcgtaccgctgagcatagccggaccgaatccaatcggtgacccaggccatcacagcagacataaacgcgaagataatccaagacgtccaatcacgataaccgccaatttgacgaagaatcaccatccacagcacaaagtaaatcacatagaagtttaatctgggcatccgcagataactggtgacataagccagcgcaaagattcccagcataccgtactgggtgtcttgaatggccgcctgatgatggagcaaattaacaatgatgccaacgccgacataaataattagaaaataggtccaaaacttcggtgaaactttcttcattgagccctcctggattttcttgaatatttttgtttaacgatctgccacaaatattttggcagcaccatcaacctgccaaagcgactgggttccttgacgacccggtacaaccactccaaatgcattttctgccaagctttgggtgctcgtttgacagttccggctaagacgtcaaatgaaccgccaattccaatccaaagggcgtcggcagcccgtcgatttttattgataaaggcttcttgcttgggataaccggttgcaacaaagaccatatccggctgggtccgtttgatatcgtggacaatgttgcgatcatcgccaaaatagccgtcgtgggtgccggcaatcgttagaaacggataattttcctggacgacttttttgagcttgcgaatcactgctggctgagcgccgacaaagtacgccgatttttggttggcgtttccccattccagtagatggacaaagagatcatatccggtcacccgttctttgagcggcgttttgagcatcttggcacccatgataatgccaataccgtcaggaacgatgtagtcagcggtcgtaatgagtttttcgtaatcgggattcgccttggcatacatgacgatctccggattggcggtgacgacaaacgtattttggtgttgattgatgacgttatgtaaaattgcttggaaatccttttcggtggtattttcaaaagggatgcccaagatatcaactggttgggtgggactttggttattcatagcagctcctttagactttgtttcatgcgaattgcaagattattttttgttaataatcggaaaaatgatagaatataaactaattatataacaaatctccggggaggatattgacacaatatgtcagaagacgataatttaacgctccataccgatttttatgagatcaacatgatggccacctactttgaaaagcatatggaaaatcgtaaggcggtttttgaagtgtttttccgcaagctgccgtttggcaacggctacgcggtatttgcaggcttggaacacattatttcatacatcgaaaatttacaattcactgatgatgatatcgattatttgcgcgaagtgacagattatccggacagttttttagaatacttaagaaactttgaatttaaaggcaccatcaaatcagcctatgaaggcgatattgtttttgccaatgaaccaattctccaagttgaggggagcttgtgtgaatgtcagctggttgagacggccattttgaatatggtcaattatcaaacgctgattgcgaccaaggcttccagaattcggacggtggtcggtgacgatccgttgatggaatttggcacccgccgagcccaggaagtttcagcagccctttggggaacccgggcaaccatcattggcggttttaacgcgacttccaacgtcttggctggtaagaagtttggtatcccaatcagcgggactcatgctcattcattggtggagtcgtttggtaatgattatgacgcttttaatgcctacgctcagacccatcacgactgcgtgttcctggtagatacctacgacaccttaaaaagtggggtgcccagtgctattcgggttgccaatgaaatgggtgacaagatcaattttgccggcgtcagactggattcaggcgacatggcctacctttccaaacgagtacgtgaagttctcgacaatgccggttatccgaataccaaaatctatgcttccaatgacttggacgaaacgacaattgccagcttaaagatgcagcatgccaagattgacgtttggggtgtcggcaccaaagtcatcactgcctttgatcaaccagccttgggcgctgtttacaagatggtttccgttgaagacgctgacggcaaaatgacggatacaattaagatttccggtaacgctgagaaggtttcgacacccggcaaaaaacaggtttggcgcattactgacagtaaagacggcaagtcggaaggcgattacgtcacactggccgatgaagatcccagaaaagaaaagtcgatcttcatgttccatcccaactatacttacatcaataagactgtcgataattttgatgcaatgccactactcaaaccaatttttcaagacggcaaattagtatatgaccagccaaacttaaagcagattgtccactacgccgaaaaggaattggcatcattgtggcctgaatacaaacgggagttaaatccccaaaagtatccagtcgatctgtcacaaaagtgttgggataacaagcgtgacatcattgaaaagattcgcaattatattcaagatatcaactactaaatttgtaatcgagggatgcatatgcgagctaaacaacaagaaattattgacgcgttaaaagtgaaaccaacgattgatcccaaagccgagattcgtcgttccgttgactttttgaaagactatctcaaaaaattttctttcctaaaaacattggtcttaggcatctctggcggccaagactcaacgctggccggcaaattggctcaattaaccatttccgagctccgggatgaaaccggcgatcctgactaccagttcattgcggtccgtctgccatatggtgttcaagccgatgagtctgatgccttggaagccatcaagtggatggacgccgatgtggttgccagagttgacatcaagccggctgttgacgccgcagtggcttcagttgaggcaaacgatatcgaagtcgccgattttaacaagggtaatatcaaagcccgtcaacgcatgatcgcccaatacgcaattgccggtgccaaatccggtgccgtggttggaaccgatcacgctgccgaagcagttaccggattttataccaaatttggtgacggagcagcagacattacgccgctttggcgtttggacaaagagcagggcaagcagctcttaaaattactcggtgcccccgaacatctttaccaaaaaacgccaactgccgatttggaagataatcgaccagcattgcccgacgaagttgccctgggtgtgacgtatcaggatatcgacgcttatcttgaaggtcgcgaagtttctgagaaggctgccgagaccattgagagctggtatgataagacgcaacacaaacgtcacaccccgattaatgtttatgacacattttggaaatagatatttagtgacttttcattagtggttaggtataattaccataaataaagggagtaaccagcaatttcgattgcgattatctcgtcaacgtgaaatactcgtatttccgggataaatcttaaatggtgagacttatgaattcttttagcgaggaatttgtgggtctcttttcttttagaggaggaagtttatgacacaggagaagaagatgttctaccaacgaacagtcgatgatgtgatgagtcaaatgaaggcccatcccactggtctgtctgatcaggaggtcaaagaccgtcgggaacaatttggtgccaacagattaacgtcaaagcggcggaccacgttaatcgagaagttcatttcccaatttaaagacttgatgatcatcatcttgattattgccgcgattattgccgggtttgccggtgaaacggtggatgctgcgattattttggccgtggttatcctaaacgcggtgtttggggttttccaggaatccaaggccgaaaatgcgattgattcattaaaagaaatgtcggcacccatggcgaccgttctgcgaaataatcaaccgatgtcaattaagagtgaggacattgtcccaggagacattgtcctcttagaggcaggagatgtcgttccagccgatgttcgactgattgaggctaattcccttaagatcgaagaagcggccctcacaggcgaatctgtgccggttaacaaacaggtggacccaatcgtggaagacgacctgccattgggagatcgaaaggatttgggcttcatgaacagcaacgtaacgtctggtcgggcaaccggcgtcgtgattggcacagggatgaatactgaagtcggcaaaattgcccatatgttaaacaccactgaagaaaccaccacgccgctgcaggagaacctgaaatcattaggtaagatgttaaccgttttgattctggtgattgccgtcatcgtgtttgctgtcgggatgtggcggggacaagagagcttgattaacatgctgctgacggcgatttccctggcagtcgcagccattccggaaggcctgccggccattgtgaccgtcacgttggcattaggaacccagcaaatggcccgccaccgcgccttgattcgaaagctgccggctgttgaaacgttgggaagcaccgatgtcattgcctcagataagactggaactttaacccaaaacaaaatgacagtggaaaaagtcttcttgaatgaaaaactgcaagattccgctgacacccatttaactttaaacgatcgattagcgcaaatcatggttttgaacaatgacaccaaatatcaagaaaatgagttggctggtgacccaaccgaaaccgctctggtgtcgttttacttacatcaagaccagccagtccaaaagtttgtcaattcccatcggcgactggccgaaattccgtttgactctgagcggaaattgatgtctacctacaaccaaatggacgatggccaaatcctaatgaccatgaaaggggcaccagatcagctgttggaacgggtcaccaagattcaagatggggacaatgttcgagacatcactgacgatgacaaacggttaattagtgtcaccaaccatgatttggcgactcaggcgctgcgggtgttggcgtttgcctaccgtcttgtagacacggtaccaactgagctcacatcagccgcccaggagcacgatatgatctttgttggtctcatcggaatgatcgatcctgaacggcccgaagttgctcaagcagttgcggaagccaaatctgcaggaatcaaatcgattatgattaccggcgatcatcaagatactgcccaagcgatcgcgaaacggttgggaatcttgggtcggggtgacaatcctggcggaaaggtcatcaatggggctcagcttgatgagatgtccgacgaccaatttaaccgggaagtcgctgacatttccgtttacgcccgggttgcaccggagcataaggttcgaatcgtcaaagcctggcagaaacagggcaaggtggttgccatgaccggcgacggtgtcaatgacgcaccagcgttaaagaccgcggatatcggtgttggcatgggaattaccggaaccgaggtttccaaagaagcctctgacatggtgttggccgatgataactttgccacgatcgtaactgcggttaaagccggccgcaaggtgtttgccaacattcaaaagtcactccagtatctgctttccgccaacttgggggaagtcttgaccttgtttgtgatgacgatgatgggttggcagatcttggcgccggttcagattttgtggatcaacctggtaaccgatacattcccggcaattgccttaggcgttgagccggcagaacccggtattatgaaacgcaaacccaggggacgaacgtccaacttcttgtccggtgggatcatgagcaacatcttgtatcagggattttttgagggctttattaccctttgtgtttatgcatttgccatcaccaacccggttcatgcttcagatgcgttggcccatgcggatgctttgacgatggcctatgcaactctgggactcattcaattgttccatgcctttaactcgaagaccatccatgagtcaatctttagaattggcatgtttaagaataaattctttaactgggcacttttgggatcggccgtgctgttgatcatgacgattgtcatcccaggattcaacgagatgttccacgtgactgagttgaccgcttcacagtggctggtcgtcgtcttcggtggctttatgatcgttgttgtttcagaagtagtaaaatacattcagagacacatttcccataaataaaattgaatggaggctgatattttgaaaccacaagatatgcagcgatatgcaaaaaccgtctcggacgtgattgatgagacgtcaaaaaacggtgaggatttaaacgccgattatgaaacactcagaaaggcaattgataaccaaacggttgctgatttgaccagtgatcagctggcgggcattcaagcccattttcaatccggaaccgataagtaccaagataacgtgaacaagcttgagcaggtggctgtgccggttaaattgttaggcaagcacaagttgctggttcgtcattatgaggactatgccaacgcctgccaggcaatgacggacagtattgacccgcaggcttcaacggtggacgttgataagttcaaccaagctgagaaggatcaggaaaatagtatcgctaaggtttccagtacgactacgcggattatgggagaaatttaaagagtgcgaagcgggctgggtgacgcggtttctaagccaactttggtttgaaccccgggtttgggtttaaatcaaagttggcttagaggttagcgtcaggcccgcgaagcacgtttcaaccagagtgcgacaagcaatgctttgacacggagagctaaggtcgctttgattaaaatcccgggtttgggtttaaatcaaagaggcttagatcgcagtgtcagttgcatcgaagcacgtttcctcaaaccaaccaaccagaaacccactccacaacaggagctcccaaaattaaaaaattaacattcaacattccgcccaaactgcagacaagtgttcctgccagcagtttgggcttttatgttcctgagaaaacctggttggagtccccggcatttgcttcattctgctataattaaacgtgacactattgatgaggtggaaatacatggacaacacattagcacataagattcagcaagacttacccaaaatccgggagaaacaaatcgtcgaaaccctcaagatgttggatgaaggcgacaccgttccttttattgcccggtatcgaaaagaacggacttccaatctggatgaagttcaaattcgagacattcaagacgctgctcatcgcatccaaactttggacaagcgcaagcaggaagtcatcaaaattattgatgaacaaaatgccttaacccctgaactgaaaaagcagattgaggcggcttcggttcttcagcaagttgaagatctttatttgccctacaaacaaaaacggcggacgaaagcgacaattgccaaagaacatggtttggagcccttagccaaatccgccatgtcgtttgcccccgatttgaagcaacaggctgcccagtatgttgacccggacaaagaactgcctgatgttgacgcagtcttcgccggagtccacgaaattatcgctgaagacgctggcgaccgggccgattttcgcgaatgggtccgccaaaacacccaacaatacggtcagttggtcgtcaaagttaaacgcggtggtaaagagttggacgaagaaggcacctaccagcagtattacgatttcaatcaacccatcaaatcaattccttcgtttagaaccttggccattaaccggggtgaaaaagagaaagtgctttcggtcaaaattgaagtcaatgaggcaccaatcatgtggcatttaaaggccaacaccgtcggcagtcatcaaggatttgctgccgatgtggttaccgatgcaatcgaagatgcctatcaccgcttcatcggaccggcaatcgagcgtgaaatccgcaagcagttgaccgaagtcgctgctgatcacgccatcgatatcttcggcaagaatttgtacaacttgctgatgcaggcgcccctcaaaggcaaaattgtcatgggatttgacccggcttatcgaaccggctgtaaattagcggtggtcgatcaaaatggcaagtatttggacaaaacggtgatctatccccataagcccgccagtgaagccaaacgtaaggctgccaaagggctgttcattgatttcatcaaccaaaatcacgttgaaatgatcgccatcggtaacggaaccgctagtcgggagtctgaacaatttgttgccgatgcaattaaagaaatcaaaacgcccatttattacgtaattgttaatgaggcaggggcgtcggtctattctgcaagtcaagtcgccagagacgaattcccggactttagtgttgaacagcgttcggctgtcagtattgcccgcagaatccaagatccccttgctgaactcgttaaaattgatccccaggcaattggtgtcggtcaatatcaacacgatgttccgcagaaacaactgggtgaacagttggacacggtggttgaaactgccgttaaccgggttggcgtcaatttgaatactgccagtcccgatctgttggtccacatttccgggttgaccaaaacgaccagtggcaatatcgtcaaattcagaaatgaaaatggcgaatttagtgcccgctctgatctcaaacaagttccccggctcggcccgaaagcttttgagcaatcggtggggttcttgagaatcatcggcggcaaaaatccactggataacaccgatattcatccggaaagttattctgccgccaaaagcctcctgaaaaagcacggattgaccattaatcaactcggcgagccggccgtttcaagtgctttgagccagcttaatttggctcaggaagttgaaagcattggagttggggttgccaccttgaaagatattatcaagggcctcgaaacgcctggccgtgacctgcgtgacgaaatgcctgcgccgttgcttcgaaaagatgttttgacgatggaagatttgaagccggggatgaaactgcagggaactgtcagaaacgtggttgactttggtgtctttgttgatattggcgttaagcaggacggtttggtccacatttccaaaatgagtcggacattcgtcaaagatcccagcaaggtggcttcggtcggcgacatcgtgaccgtttggattgactcagtggatctggatcgtcaccggattcaattaaccatggtggatcctgaaggttaggtgaacaaagaactcatgactgatcaagaactacagcaactcgttgaacatatttcgctgcaatactttgccaaaccgtttacccaccgggcctattttaatgcccgtttaaagacgactggcggccgttaccacctcaatgatcacaacatcgacattaatccaaaaatggacgacggggctgatcatgcggtattaattgggattatcaaacacgagctttgccattatcatctccatttggcaggatacagcgccaaacacaataccaagcagtttaaacagctgttaaaagcggtcggcggctccagatacgctcccagagtccagagtaccagggtccaaacgcgttatatttatcgctgtgaagactgcggtttggagtatcatagaagacgaagaatcaatctggtgaagtatgtctgcggcagatgtcgcggtaagcttcatttaatcagccaaacgcggcaaatcggagcgtagaaaggagccatcacatggcaaaaattattatcagagtacctgcaacgaccactaacctcgggtcgggtgttgattcggttgggttggcactgcagctgtattacacggtgattgttgaggaaaagacagatgaatggaaggtcaaccatgctttgggacacgacattccaactgatgagcacaacctcattgttcagacaatcttaaaggtcgattctgatattcatccgcatcaactgaccgttatctcggatgttccgattgcgcacggtttgggctccagcacaaccgcagtggttgccgggattaaaattgccaacaagttaggggatctggggctttcaattgaagatcaaattaatttgggaactaagattgaaggccacccggaaagcgttgctgctgcgatgcttggcaacttggttgtttcgacatatgacggtgaaaccgtcactgctgcgactcttcctgtcccagacgtctcggccttaatgtatattcgaccggatggtgtcagcgaggtagaaagtcgcaagaagctgccgaaacaaatcgattatgacgtggccgtccatgccagcagccaggagaatgttttcatcgccttggttgcccagggcaaatgggagcaggcggttaagctgattgagaatgatcatctccacgagccctacagaaaagagctggtcccagaaattgatcaaatccgttcaactgcccacaagttagacatctttggtacttacttgagtggtgccggtcctacggttgccacactgggtaagaaagctgctttaacccagttaagaattgatttggcacaacaaaatctaaatggtagtttgcggctgctgcaaattgatacagaaggcgcgaccgttcgcggtgaataattttcaaaaaccatttgtcaattgccaaaatttctgctataatttttaattgttgatgcggccatggcggaattggcagacgcgcaagattaaggatcttgtcgggaattatcccggtggaagttcgaatcttcttggccgcatggttaaagttcgaatcactatcatctcaatagtgattcggacttttttattgtgtagcatgtgatattttgctcaaataataagcgattggagtacaggaatgaaatattttatttttgatgtagacggaaccttgattgataccgaaaagatgtatatgttaccactacataagacactgctagaaaacggctatgacttctcttatgaagatgtcgttaagctctttgggattacctccatggacacggttcgaattcttggtgtcaagaacccggttgacattcgggaccaatggtttgccaaaattaaagattacacccaatatgcccacgtttatgatgggattgaggatgtggttaagaaactgcatgctgatccgactatcaaaaccgcgattgccacttccaaggttgaagctgaatttcaccgggatgtcacaaaatttggactggatcaatactttgatgcctttgttttttccaacgaaattaaaaaaggcaagcctgctcctgacatgattttaaagggcattgagaaattagacgctgatccggcagccaccatttatatcggcgataccaaatttgatctccaagctgctcacgctgccaacgtgcagtttgccctggccggttggcggaccaagaaaaccgcggactttgcggacacggattacgatttaaagacgcccgcagacttactaactattcagtaattccggcaaacgaaattgttattttgtgatatatttggtgtgaacagactttgtcaaatttaagaaatgggtgagtagatgatttcaattctggttgtgagccacggcaattttgccaaaagcttagtgacgaccgcagaaatgattgccggcaaacaggaacaggttggttgggtaagtctggccgcaaatgacggggtggattcgcttagtgataaggtcgcttctgcattggctgactttcctgaggacacgccaacgttgattttggcagacttgtggggtgggtcgccgtttaatgccgccgcccaatttgcagccaagaatccgcaatcgattgcattagttgccggagtcaacctgccgattctattggaggcctacatggcccgaaattcaaccctgagtgaattagttaataagatcaatgagattgctgacgattcgatccgtcagtttgaagtttctactgataatgatgacgatttgggagatgatttataatgacaatggatattcgccttgcgagagtcgacagccgcttgctgcacggccaagtggcaactttttggacacgggcggtgacgccgaaccggattatggtggtctctgattctgttgccaaagatcctttgcggaaaacattgattacccaagtggcaccgcctggtgtcaaagccaatgtcgtcaccgttaacaagatgatccgagcctatttcgactccaggtttgattccttcaacacgttgttgttgaccgaaacggtggctgacatgttgaaattagcagaaggcggcatcgatttttccaagattggcatcaatatcggcagcattgcctataacgacggaatgacgatgcttaccgacgccatttcgatgaatggagatatcgccaaacaaattcgaacattggcaaatgactttcatctagatgtctatgctcaaaaaattcctgctgaaaaaaaggaaaatttgttgaccctgttggataaaaagggcttttaaggaaccgaggggaattcaatgagcttagtttcaaccagcctggttttgttggtcgcatttgtggtcggaatggatggcattcttgacgaatggcaggtgtaccagccaatgattgcttgtacgctgatcggtttggcaattggcaacgtcggtgttggcattatgctgggcgcaattttacaaatgatcacgattggctggatcaatattggtgcttctgttgcaccggatatcgcgctgccggcagtcgtctcggctcttttagtgtgcggtccggccgccttaagtattaaacacgggattgccttagccgttccctttgcggttgttggccaacttttgaacgtcaccatccgtaaatcaattgtcaaatttatccatacggccgaccaagctgccgaaaatggtcaaatccagcagattgatcgcattcatctgctgagcttgggaattcaagggctgagagtcctgattccgacgggactcgtgatgctgatatctcctcaattgattcatcagttaatgcagcaaattccagcggggatcacaaatggcattgccatctcaattgggatggtgtcggcagttggattcgccaacctgattaacatgatggtcagccgctctttatggatttggtttatcgttggttttttaattgccatttttacgaagattaatctttttattttagcaggattaggcttggttgcggccatcagctttgtttggcttaagagtagacgacatggctcaaccggcggcgatggggaaggtaaagacgatttagatgactttgacaaagaacttgatgatttataggagttggtgggtataaatggcaaataatcaaaatatgattcacgattcccatcaaccgattcatcttcgtcagatcgattttttccggaccttttggcgctctggcactgagcagggatcgtggaactttgaacggatgcaaaacctcggatttgcttatataatggcgcctgcgattaaacgattgtatccggatatgaaccaacgtaaagctgcgttgaagcgccatttgggcttttttaacaccgcaccaattatgcagtccctgattactggagtggttttgtcaatggaagaacagcgggcaaatggtgccgatattagtgatgacacgattaatgccgttaagactgctatgatggggccaatgggtggttttggtgatccggtttggttaggcacgatccgtccggttctatcggcatttgctgccagtctggttttgagtggctatggcatgatgggaccaattctattctttattgcgtggaacgttttacggctggtctttcgttatatgactcaaatggccggttatcgtcggggagccgatattattaacctgtttaataccgggattattaagtacgttgggagcgccacttcaatgtttggcgtctttatgatgggcgtgattgttgctcggtgggtcaccgttgattttgcatcagttcggggactctttggcagttcaacgatttcccagttcgtggacacgatgattaatggcggccttaacgtgattgctccggttgccttgaccctggtttgtgtctggctgatccgtaggcgaatttcgccaatctggattattctggggctattcgttatcggagttcttggctactatgccggggtattggtttaaaaagcaaaagttacataaaattgattgtgaaaaaatagcggctcagataaaagttggtttgcttttatctgagccgctattttatggttcatgattatttaatagccattatatgtcgatgatgattgggttgccccttgaccgtcatcggtatctgtttgactggtttgaagcttggttgacttcgccaagccaagggatgttcgaatgtcgttggaaacccgcagcagttcgttttgaggaaccacttggtaggaaagaccatcgatcattgcgttttctccctgaagggtttgtgacttaatgtgatgagtggcgtcgccatattttgcccggatggcgatcatatcgtcgaaagtcatatccgtcttcatgttgccggacagtgacgagaggattgatttgtaacggggaagggaggtaatgttaagccccttcatgactaacttcttgataatctgtcgttgacgcgcctggcgaccataatcaccacgtggatcgtcatcacgcattctggagtagtccagagcttggcgaccatttagatggattttcttgcctttgacgacatttgcagccccatactggaacgtcagtggtggggtcacgtccacgccaccaaccgcattgaccattttttccaaaccgcccatgttgatgatcgcgtagaagtcgaccggaatatcgagcagattttgaacggtcttaacggctgttccggcgccaccaattgtataagcggcgttaatcttttcatatggctgggtgtcgccggggacgaccaccttggtgtcccgggcaatactggtcaaatgaatggtctttttctttgcgttgacagatgcgacaatcatcgtatccgtccgaccagtgtcgtgacgacccaaggcacctgtatcagttcccaatagcaggattgacagtggctttccttgctggatcactgacgaaacgtttcgagctttggtaacattggttgaatcgtaggtcttcttgaaggtcgacttggcactcttgtatgcgccgtatccccagaccaggccaccgcccaaggcgatcagcaggacgaaaaagatactccagccgataattcttcttcgacggtggttctttttcttatagtggggtttcttgtccgatcgacgagaatacactggttcaaaatcattattgttatctttatctgatggcatattgactcctcatttacaaaaaattctcccaaaagtatatggcagatttggacttgattgcagaaatcttcggttatttaaacattatttaataattgtaacatctgttgtgaccaacttgttcaattataccaaaaattataaccggctgtggattctaattgtgttataataattcattgttattgatttttagaattgaggaatgtttatggaagttttttataatgctgtttctggggttttaattatcctgattatgattgccttggggtttgtgttagccagaaacgattggtttgacggtaagatgaccagcatgattgcgcgcctggtaacccaggttgccctaccggcctacatgatttcaaccattatggaaaaatttactgccaagaagctgctgaccacacttcctgacttatttttcccaatcgtttcgatgctgtcactctacattgtttcaatctttgtggtcaaatttgccaagatccccaaaatgcattctgggttgttcatgtccatgttttccaactcgaacaccgtttttgttggactgccggttaacatggcgctgtttggaaaatccagtttgccgtttgtgttggtctactatatggccaacacgacattcttttggacactgggggtttatttgatccaaaaagatggcaaaggtgaggcttcatttaattggaagcaaaccctcaagaaggttttttcaccgcctttgcttggtttcatggtcggtgtcgtattggtattgatgcacgtcaccctgcctgattttttgatgcaggattttaattacatagggaatttaacgattccactgtccatgatttttattggaatttccatcaatagtgttgacttaactaacgttcattttgaccgcagcaacttcttgattttgtttgggcggtttatgctggccccaatcattatgtcgctattggtcattccaacgccaatgccggtgatgatgaaacaagttttcatcatgcagtctgcaatgccgattatgaccaatgcgccggttgtttccaggttgtatcatgctgattctgaatatgcttcaatcatggtggctgaaaccacgttgttgagtctgatcatgattccggttctaatggttttggttgagaagctttaggagaaatgctacactgagtctgttcacacaacgacttgagaggttgagaagattagaaggtggcttcggtcatcttttttatggatttatttgtgaacaaattaatttgagcaaagaggatgtaaacgtgccgacactagtcatcatgcgccacggagaaagccaagccaaccgggacaacatttttaccggctggagcgatgtacctttgaccgataaaggggttcgacaggctcacagtgctgggaaagtgatcgccaaatctcagattcagttcgatgacgttcatacgtcgtttctgaaacgggcgattattaccaccaacattgtcttggatgaaattggtcaaaactttattcctgagcataaatcctggcgccttaacgaacgtcactacggtggccttcgtgggaaaaataaacttaaagtcaaagaacgagtgggcgcaaagcagctcaaaatttggcggcgaagttttaccgttgtgccgccgcttttgaccaagcgggacgaggatccccgttatgagcgttacggtgtccaaattccattgggagaaagtctggaaatggcacaacagcgattgattccatactgggttgatcagattgcgccgaacttgttagacaacaagaaccaattgattgttgctcacggaagtaccttacgcgctttgatcaaatttctggaaaatatttcagatgaagaaatccccaacgtggaggttcctaacggcaagccgattcgatacgattttgatgagcaattaaacattatcagtaaatcgttcatggagtagttcgttgcaatttaatagaccataaaaaatacgacaaatcagataacctgacttgtcgtatttatcatttaagaacaaattcttaggctaaggcacccattggatcccaaggcttcaaaacagttggttcttgtttttgggcttcaagctgttcgtcggtgaggtactttttgttgatcacgaactggtacacgaattcgttcatccagtcgtcactcatcacgaagtagcctttggtgccgactttttcgccccagctgttttcaaccttccacttggttggttggccgtcgaccagatcgactccggtaatcaccatggcgtgggtcatcaagctttcgccgtaatccaaacgttcagcttttgacatcgacaaatctgaatcgaataattcgtcgggtgcgtagaggctggtgtccatgattccttttttggtgttggaactttggccaacgtcacttccgaaccaaacggattcgccattttgcagctgtttaattgccaactttttgagttcagacatttccaggttcaaatgtttgaccggccggccattgacaacgttgcccaacatttcaattgtgtaggtcttattgaatggcttgtcatcagtgggtgagttgatcagggaaacgtagtcttccaagtttaagttaacgtattttttgaagaattcttgtggggtgatgccagcgtcaaagtgataattcttatccttgtcgcggtattcgaagtcaaatttggtggctggttcaccgagtgcgtaggtcaacatgcggtatacttcactcatcatattgtccttggtttcggcaatcttagcttcggatgccttgtcagcaaccaattcacgtaaggcaacggcgtcatgacgaagcttcaggttcaagaacttgttgagctgagatgagcgattactgttgaaggtttccggcattgccgacttgggaacgatcccatatttttcaattagggcacaaagcatatcccattgaccgccatcttgttgtggcgttgccatcaaccaggcaactttgcgtgaatctagcggctggtcggcagtttttaagacgttttccaagaaataattggccttttcaaatttatcccagaagttggtgtagttttgggatagttcgaaatcatccggaactttataagtgttcatgaggtgaatgcgcatcgtattgagggcggcaaacatccagcatcgaccactttgcttttgatcagcaacttttccagttgaaagatcgattgaaaataccgggctcattttgccttcagcggtaaagtcctcgctgctttccaaaatgccctgatgggtaactgcccgttcaatcactttcgaatcttttcgattatcaagattcttctggtacttgctgatttgatctaaattaatttctgctgtcaaaaatgatcactctccttaatagaatcttattttacgctcatttattaaaaagggctagtgagcagggtgcttttaaacggcaaacagccggctgcgaatcgttttgatcgcatttccggctgttgtcagtttttattcaattagcgggcttgaatggtctgcggtccatcttcacggccaacaatgactgtgttaaccaggtcgaggaacagtccatgttcgacgattccggtcatttggtctaattcaagcgccaaatggtggggccgttcaatttggcctaagtgcaaatcaatcacgtaattgttggagtcggttttgacgtactgatcgccattcatcctaaactttgggtgataacctttggcatcaaggcgtttaagcagttgatggctgccgtaagggatgacttctagagggagtgggaatgaacccaactcatcaaccattttgctgctgtcgacaatccacatgtttttatcggaattaattgccacgatcttttcccaaagatgagcggcaccgccacccttgattccctggaaggtccggttaatttcgtcagcgccatcgatggttagatcaatatggtcaatctcgtctaatcccttggttttaataccgagactgttggcctgttcacgggtccgttctgaggttgggacaccgacaattgagaggtgttcggacttcactcgttcgcccaaagcatcgaccatgaatttgacggtagatccagtgcccaaaccaacggtcatgccgtcttcgatgaacttaacagcggccttccccacagactgcttcaactcgtcttgatgtttcatatttgttccctcatttcaaagttgtttaaaggttttactacaccattatactgcgatactttaccatctttgtcaatctgtgcaaacagcttcacatagtttatactacaataatagaatatattgacagaaggagccagacatatgaaacgtggatttgaaattgtctcaaaatatgcagacgaaaacttaagcctgccttaccgaacgacggagaacgcagcaggatatgactttgaaagtgctgccgatatggtgattccatctatctggaaattgaattttttgaaagtcctttgggcacttaaacatgagaaaacggttcgggaagacagcattgccgaggccaaaaaagtgcttaagccattcttaattccaacggggattaagtcctatatgcagcctgatgaagtgctcgtgattgccaatcgatccagcaacccattaaaacgtggattggtgattccaaacggtatcggcgtgatcgattctgattattataataatcgcagtaatgagggcgaaatctttgttcagatcctcaactttgggatcactgacattaagatcaagaaaggcgaacggattgctcaaggcattttcctgccgtatctgttggcggaccaggacgaccaacgcaaaaaacagacccgaagcggtggttttggttcatcaggtcaataatttataagatgatgtaaagtccgccggcatttcgtcaaccttgattcataaagtgctaaaatattgatagtgtaagtataagaggagaatttagttggcaaaagttaaaacccaatttgtatgtcagaactgcggctacatttccccaagatatttgggacgttgcccgaactgtaatgaatggaacaccttggttgaagaaaccatcaccccaaaaaatagcacaatggcaacccaaagccttcgcagaaacggtatccatgacaataagcccgaatcaattaataaagttgagttccataaggacattcgtttcaaaaccgacatggaagaacttaaccgggtcctcggcggaggcgtggttccaggatcgctgatcttaattggcggagaccccggcattggtaaatcaactttgatgctgcaggtttccggtcagctcagtaaatccggtaagattctgtatgtttcaggtgaagagagtgcttcccaaatcaaaatgcgggctgatcggcttggtgtcaatggggaaaatctttatgtctaccccgaaaccgatatggatgtcatcaaagataccattaacgagatgaaaccagatgctgtcgtcatcgactcggttcaaaccatgcagattccagagctgcagtcagcgactggatcggtggcacagattcgagaagtgaccgccgatttaatgaacattgccaagggtcagggaatcaccgtattcgtcgttggccacgtgacgaaaggtggtgcgattgccgggccgaagattttggagcatatggtcgacaccgtgctgtattttgaaggtgacctgcaccattcctaccggattttgcggactgtcaaaaaccgttttggctcgaccaatgaactgggcgtttttgaaatgcggactgacggcctgagggaggttaagaatccttcagaaatcttcttggaagaacggctgaaagacgctaccgggtcggccattgttgtttccatggagggaaccagaccaatcctggttgaaattcaggctctggtaacggcctcggttttcggtaatgcgcaacgaactgccactgggctggaccgcaatcgggtgtcgttgattatggctgttttggaaaagcgggcgggattgatgctgcagaatcaggatgcctacttaaaggcggccgggggcgttaaactggatgagccggccattgatttggcaattgcggtcagcatcgcttcatcctacaaaaaccgcggcaccagcccgacggagtgttatgtcggcgaacttgggctaaccggtgaagttcgccgcgttacccgaattgagcagcgggttgccgaggcccaaaaactcggtttcaaacgggtcttggttccagccaacaatcttcagggctggaatccaccaactggcatttcggtagttggggtttcaacccttgctcaagctttaaagcttgcacttggttaaaggaaaattgagagaaggcgatatttttgaaaagaaagagaattgttagaattgtatttacattagccggcgccgcaattggagccagttattttccgatgatctggctgatattccaagtccgctatgggacgctgtttaacaacactgcgacaaacgcagttgtgggtgcaattattttttattttatttcgttgttaaccggcaattatattctcaaagcggtcgatcgggtggaagtcagattgacaaagcaaagtccgttgtcgttattttttgggaccttgggcctgattatcgggctggtggttgccatcctgatttcgattgtattcttcagaacccgcacgttcttcttgaataccatgattccaacgatcttaatgttggtactgggctattttggtttccgaattggcaatacgcagagtgatcgctggcgaaaaatgtttcaatcccggcggaagtcagaaactgccaaggccggcgacgaaaagattatcgataaaccagtcgataagaactatcatcactacaaaattctggataccaacattttgattgatggtcgaatttatgacgttgtcaaaaccgggtttattgaaggcaccttgttagttcccaagtttgtgttgtatgaattgcagtacattgccgactccagtgacagtgtcaaacgcgttcgcggtcgccgcggcctggatattttaaacaagctgcagaacgaagatctgattccgatcgaaatttacgagaaggattacgaggacattccagaagttgacagtaagttgatccagcttgccaaagacgttgatggtgtaattatcaccaatgatttcaacttgaacaaagtgattcaattccaaaacgtccaggtatttaacattaatgcgcttgccaactcgctgcggcagaagattctgcccggccagaagttgaacgtgatggttgttaaaaacggaaccgaacgccaacagggggtcgcttatttggatgacgggacgatggtcgttgtcgaagacggtcgatacttcttgaatgatcacattgatgttgtcgtaaccagtgctattcaaacagatgcaggtaaaatggtcttcgcccgtccggaacattcgaccaagaacattaccgataagcctgatcagaataaagggaatggcaagaatgggtcaaataacaagaagtagccgccttccctttatttttggcgaagttcattgtacactttaaacactgacaaaattttgattatttttaagaaagaggcgttatacattggcaaacaatgcaattcgagttcgttatgctccaagtccaaccggccacttgcatatcggcaatgcacgtacagccatttttaactatttatttgcccgtcacaacaagggtaaattcatcattcggatcgaggatactgataccaaacgaaatgttgccgacggcgagaagagtcaactggataatctaaagtggctcggtcttgactgggatgaaggtcccgatgttggtggcgattatggtccttatcgtcaatcagaacgaaaagatatttacacaccattgattcaacagttgatcgatgagggtaaagcttatgaatcctaccggactgaggagcagctcactgccgaccgtgatgcccaaaaagcacgcggcgaaatgcctcattatgaatatgaatacgaaggaatgaccgaagaccagaaggcccaagcaattgctgacgccaaggccaagggtttaaagccggttattcgattccgagttcccaagaaccatgaatatgcttgggatgatatcgtaaagggcaaagtttcctttaattcggataccattggcggtgattttgtcatccggaaacgtgatggcatgccgacgtacaactttgccgttgtctgcgatgatcatttaatgaagattagccacgtttttcgtggagatgatcatgttgccaatacgccaaagcagttgatgatttacgaagcttttggctggcaggcaccaagatttgggcatatgagcttgatcatcagcgctgataccggtaagaaattaagtaaacgtgacgaatcagtcctccaatttattgagcaatatcgcaaattgggttatctgcctgatgcaatgtttaacttcattctgctcttgggctggtctccggtaggtgaagatgaaatctttaccaagaaagaattcatcaagatgtatgacgagactcgtttgagtaagtcacctgccaaatttgattccaagaagttggaatggattaacaaccagtacgttaaggaagctgataacagtacgatcatggatttggcgctgcgccagttgattgccggtgggaatattcctgaaaatcccgacagcaaaacaatcgagtgggctcgtcagttgattatgctctataagcgtgaaatgagttatatggctcagattaacgacatggcctcggtcttctttcaagagccggaacaaattgacggtgatgcattggcagagatttccaatgaaacggctccggtggtcttaaaagaatttcttgagcgaattcaaaaactcgacatttttgactccgttgaaatctttaaagtcatcaaagccatccagaaggacactaagatcaagggacgtcaattatggatgccaatccgaattgccgtgacccacgaaatgcacggtccggaactaccagagtccgttgaactggtcggaaagcaaaaagccatcgcgcatatcaaagaaacactggctcaaatcgataaagcgtaatttataaaaaatattattgattcgattggtctcgttgcatttacagcgagaccttttattatgggttatagttaaagtaataaaacaatgtgaattatgatattatttgaatataaaagataaagagaggaattcgaaatgttgcagatatttaataccctcacgcgaaaaaaagaaaaatttgaacccatcaccccaggtgttgttaaaatgtatgtctgtggcccaaccgtgtacaactacattcatattggaaatgccagaagcgcgattgcctttgatactgttcgcagatacttggagtatcgggggtatcaagtcaagtacgtttcgaattttactgatgtcgacgacaagatgattaatgctgctcgacagaaccatacgacagttggcgcgattgccgacaagtatatcaacgcatttatgcaggacacggctgcgctgaacatttcaagcaacgtgattcacccccgggccactaagaacattcctgaaattatcgacttcgttaaaaccttggtcgataaaggctatgcctacgatgttgacggtgacgtttatttccgggctcgaaagttcaaaagttatggtgccttgccacacatcaacgttgatcaattggaaatcggtgccagccagcacgttaatcctgaagaaatggctaaaaaggaagacccgattgattttgccttgtggaaaaagtccaaaggcgatgaaatttcgtgggattctccttggggaaagggaaggccgggatggcatattgaatgctcagtcatgtccaccaagtacttgggaaaaacgattgatattcacggtggtggagaagatttaattttcccgcatcacgagaatgaacgtgctcaaagcgaagccaacaccggccagacgtttgttaaatactggatgcacaacgggttcgtgacaattggtgacgataacgaaaaaatgagtaagtcactgggaaacttcatcacggttcatgatttgcttaagaatttggacggccaagtgattcggctattgatgtcgaccacccattatcgccgtccaatccagtacagtgatgccagtgttaaagaagccagcagcaacttgaaaaagctgcagacggctttcaataaccttgaatatcggcttcataatgctgacgagggtgatgatcccaaaaccgaccaggaagtccgccagattgtcgctgactttactgacgcgatggacgatgattttaacgtccaaaacgggattgccgccgtttatgaactggcaaaatttgccaacacttatagtgaacgcgagactgtcttcaaattgagcctgcagtttattatcaataccctgcgtcaattgtccggtgtctttggcattaagcttgagcaaagtgaactaaaagatgatgagatttggtcactgatccacgaacgggaacaggctcgccatgacaaagactttattcgcagtgatgaaatcagagaagaacttaaagcccggggaattgtgctggaagatacgccacagggaacccggtttagaaaggaataacaactttaatgattgataatttttcccagttaaacgggattgccttggcgtacatgggggatgccgcgtacgaagttttcattcgccggcatttgattgcccaggggttgaccaagcctaagcgcctgcagcatgttgctaccaactatgtatccgcaaaggcgcaggcagctttaattgatttaatgaaaacagatggtctgcttaatgaaaccgagtgggactatttcaaacgcggccgaaatgccaacagtcacacccacgccaagaataccgacgtgattacctaccgcatttcaaccgggtttgaagcggtctttggctacctatcattaagtgaccagacggatcgaatgaaagaaatcgcaaattggtgcattgaacaagtagaaagtgggaacctcaaacatgaagaatgataatcgtagtcaagatcatcgcagcgatgacagtcaggatcagcccgaagagtttgtgattggcagacaccccgtggttgcggcgttaaagagtgaaaacccggttaacaaactgtttatccagtcaggaatcaaagatgacgacaatattatctctgaaatcatgaaattggcgcataaaaagcggctggtgatttcaaaggttccaaagcaaaagctggacaagctttccaataaccaaaatcatcaaggggtggtattatcaattgcagcctttaagtatgcaacgattgacgatctatttgccaatgccaagaagcaagcggttgaaccgttctttgtgattctggacaatatcgaagatcctcataatttagggtcaattattcggactgccgatgctgccggggtgtctggcattatcattcccaagcaccgagccgtgggattaacggccacggtttccaaaacttcagccggagccattgaacgggttccggttgcccgcgtgaccaatttgtcggcaaccattaaagaattaaaacaacgcggaatgtgggtttttgggactgatgtttccggaactgattaccgtcgttgggatgccaaaggctcaatcgccgttattatcggcaacgagggtaagggaatttccccgctgttgaagaaacaggtcgacgaaatgttgaccattccaatggtgggagatattcaaagcctgaatgcgagcgttgcagccagcattttgatttatcagggctttaattcccgccacccattatcaaaataaagtcggtgagaaataatgaaagaagacctgttaattgttgatgcctataatatgatcggtaattggccgcacctcaacaagctcaagcaggccaaccgtttagaagatgcccgcgatcaactgctggctgaattgtcggaatataaaaagtaccgggacatcaatatgatcgtcgtttttgacgcgatgtatgttcccggtaattcaaaaagcttccgtaagtttgatatggagattgtctggaccagtaaggatcagactgccgatagttacattgaggccttggcccatcgtaagcaaaatcgatttacccaggtgatcgttgctaccagcgatcaagccgagcaatggacgatttttgctgccggcgcattgcggatccccgctagagaattgctcagagacgttcagcgtgccaaacaggaagttgatactgaagcgcgcaagatgactgatcaaggccaagtgtttcgccacacgccatttgacgccaaacagctccttgaattagagaagctgcgggacaaaatgatacatgatggtcaataaaaatattaggatgctgatattttaaaattggtataggtgggatattcactgaatgaacgctggttcgtcttgccggaagttgaatcctccgttaatgtttttcgtaatcgaatctgattaataaaaacatctgagggggataacaatatgttacctaacaatcgacttgaactgattcgtcaaacagctaaacgaaatgaagaggcctttgcgcagctatttcaccaatattatccaatcgtccgcaagtacaaacgccagtattatatcaacggctacgataaagacgacctggaccaggaagcccgaatggttctgtttcgctcggcgtgccggtttgaagctgcgagaaaagtcagttttggaacctttttcagtcacaatctgcgaaaccgcttgtttgacctgattcgcaccaacaatgcccaaaaacgggtgccggtagaaccattgacatcatttgaagccaacgagtatttttacgctgccaaaatcgccgataactcagctagtagtccaattgatgcggtgatcgtcgatgatgcactccgcaaactatacagcagctgttcaccattggaaaagcgggcgtttaacctgatgctcagtgaaaatggttatgcggatttggatcccaaagcccaaagaggaattatcaacgcttttgaacgctgccggcgcaaatttgacggcgagataaattgacggaattgtttttgaatgctattattactatgcttgtaaggaggtgccgctatggcacaaagaaaagttgctctggcttgttcagtttgcggttcacggaattatacgattcccgccaaccccaatcgaaccaaacgcttggagctcaataagttttgcaagtattgcggtaagtatactttgcataaagaaactcgttaatcatgatataaggggataaaattttgcgattaattaattttttcaaaaaagttgctcaggaaatgaaagtggtcacttggcccaacgcatctcagacgcggactgataccagtaccgttatcgggacttcaatcatcatggccatctttttaggcttggttgattggatcgttcaatgggcactccaatttctggcatagccttttgagtcaatctttgatatagttaagttgttgaaacctgcgaaaagtgtcaggtttttttatttgaactcatttaatggaattacgaaggagcagaaaaacatggtcgagtcagcagaaaagcaatggtatgttttgcatacttattctggatacgaaaacaaagttaagatgaatttggacagtcgaaaagaatctatggggatgcaggattacatcttcagaacggttgtccctgaacaagaagaacatgaagtaaagaacggtaaggacaaagttaagatggacaagactttccccggctacgtgctggtggaaatgatcatgaccgaccaagcttggtacattgtcagaaatactcccggagtgaccggattcgtcggctctcacggacaggggagtaagccaacgccattgctgccggatgaagttgacttggtactcaaacggattggcatgagttctcgccatgaagatttggatgtcaacattggcgatacggttaaaattgtcgatggtgccttcaccggccttgatggcaaggtaaccgaagttgataacgaaaagcaacgacttaaggttaatatcgaaatgtttggccgtgagaccagtaccgatcttgacttcaatcaaattgatacaaccctttaacttaaagtaggtggtcacgatggtatggatggctggtttgataattgttttgctgattgcgatggtggttgtcggccggctgattcggcttggaacgcccaaccaggttggtaatgactccgatccggcaaatgggattgaggcgattcccacactttttattccgggctactttggtaatcgattgtcatttggcagactcatcaatcgattaactcgacagtatggagctaacaaatcgatggtcatcaaagttgaccgccacggtaaaatccatgtttcaggccatctggcaaagtcaaaggtcctgatccaagttctttttgccgacaagtcttcccgcccaaggcagcaggcagtgtggctctctgaagttttggaggtgctcaatacccgctatggtgttgaagagatcaacctggttggccattccatgggctgtattaccattttttggtttctgacccatcagagcaaaatgacgcctgtcagcgtggagcatgttgtggcgattgccggaccattcaatgattcagagattgccagaagtactgataaagttgacgcttatcctttgaacgccaaggggccaaccaaacgaatgccgatttatcgggcgctgtcacaacgcgtttttgcaattccaagggacattaaggttctcaatattgccggccggatcagcaacacccagcaaaatgacggagaagtctcggtgaacagtgctttttcattgcgctatttactgcaggatccggccgcgcaataccatgaattggtgattcgaggcaaacgggcaacccatcggctgcttcatgaaaatgccattgtcgaccaagaaattgccaagtttctttggaaccaataatttaggttgttgaatgaaaatgtttatgttatattagtatggtatgtttatgcataccaacgtgggaggagaaattttgatctccatttaccacacacggacttaaggaggttatgtctcgtggctaaaaaagtagcgaatattgttaagttgcaaattccagcgggcaaagcaacacctgcccctccagttggtcctgcattaggtcaagcaggtatcaacatcatgggattcactaaggaatttaacgcacgtactgccgatcaggcagggatgattattcctgtagttatcactgtgtatgaagatcgttcattcgacttcatcaccaagactccacctgctgctgtgttactcaagaaagctgctggtgttcaaaagggttccggcgaaccaaatactaacaaggttgcaactgttaccaaagaccaagttaaagaaattgccgaaactaaaatgaaagacctaaacgcagctgatgttgaagcagcaatgcgcatggttgaaggtactgcacgcagcatgggctttactgtcgaaggatagtcaacccggttacgtcgttactttaacgatgacacactgtttcacatcgcgtgggaggttaatccgttataaccacaagcaaggaggaaaacacacatggctcgtaaaagaggtaaaaactacaaggcagcccttgaaaaggttgatgctgaaaaagcatacccaatcaaagatgctgttgaattgattaaagatattgattttgctaaattcgactcaactgtcgaaattgtgttcaaattaaacgttgacactaagcaggccgatcaacaattacgtggtgccgttgtcttacctaatggaactggtaaggaacagaccgttgttgtatttgccaagggtgacaatgccaaggcagctcaagatgccggtgcagattttgtcggtgacgctgacttagttcaaaagatccaagatggttggcttgacttcgatgttgccattgcaacacctgatatgatggctcaagttggtcgtttaggtcgagttcttggacctaaaggtttgatgccaaaccctaagactggaactgttaccatggatgttgccaaagcggttaaagaatcaaaagctggtaaggttacttaccggactgaccgtgacggtaacgttgctgttccagttggtaaagcttcatttgataccgacaagcttgttggtaacttgaagacaattgaggatgttattgtgaaggcacgtccagcttctgtacgtggtgtttacgttaacaacgtttcaatctcaacaacatttggccctggcgtcaaagttgaccttgactcattctcaagtgttgaagcttaattagtttcgatttaaataaaaaatccctaattgacggtttattactttgtgtgatagactgttagttgctgatatattcgcctaagactcaggtggcttctacgccttaatatcctgccgaggaaagtaagtttacttttttcctatgtctgggtgggcatagggattttttattaagtcccaacaaatttttgggaggtgaaattcgtgagtgaacaaactgttgcgattaaagcaaaaaaggttgcatctgttactgaagaattgaagaatgcttcatctatcgttatcattaactaccgtggtttaactgttgccgaggtaactgatttacgtcagcaattacgtgatgaaggcgttaagatggaagttatcaagaacaaggtaatggaccgtgctgctgctgaagccggttttgatgatttgaaaccaactttcaacggcccaactgctgttgtcttctcgtcagaagatcctgttgcaggacctaagattgtccacaactttgcaaagactaacgacaaacttaagcttaagggtggcgttatcgatggtgaagttgccagtcttgaagaaattactgcttatgctgcattgcctagccgtgaagaattgttatctactcttgctaacattcttcaagcacctgtacgtaactttgcatatggggttaaagcaattgctgacaagaaacaatctgacgatggcgacgctgcctaatcagaactaaataaattccaattaatggaggaaaataaaatggcttttgataaagataatattattgaccaattaaaagatgcttcaatctctgaccttaacgacttggttaagtcaattgaagacgaattcggcgtttctgctgctgcaccagttgctgctgcaggtgctgctggtggtgacagtgctaccaaagattcatacgatgttgaattaactgaatcaggtgaccaaaaggttaaagctatcaaggctatccgtgacatcaccggtcttggtttgaaagacgctaaaggacttgttgataaggttccatcaatcatcaaggaaggcgcttcagaagacgaagccaacaagatcaaggaacaacttgaagccgttggtggaactgttacccttaagtaattcattatctaatcataattgttctcagaactgtgtatcgacattgtcgatgcacagtttttttgtgcacctttgttgtgtgaaattcaattaattggcataatagacgaagagtacatattcaaaatgaaatgatggtggaacaataatgacacgtgtcaaagaattcatcgacaaacggatgaccatgatcaagctgatttttgtcttctccgttttgatttttgttattcgacagttggctaagattatccgtgaagtcaacggtgaacagttcaaaaccgttctggccagtcaaagtcgcggcgctcttttgataatgctggtggcgggctttatttcaattctgccgatgctggtgtacgactattcaattgttcagttcttacccactaaattttcccccggctacatcgttaaaagtggctgggtggtgaatacctttacgaatttactggggtttggcggattgttgggcgccagtttacgcgcgcatttctatggcaaaggggccactcgcaaacagatcctctatgcgatttccaaagttgccttgtttctgatatcagggctttctttactctgcttggtttcactgatcatgatctttggctttgggatcgggactgaatttgcccactattggatttggctattaggcggtgccgtgtattttcccggtgtgatgatttttacccaagtgactaattcacagtttttcagtgacctgtcaaccaagcaggaactggtcatgaccgccggctcgttccttgaatgggggagtgcactggggttctttattttgatcggttatctcatgaatctacctgttgacctccgattggttgtgcccatttttgtggttgccaacgttgccggagtcgtctcgatgatcccaggtggattaggatcctttgatatctttgtcatcattggactgggattcattggtgttgcccgaagtgatgcgctggtctggattctgctttaccgtctgttttattacttgttaccgttcattgtgggcaccggtctgttcattcacgatactgggtccaaactcaacacctttcttgatgatctaccacggcttctgtttcaacggattgcccaagtcttcttaactggctttatgtatttttccggaattatgatgttgttgtttgccacggttcccaatgtagtggttgttaataaactgtatgtcaaactattgccatattcgatttttttcgtcagtcatatgatgaatattatcgttgcattcctcttaatcggtttggccagtggtatctggactcgaaccaagaaggcatatgcccctacggtatttgtactgattatttcgatatttaacacatggtttaacgaggcgtttacctggcggatggtcttgctgttcgtgatcatcctaatcactctgcggctctccaaggcggtgttataccgggaccggatggctaattcctggggtgtgttcctgtttaatgggtcaatttttatcatcacatttgcaatttataccctcatcgggattgctgccaatcgaaatcttcatctccattttgataaagcctatctttttccatctgcgggtgcctggctggtcggttttgttggcttattgatcgccctggcggttctggttggcatgaatgcctacttgactgccggtcatccagaatggctgacacagcgatttgatgccgatcgggtgaaggctgtgattgataaatttggtggcaatgaggatagtcatctggcattcttgcgcgataagcagatttacttttacagcaaagacggcgaagatcaggttttcttcatgttcaagaaaattgctgacaaactgttaattatgggcgagccggttggcaatcgtgcccaatttgccgacgcgattgatgattttgtcaaggaagctgacaaatccgatctgaagctggtattctacgaaattgatgaagaattaaccatgagccttcacgaaaccggttttgactttatcaagaccggtgaggatggattagtcgacttggatcagttcaccctcagtggtaaacggcatcgcggcgaacgggcattgatgcacaaattcgatcgcgaaggctaccagtttgagattctgcagccaccgttttcagatgagttactggccactctgcggaagatttctgacgagtggttggataataaagcagaaaagggtttctcactcggcttttttgacgaatactaccttcaacaggcgccgattgctgtgatgaaagaccatgccggcaaaattgttgcgtttgccaatctgatgccggatggtaataaagtggtcacctcgattgatctgatgcgttcctccgccgatgccccatcaggcatcatggatggcattttgattaatctttatgaaatatcccacgataaaggatacaagtactttgacttggggatgtcaccgttctcgaatgtgggcacttcccgcttcagcttcactcaggagcggattgttcatctcatctatcaatacggttataagctttatagttttgagggactccggtcttataaggacaagtacgttgataagtgggagtcaaaatatattgcgtattatcgtcgaagcgggctggtttacgcggttctgcagattatcctggttgttaatcaaccgcgcaataaaaagccggcaggcctctccaaggctctctggtacattatggacgccaatcagcccaaataaggcggactgagtcgaaaattaattgattgtcggttaagtaacctggcaggcaatcgcattaaacagcagccggaaggtatttaacagatatctgccggcttttttgtgcggttaaatgtaaaaataccaacaatttttcatcaaaataatgtttactgaaatttaccttgatataagaggctttgtttggaaaccgatgaagcgttttcataaaaaataatccacattcacgaagtcttccccaacatccaagtggttcaatcatatcaaggattctcaattgtattttacaagtgagggaattgtgaagttaaggttgacaacgctgccaaaatgagttaaattttggttagtaaagtttactaaaatatatgtagagggatgaaatttatgatttctgatgacgtacaaaagctatttaatgacaagtttggttatgactcaagcaaagtatttttctcaccaggtcgaattaacctcatcggtgaacacactgattataacgggggccacgtatttccttgtgcaatcagcatgggcatctacgcagcttatggagaacgccaggataacaagatccgcatgttctccggaaacgtttctgatgctggaattgttgaagtatcgttggacaatttggcatataacaaagaagatggctggacaaactatccaaagggcatgcttgttcagattctcgaacacggctataagattggccatggttttgatctcgctgtttatggtaaccttccagatggtgccggactatcctcatcagcatctattgagctgttgactgcagagattgttaatgatgtcttttcactggggatcgacgaacttgacctggttaaatatggtcaactggttgaaaataaatatatcggtgttaattccggtatcatggaccaatttgccattgggatggggaagaaggatcaagcaattcttctggacacgaataccctcaaatatgattacgttcccgctaaattgggagatcgggtcattgtgatcatgaataccaagaaacaccgtgagcttcaagattccaaatataatgaacgccgtgctgaatgtgaagaggctttgaagcgtctccaagtgggattgccaattaaatctcttggtgatttgagtgaaagcgaattcgatgaaaatagttacctgatcaatgatgatgttttgattcgtcgtgcccgtcacgcggtattcgaaaatcaacgaacccttcaggcaaaggatgcgctggtcaataatgacttggaaacctttggtaaattagttaatgcatctcacgtttcactgcattatgattacgaagtaaccggtaaggaactggatacattagctgaaactgcttggaaacaaccaggcgttgtcggtgcgcgaatgaccggtgccggatttggtggttgtgcaattgcgattgttgaccgtgatcaagtcgatgcctttaccaagaatgttggcgaagtctatgagaaagagattggccatccggcagaattctacattgcagaaatttcagatggtcctaaagagattaagtaacgaattgattagaaggaggatatttaaatggcaattttagtactaggtggagcaggatatatcggttcgcacacggttgatcgattaattgaaaatggctatgacgttgcggtggttgataatttggttaccggccataaagcagccatcaatcccaaggcccgtttctatgaaggtgatgtccgtgacaaagactttatgaatcaagtctttgataaagaagagattgaaggggtcattcacttcgcagcattctcagttgttcctgaatccatggaaaagccattgaagtactttgacaataatactggtggcatgattagtttacttgaagtgatgaacgcccataacgttaagaagatcgtcttctcgtcaacggcggctacctatggtgaacccaagcagattccaattaaggaaactgatccgcaagttccaaccaacccatacggtgaaagcaagttggcaatggaaaagatcatgcactggagtgatgtggcttacggcattaagtttgtcgcccttcgctactttaacgttgcaggtgccaagcctgatggctcaattggtgaagaccaccaccctgaaacccatttggtccccatcattttacaagttgctgccggcgaacgtgatgagttgacgatttttggtgacgattatgatacgcctgatggcacgaacgtcagagactacgtccacgtgcttgatttggccgacgcgcatatcttggcactgaagtatctccaagctggtcatgatagcgatgcctttaacttgggctcatcaaccggcttctccaacaaacaaatgttggatgctgcccgtgatgtgactggcaagccgattccagccaaaatgggtccccgtcgtgcaggagatccaagcacgctgatcgcagcgagtgacaaagcccgcaagattcttggctggaagcctcaatttgacgacgttcacgaaattattaagaccgcctggaattggaaagaaacccacccaaagggctatgacgatcggaaaggaaatcagtaatcatgagccaatcagcagttgaaaagtttgtcgatttaattatcaaatctgattcaccatattcagatgttgaccggatttatgtcaccaacctgatttttagactgatcggtgatggttttggagagccaaccgaggattcatcggctgtcgacttagccaacgatctggtggatctcgccattgaacatggtaaggtcgaagattcgattaccaacagggagattcttgaagatcaactgatggacctgttaacaccaattccatcaactttgaatcagatcttttggaacaagtatcaacaatctcctgatgcggccaccgactacttctatcatatgagccaagacaatgattatattaagactcgggcgattgccaaaaatatttcatatgaaactaaaactgattatggcaatctggaaattaccattaacctgtcaaagcctgagaaggatcctaaggcgattgctgccgctggccgggcaaagtcaaccagttatccggtcggcccgttagccattgaaaatgaaggctatctcggccgcctaggctatccagcccgaagcaatcaccgggttattcggatgatgatcaacggcgaaccgtggggattccaatactcaccttatgcatactttggtgagcatgcgatttttcttaaccaaaagcacgtgccaatgtcaatcgatcaacggacatttgtcaatttggttgacattatcaagcagtttccacattactttgtcggcagcaacgccgatttaccaatcgttggtggttccttattggcccaagatcactatcaaggtggtcgccacacgttcccgatgatgaaggccaagattgatcgaccagttgatttggggattgacggcttgtcggcaggaattgtcaaatggccaatggcaaccattcgcctggtcagcaaagatgccaataaagtggtgaatgctgccaatcggattgcagaaacttggaagaactactcagatgagtcagttgacattcgggcctacacggacggaacgagacatcatacggtaaccccgattgcccgaatgaatgatgaccagtttgagatggatattgtcttgcgggacaatcaaacttctgacaagtatcctgatggtattttccatccccatcaagatgttcaacacatcaagaaggaaaatattggcttgattgaagtcatgggccgggcaattttgcctgctcgtctgaagaccgaaatgaaagaagtcgaaaagtatgtcttgggtgaagataatcagattgctgattatcataagccttgggcagatgaattgatgaaacgtgaccactttaccaaggacaatgttgaagaggtagtcgaccaagaagttggcaaagtctttggcagggttctggaagatgccggcgtttacaaatgggacgacaaaggtcaagcggcctttgatcgtttcattgagcaacttaaataatttggaatagggttggaaataagcgtccttgatttccagctctatttttattgtcaaaagggattcactcaactttggcctctgcaggtgggcttggattttgtttcaacaattatttttggtaaaatggaagcggaaccaaatttaagctgaaatcactaggaggcaactatgaaatttattgtatacaatgtccgagatgatgaaataccgtttattgagaagtggggtaaggatcacggaattgaagtgaaatacaccaccacaactttgaatcaggagacggttgaagaagcagccggctttgacggtatttcctgccttcaaacgattcaatattcagctgaattatttgagtcatttaaacgcttaggaatcaaatacttatcgctcagaaatgtcggggttgataacattgatttaccagccgctaaagccaatggcgttaaaattaccaatgtgccggcgtacagtccagaaagtattgctgaatttgcagtgatgatgtcactgtacctctctagaaaagtgggctatatgcgtcagcagttggatcaaaagcatgaatttcatttttcacccaacttcatgggccgtctgatcagtgaacagaccgtcggggtgattgggaccggacggattggccaggcagctatcaagctgttcaaaggcctgggggcaaaggtaattgcctatgacaagtatccgctgaaaaataccgacaattcgtttgtatatgccaaaagcttggaacaaatttatcaagaaagcgatattatctcaattcatatgccggcaactgatgataattatcatcaatttaaccatgaggtgtttgagcaaatgaaagatacggcaattctcatcaatactgctcgcggttcaattgtcgataccgatgatttgatttttgccctccagagcggtgaaatcgctggtgccgggattgatacaattgaaaatgaatctgctgatctccaagactccaggtccaccaaaaaagtcaatgatccggatgtattgaagatggcgttgatgccaaacgtcttgattacgccacattccgcattccataccagtgaagctgtgaaaaatatgattgatatctcactggggaatcttgagacgatggttaatggtaagacaccaaaggatttggttgattagtaattgttaaagacaaataaggctgatgcatccccgctgggatgcatcagccttattgagttactgtgaggtatttatttaaatatcgtaatctgagtctttcatcgactccacgttccccaagaggtagccattaccaacttgtgagaagaaatcgtggttggcagtcgatgttgagattccgttcatgaccactggattgacatcttctgctgtgtctgggaagagcggattctgacccaaattcatcaacgctttattggcattataacgaatgaaggtgaggacatcttctgtccagccggtttggtcgtacagaatatgggtgtacttttcttcgttaccatacagtttgtacaggaagtcatagatccagttcttcatgtcttcttgtttttcctttggcaattgattgtagccaatttggaatttgtatccgatgtaggtgccgtggactgattcgtcacggagaatcaatttaatgatttccgccacatttggaatcttgttgtggccaaggtaccaaagtggggtatagaagccagagtagaacaggaaagtctctaagaagacactggcaacctttttcttgagtgggtctggttcattggcataaatgtcgcgaattttgagtgctttgttctgtaagaattcctcactgtcactccagtcaaaaatctcatcgatttgatcaggggtgttgagggttgaaaagatcgaggaataactcttggcatgaaccgattccataaattgaatattgttcaaaacggcggtttcgtgttgagtctgaacatctttccgcaacgatgccattccttcttgggactgcagtgtatccagtaaagttaagcccccgaagacgtgaccgacaacccactgatgatcttgatccagcgtccgccagtccgataggtcgtttgacaggggaattcgggtatccagccagaattgctcggtcaatttttcccaagtggccttgtcgatttggtcatcgatggcgttccaattaattgctttataattctcagtcatgaatttctcctttaaataacgcagctttcacattcgttggaaccaacttcttgttgatcgtccgtgaaagttcgaatatagtaaattgacttgacgccctttttgtatgcgtagtttctcaagatattgagatcccgggtcgtcatcttgtctgtccggccgtttttccattcatacagaccttctgggatggttgaacgcataaagagggttaatgccattccctggtcaatatgctgctgtgcggcagcatagatgtcaatcaccttacgcatatccatgtcataggctgaagtatagtaaggcattgtgtcatttgaaaggtatggggctggataataaatcttaccaatcttggattcctgacgctcttcaattcggttgataatcgggtgaaggctggcagtcgtatcgttaatgtaagaaatagaaccgtttggcgcaactgctaaccgattttggtggtataggccgtctttcatgactgattccttgaggttttcccaatcttccttagttggaatccaatcgtctttgaacaaagcttttacttcggcagattttggtgcaaatgatccgtccagatatttgtcaaaatagctgccgtcagcgtacttgctgttttcgaagttaacgaaagtttctttgcgttccttggcgatcttgttagatgcaactaagctccagtagtttaacagcatgaagtagacactggtaaattcaatggattcaggcgagccgtagtacatatggtgcttggctaagaaactgtgtagtcccatgccgccaaggccaattgaatgtgattctttattgcctttttgaattgaagggaccacgtcaatgttggagtggtcggtgacaaatgttaatgcccggaccatgctttcaactgaatggccaaagtcatcgccagccatcatattgttaatgttggttgatcccagattgcaggaaatatccttgcccattttgatgtaatgctgctggttatcaacagtggatggggtttgaacctggaggatttctgaacataagttactcatcacaattcgaccggcaatcggattggagcggttggcagtgtcaatattaatgatgtatgggtaacctgattcttgttgcagcttactgatttcagtttccaaatcacgagccttgatcttctttttggagatcttgtcattggcaaccaaattatcatattccttggtaatgtcgacgtaagagaatggcacgccgtattcgcgttccacatcataggggctgaataagtacatgtcagcatcggctttaatcaattggtagaacttatcgggaacggtcactcccaatgataaagtcttgaggcggattttttcgtcggcgttttcctttttggcacccaaaaattcgatgatgtctggatgaaagactgagaggtaaacgactccggcaccttgacgctgacccaactggttagagtatgaaaagctgtcctcaagcaatttcatcaccggaaccacaccggaagcggcaccttcgatatgtttgattggggcaccggcttcacgaagattggaaaggttaattccaacgccaccgccaattcttgacagctgcagggccgaattaatcgtccggccaatcgtattcatatcatcggtggtttgaatcagaaaacaagatacaaattcgccgcgattttcccggccggcgttcaagaagcttggtgtggccggttggtaacgctggtggacaatttcgtcggccaaatccattgccaactgttcatcaccgtcagcgaagaagagggcgttagcggcgacccgatccaggaagctttccagatataaatcattgtcgttggttttcaaagcatattgggcgtagaatttgtaggctgccataaatgatttgaagtggaaatcctgatcgtttaagtactggtacaatttttcgataaaggatagttgatatttatgaataaaatcggcttcgtaatagttgtttttgatcaggtaatcaaaccgatcgctgagactgtcaaacttcattaagtttggctgaacgttttcttttaaaaaggcttcgagggcttccttgtccttttgcagtggaatctgcccgttgacggggatgttaatttcgttgttcaaatcaaagtaggtaacatccttaaggttgtgaagtgacatatttagtaccacgctttcttataattgcgaataaaaggggcgagaccgtttgtggtttcgcccgctaatctgaaatcaatatgttagaatggatgaaggcaattagccggcaatcgattggagctgatcaggtcgaaagccgctgaatgcttgcttaccatcaacatcgacaacggggacagccatgaaccctcgttgtttcaggtaatcaatatattgtggttgctcgttgatgttgtgttcctcaaattgaacgttatgttctgaaaggtaacgttttgtcattttgcattgcatacagttgttctttgaatatagtgtgattttagccattgttaacacttcccctgtttcgttaaaatttaatttatgattcaagtttacactaaatagtgtgaaatgcaacgattaaaacacaatatattgtgacaaaactaattgtaagcaccaaatatagataacgattataaaagatcattttaggagaattttatgtcagaacaatcattttattattcaaagaatcccaacgtgaaatccgatccgattacatggaactttgcgttgcttggaaacaacttagtgttcacttcagataacggtgtgttctctaaacatacggtcgactacggcagtcgggtgctggttaatcatattaattatgatctcattcctgacggcaaactgttagatatgggaaccgggtacggtccgattggcatttcaattgccaaagcatttccggatcggcagattgatatggttgacgtcaatgaggtggccttggcgcttgccaaaaagaatgccgacgccaatcgggttgataacgttcatatttttgaaagtaacatatatgaagcgattactgatcagtatgctgccatcgtgaccaatccgccggtgagagctggcaagaaagttgtcgatgccatgatctccggggcagtcgatcacttagttgatggcggcaccttgacggtggttcttcaaaaaaagcagggcgcaccatctgccaaaaaattaatgaccaaactatttggtgactgtcagattttaaaacgggacaaaggttactacattcttcaaagcatcaagaaatcgtgagggttcgaaatgtttcaagctgatagtcgttttatgaaagctgcactggtcgaagcaaccaaggcctacctaattggtgaagtgccgattggcgccgtggtcgtccatgacgggacaattgtcgggcgtggtcacaatctaagagaacatttaaatgacggtacggcgcatgctgaaattttagcaatccaagaggcttgtcgaacactgcggagttggcggctgattgattgcgatctttatgtgacgattgaaccgtgcttgatgtgtgccggagcgattattaattcgcggattgaaaatgtttgttttggctctcgtgatcccaaagccggcgcaaccagaagtttgtacgcagtgttggaagattcccgattgaatcatcaagtcaacgttgttgaagggctttatgccgatgcggcatcgcggatcatgaaagatttcttcaaggctgcgcgcaagaaaagaaagaataaggctggcaattctgaatcatttaagttatgatagatattgccgcaaggccctgaggcaagggtcgggttacgaactgtgtcaggtccggaaggaagcagcactaagtatcatcaaccttgtgcctcttgtacatagaacttttgctctcagcaactttgctgagggcatttttttggagaaatttcttgaaagtcagacggtcgttgattgcactctggttagattcatcatataattatttagacgtttcattgaacgattttaagaattcggcattctattttggaggatttggtaatgagctatcaagcattatatcgggtttggcgaccacaaagatttgatgaaatcgtcggccagtcgattatcaccagaacattaaaaaatgcgctaattactaaacaaacgagtcatgcctatttgtttaccggtcctcggggaacaggtaaaacttcggcagccaaaatttttgccaaggcagtgaactgtcactacttaaaagatggtgagccctgcaaccagtgcgagacttgtaaagcaattaatgagggcagtttaaatgatgtcattgagattgatgccgcttccaacaacggtgttgaagaaatccgggatatccgggacaaggcgaaatacgcccccactcaggctgattacaaagtttacatcatcgatgaagttcacatgctttcaactggggctttcaatgccctgctaaaaacgctggaggagccgccggctaacgtaatttttattttagcaaccactgaaccgcacaagattccggcgacgatcatctcccggacacaaaaatttgactttaagcggattaaacctcaggatattttggaaagaatggaatatatccttgatcaaaaaaaggttgagtacgacgacaaagccctgaaattaattgccaaagctgctgagggcgggatgcgggatgccttgagtatcctcgatcaggcgatgtcttatggcgataataaaattacttatgagaacgccttacttgtgaccggcagcgtgaccaatgaattattaaccacctatatgcagcaggtggtcaagaaggacaccaaaagcgcgctgattaccattcaaaaaatattggatgagggtaaagacgctagccgattcattgaagatttgaccagttactgtcaggatattctgttatatcaacaggatcccggaatcgttgaagaaatggaactagggatcattgatgaccagttcaaggccttaagcggccagatcagcgatcaagcgatttatcagatgattaatgaattgaatgcgatttctaattcattgcggtttaccgctcatccagatgtttatctggaggtcttgacggtcaaaattacccatttggatgccacaaatcagcccaaggctgtttcagccccacaatcacagcagtcggctaaaacggccgtgcccccggaagttaatgcggaaattcaacaattgacgcagcaagttgccgaactcaaggctgaagttgccgatctcaaacgggagtcgacacctcagtcaccaacagtcagcacaccggagcctgccaaagtcagtgaggctcactcaatggacaatcacattgagctggctaaaatctatccaattttgggtaaagccacccggaaacaattaaatcaatttaaatcggtttggccggacttgatggatgccctgtcggtgactcaacgggctgtcatgcacgtgtcatcgccggtggctgccagtgccggcggagtaatcgttgccttcgaatacccatttttgtatcagaaggctcaaggtgacactgatttgaaggatgctcttgaaaacaatttggatcgcattgtgggaaaagcccctcaaattgtgtttgttccggaaaatcagtggcccgatattcgccgtgagtatttggccagtcacaaagacaagataaaaaagactggctcccagtccaaagaagcaaacgacccaaaagctgaaccggctgatgacgatccggaaccgtcaaaagaagagccggacagtcaaccagtcgtcaagaaggctgccgaacttttcggcaccgacattttagatatcaaagatgattaattggaggaaaagaaaatgatgaacggtatgaacatgaacaagatgatgaagcaaatgaaaaagatgcaaaagcaactgggtgaagagcaggagaatcttaaacagcaggaatttaagggcgttgcaccggataacatggttgaagtgacttttggcggtgacaaaaagatgaaggatatccagattaagccggaagccattgatcccgatgaccccgaaatgttgggtgatttggtattagccgctgttaatgatggcctttccaaggttgataaagcgactgaaagcaccatgggtaaatacaccaaagggattccgggaatgtagtctgcacgaaaaaaggggaaagtatgcaatatcctgaagcaattgcaaagttaattgatagttatatgaagttaccgggaatcgggagtaagacagctaccagacttgctttttacaccgtcgatatgaatgaagatgatgtcaaagcgttttcaaaggcgctggttgccaccaagaacgaccttcattactgttcgatttgtggtaatctaaccgatgaagatccctgtgaaatttgtcgtgataaaacccgtgatcaatcaaccatcctagtggtggaagaacccaaagacgtgatggtaatggaaaaggtccaggagtaccacggcctttatcatgttttgcatggggtactgtcaccaattgaaggcaaaggacctgaagatcttaatatcagctcactgatcaaacgactccagcaaaataaagccgttaaagaagtgattgtggccaccaatgccaccccagaaggcgaagcaactgcaatgtacttgagcaagttgattaaacccgctgggatcaaagtgactcgtttggctcacggattatcagttggatcagatatcgaatatgctgatgaagtcacgttgtttaaggcagtccaaggacggactgaaatttaatttgacaaggtggggttttcgaatgttttttaatcgattaagacggcaaaatgttaaacgtgaatacgacgatcgcttgttggagttaatcaacaatttgaaagaagagtgggatcatgctgctcaaacccaagaagcggttgctgacagtgatatggagatggagcaggaaactgcgttggcccgtcaaaaatatttcttcatatataaagaggcacgaattcgaaaaattaagaattaccaaattcagccctcggttatcagttatgatcatgacaattttgaataatccggaccacctaagcgttggctgaatcgacaggcaaacgaacagcaagtacaattaatttaaattaaaagtgagggaattgttttgaatggtaagtttataacctttgaagggccggacggcgcaggcaaaacttccgtgatgaatcgcgtgattgaagtttttaaccaggaaatcggcgatcaactcttggtcacccgagaacccggtggcaataaaatctcggaagaaatccgcaaagtcattctcgaccgtgagaatactgagatggattatcgaacggaagccttgctttatgcggccgctcgtcgccagcatctggttgaaaccattttacccgcactcaagcagaacaaattggttctgtgtgatcgttatgttgacagttcagtagcttatcagggggccggccgtcagatcggtatggcacaagttgccaagatgaatgagtttgcaacggaaaagttgttaccgttcaaaacgatctactttgatatcccggttgacgttggcctggatcggatcgccgaacaccgcgaccgcagtaaaattgaccggttggatgttgaaaccaatgaatttcataaacgggttcatgagggttatatgaaggtccgtgacgaaaatgccgaccgatttatcagtattgatgcaactcaaccgattaatcgcgtcgttaatgatacaattaagattatccaccaaattgccagtgagtattttaaggagagttgattatgaaattagtcattgcgatcgttcaagacaaagatgccaacaagttgcgatcagttttcgttgctcacgatatcatcgcaacccgattctcgaccaccggtagctttctgcgagcaggaaataccacttatttggtcgctgttgatgattcaaaagttgatttaactttgaaactaatcaaagaaacctgttcggctagacaacaatttatgacaccgccggtcagcttgaacggtgatacggcagaacatacctttccaattgaagttcaagttggtggtgctacggttatgattttgccaatcgaagattttaaacagttctagaagggaacgttatggaacacgatattgttaacgttgctcaaactaaacagccgaccatctttacccaattcatgaatttaatcaaaaacaatgaattgtcacacgcatacttgtttaccggcgaagatggtgccggccaattttcagtcgcaatgggagttgccatgcggcttttttgtacgaatgttcaaaatggcatgccctgtggaaaatgtgccgaatgtgtgcgaatcatgaatcatgatcatccggatgttgtcatcaccgaacctgatggtcaaagtattaaggttgaccagattcgccacgttaaaagtgaatttaccaaaagtgccatggagggatccaaaaaggttttcattatttcagaagccgaaaagatgactaccggggcagctaacagtctcttaaagtttatcgaagagcctaccggcaacgtggttagctttctgatcagtcagaatcgcaatctggttctgccgacaattatttccagaactcaggttgtggaatttcccagcctcagtaaaaagcagatggtccaagaattacagaatagtggcgtcaagccgagtgaagtcaacttgatgatttccattaccaatagtttggatcagattaaagagctgtccaaagatgattggtttgcctcgatgcagcggcttttggagaaatggtttacctatttggtcaaagaaaacaacatggcaatgcctttcatccaaatgtctttgatgcctctaattaccaacaaggaccgtcagcggattgttatttccatgatgctgagtttgtttgacgatgttttggaaatgaaatacgggactttggcggatgatcgggtgaagtacccggcgattcttgcacagaccaaattggcggccaatcagtggaataacgatcaactgttaaccatgcttgacgagctgcttgatatgaatagccggatggcagttaacgtcaattttcaaaacataattgaagctttgacactaaagatactcgcaattgggcaatcatagtttactaaagggtgataaaatcgtggacagtcaaaacttatatgatgaattaaaagaaatggatacacagctcagtgcgagtgctgaaaatttttctcacctgcatgaatcacttattgggttgatggaaaaaaacgctgagctggagattgaaaatcagcatttgcgcgatcggattaacgaaataaccgaaaaaatggacaataattcgccacgtttgtcaaagtctcgcaagaatctcgaaaaactgtacaatgaaggatttcatgtctgcagttcttattacggtaagcgacgggagaacggtgaagattgtattttctgtacggacattatctatggcaaacgcgattaagaggtaaacagtggacacacaaaagagttttgacacattaagtgaatatggcacgctgtacttggttccaacgccaattggcaatctggatgatatgacttttcgggcggttaaaattctccagtctgcagatttgattgcggctgaagatacccgcaacacacagaaactgttgaaccatttcgatgtccaaaccaagcagatcagttttcatgagcacaatactgccgagcggattcccgagttgattagcaaactcaagcagggaatcacgattgcccaggtaagcgatgccgggatgccgtcgattagcgacccgggccatgaattggtggttgcctgtattcgtgagcatattaacgttgtgccgctgcctggcgccaacgccgggatcactgctttaattgcttccgggcttttgccgcagccattttatttctatggcttcttatcaagaaagccgaaggaacagcgagcagaaattgatgagctccgtaaccgagaagaaacaatgattttttacgaggccccgcaccgattgaaaaaaactttgaagaatttattgactcagctcggaggggatcgtcaggcagctctctgccgtgagttgaccaaaaagcacgaagaatttattcgcggaacccttgatcaggtcaatgaatgggccaattcaactgaaattcgcggagaatttgttattatagtgtcaggaaatgcccatccacaaacgcagggagatgatccgcttgccgggatgagcgttgatcaacaagttgacttttacatcgaaaatggtttgagcgttaatgaagcaatcaaaaaggttgccaaagatcatcatttaaaaaaacaggtcatctataaccagtaccatgacatcaaatagaaagaagtaatgtccatgcctgctcacagttttagcgaattgcatacgattccgttttacgagtgtaacgtcaacaaccggatttcaattccaatgttgatcaatattttgattttggcgtccgaacaccagaacgaaaatttgggacttgatcaaacttatttaattgatcattatggagttggctgggtggttacttcttactcaattcatatcactcacttgccacgcaaagattcagtcgtcaaaatgacaacccgaggcacgtcatataatcgttattttgcctttcgggaattctggctgcacgatcaagctggcaacgagctggtcaaggtggagagtatctgggtgttaatgaacgaacagacccgcaaaattacaccgattgacgaaacgattattgcgccatatcagtcggagaaggtcaaacgggttcccagattggcacgtcctgaacgaattgaagcgactgatgatgttagcgcaaaggaataccaagttcgttggagcgatatcgattttaatggccacgtcaataattccaggtatccggagtggatgttggattcattgccaatggactttttgaaccaacacgaacccactaacattgacatccgctttgagaacgaggttaagtatggcaatcgggtcaccagctcagtgcttgttgattcttcagataatgctaaaattaaaacagttcacgaaattaaatcaaatgatgttctttccgcaagtgccacaattgtttggaaagatatcaaagcaaagggtaacgattaataatgaaaatcttagcaattaacacctcaaatcaaccgctttcagttgctgttttggataatgaccaacttttggcgcaaacaaccatcaccactcatcgcaaacatgccgaattcttgatgccggtcattgaagacttggtgcaaaaggccgatttgaagccaactgatttggatcgggtggttgtcgctgccggccctggatcttacaccggcattcggatggctgtcactgcagccaaaacgattgcaagcaccttgggaatcgaactggtaccagtttccagcttgttaaatcttgccttgaatgttcaagaagaagatgtgctgatcaacccgatttttgatggccggaatcaaaacatgtttactggattataccgctaccgaagtcgtcggattcaaaccgtgattgaggatcagcacaccaatctaacaaaatggttggaaaccgttagtcgttatgatcaacggattatcattttaggggataccgatccatttgaaagatcgatgcgcgacgttctgcataaccgtctggtggttgccaatccttatttgggaattcccagtgcgaccttactgggcttgtatggattgagtcagtcaccagtaccggtcgttgatgcggttgtcccacgatatttgcggttaaccaaggctgaggctgattggaaaaaattacatcctaatgaggatacgcatgactatgttgaaaaagtttaaagagtggtttaaccaacaattttataacaaagaggttcagcttcgcgagagatatctcgacatcaaaaaccacgatgttgaaattaatggaactgagtactttttggccaaggcgatgattccggatattcctgagattctagggattgagcgggcggtttacggtggtcagactccgtgggatgatcgggcctttcgaaccgaactgatgcgcaaaacggatcgcctctatttagtgttgcgtcgaaacgactggctggtagcgtttattggctgctcgctaaacgatcatactaaggactgtcatattaccaacgttgcggttgccccaaatttccagaatcatggcttggggtattttttggtgacaacaattatcaaaaaggcccgtcaattggaatatgccaaggtgacgcttgaagtgcgcgtcagtaacacccgtgcacaaaaattatatcgggatattggatttgttgataacgggattaaaaaagattattactttaacgatcgtgaagacgctttaaatatggttttggacatcaccaaaatcggttaaaagggatgggatgaattaagtggctagagatttagtacttgcttttgaaaccagctgtgatgaaacgtcggtcgcagtgattgagaatggcaatcgaatactttcaaatattgttgcaacgcaaatcaagagtcatcaacgctttggcggagttgttcctgaagttgccagcagacaccatatcgagcagataaccggctgtattggggatgcattacgtgaggcggacgtttcttatgatgaactgacttcagtggctgttacatacggtcctggcttagtcggtgcgcttttaattggtgttacggccgctaaggcggttgcctgggcgcacaatttgccgcttgttccagtgaatcatttagctgggcacatttacgctgcccggctggtcgaacccattgagtttccagcaatggccttggttgtttctggtgggcacacagaattggtttacatgcctgaggaaaaccaatttcaaattatcggcgaaactcgtgatgacgcagccggtgaggcttatgataaaattggccgggttttggggattaactatccggctggcaagccagttgatgaattagctcacaaaggtcaggatacttttcattttccacgggcaatggacgctgacgataattttgactttagtttcagtgggttgaagagtgcctttatcaatacggtgcaccatgctgatcaaattaacgagaaattgagtcgtgaagacttggccgctagttttcagcaagccgttgttgacgtcttggctgacaaaaccaatcgcgcgctcaaagaatttccggtcaaacaattaattcttgccggtggggttgctgccaatcaaggtcttcgggagcggttaaccaaagaggttgccgcgtttgccgataccaaacttgaattagtgccactgtctttgtgtggcgacaatgctgctatgattggtgctgccggtgagatgctgtatcggcatggtgttcgtggtgatgccactttaaatgcagatccgggtttggagtttgattggctggcagatgaggctaaataattgaccaattttttgaggtgattatgaaatcgtcagcgatcctgtgatgaaggataattcaataattagatcaaaagcagcctgagcagaaggataaaatccttttcctcaggctgctttttaatttagtgggttgtcgccaattggtaaagtagacgatgtgaatcggatatcttttgcctcttgtggattatgctactcactatcttcgagcttcaaactggccgtttcccaactggactcagtttctgtgatttgggcagtcacctgatcgagctgctgttgaagatcttgcaactttcccaggtcgttaaagacgtccggcttcgtcatttctgcttcaatttgatcctttgattgtgtcaattcatcaagtttggtttccagagccttgacttctctttcaagtttgcgatgttctttttggttttgcttattaatctcgtagttctttttatcggtggtcggcacggcaactggggtcggttggcccgccgccttcttttcagcctcatgagccttgatggcttcttgctcatcttttttatcgacataataatcataattcccaaggtaaagggtggtgccatgtcgggacaattcaacgaccgctgtggcaattttgttgataaaataacggtcatgggaaacaaagagaatcgtgccgtcgaattgattgagcgctttttccaacacttcgcggctgtcgatatccaagtgattggtgggctcatccaacattaaaaagttgttgtgctgcatcgccaacttggttaggagcaatcgtgccttttcaccgccggacagatcatggaccatcttgctcacgtcgtcaccggagaaaaggaagctccccagaatgcttctaatatcgccttccggggtcgttgggtgatcatcccatagttcctcaagaacggttttagaggcgtgtagtgaggcttgttcctggtcgtagtaaccggtatcgacgccagtaccaaactgcgccttgccctttaaaaacggaatgatgcccaagatgctttttaagagcgttgatttgccgacaccgtttggaccaacaattgcgatcgcttggtgacgtttaacgtccagattaaccggctcacaaaggaccgtactgtagccaaccgctgcgttggtaacgttcaggacgttattgccgcttttggattttggtgaaaatgagaagcgggcagtttttgaatcagccgtcggtttttgcagcttatccattttttcgagttgctttcggcgggcctgtgcctgtttggtggtcgatgctcgaacgatatttttttcaacgaaggtctgcagtttttgaatcttagcttgctgcttgtcatattctttccattcttggtcaatcaactggtcttttttcttggtgtagtccgtgtaattaccagtgaagtggtggagggtaccttgtgacatctcgtaaacctcagtgacaattctgtccaggaagtaacggtcatgtgaaatgatcagaagggcaccactatagttttgaatataaccttccagccaagtgatcgtttccacatccaaatggttggttggttcatctaaaattaataattcgggcttttccagtaacagtttggctaaggcaagttgagtcttctggccgcctgacaattcattaattggccgatcgtagtcagcttccccgaatccaaatccgtggagaacaccacgaatttcagcgtcgtacccataaccattgtgctgttcaaagtcggcacggatattgtcatattgtgaggaaatcgtttcatattcttcggtattggcgtcaacgcccaaagaacccatttgtttttccagagcgtgaagttttgcttcctgctcttttagactggcaaagactgatgccatttcagcataaatgcttttatctgaattgagtccggtatcctgggccaaatagccaatcgacagattctttttagtgctgatttggccgccgtcgacagattgttcgccgatgatcattttaaccagtgtcgacttgccggcaccgttacggccaaccagtgcgacacggcttttttcttgaatggccaaattaacttttgagaaaatagtttcgccattgaatcgtttggttagatcttgtgcttgtaagattatcaagtgtttggccacctttcattttgtaactaccaacaatcaattttatcataatttacacgatttcaggaattatttgtaagtaatatttgaaatatatttcacaagatgtcatcttatggtagaatgagatgtaaataggaattcacaaagttctcttaactaaaatgacaaataggaggaaattttcttgacagctgaaaatattccacgcgcaaccgctaaacgattgccgatatattaccgatacttaaatattttacatgatacaggaaagcaacgaatttcatcaacggaattggccgaggcggtgcaggtagattcagcaaccattcgtcgtgacttttcctattttggtgcgttgggcaagcgggggtatggatacgatgtggacaacctgctttcgttcttcaaaacgatcttgaatcaagagcatctgaccaacgtggctttgatcggagtcggcaatttgggccatgcgctcttgaactttaattttcacaaagacggcaacgttcgaatctccgctgcttttgatactgacgacaagattgtgaatacaattgaagacggtgttcctgtctacccgattgaggaactttcacatcaactgcatgatcaacagatcaaagtcatcattttgaccgtgccctcaaaagtcgctcagtccattgcggacgatgctgtcgccggcggggtaaagggtgtcttgaactttacgccaattcggcttcaggttcctgaagatgtcctggttcagaacgttgacttaactaatgaattgcaaactttgatttatttcatcgaaaactttggcaagtaaaatatcgaacaaattaatgaagaaaagaccggtgatcttgaaaacgccggtcttttcttatgcgttcatttaccgtcagcaaggcaatctgcagataaattcaccaagaaatgtgcagaaatccttgcaattggtctgaaaaaataatatattatacacagtgattagcacttttatcatgtgagtgctaatgttgctaaaaattgttgcaaacggagggactaacgtgttaaaaccattaggagatcgcgtaattatcgaaactgaaaaagaagaagaaaagtcggttggcggtatcgttcttgctgacaatgcaaaaaagaagccgcaagccggtacagttgttgccgtgggtgatggccgtgtacttgataatggtaccaaggttgcacctgttgtaaaaaagggcgacaaggttatgtttgataagtacgccggaaccgagattgaggataacgatcaaacttatctcgttcttcatgaaaaagacatcgtcgcaattgtcgaataattatattttaacgagataattgctaataagtgaatcatttgaatcattcaatgaatcaataatcaaaaatatttttttgaggtgaaatttgaaatggctaaacaagtaaagttttctgaagatgcccgtagcgcaatgctcaagggtgttgataaattagcagatacggttaaggcaacgattggacctaaaggccgcaacgttgttttggaacaaagtgccgggacaccgacaattaccaatgatggtgttaccatcgccaaatcaattgaattaccggatcattttgaaaacatgggcgccaaattggtttctgaagttgcttcaaagaccaatgatgttgctggtgacggaacaaccactgccacagttttaactcaagcaattgtcaatgaaggtatgaagaacgtcactgccggtgccaacccagttggaattcgtcgtggtattgaaaaggctactaaagccgctgttgatgcccttcacaaaatgtcgcatgatgttaagaccaaagacgatattgcacaaattgcttcaatttcatctgctaacaccgaagttggcaaattgattgccgatgcaatggaaaaagttggccatgatggtgttattaccattgaagagtcacgtggtgttgataccagcttggacgttgttgaaggaatgcaatttgatcgcggctacatgtcacaatacatggttaccgacaatgacaagatggaagccaacttggacaatccttacatcttggtaactgataagaagatcaccaacattcaagacattttgccattactgcaaaagattgttgaacaaggtcgttcactcttgatcattgctgatgacattggcggtgaagctctgccaactcttgtattgaacaagatgagaggaacattcaacgtcgttgctgttaaggcacctggatttggtgatcgtcgtaaggatcaactccaagatatcgccattttgaccggtgcaaccttgattaccgatgaccttggtttgaacttgaaggatgcaacccttgaacaacttggtcaagctaacaaagttaacgttaccaaggattcaaccacgattgtcgacggttccggttcaaacgatgaaattgccaaccgagttgctgaaattaagacccaaatcgaaaagacgacttcagactttgaccgtgacaagttaaaggaacgtcttgccaagttatcaggtggggttgccgttgttcgtgtcggtgccgctaccgaaactgaattgaaagaaaagaagtatcgcattgaagatgccttgaatgcgacccgtgctgccgttgaagaaggattcgttcctggtggtggaactgccttgattaacgtcatcccagaaatcgccaagttggatgccgaagctggcggtgatgaagagactggtattcgcattgttcttcgtgcccttgaagaacctgttcgtcaaatcgctgaaaatgccggtgttgaaggctcagtgattgttgaaaagctcaaggacgaaaagcctggaattggctacaatgctgccaatggtaaatttgaagatatgatcagtgatggaatcgttgatcctaccaaagttacccgttcagcacttcaaaatgctgcttctgtttcagccttgttgttgaccaccgaagctgttgttgctgatgagcctaagaaagacgcaccagctgctccaatgccacaacctggtatgggcatgtaatgaagcgttaaatcgttgatttgaatgaaagtattgtacaataagcatcgattccaaatcgggattggtgcttattttgtgcttgcgaattaatcaattcaatattaaagtagttagcatgtggcttagatcatattttgactctgagtgcacagctgacggatattttagcttgtctggatggtgatttgctgtgagcccattcagacgtacatatcaagacttgtttttaattgtcagaaggactatcattttatggttcacaagaatggtagattattaaataaaggagtaactatttatgtggcgctatctcaaacggctccttattggaaagccattaaagaccactgatgagggtggtcaatctttaaccaaatttaaagcactggctttactatcatccgatgcgctctcgtcagttgcatatggtactgagcagattacgaccattttaattacgctgtctgcagctgcgttgatgtatcaaatttgggttgcagccctcgttttggttctgttggctgccattactttgtcataccagcaaattatccatgcttatccctctgggggcggtgcctacgtggttgccagcaccaactggggtgagcaggctggcctgattgccggcggctcgttgctggtcgattatatgctgaccgtggccgtatcaacaacttcagcgactgaagccattacatcagctattccgtcattatattcacacggggtgctgatttcctgtttgatcgttgtgggcattatgctcctcaaccttcgaggaatccgcgaatctgcttcgtttttgacgttgccagtgtatttgttcatcatcatgattatcgcgatgatcatttatggcggttataatattgtgaccggcaacatcgaatatcatgcggctgctcatatcggggcacctgtcgaaggcatgactttggtcctgttcttccgggccttctcatctggatcatcttcattgaccggtgttgaagcgatcagtaatgccgttcccaattttaacaaacccaagagtaaaaatgctgcggcgaccttagccatcatggcgaccatcttggcctgcttctttggcgggattaccttcctgagttactacatgggcattatgccaaacagccacgaaacggtcctttcacaaattggtgaaactgttttcggccatggcattgtctactatatcctccaattatcaaccgccatgattttggcggttgctgccaacactggattctcagcatttccaattttggcttataacttggctaaagacaagttcttacctcatgcctatctcgacaaaggggatcggttggggtactctaacggcattatttccttagccgttggtgcaattgtcttaattcaaatttttggtggccggaccaattcactgattccattgtatgccgtaggtgtgttcattccatttacgctgtcacagtccggaatgattatccattggcggagaaatcggggtaagaattggcagctgaagtcagttatcaacttcgtcggcgcctttatttcactgacgttggttacctgcctgttcttactaagatttccaaatgtttggccttatttgattgttatgccgattcttttgaggattttctacaagatcaatcatcattacaagcgggttgccgaacagctgcgggtggttgaagagaatactgaaattgcgacaactcatcactttgacggctcgactgtcattgtcctggtaagcggggtcactcgggtgactgccaatgctatcagttatgcccaatcgattggtgattatgtcatcgcaatgcacgtttcttttgactccaaccctgagaaggaacacaagacgtctgagcagtttaaaaaagatttcccggatgtccgattcgttgatattcattcatcctatcggtcaattgcccaaccaaccttacgtttctgtgatgtcattgccaagcgggcagctgatcgaaactattcgaccacagtcctggtaccgcaatttgtaccaagacatcgttgggaaaatgtcctgcataaccagactagtttgagattaagagcaattttaaattcacgacaaaatattattatttccacttataactaccatctgcgtgagtagttaaatgaaacgatacaggccatccgttaagcaatagcggatggcctgttttagcgtgtttttaaccgcctcgtaccggttttaccaggattgtgggcaattatcttggaagagacgaagggtgcgtagggaagggataatttggtttgagtagtcgcttagctttgggaaaaatatgtaaacaaaaagaccgcccaaatggacgatcttttgatctcgcaaggaattagtgagcgattcccatgaagttggcaaatgttggaacaacgatgtcaacaacgattgaaatgataacaaccgcgatggcagccatcgcaccagatacagaacttaactgaatggcctttgctgaaccaacagtatgtccggcagtacctaatccaagaccttgaccaatcggttcagtcaagtggaatatcttgatgagccatgttgccaaagcgtaaatcaagacggcgttcaagatacatgccatagcagtaacggcaggagtacctccgatagcaccagaaataggcattgcaatagcggtagtagcagcttgtggaagcattgaagcgattccgttgttgttcaagccgatgagctttgatacatagtagatgatgaacagtgagatgaacaaaccaataattaatgatagcagaatctctaaccagaatcgtttaacaatatcgttacgtttgtacagaggaacggcaaacgcgatggttgctgggttcaagaaccagaagatgatatctccacctggtttgtaagcgttggtgtagaaccaagtaacgtcaacaccgaacatcttagccatcaaccagaggatgaagattccaagtaccattccaacaaacagaggttggaataagaagaatcctttaccaatcttgaatagccattgaccaaacaagaaaaccaacagtgacaagcagataccaaaaattggtgtccctaaatacgcaataatagttgtttgtgtagcagacatttatattcacccctttaattactttttctcgacgtcttcactaactgtaatatcgccatggaaaacggtctttctgatccagataaagaatgatgtggtgtaagcaacaacaacaagtaagacaaccgttgaaataataatagcaacaataagttgtacaccttgagccttcatgatatcaagagatgcggtcaattgaattcctgaaggtacaaatagaaatgcgatcattccgatcataaatgtagcaaatttatcaacccattcaactttgacgatgtggaaagttaataggagataaagaataattaaaccaagaactggggttggaacagggaactttggtgcgactgctaccaaccatgctgaaattaaactggaaacaaacaataccccggcgaagatacccatttgaataagaatgggcgcatctttcgtctcggcttgtgtagtatttgttttgtcagccatgataaaaactccttccgtttgtgaaatataaaataattgaacctgttgtcttacaatctctagtataaatgtttttgtgaaatatgacaattgaaaacgttagcaaaatttaaaaatgtgaaaattcacacaattggtccgtattaattatttgagtaagctcctttactttgtgagtcagacataccttgtttttatgaattgtcatttgtataattgaattaatattgatttggaaggaaataagtgaggttacaattttgaaattcgagatcattgtgtctttatttgctaccatgattatttctgcagtcttaaccccatttattcggaaacttgcttttgctgttggggcagaggaccggccaaacaaacggcgggttaataaaattccaatgccaacgattggtgggttggcaatttttattgcctacacctttacgaccatgattttattgcgggatcagttcccaaccaaaattttgtggggggtgtatggcggggaagtcatcattattctcactgggataatagatgatattttcgtcttaaagccccggcaaaaagttttggggatttcaattgccgcgctgtgggtttactttacagccggtgttaaaatgaccaccattaccttaccgtttatcacaatccaccttggttggctgagcttgccagtgacttggatttggattttggcaattaccaacgcggttaacttgattgatggattggacggcttggccactggggttgcaattattgccctaaccaccatgggaattaccgccatgttcttcttgaacgtcggtaatattttcgtcgccatcatgatttttaccctggtggccgcttgcattggctttttgccttataactttttcccggccagaatttatttgggcgataccggtgcgttgtttattgggtttatgatgtcggtcttttcgttgtttggattaaagaacgccactttcatcacgctgctaatcccagtgatgatcctgggtgtgccgattaccgataccgtatttgccattttccgccggttgttaaataaggaaccgattacgcatgccgataagcgacatttacatcaccgtttgatgcaaattggtttgacccatcggcaaacggtgttggtgatctatggaattgccctgattttttcgtttatctcactgctttatccgatttcaaccttgtggggatcgattctgctgacgattgccgttttgattggtcttgagttgtttgtggaaacgattggcctggttggagaagatcgacagccgctgttgaacggaattaagaaattggttaaagatacgaccagtaaaaataatcattagcgcattaaaaagccgtctgacgtttgtcaggcggtttttgatataatcatgaaaagttgtatgagcggagttgttgtaagtatttttttcgacttgagagggttgaattggaaatatttccaaaattaatccacttacaatgactaatgccaagttgccggagtgtttggtggataaaaattttttgaataccattgcccgaaaaaaatcttaaataaaacgttggggatgtggaagttgttaaaacgtagccatgtttgatattcccgagctcaccatgaacaccgaatttagtaacggtgtgggacaatcctgccccttctttcatgactttatcaacgaatcccttcaacattccgggaatgctgttccaccaaaccggcgtgatgaagatcactgtattagctcttcgaaggtcatcgagatactcaattgtctgttgatcatgagacttcccttgatggaatagacgcaattcttccacgtcataggtaggattgaattgtgcttgatgaagatcaattagtttccaacttcttccttttgaagcaagtgttgaaatgacagcttctagaactgcgtgattaaagcttcttttatagggatgacagtaaataattaaagttgtattcatgttagtcttctccaatcagttgagttgctgctaaagcgaggaactctcgacggtaagtaatggcaccgttcgcaatcaatgaaccataaccttgtataaacgcccagactttgataaaaatgtcattttccggttctcttaaggaatgctgtgtggcaagattatgaatgatttcatgtgttaaaaccaaaaagctaaatgagttatcatcaaaattttgtgaatatatcttgacaattccaggattaaacaataaaaaatccattaaatttggaactgtctcgatttgatgaataacgaattcacctaaatcaatcaacgtttgtaatgcatcctccttgtttcctttggcaaggtgattggatgcctgtacaaagaattttttggaaattgtgacagtgacatgcttaaacaggtcttccttactggagaaatgcttgtaaaaggctcctgtggttaagtcgagagtcccaagaagctttcgaagagaaatgttttgatacccatgttcattaatcattcgaattgtttgtgagataatcgtttctttcgtgtggtttgtttttcctgcgatctgtatcatcccctgcttaacccaagataacaccgttatcctattgctgtaaataaaaaaacatgatcagcgaagtgaccacgtttcatgaggtatgtttgacaaatttgaaggtgataaaattaaccagatgttattttcgttcatctttttgacggtcttcacgagaatagggtacctcgaaaattttgtattgccctttcttgtaggtaaattgatcactcaataagttggtgatttgtgtgatgagagggttaaattcactatcgctaactgcaatcactagttcaattttgtcggtataattggtttcttcaactggtatagcggcgttttccaagaagtattttaatcgatcaaattgattgtaatcaattaacaaatttaattcttgtttgctgaccaatttgacgatcccaagcgaatcaatcgttgtcgatgtcgcgttgctataagcccgaattaaaccgccggcgccaagcttaatgccgccgaaatatcgggtcaccactgctaaaacgttatgtaactcattcattttgaggacttccaagatggggaccccggcggttccggatggctcgccattgtcgctttcgcgttgaatatggtcatcgtcacccaacatgtaggcgtagcaattgtggttggcttttggattgtctttagtcacttgatcaatgattttttttgcctggttctcgttatcaattcgtgccatcgtgcagagaaaacgggattttttaatttcgatttcatgggtaccgtttgatttaattgtcagtgattcatttttcaaaaaggattcctccattatttacgtaattagtgattgaggtgatgatctatgattaatgatctatcagagttgtatggccgccaaatgccacagcgtgatctggccgcgacactgcaaaattcaccggacattcgcttacgtccggccatcagtgacgaccatggattgaaatgtggtcgctgcgggtcaaaattgcgccgttcccttgccagtttacctaatcaccacttttattgctacatttgtattcaaatggggcgggtggataccttgtcgccactggcttatttggaagagccaaatcattttactgagaatccggatccattatcctggtccgggcagctgacccaattacaaaatgagtgtgccgacaaagtgattgaagtgtttcaacaacgccagcgtcacttgttgtgggcagtaacgggggctggcaagacggaaatgctgtttaaagggattagctgggcaatttcaaatggattgcgagtcgggattgcttcgccgcgggtggacgtatgcatcgaactgttcccacgaattcaagccgcgttcaatcaagtttcaatcgtgttactccatggcaagagtgagcagcggtaccagtacagtcagattaccgtttgtacgacccaccaactgttacgattttaccatgcatttgacgtcctgattattgacgaggtggatgtcttcccatattctggtaacccaatgcttcattttggtgttcaaaatgcgattaaacccgctggggcaacgctgtatttaacggcgacccccgatcaggcactttttaaagcaatttctagaaaacagttgtcggtcagttatttaccaatcagatatcatggacattatttaccagaaatctcggcgattcgggtcaaaagtcttaacgagcagcttcaagctggcaaactgcctcaaaaaatcttgcggatggtggctgacctggtaacagaaaagcagcgattcttactgttcgttccccacattaaagacttgagtcaagcggcagctgccatcaaggctgccgggatagcagcgaaattcaaaacggtgtattctgctgatcccgagcgaattgagaaagtagcgttaatgcgcagtcaacaactggatttcctgatcacaacgacgattttggagcggggcgtgaccttcccaggcattgacgtcttggtattaaaggctgacagtgaaattttttcggcggctgcactcgtccaaatcgctggtcgggtgggtcgaaatagtgatcggccgacaggacaagtcctcttttattgtgaatttaaaacggccaacatcaaatcctgtgaccgccagattaagctgatgaatcgaaaggcggctcaattatgaaagcctgtttattgtgtggctccagactaagacaggaaatcccacttgcagacttgattcggttaaccccactgcagaaacgggcgatctgtgaggcgtgttcccccacattttcagcgcttaacctgctaccaacttgttccagctgcggtcgacggcgaacaactgatatgagcgatccctgctacgattgtctgcgctgggagaaggacggccaattcaaatttattaactcggcgatgtacgaatataatccggcaatgaaagattacatgaaacgatacaagtttgccggggattaccgattacggaaggttttttccgatcaaattcacgagcagttgaagaagcaatctgcgatcattgtgccaatcccggtggggaaggacaccatggccactcggggctttaatcaggtcaccgggctgttggaaaatgaccgctatttgaacctattaagcgtcagattcgacaagaaggccgtccgccagtcggcgaaaaaccgtcagggccgtttattgcttgatcaaccgtttgaaatgattgaatcacaaaaaaatcaagttaaaaatcaggccgttttattggttgacgatgtgtatacaaccgggacaaccattaggcatgcggccgctttgatccaacaagccggggcagcttccgtgaaaggatttacccttgctcgataaagaaatccagacccaatgattgttaaaattcgaactttcaattatactaaagttgtagccagtaatgaaagtgatttcattagtggaccattaagcctttaatggtgaagggagagaacgctatgctaatttttaacattcgtggtgaaaacattgaggtaacccaggcgatccgggattatgttgaaaaacggatcagtaaactggagaaatactttgaaaaggacatgaaaaatactgctcatgtcaatttaaaggtttatccagataagcaagcaaaagttgaggtaaccattcctttgccatacttaactttgagagccgaagaaatgtccaacgatttgtacgcaagtgttgatctggtgacagacaaactcgaacgtcaaattcgtaagtacaagaccaaggttaaccgcaagtctcgtgaaaaaggatttaagaatcttgaatttgcacccgctgcagatacttctgccagcgagtcagattctgatgacgaatccaaattccaggttgttcgtaccaagcaactggctttaaagccgatggataacgaggaagccattcttcaaatggacatgctggggcatgatttcttcatctatgaagatgcagaaacttcaggcatcaacatcgtctaccgtcgtaatgatggccgttatggcttgattgagaccggcgaagaataattaagttaatcaattaacgggcatgcgtattatgcaccgtcaaaagaatggggataaattgcagcttaatttatccccattctttttcgtttccggaaacatttgtgaaccaatctgatcgtttaacctttcatatctattcaaaatgtattatcatggttaaatgccgctgatgcattgttttttgtgttttcatgggcggcctaaaatgttacactaaataagtatgtagtccacaaatactaagaacaatttgatcagtattttattttagaagggaatttactaatggctaatattttaagaacatgggttgaaagtgatacacgcgaacaaaagcggctcagtaaaattgccgataaagttggttcgtatgctgaagagtatcgtcaactcagtgatgaagaattacaagccaagacaccggcatttaagaaacgctatcaaaatggcgaaacactcgatgatttgcttccggaagcatttgccgttgcccgtgaaggcgcaaagcgtgtcttaggtttgtacccattccacgtccaaattatgggtggaattgttcttcatgaaggaaatattgcagaaatgaaaactggtgaaggtaagactttaactgccaccatgccggtttatttaaatgcacttgcaggcgaaggggttcacgtggttactgttaacgaatacctttcccagcgtgatgccactgaaatgggcgagttatataattggctcggcctgacagttggtgttaataccactgaaaaggatgccgatgagaagcgggaagcctacgctgccgatatcacctactcaaccaacggggaaatcggtttcgattatctgcgtgataacatggttgcttataaggaacaaatggttcaacgtcctttgaacttcgcgattgtcgatgaggttgattcaattttaattgatgaagcccgaacaccattgattatttctggtcaatcaagcggcacttccgacctttaccaacggactgacagatttgccaagacgttgcacgaaggcgatgatttcaagcttgatctggaaaccaagactgtttcattgaccgatcagggaatcgaaaaggctgagaagtacttcaacttaaagaatctttatgacaccgacaatactgccttgacccaccatttggaccaggctttacgggccaactttatcatgcttcgtgataaggattacgtggttcaagatgatgaggtcaagattgttgattcctttaccggacggatcatggaaggccgtcgattctcagatggtcttcaccaagcccttgaagcaaaagaaggcgtcacgatcaacgaggaaagtaagacaatggctaccattacttaccaaaacctcttccggatgtataagaagctcgccggaatgactggtactgccaagactgaagctgaagaattccgtgagatctataacatggaagttatttcggttccaaccaacaaaccggttgtccgggttgatcatccagatgttttgtatccaactttggaagccaaatttgaggccgttgtcaacaagatcaaggagcttcacaaaaagggtcagccaatgttggttggtactgttgctgttgaaacttctgaatacttgtcacaacgacttgatgaagaaaagattccccacgtggtattgaatgccaaaaaccacgccaaggaagctgaaatcgttgccaatgccggccaacggggcgccgttacaattgccaccaacatggctggtcgtggaaccgatatcaaattaggacccggagttgttgaacttggcggcttagctgttatcgggactgaacgccatgagtcacgacggattgataatcagctgcgtggccgttcaggacgtcagggtgatcctggtttgtcacagttctatttgtcacttgaagatgacttgatgcgtcgtttcggttctgaaaagatcaaaaacttcctggagcatttgaatgttgaaggtgaagacgcggttattcgttcaagaatgatcaccaagcaagttgaatcagctcaaaagcgggttgaaggtaacaactacgattcacggaagaacgttttgcaatacgatgatgttatgagacaacagcgtgaagtgatttacggtgagcgtcgtgaagtcattgatgagcaaaaagatttgaagtgggtcatcatgccgatgatcgaacggaccatcaatcgaattgttgatttgcatactcaaggggaaaaagaagattgggatctgcaaaccatcttggacttcgccatcagtgcgatggtcagcccagaccaaatttctctagaagatttccaaggcaaatcagctgacgaaattaagagtatgctcatgggtctggcaaacaaagaatacaaagaaaagcaagaacaactctacgatgaatcgcaaatgcttgaattcgaaaaggttgttatcttgcgagttgtcgattcccattggactgatcacattgacatcatggatcaattacgtcaatcaattggtcttcgtggttatggtcaacaaaatccactggttgaatatcagcgagaaggttacaagatgtttgaagaaatgattgccgatatcgaatatgacgcaacccgtctgttcatgaaggctgaaattcgtcaaaacatgcaacgttaatatgtattggaaagaatccggcaatgacgattgtttggattctttctttgaattggaacaaaattagaggagagtaatatgtcatttgaattgagtgaagcaaaaaaacaaatcgctgaaatgcaaaaagccatcgatggttttgggaggtcactttgaccttgatgccttaagtgaaagcatcgcgattaatgagtcgaagatggccgagccaggcttttgggatgaccaagaagccgctcagaaattgattgatcaaaccaatcagttaaaaaccaagcgcgacaatttcgtcggcctcaaaaataaactcgatgatctaaaagttactttggaattgatcgaagaggatgctcattccgggatggagggagaatttgagactgatgaaaagcagcttaaaactaaactggaccgctaccggttgaatctgttgcttaacggcaaatatgatcataataatgccattttggaaatccatcctggagccggcggaaccgaagcccaggactggggttcgatgctgctgcgaatgtatacccgttgggcagaagcccatgggttcaccgtgcagaccttggattatcaggtcggtgacgttgccggtctgaacagtgtttcactattaatcagcggtgaaaatgtctatggttatttacggtccgaaaaggggattcatcgattggtcaggctgtcgccatttgattcagctggtcgtcgacacacgtcatttgcatccgttgatgtgatgcctgaattaaatgatgacgtctcaatcgatattaacccggatgatttacggattgatgtttatcgatccagcggtgctggtgggcaacacattaacaagacttcctccgctgttcgaatcacccatttacccactggaatcgtggctgccagtcaggcgcaacgatcacaacttcaaaaccggcaaacggcaatgaacatgttgaagtcaaaattgtatgaacttgaagaagagaaaaaggccgaagaaaaggccaaaattgagggtgaacaaaaagacatcggctggggatctcaaattcgttcctacgtctttcacccatattcgatggtcaaagatcaccgaaccaattacgaaactgccaatgtcaacggcgtgatggatggtgatttggatccgttcatcaacgcctatctacaatggcaattaagtcaaaagaatccagactaatcggttattaaagccgcgtttgctttagcccggtgcgaatcatacgataaggttcttgacgccacattgcgttaagggcctttttttatcaacgacaggatgattggagaaccctaccaagcacccaaaggcagcaactgccggttaagccaccatcttgattagtctttcggatttcaaatcagcttaaatcagctgtcaataaatgatatactagccttataattattggtgaggaagacataatgaaatttttgattgcttgtggtttttatggattgcaacccgccttgtggatcggggttatccgcagttatttaattcatacgaggcggctgaagaaagagcgggggatttttaactccgcgatttatgaggatttttatgaaggtcgacattttgtcagaatggggctgatctttgggatactggcctccgtcgttttaggtggctttttaagcatttcactggaatggttgatcatttatgaaggcttactgctgatttcactcacgctgattcattggtggctgctgtcggtgactgttgccggtatcgccagtttgttggcgctgggattgccaaatatatcggaattgcgaccactgcttcattggtttgaaggactgggaatcaactcaacaactgtggccccgctcaatttgttgattttatttgtggtcattatcttggcaaacgccgttttcttgaacgttaacggtggtcgatttgattcaccgaccttggtgcgcaaccaacgaaacaataaaacggccgtttataaatttaacgaattgacgatttttccgttcctgctgtttgttcccggagattggatccataccagcttaccaatgatgccgctatttcaagtacacaatcatttctatgcgttgttattggtgccaatcctgattggacttaaatttaccgtcaaaagaagtgttcccagggccttatttaaaataatgagtcacggtatttacttattggcggggattggtgtttgcctggcgattgccggctacttcgtaccgcacctcattttacccgccgtggttatcctgttgttgggctactatttgattcttgggcttgccaaacaccgtgacaatcagcagtcgtttgaatatagtgaagtgatggatggtgtccgggtaattggcattcaaccggaaaccccagccgccaagatggatctcaaagttggcgatgtgatccttgaggtcaatggcatttcggtgactgatgaagattctttttatcgcgcgctcagcaccaactcaacttattgtcggttcaaagttcgcgatcgaaacgatcagttgaagatgaccgaatcggcgatcttcaagaattcacctcatgaaattggggtcaaaacatatacacagcttagtcattaggagggctatcgtgaaaaaagtgcttgtagttgacgacgaaccagcaattgttactttattggaatataacttgaagcaagccaattttgaagttcagagtgctactaacggagtcgatgcgctttcaatggctgaaaatggccaatttgacatcgtacttttggatttgatgttgccgcagatgagtggggaacaagtcctcaagcagctgcggatggaccgaaacgacacaccggtgattttattaactgccaaagataccgaatttgataaggtctttggcctcgagatgggtgctgacgactatattcccaagccatttagtccgcgagaggtgattgcgcggattaacgcggtgcttcgtcggtatgaaaagagtgctgcggcatccgaaacgccagctgccaaatcagccgaaaatgtcgaaaccactgggccgtttaccattgaccacaaaaaataccgcgtgagtgccgattcgaaaaacttaaagttaacaccaaaagaatttgaattgatgcagtacttggtcagtcacgaaaatcaagtgcttagtcgtgaccaattactccagggtgtttgggggtttgactactcaggtcaaagccggatggtcgatattcaaattgcccatcttcgtgaaaagattgaaccggatccaaaacggccgaaatatctgcgaacagttcgtggatttggttatgagttctccacgggggatgatgacgctgagtaaaatttataaacaaattttaaccgttgtaatcttaagcattgccacactggccgtgcttttttatggttttacgagcggcaatttgggctgggctgacctggcccttttattggccttggtcgatgcaattgccgggattattctcatcattcaataccgccagcatgataagctgctcaaacaactccaaataatgaccgaaaatattgttcatcatcagccggcggtgccgctttttgttgaacccgacaacccactcaaaggcgttgccgaccagctcaacgaacttcaaagcaggcagcaggacgaaggaaagagtattcgaaacagtaacgccgaactaattacgattctttccagccttccagtcggggtgatggtaattgattcaactcacgatgtgattttcgccaaccataaaatgtccgtcatgctgggacgagatattttgactcaggttcatccctatacccaagacatccgcaattatcaattgctgtctttaattgaaaatgtttatgacagtcacaagtctcagcaagaagagattcaaagcgtcggggcgacatctgttacctgggacaccagcgtggtgttcaatcaactcgaaaacgattttcacatcctggtgattatgtatgacatttcagatattattaacgtcaaacagatgcagattgactttttgcgaaatgccagtcacgaactcaagacgccgattactgccatctccggatttaccaaaactctgttgggtggggcgatggacgataagaagagtttggtagagtttctgaaaattattgatcaacaaagtgatcagctggcctcgctggttcaagacatactgacgatttcccatattcaaaacggtactaattatcattacaaaccattagctttacatgatttcattgatgcggagcttgcttcatatcaatcaatgatccaaggtaaccacgtttcaattcataatcaagtcccggaacacgttgaagtcattgccgacaccaccacgctcacgcggattttacgcaatctggtcagcaacgcggttaaatataatcgcccaaatggtgaggttaacattacctatagtgacaacgacagttattggcagctccacgtttccgataccggaattgggattgcccaaaaagacatttccagattatttgaacgcttctatcgcgcagacgattcccgaaccaagcagaaggtcagtgggaccggcttaggtctttcaatcgtcaaggaaatggtcgatgcggttggcggcacgattgatgttaaaagtcagcggggcgttggctccacttttactgtaaactttccgattgtcaaagatcgtaaccagcccaacacacaaacagactgatgtttgctgaatttcaaccaaatatttacattttcaaatcaatcaagccgggagcatctccggcttttttgcgtttcttcagccattaattaccaacacccggttatctatttacaaaacatttacatttgtccggtcaaatatttacattggtttaatacaatggtaattgaagattcaaggaggaattgagatgcgaaaacggacgatcgttaaactgttactgtgtgtggtggtaattgttgccggaattggtgcttacaatgcccgcagcaagacttcaaccaatcagcaatcaatcaccgctgttggttcaactgcgctccagccactggttgaggcggccagcgaacaatattctgctgatcatgctggcattttcattaatgtgcagggtggtggatctggaaccgggctgagtcaaatcgagtccggtgccgttcagatgggaaattcggatttgtttgctgaggaaaaggcgggcattaatcccgccggcttggtcgatcacaaaattgctgttgtgggagtcgctccgattaccaatgaccgcgttgggattgacaacttgagcaccgcccagttgattgcaatttttactgggaaatacaccaattggaaacagcttggcggacccgacctgccgattactttgatcaaccggtctcaggggagcggaacccgggtaacctttgaacaatatggtcttaaaggccatgaaagtgccaccgcccaggagcaggattcttcaggaactgtccgccagattgtctcatcaacgccgggggctatcagctacgtctcatttggctacttcaataagagcattcatccattaagcgttgatggtattaagcccacggaacaaaacgtgatggacaataagtggaaaatctggtcctatgaacacatttacacccgtgggaaacccaccggattgactaaaaaattcttaacttacttgaaaaacgatcatattcaaacgaccctctttaacaaactaggttacatctctgtgaaagatatgcattaccagagaacctggcagggcaaaattacaaaaggatcgggggaataatcgtgcaaaatgaaaaattagccaaacaactgatgaaaaaatccaaaacggcccgttacgaacgatttgggcacctgctcagtctttcggcgctgctgctgattatggcgatcgtgcttggcattattgtcttcgttgccagcaagggattggcgaccttcttcaaagacggcatttctgtcaaagacttctttaccggcacgttgtggaatcctggtaccaagactcccaacgggcaccaagccgtcggcgcgttgcccatgattgtcggctcttttcttgtgacgattctggctgctttactgtcgacgccgttcgccatcgggactgcggtgtatatgaccgagatttctcctaaacggggagctaaaattcttcagccggtaaccgaattactggtcggaattccctcggttgtctatggctttattgggctctcagtagtcgttcctttcgttcgaaatacgtttggcggcagtgggtttggtatcctatccgggacctttgtcctgttcgtgatgattttaccaaccattgtatcaatgactgtcgattccctcaggggcgttcccaagttttatcgtcaagcctcactggctttgggtgctaccaagtggcagaccatttggaaagtcgtcttgagagccgccacaccagggattttgactgccgtggtttttggaatggccagagcctttggtgaagccttagccgttcaaatggtgattggaaatgcagctttgatgccgcaaaatttaacgtcaccggcttccactttaacctctgttctaaccgccggcatggggaacaccgtcatgggatcgcttcaaaatgacgccctctggtcactagcactggttctgttagtcatgtcgctcttctttaatttattagttcacatgatcggtcggaaaggggcgtttaagaaatgaatcgaacacaaaagcaaagccgatttgccattgcctgtttaaaagccgttgctggctttgtggtggtcatcttagcctttctgattggctatatttttatcaccggactgcccaatatcagttggcatttcttaacgtccccggccaaagcgtttaatgccggcggcggaattggcattcagctatttaactcattttacctcttggtgttagcaatgttgatttctctgccaattgcacttggggcggcgatttacctcaacgaatacgccaaagataactggtttaccgctacgatcaagacttcaattgaaattttgagttccttgccttctgtggtggttggactgtttggtttcttattgtttgtcgttcagttcaactatggtttctcaatcatttcaggtgcgttgactttaacgatttttaacttaccactgttaaccagaaatattgaagattcactttccaacgtttccgatgaccagcgccaaggcggtttgggcttgggactttccaaatatgagacgattattcacattgtcgttcccgcttcactgcctggaatcatcagtgggatcattctttgttcgggacgggtttttggtgaggcggctgccttgatctataccgccggtcaaagcgccccagcgttgaattttgccgattggaaccccttcaacattgatagcccattgtcgccgctgcggccggctgaaacattggccgttcacatttggaaaatcaactcagaaggaatcatgcctgatttgacacaggtttcctccggttcagcggctgtcctggtcctggcgattttaatctttaatttgtcggccagatggattggccggaaggtatttgaacgaatgacttcagtaaagtaggtggctgaaaatgcaaaacacaactgaattaaacaacaaacccaagcggtttatttatgattttaatcccgaagaaaatgacattacgatgcagaccaaagatttggaaatttattacggcaaaactttagcaatgcacaacgcggatttgaagtttaaaaaaaataccattacggccttgattggaccttccggatcgggtaaatcaacctttttacgggcccttaatcggatgaatgatggcgtcgctactgtgaaaggtgagattctttatcaaggcgtcaacattaatcagcccaagatcgatgtttatgaggtccggcgccgaatcgggatggtttttcaacgaccgaatccattcgccaaatcaatctatgacaacgtgactttcgcgctccagcgacggggaattcatgataagaaaaccttggatcaagtggtggaaaccactttaaaacaagccgctgtctgggatcaggtcaaagacagtttgaataaaagtgccctttccttatccggtgggcaggcacaacgggtttgtattgccagagccttggcagttcaaccggatgtgttactgttggacgaaccggccagtgccttggacccggtttcaacccaacaactggaagcgactttacgtgaacttaaaaaggattatacaattatcattgtgacccacaacatgcagcaggcagcccgtctgagtgactacacggtcttcttcaacatgggtgaggccattgagtacaacaaaaccagaaaggtcttcacccggccgaaagtacagatgacagacgactatgtatcaggaaactttggttaggaggaacaatcatggcaacaccaattatttcagcagacaatttggatttattctatgatgattttcaggcactttacggaatccatttagatttcctgcctaaccaaatttctgcgctgatcggcccatcaggctgcgggaagtcaacatttctgcgctgcttaaatcgcatgaatgatatgatcgatggcgtgacaattaccggagcggttcaatttcacggagaaaatatttattctccgcaaacaaatctggtagaattgagaaagtcgattgggatggtctttcaacagcccaacccgtttccattttcagtctatgataatatcacctatggtttgcggatcgcgggacttcgtgacaaacaaaaattagatgaaattgttgaaaaaagtttgaagcaggcggctgtttgggatgaagtcaaagacaatctgtacgataacgccctgtcgttttccggcgggcagcaacagcgaatttgtatcgcccgggtgcttgccacttcgccatcggttattttgatggatgagccgaccagtgcattggacccgatttccagtgccaagattgaaaatactttgcttgagttgaaaaaagattatacaataataatcgttactcacaacctgcagcaggcttcccgaatttctgataagacagcgttctttatggaaggcagagtggttgaatatgatgacacaactaagatgttcgtgaatcctgaggaaaaacaaacggaggattacgttagcggacgattcggataggagagaagcttatggggaaagtttttgatgaagagattattacgttaaaggcggattttatgaaattgggggcactggttggtgaagccgtgaccaacgccgggcagtcgtttgtcgaccatgatattcaaaaggcggaaacggtgatcaccaacgaccacgagattaatcacctccagattcatattgaaaagcggtcatttgaaatgattgcgctgtatcagccggtcacgggggacctccgggaagtggtcggaattttaaaagccgtcactgatttggaacgcgccggtgaccatgcccgaaacgttgctcgatcggtgattgatattaaaggcaagcagcggatcgcttcagtggaagaaattattgctacaatgtctcaagaagtcagcgagcagtatgctgattcaattgagtcatatggtgatgccgatcaggacaaagccaagcggaccgcgcaacagtacgataaaaaaattgaccagctctataacgacattgcttctcccagttaccaagcgatggccaaggatccagagattgtcagttcagcgattatttatctaaacgttgccaaagatttaggccgggtgagtgattacagcacgaatatttgtgagtggacggtttatctggcaaccggaaaaattattgaattaaattaagaatggttgatattttgcactgcatacttgattgcagtgccttttttagataatcttaagctagaagttttattgtggaggcatgaggatgaatagtcataaaaaattacggcgttccagtaccaatcgggtgatttccggcgtgcttggcggaatttccgagtatctggactggaacgctgtcttggttcgaatcttgtatgtggtcttggcgtttacgcccgggatcaacgtggtcgcaattattgggtatatcattatgatgttcgcaattcccagtgatacacctggtagtggatcggcctttgaccaattcaaaaccactttatccggcggaacttctaacgacaaatccagaaaagtcattcataacgtcgaagaaaaagacgttcatgatgacaagaaaaggggtcaataattgagatttttaaccaatgtattggtcgatacgatcctgtttgttgcgatcagtggctttttccctgccaacttctacgttgccagcgtgggaattgcttttgtagcggcggtggttttagccgttttgaactggttggtccgaccgatcattacgatcttgtctttgccgattaaccttttaacactgggattattcacgtttgtcattaatgggttgatgcttgaactgacggcgacgattgttggggctaatttcagattctcatcattttgggtcgcaattggcgtggccattctgatgtctgcggttagctggatcattgctgaatatttccgcaagccataaggacttgtcaggctcaaagtgataaaattatattgattaattgaggagggatgttcttgactgaaagtgtaacggttgctgatttggttaaaaacgccaggctggatgtctattatgggaaggaataccttgaagaaaggaccatttccactgctgatatttccagaccgggcctagagctaaccgggttctttaattattaccctgtcaaacgaattcagctgttgggcattactgaaatttcatattccaaggggatgtctcatgaagagctcctcgatgtgatgcagcagatgtgtcaaccacagaccccggcgttcgtggtgtccacccaactggatccgccggaagaattgctggaggccgcaaaagaacagcaccttcccgtcctcggttccaaattgacgacgtctcgagttctcagtaacatgactaattacctcgacgataaattagcagaacgcaagtcgcttcacggagttttggtcgatgtttatggattgggaatcctgattaccggtgacagtggaatcggcaagagtgaaacggcgttggaactggttaaacgtggccaccggctgattgccgacgatcgggtagaggtttaccaacaagatgaacaaaccttgatggggactgcccctgcgattctccgtcacttactggaaattcggggaattgggattatcgatgtgatgactttatttggcgccggtgctgtccgcagtcagacgaaagtcgccttaattattcatctggccaactacaccaaggaagccaagtttgatcgtctgggcaacgggactcagaatgtccatatttttgatgtcgatgtgccgaaaatcacgattcccgttcgaaccggccggaatttggcgatcatcattgaagccgctgccatgaacttccgtgcccaaagcatgggctatgacgcgactgaaacctttgaccgtaacttgaataatttaatcaaggtcaacagcaaaaacgacgaaaagcataaagaagaacaggaacatcttgaggagaaaaataaagatctcatcgatggtcgtgacaaagattcagataaaaaataggagatcgttattttgacaaatttattgagcttagccctcaacccgatcgcctttaacctgggtccaattgaagtccactggtatggtattatcattgccagtggcgtgattctggcggtttggttggcggtccgcgaaggcgataaacgtgggattaaagccgacgatatttacgatatgattttgtgggccttgcccgctgcgctaatttgtgcgcgattgtattacgtcatcttccagtggtcttattacaaagataaccctggtgaaatcatcaaaatctgggacggtggtattgccatttatggttctttaattggtgcgatgattgtggtgatcctattttgccgccaccgcttcattccagtttggctgatgttggatgttgccgcaccaacagttattttggcacaatcaatcggccgttggggcaattttatgaatcaggaggccttcggtcaggtaacatctttgagctttctgactgggcttcgtctgccacatttcatcattacccagatgtacattagcggcgcgtatcggcagccgacctttctctacgagtcgctgtggagtttcttaggttttttggtgctgataaccttgcggcacaattcccatctgtttaaacgtggcgaagtctttttaacctatgtcatgtggtattcttttggcagattctttgtcgaaggcatgcggactgacagtttgatgcttggcggccttcgggtatcgcagattctttcaatcattttatttgttggtgcaattggaatcatcatttatcgtcgattacgccagccacataatccttggtatttagagggttccaaattaacagttaattgatcatttactaataaaggagatttatcatggctaaaaaagttgcagtgcttggtgcaggttcttgggggagtgttcttgccagtttattggacgagaatgggtcagacgtcaaattatggtcgtataacccgacacaagttaaggaacttaacgaacagcataccaacacaaaatacatcaagaatttcacgttttcagattcactggtggctaccaatgatttgaaggacgccatcgatggtgttgattacatcttattcgtggttcccacccaggtaacccgttcagttgccaaacaagttgcagaaattttggccgaccggaatcaaaaagtgaatatcatccatgcttcaaagggaattgaagaaaaaacttacttaagattatctcaagttctggctcaagaaattgatcctcagaaccgcaaatcaatttcagttctatccggccccagccaggctgaagatgtcgtgacccatgacattactttggtcaccgttgccagtgatagtgaccaagctgctactgaaattcaaggtttgttcatgaacaactatttccgtgtttataccagtgacgatgtcattggcgtcgaaattggcgctgctttgaagaatattattgctttgggcgccggcgccttgtatggattggggtataaagacaacgccaaggccgccttgatgacccgtgggttagccgagatttcccgccttggaacgtcgtttggggctaatccattgacctttatcggtttgtcgggcgtcggcgatattattgtaaccgccaccagtaccaactcccgtaactggcgggctggtaacgaattaggcaagggtcattccctggatgaagtcattaataatatgggaatggtcattgagggtattgcgacgactcgcgctgcctatgaactttccaagaagcgcggtgttgaaatgccaattacttcggcaatttaccacgttttatatgatcatgctgatattaaagaaacgattaaccaactgatgacccgtgaaggccgttcagaaattgaataactcagagaaggtgaagctcactatgaccagaaaagtaaccaaagcagtcattccggctgccggcttaggaaccagatttttaccggaaaccaaggcactcccaaaggaaatgctaccgattgttgatacaccgacaattcaatttattgttgaagaagccaaacaggcgggcatcaaagacattgtaattgtcatcggtaaaggcaagcgctcaatcgaagatcactttgactcgaatcccgagttggaaatgaatttggaagagcgccacaagaacgatattcttgaaaccattcgcaagaccaacgacatgaatatttacttcattcgtcagtctcatccccgtgggttgggtgatgcaatttacaccgcccgcagtttcattagcaatgaaccgtttgtggtcatgcttggtgatgacgtgatgcaggacaaagtgccactgaccaaacaattaatggaaagctatcagcagactggagcttccacattagcagtgaagaaagttgcccacaaagatatctccaaatatggggtcattgatccctctgaagaggtccgcccaggcttgttcaacgttaaaaagttcgttgaaaagccaacgccagagaaggcccccagcgatttagcgattattggccgctacttgttgacgcccgaaatcttcggcattttggaaaacgccaaaccggataaaactggtgaaattcaactgacatctgcaattgacaccttgaaccagacacagcgggtctttgctcatgaatttaagggtgaacgattcgatactgggaacaaattaagctggctcaaaaccaacatcatctttggtctgcgccatccagaaatttctgatggcttgcgaacttatctcaaagatttgggcgcccaattaactgaagaagacaaaaagaagtaagtgtatctactggacagacttactttttcatagtaaattaacgtgtaagtaaaatttggtaattaaagggaggatccatatggctaaacaatatgatgtcgtgattattggtgccggccccggcggcatgacagcggctctatatgcttcacgagccaacctgtcagttgcaatgatcgatcggggaatttatggcggccagatgaacaacacagctgccattgagaactatcctggttttaaatcaatcatgggtccagatctcgctcagaatatgtatgacagttcaattaactttggtgctgaatacgtttatggaaccgtcagtgctgtggaagatcacggtgactataagctcgtcaagactgacgaagacgaaatccaagccaaagtggtcatcatcgcaaccggttccgaatataagaaattagggatccccggagaacacgaatacggtggcaaaggggtttcgtactgcgctgtctgcgatggggccttcttcaagaacaaagaagtcgtcgttgtcggcggtggagattctgcgattgaagaagcctcttacctcgctggaatcgttgatcatgtgacagttattcatcgccgtgaccaactgcgtgcccaaaaggttatccaagaccgggcattcgccaacgacaagattgattttgtttggaattccaacgtcacggaagttttgggtgatgataacaaagttaccggcgttaaagtagtgaataaccagacaaatgaagaatcagttcttgagacgtctggggtctttatttacgttggtctgctgccaatgaccgatgcttttaaagatttgaacattactgatgaggatggttggattcaaaccaacgatcagatggaaacgtcaattcctggtatttatgccattggtgacgttcgccaaaaggatcttcgtcagattgcaacagctgttggcgaaggtgggattgccggtcaacaagcattcaagtatgttgaatcattggctgacacatcaaaggccagtgtttcggaacactaatttaatgattaatcaaagggaggccgcgtacaaacagttgttttgttcacggctctttttgcgaggaaaaggacggggaattatcaatgggaatgcatcagtatttggaaagtttagacgagttggaattgatcaatcgagcacctggctactttaaattcgaacagcattcggttgctgcccattcattcaaggtaactgaaattgcccaatttttaggtgacgtcgaggaaaatgccggcgaaaaagtcgactggcgcgggttgtatgaaaaagccctcaatcatgattataccgagcggtttattggtgacatcaagacgccggtcaagtatgcaacacccaagctgcgttcaatgctggctgatgtggatgacaaattgacggaaaactttgtccaaaatgaaattccggatgaatttcaagatgcctaccgaagacgtctgtcggaaggcaaggatgatagtttggaaggccgtattttagcggtggccgataaagttgacctgttgtatgaatcctttggcgaaattcaaaaaggtaatcccgaggaagtctaccctgagatgtataaagagagtctctcaacgatgctggagtaccgtgatatgcattgtgttcagtatgttttgacgaaagtcattccggatatgctggccgaaaactttacgactcaggataaattaagacgactcacccgcaaagttttaaaaaaggaagacaattccaaggaataatgattggcgaaagtatgttcgtatggtaaaatagcgttgaatagtgggctgaaacaaaatatgattttgcttgcagcccttttatgttgtgtcattttggtatagaggttagggggattcaaattgattgaacgtgaagcagatcgaaaatttgatctagtatccaaatataaaccaactggtgatcagcctgatgcaatcaagaagttggtggcaggtattaacgaaggcaaaaaagcccaaattttaaaaggggctactggaactgggaagacttttaccatttccaatgtgattgcccaggtcaacaagccaactttggtcttatcgcataataaaaccttagctggccagctgtatggcgaatttaaagagttcttcccccacaatgccgttgaatattttgtaagttattatgattattatcaaccggaggcctatgtcccatccagtgacacttacattgaaaaggattcgtcgattaatgatgagattgaccagttacgccactcggcaaccagttccctactggagcgtaacgatgtcatcgtggttgcctcagtttcatcgatctttgggttgggtgatccatccgaatatcgaaatcacgtggtttcattgcgggttggccagacaattgaacgggatcattttctccgccaattagttgatattcaatatgaccgcaacgacattgattttcagcgtggtcgttttcgagttcatggggatgttgttgaagttttcccggcatcctgggatgaacatgcctttcgaattgagttttttggcgatgaaattgaccggattcgcgaagtggatactttaactggtgaagtcatcggcgatcgggatcatattgcgattttcccggcgactcactttttaaccagtgatgacgtgatgaacgttgcactgccagagattaaagacgagatggacaagcaggttgccaaatttgaaaaagagggcaaattactggaagcacaacggttgaagcaacggactacttacgatatcgaaatgatgcgtgaaatgggctacacgagcggcattgagaattattcacggtttatggaccgcagaaagccggggcagccgccgtttacgctgcttgacttcttccctgacgatttcttgttagtcgtcgacgaatctcaccagacgatgccgcagattcgggggatgtataatggtgaccaagcgcgaaaacaacagttggtcaactacggattccggctgccaagtgcactggacaaccggccactgacattgagcgaatttgagcagcacgtccaccaggtcgtctacatgtctgccactccggggccttatgaactggatcagaccaaagatgtggttaaccaggtcattcgaccaaccggtttactggatccaacaattgacgtccgaccgattatggggcaaatggatgatttggttggtgaaatcaataagcgggttgacaagcacgagcgggtgtttgtgaccactttgaccaagaaaatggctgaagatttaactgattatctcaaagatttggggatcaaagtgaagtatctgcattctgatattaagacccttgaacgaactcaaatcattcgtgacttgcggctgggtaagtttgacgtcttggtcggtattaacctgctgcgggaaggaattgatgttcccgaagtttccttggttgcaattttggatgctgataaggaaggcttcctccgtaatgagcgttcgttgatccaaactatcggccgtgcatcccggaatgaacatggcgctgtgattatgtacgcggacaccgtgaccgattcaatgaaggcggccattgacgaaaccgctcaccgacgggccattcaaattgcttataacaagaaacatggtattacgccaaccaccatcgtcaaaccaattcgtaacttaatttcgattaccaaaggctcggatgatgccggcgaaaaggacgactttgtcgaaagtgattttgaacaaatgagtaagaaggatcaaaaggatatgctggctcgtttgacggaagaaatgcgtgacgctgccaaaaagctcgattttgagcaggctgctactttgcgtgatacaattattgaattaaagggtcaaacgagtaagtaatctaaaggagattatgcatattggcaatggataaaatcgtcattcgtggggcacgtgcccacaacttaaaaaatgtgaatgtgacaattccaaaaaataaactggttgtcatgactggcttatcgggctcggggaaaagctcgctggccttcgatacactttatgcggaaggtcagcgccgatacgttgaaagtttgtcatcatatgcgcgtcaatttctggggcaaatggataagccggatgtcgattcaattgatggcttgagtccagcaatttcgattgatcaaaaaaccacttccaagaaccccagatcaacggttggaacggtcactgaaatcaatgattattttcgactgttgtgggcccgagtgggggtaccaatctgtcccaacgacggctcggtgatttccagtcaatcagttgaccagatgatcgaccagatcatgaaactgcctgagagaacaaaattgcagattctgtcaccaatcgtacgtgggaaaaaaggtcaacacaaaaagatttttgaaaagatcaagcgtgaaggttttgttcgggtacaggttgatggcgaaacctatgatattgatgaagcaccggaactcgataaaaataagagccatgacattaatattattattgaccgaattattgtcaaagatggcattaataaccgattgtcagattcattggaagctgctttgcgccttagtggcggttatgccgtcgctgactttttgggcgagcgcgatccactgatgttttcagaacactacgcctgcccaatttgcggcttcacagtcggtgaactcgaaccacggctgttttcctttaactcaccgctgggcgcttgtcctgactgtgatggtttggggatgaagctggaagtcgatgaagatttggtggttcctgatcgaaccaagactctggccgagggcgctctggcaccttggaattccgccagttccaaatggtatccgaatatgctcaagcaggtttgtgatgctcaaggcatcgacatggacgtgccatttaacaaactgccgaagaaacagcaaaactttgtgttatacggttcaaagaccaaatcattccactttgtcctccaaagtgactttggcggcatccgtgatgtggacggcccgtttgaaggggttgtcaacaacgtcgaccgacgctatcacaacaccagcagcgactttaccagggacaatttaagtcagtatatgaccgaattaacctgtcagacctgccacggctatcgattaaaccgccaggcactggctgttaaggttggcaagcataacgtggcccaaatttcagctcttgatgtcactgcagagttgaacttctttcagtcgctgacatttggtgaacaggatacaatgattgccaaaccaattatcaaagaaattactgatcgactgacttttctaagaaatgttgggttggattacctgaccctctcccgttccgcacggactttatcaggtggagaagctcagcgaattcgcttggcaactcagattggttcaaatttgactggcgttctttatattcttgacgagccctcaattgggctgcatcaacgggataatgaccgactgattgcctccctcaagaaaatgcgcgatttgggcaataccctgatcgtggtcgagcatgatgaggataccatgcgggctgccgattatatcgtcgacatcggcccgggtgccggtcagcaaggcggtcgggtaatggccgtcggaacacccgccgacattgaaaaagtaccggaatcgatcactggccaatacctctcgggcaagcggtttattccggttccagataagcggcgcaagggaaatggtaagaaaattcgtgttactggtgctgctgagaacaatctcaaggatttgacggttgattttccgctcggcaagatggttgtggtgacgggtgtctccggctccggtaagtcgactctggtcaatgatatcttgaaaaaggcccttgcccagaaactcaatcataattccgagaagccgggtaaatacaagtccatttccggttacaaaaatattgaaaaaattatcgatattgaccaaacgccaatcggtcgaacaccacgatccaacccagccacctataccggtgtgtttgacgacattcgcggcttgtttgccaataccaacgatgccaaacttcggggcttcaaaaagggccgctttagttttaacgttaagggcggtcgctgtgaaacctgtcatggtgacggcatcttgaagattgaaatgaactttctgccagacgtttacgttccttgtgaagtatgtcatggcaagcggtacaatgctgagaccctcgaggttgaatacaaaggcaagaatattgccgatgtattagacatgaccgttgacgaagccgtggattttttcagtgccatcccaaaaatttctcgcaagctgcaaacaattaaagacgttggtctgggatatgttcatttgggccagccggccacaactttgtctggtggggaagctcaacgaatgaagttggcttctgagctgcataagaaggccaatggccaaaacttctacattctcgatgaaccaaccactggccttcatagtgaggatatccggcgattattaggtgtccttcaaaagctggttgatcaaggcaataccgttttgatcattgagcacaacttggatgtcgttaagagtgccgattatctgattgatttgggaccggaaggcggcgatggtgggggaacggtcgttgcgaccgggactcccgaacagttggccaaagtccctgagagttacactggtcagtaccttaagcccgtccttgaaagggataagaaattgaccaagcaggctgaaaagcaggcagtcaaagcaagtaaataatttggttgagccatttcaatgaactgattggaagtggctcttttttgctgtctgaagttgccccattactgctagaatgctcattcggtcggggacaagtacctccgggtgtttctttcattcacatgacacacccggtatgttatactggttgaagttcgttatacgaaaggaaatcattatggctgttaacaaccaattcgtcatcatcaccggaatgagtggtgctggtaagactgttgccatgcaaagttttgaagatttggggtatttttgcgtcgataatatgccgccaaccttgctgccaaagtttaaagaattaatccgcatggagcgggatattaataaaattgctttagtaatggatttgcggtcacaggtcttttacgatgaaatcatcgatatgtttaacgatttaaagaaaaatgatgacaataatgttgacatcatttttcttgattcatctgaccaaaaactcgtttcccgatacaaagaaacgcgtcgggcccatccgcttgctcgcaatggacgcgtcattgacggtattaaaaaagagcgtgaattgttggccaacgtcaaacaggctgctgacctggttgtcgataccactaatatggcgccccggcggttacgtgaagaagtctttcacaattttgaatcaactgatgaaacacatactttccacgtggaagtgatgtcgtttggtttcaaatatgggctcccgttggacgctgacattgtcatggacgtccgatttctacccaacccatattatgatgccaaaatgcgttacaaaaccggccttgataaaccagttcgtgattatgtcatgaactcccaaggggccaaagaattttatcaaaaactattggatatgatggtcttcacactgcccggttaccaaaaggaaggcaaggccagcttaactattgcgatcggctgtaccggcgggcaacatcgttctgtggcaattgcccaacagctggcaaatgacttgaaagatcagtatccggtgaacatcacccatcgggatattgaccgccataaaacaaaggagggtaactgatgcttgacgcacttcatacgcaccaaccgcgaattgtcgtgattggtgggggaactgggctgccagttatcctcaaaaacttacgaaatcgacacgtcgacattactgcaatcgtcaccgtcgccgatgatggtggttcttctggtatcttgagaaactacattaacgtcgttccgcctggcgatatccggaacgttatggtggcactatcggagatgcctgagttgtatttggatttgtttcaataccgatttcgaagttcagaccaattctttgccggtcacgctttgggcaatttgattattgcggcactttcagagatgaaaggcggtatttttgattccgtccagatattgagtgacatgctcaaggtggatggccatatttatccggctgccaacgagcccctggaattaaacgctgaatttagtgacggcacgacaatgagcggtgaatctgaaataaccgctgccggcaaattgattaagcgcgtttgggtcgagaccaccgatgattctcataaaccagaggcggttcatcaagtgattgatgcgattatgaacgctgatcagattgtcttgggtcccggaagtctgttcaccagtattttgcccaacttaatgattgaaaacgtgggtgaagccttacgacaaaccagcgccgacatcgtctatatttgtaatatcatgactcaaaagggtgaaaccgagaacttcactgaagctgaccatgttcgcgtcctgaatcgtcatttagggatgaactttattaataccgtcttggtgaacatcaaagaagtgccggctgaatacattgattaccaaaaatggaatgaagtctcacaaccggttaaacatgattttgccggattgcgggccatgggctgtcgggttatctcagccgattttctggaattaaaggatcgcggtgcctttcacaatgggcaagaggtcgctgacgaattgatcaatttactgggtcgatcattggacgaccataagtaggccagtcactcaagaaatggaggggattaaatgtcatacgcaagtgaggtcaaaaaggaattaacctctttgaccgttcaccgggataatgccaaggctgaattaatggccttgattcgaattaatggctccctttcaatatccaatcaccactttgtgttaaacgtttcatccgaaaacccggcaattgccaggcggatgtacaagttgctttcaaagttctacgggatcactggcgagctcagtgttcgtcgtaaaatgaagctgaaaaagaataatttatatattttacgagttgaaaataaggcaacccaactgttggatgatctgggtatttttgatggtgcttcaatcgttgaacgggttcccagtcatatgttgacagaagattcgcagatccgctcatatctgcggggagcctttttagccagcggctctgttaataacccggaaacttccaggtatcatttggaaatctattccctgtatgaaaatcataacgaaatgattgcagaaatgatgaacaagtatcacctcaaagcccgcactacgcaacggcgaagcggctacatcacttacctgaaagaggctgaaaaaattgccgactttttgcaattgatcggtgcgaccagctcgatgctgaaatttgaagatattcggattgttcgcgacatgcgcaactccgtgaatcgactggttaattgtgaaaatgccaatctcaacaaggttgccaacgctgccagtaagcagattgaaaatatcaaactgattgacgagatggtcggattaaataaactgaaccctaagctggcccaagttgcccgggcgcgcttgaaacatcccgaagtcagtttgaaagagttgggcgacttggtggagggtggaccaatttccaaatccggagttaatcaccgattgcgaaagattaacgaatatgccggcaagctggctcagggactgacccctgaagtttagttttgaccaagctagtaaagtttcaacacatttttaaacctaaaaaaggattctaattatttcgctgtgaaatagttagaatcctttttgaatccaatcatttaactgttaatgacagaggttagccctcactaactcttaaaacacaggcaccacgaatatcacctttggcaatatatttcagcgcctcgtcagctttggccaacggatattcagtgacctccggatggatattgagtcgatcagctaaggtcaggaactcttcaccatcccgacgggtgttgctttcgacactggtgagatttttttcatggaaaatgtgacttggataactcatttgcggaatatctgttgagtggataccggccattgccaacgtgccacctggtttcagcgcttccatggcttttggaactacgtcaccaaccggtgtgtagttgattgccgaatccagcttaacgggtggcatatcataggttcctctggctgaggcagctcccagttgcagggcaaatttcctggcatcttcaccacgggttaaaacgtgaacctcgatgccttgcttcattgcaatttgggcggtcaaatgagccgagccgccgaagccatacaggcccaaggtgccgcctgcagggacgttagcccgttcatatgcccgatagccgatgattccggcgcaaagcagtggggcagccgtcagtgaatcaaaccgggccggaatccggtatgcgaaaccttccggaacagtgacgtattctgcatagccgccatcatgatcccagccggtataaagtgagttggggcagagattttctctcccggaccggcaatattcacaaaccccgcaagtccaacgtaaccaaggaatcccaatccgatcgcctaatttaaatcgacgggtttcagcacccatctgaacgacccgaccaacgatttcatgaccgggcgtcaaatgttccttatgaaccggcagatcgccttcagttacatggagatccgtgtggcagaccccgcaagcgatgaccttgaccaaaacttcgcctcgttttggttttggcaccggcttggtggtgtaacgtaaaggagaaaccgcaccgttaattgaaccgggcttaacaatttcccaggccttcatctcagtagggattgattcatcagcagtttgtttaacttgttcttttgtttgattgacatccatattaatggcctcgattcatcattcatcatgttaattttttaactaacttcacctatattctagtcggtcatcaaccaattatcaatcaggtggattatgtaaaaaaagcagccctcacaaaatgaggactgctttgaaaggcatcatacaattcaattaacgaattgaattactgcttttcggaactgctggtcataatgccatccaaaaggccataatcaacagcttcttgagcagtgagataattatcacgctcggtgtctttgttgatcttctcaattggttgaccggaattctcagctaagagattgttgatcatcttacgagctttgagaatttcttcagcagcaatttcaatttcagtttgttgaccttgagcaccaccagaaggttggtgaatcaagacttgggcatgtggcaaagcaaatcgcttaccctttgctccagaagaagcaaggacagaagccattgatgcggccattcccattacgatcgtttgaacgtctgacttaacaaagttcatggtatcgtaaatggccatgcctgaggtgatcacaccaccaggtgagttgatgtagaggtaaatatctttttctgagtcttgagcatccaagaaaagtaattgggcgataatcgcattagccatgtcgtcttcgatagggcctgataacatgataattcggtcttttagcaaacgtgaataaatatcatacgcacgttcaccgcctgcggattgttcaatgacggttggcactaaattcattcaagatgcctccttataggttttatgaaagatggcttacgccaagttcatgttaatatgatagtttattggtcaaaaaaggtcaaatgttttgctcacatcaaatcattaatttttccggtcaatcttcactgtgcttcgataaagaaatgcttataataagaaagcggattcattcgtgatacaataacggtaatcagcaaataccgagtcgggaggatatactatgagaactcatcatatttcactgttaaccagagatgctcaacaaaacattgatttttatacccgggttttggggatgcgcctggtaaaaaacaccgtcaatcaggaaaatatccgcattcgtcacttattctacggtgactatctgggaacaccaggatcagtggtgacattttttgtggtgccattattaggccatcggactgacggtaagcatttcttcaataatatcaaactttcgattccaaccgggagcactgatttttggaagaaacggttaaccgaccattcagtggctgttcaagatattgaccatggcctggtgttcgctgaccctgatgatgtcgaagttaaattattggagacttcggaagttttaaccgatatgcgggtggttcctgataatgggatccccgctgaaaaacaaattacgcatttaatgggaacagaactccacgtgccggatcctgaagctaccagtgcctttttccataattggttgggcattccggtagaaaataatgttgtccaattggaggacggccagtccattgaattatttgaaagtgaccagcaagatgtccggactcggtttggccggggcagtattgatcattttgcgattcaagccccaactaaggcggccttgttcaaattctgggatattgccaaagaacagcacttaaacattgaagagtatgccgatcgtggctggttcaagagtttgtacgtccgagatcctggtgataaccgggttgaaattgccacgacgactccggggtttagtctcgaagaacccattttgacgatggggcagggactgtcattgccaccgaaatttgagtcccaacgtcaagagatcatggacttctatgctaaagaaggcgttgattttaccgaaggtgttcgagagccaacgtccgtcccggattaaccaggggttgttgaattgcgaagaaaagattaaccatcaaaaaaagaggttcaaggattaagcttggacctctttgttgtttgtgaaatcaagccgaccattgagaggaccaaacttcagaaacatcccatgacttacctaagatattttgggacttgatttggcactccagaagcgataaattgaattgtttggcataggaacagacacacgctagtcagtttgcatgaaagtgagaaagagaatgaaaattgtcgaagaaaccaaggtcagtcccaaattggtgaaggacttgttgacggtttgggagagttccgtcaaggcgacccatttatttttgacagataacgagattcaaaagattaagaaggtcattccggaagctattggcggcgtccagcatttaatcgtgattgaaaacgacaatggggatccggttggcttcatgggaattaatgaccgaatgcttgaaatgttgtttatctcaaatcaataccgtggtaagggtttgggcaaacgactattggattatgggatgcagcagtattcgatcgaccagcttggtgtgaacgaacaaaacccacttgcgcgcggattttatgagcacatgggatttgaagtttacaagcgcacggaatttgatgaacagggcaatcactttccaattctgtatatgaaaaaagcggaatgacgatcaagctgattgcttacaaaaaacagcggggcatctgcctcgctgtttcgttgattaaaattgttttgtgtccactgaacctagtttcaccactaacacaattacctatgtgtcaaaaatgacctaatgaaacatgaatccttgcttgcgatgggtcagtgaaatctgatgcgcccggggggaatcgaaccctcatttcaagaaccggaatcttacgtgcgatccattacactacgggcgcaacttcctataccaatatactagaaagtgagaactttttcaagaacaaagaaaaattgattgtgaaaacgcttactaaatccatttgcattgcaattctcccgcggtctgctatactcgaatttgggtaatattttatggttactcgatgcatactttgaactttcgttcacaagggtgctgactttgttttcatttcatggtacgattaacgtgtactgtgtcttaatattttcttatttcctaaaggaggaaaacttagtatgactgtaaagattggtattaacggttttggccgaattggtcgtttggctttcaagcggatccacgaattacactccgacgagattgaagtggctgcaattaacgatttgaccactccatcaatgttggcttatttattgaagtatgattcaacccatggacgtttccctggtgatgtttcagcaactgacaagggtatcgtcgttgacggtaaagaaattcctgtttacgcagaaaaagatgcttctaaccttccttgggttaaaaatgacggtgttgactacgtacttgaatgtactggtttctacacttcagaagaaaaatcacaagctcatatcaaggctggtgcaaagcgtgttttgatttcagcacctgctggtcaaattaagactgttgttcctggtgttaacttggatgaattgaactcaaacgatgtcatcgtttcagctggttcatgtaccactaattgcttggcaccaatggcttacttcatgaacaaagactttggtatcaaagttggtactatgacgactgttcacgcattcactgcttcacaacaaattcttgatggtcctaagactaagaagaagcgtaacaaccgtactgccagtgctaacacgattcctcattcaactggtgctgccaaggctattggtttggttatcccagatcttgccggcaaactccaaggacacgcacaacgtgttgctgtcgttgatggttcattaactgaattagttgcagtccttgacaagaaggttactgctgacgaagttaacgatgctatgaagaagcacaccgctgacaaccctgcatttggttacaacgctgacgaaattgtttcatcagatatcattgatgattcacatggttcagtatttgacccaactcaaactgaagttactactgccggtgacagccaacttgttaagactgttgcttggtacgataacgaatggggcttcacttgcaacatggttcgtaccttgttgaagttcgcttcactttaataattaattgtaattggcggaggagggtggccttctccgtcttttactatctcgctatgttctctagatcacaaatcaaatcgattttgggaggtttccaaattggcaaaattaacagtttctgatttaaatctcgaaggaaagaaagttttgatgcgtgtcgactttaacgttccgatcaaagacggcgttattggtgacgataaccgtatccaagctgctttaccaaccattaagtacgttttggaccacaaaggcaaagcaattctttgctcacatcttggccgaatcaaaaaagaagacgacaagaagggcctttcattacgcccagttgcagaacgtctttccaacttattgaacaagccggttattttcgttcccgttactgaaggtaaacagcttgaagacgccatcaacaaaatggaagacggcagtgttctcttatttgaaaacactcgttatgaagatgtcgttaatggtgaatacgtcaagcgtgaatccggtaatgatcctaaattaggtgaatactgggcttcacttgccgacgaattcattaacgatgcttttggtactgctcacagatcccacgcctcaaacgctggaatcgccgaagcaatgcacaaagacggcaagccagttgctgctggtttcttgatggaaaaagaaattcagttcttaggcgaagctgttaacaatccaaagcgcccatttgttgctattctcggtggtgccaaagtttctgataagatcggtgtgattgataatctgcttgacaaggcagacaagatcatcatcggtggtggaatgacttacacattctatgcagccaaaggaatcaagattggtgactcattgatcgaaaaagacaagattgatgttgccaagaagatccttgaaaagggtggcgacaagatcgttctcccaactgacaacgtggttgctaaagaatttaagaacgacgcagaacacaaagttgttgccggtgacattgatgacggctggatggctttggacattggtcctaagtcaattgaagactttgaaaatgttcttaaagatgctaagaccgttgtttggaacggaccaatgggtgtctttgaaatgcctaactatgcccaaggaacccttcgcattggtaagttccttggaacgttaaacgatgcgactacaattgttggtggtggtgattcaactgccgctgtcaaacaattaggcgttgctgacaaattgacccacatttcaactggtggtggtgcttcacttcaatatcttgaaggtaaaacactccctggtattgcagcaattgacaacaaataattgacgaagagcttgctatttagcgagctctttttcttttactaaaaattggtataggagaaaaatgtggcttttaaattctcttttggttacaatggcattaagctaaaaaatgtaaaggatgattcttatgagaattccgttcgttgcgggtaactggaaaatgaatttatcagtcgctgaagcagtcaaatttcttcaagccatcgagggtgaattacccgatcctaagataaccgagacctgtattgcggcttcaccactctttttggagagcatggtcgaagaaaatggtgattcaccactgattatctccgctgaaaattgtttttatgaagacgagggcgcatacaccggggagactagccccaaagcgcttgccgaaatgggcgtgacccacgttattattggtcattcagagcgtcgtaagtactttaacgaaaccgacgacattattaataaaaaggttcacgctgcttttcgcaaccaattaacaccaatcatctgctgtgatgaaacgatgagccggcgtgaatccgctgatcgaatttcctgggtggtcagtcaagtgaccaacgcccttaaatcgattaccccgcaacaagctgagaagatcattgttgcttacgaacccagttgggcaatcggcagcggcaaaaccgccagcagcgatgaagccgaagagggttgttatttaattcgtcaaaccattgctgatttgtatggcgatgatattgccgatcaagtccgagtcttgtatggcggcagtgtaaacgacgaaaacgccgatgacattctgtcacagactgatatcgacggtgttttggccggtggtgccagcttaaaaccggattcattcttaaagcttgcaaactttttacaaaaatagttaaattcgctgatttatgttgaaacttcggcgagaaactaatagaattgaagttgaaccttgtacaaaaggtcacaactttcgctaaggagagaaaaaaacatgtcaattatttctgatatttatgctcgtgaggttctagactctcgtggtaacccaactgttgaagttgaattgtatactgaagcaggtgcaatgggccgtggaatcgttccttcaggtgcttcaactggtgaacacgaagctgttgaactccgtgatggtgacaaggatcgttacatgggcaagggcgttaccaaagccgttgacaacgttaataacatcatcgctaaagaaattgttggctacgatgttactgaccaattggctattgataaggctatgatcgaattggacggtacccccaacaagggtaagttaggtgccaatgcgatcttgggtgtttcattagctgctgctcgtgctgctgctgatgaattggaagttccattgtacaactaccttggtggtttcaatggtcacttgctcccaacaccaatgttgaacgttatcaatggtggtaagcatgccaacaacaaggttgatttccaagaattcatgatcatgcctgttggtgctccaaccatcaaagaagctattcgttggagttctgaaacattccacaacttgaagaacttgttgaacgaacgcggatactcaactgccgttggtgatgaaggtggatttgcgcctgacttgaagaacaacgaggaaccatttgaaatccttgttgaagctattcaacgtgcaggctacaagccaggtaaagacattgccattgcctttgactgtgcagcatcagaattctacaacaccgatactaagaaatatgatttaaagggtgacggtaagtcatacactgctgatgaatttgttactttgcttgaaagcatcgttgacaaatacccagttatttcaatcgaggatcctcttgatgaaaacgaatgggctgattggcaaatggctactaaacgccttggtaagaaagttcaaatcgttggtgatgatttgtttgttaccaacactgattacctcaagaaaggtatcaacatgggcgttgccaatgcgatcttaatcaagcttaaccaaattggtactttgactgaaactgtcgaagctgttgaaatggccaaagaagcaggctacactgcaatcatttcacaccgttctggtgaaactgaagataccacgattgctgacttggttgttggcctcaatgccggtcaaatcaagactggttcaatgagccgtggcgaacgaattgccaagtacaaccaattgatgagaattgaagaccaactcggtgacgttgccgattacaaaggaattcactcattctacaacttgtcagaacaagcacgccaagacatcttaaacaagtaatttgaaaaaagtcgtgaaagcgactttttttgtacataaaacgcctccatttttgcgtatctaactcttagatcataaataatggaggtattattttgaaaaaaacacttttattatcagtttcgttaggcgtgctgggattcgccagtccactggtgcatgagcagattgttggtgctgaaatcagtcaaacagctacccaggagtttcctgacaaaattaccatccaccaacagtttcaagttagaaacatccgtggtgacaagtcggtgcttgacaaacaagccacagtcaagatgtacattgataagagtaagtcgtcaacctttagtgccccggacaacgttccacattaccatccggtcgtttccgaagtgcattattctcccggaatggtggttaactatatggcagaagatgctgtggtgaccatcaagtaccttgatgaaaacaaccaaccaattcaggacaacaaggttttcaatcaagcaactatctttgggacctaccgccttaataaaaacgaatttgacgtttcaggttatgaactgctcaattcaaaggatatcaatggaaaaatcaaagagaccaactgggatgtgaccctcaaatataagagccttaatccattgattgctgcggattggttggctaatgtggttgtaccagaccagccagaacctggtaattccaagtctggtgaaactgggcagacaagcgaaccaattcagctcgttagtgaaaagcccatgagcgagtctgcttcaacgccggtggtttcaacgactgcgacaactgacatgcaaccatcaccaagtacaccgagcgaggctggcaatcatgtcgttccatcggttacccaaactgaaccaacgcaccaaccggctgtcaaaccagtcgaaacgcccgataaagaagtcaaggacactaccgcttccaagtccggccccaaacatgatgataaaaaggtgaaggtagtgggtgccacagggactgaaaacagccaagtaaccccaccagtggcggcgccgggaaccaaattgccggatcctgaaccaaaaatccagcccaccactaaaaccaatggggcgtcatcacggtccgataaagagactcgtgttactaaacctgaaagcaaaaaggaaggcgcagttgcagattcgtcgactaatgcaaagtcgacatcatccgttcagtccgaaaccggcaaaaaatccccatcatccaagccggtagaaaccacagccgaatcactcaaacccgatgaaaaagtgcagggaatttcaaaaacgtctgcgaagccgtctgaaaagccagccgaccttcctggtaaaaccacagatcaatccggctccacaaagaacacagttaagacttccgaatctgattcaaaagactcagaaaaaccggtcgttcaaacaaaacccaaaattccgaaaatcaaccagacaaaggtacccgaaaaatcaaccgatcatcaggaaatgcaaccaatgaccacaacctatcaactccatgggatcgacactcacggccacttactcttcaataaagccctgcatctcacttcagaagaggctcgggcattccggtcaaagaacgtcgaattttatggctatgaattacagtccaccgacctggatgcaagttcgaaaaccctgacattgcattatactgctaaaaaagtcacctttaatattatcaacgtggatcaggatggcaaaaccatctctaaagactcagtggaacttgaatatggccaaaccaagacttacacggccaagtttatttcaggttatcgggttcagcaaccaactcaggaactgaaggctgacaatctgatgcctgaagatgtgcacttcacttacatcaaattagctgacaaatcaaacaagccattagctgaaccgactgcactcagctcaaagactggccacaaaaaagggcgtcaatcagctatcagtggccggaatccgtctgaaaccaaatcaaagcgacacagcgaaaccaaagacacttcggaagtttcagaaaagcttccccaaaccggtgaatcgcagtccgttgtcggtgttttatcgggggtggcacttcttggcgcgttaatcggcaaaaaacttttcaaacgactcatttgattatgatataatggatatcagaaatcattaaaggatgagcaaaattgcaggtaagaggaagttacaagctgtctcaagtaaaaacaatcgttaacgggatcgtcattggtgtacttgccggttcggcagtctcaatgtttcggtggtcaattggccatatgacggatttgatgcgctatctttatatcaattcgatccatcatctgtcgtttctactgacgacaattgtcattaatattgccattggcttactggttggctggtttctaaagcagcagccggatattaaaggatccggcattccacaagttgaaggtcaattgttaggtgaggttgattacggctggtgggcgattctgtggcggaaatttgttggtggcattttggcgattggaagtggtttataccttggtcgcgaaggtccctcaattcagttggggtcaactttggggcagggagttgcccatttcaccaaacaagttgggtttgatcgccaagtgctcatttccagtggtgccgctgctggcttaagtgcggcttttaacgccccaattgccagtacgctgtttgttttggaagagatttatcataacttttccaccaatatttggattgtttcgctcacatctgcggtcacttctgacatggttgcgacgtatgtttttggcctcaagccggttttatacatgcgaagtacgccactgccactcaaatattttttgtgggttgtcattttaggaattgtccttggcgtgttgggccggttatatcagatggttattcttcggatgggaaagtggtatcggcatactcatattccctggtacttcaacggaattattccgctgttgttggtgatcccaatgggagcgtttttcccgcacttgttgggtggcgggagtgacattattctgaggttgagttcggcaaattatccaactctgattttatgtctttatttcataattcggtttgttttctcaatgctttcatacgggagtggccttcccggcggcattttcctgccaattctttgccttggtggtttaatcggcgcgattgtcggcagtatcgctgtcaatcttgggttgatgaatccactgtatttctcgagtttcattattatggggatggccggatactttgcggcaatcagtaaggcccctttcacggcaattcttttgattacagagatggttgggactctgacccatctccttggcctggcggtcgtgtctttaatcgcatacggcgtcttagacctgttaaacggcaaaccagtctattactcgatgcttcagcagctgctgaaagttcagaccaagatgaatttgggtcgaactgctgaaattatggaaactgtgtatgccggttcacagatggatggcaaaatggtgcgtcagatcaaatggccaatggggtcactgctgaccaagattcaacgaaatggtgtcgaaattgtgcctgctggcggcaccttgattcgatggggcgatacattgttcattaacgtctcgactaaaaatcagcacgcgatcactcaacaaattattgccttaacaacagaaacttaatcccaaaaggtagcgaattctgctataatgtgttagtttagtaagagtagtattaagccgatttaacggtaggaggctatcaacgtgtacaactttttgttaacattattgctgatcgactgtgttttaattacaatcgcagtgttaatgcaaccatcaaagactaatgacgccatgtccgccttaactggtggggccgacgacttgtttgcaaagcagaagccacgtggctttgaagcattcatgcaaaaaactacacttgttttagggattattttctttctcttagcacttgcattagtttggatatcatctcattagtattcaatcctcctgtttaaatgcaggaggatttttattataattgaatgggtggacatgaaaggatgggtgctatgcaaacaccagtcaaatctttttattttgaacacggaccgagagcaattattctgttgcatgcttttgccagtggcccggttgacgttcgaatgctcgcgaggtatttggagcgtcagaattataccgtgtatgcgccaatgtttacgggccatgggacggctgattttaccgatatcctgattcagggaacgcccgagcgttggtggaatgatgccaaacgggccgtccagtttctaaaggacaagggctatgaccaaatcagtatctttggcatctcgctgggcggtatttttgccgctaaaacgctggagaatgatccgactttactcggcggcggttcgtttggatcaccaattgttcgaaagcgtcagtttagtgttcataatacctttatgcaaatggccaaagccaattttgttcagtatgataccaatgaagcgattatgaattcaaaactcaagtggcttgacgaaaatattgatatactattaggtaagattgctgatttcacagttggtgtggcgcaggatctacctaaaatcacccaaccatacttcatcggtcaggggttaagcgatgagatcgtgaatcctgaaagtgccaagtctttgagggatggattggtgaacagtcgggtcagttaccacgaataccccaacgccagtcacatgattaccgttaatcctgctcacaagcagcttgaggctgatttaaccgaatttttaacacaactttatgaataataagaggaatatagattgcaagataatgatttgaaaaatcaaatagaaaacgttctccgaacctatccggataacgtgtttactgtcgagaaaattgctgacgtcctgagatcgcatggttcagcagcctttaagctgattgttcaagaattggcttctttggaacgcgataaagtcgccgttgtgactgaagacggcaagtttcaattgaatcctgataaacaacaattaagtggtattttccacgctaatgacaaagggtttggtttcgtcgcttatgatgaaaatgctccagatgcttacattgcgcccgataacaccatgaatgcactgaatggtgatactgtggaaatggaaattgtccggccggcgcaaccgggatctgatcggggcccggaaggtaaagtcactaaaattgccgaacacaaatatacccgcgtggttggaccgtttgaaaagactgatgatgacaaaggatacattggtcaattaaccctcaacgataagaaaattgccaagtacaaattttatatcaacgacgttggcctgaaaccaacacctggtgaagtgatcactgctcaaattaccgaatatccatctaccaagcaccctgattacatggtggggattgccgatgaagtcatcggatcagttgatgaccctggaattgacattttacagattgtttatgcccatgatattcccgctgagttccctgaagatgtcattcaggcagcggatgccatcccagatcacgtgactgaagccgagaagattggccgagaagatattactgatcaggacttggtgaccattgacggggaatcttctaaagatttggacgatgcggttaccgcttggaaactccccaatggcaattatcatttaggggttcatatcgctgacgtgagccattatgttcaacccggcagcgccattgacaaggaagcattccgtcgtgggacttccgtttatctgactgaccgtgtgattccaatgctgccaagacgtttatccaacgggatctgttccctcaacgaaggcgaattacgattatgtatgagttgtgagatggagattgatccatccggcaatatcatcaagcatcggattcaccccagtttaatgcgttcaaccgcccgaatgacctacacagcggttaacaacattttggaatctcacgatcaaaaaaccatggaccgttacgataaattggttcccatgtttgaaaccatgggtgagctgcacaaaattttatacaagcatcgaaaagcgcgtggggcaattgacttcgacgataacgaagcagaaattatcgtggatgacaaaggccacccaatcgatattaagctgcgggttcgtggtactgccgagcggatgattgaatcattcatgctggccgccaacgaaacggttgccaagcactactatgaaaaacacgttccctttatttaccgggtccatgaaacgccggatgccgatcgaatcagaaccttctttgagacgttgaccgcattcgggattaatgtgaagggtgatccagagcacgttaccccaaagactttacaaaatgtcttgaaaaaagttgccggcaagcctgaagaaatgatggtttcagtgatgctgctgcggagtttgaagcaggctcgttacgccgatcagtctttgggacactttgggttggcagcaccgttctatacccatttcacatcgccaattcggcgttatccagatacaatggttcatcgattgattcattattatcaagataacgggattaacgatgagaccaagaaacgttatgccaacgtgttggatgaaattgcgacgacgacttctcaatacgaacgtcgggccgttgatgccgaacgtgataccgattcaatgaagaaagctgaatatatgaacgatcacatcggcgaagaattcgatggggttgtcagttcagttatgaaatttggtctgttcattgaactgccaaatacggttgaaggcttggttcacatcagtcgaatgaacgacgactactaccaatacgtggaacaatttatggccttggtcggtcgaaacactcgtcgaacctacaagatgggtcaggcaatcagagttaaagtggtcaatgttgacgtcaagcagagtgccgttgactttgatattgttgatcctgaaaagacgccacaaagtaacatgctgccaaagcggacttatcataataataactatcatggcaataacgagcgccacggcaattcgaataacaattcccgttccaatcacgccaacaacaaccgtgggagaaacaacaaccatggcaacaacggacatcggaaccataataaacattaagctgtaagcgaggtgatttgatggccaaaggcaaaaagcagcataataacgataatttgatggcgcaaaataaaaaagcccgtcatgattattcgatttcagaaacctacgaagctggaattgtgctgacaggtaccgaaattaaatcgattcgtgctcggcggattaacctaaaggacggcttcgttcaaattcgaaacgatgaggcctacatgatgaacgtccacatcagtgagtacgctgaggggaaccaatttaatcatgacccgctgcgcaatcgaaagttgttgctgcacaaaaagcaaattcgcaaattggctcaaattactcaagacaaaggggttacaatcgttcctttaaaggtctacctcaaaaatggttttgccaaagttttaattggggtagcaactggtaagcatgagtacgataagcgtgaaaccatcaagcgacgtgatcaaaagcgtcaaattgaacgagttatgaaacattattaatcaagctcaaacaaaaagcgatgaaatcaattggcaagctgccgactgattcatcgcttattttcattgtgcagggtcgaaatattttcactttcaagatttggtttgacgggtgctttattcaaaacacccaacttcaatcgggaagcatgtgccaacgagggatgattgagaatggcggcaatggcaagcaccagtggctcatgattggtattgtctacatccatgatccgaatgacttgatcggactgactgtatgacttgattgtcgcaatccgctggcgtccgtgcatgattcggtaagtttgtttgtcctgattaccggcaaccaaccaattaattccgttgataaaaatcgttgtgtagtgcatcgtaaaatggatcacggaaccgcccacaaattggtccaggtaatacaaatcaaatttaggcgtcatgcccagagattgttgacggacggttgccacgacttcacctgaaattgagtaaattgaaaaagtgtcgtcaatcaagccccacttgccgacaattaaatattttgtgtctcgatattgatcggtgaccttagtcgaacgggtgtgatccagttcggttaaattcaactgtaattttcgactcatagacgcatttcctttacttgtattattttcattttaacacgttctgaaattatttacgctggtgttattttaaaaatggtatggtagaataaaacgtgaggtgttgggaatgaaaccgtttataaaaaatgactggtgggatgttttaaagcccgaatttgagaaaacttattatcagcagttacgccaatttttgatatcagaatacaagacgcaatatattcatcctgatatgaatcacatttttgaggcgtttcagctgacccctttcagcaaggtaaaggtcgtgattttgggacaggatccctatcatgagcctcatcaagcccagggattgagtttttctgtcatgccgggcgttaaaattccaccgtcacttcagaatatttataaggagcttcagtctgacctcggaatcaaaccggttgaacacggtgatttggaaagctgggccaaacagggcgtattactgctgaattcagttttgaccgttcgcaatggccaggccttttcccacaaagggaagggttgggagcaactgactgatgcggccatccaaaaactgtccgctcgtgagaagcccgttgtctttattctgtgggggagagctgcccgagataagattgcgttgattgatacgaagaccaacgtggtgattcaatcggcccatcccagtccattgtctgctcatcgaggattctttggttcgaaaccattttcaaagaccaatgaagcactggaagcaatgggcgaggagccgattaactggcagctgccggaaaaggtatcgcaaacatcttagactgattttgtagaattggaggatttatcatggaattatttgaaagtcttaagcaaaagatcaagggcaaaaacattagtatcgttttcccagagggtgacgatgtccgaatccttggtgccgccagccgtctggcaaaggacggactggttaatccagtgattctgggggctaaagacaccgttgaaaaagttgctaaagacgctgacattgatttggggaacgttgaaattatcgactacctgaaccaaccagcggatcaaatcgatgaaatggttgcagctatcgtggaacgtcgtaagggcaagaccgatgaggctaaggcgcgcgattggctgaaggatccaaattactttggaaccacattggtctacatgaacaaaatcaacgggatggtttcaggtgccaatcatccaacgggcgacacggttcgtccagctctacaaatcattaagaccaagcccggcgttaaattaatcagtggtgctttcattatgcaaaagggtgacgaacgatacttatttgccgattgtgctatcaacttggacccagatgccaatgccctggcagaaattgcggttgaaagcggcaaggttgccaagaccttcgatattgaccctaaagtggcgctgttgagcttctcgaccaaaggctctgccaagggtgatatggtcaccaaagttcaagaggcaaccaaattagctcaagaacaggcacctgatatggcaatcgatggtgaaatgcagtttgatgccgcatttgtcccaacggttgccgagaagaaggcaccaggttcaaatgttgccggtaaagccactgtctttgttttccctgaattacaatcaggcaacattggctacaagattgctcaacgattcggtggttttgaagcgattggtccaattcttcaaggattgaacaaacccgtttctgacctgtcacgaggcagcaatgaagaagacgtttataaagttgctatcatcacagcagctcaggccttataatagaaataattaaacagggtaggattgcggtggttattgcgtcgcaatccttcctttttgaatgaggtgattaattgactaaaacgataacagtccattccgcggatcaaaccatgacgatcggtgagaaattagccgcatacttggcgccacaagatttgattttgctcgatggtgatttgggagctgggaagaccacctttaccaaaggacttgccaaaggattggggattacgcgaccaatcaagagtcccacatttaccattattcgcgaatatcaagacggccgaattccgctgtatcacatggatgtgtaccgacttgaagaaggcggtggcgatgatctgggcttggaagaatattttaatggcgacggggtcaacgtggtcgaatggtcaaagtttgttgccgacgaactaccggatgactatctccggattatttttcggcgggatgattctgagggcgacaacgtgagaacattgacttttgaggccaccgggcaccgttttgaacaactaattgatgatatattttcagaataacaatggaaagcgagcaatgatgtggcagaagaagtagactttcggttagcagaaccgagtgacggtcaggcaattttggatttgttgaaggttcttcaaggcgagtccgatacgtttttggtcgattctgatttggatgacattaccgcagccgacgaagcccaacaaattaatttgatcaatcattcccggaccaatttgatggcggttgccacctatggctccgaattgattgggattgtgaccgttgacagtgttgataatggagtcggggaagtcggcgtggccgttcttgcgggttaccaaggatactcgattggcaccaacttgatggaactggccattgactgggcaacagattttagctcgcttgatcaactggtgctgactgttttctcgaagaatgagccggccattcatgtttattacaaagttgggtttcacgataccgacgtgtactttcaagacggtcgtgaagttgtgagaatggcctttgatgtcccaaaaaaggattgaagccttgagtgacgtggttgcttattgcaactaagaccgccacttttttattaaacggacgtgatgactggttgatctcaggcacttaatgaaataacgcaaccatccctaatcttggaatggttgcgttattttgttgaatgctgggatgaaactaagttcgttccaatctctttagattgctttgacaaatggccggagcatatcgctgccaaattgggcctgttcggttaatagaatattggcacaggcaacactatcgtccagcgcgttatggtgatgttccaaaacgatgttgagcttatcgcaaagggtgttaagtttgtgattttccaacgtcgggtagaattgcttggaggtccttaacgtgtccagtgtcagatagtgcggcggttgaacttcataacgttccagtgttcgtttcaagacgctgttatcaaatgatgcgttgtgggcaatcaccaatttattggctgaaaacagcggttgaatgtggcgccaaacttccggaaaggtcggggcatcgacaacatcacgttcatgaatgccatggacgttgatatttcgccaactaaagtccatttccggattgattaatgaataaaattcgttagtgatttgattatctcgaacgatggccagtgcaattgaacatgcgctggctctttttgcgtttgcggtttcgaaatccatcgcaacaaaattcatatttttcacctcaagttaatcacattgtacaaagaacctcgtgaaaacgcaaccggagtgcttcccggctattccgccccatagataacttgtttcgtggtaaaattaatgtatatgttttgaaaccgaggaattgaaaaatgatgcaatcaaaaactgttgtagatttatatccaaaaattgagattctgttaaatgaacctttatccaaatacacccacacgttgactggcggtccggcagatattcttgcctttcctaaatcgattaaagaatgtcaagaaatgttggattatgccaacgagcaatcgctcccggtcactgtggttggcaatgccagcaacttaatcgtcaaggacggcggcattcgtggcctgacaatgattctaaccaaaatgaaccggatttcgtcacatgataatgaggtcgtcgcggatgccggagcggctttgattgacgtgaccaaggctgcccaagcccattcgttaactcacttggagttcgcagcggggatccccgggagcgttggtggagcggtgttcatgaacgccggtgcttatggcggtgagatcgccaatgttgtcagtggggcggaagtcttgacacccgacaaccacattattcacttgaatcatcaagagctggatttcggttatcggcattgcagcgttcaagaaaaccatcaaatcgtcatttcggcgaccttctctttagaagtcggcattgctgacaaaattcaaaagcggatggatcatctcaatgctctgcgggcctctaaacagccgttggaactgccgtcctgtggaagtgtcttcaaacggccaaccggctattttgccggtaaactgattcatgatgccggacttcaaggcttccagatcggcggcgcccaggtttcaatgaaacatgccggttttatcgttaatgtcgatggtgccactgccactgattatttaaacgtcatcgcccatgttcaaaagaccgtttacgacaaattcggcgtgcatctggagacggaagtcagaattattggagaagaccccaagtcaaactaggagttggtaatgcgtgcacattcttgaagcggtcattctgttaatgacgttggttgttttttccaacgttgttgaccattttgttccagcggttccggttagtttaattcaagttgttttgggactgggagccgctttgattatgcgggtgaccattccgcttgaaactgattggttcctgctattatttatcgcgccgttgctgtttaacgacgggcgcaggttccccaagcaggagttgtggaagttgcggggacccatattggccaatgcaattgtattggtttttttgacgacaattttaggcggcttgctgtttcacttaattattccaactatgccgttttcggtcagttttgcgctggcagcgatcctgtcgccgaccgacccggttgccgtgcagtcgatttccaaacgggcaaagcttccggaaggaattttacacattgtcagtggcgaaagcctgatcaacgatgccagcggcctgattgcctttaaatatgcaattgcagccacggtcaccggcgttttctccattaaaacggccgccattgactttgtttatatcagtattatgggcttcgtcagcggtctggtcattatggggctgattttgatgattgaaaactggctgtatcgacagggaatcaacgatgtcatttttagcacggtcctgcaggtcacaacgcctttcgtggtgtacctggtgactgaagaatttttgcatgcctccggtgtgattgcggtggttgccgcagggatcatcttccacttttacggaacggcaccggatcgcagtcaacccgagctcaaattggtcagtgaaaaaacctgggacattattatctataccttaaacgggattgtcttcttaattctgggaatcgaactgccgttagcaaccaccaatgtgattcaaaataacaagattaatacctttgctgcactgggaatttcttttctagcctggctgattttgttggccattcgagttgtctggatctacgcctaccaagcggtcagcagtattcgctcccgaaaaatcaaatcaattcaaaccaagcaaatgcccacctttaaggcggcgctgttggcaggattgtctggcgttcggggggccgttaccatggccggagttttatcgattcccatgacgattgataatggcagtccgtttccgtccagatcactggcgttattcgttgctgccggtgtgatcatcatttcactggtcgtggccaccgtcaccttgccgttgatttctgaggataaggcaccactgttgactcgagccaactcaacggatgatccggatgaaattgataccggttcagccgacagcgatgcggaatacatttctgaagatgaggcccgcgtctatattatgaaattggcagttcaacgaattgaagaagaacggcggcccaataatcaaaaagaggcttttgacttaattctcgattatcagtttctgattcgaaggctggaattaaaactccaagataaaaaagaaatggactccatcattgctgatgaattggcacttcgaagggttgctcttcgtggtgaacgggctgccgttcagaaattatttgacgaccaaaaaatttccaaacaggctttcttgattgccaatgccaagctgcagcgtttagaaaatcggatgatccgctcggttggtcggaaagtcaaacttgggcatggaaccgcgcggaatttcattaaactgcggaatcgcgtctctttgtggttgattcggcgcaaaacgaatgaagatatttctgatgagctggccctgattcagcgagaacaggcgaaggcggctatctcggcattatccgactactttgcccgtgacgatattgacaatcaacggtttgacagtcagtcggtttatcatttaattgtgcattatcgaaatcagattgagctggccaaggatcattccaaaaagcagatcaatgatcaggcgatgaactaccagagcctgagaattaaggccttggctgccgaacgtgaaggcgtgcaggtgctcctcgaacaaggcaatattgactggtcgatggctgcccacttaagacaatatattaactattctgaaacagttttgattatggattatcaaaacgagtagggggacttcaaatgaatgacaaagggttagtgaactttagagacatcggcggaatcagagttccttccggaaaattgcagtcaggatacttttttagaagcggtcaaattgccgggatcagccaggaacaaacggccttcctgcaagaccagtgccggatccgggatgtttacgactttaggagtacggatgaagtcaaacaggcaccggatagtgcgatttctggtgccaaatattaccatattgatattttgtctgataaaacgtctaatggggctagtctgggggctatgattaccgacggcaacaaggttcatgagaatatgcttaaaacttatgaatcaattgttttaagtcagtctgcccaacaggggtatcatgatttcatgacggatttgctggcagatgatgcaccgatcctatttcattgcttcgctggaaaagaccgaaccggctttgcagcggccgtgattttaaaggtggctggcgctgacgatcaacaaattatggatgattatctgctgaccaatcaacttcgggtcaaggccaatgaagatttgctcaaccgattcaaaaatgaaatgaatcagcagcaattggacaacctgcacacagccttgctggttgatgccgattatttacgccacgccaacgatgttttgctggaacactttggctcatttgatgggtatttgaaaaatgggttggatctgcccagcgattacattgcgcggtttagagaaaagttcgtgacggattgatattgaagcaaataaaaagggatgaaccgtcgaattacggtagcatcccatttattttgattgtggtttttgaatgagtttgagtgtgtagtagaataccagttgaactgccgttaataaaacaataaacacaattgtcggccggctccacatgttcaataacggtctgataaataattccggggttaagaacaagtaaatcgtgtgaatccgcaagaaacggccaatgaagatcccgattgatgccagaatggtgagcgccacaatgacggcgtgtttgaccaacagattgtgggcatggaacctggctgtaatcgcatcgccaaccttatccaagccccaaagcccgaccaaagttgagaaaatggttgaaatcaatagcagcgcaaacttgaaccacatcagatcgtccagtcttagcaatccgttgacaccataaggattcagtagtgacaagtggaataaatccgtcagcaggtaaggggtatttggataaaacaacagccagacgatgatcagcacccaaaacagcaggccgttttggggtttgccaacgtcaatgtggaagctgagttcaattgggataaatgccagaaacgtatttaacactaaaaaattaaacgggggttgttttaaatatgaatatagtaaggcgatccagaccagaaaaagtccccggaccagccattttgtttttgtgttcacgttaaaaccccctatcaatatataattaaactatttttcgcggagaaataccatcaatacttgatcgatccggtcatttttaatgttttatttaaacatcgtcacaaattttaatcgattatcagtttgacaggcgacaatgatataatatttctgaaaactaattaggggagagcgtaatgaactggtcagatatttttacgatacataacttgacgagcctgattgatattttggccgtttggtttctaatttataatttacttttgattgtcagagataccaaggcagtccagcttttgcgcgggattgtcctgatcttggtggttaaaattattagtgcctataccgggctctccactttatcttggatcatggatcaggtgattaattggggtgttattgggctgatcgtcattttccaaccggaaattcgtcggggcttggaacaccttggccgtggatccatttttgtcaaagggcgcaaggaaaacgaagctgcgcaaaagatgatcaccgctttggatcgggcaattcaatatatgtccaaacggcgaatcggtgccttgattaccttacagatgaatacgggtctggaagaatatattgagactggaattgcgctggacgctgatgtgagcggtgaattgttaatcaacattttcatcccgaacacaccactccacgatggagctgtcatcattaagaataaccgggttgcggctgccgcagcctacttaccgctttctcaaagtaacctgattcccaaggaattagggactcgtcaccgggcggccgttgggatctcggagttgaccgatgcgatgacagtggttatttcagaagagaccggtgaagtgtcaattactcaaaataacgaattactccgtgggatgacccgggatgactacctgaaatacttcaaagatcaattgtttaccgatgaagatgatcagacccaccggacatttcttagtacggtatccggctttattgacaagcatttcaaagggggacggtaatatgcgacaatggctcttaaaaaactgggcatatcgtttgctgtcgctgttctttgccatcctgttattcatgtatgttggcagtacccaatccagcacaaccagcaatcagtccggcaacaccaattcaacctcactaacttcaaaccggacccagacattttcagttccactttctttaaccgtaaatagtaacaaatattttgtgaccggttatccacagaaggtcaaagttcatctcaccggcccatccgcgttggtgaccaccactgcgaatacgcaaaatttcaaagcctacgcggatctctccaaattgggagtggggacacataccgtcaggattcagcaggacggtttaaataatgatttgagatatcgcttcgaaccagctacaattaaggttgatattcagccgcgggaaaccgtttcgtatccattgaccgttaaatactctcaaagaaatattgcttcgggatatcaggcaggcgaggccaacgctgacgtcaagaacgtcaagattaccggtgcgtccgatcagattaaccggattaagtcggttgtcgcccagcttaacgttccgcaaaatgccaagtcatcaatttccagtcaggcaattattgaagccctcgacgccaaacaaaacacggttaacgtggtgattaccccggctaccgcggacgtcaccttaccaatcacgccgggcaatagtaaagaactgccgatcaaactggaaccaaagggtgtcactgatgacaacgagagcttcacgctcacttcggcaaccaagcgggttcgggtatttggaaccaaggcggaattggccaagctggcctctgtcaaagtcgaagtcgacaccagcgatgtcaccaagactaagaccaagcaggtgacgttggatcctaaattaaacggcgttaaaggatttgatccagagcggatttcggtcaaaatcaccagaaataactaacaaatatttaaaatatttaaactgaaatgaggaatttttaacatgaagtattttggtactgacggcgttcgcggtatcgcgaacaaagaattaacccctgagttggcctttaagtgcggccgagccggcggttatgtgctgacccaccattcagaacgtaaacagcctcaggttctggttgcacgagacacccgaatttccgggcagatgcttgaagaagccttggttgccggcctgctttcggtaggaattgaagtgttgaacctgggaatcgtcacgacacccggagttgcttacctggttagaaatcaggaagctgatgccggtgtcatgattacggcttcacataacccggttgaatataacggtatcaagttcttcggtgccgatggttacaaattgtccgacgaactggaagaagagattgaaggcatcctggaaaggccggaagacattctaccccgcccagccgccgatggcttgggagtcgttggggattatcttgaaggtagtcaaaagtacattcatttccttgagcagacaatttctgaggacctttccggcatgaaggttgcagtggacgctgccaatggttccaccagcaagctggttaccacgttgtacgcggatttgggcattgaatttgaaacgttagccactaatccagatggccttaatatcaacgatcatgttggctcaactcatccggagcaactgcagaagtttgtcttggataaaggggtttccgctggaattgcctttgatggcgacggtgaccgttgtatcgcagttgatgagaacggtaagttggttgatggtgatgccatcatgtacatttgcggtaaatacatggctgaacgtggccgcttgaagaagaataccattgtgacgactgtcatgagtaatatgggaatgtataaggcaacggaacgtgaagggatgaccagcgtgaagacccaggttggggaccgttacgtcgtcgaaaaaatgaatcaggacggctacaatttgggtggcgagcagtccggtcacatcatcttcttggatttcaacaccaccggagacggcatgctgaccagtttgcaactattatcagtcatgaaagccaccggtaagaaactatcagagttggctggcgagatcaaaaaatatccgcaacgcttgattaacgttaaagtagctgataagaaacacgctttggacaatgacaaggttaaagacgtgatcgcccaagttgaagaagaaatgcatggtgatggccgcgtcttggttcgtcccagtggaaccgaacccctacttcgagtcatgaccgaagcaccaacgcaagatttggttgatgattacaccaaacggattgcggatgttgttcgtgacgaaatgggaattgaatagtttagacatttttcagagaatcatttatttaaatatgattttgagcagatgttgtaagtaaaacgaaagtttactgcaacatctttttattttggtctccgcgcaactgccaaagttgatatatcaatttttaagatttggtataccatttgacatcttttgttgacttttatctcgaagttaggtagattatacgtgttatataaatatatagagttcatattctgtatataccaatttatgaaatttgaggagaatactaaaatgtgtggaatagttggagtaactggaaatgataatgctgtttcaattttattggaagggcttgaaaaacttgaatatcgtggttatgattccgctggtatttatgtcaacgatttgaatggcaacgactatctggtgaagcgtaagggccgcatctccgaactcgaagctgccgttggaccggaagttcacggttctgtcggaatcggccacacccgctgggctacccatggggttgtgagcgttgacaatgcccatccacaatattctgaagaccaccgtttttacttggttcacaatggggtcatcgaaaactacaaggaattaaaagccaagtacttgagcaacaccacctttaccagtcaaaccgatactgaagtggttgttcaattggttgatcgatttgttcaaacagaggggatgacgactaaggaagccttcttgaagactttgagtttacttgagggatcttcatatgccttcttattgattgacagcacagatcctgagactttgtacgttgccaagaacaagagcccacttttgatcggggttggtgacggctgcaacgtggtctgctcggacgctttggccatgctgaatgtgacccatgacttccttgaattacatgacggtgaagtggtgacaattaagcctgattcagttgacattgaagaccgtgacggccacaaagttcagcgggacactttccatgttgatatggatgcccaagagaccgataagggtccttatccatactatatgttaaaagaaatcgacgagcagccaaacgtgatgcggaaattggcctccctttacactgaagaatccggcaagccaaacgttgattcacaattgatcaatgcaatgaaggaagccgatcgtttgtacattgtgggtgccggaaccagttaccatgccgggttagtcggtaagaaattattcgaaaaattggctcacgtcccaactgaagttcatattgcttctgaatttgcctatgacaatccgctgttgtccaagaagccgttcttcatcttcctgtcgcaaagtggtgaaactgccgacagtcgtgaagttttagtgaacgtcaatgccaataactatgagagcttgacgattaccaacgttgaaaattcaacgctattccgcgaagcaacttacacgatgctattgcacgccggccctgagatctctgtggcctcaacgaaggcttacaccgcccaaattggggttgaagcgattcttgccaaggcgttgggtgaagctaaagagcaaacgatcgccgaagagtttgatattcgccagcaattaggattggtcgcaaccgggatgcaggcgattattgatgagaaagatgtcattgatgatctcgctaaaaagtattttgttccagccaaccgggccttctatattgggcggggaattgaccaaaccgtttcattggagtctgccttgaagctgaaagaaatttcatatgttcaagcagaaggctttgcatccggtgaattgaagcacggcacgattgccttgattgaagaagggacaccggtcgtcgggattatcacacaaaagcggacggctaacttaacccgcagcaatttgcaggaaactgaatcacgtggtgctgcaacctttaccatcgttcgtaagggattggctgaggaagatgatactttgatcattccagacgtcaatgagttgatcacaccgctgctcagcgtggttcctgcacaactgattgcttattacacaagtttgaacaagggactggatgttgatcgtccacgtaacttggctaagagtgtcactgttgagtaaatttgaatagcgtttctatagaggacaggcagagaatgcttgtcctttttgtttatcaatcattttttgatgaggcatgccataaaacagacacactggataaattgagatattgtccaaaaattttcttgatatctcaaaatggtagtttctttttttgttttcaaacagaaaatgatatattataagagttgttaaagttattaagaaagtctaaagcttctttggctaattaattctatttagggcttcattttttctctgttatctaatatgatagggatgtggcctaaacggaggtgtggatcattgaataaaataattaagcatggactaactgccttacttgttacggggatgggggttttattcacagcattttctgcccaaagtacataccaacaagcttatgcttccacagcaagcagttttatctcaaaatataaaaatgacgttaccaaagcttcatcgaagtacaacttatacgggtcggtcatgatggctcaggccggattggaaagcggctgggggcaaagtcagctgacgatcgaagccaataatttctttggaattaaaggggcctataatggtgcctcggtttcgatgccgacgaccgaatataatagcaatggtcagatgattaataccactgccaattttaaaaagtatccaaccgcgtacgcttcttttgccgacaatgggtccactttaagaaacggcaccagctggaaccccaagtattattccggttcttggaaagagaacgcggcaacgtatcaagacgctgcaaatgctttgactggtaaatatgcgacagcacctggatatggtcagtcgttgattacagttatccaaacctataatttggatcagctgtttggcgagaccggggatgggtcgtcagcatcatcgtcgacctctgcttcatcatcatctgcagcatcgagttcaacagcaagcagctcaagtgccagctcagcaactgcttcgtctaccgagacttcgatgcctacagcaccaaaacttgccaaagttaaatactacaaagcttcaggcaaagatttggtaccactttccagtaaatacaagaaatattacgtatataatcatgtgaaggggtcaaccacctctgagaaacgttatacttggtcacagctgggtgttaacagtcgggttcaagtctacctggatatgcgcggagtcaagactaacagctcaactaactggtaccgtctacgcttctatagcaatgccaaagccaaaaagttctgggttagtgctccggcattgtcatttgccacgacctattctggaacggcgactggtgcgttaacgccaagtaaaacttcttcggggtacatctataaccacattgtgggttccagctatctgtcaaaaccggttaaaaaggtaaagacgattgcggccgccaacaaaggttacaatgttaataaaaccgcccttcaaaagaccaccaaggggcttattctctggtatcggattgcggacggcaagacaaagggttggattaaagcttcagatgtagtatcatatcctggatcggttgcggttgtgaaccacaaggagaccaagtcgatttctaagaatgccaattcgacttatttgtacgatcatgcaaactcgacggggaatttgcagaagcattacaagctcaatcaggttgatttacaagttggcactaaggtgacagtcgataaaattggctataaggtcagcgaccattcactttggtatcgaatctcaacgcctaattcttcaaccaagtattgggtttccagtgcctttttatcataattgaatatggaaacagccgatgttgttgaccattcgtcgtaacatcggtattgggaggtttttagcatcattaagcaattcaaacatgtcatgatgaaagccctaatcgccacggttgcggttaccggcttttgttttgtccaagcaaaccactcgcatgccagcgtggaaaccgatttcattaatcagctgaaaacgccggtggtgaagattagtaaggctaaccatctctatccatccgtgatgatggcccaggcaatcgttgagagcgactttggccgttccgagctatcattggacgccaacaattacttcggggttaaaggcgcttataatggccaatctgtgactatgagtaccggggaatatacctccaaggggaagcattatatgactgcggccgcttttaaaaaatatccaagcgttgaagcctcaatcaaagataatgcttatctgttacgccacgggacattgtccgatccgaattattatgagggaacctggacgacgaacgccatttcttccagtgatgccgccatggcactgtcactaacttatgccactgatatgaattatggtaataaattaaatgcaattattaccaagtatgatttaaacaaacttgatgggtctgtcagcaccggggacattggttctaaaattgatgcctctctcaataagcaattagctggtgactccaaaaaatcagctttaattcgagcagaaaattcacgttccaaaattaacagtattccaaagcggattattcccaactttgtttttaacgacaagggagccgtcgccatcaatcaaggcgacgccgtgatccaatttaatagtttgcctttgcagcgcgttgttcgccgatagatgtttaagggttcgcaaagtttatttgggaatccttttttcagttgcaaagtttgttataatgttactcgtgaatttagtctctcttaaattaggagcggagcaatggaaaacgattataaagtaaaagttgaaaatgttaccaaagagtatgaattattcaagacccagtctgaaaaattacgctcattcttttcgattaccaaaaaacaggttcctcatttttggtcattaatgggggtttctctgacggttaaaccaggggaaacccttggcctcatcggagttaacgggtccggaaaatcgacgatttccaatatcatttccggaattatcccccaaaccaccggttatgttgacgttcgcggggaaacttcgattgtggcaattcatgccggcttgaggagcagtttgacaggccgtgaaaatatccgtctgaaatccttgatgcaagggttaaccaatgaagaaattgacgaattaatgcctgatatcattgcgtttgccgatatcggcgattttgttgaccaaccagttaagagttattcaagtggtatgcgctcccggcttgggtttgcgattgccgtccacatcaacccggacattttgatcattgatgaagccttatccgttggtgatgatacattctaccaaaagtgtgtcgacaaaattaccgaatttaagcaggaaggtaagacgattatttttgtcagccattctctcaaacagattgaaatgttgtgtgacaaggttgcttggatcaactatggtgaactcaaaatggttggtgacactaaagaagtgacccagaagtatcgcgagttcacgcagtggtttaagaagttaagcaaaaaagaaaaacataagtttgaaactgaacgcaagagtgttcagaaaaatttcagtattaaaaattatcaaaagcaaatcactgaacaggaacaaaatgctcacccggatgagaaggatgttcccgctaagatccataaacgtttttacggctcggtcattagcgaaaaaatgtcagtttggaatcaattattgacctgggctgtgttgattgtggtggtcttcttctgcttggttaacgtttccggccattcagtcgagcacgtgattaataatccttctgcgattgttcatccatcgcacacgcttcatctgccgggtaaagaatgactttcaggttgccagatgattgtttggcaaccttttttcgaaatttagttgacagcgctttcaatattgagtatattatgttcgggtactaaataaataccttctaatcaattctctttctctcttaaaaaactgacgtctttataacgtcagtttttttatgtataatgttcttcgtgagtaaataaggggaggtcacacgttgaagagtcatgaagtattgacattaattgaagaaattaccagaaacgatggcagcaagtatattgagatcagcaatatggtgcagaatggtcgggcagaattggcagctgagcgaggttttattaagcaggtcaggatcttacagcttaatatcccacattctcctcatgtggccaaatatgagcaatatattaacgaaaattatacgatgccgactgaagatatggaccactttgaagaatggcacaaaaccccggaaatgcagaaagaagtcgacatcattcttaaagaaaatcacattagttagtgggttgatgaaatttagatgataaaatagtttgcatattttcgctggatatgatataaatatatatgtcgtttttaaagaaaatatttttgctccgtagttcagtggtagaataattgactgttaatcaagaggtcgctggttcgaacccagccggagcagtaaagatcttccgggggcggttgatcccccaaaatctttttttatgcaattttgtagttgtcagtcactcttagatatgatatattatctaagtggtcgttaagtaaatatttttgctccgtagttcagtggtagaataattgactgttaatcaagaggtcgctggttcgaacccagccggagcagttacacaaagagtaggcaatttgcctgctcttttctttttatcattttttcatttagaagtctggttatttaatcttcaatctaaccgatggcccttaagtggaatgattctctcagggcattcaaaaagacctaaccgaaaaaacttccggtcaggtcttacaacatgcaaagtaactttataaattgatttcagatggggtcgcaatgatttgccggtcaccactgtcatagacgaccagggattttggataaccattgtcgtaaggatatggtgaatcaaaagttgccaccaattcatttccttgaatgaaatcataggacaaattgccatcgttattaactaaattaaatgtgatcagatttgataattggaaaacgccttgcaggtcgttatcgatgatgtaccaaacgttatcaattgcctcatcgggtaatgatgaaacgatcgtgtagctggcgaatctggattcattgggattaaacattcataacaccttcatttctgcattgcttgtcatatgtaacctaccaaattaatcaggccaacgcaagtaattagttagagttcaaactcttgattatcagtgattaaacggacaatgtgtttttcagttcgggcattttccggcggcagcgtcatataatcgccatagattttggtcaagatgccatcgtaatcagcggggacccgaatataagtgtcctcaaatggcaacacaatcgtatcatttagttggtccaggctcagaatttctttttcataggcatattgtgaggcgagattcttgacgttcattaacgccgctttgtcgttatacatggtcatgacgctttcgcgttgttttttgaaatcttctgccgtctctgcctgctcggcagaaagggaggcatgaaacttgcgaattggattatcgatcacgttataacgcagtttcaaataaattcggctgtcgagtcttcgcatgtccaaaatttgccgccgttgacgggcaggagagtctggaattcgatccaaggggaagatatccaggaaaacgcctttccgggcgttgttaacgttgttcttctcctcaatgaaggtattcctatccaatagtttggaatagctcagagcgtaattctcgtccgtccatggggtttgaagaaaatagtgagtccctttaaggtcttgctcagccactttcaaaaattgctcgtaatccacccgcagcattccgacgtccatatcatcgtcccagggaatgaacccctgatggcgaacagcccccagcattgtcccacccaaagcaatgtaatggatgtggtgttggtgggtgattttggcaaattgtttgaaaagatccagttctacttggtgaattagtgaaattgcatcatcagccataaatatcaatccttttttgttatgtcataattataaagcataatgccataaaacgataaagttaatccatttagttgcgacactggttactaaaatatataattaaggtgatataaggtttaataattaaaggggaatggtgacagatatgagtaaaacaaatcaggatctattaaaagaagcaatcgacgtttatttgtcgtcacttaaatacttagataactttgtttctgaacccgcaactaagtacggattgtcgtttgaacaatacttaattttgcatacaatcgctgaaaaacaaaacgtctcattgatggatattgccagtgaacggcgagtaacccgaagcgcaatttcacgccaaatcaaagttctattacagcatgattatatttttcaaaaaccagctgaaagtgatcgtcgtcgactttatttacatttaactccaaccggtgagcaaactgaaaagcacgtcaacgatctgatcaccaaacgttttgacagctggatcagccgttatggggacgacaaggtcagagccattttgaaatttattaaggaattcgctgcagaagaaatgaatagcaaagattacaccaacaaatagcattctgggatccatctggaccggggcaaaactgaggctttgctgccggccttttatttgtcgaatctgttgaattcaaaagggggaacgagtatgtggatggtggctttgacaggcgtcgtttttgccgttttgacggtggctttaggtacatatttgatcaagaaccgaaacacgtcggttcttggttggctggccaatttggatttactggcattattggccctcctggttcaattatttgaggtgtttggcgaaaaatataatgcgttggtgattgccgtggccgtcgcaatcgttggtctggccgttattttgggattaattttgagttttattttctggtttatcaacgcaatcgtcgtttggcgaaaagaaggttatagtctcagcgggtcgttgacgttaatcgtcgggatcggcgttgtcctcattgatgttttgattttctttaacccaattgacctgccaacaccgattcaagcgtttgtcatgacttttttgacgatgctgattgcttatattttgctgactgtgtggaatacgttgtcttcgatgctgttgtatcaattatattttccccggagcaataaagattacatcatcgttttgggagctggattggttgatggacacaaagtcggtcgcctgcttggcggtcgcattaataaaggaatcgcattttataatcatcaaatccatcgaaccaacaagcgcgccaaattggtcttttcgggcggccagggtggtgacgagttactccctgaaagtatcgccatgcgtgactacgccttggaacatggtgccagaggggcagacactttgattgaagaccagtcagtgaatacttttcaaaatatgaagttttccaaagccttgattgataaggacgccggttcgactaatcatagaattgttttcgttaccagcaattatcatactttgagagccggtatcctttctcgggaagttggtatgcatgcttttgggattgggtcgaaaacgccattttattacctgccgaacgcagtcattcgtgaatacctggccctggttgtcatgcataagaaatttcatttggtgatgctcggcttgatgttggtcgcctcagtgattgtgggggtgctggcagggcttggaattgcttaatgtttggattgaggagttgaccgtttggttgacgccttttttttggttaaggcaaacgtgttcccccaaaccggcttgcctcacactccgatgtaaatgtgttcccccaagcagcaacctgcacataagccaacttccggcgaaatcaaactcgatttccccgcaagtcagcttatgctccggttgctaaccgctcggactcacactctaaacgtgttccgccgcaactgacgcttgtttctaagggatctttaactcaaacccaaacccaaacccggggtttcagtcaaagctcccttagaagtcgcgccacccgttggtcctcacactctaaatgtgttcgacaagccagctttctccgcttagtccgataacagcagtcaacgcaaaactagcgttaactactgttatcaccctaatgctcaaaagctaatcagcttgcctcacactcttttcatcttttcttcacaccttattcacacaataagatattaattattataaaatataactatagcaagggagctataatttccacaatactatttgtagaaaggatgattatcatgtttagtttactctggacacttatcattggtggcatcattggcgcacttgcaggagcgattgccagtcgtgacatgcccatgggctggatcggcaacattgttggtggcctgattggcgcctggctcggagaagcaatttttggttcctgggggcctcaattagctgggatggcaattttaccggccattgtcggagctgtcattttagtcctggtcgtttcaatggtgactcggggaatggcacgttaaggttacctcttttaagaaaggaggttgcaaattgaataagttttcaagattaatgatctggattgtcagcctgattgggattgcccaatcggtttggctggttgggttagtcattccaatcgactatttgtcaccagtcgtgactcagacaattcaaacggatactccttggatgatgattggtgctgcgattgtatccgcggtcgtcgccctagtcagtctgatgatgttgataacggcaatctttgcgccgaggaaggctgaccagttgcggtttgagtctccacacggcaggctgagtatttccaagtcagcggttgaaaaaattttgcagaatcgaattatgacgcaaaacaacgtcaatcatgtgactgtcaaattgcgattgaggactcggaatcgggtggttcgcgttagcgtcaacgccgttgataaactcaaccaagatctggtcaaactgggtgaggcaattcagaacaatgtcgtggatgagatccagcagttgatggatgttgaagtcaagaaagtgcgggtcaaagtgaccccgtttgaagcttcaagcagacgcgaaaaagccagtcgcccacgagtagtttaggaggaggatgtcgatgaatgcaattatgtacggagccgtcttcggaatggtcgcaggcgtcgtgtgggtctttggcggcctcagcggcatgctgacggtgttggcactgaccttgattggtgccttgatcgggaccgttatctggaagtttggcgggctcaagcgcttaatcagccaattagtgagtgatgattaaataacagaaggaaagtgagatgactgtgatggatgcaacgattcaaaaatcagatttaaacaagaagttaacctttgaaaactcggtaattgaaaaaattgccggactggtttccagaaatgtggacggcgtcctgtcgcttgatggcgggatgatgagtgaattagcggatcggttctcaaaaaccactgatccgacaaaggggattgacgccgaggttggtgaaaaacaggttgccttggacatggaagcaacgattgaatatggcgccgacgcccggcagatctttgatgaaatttgcagccggacccaaaaagccatcaagaattataccggtttggacgttgttgaaattaatttaaatattaacgatgttctgaccaaaaaagaatgggaacagcaaagtacccgaaagaaagacgatatcgcaaacactgtcaatgatgacagggtggaatagccaatggagggaaaaaccatgacacaagaaaacagcagtgtagcaaccgtattaacttatgatgacagtgtgttaaccaagattgccggtaataccgttcgtgatgtggatggggtgctgtctttagaggggaacctgattgattcggtcactgatcgtttcagtgacgagacggatccctcaactggggtgaaagtagatttagacaacgatgataaagaagttaaattggcaatggatgcagtcttggaatatggcaaatgcatcccaacggtctttaacaaaattaccactaaattaactcagacaatcaccgaaatgaccgatttgaagccaaccgaaattaaaattcacgtgaaggatttacagacacgggatgaatttctaaaaaagaaccagaagaaagataagggtgagaagaaaaaataattaaagaccattttgatcaaccagacagcaaaggggctgcgacagatttgtcgcagccccttgtggttgtcgtcttaactatgcgattgttttcgattcaggatctttttgattgtcagcatgatggttaagccaattgctaacaccgccaaagtgattgcgaacggacggttgttggttacggtcatcaaaataaaaccaatcgcgattgtgatcaacatggaaatatcaaaatgagacattttgccacctcacttactaagccatggcctcgtcttcctcaagctccaaccaaagggccagcgccgtcgggttgaagtccggccaactggaaatatgttcatatccgcgcgccaaaagcgagctttgctttcgttttttaaggtcatcaaaaatcgttaatgcaaacaggttatcttcaaggtcggtgataacggttcccaatttgtgctgccactcggcaactaggtcctggtagatcaataatttccgggcattcttgattgtatagtcgaccccttgatcccgcagggtttgtttataatcttcatactcttgcaaaacagattctttagcggtttcccactggtcattattgtatctggacactttattagccattgtcgttcctccctagtccaaaataaattcacaaacactaagaagatggtcacaaaacaatcgtttcatcccatcttcgatcgaaaatatattttgtctactgaagaacattaaacactaaatcgggaaattttgcaaagcaactcgccattaatcttctacagtggctcccagaacatgttcgaagtgatccaatgcccagtcattgccggcttgggtcaatccggcaacgccgctcttgtgaacaacaatgttgtagcagagattataagcgtcgacggcagtgtgtaaaacgcagatatcgctgcagacaccgactagatgaacggtgtcaacgtggcgttcacgcagccggatatccaggtcggtgccggcaaaggcactgtagcgggttttgtcatacatatacaccttatcatctgcttgatgctctttaaaccaaggtgataagccaccataaaattcacggccccaagtacctcggacgttgtgaggtgggaataacttggtttcaggatggtatgggtcatttggtgtatgcacatcggtcggtaaaatcacccagtcgccattggccacaaattcgtcagctaattttaaaatatgcggttccagtacctgtccagggccgccacagctcagtgcccctttatcggccacaaaatcgttggtataatcaataatcagtaaagctgtatgagattccataaatgtatccctccataatgactcgattaaaagtccaattaacttttattggctcaaagatactcgatattggccgaaaaatcaactaatttgctgattaaatttcgtctttgttcttcatccgtgaacatgtgttgacgatttggggttgacatttcaaatatgaaccgtatactggtaaatattcacagagagctggcatttgctgaaagccggcaactaaaatggcaatacttaatggcggcagccttatctgcaattagaggcaatacatattgtattgtggaacttgggtggaaccgcgttgaagaacgcccctggtactgtaataggtactgggggcgtttttaatggacatttttaaggaggacactatggaaacgaaggatcaaacaaattcactatcgcgttcactaaaaagccgacacattcagatgattgcgattggcggggcaattggaaccgggctgttcttggggtccggatcggccattcacacttcagggccatcaattattttatcctacttgattgttgggatcttttgtttcctgctgatgcgggggattggtgaattgctgctgtcagataccagcaaacattcatttcttgattttgtaaaaatgtatttgggtgaccgctgggagtttgtgaccggctggacttactggttctgctggattagtttggcaatggccgatttgactgccaccggaatttatatcaagtattggtttcccggagttccccaatggattccaccgctgattattctcttatgtctgttcgccgccaatctggtcaatgtcggattgtttggtgagatggaatcctggttttcgatgattaaagtcgtggcaattattctcctagtcgttgtcggagtgggactcgccgtgttccacgtgaatgttgacggctcgacggcttcgttcagccagctggtcagccatggcggctttttcccaactggcgcccacgggttcttgatgtcatttcaaatggtggtgtttgcctttgtcggcattgaaatggttgggttgacggccggcgaaactgacgatcccaaagccaatctgccaaaggcgattaacagtttaccgatccgaattggtttattttacattggttcgatgattgcagtcatgagtgtttatccttggaataaaatcaccacgaccgccagcccatttgttcaggtgttctcgggagtgggaattgtgggtgctgccgggattttgaattttgttgttttgactgccgcggtctccgccactaacagttgtttattcagtaccagccggacaatgtacgcgttgagtatgggtgggaatgcttcatcatttttaaccaaattggggcgtaacggggttccaaacattgccctgaacttttcaaccgcctttctgttaatcatcgttgttttgaactactttattccagcgggtgtcttcaacctggtttcaagtgtttcaaccattaactttgtcgtggtgtgggtggttttaatcatcgtccacattaaataccgccgagctcatccgaagggcagtgaggtctttagaatgcctgggtatccgttgagtgattatttgacactggcattctttgtcttcattcttggattcctattggtgaacagctcaacacgggtggcgatggtcatttcattgatttcaattggctcgatgctggtgatttaccaggtgatccaacggcgtcatggcggcaggtagttggggattgaaattgctttcggaaaaaattagactttagttattcataaaatgacgattgaagaggcaataccatgattaaaattcataagtttgacacttacacctgggtcgaggcaatttcaccaactgaagacgaattaaacgacattacgattgactatcgggcaccagccaagttcaaaggctatatgctggatcgtcatgagcagccacgggccacttttgatgatctgtcagggtttagtgcactggtggtcagggcaattgcggatcctaagcaaagccgaatgctcacatcgccgatttttctgggattcagtaattccctgctgattacggtgtgtcacgcccaagagcaggctaagctggtttcagaccattccaagttggcatatgacagtgttgccgagcacattttggcaatcctgtttgcattgatttcgccgttcttcgataaattagacgagatcagtcagaaagccgagaagttggaagggatgcacaaccgggcaatcagcaaccacagtttggatgaattggcagcactaaagaccagtctggtctatctgcgctcggccacggcaggcaacttgatcgccctgcaggagttacaagccaccatcaaggataacttgaagatgtctccggaacttgccagcaaaaccaatgaatccattggtgacctgttaattgaatacaaacagtgtcaaaccatgtttgatgtggtcggcgacgtggttcgggaaaccgagtcggcatttgggaatattttgaataataaattgaaccaaacgatgcagtttctgacgatttggtcactgattctagccattccgccgattgtttccgggttttatgggatgaacgttaaactaccatttgcaggtcgtggggaagcttggttctatacagtcgttttaacgatggtaatggtcttattgatgattgtgtatattaagaaggatcgccgcttcaagaaatagaacataactgaaagccgcttcgtggatttttcggtatacaaaaagctcgtcattcaagatgacgggctttttgtatggggcaatttgcaaataccgacgggtaagtttcacgactacatcgcaaaaacgtgcttgccggaatcatatcgtttgagtgcgttcacagcctcagtaatgttacctcgtaaaatatcattatggtcaatgtcgattattttaaagttcatcagcagttcgtcggggagatcatcgatgatgcgcctgtccatcaaaatgatgtcggcacatggcttggtagcatcgaagaaatggtcgggaataatatcaacggatggttgcagtgaatttaatttttctttgagtcgatcacaaaaatgttgaatgaggacatcgtcaacaatgggattcccagttaatgaaggttgtattttgcctactcggatatcaccaactactttaatgttcacgcttgtcaccgtccttgtcgaatttatcaatcaacgccatactacacgattgaatgacggtgggtgacaaagttggtgattcttttcttaaaattaaccatattaacaaaattataataaatgaaccttaaaaacagaccagcattgaaaacaacaggaaggaaaccgtcgaaacattggcccgtttttcaaaattacggaaattaacccgggattcaaaataagcgtagaatgccagaatgccggcgataagaatgattttaaaaaatgagatgttgagcgtgagacacaacattaaaatcagcaccgacacgatcatcatggacagctgattgttttgtttcataaaggcgtagtaggaaaagaaaatatttgcaaaaatcatcagggtgatatacatcagtgagaccagggaaaaatagtgatggtaggtcgttgtgaacaacaagacaattccggttccggaaatgaacccataaataatccaacgacagtgaggttcatcgattaaattagagactaacagcaggttggcgagcaaaaagccgatcagaatcagccagacgttaatgctcggcgtatcgaggtacagcgatgccaataagatacccagtaaaatatcggttaagacgaccatgacggcatttttgtgcggtcggctgacggcggtcaataaaacggcaaacacgaacccgatcaccaggagatgcagaaggcgcggattgacgaaaaatccctttaacgagatattggcaaatagcatccagataaagaccatgctgacggcgcgcagtcctgattgaattaaaatggagcggtcaaattttaacaaatcctcaacttcctcacatttttaatagctaattataaaaataatcctactggttttctgtcagatggtcaatggacagctgaaaataaggcttgaaaagcaaatcaaatatgataagattgtagagttatgagttcccgataggattcacgtgatgcgtgaagaagccttgtaaccttaaaaaataatagggggaaaatagaatgcgcgaaaaacatttatttacttcggaatcagtttcagaaggccatccggataaaattgcggatcagattagtgatgcaattctggatgccttgttagcaaaagacccggatgctcgggtagcatgcgaaacctcagttaccaccggactggtgtttgttttcggtgaaatttccacgactgcctacgtggatattcaaaaagttgttcgcaacacgattaagcgaatcggctatgccgatggccgttacggctttgatggtgattcatgtggtgttatcgttgcccttgatggtcagtcacctgatattgccttaggtgttgatgacgctttggagcaacgtgaaggcaataccgacccgttggatcaaatcggtgccggtgaccaaggactcatgtttggctatgccattgatgagacacccgagttaatgccgttgccgatttcattagcccacaagctgatgagaaagcaggcagacttgcgtaagagtggcgagattggttatctgggcccggatgccaaggctgaagtcactgttgagtatgatgacaacgccaagccggtccgagttgacacggtcgtcttaagcactcagcatgacgatggtgtccgattggatcaagttcggaccgatgtgatcaaccaaatcatcaaacaggtgattcctgccaagtatcttgacgacaagacccgttatctggttaatccaaccggccggtttgtcattggtggtcctcaaggggatgccgggttaaccggacgtaagattatcgttgatacctatggtggttacgcccaccatggtggcggtgccttttcaggaaaggatgctaccaaagttgaccgttcggcaagttatgcggcgcgatacattgctaagaacattgttgccgccggtttggcaagcgaagctgaaatccagttggcatatgccatcggggttgccaagcccgtttcaatcgacattaatacatttggtaccggtaaagtgcctgaagatcaattgattgatgccacacgagcattatttgatcttcgcccggcaggaattatcaaaatgctggacttaaaacgaccaatttatgaacagaccgcagcgtatggtcactttggaagaaccgatattgatcttccatgggagcataccgataaggttgatgcgttaaaagactatttcaagttataaacagctgacaagcaaaacgcccttgaaaattcaagggcatttttttgtttaattttaaagaaaagaggtcatttcatgacgaaaacagcaaccaaaagtaatgtaaccttagtaacgattgccctctttgtggccacctttatggccgcaattgaagggacaattgtttcgactgccatgccgacgattgtcggtgacctgcggggagtttccctaatgaattgggtcttttccatttttctgttaaccaatgcaattgcgacgccaatctatggtaaattggccgacagtattggccgaaagccaatgtttattggtggaattttgatctttgtctttgggtcggtgatgtccgggttatcgcactcaatggtggttttgatcttttggcgggccgtgcaaggggttggagccggctccatcatgccgatttccaatacgattatcgccgatatttatcccctggaaaagcgcgctcaggtgttgggcctgaactcgtctgcttggggaattgcttctgtgatcgcgccactattgggtggtttcattgttgatcacttgagctggcactggattttctttatcaatttacccattgggttgattgtcatggtcatggtccagattttcctgcatgaagacaaacaccacagtaccactaaaatggacattgccgggaccacttggctgacgatgatgctgttggcagtgatgtatgcgttccagttggtcggccaggatccgatcaactggcagatcgttgcggtctgcttcttggttacagtgatcgccacggtcatgtttattcggacagaaagactggcggccgatccgttaattccgatggaactgtttgataatcggaccttcgtcgttcaaaatatcgtggtttttttggtcagtggctttctgatcggctacgaagtttatctgccggactggacccagggaattttgggcctgcgggcatcgatggccgggtttgcggtgacgccgagttccctgatgtggattgtcggctcatttttggccggtaaattgctggccaggacgtcaccttaccgcattattaacctcagtctcttctttatcttggttggggccattattatggtgctgattccggcatatacgccgtttgtggccttcttggggatttcaatgatctgtgggaccggctttggcttaacggtgacaacgtcgattattagcgttcaaaatgaggttaaaccaactcagattggtgtggcaacttcctttaatactttgtgccgaacgctgggtcagacactgatgatttcaatctttggtatcgtcatgaacaccaccatgctgcgtggggtccggcaaacggaacatacatccttgaaaatgatggacaaactgattaacccattgactgccaatcagttaagtgacaaaattttgccgcagttgcgaaatattttgtacaattccctgcataatgtctttgtggtcggcttgattctgattatcattgcctatatctgcaatttgtttgaccgcaaaaataaaaaacagcgaatcaattaatcgatccgctgaatcgccatcaatattggtggaaaatgctgctgatttaagaagctgtatttcaaaacactgtatcgtttttggtcgagttgactgccaaattcgaggacggtgtttttttcgcgttcgccgcctggatgaccatagtaggcaaccacgacgatcacgccattatggcataagtggttgaggcagcctttaatcgccgcaatcgtcgtttcagggtaggtgacaatcgtcttatcgccgcccggcagatagccgagattgaagatggcgccggaaatcatggtctcgtatggtaaaatttcatcaactttggcatggctgatattgtacaggtagacgtttttggtgcgaacgtgattggtttttagaagtgctttggtattttcaactgcctgggcttgaatatcaaatccatacacggtgccttgtttgccaactaaattggctaaaaacagggtgtcgtggccgttacccatggtacagtcaacgacggtatctccggaatcgacagtttctgataacagttcatggctatattccaatgctgatttgattttcatgagatacctcccgcgaatcgattaaatacccattgtgacaccattaaggtcactaggccaagactccagccgcccagaacgtcactggcataatgaacgccaacatatatccggctgatgccgataccgacaatcatgatgatcaaaatcagatcaacgatcagccgttggctacttcctttaagcatgcggttggccagcaaaatcaggctgccggcaaccaccatgatactcattgagtgaccactggggaaactactgctgtgaacagccatcagatgggtcagagatggtcgcggccggttaaccatgtgtttgaccagggtatcaatcggggctgccaagacgacgccgttaatcaacaagaataaggcggatttgattttgcgaaccaaaaataaaatcaatccggcaccgattgtgaaacccaatagtgactgataatttcccaactcggtaaaatgaatcatgaagctggtcagtgagggcgtttgaaagcttctgaccatgtggccgaagtaggtgtcaaaggtattgatccattctttatgtaaaaccacgccgtaagtcagaatcaaaaagatgaccagtgaaaccaaactaacggtgcttgaaattttttgtgattgttttttcatgttttcaactccaataataaaattatagcacgctgagcagttgttttttaagacctgttttggtatgataataagcaataatttcaatttgtgaaaatgcagagacgaattagtaaccaactgcctgttttccagaaactgagtggctgctgtgaactcagaacaggtcgtggcgaactcatcgtcgaatgcttggtcgaacgaagtaaatcaagccggtttgtcgccgttattgattcgagagctcaagtaattgagaatataggtggtaccgcgataaatcgtcctataagaagcccagtctggtttcttatgggacttttttcattgattgagaaatatgaaaggtggaagttgcaaaatggcatacaatcatgaggtaattgagcgcaaatggcagcattactggaaagaacacaagacatttaagaccgaagaagttgctgacaaagacaaatactatgtcttggatatgttcccttatccatcgggtcagggcctgcacgttgggcatcctgaaggctacacagctacggatattatggctagaatgaagcggatgcaggggaaaaatgttcttcacccaatgggatgggatgcttttggattacctgcagaacagtatgcactgaagacggggcataacccgcgagactttacggctaagaacatcaaaactttcaaacgccaaattcgttcgcttggattctcatatgattgggatcgtgaaattaacaccaccgacccaagctattacaaatggacccaatggatttttgaagaattatacaaacgcggattggcttatgaagacaatattgaagttaactgggcccctgattttatgggtgggaccgttgttgccaatgaggaagtcgttgacggtaagactgaacgtggcggctatccggtttatcgggtgccgatgcgccaatgggtcctcaagatcacggcttacgctgatcgattgattgatgacttggacgatctggattggcctgaaagtattaaggaacaacaacgcaactggatcggccgttcgcgtggtgccagcgtgttctttgaggtcaaaggtcatcctgatgacaaggttgaagtgttcaccacccgtcctgacaccctatttggggcaacatacatggtgctcgcgccggaacaccagctggtttcaaagattaccacccctgaacaagccgctgaagtcaaagcttatcaagaagaagtttcccgcaaatccgatcttgaacgaaccgatttgaacaaagataagagtggggtcttcactggtgcctacgggattaatccaatgactggaaaagaagtgccaatctggattggtgattacgttcttgaatcgtacggaaccggtgccatcatggccgttccagcgcatgatgatcgtgattatgattttgccaagaaatttggactgccaattgttcccgtcattgaaggtggtaataccgacgaagctgcctatacgggtgacggtcctcacttcaactccggcttcatggatggcatgggcaaagatgacgccattaaggcagccattgattggttaactgaccataaagccggtcatgaaaaggtcaactaccggctgcgtgactggatcttcagccgtcaacgatactggggtgaaccaattccagtgattcattgggaagatggcgaaacgacgctggttcctgaagatgagctgccgcttcgattgccaaaggccaaagatattcagacctctggtggcaaggaaagcccactcgctaacttggatgactgggtcaacgtggttgataaaaacggccgcaaaggcaaacgtgaaaccaacacgatgccacagtgggccggaagttcatggtactggctgcgttacatggatccgcataacgaccaagccatcgcttctcctgaaaagttgaagtattggtcaccagttgatttatatgtcggcggggctgaacatgccgttctacatttgctatatgcaagattctggcacaagttcctttacgatttgggggttgtgccaactaaggaaccgttccagaaactggttaaccaggggatgattcttggaaccaaccacgaaaagatgtcgaagtcaaagggtaacgtgatcaacccggatgatattgttgatgaatacggtgcagatacactccgggtatatgaaatgttcatgggcccaatcgatgctgccaagccttggagcacggaaggtattcacggggcctaccattggcttgaccgggtatggcgcttactgatcgatgataacaatcatttgcgtgaccgcgttaccacgatcaatgacggcaagctggacaagatttataaccagacggtcaaaatcgtttcagatgactttgaacatatgcggtttaacgtcggcatttctcaaatgatggtctttgttaacgacgcctacaaggcagattcactgccaattgattacatggaaggcttcgtcaaactcctgtcaccggttgccccacatatcgccgaagaattgtggagtttattgggtcatgacggcacgattacctatgaaaagtggccaacctatgatgcttccaagttagttgagaacaccgttcagatggtcgttcaagtcaacgggaaagttcgttcacacattaaggttgcccgtgatcttgataaagaaaaagttgaacagactgccaaaagtgatgagaatgttgaacgatatctggaaggcaagactgttcgtaaagtgattgtcattccaaacaagatcgttaatattgttgtcggttaacgtgatcaagcaaacagctggggaattgtcctcagctgtttttatttgaacagttgaattattttcaaaaaaataaaaaaattccgccattttctccgtatatatattacgaacgggacgagttgagtcgtcttgaaaaatgttgaaggagaaagatgatggataaatttgataaagtgactttggggaaagctaatggttttaaattttggagcagtttagcgctcatggctgccagtgggttaatcatgctgcaggcaccgttggctcacgcggatttcccagcagacaacgtgcgcacgactgagttggggcagcgggtgacattttatgttcagccggtgtccaaatcggattccgctggtgactggcaggtgattcccggagtcaagccaattaagatggtcggcaatataggggagtcatttcaagtaccggtttatcagaactttgttccaaccgcaacgatttctcatacagttccagattctcgtgcagacttgcagcacccgctgttgctcaaatatcgccaggaaagtactggcctctataccgcaacggtgaatattaactatatgaatcgtcaagatagtcacacgctggacaccgccaccaaaacgctgcattacgctgaccaagtaaccattaagccaaagaagattcagggctatcagccggttgaggcaaccttcgaaagcccgtatttcactaaaaataacgatcaatcggtgaacttctggtttagagaattaagggatctgacttgcttggtaaaattctggtatcggccagtgaatgcttctcagccagatcagcctgagcaggtcaaagaagcccaggcaaagccgaaccacgctggtgtgtctacgagttctcactcaggcaccgattcaaaacttgtggaagctgccaaaccggtgacacaagacagtggcgacacaaagccagccagttcgaatgtagcgccggtattaccagtcaactcaactgatcaggcgcaaaaaagtgctccccaagttgaagttaagcaacaacggcccacggttactcaaccaactttagtaactaaagaaccggtgttccaggcggttaagcctgttgagacgaaagctgcaagtcttccgtcagatttgtctcaggttgcacaacaatcgccagtggtcccgtcaaaaccaacgaattcgacgagggttaatgtggcgggaaaaagtcaaatctctgttagtcggccaacagagagtgtccgcacgtcatcccggccagcgactgattcccacctgggagcaattggggtcgcgatcttaaacaacccaatgaacgcaggccaaactacaataacccaaccgactccaaacaaaaaagtcgccgtaaaaggggtggccgtctacgccatcaaaacggtcgggctatacaattcccccaattttaagtccggcaatcgacttttccgatatccagctcaaaagcgctatgcccgacccatgtttgtggtgaccggctatgctcgttcagccactggccagttgcggtaccgggtacgggatgtcaatcatcaaagtccttcccatggcaaggcaggctatctaacagcaaactggacctatgtgagaccagtttattatgccagtcgtcacccaaaaatcaaagtgatcaacccgactggcattcatggctatcaaggtaagaatttgactggtagagttgccacatacaaaaagggccagactgtcaatgtcaaacgcatggttcattatcatttaacaacgcgttttgtcttagccgacggttcatatatcacggctaatcgtaaattagtgagtgcttttaaataatcagccacaggaatgaaaaacagccaaaatccacaatggattttggctgtttttgagttgctattgcattaattcactcgcagaactatcttggtaatttttattccacaggaattccgttagaattttattgacggcaatgttgttattgtgcagggcactgtgttgcgccttgggaccaaaagcttgaaatgtttgataaaagctgacgtgatctcgcaaaatatagcctaatgatagggcagaagcgttggtgacaacgccatctgaatttgaaccatcgcccaagttaccataaatattcaaaaccctggcttgacgagggaaattttttctcagccgatagagtaacttgtattcaggatggatgatcttgggtttaccagtcggcaaaatgcgatttttattgggcgcatcatcccataactgcatcagtgggccggatgtcggctgattggacttgtgattatccatgatcccatcataaggcccggcgatcacacataacttattggttcgtggcaaatcagatcggttgccgttcaaaaggttatagtagacgacggcgtaagcccccatggaatggccgacaaagtttaattgattgacatggtatttctgcttgagtaacttgcagaccttggtcagccagcgggcatactgaacctcgccggcgcggttattgtccattcggaccataatgattggattaaccatccatgacttaaccgttccagtgactgacaattttccgttggctctcacgcggacaatcattcgccttgaagcggccccactaacctcggctgctgagatcatatctttttcggaacgaagggtggcaccccagccgtggacaaagatagtcggcgtactggagtcaatatagttggccttgagctgatccgaagcacgctgatcctgccaaatgttaaaaccgaagcccaagatgatgagcccgccgattacaaagtaaagtattcgcaagtttcttgagcgccgataatttatcaactaattgaccgccttatacgtgaattctttattttttgtttgacatagccgtagcccagtgacaggataaacgaaattaaaaccgccagaattgtttccataatggcaccattgtagccagcttcatcaataatgtcgatgacagccttgtgcagatacataattcccaatgtctgttggcccaataattgaaccggcttaatgagaaactggggcatgaatttgcagaaatagtaactggcgctgaaaacgactagacaaacaataatcgggataaaagtaatgtaggaaacccgagaaatcggaatgtggtgataggaagcgtgaatgattttggacttcaggaagaacgcgaagttgaaccggtccatgtgctgcatccaaaacaaccagacagtcagcatggctgctggaataatcacccacaggtccttaacgaattgctgaattttatggaaataaagatagccaaataacatgaagaacatggcgataaaagcaacatcgaagtcccaaggcacgtatttataacttaggaagtaaatgtgcttgtaactggtggaaatgattaatgaagcaaaggccacaataatctgtgcttcccggcttttgacgtatgtaatgacaatcgatgtgaaaaccagggccaacaggtaaacattaatgtaccaaaaaacactgaggtagtggttcagtgtccgtccaccgtacagtaatcgggcaaagtagaaaatcgtatacgaccaactttcgcctctgatgaagtgtgacagtaaaatcaaaaagccaccacagattaaatatgaaattagcagtggtaaaatccgtttcttgaaaaaaccgatccaattgttattgacgattggctttaagaaaaagccccccatgatgaagaagatcggcatgtgccaccaataaagaaaatggaacatggtgccgtgtcgtgtcatggcgtgaccgaaaacaacggcgacaattccgaccgctttggcaacgtcaatccactcgattctttttttactcacaagtgtttcacctcgaaaattattaagaccacatataaaaatattctagtgcatttagggtgttcatgacaatactttttcattacatctctataaaacaattgatgcttaagtaatttttaatatatcaccccgttattgctattcattagcaacttgattaaaatgaagcgagtgtcaaagtatacgaaagtaggaacaatcatgattgataatcatcaaaacctgacggaaaagtcgcgtgaccagatgttatccgggtcagcgtggatgacggccggtagtattttgagtcgatttctcggtgcagtctatattattccctgggggatttggtttggcaattatttcttccaagccaatgcgctgtacggactcgggtataacatttacagtttcttcttgatcgcggccatcgcagggattccctcagcgatcgccaaacaagtggctcattacaatgccttaaatgagtatggtgtcggcgttcggctttataaacggggcttggtgttggccattgcgacaggagttatctgtgcggtgatcctgtattttggtgcgcccttaattgacggcggcaatcccaacgtcattccggttttgcattcactggcatgggcaattttgattattccgacgatgagcctcacccgtggttatttccaaggttaccaacaaatggcgccatcagcgatttcccaatttgtcgaacagctggctcgagttgcctacatgcttttaacagccttcattatgatgcgggtgctgcatggcagttgggtcaatgctgtttctcaatcaactttcgctgccttcattggggcggttgccggcctggcgacccttggcgtttattacttccgccgccgcgaagattttcgacagctggttttgtccagcaataatgagatccacgttgaagcaaaacaattatatcaggaaattattgcgcaggcagtgccctttattatattgggtgccggaatcacgatttttatgctgattgaccagttcactttcttcaagattatgcggatggcgactgattacaactacgcgaccctgtccgatctatatgcaatgtttgctgtgaactcaaataaattgattatgattactgtgtcgctttcctctgctttggcgattaccgccgtgccgatgctctcagaagcgctgaccagcggggacaacgtcgaaattcgcaaacaaaactccaatgtcatggcattattcatgtttgtcatgattcctgccgccttggtaatgccgcaattgccggaccgcttaaccgggtcttctatggcaccactcatcaggcactcggcgctaatattctaacgttttcatccattatctccattccgatgggattgtttgttgttatttctgccgtgatgcagggattgtctcaaaacagacgggcagttaagttctttgctgttggaacagtggttaagtttgtgcttcagtggccttgtacctattttttgggttcatttgggccactgctttccaccgggattggcttgaccgttgccaactggctgattcttagatatttgaaccgccatttcggttttgaaaaacggatgttggacattgcttttcggaagatttcgaaatattcattgtttatgtatgctgctgcactgttgacggtttatgggttgaattttgttgttcagttgattggtaatccatttggacgggttgtcagtctgatcgtgaccttggtggccgttttggttggtggggtaatttatctctacttagccttgaagagtcgaattgctgatatgattctgggcccgcgaagtgacaagttgcgacggttgcttaaaatcgaataaccagccgttttcattcatatttagccaggataaaataaacaagtctccatcactgacaattcagctgatggagacttttgtgattcaatttagttatttagcttgatgcttatacataaatttcggcagggcctcactgatttggtggggcagaacaacatattgcttttcagctaatttatctgcaatggcactatgagaataaaccgccgctaacacagctttttgcggatttttgaactgggcggcaaagcccccgaccattccggccaaggtgtcacccattccgcccgttgcctgggcaggagtgccgccagtgttttcgtagacgtggttgtccgcataaacttgcgttcgatgtgatttaaccaccacgattgcgtggagctgtttggcggctgcctggtttttctctggcgtctggtcggcaatcttaatgccggatactcgctgccattccatttgatgcggcgtcaaaatgttggtcgaatctttgggcagcggcaagttgttagcagcaagcaatgtcagtgccgaaccatcaatgactaacttttgttcgctgccggcaatccgaaagacttttgtcaacagggtcaacgcactgggatcggttcccagaccaggcccaatgaccaccacgtcggcacttttaatgattggttctgcctgatcaaaattgttccaatccacaaacattgcttcgggcagccagtcatgcagactggtttgattactggggtccgtaatcgtggtgaccaagccggctccggaataaactgctgccagtgaggccatgataatcgcaccgccaaagttttggctgccgccaatcaaagcgattttgccgtaagtgcctttaaaactatctgccggtcgcttgcgaatgacatctgttaaaatttgacttgtgatttttttgacatttatcatcatcagatctcccatccgaatctgtttttcaccctaattatagcatttctggagtggacagattgccaacgccaattgaatagtgtgataaaattgaactataagaaatggacaggagcgagaaaaatgacagttgattggaaaaagcgcgcacaaagttatcaagacgagtatttgaacgatttaaaggaattgatcagtattaacagtgttcgtgacgatgagcacaagaccgatgaatttccactgggcgaggggccaacccaagcgatgctcaaatttttatcatttggggagcgcgacggctttaagacgcaaaatatcgacaacattgttggctatattgagtatggttccggcgatcagacaatggcgatgcaggcccatgcggacgttatgcctgctggagacggctgggaaaccaatccatttgaaatggtggaaaaaaatggcaacgtctatggccgtggaacctcagatgataagggacctgcgttagccgcttattatgggttgagaatgctgaaggacaatgggattatgcccaaaatgaagattcgtttgattattggaactgacgaggaaagtgactggaccgggatgaagcattatttccaagttgaaccgcaaccgacctttggtttttccccagatgctgaatttcctctgattaatggtgagaagggcaatgccacttatgtcacgacctttggccatacaaatggttccgaattcactttgaagcgatttgattccggattgcgcttgaacatggttcccggatctgcggatgcgctggtcgaagtcggtgataacgaaaaatttgtcgacggctttactgaatttttggatcaaaacccgattgccggtgatgtcaaatcaaccggtcagggcgttgctttgcacattaccggtaaagctgcccacgcgatggaacccaagaacggcgtcaatgccggcacgtatcttgccaagtttttgaatgcctatccatttgacggggccgctaaggaatttatttcctacctggctgaagacctgcatgacgattcccgggcaaccaagatcggcgctgcgcacgtcgacgacatcatgggagagttaaccatgaacgttgggattatgaaatttgacacgcagcacggcggcagcgtcaacaccaacttccgttacccgaaaggaactgacgatcaagagattttagctcacttgcaacaggctgccgagaaacgccatggaaccgtgaaggaaatcaacaatatggacacccactacgttgatccaagtgatccgattgtcagtaccttgatgcacgtttaccaggaacagacgggcgatatggattccaaaccggaagtcgtcggcggcggtacttatgcccgtttgatgaaacgcggggtggcgtttggcgcattgttcccgaacgcccaagataccatgcatcaggcaaatgagtttcagccggttgccgatttaatcaaggcaatggcaatttatgggcaatcaatttatgagttgacagccaagtaaaaacattgaggtggttagtatgttggactttaattattcgaatattctggttgggattgatggttcaaagactgccgccaaggccgttagacaggcaatcacgattgccgagcacaaccatgccaaactgacaattgtggcaattatcaacgaccgtgaaattctgggggtgtcaaaagccgccttgatcggttttggcaacgtcaatcaatcaacgatcgatgaggtcaaatccagatttcaacggctcgttcataaatacgaattgatggcaaaagaccgaggacttgctgtcagtgcctttgtgacatcaggcgatcccaaaaataaattggcccacgagttggtggatgacgaacatgtggatgcaatcgttgtcggggccaccggggcaaattttgttgaccggatgacaatggggtctacagctgcttttgttattgcccaagctccctgtgatgtgtttgtggtccatcgcgactagccggtttcaagtcggttagaacaactgaaataaaaaaagaggtgagccggtatttcgagaatacctggttcgcctcttttgtggtccattattcaattttggttggctgatttttctgcggattgttaacaattaatccccagattccggaaatcacgtacaagaaactgcccaagacgcccagcacgattaaaacaatcggccacacataactttcattgtagtgaagtcgtttaataccaaagaacgcaatgatttgctggattccatacaccagcaaaagaaaaatggcgatcatgtgataattccatgagttatgaacgcctgcagcatccgtcgttctggtcagcataaagattgccagcgccaaaacgacaatggtgatcacccaccagacgatccagccgcaaatttgagcggcagataatttatgttgttttgtattttgcaaatctacatctcccccaatattgtttatatcaagcctaccaagagtggcctgattcagtcaaataaaagttgcatccaggccaccaaaaaagttatacttttcgaagcacgtcattgagaaatgacaatttcgaagggtgaggtttggtcatgattgacatcgtattcagtgatagttttgcatcaacattgaagtattactatcagaaaagacatcttgacgggcaggttttggcattgccaatgtacctgagcttgggggacatcagtcaacgctcgtttatggaaagtcgacaaactatttataaaatcgaatacgctcattatcaagcctctgaacaattaactgtcgaagcggtaaatgctttacggcaggggcttgatcaactgagtcaaatggctcaggccggcgaatcgtttcgcatttggtggagtgagaccgctgacgactactgcggctttttgtggatttgcgattatttaaaggatttttcagttcaaacgacgagtgtcaaggttccaatgaccttggtccgagaagacagtttgatgattatttccaaattaggtgaaatcagtgaagacgccattgatgaacttcaattggcatcactacaaagggacctgtctgctaattcccggagagccttcagttactattggcatgacttaaggagtgaaaataatccgatcagaacggtgattaacggcaccgttgtcagtcaatcgattgacttttacgatcgttttgtccttgccaatctcagtcaaagacggtttagaaatattctgcgggtaattggtgagactttgggcgattatccgttcacggctgactggtggtaccgccaccggattgattacttggtgtcaaagggaagcgtcgattataaggcggatccggacgcaatcgttgggaaaattaaattggcaaaataaaaaagggctgtttagctgtgaaatgatcagctgaacatctccttttaactccgtggccttttcatcgtatctggtagacctgaaacttatgactgtctgttagagtgtctcactttgtggttggcgaattttagccaaagcatcatcaatctgtccgagaacgattgtgacattcttgggatcggacaagtcatacttttgcaagtcgattttgatcttgggactgacatcgtattcttggaaccatttcttatatgcagcccacatcttgaagtagtattcctgaaggcccgggttgtcgtcaaactgttcatagtcgcgaccgcgttttttgatccggtgcttgatggtgtcaaagtcactatcagcatacaccagcaaatcaggagccttttttggcaactcgtcgagttctgccatcatgttattcaataacttgaggtaaaccgccaattcagtgtcggtgatgtttccctgagcattattttcccgggtgaacagtgcatcttcatagattgagcgatccaagacgttattatcatcactcaatgcttgtttgatcattgagaaacgcttgtttaaaaagtaaatttgaagtagaaatccgtattgttttggattggagtagtaaagcggtaaaacgggattgtcgccaacgggttcaaaaaacgcttttgtcccgagatgttccgcaatttttccggttaaagtggtctttccgaccccaatcattcctgcagttattatcaccatggtagcccctctttataataaaatgacaatatatagtgtaccacaaaatgtggtaacacaatatatataatttcccgattcggaagttaaaattgggaatgccgcacatattaagtagtacaatatagttaataagttaaatggagggaatttaatgtataaagcggttgtgttctttgacttagacgggacactttttgataatgaaaaaaacgtgtccgacgaaaatgtagcggcaatcaatgaattacgtgccaataatattttaccagtgatctccactggtcgaaatatttttgaaattcagtatgtgattgatgccactgggattaactcgttagtcagcgctaatgggagttatgttcagtatgaaggcaaaaaactcaaagcagaacaaattagtgatgatgtgattgaggaaatccttgcctttgcaaaacagcagggggatgtcatttccttttacaacaataaggaatttgcgttgacttttgaaaatgacatgacgaaagtgaactatcgtctgttgcgattaacaccacatgttgacccagaattttacaagcatcacgaagttaatttcttaaacgtctttaattacgacaaggataagctttaccaagacaagttcaaagggaagttgtctttggtccgtaacaacccgcgttgtttggataccatgaagtggggcgtttccaaacaaacgggaattcaggctttgatgaaaaaactgaacctcggtgacgttccatcatatgcatttggggatcaaatgaatgatttgcaaatgttttccgaagttaaatttccaattgccatgggtaatggtgtcccagaagttaaggaaaaggcgtcttttgtcactaaatcaaatattaacggtgggattgtgaacggccttaaacattatgggctgattgattaatatctcgccaaaggttgttctcgaccatttaacgacgaaaggcaactaccccgaaacagaggtagttgcctttcgtcgttaatcatcagaattagggatgaaacgaacccttaattcatttgcttttcaatattagccaacgtcatttctgaagtatcggcaaaattaatgtcggcatcctttaagatatttttgtcgccgatgccaatcgaggtttcgccagctgcgttaattgattcaacaccagctgccgcgtcttcaacgccgatgcactgttccggcttgagatcaatcaattcagcaccctttacataaatttctgggtcgggcttgcctttactcaatgtttttggatcaacaatctttgggaaataatcggttaaattcagcttttgcaagactttgggcgcgtttttagatgctgaagccaatgacaataaataaccgccatttttgatttcgtccaagaatgctttaatccccggtaagatattgtcaggggtcatttgatcaaccaacttcaagtagttggtatttttttcagttgctaaatcaaccttttgctcatcagtgtatttatcttgaagatttccagctttcaaaatcatttccaatgagtccattcgactgatgcctttcagaccgtcttcaagttctttggaccatggagcgccgactttatcggcaacttgatgccatgcctggctgtgaaaaaccgaggtatctgtaatcacaccatctaaatcgaacacgaagcctttaatatcggaaaattttgccattatcattcactccttattatttgtaggtaattgttgccatcttgttcttagtcagtgaataagcctttttcgcaacactgacgtgagtatcggcatctgcggtcacatcgatccgatgatgaccgatgacgaagtggtaattgattccttggtaagtttctttaaatgaaattttagaccaagtgcttggcaggtgaggattaatcgtgacctcgtcggtatcaaaccggacaccgccatagcatttcgtttcaatttgaagggtcgcacccattacacctagatggattccttcggcagtcgtcccgccttgaatgtcgtagtaatctgagaacagggcagttgaaaacagctgccatgactggtccatgttgccgtcaatttcgtccagaaccgaataaacaattctggaaagcgttgatccatgagtcgtccggtcaagatagaaccgtaagttgctggtaaagaagttggcgggcagcttgtaccccagacggttgatgacttcttgcacttcgtcaaacggcagttcatagtaggccatcaatgtatcagcctgcttggcaacttggtaggcgtccggtgacttgccttcgcccttgagcagtcgatcaattctggaaatatcaccatacttcttccggtatgaatcgaaattcagtttggataggttgaagtaccctgagaactggccgataataccttcttcgttgatgtccaatcgcagtttatgggcaatatcgttcatcttggcgagaagtgcgtcgtcaaagccggctttttcactggcttgctttaaaacggcgctgtcttcctgcgataccagggtattgaccttgtcaaacagccaggaaaccatgatattcgtataggcattattggttaagccatgatcgttggagttagggtactcttcgtgaaattcgtcaggccccatgacatgatggatgtcataacggtcggctgattgatcgtagtcggtcatgctgacccagaacttggaaatcgacagcagcatttccaatccgtattgatccatgaattctttatcgcccgtgatgtggacataattgataatgtcataggcaactgaaatggaaacgtgccgttgtaggcggctgttatcgggatcccatttgccgctaaccggattcaagtgaacaaattgtgattgctcatcgccatacatccctgactgccaaggatacattgcaccttgtttgtcctctgaggcagcatactttcgcgcctcagctaaccggttgtaacggtaaagtaggcactgtttggcaatcgcagggtaatgaattgcatagaatggcaagtcaaacgtgacatcccaaaaaatgtgtccacggtaagcttcaccatgcagcccacgagcaccaacggatgcatccaatttaccggaggacaaagcagcactggtaactaacatgtggaaaatattgaccctggtcaacttttggctggtaagatcattatcgataataatgtcggagtgttgccaaacattgctccagaatttttcactatcgcttagcgtatcttcaaatgaggagtcatcaagttctttttgtgcatcggcttccaaatgatcattttcgtcttgggaagtaaagacggtgacattctttttgaattcgtattccttgccgggctcaacgttaatgctcaaagcctgttggactttaccttcctcagtcgtggtatcgattaattttttggtatcgaaatctggactgctgagtttggagttaatcacaaattgaacgtgtgaggtcttggtttgaccggtcatcgagacttgattgtcatgagctgacatgccgatgacatcaatgtggtgctgatcaaagtcttgataacgttccacgttgccgttaataacgttgccatcaatgccggcatagatttgtaaactgccggagaaattgatgggctttaattcatatttgattgcgtaacggtgccactgatccatgttggcgactttcgtagcccggacttggatgatatggccggttgaaagctgaacgtgcagcgtggttgtcaaagtaccggtcttcagatccaagcttcggtaaatatcttgaatatcggctttcttaatggtaaatggcagttgatggtcaacaccgaaactaatgtattgggcattcggtaagtttaccaaatcctcgttcacaacgtcgcggtcattaatcttagtcgtcaattggttgtaaacaccggcaacgtacatacccgggtaattatccttatcagcgtgggactcaacgtaggccccccggagaccaaagtaaccgttcccgattgtcagcatggcttcttggccgtagttccgtttaccggcatattcaccatagtaatccagatgccacttaaggtattcttccttatcggcaacggcttttttcagcccaacttctttgatcttttgcagattaacaaccggaatattcatcatgttggcaattgccaatccgatatcaatcttttggtgattaatgccaataatcgtatctgaaaactcatagtttaacgaattttcgataatggcggcgtcgatcggcaggccggtcagcgctgctttgatattttcaagattatcgccaattgaaaatttggggttatatgtgatcataaactttcgaaacggcggtttgttggaatcttctgaataatttaattccatgaccccatcgcgggccctaatagcaaacgttctcataacaaaacctcttctcaatttttgggaaataaattaaaccttcacacttttaattctagcccagacatcatgcaatcgcaatcaattaccgttttggaatggtctgcggtgcgtcattgacggctcattgtttattttttaacagatcccggatctcggaaagtagtacttctttgttatcgattgcaggctttgtcggctgacgcttgaggaccttgttaatgagtttgattaagataaaaacgacaaaggcaacaattagaaaattgatcagtgaattgataaaggccccgtaacgaaaagttgcatcaccgactttgaaaatcaggtttgacaagtcaatttttcctaagaagatcccaattaacgggttgatcaaattatttgtgagggaggtgacaattccagtaaaggcgccaccaataatcaccccgacagccaggtcgatgacgtttcccctggcaataaaagccttaaattctttgagcatgatttttctcctttcaactagcttattttcatgatgtatttattatatcgactttaaataccccaagacaaactctaactttcccaattcaaacgtgaactccattggcaaagtatgatagtatgaaataagaaattttacaggagaattcatttgaaaaagtctaaattattcttaatcgtcggcgccgtcgtattagtgttagcagtggcgtttttcatcacaaagtcttggcatttatcagtcctgtcgttcgcactgatttggctgattgcaattattgccattcgcctgattttgacgccgctggtggtgatgattgttcgccaacgcgatgaaagaaaagcccaacgagaagcagacgacaatagtcgtgacaaataagattgtttgaaggggattgtatgaacaaggattggctccacaggattttcataaccgcaggattgatcttgcttgccattggtggctctgcggcaaccagcgggcaggcagctgccaagacgaccaacgttgctgactccaaacagcagttggttgatattgtgctgcggccaaaaagtcagtcggcacttcaccaatttgtctacaacacagtgacgccgagttcaccgacttatcgcaaatttgtgtccccaagtacttttgccaaacgattcagtcagagcccaaagcagattaaagctttgcagacctatctcagacaccatcatttaaaggcgcagacttacaaaggtaatttgattatggtggtcaagggatcaaccaaaaacgttgagaaggcgtttaaggttaacctggtgaacgtcaataacggtgaggtcaaatatcaaaaggccagccgaaatcctcaactacccaagaaactttccaaggttgtctataccgtctttgggttatcaaattactcaccgttttcttcatataaaaccaaatttcagccctcttcactgcataccagagctgccagcgggacgacaaccaccaagaagtattcaccgacgcggtttgtccgtcgctacaatctacagtccctatacgataatgggtcgactggccgcagtaaaaccattggtatcatttcatttgccaacttccatcctaatgatgtgtaccgctactgggatgatgagggcatcaatgtgaaatccaatcggctaagcgtttatcggactaacggcttcaagggtacctgggatggctatgatgaaacgaccatcgacgttgaacaggccggcgcaatcgcaccggacagcaacattcggacctacattgcccgcccaaatattttggggatggtgaattcaattgctgccgcagttggtcaaaacgtggccgacagtttgtcacttagttggggccaaagtgaagcccaagtggcttatgaaatgaaacaggggattaccccgaaaaaatataatcaaatcatgaacttattatttgagcaggcagctgcccaaggaatgagtgtcttcaccgcgactggtgataatggcgcctatgatgggattaccaccggtttaacgtcaggattgtccgttgacacgccgtctaattctccatatgtgaccgcagtcggcggcacgacactgccgaaaacctatactgtcaataagaaaaaagtcaccattcaccaggaacgcgcctggggggctgactttttataccccaactataaacaccaacgatttttcggaactttggacatgcttcaaagcttctttgccggaggtggcggcggttttagtaaatataatgccagacccgcctatcaaaaagggatcagtggtgtcgggacgtatgatgcgactaatctttggaaatttaaatatggccggccggaattgttgaaaaagccgattaatcttagcggtaaatccagcggcagaaaccttcccgacatttcagcgaatgccgaccccaatacgggttacagcatgttcattaccccgaagaataatcgaaattccaaggggcaatggctgattaccggtgggaccagtgtcgtcgcccctcaaatggccgcagccagtgttttgatgtctgatttcactaccaatggccgcttgggcttttggaatccacagatctatcgatttgccaaacgatcaacttcgccgttcaaaccgttggacagtcggacaaataacaccaatttgtactataccggacagccggggaagatttataaccaggcgaccggacttggaaccattgattttacagctttgaacaaagcttttaatagttaaggagacgctgcatggaagagcaaagaaagttaacttttggtgactactttgaacgattaatgatcttttttgggctgattattttggtcggctcagttcagctgccactgatgttcattgcccaaggcaagctgtcagcagttgccaattacgctgttggagctttgtatttgttgggctttctaatcgccatttggctggcacagtatgcctaccggaagtatggccgctacgaagtcaaaaaaatgacctggccaaatgtcaaaacaattgtcattgcttggattgcttttttggtgattgagttcttattgggaaaccttaataaactggtctatcacgtcactcaaacggacaacaatcaggaaattcaatcattgttgtccagcaatcatcttaccctgattttgatgggatttacggcaatcttctgttcgccgattcttgaggaaaccatttttcggggatatttgatgactgcgttctttcggtcgactgaaaaatgggcaccaattattgtcagtgggatggcttttgccctgccgcatatggatcctgatctttcccattttaatatcatcagttttttgacgtatgcgatcctaggttgtattttggcctatttgtatgtaacaactaaaaatttgaaggtatcaattggcctccattttttgaataatttaatcgcagtcggcggaatgattgcgatgatttttgctgtgtaattaattgtgagaggtgttaatcatgggattatcggttaaattgatgaatgatctttcggatggcctcaagggtcggcgaaatctgattacagatgttggcggcgtcaaggtcgggcaggtgactattgatgatggtgatgttcatagcggtgtgaccgcaattctgccccataccggcaaccttttccggcacaaggtaccagctgcctcttgtgtgcttaacggcttcggtaaaagcgtcggcctcgtccaaattgatgaattgggaaccattgaaaccccgattgtgatgacgaatacctttggcgtgggcacggccctaaatgccctcaccaaacaaatgctggctgacaatcctgaaattggggataccaccagtacagttaatctgattgttgctgagtgtaacgatggcgacgtgtccaatatccgcaaaatggcgattactgaacagaatgtgtccgatgctttggctgctgttaacgatgactttgaagaaggtgcagtcggtagtggccgcgggatgatgtgctatgatctcaagggcggcattggctcttcctcgcggattgtgaccgttgataagaagcaccaatacactgttggcgcactcgtcatgaccaactatggttatttaaccgactttattgtcaatgggatgcctattggagcccccttggccaaaatgttggccaaggataagcaaaaagaagaaaaggggtccattatcacgatcctggcaaccgatgcgccattgaatgcccgccaactcaagcgaatggctaagcgggcaacggttgggattaatcgttccggtggctacattggcaacggcagcggagaaatcgttttagcattttcaactgccaatctggtggaccattttgaaaccagcgagtttgatactgttacccggtttaacgataaccaaattgatttattcttcagagctacggcagcggtcgtcgatgaggcgattttaagttcaatggtgcacgctgaatcagtcgttgatcgaaagggacggctccggttaaatttagttgatgcatgcaagaagttgatttctcagcagccggattataccgatatggttgagcaggtcttttcacagcttggggtggtcaaatgagtgcgaagattttattaggtgctgaaaacattcgccaacttgcctggggtgccgtcaacggctgtgaagcagccagcttgctggaggggctccattatcagggccgagctttagacctgaattatggccaatttctccttcagatgccaatttcaccagatagcaatccttaccacggctttggtggttcacctttcaccaatcggcccggcaagtttgaggcaatctttacccgacccttgatgtggtggggaaatcgttatggtaatctgcaagaactgagtggggcagatccccagtggttgtatgactttgtggcaaaaggggagccggtgttaacctttgtgaccgtccgttttgaacaacctgagtgggattcgtatccatttggtcaggttccggctaataatcacgcggttttgttggacgggatcgatggcgaccaggtccacgtgagtgatccgattgacggtcaatactggctgccaaaaaccaaatttgagccgatttatctgtctcgtaagatggcaatcgcaattactaagtaaaattcacagcaaaatcgcatattctaacaggctttctgaactcaatattagaaaaggcctgtttttttgacacttttatgctaaattagaaccaagatgagtttgttacgcgtcttacatattagaggaggattatatcatgcatttatctcgaggagtggctgcactcgcaggtgtagcaagcattgcattaattctggcaggttgtggtcaaaagtctggtcaagccaacaagacgattaagacttcaaccgattctgaactgacgactgttgatccatcgaagaccacggctgttggaactttcaacgttttaaacaacgtcgatgaagggttggttcgtctaggcaagaatagtaaagttgaaccgggaatcgccaaatcatggacggtttcaaaggatggtaagacttacacttacaacttgcgtaaaggtgccaaatggagtaatggcgatccggtgactgccaaagacttcgtttattcatggcagcgaaccttaaatcctaagacggcttcacagtatggttacctgttctcaggaattaagaacgctgacaagattcaaaacaaaaaagccaaagtttcttcattgggaattaaagcagatggtaattataaactgactgtgaccttggaacagcgaatcccatactttaatttgctgatgggctttcctgtcttcttcccacaagatgccaaggcggttaataaatatggcaacgattacggcacttctgccaagacccaagtttataacggaccgtttacgctgactggatggactggaaccaataacaagtggactttgaagaagaacaccgattattgggacaagaaagctgttaagcttgatgacatcaagttcagtgtccaaccggatccttcaacgtcattgaacctttacaatcaaggcaaacttgatatgtcgcaactttcagctacccaggccaaacaaatgggtaacaagaaagatatgatttcacgaaagcagtcttccaactactacattgctgttaaccaaaagaacaaggtcttcaaaaacctgaaaattcgccaggcaatgtcaatgatcattaatcgaaagacattagccaacaaagtcatgggtggcggcgcaatcgataacaatagctttgtttcagagggattggccgtttcaccgaagaacggaactgactttacgaaagacacaaccgctcccgcatcaatgacttataacccaaccaaggctaaacagctctttaaggaaggccttcaagaagttggtcgttcgtcattacactttactttgttgaactctgatggcagtgaccaaaagcaattgagtgagtatctgcaaagtgccttgcaaaagttacctggcttaacggtcactttgaacaacattcctggtcgttcaattttatctcgacaagctgatggtcagtttactgtgaccgttgccaactggtttgccgacttctccgatccaatcacattcttgaacattttgacttccaataacccaagcaacatttccggttggaagaattcagagtatgattcgttaatcaaagccagcaacgctgacgatggcagcaatgccaacgctcgttgggatgacatggttaaggctcagaatttggccttgaaagatcaagcaatcattccactttaccaatcaggtgaaaaatggatggttaattcaaaagttaagggaattgtttacaacactgctggtgccaactacaatttcaaagaggcttacgttaaataattaatgaggagtgacacttattggaacccgtgattaaaaagattgatgtccaggaagctgctgtgccactcaaacggccgttcaaaactgcattaagaactgtcaccactgcccagacgctgatcgttaaaatgactaccagtgatggtaaagtcggttatggcgaggcagcaccaacgccggtgattaccggagatacccttccaagcattgaaagtgccattaacgatgtgattggcccgaaattgattggcaaaccattgtttgactcagcggatattaaggcgactatcgatcagtcaatggtccataattcgagtccgaaggctgctttgaatattgccgttaacgatttgctggctcaatcgtatggggtgccactatatcaactgttgggtgggcactcggatcacatcacgaccgattatactgtcagtgttgggacgattgaggatatgatcacccaagcacaagacttgattaccaaagggtttaccactttgaaaatcaaggtgggggatgattctgaagaagccgacctcgataaaattgtggccatcagaaaagcagttgggccagccattcaaattcgtttggatgccaaccagggctggcatccaaaacaggctgtcgccgttattaatcggatgcaggatttgaatctgaacattcaactggttgaacagccggttaaagccactgactttgatggtctggcttacgtgaccgccaacaccacgacgatgattatggctgatgagagcatcttttcaattgaagatgccgctcgcatcattagtatgcgtggttgtgatattatcaaccttaagttgatgaaggcgggcgggattgataatgcggttaaaatcaatacccttgccgaggctgccggaattccctgcatggtgggtagtatgattgaatcgtcggtttccgttactgctgcggctcacttggccgccgccaaacgaaatattcagtatgtagatttggacgcatcgatgatgttctccagcaacccaattgtcggtgggatcatcaatcaaaaaaacgaaatctcttttccagatttaccgggattaggatttaagtaacctaagaggctcggacataaggattcctcatgttccggcctttttgagtagggtgaacaagccggcaatgctttttatgctatctagcaggtagttggtggctaatgaggtataatatatgtatactaaaatttaacgaatggaggtgcccagatggaaacaagacgagtcaaagttccagtggcaactatttggaagtctaaagaatcaccaagaaaagttgatcaaccagccttagacggcgatggtaaaaaatgggttgaacaaatgagtgatgagcaatcagttgcgctttccgatgatgacttattagaaacgcaggctttgtttaacgatgaagtcattattgatcatttcgacggtgactgggccaaagtctatattcccagtcaacgagatgattctgattcaaggggctatcctggttgggtgccaagtaaattattaagcgatcagcagattagttatccaccggttacctcaattgtgagaattgctgttcggacagccaatttgtatgatgaaaacaaaaagccggtcctcgaaatcagcttgggaactgtgctgccacaaacaggcaccagtggtgactacattgccgttgtgaccccgcttggaaagggcttcattgacaaatcagcagcagtactgccattcgttgggagcaatgctggtgaaacgatggttgagatgggacgccaatttttaggcgagcgttatctttggggtggaaccagttcctatggttttgactgctctggatttgcgtacacgcttcatcgggtacttggatttgatattccccgggacgctgacgatcaacaagaaaacggcttacctttagcaccggaagaaatcctaccgggtgacttggtatttttcgcgtatgatcacggcaagggctacgtgcatcacgttggcatgtacattggtaatggaaagatgattgaatcaagaacgccaggcgccaaagtcgatattgccgaactgactgaaccaaaatttgcggccgagtttgccggctttaggagatattggcgatgagtgagctttctgaaacaattgaacgggtgatggctgacagttcgtttaagtatggcttgttaattcaaagcaacggtcagaccttggtggaccatgatagccacgaggctttcccatcggcttctttgatcaaattggccatcttaaacgatgttttggacagcaacgttgatctggatcaatccgttgatgtttcgacggatgagttggtaggcggtgccggaatcttacaattgatgtctgttcggtcatggaagcttcgggacttgttggcgttgatgattagtgtgtccgataattcggctactaatgtggtgatctccttgatgggaatgaaccatattcagcattatcttcaaacccatgatttccacgagaccaggctggaacgttatctgatggacggtcgggcacttgccagtggcaaaaataactataccagtgccactgaaagtttgcggctgcttcagcaagcacttcataatggttccgaagtccagagctggttcgtcaatcagcagttccgatacaaactaccgggtaattttgatgaatcaggcgagaatgttgctgtatacaataagactggtgagggcaatttgattgaccatgatgtcgctcaaattgtatataacaaccattctgttgacattgccatgttgactgctggatccttgaaccgaatggaaacgatccaaaaatttaatcaagttggccagtcagtggttgattggctggcatgaataaaaaagcaagcgtcggccaataagcaattaggctccacagtataaagggattacctgaattccagttggatatttggataatcccccttatacggtcggaagctgcttattggcccacaattataccagataacattcaaacacaaatcgaggctggaacaaaatctttcattttgtcccagcctcgattttaaattggatttatgattagattatactctgcaccaaaatcttaacattttggtcagagcgtttagatctgtgtttgattgtacaaatcaagcttttgttcaatggtcgccatcgtctgagaacaagcttctttttcagctggggttaatcccaaaacatcaaagcagctgttcacacgactgaagacattgtcctgttgctctttggctttgtcggttaactggatgacaacggttcgctcgtctgcttcgcaacgggagcgggtgatccagccatgattttccagccgcttgagtaatggggttaacgtgccgctgtccaggtggagatattcgcccaattgcttaactgagagtggtgcatattgccacagagtcagcatcgcaatatactgtgggtaagttaaatcaaaaggcttcagtgcctgctgataaaaatgattaaattttttgttcgctgagtagacttggaaacacaattggccgtccaagcgaattggttgggtttgaggcataatttcaactcctattatttttgcacatactgccgtgaaacacggacagcactagtcgaatcaatttaaatactttatgttattattgtaatgtatttatatttaaaagcaagacttaacacagggagtcaaattaattgcggacaattaatttgacataaaaggggattgttacatatgaaaattggtaaacttagatttagtacctggttattttggattacggtggtctcaatggctgcttatcttggttactatggttattggttaatgaaaggacaaccaaaatttcacgggcagacgttgctcttggtggaggtctttattgggatcctcattgccagcttgccatttttaatcgagaagttgggccggttttattttccacagattgaattggttttcttttatattttcttatacatgtccattttcctaggatccggattgcaattttacagtgtaccgttttgggataagtatgaacacgttttttccgcaatgatgttggctggactgggattttcaatttttcaaggattgatgagtgccagagataatgcaaccaacaagccattcttgatgagtctgtttgcctttacgtttggaacgacttgtggtgttttctgggaaatgtatgagtttaccgctgatggactgggtggtttgaacctgcaacggtatgaagaagctggcaagttgttgctcggccgagcagccttgatggacacgatgactgacctgatcgccgatttggcaggggctttcctcatggctttgattggttacctgatgatgaaacatgatccaagttccagccgatatctggttttcaaaacaaaacgacaaaacttcttttcaagttactacttttagtgtaaaataaaacatgttgttgccctcgtggcggaactggcagacgcgcagcgttcaggtcgctgtttgagcaatcaagtacaggttcgaatcctgccgagggcatcatataaagttaagaggttgagatcactattgcacgatagcgatctcaacctcttttttgatccgtttttttaaaaaattagtcggccgattatccataagcaggattggccgactaattttaagttatcaacatgttaaaccttgagtgtttcgttggcgaatctcgagttaaaacaacgattgtcttaatgggcccctctgacgagaacttggtatacaatttggcgaagttgacggttcctagtccagtggcttgattgtaaagtttaccaggttggccggtgtaatacaggttattattgttatcagcatcgtcaagcacagtaaagggtgaatcaggttgcaccgcaaattgatagatttgtgggttccaaaagccgattggcgaatttgtcccgctgttcatcaccgcgttggcaccagccatttgtggcgatacaaagctggtgccgccgttcactgtccattgtttgactggaacgctgatgaccgttttgccatccttggcataggcgaggtcttgtccggagacgtaggtcgcgtaaccggtgtaactgtcggcattggctgaaacatcgggaacgtttcgaccagatcccttgccaatgataatttgtggatctttattcactaagaacccaccgctcttatatttcagcagatcgattgcctggaaggtgttaacgccggaaaatccttgctggtagcggggcgtcggattcaaaattgaaaatccgccgccgctgccgccataattagccggtttggtttgtggattgctgtatgtgtcgccccaagcccgttccttatcaatggtgattaagcggccatcggtaattttagtatagggtaatgtggtgccgccggtaatgacttgatatggcgaagttgagaaaacgtggttgaattgtttaagtgccaattcacgcggaccatagtcgccacttgcccgaaagacggagatgccctgaacagctgcttgttccaacagcagattaaaggcgtcgttgtactcacccaaagaggcactggcaccttgttcccattgactggcaagctccgtgttgggtgaaaagctggttgaaatttgtttatcacgatcatccgaaacggcctgcataaaggcggtgtaataagatgatgtcgttgaagtgacgttttttaatgataggccgatataagcatcaattttggcatcgggtgcgacggctccagactggttaacatccagcgttgattcaatttgagccgggtttaatcccatcgacaggatcaagtggccggtcttggcaccgtcaattgaataaattttattgatccggctggggtcggcgttgacaccggtttgctgccaatatttgagcacgtcttttgcattaaagtcgtccatggcaataatgccaattcgctgtccttgaccggttaaaccttgtttatataaatcactaacctgataatgatcagcgaattttaaggcaccatattttttggcaaaactggttttactcaaatcagtatttggcggggtcgggttttgtgggagtgagggtgttactgcaagacttgtcttcttacttttgggtttcgttgcgtacacaccgatgacactgactgtttgggccgaaagctttgccggtaatttaactttggttcgataatcgtttttgctgaccttcacttgtttggcgttaaatgcccgaatcaaattcttccgagtgccaacgactttgatggccaagtttcccggatagacggatgccttgagatgatatttccctaagtagcttttaaaatcgttgatgtctgtcgtcgggcggccgaattgactggcaaattggcccggcgttaagtattgatgataatttggtgaacttggatcgacggtggcatagacataatctgtcagttgggatgaactttgcggttttaaagcaatatttgccacaactgttttcgatggtgaaacttttggcatcgtgtacgtgttggattttgcactggtcgacacgctgccagcaatcacaaaaatcccgctcaatatgccaataactaatcttttgcccctcatgaaaaccacttcctccataatttgataacatttaaattataacattaattagtccattgactgaattggaaagccgtcataccggaaaattgtacctgcttgtgattaaaaatatatcttcagacttattaattgcttttcggatataaacgtagcattatagtggtgtagacagtaatgtgtccgcttacaagaaagaagggtgatatttatgtatgacaacattttggtaccacttgatggaagtaaaaattctcaacaggcactggaggaagcttgcaagttggccaaacaatttgactcaaagctccagttggtaacggttattaacaacaccaacttctactatggtgcaggggcagccggcatgccgccaagcatgtatgacgatcagcacaagatcgctgagaacattattgacgaagccaagaagtatgctgattcacaaggtgttaaatatgaaacagccattgatattggcaacccaaagaacattatcgcgcacgtttacccggatgagcacgacgtagatttgattgtgattggtaagtcaggtgtcgatgcgattaaccgactgttaattggatccaccaccgcctttgttgttcgaaacgcgacaacaaaagttttggttgttaatactaaaggctaaagataaatttatctataaactaaaagggattcaaaattgctcccaacaattttgaatcccttttcctgatgaaatttatatatcactaaatccgatcagaaatcttataaggtttttgaatcgcatttctttcattgtcatgactaatgatgtcgtcggccataaaaatatcgaagttcttgttgtcgacaccatgaacaaccaaaacctttttgttgtgttctttttccttgtaaatttgagcggttttgacagcttcattgtgatcatggaagttgccgatagaatctcccgggttgaaaaatacgatctcgtccatttgtatctctcccttcaaaaacaatttgatactctatctaaagtataacttaaaagaatggtaaaatgaaattcgaaagtgttttaatttcctttagtcaagccgttctttaagaaaggtttatactactggtagcaatctatgtaatctgataaaatataaaacgttattaatttcagactaaccaagaagatttgataaaggggtataaaatatgtgcggatttgttggttacgttaaccaaaaagatgttccagaaggtaccattaatagcatggctgatcggatcaagcatcgtggccccgacgacgaagcttatttctccgacgacaatgtttcaatgggatttcgtcgactttcaatcattgatttagcacatggccgtcagccgatgttcaacgctgaccaaactaaagtactgacttttaatggtgaaatttacaattataaagaaattcgtgaagaacttcgcgatttgggatatgttttcaagactgatgttgattcagaagtcttggtatacggctacgaagaatggggcccagccttgttagacaagcttcgcggcatgtttgcatttgtgatttatgataaaaagaacaatgaggtcttcggtgcccgggatcacttcggaattaagccactgtactattacgatgacggtgatacgttcctttggggatctgaaatcaaagcatttctggagcatcccaatttcaataaggaactgaatttgcgcctgctgccaattcacttgagctttgagtttattccgtccagagaaaccatgttcaagcacgtctacaaacttttgccaggtcaatatttccttcataagaacggcaaaaccgaaacccatcgttactacaaattcaactacgatcatattgacaatagccaaaccattgaaggagacgccgacaaaattggtaagttgattgatgattctgttaaggcccacatgattgccgatgtcgaagttggtagtttcctgtctagtggaattgattcaagctacgtattaaacgaagctgccaaattaaagccgatccagtccttctcgattggttttcatcactccaaatatagtgagttggcttggtcgactgagtttgccaagaccattaaccaaaagaatacgccaatctacatgaatggcgatgattacttcaatttcctgccaactatgatgtactacatggatgagccgctttccaatccagcggccattcagctgtattatttatcaaaggacacttccaagcacgtcaaggttgctttgtccggtgaaggggccgacgaattctttggtggctacaacacctatctggaagctatcccattcgatcgttatcagaagtatgtaccaaagccggttcgtaaggggctggctgcagttgccaaacggctgcctcgtttccacggtaaacgtttcttggttcgtggtgcccagccgttgagtgaacggtactatcgtgtgaactacgtctttaattacgacgaccgcaatcgcgtgttaaaagatccttcaattaacacagattcaggcgcctacaccaagcacatctttgatgatgtgaagggcaaagacgaaatgacccaaatggagtactttgatattaacacttggctgccgttcgacattcttcataaggctgatcgaatgagtatgtgtaactcacttgaagttcgggtaccattcgttgataaggaagttgccaaatttgccgaaaccatgccggtcaagacacgaattacaccggatgagaccaaaattgcgttgagaacctcagcagaacgggaaatgcctaagaagactgcccttaaagagaagctcggattcccatctccaattgccagctggattaacgatcccaagtatcacgaacgaattgtgaatgctttccattctgatacagggaaaaagttcttcaataccaacgaattggatcgtctgttgaaggagcatgctgaaggtaagtccaacatgcagaaaattttcaccatctatacctttatcctctggtatcaagtttacttcccagaagatacaactgagaacacggtcagcttggttcatcgtacccagatttagaaatatgcaaagaatggaaggtgcacatattggcacaaattactgttgctgaggttttagttttactcaaagaacataatttattgcttgaaagtcaattgagcagctcaagtcatccctttgaccagattgcatataactctaaattggtcactgacaactgtttgttcttctgtaaggggaacttcaaatctgcgtatctggatgatgccagacagaatggcgccaccgcgtacatgtccgaaaagacataccaaaatgccggcattccaggcattattgttaagaatatccaaaaagcaatgtcgctcgtaagtgcggcattttttgggtttccacaagatcaattgccaacgattgcctacactgggacaaaggggaaaacgacatctgcttactttaccaaagcaattctggatcaaacttatcagcgaaaggttgctttatcctcaaccatcaatacggttgtcggattaaagcccgaagatgttgttaaatcaaatttaacgactcctgaatcgttggatttgtttaccatgatgcgaaaagccgctgataatggaatgagtcatttagtgatggaagtttcatcgcaagcctacaagaagaatcgggtttatggtctgcattacgatgttggggtttttctcaacatttcacctgaccatattggtcgcaacgagcacccaacttttgccgactatttgcactgcaaagaacagttgttggttaattccgacgtttgtgtgcttaacgctgacgggacacatttaaccgacatcttttacacggctaaagcaaccacccaacctgaaaatatctttatttatggacgggctgggcagaatcaggaaactgaatttccagtagatgtcgagtatcggtcgttaaaggattcgctgacggaaaatcaaatccaagtgactgcccgaaccgccaaggcgaagcaattgaacattgacggtgtataccggattggaattcctggagattataacgaaggcaatgcagttgccgctgcgattaccagcgccttgatgggggccaaaccgactgagatcgcttatggtctggccaatacaacggttcccgggcgaatggaaatatatcagacccatgatcatggaacaatttacgttgactatgcccacaactatggcagtttacattccgttctcgatttcttgaaaaaacaggctcctaacggtaaagtgacggttattacaggcagcacgggtgataagggaattgatcgtcgcgagggccttggcaaagcaatcaacgaggctgccgatcaggcttatttaacgactgatgacccggcaaccgaggatccgcaacaaatcgccaaagaaattgccgctcatatcgatacctcaaaagtggctacaacctacatccccgaccgcaagcaggccatcaccaaggccgtttccgaaagccagaagggtgacttggtagtggttgccggtaaaggtcatgatcagtatcaaaagattaatggcaaaaacgttccgtatgaaggtgatgcggcaattgttaaaaatctcgtgaaaggactctagtaatgaaaaataagcagcttgattttacacccgttctgttaggcagtgactttaacgcctatggaatggccagaagtttatacgaaatttatggcaagccggtcaaagcatttgcccaaacccaattggcaccgacgcgcttcaccaaaattgttgatttggagctgatcccaggctttagtgaggatccagtctggattgatacgatgaagcagcttaagaaacgttatgccaatcatcaagaaccggtgattttgattggttgtggggatggctatgcggaactcattgccaaacacaaggccgaactagaagatgttttcatttgcccatacattgactatgatttacttaagaagctcaacgacaaggaaaacttctacaagatgtgtgatcaatacgacttaccatacccgaaaacgaggatcatttccaaagccatgtatgcttcgggcgagccgattgaacagccatttggctatccggttgcgctgaagccggccaacagtgttgagtggcttgatattcactttgaaggacgcaaaaaggcgtttatcattaagagtgaagcagaatttcgggagattgttgccaagagttatgataacggctatacatccgactttattctccaagacttcatccccggtgacgacagtaatatgcgcactttaaacgtctatgtcgataagaatcatcaagttaaattgatgtgtctgggtcatccactactggaagatccagcgccggcagcgattggcaattatgtcgcaatcattcctgaatttaatcaggaaatctacaacaaagttcaggcgttccttgaaaaaattaatttccacggctatgccaattttgatttgaaatttgaccaccgagacaattcttacaaactgtttgaaatcaatttgcggaccggccggagcagtttctttgtaaccttgaacggccatcatttagctgattgggtgattcaagattacgtcttcgattcactgaaggaccagtcgaccttgtatgccaacaaggacccacgccaatatttcttgtggcttggtgtcacgccaaagatctttgaaaagtatgccaaagacaatgctgccaaaaagcaagccatggaaatgatcaacgaaggccgatatggcgacactttctggtacgccaaggataaaaatatcaaacgttttgcattatataagtggatgatgcacaattatgccaagagctttaagacatactttgtcgaaaaataagggactgatttagttgaaaaatttctttacaattattggtggtatgggcaccgaagcaactgaaaccttcattcatattttaaatgatcggactcaggcgacgaaggatcaggactatctgaactatattttggtcaatcattcgaccgttcccgatcggacagactacattttggatcactcaaagcccaacccattgatcccgctggcagaagacgtcaagcagcagagtgccctacatcccgatttttttgcgattccttgcaatactgctcattacttctatgatgagctccagaaactcacggatgtgccgatcttgcatatgccaaaggaaaccgttgcagccattaaggattatgcgccaaatgccaaacgggtcggtttaatcgcgacagaaggtaccttacatgatcaaatttatgatcatgaaattattaatgccggctatgaattagttaagccaaccgacaagattgccgatcagacgatgaccttaatctatgatgatatcaaggccaaaaacgaggtcgatgagggattgtatcacctgattctttctcaaatggttgaatcgttaaaatgtgacatcgttattttaggctgtactgaactgtcagttgcccagcagcgggcgggtaatcacgattatccagtgatcgacgcccagacggttttggctgataagtgtattgaattggccgaagcaaatcgggcaaaataaatagccaactaacttaatagttgaccaaagtttgtaagcatacggcgattggcgtggcgagcatcaataaccacagcagtttggggctgtagttgacgtcttgctttcggccataagcggtttcggttaatgcaatcactgccagcgtcaccactgtgccaatgataaccagcagtggatgacggtgaaatgaacgaagtgaaatgacgacttggctaatcatgatgagccagtagaagacgcgggcgatcatcatcgaatcgatgacgtgctttttcatggatcgggttaacccccagataaaattgacgaatagaattgcccaacagctgtagttcaatatgatccacattcaaatcacctcttaagttaagtatctgtattttgggacaaaaaagcaatcttttccaaaattctttagagatttcaaatctttatgacaaagataatttaaaatgatataattgtttttgttatgcgggtatagtttagtggtaaaacacaagcttcccaagcttgcgtcgcgggtccgattcccgttacccgcttagtgttggttgtctcagcactggggtgtggtgataaatgttgacatataccgggtcaacaagttattatacacattgaacgttataaatattcaacaataaaagaacagtagctggtcactgaattgtcagcgatttcgggatggtgggagccgaaaaattgagtcagcgaagcgcgctttttagaatatgaatttaatactttgagcggatatttttatcaaatagagtggtaccgcgggtttactcgtctcttacaattattcttgtaagagtttttttgtatatttatagatggagggaacattaatggactacaaagcacaggttacgaactcaattttaagtgttttaaatgacgaattgtcatcagccgaggtttatgagaagctcgaaaagcctaagaccttagcaatgggtgatttggcatttccagccttctcattggctaaagttttccataaagcaccaaatgccattgcgcaagacttagttgagaaaatcgatcaatcctcttatgagaaggttgaagcaaagggcgcctatctgaacttcttcttggataaaggaaacttcagtaatgaaattttgaatgaggttttggaagaaggctcagcctatggtcaaaacgacagtggtaagggtggcaatgtcccaatcgacatgtcatcacctaacattgccaagccaatttcaatgggacacctgcgttcaactgtgatcgggaactcaattgccaagttattggttaaaaacggctatcatccaatcaaagataaccatttaggtgactggggaacccaatttggtaagctgatcgttgcctacaagaagtggggtaacgaagaagacgtcaagaaagatcccatcaacaacctggtgaagtattacgttaagttccataaggaagataaagaacatcctgaattggatgatgaagcccgtgaaactttcaagaagctggaagacggcaatgaagaagaagtctttctctggaagtggttccgtaaagtttccctggaatcatttaacaagatctacgaaaaattaggcgtgacttttgatacctacaacggtgaagccttctataacgataagatggacgaaggaattcaaattctcaaagacaagggcctgctcgtagaatcccaaggtgctcaagtcgttaagctcgataaatataatttgaatccagcccttatcttgaagagtgatggcgccacattgtatattacccgtgatatcgccactgccatttaccgtgatcgaacttacaaaccagccatgaacttatacgttgtgggtgccgaacagacttattacttccagcagttgaaggccgttttacttgaaatgggcttaccatctgccgaaaacctgcatcatattccatttggtctgattacggttaatggtaagaaactgtcaactcgttccggccggatcatcttgttggatgaagtgctggatgatgcaattgacttagccaagaagcaaatcgaagcgaagaaccctgatttgcctaacaaggatgaagttgccaaagaagtcggtgttggcgcaattatcttcggtgatttgaagaatgagcgaactaacaacattgactttgtgcttgaagaccaacttcgatttgaaggcgaaaccggtccttacgttcaatattcacacgcccgtgccgaaagtattttgagaaaagccggggacattgatcttcatggtgccaacaagcagcttgatgatccagcagcttgggaaacggtcactgcattgaaggacttcccagacgttgttaagagtgcctgcaaggactttgagccatcagaaattgccaagtatgccttgagacttgctaaatcctttaacaagtattatgcgcactcaaagattttggtggaagatgatcaattggcagctcgtttgtcactggtcaaggcggtttcaattgttctcaaagaatcattgaacttattgggcgtcaaagcaccggacgcaatgtaatctaattgtatttgaaaccaaggctctctaccaaccaggtagagggtctttttgtttcgaaaaatttcagattgatcaatagcttgtggcgggcgctcttttttaaatcctcgttaaatttttccaccctgaatttcgccacttttcagatatgatacaatattgaggtattcacaaaaggagtatcgcatgaataagaattctaccaactcatttagaaaatcggtcgggacctttttgaaacgtttcaaccgattttgtcgaagattccacttggttaagtggcttgtggtcatttttctgagtatttcacttgtgaccagcacctacttggtgttccttgccaaaaccgcccacgtccagaacttggaatcctcgctctcaaagacaactgaaatttttgacgttaataataaaaaagccggcgaattatacgctcaaaaggggacttatgttcatttaaatcaagtctcggcaaacattccaaaggccgtgctatccaccgaagaccgtaacttttatcatgaatacggtttctcgttcaagggaatcgcccgggccatgtttttactggttaagaacaagctgcttcatcgcaactatattagtggtggtggaagtactttaacccaacaactggtcaagaatgcttacctgtctcaagagcagacgatgactcgaaaactgaaagaattattcctctcaattcaagtcgaaaatgtatactcgaagaacgaaatcctgaccatgtacctgaacaatgcctactttggtaacggcgtttggggggttcaggatgctgccagaaaatattttggtgaaaatgctgtcaatttatctgtacctgactctgccgttttggcggggatgctgacatcgccaagtgcctttaacccgattgatcatccaaaggccgccaagtggcgacgaaacgttgttttacagctgatggttgaaaataataagctgacccaggcgcaagcaaattactacaagaaaacgccaatcacactgcgggatacctatgttcgaaaagacggttacaagtatccatattactttgatgccgtcattgatgaagccatcagcaagtatgggatgacggaatctgagatcatgaaccggggttatcggatttacaccaatttgaatcaggctcagcagcaggcgatgcagaacaactttaataacaatgccatgtttccggccaatgcggctgatggcaccgaagttcaagcggcatcaattggggtttcaccgaccacaggtggcgtgactgccgttgtcggtgggcgtggtaagcacgtctttcggggttacaaccgggccactcagattacccgtcaacctggatcgacaatgaaaccgttggctgtctacacgccggcccttgaagccggctataagttcgactcggaactggttgataagaagaaatcttatggcaccaatcattacacaccaaaaaactataacaatgtttatcaaggaaaagtgccgatgtacgaagccttagcgcaaagtatgaacgcgccggcggtttggctgctgaatcagatcggcgtcaatcgcggttatcaatcagtcaaagactttaacattccggtcactaagaaggacaagaatctggcgctcgctttgggcggaatgtccggcggcgtttcgcctcaacaaatggccggagcttatacggcctttgccaacggcggtaagattgttaaaccattttatattcgtaagattgttgattctacgggtaaagtggtggtcgataacacggccaagcaggaaggccgtcaaattatgtccagttcggttgccaaacagatgaccagcatgatgcttggggtatttaacaatggaaccggtgctgacgccaagccgtatgggtatcaggttgcgggtaagaccggaagtaccgaagccgataataccggctctgctgacgccacaaaagataaatggatcatcggctatacgccagatttggtggtggcgacttgggaaggatttgataataccagtcaggcccaccatttggaaaacttgagtgggactggtgtcgggccactgttcaaaaacgaaatgcagacaatgttaccatataccaagaattccagctttaacaccaaggatgcccaatccatcgttcaaggtgaaagcagcaatgacaatctttgggataccattcaaaagaaaacgaatcaatatggtaatcaaatcgaacaaaaagccaaagatttgattgatgatgccaaaagctggttcaaacactaactttggcaggaagccatttcagtaatgtgttagaattaagtaaataaaattgttaggggaccctatttaatgaatgaaaaaatgaccgcaacaaccaaccagcttcaagccgaattgattgcatccgatgaatttacagagatcaaagctgcctatgacgcactcaagaagagtttggatgactacaaattattcaatgactttcaagatgctcaacagaatcttcagcaaaagcaaatgcagggcgttcaaccaacccaagatgagattcaaaatatccaggcgattgctgggaaaatgcgcgagagtcaattaatttccgcattaatgaccaaagaaaaggcactgagccagttattatcagatattaatgagaccgtgacaaaaccaatcagcgacttgtacaaatcataagcagatcaagcacgtgacaaaaggggccgagacaaaaagtgtgtgcacttttgcctcggcctttcctttatacataagttgaagaagggacctatcatgaaatttattcacacagcagatttacatctggacagcccgttcttgggactcaaaagtcatgttttacccaatgagctctgggagaaagttcatcaatcaacttttgattcctttcaaagaattatcgatgacgcaattgagcagcaagtggactttgttttgctggccggtgacttatttgaccgagaagaacgaagtgtggccgccgacgcgttcctagttgctcagcttaatcgattgaacgaacatggaattgaagcctttatcagctttggcaaccatgattactctacggcagatccggcttcatttggctacccggcgaatacactggtttttggcaaccaggttgaaaccaagcagtataccttaaatgatggggaagttgtggccgtcagcggctttagctttgataagcagtggattacccaacccatgattcaagactacccaacggccgttagtgatgttaattggaacattggcatgttacacggaagcttaagttcactcaattctccggaggccaattacgcaccattcacactgtctgaacttgaggaaaaaggttatgactattgggcattaggacacattcataagcgccagtcgttaaatgagcagcaaaccatcaattattccgggaacacccaaggccgccatattaatgaatcgggtgagaaaggatatttgctggttcaaagtgacgatcagcaccttcaaaccaaatttgtgccaaccgcaccgatcgtttgggaccgggtcgccatttctcttgataaaatgtctgcagaccagatcgttgaatcaattttagaaaaaattgctaatctgcactacgacaaattacatttcattcggatccagttggccagccaaacggcgattgatgccgacttactggccaaaattaataatggtgatctcttggatgacctgcaggacattaatgccgacaagtggcagcagctcaactgctggattacttcaattgaagccccacaagtaaaaagtctggtctatagcagtattgatcaggattattttaatcaagccaaggcggcaaccttgaatgacgaagtttttgatcaaattctcaaggactttaataagcagccaactttcatcaaggacgaagtcggatctgaagaatccaaacaggagatctttgatcaagccggggcgattcttcaggaaaatgtcgttcatgaagatactgaggaggataaatccaagtgataatcaaacaactcaacatttatggttttggccgctggattgatcaaaaaattgatatcaaaaatccacttcagatgatttatggtcctaacgaagccggcaagagtaccatcatcgcgtttatcaaagggatcctgtttggattcactgataaaaagcattccatccacggtcagtaccagcccaagggcagtgccccatatggtggtgaaattattttttcagctgatcaacataactataaggttgtccgaactggtttaaaatacggcgggacggtaaaattctacgatttggataacgatactgagcttaccgctgatgactaccagcagctcattgcgccaattgaccgaaccgcttatgaccaactgttttactttggcagcgttgatcagacggccttctacaaaataggtcgagacgaattacgactgcgaatccaatcacttggtgtcgccggggcaggcgattggatggacctccagaccaatttggataagcagtcggcaaaaatgtatgcgccccgcggtcgtacaaaaaagattaatattcagattgcggaatataaaaaactcgaagatcaggttagcgctgccaaggcccacttcccacactaccaggatctgcaggttcaattaaagcaggaccaggcgaaatcaaaggacctccaagctgatttaaaaactgctaatcaccagttggataacaaacgccgactgcagacggtcatgccgctggttaacaggctaaacgatctcaacacggtcgattcatctcagttgaagccacaattcggtgatgctgatctcaacgagtttaataaattaaacatggcactgacagctgaaagcgcggatgttcaaaaggctgaaacggccgtcgctgaagtggcccgccagtcatccagaaaaccggttcaaaccttctatgaggctcatagcgacacgatcgaacggttataccaagagctgccagccgccagaaaggttgctttggcaatcgaattgggcgattctcagctgcaggacgttcaacgacaaatccagacccagtctgcctcaattgcgaaaaatgaacagggaaatctaccacaagcatttgacgatcagaccttttctcgggtgaacgaactgctgcgggagcaacagaatctccaagagaaacgggcggaggtaactcgaaagaaaacccagtctgccgaacagcctcatggtaatggtgggctaatctggtatggtgtggcagccgctctggtggtattagggttcttattaggctctagttcgtttggatggattggatatattctggcggtggtcgcggccctttggggatggtacagtgccaaagggagttcaaagtcccagccaacctcaagcccaagtcatgaagacccagttgagatcgatcagaaacttgagcaaatccgaacagagttgacggctgttcaaaagcaatttgggctccagggaattgatgaagccaaatggctgccgatgcaaagttcgcttcgagaaattcagcgcctgcaacagagttatcaacagcaaaaaacagcactcaatgaacagcaggctaagtaccaggattaccttgaccaatggcaatttgccagtgattggctgaagtttgatcaaacaaagtattcgaccgccattgaaaccatcggcaagaccgttgctcattggcagcagttgtctaccgattatcagcaccaacaagcagtactcactcaggagaagaagacactggctgccgcaaaagccaagctggtcgaactgacccagcaaaaacaaaccttcttgaaggatcgacatgttgaaaacgacgaagcatttcaaaaaggtgttgcctttcaggccgaactggccaagcaactggatcaaaaggccacgcttgaaagtcaaattaaggccgccaaaatttcaattcctgaaaatattgaccaagatgccttgaacaccgacgttcgtgaagctaccgaaaaagtgcagtccttacaagatcaactgaatgatttgagccgggaaatgacccgggttcagactgaaattgccggtttaatcaagaatggccaatactacgatttgcggcaggagctggccaatcaacaaactgaaattgttgagaatgttcagaagtacctggctttgaagctcagttcccagtggatccaggcggtgttggacattgccagcaagggtcgactgcccaagacactggcattagcaaagcaatatttcgccactttgacgaatgatgcctacaaggagattatttttaaaaaagaaatttctgtcgttcgaaaagatgatgtctcctttccaatcaacgaattgtcaaccgggacgttggaacagctttatttagcactgatcttttcgatggcggttggcttcagcagtcaatatccaatgccaattatcattgacgatggctttgtgaactttgaccagcgtcgaaaagcggcagctctggcaatgctgcaacaggtgagtgagaagactcaagtgctttacttcaccgccaatctcgatgcaaatactgattccaagctcgtcttagatcttaaaacgctttaggaggcgattttatggcaaaacaattgatggatatcaagttggatgaagaatttgagatgtatgtcttactaaaagacgcctccaagcgggtggctaaaaatggtaagccatttctgtcgttggtctttcaagatcagtccggccaaatctcaggcaaatactgggatgcctcgccaacagatgtggagcagtttgtttcaggcaaagtcgttctgctgaaaggtaagcgggagaactatatgaattctccccaaatcaagattctggcaatgcggctggccaaccaaagtgagccccacgatccggttaattttgtcaaacgggcggggatgtctcgcgatcagatggaagaatacattgaccaaaccatctttgagattaccaacgcaacctataatcgaatcgtccgcagtttgatttccaagcacgccaacgcgttttatacctttccagccgcaaaatccaatcaccatgattttgccggggggctagcttttcacaccatttcaattctcaaactggcccattcgatcgtgaatcagtatgagggcattaatgccccattattgtacgcaggggccattttacatgatctgggtaaaaccattgagctgtccggtccaattgccacagagtacaccttagcagggaatctgttaggacatctcagcattatggatgccgagatcgttgaagcggctgacaagttgggaattgatcccaaatcccaggatctgattttactgcggcatatgattctgtcgcaccacggattactggagtatggttcaccggaacggccgaagatattggaggcagaaattctgcatcatttggatgagttagatgcgacgattatgatgattcaaagcgccactaagaatgtcgaacccggccaattcagtgatcgggtctttggattggataatcgacgattctacaaacctgagaaatcagttgaccccaaacaaaaaccgacccaaggggaattgttataattgacgggatacaaaaaggattggacaattaattgtccaatccttttttgtatgaatgatttaaaaattacttcttagctgatgagctggttgaaaggtagtctgataagacgttttgcaggtctttatcttggatggtaactttacccttcttaagaaccttagaaacaactgaatgtaaggtattgctatcagacatcttgctggtaacgatttgatcctttaattcagattcgtgttgcttccaagttccctttgatggatggttgaccatttggattacttggtaaccatactgagtcttaacaggggtcttggtatattcaccgttcttcagcttgaaggcagctttcttgaagttggcatcaagtgacgtgttggtgttgtcgaatgctgcgattcggccgcccttgttcttagttgctgtatcagttgaatactttttagctaagcttgagaagctcttaccgtctttaagttcactgataactttttcagcagttgatttctttgaaaccaagatttggttaacagttacttttggttggtaagacttgaattgagtttcaagttgtgcgtcggtaatcttgacgttgtccttaacggcttgcttcaataagagattggaacgaattgaatctttcaattgtgaagcagtcataccgttttgttggagaactgagttgaatgatgaaccgtattgcttcttgtatttagcgaattcactattaacttgagagtccttaacatctttaccgtattgcttttccaagaccttgttcaagatcatttgctgcaatacttgtttaccgcttgaagtactcttcaaactgctgtaataagcactttcagtaatcttaccaccgttggttgttgcaacagttttgctgccacaagctgcaagggtaaaactcatcataatgccggctaaaacgattagccattttttcatacaaaaacacatccattcctaaaagtattcgtctgcaaagcaaacgttcccgataataataacataatctgcgtcgtttatataatgacctcaagaatttaaacaaatattcatattttacttactttaatttgtcggtatacttgttgatttcgtcaagccgtggctgaattttgaacatcgcttcatccacatcccgtgagatgtcgttaatggtcttctcaaggaccggcatctgcgctgtgaaagcattcatcgacttcttaaagtcatcataagcgcttttccagtcagcggccttttgctttcgatcatcaaaggtcgacttggcccgctcaacgaactcttggggagtttcttttcggctgtataaataaactccggcgacaacggcagttgcaccaacaattttaaaaacggttttcatgattaatcacccatatgttgttcaatggattcttgaatcgcctttaactgttccggtgaatatttgttggagttatccttgaagatcatcttaaagtcgtcgttactggtatatcgggggaccaggtggaagtgtgaatgaaagacggactgataagcgacttggccgttattatttaaaatgttcatgcctttgatgtcgggatttgaagctttgactgcccgagcaatctttgggattctggcaaaaacttcactggctaattcttcatcatattcaaagatattggcgatgtgcttctttggaatcaccagcgtatgtccaggagtcccttgagaaatatccaggaatgctttgacaatgtcgtcctcatacacggtgtagctggggatctcatttcttacgattttacaaaaaatacaatctttcaaaatttctaccttctttctgtgaatactaatgatattataccattattgcgtttttggcccagctcaaaggctaattttgtatggtataatcttgtttgtacatttatcatgatacggaggtaaacaatgaccttacaagtttcgaatctggttgggggctattcccaagtaccagtgttaaaggacgtcaattttgacgttaaggatggcgagttggttgggttgatcggcttaaacggtgccggcaagtcaacgaccatcaatcatattatcggtttattaacgccatttaaaggctcaatcaaaatcaacggcgtcggcttaaacgatgacgtgaaacaatataaagagcagattgcttatattcccgagcagccaattgtctacaaggaattgacgctaaaggagcatttggaaatgaccatgctggcctatggacttgatcaagacgaatcctggaaacgggcacatgacctgctcaaacttttccggctggataataaattagactggttcccggacaacttttcaaaagggatgcgccaaaaggtgatgattgtctgtgcctttttgactaacgccaaactctttattattgacgagccgtttcttggcttggatccactggccgtaaacgacttattgaacctgatctctgaaagaaagcaacagggagccagcattttgatgtcgactcacgtgctggataccgcgcaacgttattgtgatcggttcgttttacttcatgacggtcaagttcgcaccgaaggaacgattgaagagctgcggaaattattcccagatgccggcgattctctcaatgatatttacctgactctggcaagggaaggcgatgcctcatgaagcagttattcaggcagcgtttaacgacgcatctaaaggaaatgatgcgctatctcagattggtttttaacgactactttgtcttggctttgttgtttgtcattggtggcttgggatactattattccaatgcgcttaagcagctgcacaccggtctgtggtgggcaccaattgtgattatcggtattttgttggttagcgttcagctgggcaggtttgcgaccttgattgaagccccagactatgtttttttgttgcccaaagaatctgaactttataactatcttcgaagcggctttcggtatagtctttcgattgctgtcgcaatacaagtcctgttttggatcttgttgatgccgtttgttcaagttaccatgcgcgccacatcgacggagttgtatctgcttttggcaaccattttaatcttgaaaataacgtggctaaataccgactttgcccgtaaataccatttgcagcaatcctggttggccagtcggctcatctttcgattgctgctcccagtgattgcattggggtcgtctatctacatcaactattggcttgggttgggcattgctgtggctgcgcttttcgtcagttatttttcccgccggaattgggtcagccgatcacttgactggacgacgatgattaccgatgaaaacagtcggatgcacaccgtctatcaattctttaatttatttacggatgtgccaactctgcaaggttctgtcaaacggcgccgttacgtggacgggatcttgagccgaatcaagctgattccaaaaaacacctacttatatctctacgctcacggaattgtccgtgacaatgagatgagtgggctatacgttcgtctgctggtgatcggaaccttatttctggtattcgtcaagggcgagctgttacccatctttttgagcctgctgtttgtctacctaattgggttccaaatgattccgttttattttcatttctcggataacgccttcgtgcacatttatccaattaccaatcagtaccaattgaagagttttcaaagggttctgctgtacttgttgagtacggttggcgttgtttttgccgtggcagttctcgctgttaatttggccacgccggtcacgatcatcggcgtgattgtcggcgaagcactcgaaatctgggcatttgtctatctgtatttacccagacgtttggctcgaagcgagcgaaccagataaattgttgaataataggagaatgatatgcgcgtaagaaaaaagccgtgggctgataaatatatcaaaaaccacggcgactatattgtgaccgatccaaagaattggttgggtaaatggcaggaccggtttgccaaagtccaacccttaaacgttgaggtcgggattggtaagggccggtttattatcgagaccgctcgagccaaccccgacatcaactatattggcattgaactgcagacttcggtcattgccacagcactgcggtcgtttatggcggatccattgccaaacgtgcagtttgttctgactgatggcgccaatcttgatgaattgttttatgaaaatgaaattaaaaagattttcttgaacttctccgatccttggccaaaaaagcggcatgccaaacgtcgtttgacatcaccactatttttgaagacttataatcacgtgctggaccaggatggggatatcgaattcaaaactgataatcgcggcttattcgaatacaccttggtcaccatgaataatttcccgatgaagttcgattatgtttcgttggatttacaccattctcctgaaaatgaatcgaatattgaaacggaatatgagcaaaagttcagtcccaagggacccatttataagctgattgcgcattttacagcgtcatgacttgatgcttaaccacttgctgtgaggtttggtcgacccagaattcttctgttttgcgatcaccttcagggttcaaataattgaagccaaagtgaaaaagcggcgtggagtcagtggtcggtagaatgctccaactgccaatatatttgaagccttttaatgcggctgattgtttggtatccttgacgatagctgctaaaaacttttcgtgtttgcgatcggacttggccacgatataggcactgccggcaagcgctgcgagtgccaggccatagaagacggtttgttttttcatcatttcaccttttttgtatatgatatgtatactttagactattagcagcggatgagcaaactgatttggctgggcggaaatttgtgctatgatgtactttacattagtaagtgaaaggatgataattttgcaaaatttacctaaaaccaatttaaaagatttaaccaaacaacttgagaacggcaagtatatgctgttcttcaccgctgactggtgcccggactgccgcttcatcaagccggcaatgcctgcaattgaagccgaatatccagagtacacattcttacaggttgatcgtgatgaaaatatcgatcttgccggtgaaatgggcattatgggcattccaagttttgttgcctattcagacggtcaagaaatcggccgcttcaataatggcgaccgcaagactaaagccgaagttgaaaactttattaactcgttagcaagtaccgtagcaaaataattaattgttggaaggaattttgaaatgttaataaccagttataacccaaacagcacaggtgacacaatggtcctcattatgaacccggatgtgggtgaacaaagtgtgacaattcatgataaggttgcccggatttttgccgctgatagcaatcagacgttggggtacaactttttagaagcaagtaaagtccttccagaaattgtccatgaaaatggccaagttcatttaaccgaagaccaggttactcgcttgaaccaatatttgggcgatcacggttttccggcagatatccgttatgataatcagcccaagtttgttgtcggctatgtcaaatcagtggaagaccaccccaaggcaaatcatttacagattaccaaaactgatattggcaccggtaaggacgtccaaattgtcagcggctcgccgaacatgcgcgaagacattaaagtggttgttgcgttaagtggggctatgatgcctgacggccagattatttggcccggtaaattgcgtggtgttgaaagcgatggcatgatttgttccggccgcgagttggggttgcccaacgcaccgcaagtccccggggcactgattttacctgatgattatcaggtaggggatgcctttgattttgacaaggcacagcatttatttgattaaaggactttgggtggatgagtaatgaagcattatgatggacccgcattttttcggcggaagggcattacccgaaagcctcatcaagagcgggaaataaaacagaataatcagccggtggcaccgaaaatccaagatacacgatcaagcaaggtccctgattccaagtttgatcgtcgggatgagaccccggcttttttgaaagaaattaaaaatttcaaaccgcaaaagcggtcaaaatccgataaacggaaacagcaaattcaaacgaattattttctcagccaggcgcatcgtcgtcaccgtctgtacgatgaattgacacgccggctgaggattacatatgatgatctcattgtgattgccgataagcaaccaacaattgatcagcctcgtgagcagcatccaaagcaacccgttcaatcaccaaaacccgccaagccgactgaaggccaacctcagacatcacctcaaaaatcatctttgacagatcaaccaaagatcagctcaggagaaggggtacggcatttaaatcgtcaaccacggaaggctttgaatcaccatgggttgggacagtcattcaattcaattatgcataaccaaagggccagcgaatctgacctttctttgtttaacgctcaacaactgagtcacaatgcccaggttaaaaaagtgaatcacgttaatcaacccacgaagggtgttcaacattcattggctgaaccaaacgtctcagagaagccgactgaagacaggggttaccaatttccgccgctgtctttattagccaagcctcagcaagccgaatcagaatcgattgatgactggattattcaccaatctgaaatcctgaatcaaactttctcagccttcaaggtcaatgcccaagtggttgactggacaaatggcccaacggtcacgcaatttcaagtcaaattggcactgggcgtcaaagtcagccggattaccaacttaaccgatgacttaaagctggccttggcagccaaggatattcgaattgaagcgccaattcctggtaaaacgacagtcggaattgaaattcctaatcccaatccgagaccggtggtcctttcagaagtgatttcaaccaagcattttcaagatagtcaatcgccactcaccactgccttgggtgttgatttgtcaggagttcccagaacgacagacattaaaaagatgcctcatgggttgattgctggggcaactggatccggcaaaagtgttttcatcaacagtttgttggtttctttgctgtacaaagcgaccccggcggatttacgattactgttaatcgatccaaaggcagttgaactggcaccttatgacgggattcctcacttgttatcacctgttatttccgatcctaagacggccgcagcttcccttaaatgggtcactgaggaaatggatcagcgttatgaaaagctcgcagctgctggtgctaaaaatattgaacagttcaatcgacaggcaagtgaggctcacgagtatgggctgaaaatgccttatattctggtgatcattgatgaattggctgacctgatgatggtcgcttccagtgaagtcgaagattacattgtccgcatcactcaaaaagcccgcgcagccggcatccatttgattgttgccacgcagcgtccaagtgttgatattgtgaccgggaccatcaagaataacattccgactcggattgctttcatggtatccagccaagtcgattccagaacgattttggattcggccggagcagaacgtttacttggccgcggagatatgctatatctagggagtggtgcaaatcagccggtccgactccaaggtgcttttgtcaccaatcaggagcttgacggcattgttgattatgtccgccaacagggagaacctaaatacttatttactcctgatagcttgaaacgagctagtactgaaaccagctccgaggatcgtttgatgccccaggttttaaaatatattggcaatgaagagacaatttccacttcaaagcttcaacgggtattttcaatcgggtataatagagctgcaaacattattgatcatttgcaggaaaagaacttggtttcagagcagcaggggtccaagccgcggacagtgtattacaagccggcagcagatgaatccgctcgggaatcaccgcaaaatcatcaaaaataacataatggataggtaggatgtctaatgaattcagatacggtatatcattttgtaggaattaaaggaaccgggatggccgccatggccttaatcttgcatgaccgtggtgagaaagtgcaggggtcagacattgaccagtacacgtttacacaacgtgggcttgaaaaggctggtattaaaattttacctttcgatgaaaacaacattcacgaaggattgacggtaattgccggtaactcctttactgatgatcatccagaaataaaaaaagccagagacatgggattgacggtttaccgttatcacgagtttcttggcaaaatcatcaagggtaagaccagcatcggggtttccggtgcccatgggaagaccagtacgactggcctgttagcccacgtgctttcaggaattgcaccaaccgattatttaatcggtgatggttctgggaaaggtgttcccaatgcccggttctttgtctacgaagctgacgaataccgtcgtcactttttggcaactgaacctgattatgccattatgaccaacattgactttgatcatccggattactacaagagtatcgatgatgttgccgatgcatttcaaacgtttgcgaaccagacgaagaagggcatctttgcttggggtgatgataaacgtctccgtcaactaaaagccaaggtaccaatttattattatggcctcaaggatactgatgatttccaggcggttgatgttaaacggacgaccagtggttcgagctttgatgtcacttataaaggtaaaaatctgggaaacttttcagtaccgttgtttggtgagcataacattttcaactcattggctgtgattgctgtggcttactttgaagatgttgatttggatgaaattcgcaaagaattgaagactttccaaggcgttaagcgtcggttcgccgaacgtaagattgccgggatgacgatcattgacgattatgcccatcatccaactgaaattaaggcaaccatcgatgctgcccgtcaggaatatccaagcaaaaagattgccgtggtatttcagccgcatactttcagccgaacgatcgctttgatggatgattttgccaagagcttgaacttggccgatgaagttttcctgacctcgatttacagttcgccgcgagaaagtcacggaaaagtttccagtgaggacctgtcaaagaagatcaccaagggtgggcgcatcttgtccgttgacaatatgtcgccactattggactacgataacgacgtggtcatctttatgggtgccggcgacattcaaaagtatgaaaaatcttacgaagatctgctaagccatttaagcaaaaaaattaattaagatatcttataaaagccgttagttgagtcctaaatacttgattaatggcttttatttggtagaattacttaacagtataagtataaatactgcaaattgtttgaggcaatatttgaacttacaaacaaaagggagcggatttaatgaacaattatccaaacgaacaacaggaagctcgacgagtcgttaacaacgcagccgggttgaatgcttttttaactaaaatgtatggctggatgagtttggccgttttagtttctgctgcaacagcatttttagttagtgggtctgttgctggtggaatggcggcttacattgcaggtcaccaaggtgtgatgtggggatcaatgattttatggtttgttttgccatttgtcatctcacttcaagcattgaaacggccgaccctcgcgtttacagtactgatgttgtattcaattctaagtggttttgttttcgccacgattgcgtgggcgtatacaggtgcctcaattgcggcagcttttgtttccgcttcggcaatttttatcacaatgacaaccgttggattggttacccacaagaaccttgatcgttggggtgcccaagcaactgctgctttaattgcgttaatcattgccatgattattaacatcttcttgcgtagttcagtgatttcatttgttttctcgatcatcgcagtgttaatcttcacggtcttaaccgcctatgacacccaaaagatgaagcagatgtataaccaatattctggtaatggtgaagtttccatgaccggtttggcagtctttggtgccttacaattgtacttggactttgtgaacctgtttctccaattactctcgatttttggtaacaacgaccgttaattcagatttcgtcacaacgattggccattgatttggttgatcgttttttgttatctgtcgtggtaaaattaaagtaacagttttcaccagaggagaagttaatgactaaaaaattattattaattgatggtaatagtattgccttcaaagcgttttatgctttatacacggccatggacaaatttaccaatccatctggcctacataccagcgccatctatggctttaaccggatgctggacaaagtattagcagacgagaagcccaccgatgtgctggtcgcatttgacgccggcaaaaccacttttcgaacgaaaatgtacgctgattataagggtggtcgggcaaagacaccaactgaactttccgagcaatttcccttcttaaaagaattaattaatgcccgtggcatctccacctatgaattaccggattatgaggccgatgatattattggaacgctcgccaaaaaggctgaagaagctggtgactaccaagttgtgattgtcactggcgatcgagatttgacccagttaacttcagataagaccacggttcaggtttctaaaaagggcgtcaccgaactggaaacatatacccccaaacacgtcgaagaaaagttgggtgttaaaccgagccagattattgaaattaagggtctgaaaggtgacaactccgacaactatcccggcgttgaaaaagtcggtgacaagacagctgtcaggctggttcaacaatttggcacgattgacaatctctatcaaaatatcgaccaggtttccggtaaaaaattaaaggaacatttgattcatgaccaagcccaggccgagcgcgcccacacgttggcaacaatcaaccgcgacgcgccggtaacagtctctttggatcagttgaagtatcagggagacaatatcgataaactgaccgatttttacgagcgaatgggcttcaaatcgtttctggccaagttatcagttgatgatcaggatcatgccgatgatcaggcagatattcaatacactgtcttgtccgccaagaatgcggctgagctggatcagttcacagatgaagtgacttttcacctggaaatgtcagaagaaaactaccacacatcgccgttggttggctttgcgattggacagggtgacaaatggtatgtgaccaacgatcctgaattgcttcacaatcagcatgtcattgaccttttgaccagcaagactatcaaaaagaatgtctttgatgccaaacgaacctatgtcggtctttatcgacaagggattgagcttgccaacgtggacttcgatatgctgctggtatcatatttgcttaatacaactaataatagcaacgacgtcggcaccgttgcccatttacacggattctataatgttaaaaccgatgaagaagtctatggaaagggtgccaagcgacacattgacccgcaatcacctgcctttttggcccatttggttcataaggtcaaagcgattgatgctcttcacgacgggatgtttaaggatctggatgcccataatcaatccaaactgtactgggatatcgaaatcaagattgcctttgtccttgcccacatggaaatcaatggcatcaaagttgatgcagccactttggagggcatgggcagtaaatttaaagagcggctggctgaaattgaacagaccattttccaagaagctggtgaagaatttaacattggttctcccaaacaactgggaaagattctgtttgaaaagctccgcctgccgattctaaagaagaccaaaaccggttattcgacctcagttgacgtgttggagaaattggctccggatgcgccaattgttcaaaacgtgttggactaccgccagatttccaaactacagtcgacatatgttgatgggctattaaaggtcattcatccagatgattccaaagttcacaccagatatctgcagacgttaactcagactggtcgattgtcttcagtcgatcccaatctgcagaatatcccggttcgctccgaggaaggccgacttattcgccaggcgttcattccatcacatcccggttggcagattttctcctctgattattctcaaattgaactgcgggtgttggcgtcaattaccgacgaccaaaatatgcaggacgcctttaaaaacggcgaggatattcatgccaccacggcacggagaatttttgggctgccgtcaaatgaagaagtcaccccggaacttcggcgtcaggccaaggcagttaactttgggattgtttatgggattagcgattttggtttagcgtccaataccggcattaccagaaaacaggcgcatcagtttattgaacgttattttgaagaatatcccggagttaaaaaatataccgaagacatcgttgaatttgcccgtaaccaccgctacgttgagacgattgcccatcgacgccgttatttgccggatattaattccaagagctttaatctgcgttcattcgctgaacggactgccatgaacacaccaatccaaggcagtgcggccgatatcatcaaaattgcgatgattaatatggccgatgcaatcaaggatatgaaaacccgcatgctgctgcaggttcacgatgaattaatttttgaagttcctgacgaggaattggacaccgtcaaacaactgattccaagcgtcatggattcagcgatccacttgaatgtgccattaaaagttgaaagccactggggtaagacctggtatgatgcaaaataagttgaagcaaatgggggatctcaatgcctgaattacctgaagttgagaccgttagacgcggcctgacccaattggttaaaggaagcaccatccaatcggttgatgtgttgtatgccaaaatgattaatttaccaccaaacgatttcaaaaaagccctccgtggcaaaacgattgaaaaaattgatcgacgtggtaaatacctgctgattcgattgagtgacaacctaacgattgtttctcatttaagaatggaaggcaagtacgatgtggagcccgaagatgcaccggtcggtaagcatacccatatcatttttcatctgaccgatgggcgtcagttgcgttacaatgatacgcgaaaatttggccgaatgaatttggttgataccggcactgaaatgcaggttgccggtttgaaaacgattggaccggagcccaccgaagataatttgaccgtcgattacatgcagaaaatttttagcaagagccgtaaagtgatcaaaccatttttactagaccagagtaatattgccgggttgggtaatatttacgccgatgaggtcttatggctaagcaaaattaatcctcaacagcctgccaacacgttgacgttgagacaaattaaagagttgcgaaaaaatattattgccgaattagccaaggcgatcgccggtcatggaacgaccgtccactcatattcaactgcatatggggaagctggcagttttcaaaatcaattgaatgtttatggtcgtgaaggcgaaccctgcccgagatgcggcacaaagattgttaaaatcaagttggctcagcggggcacccacttttgcccaaaatgccaacctttgcgtggtgtaaaaaatgactaaattaattggcttaaccggcgggattgccaccggaaaatcagtggtcagcgattaccttcatcagcaggagattcctgtgattgacgctgacatcgtgacccatcaagttgaacaaaccgggactcctgggctccaagcactggtggacgcatttggacagcggattttgctggctgacggcgcacttgaccgccaggcaatcggccggattgtgtttaacaatccagctgatctcaaacaactggttcgaatcattgacccattcattcgcgaagagattttttctcagttgaaacgttatcgggatgctgaattgaccgtcttggacgcaccaactttatttgaaaatggctatgtccatctggtcgacgaggtggtggtggtttactgtgatccggtcactcagttgcagagattgatgaaacgcaataaactgagtattgtaagtgcgactaaaagaatcagaaatcaatggccattgcagacaaaatgcgatttggctgatacaattatttataactcaggaacaatgacaacgacgctgacacaagtcgacagatggttggcgaaggaaacgaaatagacgaggtgaacaccatgcaatgtcctcattgcggatacaatggttccaaggttgtcgacagtcggccaactgatgacggtcgggtgatcagacgaagaagagaatgtgaacactgcggttttcgatttaccacatttgagcgggtcgaagtaacccctttattagtggtgaagaaaaatggtaaccgcgaagaatttaatcgtgaaaaactgttaaaggggatcgtcaggtccgctgaaaaacggccagtttccatggatgccattaccaatttggtggaccgggttgaaaataaattgcggtcactgggcgagaatgaagtttccagccaacaaattggtgaatacgtcatggaagatttggccaatttggatgaaattgcctatatccggtttgccagtgtttaccgtcagttcaaggatatgtcggtcttttataaagagcttaaggaaattatggaaaaggataagaaaaagggtcaggatcactcgggggacaaataatggcagagtcgttcgataaattaacacccgatacaaaatatctcacgaccaatgcccacattaatcggagcctcgatcacagtgttttaaccaacttgtatctaccaatcattggtgaaaaagcattgggattatacaatttgttgtggtcgatgagcttaaatgatcacaatcagttggttttgcataagcattacgaaattcagagcatgttaaattgcaaaattgatcagctggtggcgattcgaaagcaattggaaggcgttaaactgatcaatactttggtttcccaaaacaaaccggatgtcttgatctactcgttgaatctgccgctaactgctgaacagtttttacgaaccgatattttgtcgattattttattgggcaaagtgggcgaaacaacctacaagcagattgtcgaccgactggtgctgccacttccggatctcggggagacgaccaatatttcggcttcactgctggatttatttgctgtaccccagaacctgattaaaaacattccaggcgcagtcaatgacgccaagcagaccattgttcgatccgctgcaaatgtcagtgagaacagtttcgaaccggatagtcgccaatttaacttcaagctcttattaagcatgttggaaaattcatacgtcgatcttaattctgttaaggccgctcgtgatttgattttgtcagagaatttgctctatggaattgatgagatccaaatggctaaactcattcaaaaggcgactaatctcagcaccaatgaattgaatcaatcacagttgaaggcaattattactgataatttcagccggcatcaagcagagaacgtggagaaagcagcatctactgctgagatcacgccttcttccgcaaaattcgacacggcaaccaatcaactgatttcaattagtaaaaagacggctccagtcgtgtttttggaacaaatcaagaaacaaaagcacggtattgtgaccagcggtgagcagcgaaccttgcgcgagcttgtcaacctgcgcgtgttgccgaatgaagtcatcaatattttgatttactatttattagttgatgaaaatcgttcgactctcaataaaaacttgatgtcaacgattgccgatgattggtcacaacacgggatttttgatgccgagcatgcaatcgatgccattaagaatcgaacaatcgacaaacagaaaaaggctgatcagtgggctgccaagtacaaacagcggcgggttaatgtcaaagagaccctgccggattgggcgaaggatgatcagccttcctctgccagccagccgacctcacagttgactgaggcccaaaagaagcagctcaaagcacagcttgataagttaaaaaagccggggagtaggtgagattgaatggaaaaagtaagtgatttcgtcaagaaactaatggaagaccgtcaatttaagggtggcaatgtcgcatcaggtttccaaaaaattattgaacagatcaaaaatgaccctgagatcgccaaatttcttcaggatcatcaaggtgaactggctcctgatgcggttgaccgttctgctgccaaattgtatgagtatgtgaatgtcaaaaatcagattaaggccaagaaacaatcatttgcacctgggtatttgccccaattggtcattaacgatcatttgattgatattgcgtattcagcctctccagaggtgatcgaaaaacagcgcagtcagtccttggcacgtcgaattaagacggtttcaatgcctaaagatatcaaggatgccaggatcgccgaattcgacggggctgatcccgataatccagaccccaatcgttatacagccctttcaatggcattggattttattgcccaaatgaaggccgacaaaaagactttccatccgggtctgtacatatatgggccgtttggtgtcggtaaaacatatctgacaggtgcaattgccaacgaacttgccgataacgggattcaaaccactatggtgcattttccaagttttgctgtcgaaatgaaatcggcgatcaccgataactcggtcaccgaaaaaattgatgtgatcaaaaagtcgccggtgctgatgattgatgatattggggctgactcaatgtcctcgtgggttcgtgatgaagtattgggagtcattttggaataccggatgcaacagcagctaccgacgttttttacgtctaatttttcaatggcccaactcgaacaggaacatttgcgtatcaatcaaaaaggcgacgatgaaccattgaaagccaaacgactcatgcagcgaattcgattcttgtctcgtgaggtcgagatgaccggtaaaaatcggcgaccagtttaatttacaaattgaattgacatttttgaacggcaactctatactaaatgtcaatgaatcaaagagacatgacagtgatgactcatcacagggagaatggttccagcctggaagaccgtttgttgagaaattgtttgttaccactctttgagaatggattgcggataatgctttcccggttggtaccgttagcagccacttgagagctttttggataattgtatccaaaaatccaatttgggtggaaccgcgctaattgcgtccctgatgtacttgtataagtatgtcaggggctttttttgtggctccaataaaatataaagggagtaagaaatatgtcacaactttcatttgaatttccagatggtagtgttaaacaatttgatgacggcgttacctcagaagccattgccaaatcaattgccgtaagtttaggtaaaaaagccgttgccgccaaggttgacggaaaatgggtcaacaatgacgagcccctacataaaggcggcaagattgaaattgttacgtcagatagtgacgaaggcctcagtgtattacgcgcaactgccgcccagattttgaaaatggcaattgccaatgattttgataatatccactttggtgaaagcgatgccgataaagacggcttcttcgttgatactgacaaaccagacactcaaatcagtgttgatcaattgagttcacttgaagactcaatgcataagattatcaaacaggatctgccaatcaaggtggtcttcttaagcgctgctgatgctgcaaaggttgccggcgatgatccttatcaaaaagaattggtcaaagcaaacgaagttaacggccaagttaaattcttccaaatcggtgacttccaatcaatcgccgaaggagctgttttaccatcaaccggcaaagttaagatcttcaagctgctctcagttgccggagcttactggcagggcaagtcatccaacccaatgcttcaacggatttatgcaactgcttttaacaagcaaaaagatttggatgccgaccttgagaagcgcaaggaagcccatgaacgtgatcaccgagtcatcggaaacgaactggatctgttctttgttgatccaaaagtcggtgccggcttgccttactggatgccaaacggtgcaacgatcagaagaaccattgaacgctacattgttgacaaggaagttgccaacggataccaacacgtttacacaccggttttagccaaccttgatctgtataaacaatcaggacattgggatcactaccgtgaggacatgttcccgccaatggacatgggagacggtgaagagcttgaactgcggccaatgaactgcccaagccatattcaaatttataaccaccatatccgttcatatcgtgaactgccacttcggatcgctgaactcggaatgatgcaccgttacgaaaaatcaggtgctttgtccggacttcaacgagttcgtgaaatgactttgaacgatggtcatacatttgtcgccttggaccagattcaagaagaattcaagaatatcttgaacttgatggttgaggtttatcacgattttgatattaacgattataccttccgtttgagctaccgtgaccccaagaacaccgaaaagtacttcgatgacgatgaaatgtggacccgtgctcagaccatgttgaaaggtgccatggatgaaatgggcttggattatgttgaagctgaaggagaagctgccttctatggtccaaagctggatgttcagaccaagaccgctctgggaaatgaagaaactttgtcaacgattcaattagactttatgcttcctgaacgcttcgatcttcactacatcggcgaagatggcaaacaacatcgtccagtcatgattcaccgtggcttggtttctaccatggaacgattcgtcgcttacctgactgaaatctataagggtgccttcccaacctggttagcaccacatcaagttaagattattcctgtcagccaagacaagcacctggattacgctaagaagattaatgaccagcttcgagcattgaagattcgttcgtcagttgatacccgtgccgaaaagatgggttacttgatccgcgatgcacagactcacaagattccatataccttagttgtcggtgatgaagaagtgagtggcaacagtgtttcagttcgtaagtatggtgagcaggatacccaatcagagtcagttccggacttcattgatgaagtatctaaagacattgcttcatattcacgtgaagaagattaacggattaccaagtcacttattaatgcgcttaacggttcatagttgacacataagtgattagatgatattctgtaatagttgttcaaatgaaagcaggagctacccgcttctcgcctgagtaaatttctgaatttgctgggcatgatatcgagtaagagcttggtcagccaagttctttaattgagagcgggcgcaaatgtgtgcccgctctctttctgctttttcaaattattcggaggtgaagtaccatagcaaaagatatgatggttaatgatggaatccgtgctcgtgaggttcgtttgattggtgctaatggtgatcaacttggtgttaagactaagtcagaagctcttcagttagctgaagatgccgacttggatcttgtcctggttgcaccgaaagccaagccaccggttgcaaagattcttgattatgggaagtatcgtttcgagttgcagaagaaggaacgtgaatcccgtaagaaacaaaaagtcatcagtgtcaaggaagttcgattaagcccaacaattgatgtgaacgattttaacaccaaattgaagaatgctaagaagtttttggcaaagggcgaaaaggttcgggtctcaattcgatttaagggccgtgccattacgcataaggatatcggccggaaagttcttgaccgaatggctgctgaaacggcggacgttgccaccgttacccaacgacctaagatggacggaagaagcatgttcttaatgctttcaccaaaagaccaagatcaaaaataatagttgttaaatacttgaggaggatttttaccaatgcctaaacaaaaaacaaaccgtgctgcagcaaaacgttttaagagaactgccaacggtggatttaagagtgcaaatgcttataccagtcaccgtttccacggtaagacaaagaagcaacgccgccaacttcgtggtactagtatgatggacaagactaatatcaagacttacaagaagttattgccacatctataaaatcaactatacattcaattattacttttcaaaatataggaggaattcaaaatgccacgagtaaaaggtggaacagtcacacatgcacgtcgtaagcgtgttttaaaattagctaagggttatcgcggtggaaagtctcgtttattcaagactgccaaagaccaagttatgaagtcacaggtatatgcattccgtgaccgtcgtaacaacaaaggtaacttccgtaaactttggattgcacgaattaacgctgctgctcgtcttaatgacctcagctacagccaatttatgcacggtttgaagcttgccaacatcgacatgaaccgtaaaatgcttgctgatttagcagttagtgatactgaagctttcaaagctttaactgacgaagctaaaaaagcacttaagtaattttgatgtgctaaaatgactttcaccgatagtttggtggaagtttttttaaataaatttactataatttaaggagcgacatatgttgtctcgatttaaaccaacatggatgattggggatatttacacgatttctccccaattcctgcgggatcataatatcaactgtgttctaaccgatttagacaataccttggtaccttggaactccaagaagggttctcaagcgttacgcaactggttgtcagaaaataaaaaatttggcattaaggtgattgttgtgtccaataacagtcacaagcgaattcaacgcgcggttcaagattacgagctgccgtttgttcccagggcaatgaagccgctcactatcggtatccggcacgctctcaaggaatttaatttacaaaagcgcaacactgttatgattggcgaccaattgatgactgatgtggtggctgccaacagttgcggtgttcgcagcattttggtgaagccactggtgcgtgacgatgcttggaataccacgatcaatcgttactttgaaaagattgtctggaataaattatcgaaaaaatatcctgatttacattggaaataggaggaattatggcaaatagtgaagttgttgttgacggtgaagtcgttcattgtgtgggttgtggggcagctgtccagacgactgacaagaacgcactcggatacacccctgaatctgctttaaagaaggggcttgaaaatggggaggtctattgtcagcgttgttttagacttcgccactataatgaaattgctcccgtcagtttatcggatgatgacttcttaaagctgttaaccagtatttctgatactgactctttgatcgtgtacgtggttgatatttttgatgtgaacggaagcctcattcccggtctccatcggtttgtcggcagcaatccggtcctgttggttgggaataaactcgatattttgcccaaagccttgaagcataacaaggtgaaggattggttgcgacaacaggctaacgcggccggtattcggccaattgatgttgagctgatttctgctaagacaaattttgatattgatcgtttgttggatcaaattgaaaagtaccgtcagggaaaagatgtttatgtcgttggggttaccaatgttggtaaatcaactctgatcaactcaattgtccgtcagtcaactggcatcaaggagttaatcacgacttcccgttttccgggaacgaccttggatcggattgatattccgctcaatgacggtcataacttagtggataccccagggatcatccagcctgagcaaatggcccaccatctgtcgggtaaagaattgaatttggtgacgccacaaaaaacaatcaagccgaaaggttaccagttaaacccgggtcaaacgctcttctttgccggcgttgcccggtttgattacaactctggtgacaagcgtcatggattcacagtgtatgctgagaataatttattcattcatcgaacgaaattagaaaatgccgatgagttttacgctacccatgtgggttcatttctaacaccgccaaccgaagatcaaaaggctgattttccagctttggaacctcatgaatttaagtccactgaaaaaagtgatttagtgatcgagggcttgggttgggtaactgttccagagggcgtttccgtcactggatgggctcctaaaggcgtatccgttttgatgcgcccagcaatgatttaactaaagagggacttatgaaattaacaggaaaacaaaaacgatttttaagagccaatgccaaccgcatgcggccaatctttgaagttggtaaaaacggtctttcaccagtttggcttgaagagattcaaaaagcacttgatacgcgtgaactgattaaaatcaatgtcttacaaaattccgcagcgaccgttgatgacatcaaggactatattgaaaccaaaagtgatgtgacggtggttcagacgatcgggaagactttggtcctcttcaagccgtcaaaagatccaaataagcaaaaattatccaacgaagttttggcgatttagaggtaatgaaggatgagcaacgtcatgaatcatgtcgaaacattaacccagacgaaaacaattacaaaacaaaacggtaaacgcatcgggatcttaggggggaccttcaatccaattcataacgggcatttaattattgccgaacaggtcttggatcaactggggctcgacaaagtttactttatgcctgatgccaatccaccgcacgttgaccggaaatttgcgattgatgccaaagatcgggtggccatgattaactgcgctattcgggacaatcccaagtttgccattgaaatgactgagattatgcgtggtggcgtcagttattcctacgacacaatgaaacagttgacccaacagcaccccgagaatcaatattactttattatcggtggtgatatggtcgattacctgccaaaatggtatcgaatcgatgatctggtcaaattggtttcgtttgtcggtgtcaaacgtgacggctacacaccagcttccaaatacccggtaatttgggttgacgtgccgttcatcgatatttcatcatcgctgattcgctcgaaaatgcgacagcaccagtcaattaagtacttggttccggccgctgttgaacattatataaaggagaaccatttatatgaaaaatgatcaactaatctatcaaggccattttgttccatacactcgtgacgagctggttggcaaactacgcgccgctctcagtgatcaccgttttcagcattgtctgcgtgttgagcagactgccatggacctcgcagaacaaaacggggttgatattgaaaaggcggcgattggtgggttggtccacgactatgccaagcaacgtccggatgacgattttattcaagcaatcaaggactatcaattagagcctgaactgctgaattatggcaacgcaatttggcacggtgttgttggttggttgtttgtcaaaaatgagttacaaatcaccgatattgatattttaaacgccgtcaggtaccatacagttgggcaccagtatatgacgccattggaacaaattgtctatatggccgattatattgaaccaggtcgggattttccaggtgtcgatgaggcacgcaagattaccaagaataatctgcaagatggcgttgcctaccaaaccaaacaaacgttgggatacttggttgcccacaataagccagtttttccacagacaatcgtgacttataatagttgggtaccaagttcaggaatagattaaggagtaaatatgaacagtaaagaaatttcagaagtcgttgttcgtgcggcagacagtaaacgtgccaacgatattgtggttctcgatatgcaaaaggttagtctgatggctgactattttgtcatcgctgacgcagcttccagtcgacaggtcaaggcgattgccgatgaaattgtcgatcaggttgaagccgatgacgttaatgtctacagtgtttctggtaaagattctgcccgctggattttaattgacctcggtgacgtggtcgttcacattttccagaaagatgtccgtgatttttacaatttggaaaaattatggtcggatgccccaatcgttaataccgattcgtgggtggaggcataatgatctatacagaattcgccaaattttatgatgatttatttgacgcaactctctatgatcgttgggcccattttgttgtgaacaagacaaaagggatccaaaaaccgccttcagaaattaaaattttggatctggcctgcggaactggtcgcttggcgattaaattagcccaaaaagggtttcaggtgactggggcggatctatcagaggacatgctgacaattgccgagcaaagagcacgcgaagcaagtgttgacgtgccctttattcaaactgatatgcgcaatctggacggccttgatcagtatgatttgatctgctgttttgatgattccttgaattatttgattgatcaaaatgatttggagacaactttcaaagcagtgtatgatcatctcaattcggacggtcagtttctctttgatgtgatttcaccttatcaggcaaccgaggtttatcctggttatatgtacaactatcggagtgaagatgccgcttttatgtggaccagctacgaaggtgacttcgcgccaatggctgttgaacacgagttgaacttcttccaatacaatgaggagaaggatgcttatgatgcgtataatgaaatccatcgtgagcgcgcttacgatgacacggtgattaaagatctgctgtcacagactggtttcttggtaactctggcaagcaccgattttggggacaaccccttcgtacgggaaaccaagcgctggttctttagtacgggaaaagactaaggaagtcggagaatatgcttcaagctgttgggattgtttcagaatacaatccctttcataatggacatttatatatgctcgaacaggcaaagcaggcaaccggcgcagatgttactgtcgccattatgagcggcaattggctgcagcggggtgaaccggcggcgtatgacaaatggcaacgggctcacgctgccctgctgggtggagttgacctggtcattgaactgccattattttcggcggttcagccttcccacctattctcaaaaggggcggttgatttggctgccaaaataaagtgtcggtggttggcctttggtgcagaacatccagaaatggattatcaaaagctgattgaccatcagccaaaaaatcctgccgattttaaacgatttgatcgtccatacgcctccgtcttccaggattatctatttgagaaaaccggcattcggttgaatcaacccaatgatgtcttaggatttggatacgcaaaagccaatgttgaagcaggcaggccgctttcgctggtaccaattaagcgaaagggcagccaacatgatgcgactcaaattgacgatgtcagtcctattgccagtgcgacagcgattcgccaagcggtcgttaaacatgacttgaaggctgctgatcgagtggttcccaaggggacaatggggatgcttgagcatgaccgaatgctcacctggcaagatttttggccgtttctcaggtttgaattggttgagagtccgattgaaaagcttcatcagatttatcagatgaccgagggaattgagtaccgtttaaaacgggccgcaatcaaggcagaaagcttcaccgagttcctacatttggtcaaaaccaagcgttatacgtatacaagaatccagcggctgtgtacctatgtcttgttacatgcagttccaagtgatatgcttcaggcggccggatatgtccggctgttgggctttaacgcggtaggtcaaagatacttgaatcaaatcaaaggagaccttgacgttccattgattaccaaaattactgacgacgttgttgccgacacaatccaaatggattttcggggcgggatgttaacccagatgattaatggcttgtctcaagattattatcgacatccaatcatcatggaataatccgtaaactcctatcaaggaaattgccttgacaagcctatttgttgccggtataataagttttgttgcattggaggaattatattgaaatggtactttagagacttgcaaaagtactcggatactgatcctttcacattcaacgagaaccttcaaatcaaagccgatttgcttgatcgatatgctgatgaagtgatcgatgcatccgactttcacgttgaagggactgcttttgccgatcgcggtgatgtgattattgactcccatattgttgggaagttggtcgtcccgtcatcccgttcattgacacccgttgacctaccgcttgattttacagttgaggagttctatgttccttccaaggctgctgaatcacggtatggaaaagatgacgttgtctttgttttagatgaagatgatatggttgatatgcaaagagcagttgttgataatgtgattttgcatattcctatgcacgtcctgtctcctgaagaacttgcaggcaaagagatgccaagtggtgacgattgggatgttatgtccgtcgatgactacagcaagcagaaggcagaattgaaaactgttgatccacgtctggccgaattgaaggacttttttaagaatcgagattcgaaatagctggacttaaaatttcactagtggatattttattttgacgaggagggaaaaagaatggctacaccagcacgtagaacttctaaagctagaaagcgcatgcgtcgcggtcacatcaagttgacgactcctaatttgagcctcgacccaaagaccggtgaatacaccatgccacatcacgtatcaccatcaggcttttacaaaggccgtaaagttatcaaagataacaagtaattaataaccaatttagaacgccatggattctaaattggtttttatatacataaaaatagggccgccagcgagatgcgtttcgctggtggcccttaattcatttggatcaatattatatttatttagtaaaatcaacaaccattcggccaacaatcttattggctttcatttcatcgataatgtcattgacctcatcaagtcgacgagtttgtacgattggctttactttgccttcagcgccgaattggaatgtttcagcgaggtcctgtctggtaccaaccagtgaaccggcaacttgaatgccatcgagaaccgtcttatcgatgttaagtgccatatcacccttaggaagggcaacagcaaccaacttgccatctggacgcaaagcgttaacagatgtagtgaaggcctcagttgtaacggcagtaatttgagcattatgcacgccgccaaccttcttttgaatttgatcggcaacatctggatcatgacggttgatggtgatatctgcaccgttgtccttagctgcttgaagtttttgctcattaccatcaacggctaccacatgggcaccaaagacgttatgggcatattgaacagcgaggttacccaagccaccacaaccaacgacttcaacccattggccgggacgagtgtcgccaactttgagtgccttatacatcgtaacgccggcacaggttaatgaagtcgcttcaattggatcaagtccttctggtactttaacggcgtagtctgcagggacaatgacttgttcagccatagcaccatcaactgtgtagccagaattttgaacgttacggcagagtgtctcacggccagtgatacagtactcacagtgaccacagcctctgtagaaccaagcgattgaaacacggtcgccaatctttaagttagtgacatcgtcggcaacttgaatgacttttccgacgccttcgtgaccaatgattcggccgggaaccttaccaaagtcgccttcagcgacgtgtaaatctgtgtgacataatccacaatattcaacttgaactaaggcttcaccttggtgaatggggcgtaaagtaacatctttaatatcaacatatccatcaacgggatctcttacaacagcagctttcatagggttaatcatcctttttgtaatatattttcaaacaagttcattataaacgtccccttgggcattatcaagtgaatttctacacaaaattagtttaaatgaaaaatatttccaagcaattttagccgtttttctaagttttattaaagtaaaagactaaaactctcataattatggtaaaatgagagttatgttaaaaggtttctacgttactaataaacaaattaagatattttatgggagagctgatcatttatgagtcgaattttgattattgaagacgaaaagaatttagcacgtttcgtcgaactggagttaaagcacgaaggctacgatacccaagttgagctaaacggccgaactggtttgcaggctgcattggatgagaactttgatgtcattttgcttgatttgatgttgcctgaattgaacggaatggaagttgcccgccgattacgtgaaaagaagaacacaccgattatcatgatgaccgcgcgggactctgttattgaccgagtttcaggctttgatcatggtgctgatgattacattgtcaaaccctttgcgattgaggaactcttagctcgaatccgggccttgcttcgccgaattcaaatcgaaaatgatcaacaaaagaacaacaagaaatcagtcacattcaaggacttgaccattgaaaaggaaagtcgaattgttcgtcgtggcgatgaagtgattaacctcacaaagcgtgaatatgaattgttgctgactttgatggaaaacgttgacgttgtcctggcccgggatgttctgcttaccaaagtatgggggtacgattccgaagttgagaccaacgtggtcgatgtttacatcagatatctccgaaacaagattgatcgtccaggtgagaacagttacattcaaacggttagaggtacggggtacgtgatgcggtcatgaaccaacccaacacaaaaccaaagagaagaaagacatcgctaaaatggaagtgggcgttttttacgtccattggtgttttagcgattgttgttattttctcatgcttaatttttaatcgatttaccaacgtcttatttcaacaggaacgttcgcacattgacaataccttgagtaccgtttcttcaaggttgaccaattatgcctcaccattgaccaaaagcgatgtgggacactatttgaagccaaagatcaccgacagtaacgatcaggtaacacaagctgatggcaacgatttgtattccaattcgttgatcgttaatttttcccgcgataacattttagtcaatgtctacagtgtcaatggcaaggaattatttgaatcgcggaagagtacggccaagttttattctgccagcaagcggaaaatttttaccaccaggcataatggccaccaaattctggttggctcagaaccgctgctttcaaagaagaatggctcattgattgggtacgcacaagtcactgatcaattggacaattaccgagcgacggctaacaagctgctggttatcttaattattctggtgctgatttctgttcttttgacgatgatttttgcctatattctagctcaggaattattgcggccaattaatgatattcaaaaaacgattaatgaagttaagagcgatcccgactcagatgcacgggtaccggcctttcgatccaacgatgaattaaccgacttggctcagttgttgaacggcatgttggatcaaactcagcgctatattgaccagcaacagcaattcgtggaggatgtttcccatgaattacggacaccggttgccgtcattcagggtcatattgatatgctgctgcggtgggggaaagatgatcccgaagtcttggaagaatctttgaaagcttcactgcaggaaaccaatcgaatgaagagcctggtttctgaaatgttggatctttcgcgtgccgaacagattgaaattaattacggcgaagaaattaccgacgtcaatcaagtgtttgaacaagtttataatgatttcaaaatgattcatccagatttcacctttacgtttgatgatgacaccgatcatgacgtttacgttaagatttatcggaatcatcttgaacaagtattggtcattcttctggataatgccattaaatattcaaccaagcgaaaagaagtccacctgtcactgtctacatcgatggcgatggttaacattgctgtccaggactttggtgaggggatttctgaagaggataagcaaaaggtcttcaaccgcttctatcgggtcgataaagcccgcagtcgtgacaaaggcggtaacggactgggactttcaattgcccacaggctgatcgaagcttaccatggtaacatttcgattgaaagttcacttggttccgggtcgattttccaaatcaatctgccaatcttgcagcatctgccaagcgaagaagaaatggagaaaaagacttcatcaacctccaaagaacaatcggaagattcaggactcccagaaggaatcttggatacttccaaacatgatgatcgtccattaaatgacgatgaacatcatgaaaaataagtttaaaaaggcgtcacatccgttgcaaactgcaatgaatgtgacgtctttttaatgggtaagagtcattgtgactaattaagttttccaagttccctacgaacttctggtgcctcggctttgctgctggtaaaaataatccgatcatttagttttaacgatgtgccgccggttggccggataaaccgtttgtcacggtaaatttgggtaatggtaactttgtcgataaatggaatgttgcggacctgaatgtcagcatacagccggtttctcagggcaacttcgtagacactggaatctgtggacgtcattaagcgcattgttgacggcgcttcgatcaacgctcttaacatgctgatattaacatccggggtattataaagctccactcccagtcgatccaactcgtctctgcgatcgtctaaaatattgcggtcttcgaatcggacgatcacccggcggacaccatattgcttggcaattttcgccaattcataattcttttcggaattaatctgaccaaacaccacgacatcagcatcaaaaacaccgtttttaatcatgacttccggttccaaactgtccagcagatggatggtcgtttcactgttgaaggcccgataattgtgctggttgttggtatacatggtcacatcataccagcccttggctaattgttgcgccacagggacagtcgtcaaattggtgccgataaagtgcacgctcgtctttttgagatcctcggcttctgatgaatacagcttattaaaaatcagtggaccaaagacacaggtgatgacggctgacagcaagaatgcacctgactgttggctggtaattctgtgtaagtggttggcaacctgcagcactgccaaaacaacggtaatggtggtggcagtcatcgcagttcctgcaactgcgtttaggttcttgaaacgcaattttaaggcactgaataccaagctctttgccaaaacgtagccgacaaaaatcacgggaatcaacaccagcgtttgtggattcgtaattaattcttttaagttcaaattaacgccactcatgatgaagaaaattgggatgaagaagccatacccaattgagtccaaacgaactttggtttcttcatgcggttcaagtaatttgatgacgattccggcaagaaatgcaccaaggattccctcagcgccaaccgattcagcgacggttaccagggccacgatgataaaaaatgaaagccgaatatccagctgggtggtcgacttgttgatccgatcaaagaagcggaaaaaggctttgaaccgccagaacaagagcgcagctgcaaccagaatcaacaagatcagccataaggatttggaatggggactgtaggctgaagcgtaaaaagtcaacccaaccatcgggacaacttctcccagggcggcgattaagaggattgcctggccgaacggcttgctaagcagctccttttcttttaacccggcaatgacaatgccgagtgaaatcgtcatgaacagaatcgcggccagccaaatatcggtgaacaagccgctgagttgaagcagataagcgatcacaaacgacatgccgacaattgaggcgtaagcgattgtagccacttgtaatactgagtacttcggctgatcatgctggcttttcttctcgagcggtgaaagagtggtgggcttctttttaaagaggctgaaatcaatctccatcccgcttaagaacaacaggaagatgaccccgacattttggagaatctccaaggtttccgagttggtgatccagttgaacagtgacggtcccagcaggataccaacaataatttcaacaaccgctgttggtagaaaagtgattttaaaacgggccattgccaatgggatgacaagggccgccaggagaatgatcaatagcgaaatttgattcataaacgaaaacaactcttttcctgaaaaatatacatgaatatcctaccattcttatcctgagtttgggtgtcatatcactcaaaatcttgcagaaataaaaaaatcacaccaaaagatgtgattgagtgtgattatttatgatgtcgttgttgtttaccagcgtttcgaggacgcttagccgctggtttttcagcttgcttatccaccgtcgttttggttggctgagcagctggacgagcctgaggctgatgcccggattgctgcttgccggtatttcgttgacgatttctttggtgaatatcggaaccggtcgattttgtcccactggcagtcggcgttggatctggcatcagatcctcaaccgtcacagcttttttgccttcattttctttggcgatccgctttcgaattcttggtcgatacatattgatgatcaacgtctgcaaacatgcgaataggccgccaatgaagaagtaaattcccagaccggctggggcactcagcgtgaacaccaagatcatgattggactgagcagcatcatggcgcccatttgcttcttttgcgctgcaggggtgcccagcatggcaatgtagccctgtaatagataggaagcaaatgacaaaacggctaacagccaactcgattggccgagtcgaatgcccatgaaaactgtatgagacagctctggcgagtaacggattgcggcgtacaaagcagtaaagatcggcatctgaatcaataatggtaagcaaccgatcccaccggtcatcgaaatgccgttttgtttgtacaatgccatcattgcttggctggcagctgtctgttcttcaggggtactggctgctttttgacgcttctgtaattcagccatttgtggtctaatcaactgcattttttcctgttgaatagttgaagccttcatctggcgaaccatgattggcaagaggaataggcgaacaaccacggtcaggacgatgatggcccagccgtaactaccgacaaattgggcaatccattccataattgcctgagcagggcgggccagataatcatagacggctccgtaaggcttaccggacttggttgttcggacacagccactcaaaagaagggccatgccggaaagcaatcccagcgtggtgaggtgtttaaattttttcatgagtaagacctttcttaagttagtacgtaaacaaaacaatcttactagattattgcctgcttttcaatttaatatttcacattaaaccctttatttacccttttcgcgatataattgacttggagacttttgactttggcaaatggggtgggtgaattcttgattttttggataaattgcgccagattttcactttcgccgcttgcaagaattgaaacgctgccgtcgatttcatttttgacccagccggaaatgttgaggctttctgccagctggatggttgaccatctaaagccaacgccttggactcggccggaagcgttcattttgactgtttgaattttgtcgttcaaatgatcaccacctacaattaataatgaaagagagatattttatggatattgaaagaattacatcgaatcagaataaccgggtaaaagaatggaccaagatgcagtccaagaagggacgggttaagtccggcgaatacgttattgaaggctggcacattgttgatgaagcaattcgccatcgccagaccatcaaacaactgatggttgtcgacgagagctatttgggcgatctgccggttgacgatgataccgaaattttcttaatcacgccagaaattgccaaacatatctcgtccacagagacgccccagggtgtgtttgccgtgctcaataccgaggactaccatgaacagattcccgatgacttaaagggtgcctggctgttattggataacattcaagacccgggcaatattggcaccatggtccgaacagcggatgcggcgggattaaacggcattgtctttggcaagggatcggctgatctttataacccgaaagttgtccggtcaatgcagggcagccaatttcacatgaagctgtttaccggagatatcttggaatggatggcagcctttaaagaagctggcgttaagacttatggcaccgaattaaatgatcaggccatttcctactatgatataacacctaccaagcaatttgcactgattatgggaaatgaaggcaatggggttgacccaaagattttggagaagaccgatcaaaacctttacattccgatgaatggtgaggcggaatcgctaaatgttgccgtagcgaccggcatattacttttcaagtttgttaaataacggtcgttttcattgatatttggggcgataccatgtatcatgtttgtaaataaagacaaaggggtattacatgcaaaaggatgaatggaaaaacgattccgagtatcgtgaaatagtttctgacctgatggcgactgacatggttaagaaattggctaactatactcagcaccatcactcaactcgacttgaacattcaattgctgtttcttttgacagttataagattgccaaaagaaggggcttagattatcgtgccgttgcgcgtgctggtctgcttcatgatctgtttttctacgactggagaaccaccaagtttgatttgggttctcacgcatttattcacccacgggttgccctgcggaatgccgaacggatcaccaagttatccccaatggaaaaagatattattcttaagcacatgtggggattaactttggcacggcccaagtacgaagaaagtgtcatcgtctccttggtcgatgactacgaagctgttcacgaattcgtgagtccacttaaatcaaagttcgaaacgttaaagaagcaagttaagcgaacaactgctgttaaataacggttgtccgatgagaggggggaatttatatgcgacaagtagttggtctgcaagatgccattaattattatttgtgtcctaagttcgagaagacattttcattccttggtaaaaaatggaatggcttaatcattgacgtcctccttcaggaaggtgttttgagattcagggagattgcccgacaaatccccaagtgcagcgatcgtgtgctggtagagcgcctgcgcgaactggaagacgatggtgtcgttgtcagaaccgaacacgatgattcatctttaatcgagtattcattgactgaacaaggcaaagaattagctccaatcatgcatgaaattcatacatggtcagaaaaatggtatccaagcgttgaaaagtagcttgaccatttttttgttttagcttattattcactaatgtaaagcgtttgagaaaaaagtagtaggttgataacctatctgagagacttcgtggttggtgaaaacgaagtaggaaatcttcacgaattcatttttcgagctgaaattgggcgttatttaacaaaaaatttccggttaatcaccgttagcgatgtcttaagtgtgttgtcttttgacagcaaattagggtggtaccgcgttgcttcgtcccttatcgggcggagtttttttgtgtttaaaatttgaactggagggatactatgtcactgcgagatcaattgacagagatcaaagaaaaagggcttgctgatattcagcagaccaatgatttaaaagcattaaatgaaattcgagtgcatttgctcgggaaaaaaggcccgattaccgctgcattgcggggaatcaaagaattaacccctgaagaacggccggaagtcggcagttatgccaataagattcgggatgccatcaccgaagccgtttctgatcatcgtgaaaaattggaagatgctgccctcaatgcgcaactggcagctgaaaagattgatgtgacgatgccgggaaagccggttgctcaaggccaaccgcacgtgattcaacagatcattgaccaaattgtcgatttgtttttggggatgggctatgaagtcctttccggtccagaagttgaagaagataagtacaactttgaaatgatgaatctaccgaagaatcatccagcccgggatatgcaggatacattctacataagtaaggaaatcctaatgcgaacccaaacttcaccaatgcaagcacgggcactggagaaacatgatttttcaaagggaccgctgaagatgatctcacctggaatcgtttaccgtcgggatactgatgatccaacgcattctcatcaattccaccaagttgaagggctgtttatcgatgaacacgtcactatggccgatttgaaaggtactttgatcacgatggcccaaaatatttttggtgataaattcgatattcgtcttcgtccaagttatttcccatttacggaaccgtctgtggaggttgacgtcacttgctttaactgcatgggtaagggttgtgatgtctgcaaacacactggttggattgaggttttaggtgccggaatggttcatccaaatgttttggacatggctggtgtcgactccaagaagtacggtggttttgccttcggagtcggtccggatcgtttcgcaatgcttaaatatggtgttgacgatatccgtgatttctatttggatgacgttcgcttcttaaatcaattcagtaagaggggtaattagagaatgaaagtttcatataaatggctcaaacaatatttagatctgaatatgcccgctaaagatctggctgaaaagatcgaacgaacagcggttgaggtggattctgtcaccgttgccgaagacggcctgaaaaagctcgttgtcggccacattttatcaatgaccaaacatccggaatcggaccacctccacgtttgccaagtggatgtcggagaagacgaacccttacaaattgtgtgtggggccccaaatgttgacgttgaccaaaaagttatcgtggcgctgcccaactcacgaattggcggcaacgttaaaatcaagcgttccaagatgcgcggaattgaatcatccggcatgatctgtgctttggatgaaattggcttcagcaaagacgtcatccctaaggaatgggcagacggtatttacgtttttgatgacgatgtgcctgttggtgaaccaatttacaagtacttgggaatggatgatcccattattgaccttgatgtcactcccaatcgtggtgatatgttaagcattttgggcactgttcacgacctggctgcaatctataaccagcaaccagaaattaaaaaaccagtggttgatgaagacagttcattggatgccaatcaagaaattcaggcaaaagctgacgatcaacttgccaaaacctacaagctgcgggttgttgaaggagtcaaaattgcgccgagtccttcttggctgcagattgttctttggaacgccggcatccgaccgatcaacaatgtcgtcgacgttaccaactatattttgctcaagtacggtcagccactgcattcatttgataaagataaaattaacggtaacgtcaatgttcgcctggcgcaaaagggtgaaaaattaaccacgcttgatgaggatgaacacgagctttccgcagacgatattgtgattgccgatgacgacaaaccgattgccttagctggtgtcatggggggcttcaacacccaaatcgatgacaataccagcaacgtggtgattgaatccgcgatttttgattccttcaagattcgtaagactgcccaacggcataatttgcactctgaggcctcccaacgcttcgaacggggaattaatccagacggtgtccaagatgctgttgacgaagctgtcagcatgattaagcagcttgctggaggcaagatcgccaaaggcacggtgactgccagtgaatatcatcctaaactgccaacgatttatattaccgctgaacgaaccaatcatgttcttggaacttcattaaccaccgcagaaattaaaagtatttttgatcggcttggcttttcaagcgaagcccacgatgacggtttaaatgtgaccatcccggcccgtcgctgggatattttccgcgatgctgacttgtatgaagaagttgccagaatttacggttatgataatctcccggcaacgctgccgaccggacgacaaagtattggtgttttgacgccgattcaaaaactgcagcgcgcttccagaactgccttggaaggcttgggcctgactcaggcgatctcttattctttgactactgctgaaaaagcaaaaatgtttttgatgcgtgatagtcaagaaacgaagctgctgtggccaatgacccaggatcatgcggtgctgagaatgaacatgttgtcaggattacttgatgatgttgcctataaccatgcccacaaagttgacgatgtggccctttacgagtctggacgggtcttttacaaacatagtgcggaccaaattcggcctgaagaagttgaacacattgccggagttgtcacgggcaatttcactgatccgctgtggaataaccatgtcaagccggtcgactttttccagttaaaaggcattgttaaccagttcttggttaatttgggcgtcaaaggtgacattgagtacactgccactgatcaatatcctgaaatgcatccgggaaggacagccaacatttcgatccacggccattacgtcggtttcctgggccaaatccatccacgaattgccaagcagttcaaaatcaaggaaacttatggatttgaactcaatatgcaggagttgattgatttgccaaaagatgacaaccagtaccaagctatctccaaatatccatcaatcaaacgggatatttcattagttgtggatcaggatgttaccaacagtcaaattttggcggttatgaataaacgtggtggtgccttcttgaacgatgtgcgtttattcgatgtctatgaaggtgacaatgttcccgacggcaagaaatcgatggcttactccctgacttatgtggatccccgcgaaaccctgaaggacgaagtggtcaacaccgcctttgaaaagattaaaaaacggttaacagctgatttaaatgcagaaatcaggtaatttggaaactataattaaattgaacagataggaggagcttctcatgaccgatgactcaagtcgacgaaaccccaaacccaataaaagcctcgggcgaagaattattatttctgtcattaccttactggttattttagctgcaacaatcgggctgatgggctaccggtattttcaagatgccttaaagccactgaacccacagaacactaacgtcactcaggttcacattccgcttggcgcttcgaacaagcaaattggttcgatcctgcaaaataaaaaaattgttaaaagtggcatggtctttgattattatgtcaaatccaataacatggccaactttagggctggatattatcaattgaaaccctcgatgagcctcaaaacaattgccaaacggcttcaacgcggcgggactgatcaaccgatccaaagcaccaaggggaaagttttgattcgagaaggcgccaacattgaccaaattgcgacccagatttcagtgacaactgacttcgatcgtggagatttcttgaaattaatgaagaatcagacataccttgaacaactggccagtcgttatccgaagctgcttaatccggcgatgaaagccaaaaacgttcgataccgacttgaaggctatttgtatcctgcaacttatgaagtggaaaagaatacatcgttgaagtcactggttaaccaaatggttgccaagaccaatcagatggtttcgccgcactttgctgccattaaaaaatccgggatgaacatgcagcagttcatgaccttgtcgtcattgattgaacgggagggtgtcaaccagaccgatcgacggaagatggctggagtattgttgaatcggatcgatatcaacatgccattacaatcagacgtcgcggttttgtatgccattcaccggaataacaaagtgttgacgaacaaggatctgcagagtgattcgccatacaatctttataagtataccggatttggtccgggaccatttgacagcccaagcattagttcaatgagcgctgtcctgcatcctttggatcgttcaaagaactatctgtacttcgttgccaataccaaaacgaaaaaagtatattactcaaagacgtatgctgaacatcagcagcaaattgcagcgcatacttccgataacaactaattgagagggcatctatttacatggtaaatcacaaaacacggccagtcgttattggcattaccggaggatccggtagtggcaagaccacggttgcacgcaagatttttgaccaattatccaattattcgatcacgatcattcaacaggattcatattataatgaccaagctgacatgaagatggccgatcgcaaaaaggtgaattatgatcacccgatggcatttgattttgatctgttgattaagcagcttaagcaactgctgcaatatgaaccgattgaaaaaccggtctatgactatggtcaatttacccgcagtcagcagaccattcatcaagaaccgcgcgaagttatcatcttggaaggaattttaatccttgacgataagcgattacgtgatttaatggatattaaagtatttgttgacacagatgatgacattcggttaattcggcgaattgaacgggatacaaaagaacgtggtcgttcactggataacattattcatcagtatttgatgactgttaagccaatgtatcaccagtttgtcgagccaaccaaacgttacgcagatttgatcgtccccgaaggtggggagaaccaagtcgcgattgatttgctgacgaccaaaatgcgttccattttgatgcggcgtggcaacaaagaaattaagaataaccttgattcaacaatataaagataaaaaggggaaattaccaaatggctgaagacacatatccaatgactgccgatggtcgcgataaactcaaggcagaattagaagacttgaaagtaaaccaacgaccaaaagtggttgaacgtatcaaaattgcaagaagttatggggacttatctgagaactcagagtatgagtctgctaaagatgaacaaagtatgcttgaaagtcgaattacaacgattgagcacatgcttcaatatgcccaaatcattgattcaaatgatagtgacaaggatgaggtaacggttggcaagaaagtgaccttccaagaattgcctgatgaagatcccgaaacgtatcaaattgtcggggcggccgaagctgatccaatgtcaggtaaaatttccaatgattcaccaattgccaaggggctcattggtcaccgtctcaatgaagaagttaatattcccattccggccggaaccatgaaagttaaaatcactaaggttgaatagagctacttgcatattacaaataacctagtatgtgaaaagagctaactgtgagcatctttgctcaacggttagttcttttttgataagttaaattaagcccgcaatcgtcacgttttgaaaggtgaacagccccttgatgaacaatgttagcgtctaatcggcttgcatatcgtttgtgaaataccttaatgatgttataatcgattgtaagcgaatacaaacacagattttaggagtgtggcataataatgaaaattgatgtaactgattccgcaagcaaatggttccaatctgaaatggggttaagccaaggcaatggtgtgcgcttctatggaaaggtttatgggaaaactcccgtccatgaaggcttctcgttagcgttaacccgcgatgatcatccaggtgagacttataccaaaactgaaaaggacggaattacttatttcgttgacgaagatgaccgctggttctttgtcggctttgatttgaaagtcgattttaatccagaaaaagatcctgaaaatgttgtgtacacatacacacctaatggggatcttgataaataaacgtaaccaatcaaaaagggatggaagccaaaatggttttcatccctttaatcatgcaatttatttggtatttgttggtgtctcagtgtgcttggctttttgtttcttacgatgtttcaacgttgcctcggtgccgataaatgctaagccaaaagcagtgattagtaggccgactctcagcccttcaggccagtaagtaaagacaaccttatggtgacccttgttgattgggatatacaggaacatctttgcccagcgttttggtttaactgatttaccatcaaccttagcagtccagccattctcaaatggaatggtcgtggttaatgcttgattgttggacttgacgtccactgttccggttaactgatggtggttccacttcgtaactttatacggcttggcgtttaagtccttagagaactgagcaatctttgaattatgaactttgtacaatttcacgtcttgtaagagggcgttattcttgttgacaaagatttgaacatttgcagtggtattgatgctggtacctgtggcaatgttagcaatgatggttttttcagatggtgtaaattgagtctgcgcttgaccatcaaccgaaattgaaatgttgcctttattgatttcggttcccaacgtcatgtagtaagacgtgttcttctcaattgggacagagaaaatgatgtaggacatttccaagaggttctttttcttcaagacagcattatctaattgagaaatcggttgaatgttgttataccgcatgtcagtgtaagttgctggttcaaacaagttcttgatgtttggatccagacgatgggcaatttggttttggtaagtaatcggactcttggcaattgaattatgttccattccggatttaggcgccaggaaaccaatcgggaccgcatacggattccggtaggtaccaatcaaggcgtcctgtgacaacaaggtgtaattgttataatcaggctttcttgtcaaagtagtcaacagctgcttctttggttttttgttcggattagcttccggaatttggtgactcatgtaatacttcatgttcaacaatgaatcagtaaacatggttccgtttgagtaaaggacaaatgaatccccatttggctgaccgatatttttgaagaactgagacgtatcggattctagggttgacgagaagattgagccgccattgtaattaccagtgaaggcatcgttcttggtccgcgagaaagtggttcccaatcgatagaatcccttatctttttgcttaattttattgacatgtttgcgcatcacccgctcaaactgggtgtaattgctggccttcaaataatcaagatgattcagtgaggtgaccatgttaagggccatttcaccactcatcagcacggccaaggtcatcgccagaacaatgtttctgcgataaatgcctaagaagacaacgatcccaagggaaacgaccaaataaacacagccccagagaaagtcgaagtggcgcatgtattcgagatgcttccagcggagttcgacgtaaagaacgcccaaagccatgataccggcagtgaccagataacctttccagttgatgccttcatccaagatatgcagaaaggcttgaaaggcggtcagaatcatccaaaacgagaagaggtaggagaaacggaaagtgtaccaaaccggcagctgcataccgtgccagaacagatccagtggttggaaacacattgatagaatcataaatgctgtcaacgaaatattggcaattttgacgtttcgtttgatggttggaataaagaagtagtaaacaaataggatcaaaacgacactggcgacaaagacgttggctgttccggcaggcagttcattgaaattaactgatccattaaagaacttgcccaacatgtccagtgggttatattcaaacttgattttgtattggccctttgaatattgggttttgcttcccagaagcgagaaaaaggtcggcagcagcagccaggcagctaaaataccgctcagaattgacgccttaagccatttgagaacggttttggtcgatgtttggttttccaccggcaatgccttggcagcccagtaaatgaacatgaagagggttaaaaagatggcgatcatgtaactcatgtagtaattcataatcaacatggccgttaaactgatgatgtagatggcactcgactgatttttcaagatcttgaagagcccatagaaaatcattggcaaaacgaacaacacgtctgtccaaagcatgttgaattggttggcaaccatccagcccatcatcgcatacgaagcagagaaaccaatgattgaccagccaacgtgtttggtaactttcatcaagaaatagccaaaacttaaaccagccagaccatacttgataatcgtgatgatgcccaagacactgggtaatttagaaagtgggaaaagcaacataatcaagttcagtgggctcattaagtagtaagcccaagttcccatcatgtcgcctccaagagcctttgaaaatgaaaagaaaaagccgcttggactatgtaggagggtgtcatggaaattggtataaaagtcaatatactgttgacccaagtcaacggtcataactgacgagccgccaaacggagcaaagtggcggaaaataaagtaactggtggaaattagcaccggtaccaaaaagcacagcactaatatggaaattttcgttgtcttctttgaattcataatctacatcctttttaaaagtgattaacaacatatagaatatcataataagttaaagattgactaccggttgtagtttttagttggaaaatttgatagaataagtttcatggcaaggagttaatatcgtgaaaatttttaaaaagcgcaccaagaaaacgaacaaagcaaaggctgtttcactgccttttcgaatcaacattatttttattatcgtcggaattttatttgttgcattactgacccagttggcgtatttacaggtgatgtacggttctaaatttaaagccgaagtgaaccgatcagacacctcagtagttaacgggaatgttcagcggggaatgatttttgattcaaccggacacgttttagtcggcaattccgcgcaccaagcaattatttataccaagggcgtgaatgtgttgtcctcggacatgtacaaaaccgccaaccgattagcccaatatgtgactgttccaaccggcagtttaaccaagcgccagctggctgattattatttggcaaatacagataatctagccaaagtcgaaaagtcgatccctgggatttccggttattctgaggatgccaaatacgacaaggctgtcaataaggttgagagttatccaaatgccactttttcatcagcactcaaaaatgctgcaaccatatttgccaagatgagtggtgcctaccaattatccaccgttaatattaaggatgacaacgtttctactaaagaagttgccatggtgggggaacatctggccgatatgccaggggttaatgttggaaccagttggagtcgcaactatccaaatggccgttcaattcagggaatcaccggaactgtctcgaatgaaaagagtggtctgccaagtgatcgggtcaatgaattattggcacaaggttactcacgaaacgacagtgtcggtcaaagttatctggagcgccaatatgaaccggttcttcggggaaccaaatcccagacccaaatcattttgaatagcgataatcagatcaaaaaggaaattaagaaatatggcggtcaaaaaggtgacaaccttcaattgacaatcaatgccaaattccaaaagcagctccaatccttagtccgttctgccgagtccggtgccggtggtaattcaaccggaacttatgcggtcgtcatgaatccgaataacggggccatcatcggaatggcaggggttgaccgcaatccgaagacttccaagatcactgataatattttaggaaccattaacagctcaattgttatgggttctgttgtcaagggtgccatggtttccggtgcattgatggatcatgtcattacaccaacgaacagtaccttaaccgatcagccaattacgaccggtggtgttaaaaagtcgtcttggttcaaccacaacggtcatgcaaatattgccgttgatgccagtgatgcgctgcaagtttcttccaactcttatatgatgcagttagcgatgaaagaaggtcacttcaactatgttgaaggtggcgcattaaccatgagtcccaacgtcttcaacacgatgcgcggttacttcaaccaatttggcctgggtgtcaagactgggattgatatccctggtgaatctaccgggttacagggtgccagcggctataagcacattggaagtgccttggatctttcatttggtaactacgatgcctacacaacgatgcaggttgctcagtacatgtctaccattgccaacggtggtaatcgaattgaaccgcatgtcgttcaagcaattcgcggcaccagcccagatggtaaattaggaacggttaaagcgacagtgatgccaaaggtactcaatcatattgatatgactcaagcgcaacgaaacgtggtcacaaccggcttgtatcgggtggttcatggaaccaacacctacaagaccggtgggatgttggattccatcaaaccggaaatttctgccaaaactggaactgctcagacattttataatggcaacgaaacagttaccctgagtttagcttcatatgcgccatcgactcatccacaggtggtggttgctttggcaatgcctaacttgggggttaacgctgaaagtaataacatggcgctggccaaacaaatctactcggcttattggaagacggtccaatcaacttcgactgttaagtaaaaacacttaacatttatcgattttgtcctagtaatttatcaggattgatgataaaatattttaagttgaggctattagactagctactctataaaagtttggaggtcgtattccatgcgagtacacattacaatggaatgtactgaatgccacgaacgtacttacttgtccagcaagaaccgtcgaaacaatcccgaccgtttggagcttaaaaagtattgcccacgcgagcgtaaagttacattacatcgagaaaccaaataaggcttgggtaaatacccaaaccttttttatatacaacagagtctgtcaattagatttgactgaagaatcgggtgaggtaaatggccaaaagtaaccaattaaaagccgccctgcgagatcagcagatcgctcggcttcatgactttttacaagatccacaacaaaagccggaaattcaacgcttgtatcagcagttattcgccgagccacactttgcgaatagtgagacgctggggatcaccctcagtatggatgatgagcttgatacccagccaattattcactgggcgttaacccatgataaacaagtagcagttccccgaacacttccgcaccgccagatgacctttgtgctgctggaacctgatacggtactcagtgagaccaaatttggtacgattgagcccgttggcggtcaagtgctggcaaaaagccagctggatgttttactggtaccgggattggcgttttctaaaaatcactttcgagttgggtttggcggcggcttttacgatcgctttttgaagggctttaccggcacaagtatcgctttggtgacaccggttcaactatttgacgaacccgtctgggatgtggaagattttgatgttaaagtcgacaaactcatttactaaacggataacaggaggggttcatgagtaatttacgaaatcagccttatatcacatatggactattaatcatcatggtggtggtttttgcgatcatgtcagtaatgggcggaactgaaaaccccgtcaccttggtcgaatttggcgctaaatacaacccactcatccgtgctggcgagtattggcgattgatcacgccaatgtttattcacattggcttcactcatatcttaatgaacggcatcaccttatactttatcggtcagtacgttgagcaattgtttggacactggcgatttgcggttatcttctttgtttccggaatcatgggcaacctgggcagttttgcttttacagacagcttgtctgccggtgccagtactgcgatctttggactgtttggtgcttttatgatgctgggagaaagtttttccaaaaacccggcaattgtttcgatggccaaaacattcctgttgtttattgtcctaaatatcggaaccgatatttttgtttccggcattgatattgctgggcatctggggggactggttggtggattccttgtggcgtatgtgacgggcgtcggtttttccaagaccagccaaaccaaacgaattatttcggcaattatgctggttgtaatcgctttcgttttgtttacaataggtatgcgggcaaaattttaaattttgtgaaaatgaaagaaatttacatgaggatgtgagataatgaaaacgctgtatgatgttcagcagctgctgaaaaaattcgatatttatgtatatgtcggcaaacgactttgggacattgaagtcatggcgttggagttggaccatctccatgatgccaagctgatcagtcatgatgagtttattcatgccaaactgattttaacgcgggaacatcgaattgaagaaaaacaagaaagtaggggaaaatacattggctaagaaattaatcggaattgatttgggtggaacgacagttaaatttgcattcattgatacaaaaggaaacgtcctgacgaagtggcgaatcccaaccaacattagtgaacacggcagtcacattgtgcctgacatgatcaaatcaattagtgatcaaatgagaaaagacgactataacgcaagtgatttttatggtatcggcatgggaactcccggtgctgtgaaccgcgaaaagggaacagttgttggagcatataacttgaactgggacatcgtgcaaccggttggagcaaccatttcagccaatctcaatttaccaattctgatcgacaacgatgcgaatagcgccgctcttggtgaatattggaaaggtgccggcgacaaagcaaaagatgtcgtcttcattactttaggaactggcgttggcggtggtgttatcgccaatggcaagctggttcatggtattaacggtggtgccggagaagtcggtcatatcacggttgtccctaatggatatcaatgtacctgtggaaagcgcggctgtttggaacagtacgcttcagcaaccggggttgtccatattgctaaagatatggccaagaagtttaccggccattcacggattaaagaattgattgatggcgacgaagatttgtcatcgaagatggtcttcttcctagctgataacggtgatatcttggcgaaccaaattgttgatcgggtctgctcatacttgggattggcactttcacacattggtaacacgttgaacccggagaacatcattattggaggcggtgtttccaacgccggtaacaccttgcttcagccaacgactcgttatttccaagagaacgcctttccttctgttcgtgactcaacacggttgaagttggctcaactcggtaatgacgccggaattattggtgccgcatcattagccttgcaatttagaaataatcaaccatttggaaccaaataatcaaattatttgagagaaagagggatgtttttgttgataatcggtgcaatcaccgccaatctggtgacaaccatcattttgatcgttattttacttgcatggggtggctataccatttttcaaaatatgcgtgttaaacaggttgcaacgtatttgaaaaatgatgagtttcaaaaaggcatgagaaaagctcaggtcattgacttgcgagaacaaaaaagttttaaagacggccatgttttaggtgctcgcaacatgccttactcaaccatcaaaaacttttacagtcagcttcgtccagacttgccggtttatatgtatgatcaaggcaaaacgatcagcaaacgagccgcactctttttaagcaaaaagggttataaagatctttatatcttaaaaagtggttatcaaggttggaatggtaaggaaaaaaagagtaattattgataaaataggactatgaacaaagcattcgttttgttcatagtcctatttttataatcgttattagtgtaatggattggataatgttttatccgtggtgggcagctcggctcttacgcattgccttttttcggttatcctcgaatttttgctcttcatcttcgattggatccaccactgactttttaaatgtcagcaaagcaccaaccccagcagcaacggttccgagaacaccaacaatgagcccattagtaaactgtttcatatctaaaccctccaatactcgtttatactttcattatgctttattttttcatagatatctagttaattgattaattaatcgttcaaaaaggagtttattgtgaaaatcaataccaaaattattgcccatcgcggcagtaaaggaacccgaccggaaaatacactgatttcttttcaaaccgccattgacgatggggcagacggcctggaaaccgacgttcatttctcaaaagaccatcagttaattattatgcatgatgaaacagttgatcgaaccaccaacggttctggcagaattgttgacaaaaatctggctgagattaaacatttggacgcaggtgttcgattcagcagtgaatttaagggaaccacggtccccacgctccaagaggtggtggaattattaattaaagacaacttcacggggatttttaacttagagttgaagaccaacaagattcagtatccagggattgaaaaagcggtttttgactattttgcctcaatcgactacccgtttcagctgatttactccagctttaatgcccggtcacttgaaattctcaaccggctggatcctaaattagccggtgccaaattgttcaaaactgccgctaagcaggccaaaaccctcaagaaggaccatttaattgccgatttccatcccgacattcgttggcttaaacgacatccattttttgcccctgctcaaaatttgcgtccttggaccgtcaattccactgaggatatgcagtactgttttgaacgcaatctggccgctatcatcaccgactatcccgccagagctgttcagatcaggtcagagatgcgggagggagtggaatgatcaaacttttagcaatcgtcggaccgactgccgttgggaaaacggatttgtcgatcaaactcgctcaaaaatttaacgctgagattatttccggagattcaatgcaggtatatcgacacttggatattgggacagctaaaattacccaggaagaaatggcgggcgtcaaacaccacttaattgatgtcagaaatattgacgaacgtttttctgtcgccgatttcgttcatgatgcctcggaactgattgaagccattcacgaggccggcaagctgccgataatcgtcggtggaaccggtttttaccttcaggcacttttatctgggctggagcttggtggcgaccagtatcaaaatgatgacttgagaagacaattgctggctgaagccaaagaaaaaggggatttggcactgcaccaacgactcgccaaagtggatcctgctgcagcaagggccattccggttcacaacgtcaggcgggttgtccgggctttggaagtctacataaacaccggtcaccgattttctgatcagcataatgtcggatcaaaatacgatgccttcgtcattggattaacgacggatcgggcgttgttataccagcgaatcaatcagcgggtcgatcaaatgatggcgcagggactgctgtccgagggtcgctggttgttcgaccatgacggacagcaatttcaagccggcaaagggatcggctatcgtgaattattcccgtattttcagggccaatcgaccttggaagaagcaattgagctgatcaagaaggattcacgccattacgccaagcgccaattaacttggtttaggaacaaaactgaaccgcaaccaaattggtataacctggttcagcgaccaaatcagttaactgagattgaaagcgacgttgaaaaatggctggatgacaacaatcaataaattcatgttataaaatgtgacatttagtcttgactttgattatgggaatggtattatgggtacaagatttaggaggtgaacaatgcgagagaaggaattacggcgttcaatgtcagttctgccgattggaactgtgatgaagctaactgacttgacagcacgacaaatcagatattatgaacagcaggaattgattaagccgcttcgtaatgaaggcaatcgacggatgtattcattgaatgatgtcgatcggcttttggaaatcaaagattatcttgacgacggtctgaatatctctggtatcaaagaggtgtacaagaagcagaatcaattggaagacgagcggaagcgtaatctcgagaaaggtttgactgacagtgatgttagaaagattcttcaagacgagtttcttaacattggtggattgaagccgccttcttcgtcatttgatgatccgaataatttgaacaatttaaacaaactaaatcattgataggagcgatggatagatggccacaaagcatgattattcaaaagatgatattcgcaagatggtaaaagacgaggacgtcaagtttttacgtctgatgttcacagatttatttgggacaattaagaacgttgaagttccaatcactcagttggagaaactactcgataacaaattgatgtttgacggttcttcaatcgaaggctttgtccgaattgaagaaagtgatatgtatttgtatcctgatttatcaacttggatgattttcccatggagtactgatcgtggtaaaatcgctcgagtaatctgccaggtctaccgtccaaacggcgagccatacgcagccgatcctcgtaataacctgattcgtgttcttggcgacatgaagaaagccggctttacttcatttaacattggacctgaaccggaattcttcttgttcaagatggatgaaaatggggaaccaacccttcatctgaacgataagggaagttacttcgatatggccccaatggatttgggtgaaaattgccgtcgtgaaattgtcttgacccttgaagaaatgggctttgatgttgaagctgcccatcatgaagttgctcctggtcaacacgaaattgatttcaagtacgctgatgccttggctgctgctgacaatattcaaacattcaagttggttgttaagaccgttgcccgcaagtacggcttgtacgcaaccttcatgccaaaacctttgagtggtattaatggttcagggatgcatttgaatatgtcattattcaacgataaaggcaatactttctacgacaaggatggcgagttggaaatttctcaagaagcctattacttcttaggcggcctcttgaagcatgcccgttcctttactgctgtatgtaacccaatcgttaactcttacaaacgtttggttcccggttacgaagcccctgtctacgttgcctggtccggttcaaaccgttcgccgctcattcgaattccaagtgctcgtggtaattccactcgtttggaacttcgctcagttgatccaactgcaaacccatacttggcaatcgcttgtgtcttggaagccggcttggatggcctacgcaacaagatcgaacccgaacacagcattgatcgaaacatttatcgaatggatgctgaagaacgtcagaagagccatatcactaacctgcctgataccttgcataacgcattgaaggatctttcagctgatgaaacgatgaaaaaggccctcggcgaacatctctacagtagctttattgaagctaagaaccttgaatatgattcataccgcacgcaagtttccggttgggaacgtgaccagtatcttgaaaagtattagtgtgttaaaataactttgccgcacttgtaagagcgtgatcgattattcaaagagctcatggtggtgcacgatggtgtactgctgtgagccctttttataccgattatctctcattaaaatataatgtgtttataattgaatgtatttcagtctcatatagatcatgaaggggtgtctgttatgtcaaatattcaacttggcttaaaagtggggttagtgatctccgcagccttaattctcactggttgttcatcgcaaaagagcggttcggggaaactggcggccaaacaggaatttaccactgccgttgattcggaactctcaactgttgacctttccaaaacgacgtcggttcaaacatttgaagtgttaaacaacattgatgaaggcctttatcgtctgggtaaggacagcaaaattgaaaatgcactggccaccaaaactaaaatttcaaatgatgggttaaaatatactttcaatttgcgtaaaggcactaaatggagcaatggggatcccgttacggcaaaagatttcgtgtattcctggcgaagaactgttaatcccaaaacggcctctcagtacggttatcttttttcagggattcaaaatgctgatgccatccaagctaacaaaaagtcacccaatacactgggaatcaaagctgacggcaattataaactagtcgtaaccctggaaaagaaaattccgtacttcaaactgctgatgggcttcccgttgttcttcccgcagaaccaaaaggtcgttgagaagtttggcgacaattacgggacgaagagtgcggatatggtctacaatggaccgttcaagctaaccagctggaacggaaccgggatgacttggacgcttgccaagaatcaaaattattgggacaagaaagctgtcaaactggacaaactccactatcaagtgactaaggacccttcgaccggctataaccaatttaagaccgacaagctgcaatacgttggcttatctggtgttttggccaaaaatctgaagaacaataagaatttggtgaccagagaaacttcgagttgttactacctggcattcaaccaaaagaagaaactgttcaaaaatttaaaaattagagaagcaatttcgatggccatcgatcgcggccagttaaccaagaagattttaggagacggttcctttaattcacaaagttttgtttccaaaggactgtcaattaatcctaagaccggcaaagattttacagccaccactgccaaaccggattctttaacctataattcaaccaaggcaaaggcactttggaaagccggcctcaaagaactggggatcaccaaaatgagctttacactgctcagttctgacgaattcgcgcaaaaacaagtcagtgagtatctacagtcgcaactagaaaagaatctgcctgggctcaaggtgaacctaagaaatattcctttccaaacgttgctgtcacgacagaaatcacataattaccaagtcacgatgggtgattggtacgcagattttgccgatccgattaccttcttaaacatcctaacgtctggcaacccaagcaacgtcccacagtggtcgaacaagcagtatgacaagttgattaaggcatcttcaaccaccgatgctgggaacgctgacaagcgatttgaggacatgaccaaggcacaaaatatcttactggacaaccagggcattacaccgctatatcaatcagcaagtaaaaacctgttgagcagtaaggtgaaaggcattatttacaatacggccggagcaacgtacaactataaaaatgtctacattgtcaaataagttatcatgcagcgacacgggacggtttgacaactccatataggcaaatggaaaaagaaagtcaaactttcaactgaaaacaatcgaatacaggggcggccaggtcatcattaacccattatgatggtctggtcgtttttgtgatttcaccgaattttcaaaagaatggattgttttctcatcattttgacaaatctttcataaataaatgcgattagccctttatttatgtacgtttttcagataacattaaatgtataaataaggggaatacgaggcaatattatggataacaaaattgaaaacgatccattcagccaaaacgactcgattttagcttccgcgttaagcgaaaaggtaaaatatctgtcggatttgaatgactcgatcaaaaatggcaatgatttaaaagtatacgaattgatggatcccaaccgctttgcaacagaagtcaagggtgaacagcctgatcagccggagactaatttctttggcctggccactgatctgaaggctcagttaagtcatcatttgagtgacaaactcattgattatttaggaaccacctatccattcttctattaccacgaatatgatttggggaaattcaacatttactttggtaactggtgggaccatcggatgtttggggagttggatacaattaacgttcgattcaattttgctgaagatgaatataataccttggccaaatcatttgaacttgaagctcaaaacaaacgggtaaacgacgatcaaatgcgcgaactgggacaaaagaatgaaaaactgactcaattgattgaagatcaaaccaaacgcgatcagcgtaaggaagagattcgcaaacagatcaaggaaaatgaagagaagtcgccaatgccttgggaagctggcaaggttaaggaagagcatcagcaattacaaaacgctctgcttgagttaacgaatattgatgaacaagcttcaggcgcccggtccgaaatcaaaaagaatgaaaaccaaattttggcgctgtccaaagaagagaccatttacaatttggaaaaacaaaatattcgagcttcatttggcagttttgaagcatttattgagaacaataacaacttatacgccaaatacttgcaaagcttgagcaaagaatcgcaggtgactgacggtgagtaatgaaaatactgaaacagaaaagaatgttttaacgacgactgaacttttgaatcactatactcagtcaattcaagccggattggacaatgggtccaagtatgtcaatgcatttaccagcctaaatcagacccaggacctcgatgaattgttgactgcagctgtttcgttgaccaattatcaactcaattcagattttgtggaatttccacaccaattttctgatgaagatgttcagctggtattctttgaacggttattgaagttgtctgaccacgccgatggactttcaattagcaactctgaacacgttcaaaagctgctggctaaattttcatcacttggtgataatacctttacctttaccaaatcgaccaagaatgctgccggattcttctttggccccacggcccataaccgaccgctattctacttgaatctgaagagtaaggaaatgatgtttcatgggtcggccttaatcgattactttgtcgttgatttggagggcttggacgtttcggctcttaaagatgcgatgaacgtgattatgcgggctgctgaagtgctcaaagaaagcttcggctttaagattgactttaacgtcttggacggcgttaacggtgagttctatgaattcgctgccggcgcaattccagagccgattttggacgagctatttgttaagtcggctgataaccaatatattttgatgtctggtgaaaatggtggggcctccttgaccttggataacgatacccagctgaacgtttataacgccggtgatgaagatcggcccaagtggggagcaaccatccacgatcaggatcaaaaagaaagctggctgaatctattattggattacccgttcatcaaagactggtatttggataacaaaaagcagctcgaaattttatcgaacaagtttatttttggataggagtttgaaatggatttacaatcattgattgcttcatcggtgtatttgaatcgccagatcgaatcaaagaagcaacttcactggtcaaatgacggcagagtgaaaaatgcctttgtggccctggacgtggaactggctgaaatggccaacacttccgagtggttcaaggtctggaagacgcatcgtggtaagcacgatcccaacaaaacgccgcgggaaacgttgctatacgagtacgttgacgcaatggatttctacctattgatttccaacctcaaaaattggaatcacgtgattttaaactcgcaggatgatctggacaaaatcaaacagttcaaaaaagaagataacctggataagcaatatttagccttaaaacgcatgttgtttgacgcttactttgatcacagcggtgacagctttagccattcctggcgactgtttcttaaatttggcttggttgatttcggttatactgagcaggagattgaacaggccttcaaagataaaaacaagattaatgaagatcggcaggatcaggattattaattgaagataataagaaacggtcgaaacgaagagattcagcttcggttcggccgttttgataacactaagtaagcggactggtattttgacatttcctagagtgcggcgtaaatagtggtgtaaataaaaaataccttcaatcccgttaaaataggaattgaaggtattcagcaaacatctctaaatgtctgatgtgatgtcagaatgtcgcaagagagattcgaactctcgacctacggtttagaagaccgttgctctatccagctgagctattgcgacaaatcaacaataacaattatatgaaatattaacagggtagtcaatgtttaatcagtcttttagggcaaagatgtcaatatgattatgaattccttaagaaagttgcatttttattaaaatttgagttggttgaattcaaaaatttgaacgttcgctgacaaaactggataatgtagttgtgcagcaatctgctgtcacaacaattaggaggtggacgttgtgggatttgtaatctttattgtcttcattttcatcgttagtggcattattcagtattttaccaattcttcaaccaccacgcgagccaatggcagacatttagctcaacgtaaataaaacagccgtgggtagcggttgtttttttatgggatcaggtttctattgacgaacacctgccaattatgtatactagtaacgttgtaattgtggcttccacagctacaaccgctcgattcaagctgataagtcttcgatagtgatcggagcgcttgttctcggcgagtctaagcaaacttataaggaggtgcacaagatatgtacgcagttattactacaggcggtaagcaatacaaggtttccgaaggcgatgcaatctacgttgaaaaattagacgcagaagaaggcgcaaaggttacttttgatcaagttgttatggttggtggcgattcagttaaagttggtacaccattagttgatggcgcatcagtaactggaactgttgaaaaacagggtcgtcaaaagaagattatcatcttccgttacaaaccaaagaagggctcacgttcaaagaagggccatcgtcaaccatataccaaggttgttattgattcaatcaaggcataatttactttgaggtgactgatatgattaaggcgaccattaaacgttatcgcggtcatgtaagtgggttcaccatcaccggccatgccgatgcgggtgaatatgggcaagacattgtctgttctgctgtttctgtgttaagcatcacaacggttaacggtcttcaagaggttattggactggatgtcgatgtcgacagtgacgatgacaatggtggctatttatcagtcaatgtaccagttgttagcgattcaaagaagcgcattcaagctgatgcagttttgaatacttttgcgaacggaatggctgatatagccgaaagttatagtaagtatattaagttaaacacagcgaaataaatcaattaatctggaggtgtaaacctatgttagcaatgaatttacaattcttctctcaccataaaggtggtggatcaactgccaacggtcgtaactcagctggtcgtcgtttaggtacaaaggctgctgatggctcatcagttcacagtggatcaatcatctatcgtcaacgtggaactcatatttacccagggaacaatgttaagcgtggtaacgatgatacattgtttgcagtcgttgatggagttgttcgtttcgaaagaaaaggacgcgacaagcgtcaggtttcagtttatccagttgctgaagctgcaaagtaagcacaatagtttaattaaagaggctgggacaaaacgcgtgttttgcatcccggctttttaattgctcaggatcagaatgccattttcattggctattttgaccgaaagtattatataatctatttatgttacattacatttaggaggaacaacaatggcaatttcaactgctgattttaaaaatggtttaaccatcgaggtcgataacgcaatttggcggattttaagcttccaacacgttaagcctggtaagggtggcgcattcgtccgttcaaagctgaagaacttgcggaccggtgctgttcaagaaaaaactttccgttcaggcgctaagatggaacaggctcaaatcgatacgcgcaaaatgcaatatctgtatgctgatggtgatcaacatgtcttcatggatatggatacttacgatcaaatttcaattcctgctgaacaaattaaaagcgaactgaattatttacaagaaaacatggaagttcaagttattcaatacggcaacgaaaccttaggaattgaattacctaataccgttgttcttgaagtagcttccactgaacctggtatcaaaggtgatactgcttcgggtggttcaaaacccgcaactatgacgactggattaacattacaagttccattctttgttaaccagggtgacaagttgactatcaataccaccgatggaacttacatttcacgggcatagtagccgattgatctgaaacggaggctttataatggctgaagacacgaatatcattcttcattcaaatgatcccgaacttggcaaaattgagattgcacccaatgtcctggaaattattgctggggtagccgcatcgcaaattgacggcgttaaccggatgcgtggctcattttcaacgagtgtcaatgaattacttggaagaagaaaagaacacggtaagggcgttaatttgacatacacagatgaggaattaacgatcgacgtctatgtatacttgaactatggcgtttcagttccaaaagttgcattggaaattcaaagtcaagtcgaacagcagctgttgtttatgaccggcttgaaagtcaccgaagttaacgtgcatgttcaaggcgtgattccggaaaaaaccaccagtacggttgatccgaataatccgttcgctgacaatgaagaaaatggtgaggaatagtggaattaacacgacaccagatcagagaaattgcgtttcaaacactgtttgccttaaataccaacgatcaaactgattggaaggatttcttccaagttttgacgagcggtaaatatggcgacgactacccagaatacctgcaccaacttatttctggcgttttggaacacaagtctgaaatcgatcatacaattgaaaagtatttagcttccagttggtcacttgagcgaattgcccgaaccgatttaatcatcttggagattgctatctacgagatggtttatgtggatgacatgcctgccaaggtatcaatcaatgaagcaatcgaacttgcaaaaaaatttagtgacgaccgttcacgaaaatttgttaacgggattttgtcacatgccttagaagaactggtaaaatagatttacacatgtgtaaatctatttttttgtacatatgatttctcacgatgaaaatataaaggagcggtttctagatggcaacgattattgatggaaaagcattggcaaagaagttaaacgcacagacgagcgaacgggtaaaacaactccaaaaccaacacggaatcactcccgggttagttgtgatcattgtcggcacagatcctgccagccagcgatatgtcagaaataagcatcggacggccgttagattgggaatctattcaattgtcagggaattaccggataccattacccaagatgagttgctgaaagtggttcaggagtacaatcaggatcccaagattacagggattttagtgcaggacccactgccaaagcaaatcaatgaaaaacaaatcacccgttccattttgcctgaaaaagatgtcgatggttttcatccaattaacgttggaaaattatacttaaatgattcaaccaagtatccagttgcatgtacgcccaagggtgtgatgacaatgtttgatgaatatcacattgacttgaaggggaaaaacgcggtgatgatcggccgaagtgccattgtcggtaaaccaatggctgctttaatgttaaatgctggtgcttcggtttcaattctccatcttttaacaaaagatattactgaatatactaagaacgctgatgtgattgtttcagcaaccgggagtcttcataccgttactaaaaacgatgttaaaccgggagccgtcattattgatgtcggtcaaaatattaacgaagaagggcacctagtgggggacaccgactatgatgatttatttgacaaagtttcttacatcacacccgttcccggtggtgttggtccaatgacaattgcaactttgatgcagcaaactgttgatttagcagaatggagccttgaacgtggcgaatgattatttaaccgttagcgccttaacaaaatatattaaaagaaaatttgatgttgatccgtatttaactaaggtatacctcactggggaaatctccaactttcgattgcgccccaatgcccaccaatactttagcttgaaggatgatcacgcgaaaattagtgcgatcatgtttaaatcggctttcaaccggctaaaattcatccctgaagaaggcatgaaagttttagttgtgggccatatttcggtctatgaacccagtggaagttatcaaatctatgtggaacagatggaacctgacggcgttggtcagctataccaagcttacgaacagctcaaacaaaaactgtccaccgaagggttattcaatttgcccaagcagcagctggcaaaatttcccaaacgaattgcggtcgtcacttcgccaagcggcgcggttatccgtgatattattaccactgtccgccgtcgatatccgattgcccaaattgtcctgtttcctgccctggttcaaggaaccgaggccagtgcagacattgtccgacaaattgagcgggtcaatcaaattggtaattttgataccctcattgtcgggcgtggtggtggatcgatcgaagatttgtggccatttaatgaagaaaacgtcgccagagcgattgttgccagtaaaattccagtcatttcctcagttggtcatgaaaccgacaccacaattgctgatttagttgccgatgttcgggccgcgacaccaacggcagctgccgaactggcagttcccaggttggatcaagtgttagttgacctcaggacgacccaaaaccgcatcattaatgcgacttaccaggttgttcagcaagacaagcagcgattgaagcgactccggcagtccactgttttcacgacacctcaacggatttacgaaacttttgctcaacgtttggatctactgacgcagcgactctataatcaatctgacaagattaccggtaaacgaaaggatcgtttttctgatcttaaattgcgcctgcgtttggtcgcgccaacatatacgattagagaagagcagcaaaaactggcaacactcaaaggtcgactcaaccgggcaacaactcagaacctgaaaaatgtttcccaacattatcagatgttggtcggctcacttgaccacttgagcccgttgaagattctcagtcgaggttatacgtacaccacagacgaacagggacattttattaaacgggttgccgacttgagcagcaaaacaattgatgtccattttagtgacggtatcgtcaacgcttctgtcaatcagataaatgcaaagaaggagaaataatatgcctgataaacaagacaatcaaacctttgaggaaaaaatggaccaactggaaaccatcgtcaatcaattggaacagggaaacgtttccttggaagagtcgatggccaaatttaaagccggaattcaactgagtgaacagcttcaagacaccttaaccaaggccgaacacaccatggccaaaatgatggacaaagatggcaatgaagtggaatttgaagcacctaaagatgaaaaggatgatagcgatggcaaccaagctaactgattttgaacggttgtgggttccaaaaatcaatcagattttggaaaatgacatcaaaccggatacggatcagaccactctggaagcagcgatgagttattcagtcaacgctggagggaaacgcttacggccattgttgacgcttgcggtattggcgagtttgggcgacccaatcgatcagaccgtcttaaaaaccagctgtgcgctggaactgatgcattcttattctttaattcatgatgatttgccggctatggacaatgatgacctcagacggggaaagcctaccaatcacgtcaaatttggtgctgggatggcaactcttgctggtgatggcctccaaccactggcgtttcagtggctggtggataatgatttggacagtcaaacccaagctgaactgactttggcacttgccaaagctgccggcccccatgggatggtttcaggtcaggccgacgatatcgaatttgaaggcacccggttatcgttgtcagggcttcaaaaacttgaccgcaacaaaaccggtgccttgattcgctatgccgttgaagctggcctgattatgggccgggttattccggaaaaacgcaagtcactgttaacctttgctgagaagtttggtgaagcttaccaaatttacgatgacatcttagacgttgttgggacagaagcagaaatcggcaaaccggttcaccaggacgctaataaaaatacgtatcccaatttggttggtttggcaaaatcatatgaaatgctgaatcagacggtcgccgatgcccagcaagccctcgtaaccgccagagaagcgttatcaattgataccagtctgttaaatgatttcacaagctattttaaaaataaggacgaaaagtaatatggaaaagcaacgagtcgatgtactactagtaacccaagggctgttcgacaccagggaaaaggccaaacgtgccgtcatggcgggtgagattcttggtgataacgaagaacggttggacaaaccgggaaccaaaattccggtggataccgacctgcaccttaaaggcaagccaatgccgtacgtcagtcgtggcgggttaaaactcgaaaaagccctcaaagtatttcatctgaatgttaaagggctgaccgtgttggatattggctcctcaaccggcgggtttacggatgtgatgctgcaaaacggtgctaaattgagctatgcgctggatgttggcagtaatcaattggtctggaaactgcgggaggatccccgggttgtggtcatggaacacaccaatttcaggtacagtaagttggccgatttcacccatggacagcctgagtttgcctcaattgacgtttcattcatttctttagagttaatcctgccaccgctgaaacagatcatcactaaaaatggccatgtggtggctttgattaagcctcaatttgaagctggtaaggccaacgtcggcaagcatggtatcattaaggatcccgctgtgcataaaatggtcttggaaaagattttgaactttgctgtggccaacggttattcagttcaaaaccttgatttctcaccgatcaagggtggcgctggcaatattgaatttttagttgagttagaatctgatgatcaaccagtcatgtcaccaaatgtttcgattgaaaaagttatcgagaacgcttattctgaattaaagggttcgtaaacctgtatttttattcaattttattgttgggggtgtaatgatgcgtaagaaagaacgccaaaggctaatcaaacaattactgacaagtaataatattcaaagacaggaagattttgtctcgctactggataagcaggggataaaagtcactcaggccactgtttccagagacattaaagatatgcagctcgtcaaagtaccttcagttaccggtgggtatcgatacagtttgccgacgcaaaaaaatattgatactgaaaagaaactggttcaatcgattcgagattcgtttgtgtcggttgactctcaagacaagttggtctttatgaaagtcttacctggtagtggaccggtcatttctagtttgatgtaccagatgaactatagcgggattttcggcaccctcggcgatgacaacacggtcttgattatcggcaaaaccgaagccgatgcgattaatatgcgcaatcagatcaatagtatgttgggaactgaatagaattattgagaggttgaaaacatgttactcgaactatcaattaccgattttgcaatcattgaacacttagatattgattttcaggcaggaatgaccgtgttaaccggtgaaaccggggctggaaagtcgatcatcattgatgctgtcggcctcttggttggcggcaggggatcccatgatctcattcggaccggggcttccaaagccgttattcagggaaacttcatccttcatgatgataaccccacctacaacgtccttgatgaccttggaattgatcacagtgacggtaacgtgattatcgagcgggtcatttttgccaatggtcgcaacagctgtcgggtaaacggaatcatggtcaatattgccaccctcaaacgaatcggcgaaacgatcgtcgatattcagggtcaaaatgatcatcaggagttaatgcggccggaacggcacattcaattattagatgactatgccgaagatgaattggccgatgtgttgcaatcctatcaagaccaatacgatcaatttattaagctgcgcgatctaaatcaaaagaaacatcaaaatgagaagcagtgggcacaacgggttgatatgctcaaatttcaaattaaagaaatcgaagctgccgatctccatgagaatgaggacacagatttagtcgctgaaagagaccggttgaacaattttcaaaagattcatgatgccctcctagccagttatgaaggcattaacggcgacgaggaggccagcgggtcaattgattcaatcggatcggcaatgagttcgatgcaggacattgaagatttggatcctgaatataaacaaatttcggataatctatccggagctttcttcgcgcttcaagatgttgccagtcagatttccgatcaattgagtaatttagaatttgatcaggaccgtttggatcaagttgagcagcgcctcaacaccatctatcaactcaagcacaaatatggtgattcggtcagtcaaattttggactatcttgccaaaatcaaacaggaactgaaacaaatgtcgggggatgccgaagccagcgacgatttggataagcaattagccacgctcaaatccgatttaattcagcaggcaactaagatctccgacattcgccaccggtgggctaaaaagcttgaaaaagccgttcaccagcagttatccgacctttacatggataaaacggtctttgaggtcaatatccagcaaaatcgtgctttaaaccggctgggtgcagatcgagttgaattttatattcagaccaatcctggtgagaaaatgctgccattggtcaagtcagcttctggaggcgaattgtcccggattatgttggctttaaagaccatgtttgccaaggctgctggtgtcacatcaattattttcgatgaagtcgataccggcgtttctggacgggttgcccaggcgattggcaataagatttatacgatttcacaaaaatctcaagttttatgtattacccatttaccacaagtggctgcgatgagtgatcatcacgactttattgaaaaaaagattgctgacaatcggacaaccacgacgattacggaactgacaaccgcccaaagtgtcgctgaaatctcgcgaatgctttccggaacggcaattaccaagttaaccaaggaacatgccagtgagctgttgaaattggcggatgaggaaaaacaaaagattaaagcatcttaagtgctgtcgaaaaataaatgattagtttccgctatccacttggaaactgctgttggacgcactgtttacccagataaatcataaaaatgcaaaagggcttgagacaaaactgaatgttttgtctcaagccctaaaatataatctgatataatcttagtatttacgaatcgctttaatttctgacaacttcacaattcgagtgaaatgattatcatctgaagtcaataggtaacggtctgcggaaagtttggttaagtagccggtctgttcattatcctgatcgttaaattcgatcgtgatggggaagttgttttcgagtgtctgttgaatgaaataattcagctggaaagtcggcatttgtttgatttggtgagtgttacggacaatttcgaagaagcgatcatagttggttcgaaaggtcttggtaatttctgagagatatgattgtttgttttgcattttgttcaccccgaacatttgtttgtagtttcattatacgaacgttcgttctaaaacgcaacccccaaatgcaaatttcttaatcagtgccctaggacttgtcaaatggggcaaaaagggcgataatagcaggtattacaaataattgaagggattttttcgatggctaaaagaggaatgttgattgttttatcaggaccgtccggagttggtaagggaacggtgcgtaaggcgttgtttgaggagcctgatgttgattttgaatattcaacttcaatgacaaccagaaagccgcgtcccggtgaaaagaacggtgtcgattattattttgtttccaaagagcagttcgaagagaatattcagaatggtgaaatgctcgagtacgccaagtatgttgacaactactatgggacgccattaaaatatgttaacgagaccttggaatccggcaaggatgttttcttggaaattgaagtcaatggtgccatgcaggttcgcgccaatgttcctgatgcggtcttcgtctttttgactccgccagatctaatggaattaaaacaccgtctggttggtcgtggaactgacaagatggatgtcattaataagcgcatcaaaaaggccgtcggcgaaatcagcatgatgcgtaactatgattacgccgtcttaaacgaccaggttcctttggctgttgaccgaatcaagtcaattattagaagtgaacgattaaaagttgctcgggtgatgcccgattatgagtcaatgttaggagataaataattatgttactttacccatctgttgataaattgttagataaaattgattcccgttattcattaattgcgctttccagtaagcgggcccatgaattggatgccggtgccaagccattattggatcactacaaatcacaaaaatcagtcggcaaagctttggaagaaattgctgctggtgtattgaaaatcgatcctaaagcaaaagattttgaataagattgatcgttaagggactgcggcaaaacgactgttttgctggcagtccctttgtctttgttggacaagctgataccagccaatcctgttatcagcttatcttgtgatcccggccgaaactcggcgttagcaatccggggggatcattttggagttaatcgccttttccactggggtgcagccaacttttaagacgccgactgtttttatccgtcttagatttggtacaataaagaatgaaatctgaaacggggtggaaaaatgtttcaaaacaaaaacgttgccgtatttgtgacgggcagcattgccgtctacaaatcactgtcactggtacgcctattagtgaagaaccacaacgatgttcacgtcattatgagtgaagcagcccaaaaatttgtgacaccactggcatttcaaactgtcagtaagaatacggtcctgaccagcgattttgacagtaaagatccgacaatcattccccacgtcaagactgctgatgatgctgatttggcaattgttgccccggcatccgcgaatacgattgccaaattggcgaatggcattgcggataatattgtcacttccacattattaacgatggcagtgccggtatttgttgtgcctgccatgaatactcatatgctcgccaattttgccacccaacaaaatatcgccaacttaaaacaagccggtattcaaatcatggagccggctgaaggcttccttgccgagggctattctggaaagggccggatgccggaacccggcgaaattttaacgtgggttgatgaaagcttaaagctgaagggtggatccttagccggaaaatctgtcgtcgtcactgccggagggacccgtgaaccacttgacccggttcgctatttaaccaaccattcatctggaaaaatgggtttcgcagtggccaacgctttcaaaaatgccggtgccaatgtcacgttgatcgcggctaatccgttgattaccccgccatccggcgtcaatttcattcgagttgaaacggcggctgaattgttagcagaggtcaaacaagcctttgttcacgctgatattttggtaatggccgccgctgttgccgattatcgaccggccaaggtagccaataaaaaaatcaaaaaaacagctgacaatcaaaccatgaccttggaactggttaggaatcccgatatcttaaaagaaattgccactatcaaacaccctggccagttagtgatcggcttcgctgccgaaaccaatgatttaatcagcaacgccaccaaaaaaattcaatcaaagaatttggacatgattgtggctaacgatgtttcccaaagcgggattggctttaacgccgataacaaccaagtgacatttttatttgctgccggcaagcaaattaagacgaatgtcgagagtaaggcaaaggttgccgatcagttaatcaatattattgctacacaaatgcaaaatcagtgaaaggagaatctgccttgcaggttgctcaagttattgttgacgtcccagcacgccaaaccaacagtccgttcagctattcgattccagatcatttagcggatcaaattcaacctggcatgcgcgtccaggtcccttttggcaaccgcaaaattactgggtttgtggttggcctttccgacagttccagcttcaacggcaagctcaaaccgattgccgacctgattgatttatacccagtcgttaattctgagttacttaacttggctgagtggctggctgatcaaacctattcctttaaaatcagctgtttacaaaccatgctcccaggtggaatgcggactaagaaccaaaagaaactaattgccaaaaatgaacaagtttgccagcagtatccggaaatcttccaaggacagccagaagtcgaatatgaccgccagaaatataataatcaggttttagcagagattttaaatctgcagaaagccggcgatattcaagttgagtatgatctcaccaaccacgcccggccaattatgcgaaaagcttatcgaggccaattaaatgacgcccagattgctgacgccctcaaaaccgtacggaaaaatgctcgtggacaaattcaattgttaaacctgctcaagacccatcaaaacgatacactgctagtttccaaatgggcgtcccttggagtgaccagcgccactttgaaagctgccgaaaagaaggggtgggtgacttcaacattgaagcgccatgttcgcaacccatttctcagagatgtcgcccccagtcagccgtttaagttacagcctgatcaacaagcagcagtcgattcgattgaacaggcggtcgtccacaaaaaagatcaggtctttttattggaaggcgtcaccggttctggaaaaaccgaagtttacctgcagtcaattgcccacgcgctggagctggggcggacggcgttgatgctggtgcccgaaattaccttgacccctcaaattgttggccgcattcgcagccggtttggtgatcaagtggcgatgcttcatagtgcgatgtcttccggcgaacgctacgatgaatggcagcggattaaccaagggaaagccaaagtggtcgttggggttcgctcagccgtatttgccccgctcagcaatattggcttaatcattatggacgaggagcatgacagcagctacaaacaagccgacaacccccgctaccaaacccgagatgtcgccaaatggcgggctgcctacaataattgccccgtggtactgggaagtgccactccatcgctggaatcccgtgcacgggcaatgaagggtgtctatacactgttaaagctgccgcatcgcatcaatcagcatgctttaccgcatgtttcgattattgatatgaagactgaactggcaaaacaccacagtgcactatcgacaaaattggccgatgcgatccaggttcgcctcgacaaacatgagcaagtgattttattgctgaatcgccgcggttattctgcctttttgatgtgtcgggactgcgggtacgttcctcggtgccccaactgcgatatttcgctgacgatgcacaaaaatacacatactcttaattgtcattattgcggccacaaagaaccggtgccaactgtctgcccacaatgccacagtaaacggattcgcttttatggcatgggcagtgagcagcttgaagaacaggtcaaagacatgtttccaaccgccagagttctgcgaatggatgttgataccacccgtaaaaaggggtcccatgaggcgattattgatcaatttggcgctcacaaggcggatattttgctgggaacgcaaatgattgccaaaggattggattttcctgaggtcactttggtcggcgtcttaaacgcagattcagcgttgcagtttccagattttcgatcaagcgaacggacttttgaactccttacgcaggtctcaggccgctcggggagagccgacaaaaccggggaggtcatcatccagacctttaaccctgatcattatgcgattcaattggccaaaacgcaggattacgagaagttttacgccaccgaaatgcgtgtccgtcacgatggcaaatatccaccgtactactatacggttaagttaaccggcaattctcccagtgagaatcaaacggcttcagagatgtttgggattatgaactttttaaaaaaacagctatccccacaggcaatcattctcggcccaacgccaaaaacgattacccgaattgacaaccgttactattaccaaatcattatcaagtatcgaaaggaacctcagttaaaggccactttagacgagattttagtccagtcacaaaaaaagcagcgtcaaggcctccaaattgcaattgataatgagccgctggactttatgtaatttgaatcacgaaaggaaacgataaatttgacgacagttgtgttcatgggaacgccacagttcgcggtcccaattctacaaggattacttgatcaaaaatacgatattttatgtgttgtcacccaaccggatcgaccagtcggccggaaacaccggatttcacaaagcccggttaaacaagccgccgttgccaatcatctgccagtgtttcaacctgaaaaactcagtggaagcccggagatgcagcgggtcattgactttcatccagacttgattgtcacggcagcctacggtcaatttttaccgacgaagatgttaaacgccgtcaaaattgcggccgtcaatgttcatggctcacttttgcctaagtatcgtggtggcgcgcctgttcagtacgcgattatgaatggtgattcagaaaccggcatcagtctcatctacatggttaaaaagatggatgccggcgacattttggcacaaaaagcggttccaattcagccagatgatgataccgaaacgatgtttgacaaactcagcatcgtgggccgcgacctgctgttagccactctgccaaaagtgatcgccggcgatatctccccagtgcctcaagatgaggatcaagtcgtcttttcgcccaacatcaaaccggaagaagagcaactggacttcaatcaaaccgcgtttatggttaacgccaaagttcgtgccctgcggccggatccggtcgcttatacggttatcaacggtaaacgaaccaaaatttggggggcacaagttgtcgatcaaaccactgaaatggcgccaggatcagtggttgagaaaaccaagcaccaattattattgtcagcaggaaaaggcactgttttatccattcaggagcttcagcccgccggcaagccaaaacaacaaataacagattacttaaatgggattggtcagtcacttaaagttggccaacaggtgattaaataaatgaaatatacaacaaataatccacgccaacttgcagtcatgacgttggttcgcaccagtaatggttcatattcaaatctgcagattaatgccgtgattcaatctacttcaatgggtccagctgataagggactgttcaccaacattgtgtacggggtcattcagcatcgattaacgctggaatatcaactccggccatttttgcgtgaaccggaaaagactgaaacctgggtcaaagagctgctctataccgcgatgtaccagttggagtatctggatcgggttcccaagcgggcaatctttgatgaaacaattaaaattgccaagcagatgggacatgacggtacccgccgatttgtgaccggtattttgcatcagatggatcggcaggggatgccaaacttggatgacattcaggatgaaaagacccgactatcgattgaatatagtgtgccaacctggttggtagaaatgcttgacgaacaacttggcaagccaaaaacggcttcaatcttagcatccctgaataaagcgccaaagcaatcggttcgtgccaacttagccaaaatctctcaaaaagatttgctggcagatttggccaaggacggctatgatgccgaacccagccaagtttccagtgaagggattattattaacgatggtcaaatcattcacagtgactttttcactgacggcctgttaaccattcaggatgaaagtgccatgctgccagttgaatcaatgcagatttcccctgatgacaacgttttggatgcctgcagtgccccgggcggcaaaactacccaaattgccagccgtttgaaagccggcaaagtctttgcactggatattcataaaaacaaactgaaaaccgtccagcgaaatgccactcgcctgggagtctacaagcaagtcgaaacttttgaattggatgcccgcaaagtcgataccaaatttgaagacggcttgtttgattcaattttagttgatgcgccgtgttctggcttgggactcctcagaagaaagccggagattcgttatgacaaaacaattgctgatatcaatcgtctaagtgagattcagttacaaattttgaacgcggtttccgctaaagttaaaactggtggtactattacatatagtacctgtacgattgttaaacaggaaaatcaagacgtgatcgccaagtttatcagcgagaaccctaattttgacatcacgaagacaaagactgccaatcatttgaatccggatagcaagatggttcaaatctaccccgatgactatgattcagacggcttctttgtttgctccctcattcggaaatcataacggagttgatcaatttgcaaattgcatatcaatcctcaactggaaaagttcgcgacaaaaatgaagatgcggtcggcgcgtttaaaaatcaaaccgggctcattttggcattaattaccgacggaatcggcggcaacaatgctggcgaagtcgcttctcaaatggttgtcacccacatgggagccgcttttgaaacgaccagtatttctagtctggataaaattgaaacttggtttgaaaaccagttggcaaaagaaaataccgcgattatcgatgaatccaacacggacacacgactccatggtatggggacgaccatcgtggcgacacttattgatggcaaacagagtctgatcgccaacattggtgatagtcggggttatgtctattccaacgggcaattcactcagatcacggaagaccattcctatgtgaatgaattggtcaaacacggtgatatcactccagaccaggccaaaaccaacccatacaaaaatattattaccaagagtctgggaatcaacaacgattcggccgccgacttcaaaccgtataccgcccaacctggagatcaaattttactctgtaccgacggtttgaccaatatggtcgacgatgccgacatcgaaaaaattttgtcaatggatgaagaattacagactaagtgtgacatgttggtgtccttggccaatcaaaacggcggcttggacaacattactgtcttgatcgcccaatacgattcggaggtgaccgccgatgaataagggctatgtattaaacggtcgttatgaaattatcggtcgcttgggcgagggtggaatggctgacgtatacctggccgaagacctcatcttgaagcgaaaagttgccgttaaactgttgcgacttgatttccgagacaaccccaaagccaagaagcgctttcagcatgaagcaatggcggcgacccaactggataatcctcacattgttggcatttatgatgttgacgaggttgaggggatgcagtatttagtcatggaatttgttgacggtgaagatttaaagaaatacatcaaggataactttcccattccttatgccgaagttgtcaatattatggagcaaatttgctcagctgtcagtgaagcccaccggcataatattattcaccgtgatttaaagcctcaaaacattttggtcgataagaacggttatattaagattaccgactttggaatttcccgggccggcacagaagatacgatgactcagacccgttcgattattggctcgattcactatttgtcccctgaacaaattaagggtcagatggcgactgcccgatcggatatttactcattagggattattctctatgaaattttgaccggcaaagtgccatttaacggtgataccgccgtttcaattgccattaaacattcacaaacaccaatgccttcagtcagggattttgatccgcgcattccccaggcaatggaaaatgttgtcttgaaagctaccgctaagaatcccgatgatcgttatcaaacagttaatgaaatggctgctgatttgaatacgtcattggacaagtcacgggctaatgaacctaaatttacggttcagccaccacaaaacccggttgatgaagcaacccgggtgatgccattttcaccattggatgatacgactgcctcagcggatgccaatccggccaaacgtgaggaaaagcctgccggtacctcgaacgacaaaccaaagccgccgaagaaaaagcggcgacgaaggtggtggattatcggtgggattgtcggcctgctgttaataattctggccttcatcatgattgtttcagccaacgggaaaaccacggtgccaattgtctccgggacgttggaaaccgaggcggaagccaagattaaagcggctaatttgaccgttggcagtgtcaaatatcaaagtagtgataaaattgatcgtcatcgcgtcatcagttccagtcccaaggaagaaaccaaagtcaaaaagggcaccaaggtcaatttggtcgtgagttccgggccccgtcgcgttcgggtcggcaactatgtcggtcaagaatatgacgttgtcaaacagaaattggaagacgaagggtttacggttcatcggcgtaacgctccttcaagttcatttggctcaggcagaattctccaacaggactttgagtccggcaaacggttcaatccggctaccaagacactgacctttgtggtttcaaccggtgttaaacggattacgctgaaagacttaaccggcatgaccaaggctcaagtggtctcatattctaacaaggtggaaattaacccaacttttgattatgtttattctgacgaccagcccaagggccgagttgtccgccaatcaccaaatgccaacgaatcaattcaacagggcagtaacgtcgcggtttggatttctcgtgggcctaagaaagacagttcggatgaattgaagagcttcaatgtcaaaattaccatcccgtacctcgacaacagttcggcggcatcatctgactccacattgaatgaaagtggcatctccagtgatgctgcttccacagatagttccagtggttccaacgagaacgtggtcttgatttatctcaaagaccatgatcatagtttgtcgacggtttacaagcagatggtgatcacaaaggatacgcaagtcaccttgccatttaaattatccggcaatgaagtcggtcaatacaaagtggtccgcgatggtcggacgatcatgcgtgataacaacgtgacctacgattcacattaataattactgcaaaacaaagtcacttctcttataatgtaagggaagtgattttttatcgaggtgatcaattgaaacaaggaaagatttttcagtctttgagtggcttttatgatgttcactcagaaggcaaggtttatcgaacacgcgccagggggaattttcgaaagcgtcaaattacaccgttggtcggcgatgacgttgagttccaagttgaagatggcgacaaaggatacatattgaagatgctgccacgaaagaattctctggttcggccaccgattgccaatattgatcaggcgattgtggcgacggcaaccactcagccggagttttccagtaacttattggaccgtcagttgattgcattggaaattgccaatatcaagccgatcatttatttcaccaagacggatctgttatctgaaaaacaactgaattattttaaagatttagcagttgcctacgctaacattccttatgacgttattctgccggaagccgcgtttgatgaaaattcgttgaaccatttacggcaattgttttcaggaaaagaaaatgtgataatgggacagacgggtgccggcaaatcgacacttctcaatcacttggcaccggatttgcagctcgctaccggtgagatttctgcggcattaaatcgtggaaaacacaccacccgaaaagttgctttattgcgggtcaacgatgggtatatcgcagacactcccggattttcctcgtatgataccttggagatcgattaccgccagcttgccagttatttcccagagttcaagcgggcatctgtgaagtgccgctttcggggatgtgtgcatgtcaatgagccggactgtgaagtgaaaaaagaagtggccagcggtgacatcatgcagagtcggtatgagaattatctgcagttgtacaccgacattaaaaaccggaaaccaaattataaaaagtgaggaagttagttatgattaaagttgcaccttcaattttgagcgcggattatgtcaatttacaaaaagatattgaaaaagtcgaccagggtggggcggaagtcctccacatcgacatcatggacggtcagtttgtcccagctttatcctatggacctgggtgggtcaaagccattcgtccgatcaccaagatgatcttggatgtccatatgatggttgaacaaccggaacgtttcattgaccaattcgccgatgccggtgccgatattatcggagttcacgttgaggcaacccctcatattcaccgggctttgcagatgatcaagaacaaaggggtcaaggctgaagttgtcatcaacccgggtacgccggtatcagccatcaagccagtactatacatggttgaccaggtcttggtaatgacggttaatcctggatttggcggtcagaagttcctgcctgaaacggttaaaaagatcgcagaactcgatgagttgaaaaaaactgaaggcttgaactttgacatcgaaattgatggtggcgttaatgaccacacggttgtgggtgcctatcaagccggtgcaacggtggcagttgccggatcatacgtttttgacgccgatgatcctgttagccgaatcaaagcaataaaggatgcgaccaaataaatgaagatcttaaatctattggttggcggccccattgacctctggccagacgaattgaaaaatggacagattaaaggtgattggatcggcatcgatagaggcaatctccatttgatcgagcgggggatcgacccacttgtcgcgattggtgacttcgattccttaaaaccggcagaacttcaactagttcgtgaccacattaaggatatccgccagtcaattcctgaaaaagacgatactgatacccaattggggttgaaggtcgctttgcaggaacatcacgccgatcgacttgatatctacggtgcgacgggtggccgactggatcattttctagccaatctgtggatggttttggaaccccggttcaagccctacgcaccgaaaattcgaatgattgacaagcaaaatacgattactttctttttgccaggaacttatcagattgaaaaggaacctgataaaaaatatttggcattcgtggcgttaacaccgatggatcatttaactttgtttgatgaaaaataccagctgaatgactatcaggttaaacacccaatgtcgcttgccagcaatgaatttgttggtgaaactgccaggtttaaatttggcagtggggtgatgtgtgttattcaaagcaaagatattaatcgttataactaaaaaaggggcaaccctcagctcaccgaaaacggctgctgagagttgcctctatttttgaaggtaataaaaaagaccgattaacatcgatccaagttattactatacacgggttactttacctgatttaagtgttcgggcagaaatccaaaccttcttaggcttgccatcaacaagaatgcgaactttttgcaaatttggcttccagctgcgacggcttgagtttaaagcgtgtgaacgtttgttaccaaagtgggtacgcttaccgttaataaaatcctttgccatgggtaacaaatctcccttctctttgattttagtgttaaagtctgtttcattacactagaataatttatcatacatacattgatattgcaatacttttctttcaagtaattatacttgacagtcttcttgggggcatcaagattactttggtttttagcgttattgtggtaatattaactatcgttaataggttaatagaaaattaaggaggctgctgcacatggccgtcaaaatcaaaaccagatttggaacagttgacatcgacaacaacgtcatcgcaaatgttgttggtggggctgccaccgataattacggagtcgtgggtatggcaagtcgcaatcagctcagagacaatgtcaacacgattttaaaccgcgagaattatttcaagggtgttgtggttaaacaacacgataatgaaattgaagttaacgtttatattatcgttgcttatggcaacaaaatttcagaagtatctaaaaacgttcaagcaaaggttaagtataacctacaaagtatgcttggggtatctgcaaattcggtcaatgtcatcattcaaggcgttcaggtaatgaatgactgattatgcaagtgaccaaggaggacaagttgttgaaagttacagaaattaccaacaccgaatttacggcaatggttcaagcagccgcaactaaactaaataaaaattctgattttatcaattcactgaacgtattcccggttccggatggagataccggaaccaatatgagcctatccatggcttcgggttataaatatgtgaataaagatgtcaagacaaacgttggcgatttaaccgctgctttggctaagggacttctaatgggagcccgaggcaactcaggggttattttatcgcagattttccggggcttttcgaagtccacggagggtaaagaaactttgagtgcccaagatatttctgatgccttcgttgccgggacggaaatcgcctataagtccgttatgaagccaaccgagggaaccattttgaccgttgtgcgaatggccgctactgctggtaagaaagcagccgctacgaccaatgatgttgtcgctgtcatggatgccatctaccaggcctcacaatccgctttggagaaaacaccggatttattgccggtgctgaagcaggttggtgttgtcgactcgggtggacaaggattggtattcgttttggaagctttcgatgatgtcttgaatggcagaaacgaagctgaatccggtgaatatcaacctaacgatgcggaaatgaatcagatgattaaagtggccgatcaaagtgttcaaagtaaattaaatccagaagatatcgtgtatggctactgtacgcaaattatggtccgaatcggcaaaggccgcgaagttgatcatcaatttgactatcagaccttttatgattatctcgccaagcttggcgattcattgctggtgatcaacgatgatgatattgtcaaagtccatgttcacactgaacatcccggcaaagtgcttgcctggggtcaggagtttggagatttggcaactgttaaagtcgataacatgcgacttcaacaagaaaccatcattgaagaagatgaggacagccaagaggacgcttcaccaattcaaaaagctgaaagtatcagcacccagcagccaacttcagatactgccattatttccgtttcttcaggcaaggggctgaaccaactgtttgaaagtttgggcgtcaactacattgtcagcggcggacagacgatgaatcctagtaccgaagacattgtcaacgcaattcaaaatacaaaagccaaacaggcaatcgtcttgccgaataacaaaaacattttcctggcggctgaacaagctgccaaggtggttgatattccgacggtcattgttcattcaaagacgatctcacaagggattaccgccatgcttggctttaatccggaaaattcgctcgaagataaccaaaaggcaatggaagataatttgccaacggttaagtccggccaagtgacgaccgccattcgtgagactaagattgatgatttggatattaaaaaagatcaatttatgggcatcgttgacggcgatattgccaccgttggtgataaactgattgacacggccattcagatggttaagaagatgctggatgacgatagtgaagccattacgatcatttacggtgaaggcgctgatcaggcggctgccgaaaaagtccaggccggcattttgaaattggatgacgaactggaagttgagattcacgaaggtgatcaaccagtctacccattcttaatttcggttgaataaacaattcctaaaagtttggtcaacactggccaagcttttatttatatcaatgacaaaggagggataacattggccagcttaagtgattcggttagggttctcaaaggagtcggcgaaaagcgcctgactgctcttaataagctcggaatcaataccatcaacgacttactgacttattatccccgccgatatgatgatttatcgctaaaagatttaagaactgccgtcgatggccaaaaagtcaccgtcaaagggatcgtgattagcgagccaactgttcgtttttttggtcggcgcaaaagtcggcttggttttcatttaaaaattaatgatgaaatctataacgtcactttttttaatcagccgtggctgaaaaagcagcttgagttggaagcccaagtgattatttttggtacctttgaccgcaatcgtaaccagattcaagggatgaaaattttaaacggcgaaaaaagcgacacctatgattcaatctatccaagtaacaaagaagtcaaacaaaataccattaaacaattgatcaagcttggatttgatgaataccaggatcagctagttgacgtcattccagagtcaattcgcaccaagtatcgattggaatccttccgtgataccattcaaaatatccattttccaacatcaccggtcgctgcccaaaaagcttttcgaactgccaagttcatggaatttttcttatttgccatgaaaattcaaattttaaaacagcgccacagaaaaccggatccggcagccaaagttgcctatgatccagatctagttaagcagttcaccagtcaactaaaattcaaactgaccgattcccaaaacaaagttgtcaatgaaatcttgtccgacttgggcaaaccattggaaatgaatcgcttgctccaaggggatgttggtagtggcaaaactgtggttgctgcaattgcaattttggcagcgattagtgccggcaaacaagccgcaattatggccccaactgaaattctagccgagcagcatgccaacacgtttgccaagttgtttgaaaaatttgatgtcaacatcgccctgttgaccggggcgaccactggcctagctcgtaaggcgatgctgccgcggatcgctgacggtgaagtcaatctgattgtcggcacccacgccttattccaggatcaagtcgactatcacgatcttgacttggcggtcattgacgaacagcatcgcttcggggtcaaccagcgccaggccttacgactgaagggaaatagtaccaacatgctggcaatgactgccacgccgattccgcggacactggcgattacgatgtacggtgatatggacgtctctgtgatcgacgaattgccaaagggccgcaagccaattaagacaacttggattacctccgctaaaacggatagtgccattcgatttgttaagaaacaattggatgccggaaatcaagtgtacgtcgtcacaccgttgatcgaggaatcggaagctgtcgatatgaagaacgccatggcgattttcgaccgtttcaaagcgatttttgaaccgcagtattcagttggtctcctacatgggcgaatgtcggatgaagaaaaggatacggccatggccgattttaagaacaatcaattccaagttctggtggcgacaacggtgattgaagttggcgttgacgtgacgaatgccaataccatgctgatatttgatgccgatcacttcggtttggcacaactccaccaacttcgcggtcgcgttggccgtggcgacacgcagtcctactgcattttgattgccgacccaaaaaacgagttgggtaaaaagcggatgacggcggttgccagcagcaccgacggctttttcctctcccaaaaggatttggaattgcgtggccaaggtgacatcaccggcagtaaacaatcagggatgcctgattttaaagtggccgatccggttggtgatttgaacattttacaagttgccaatcaggaggcccagagtattacggttcatcaagactggcaaaagcagccagaaaatgtacaattatcacagtatctaaaatataacgaaactattactacggattaaataggagttaaatatgaaaattgcagttgacgccatgggcggcgattacgcccctaaagaagttgttgaaggaattgaattggcacgggatgcttatgccgatgttgaattccaactatttggtcaaaccgaccaaattaaaaaatatcttaaaaatgatgatcgaattcagattgtccaagccgatgaagtcatcgaaatgggtgatgaaccggttaaagccgttcgtaccaaaaaacaatccagcatcgttctggcagcaaccgctgttaaagaaggaactgcggatgcgttcttctcggcagggaacactggtgctattttagccgccggtttgtttatcgttggccgcatcaaaggaatcgatcgtcccggattgaccaccactttgccggtcatcggcgttaagaatcaagataaatttgtgatgattgacgtgggggccaatgcagacaccaaggttttaaatatttaccagtatgccttgatgggaaaatattacgcccaaaacgtcaaccaagtcgaaaatccacgaatcggtctcttgaacaatgggaccgaagcggataaaggtgatatgaatcaccggaaagtgcatgatctgttggcagcggacaaagatattaattttgtcggcaacgttgaatcccgtgaattactcaacggggccgccgacgtggttgtgaccgacggctttaccggaaacgccgtattaaagagtattgagggaactgctttgtcgatgctcagcttaattaagacgaccatcatggatagcggcactaaagcaaagtttggggctttgatgttaaaagacgccttccacaaaattggcggttcaatggactattcacaatatggcggcgcagttttactgggcgttaaggcaccggtcgtcaagacacatggcagcagcaaagcagacacggtgaagaatacgatcggccaaatccgccagattattgcctcaaatatgattcctgatctgaatcaatacgtcgtcgaccataatgatgaactgcagcagataaaagatagtatcaaaagcagtaaatagttgatataataatcattagcaaattaattttatgaaataggtgtttatcaaaatggacaaagatgaagtgtttaacaaaattgccgatttggtggctgaccagtttgatgtcgaccgaagtaaaattaccggtgacttaaattttaaaaacgatcttgatgctgattcaattgattttgttgaattcgtattggatatggaagatacttttaacgcagaaatttccgatgaggatgctgaaaagctgaataccattaacgaggccgttgattttgtcatggctcatcaaaaataataaaagtaatcttaaattggaattatctcaagtttgatataatttcaattttttactgttatctggattttatgtggaggtaaaagattgataaagggtttaaatgagatgctaaagcaagattttggcatccatatcgatgatcaggatttgcttgatgaagcattcacacaggcttcttacgtcaatgagcatcgcggtgaaggcttaaaattttatgagcgtctggaatttttgggggatgctgttttacagctgatcgtctccgactacattttcaaacgttatccaaagatgcctcaaggacggctcacgcgacttcgagcagcaatggttaatgagcaaagtttcagcacctttgccagagaatgtcattttaatcagtatatccgtctcggtaagggcgaagaaaaggcgggggctcgtgatcgggactcgctgttatgtgatatttttgaatcattcgtcggctgcctttatttggaccaagggcaggccgaagtgacacgatttgtgaccaaagtgatttttccaaagcttgatgaaggcatgtttgcggaattctttgatcataagactgagttacaggaactcgcccaagcggacggtccggtggccatcgattatgaattagtggacgagtacggacccgacaacgaccgttcgtttaaggtcaacgtctcaattgacggcaaactttatggtgttggaattggccattccaagaaaggcgccgagcaaaaggccgcccaacaagccctggaacagtttgataccgagggcgacaatctagtttagactggagaatgagtgtgcaacttaaatccattgaaattatcggttttaaatcatttgcagacaaaactctcatcaaatttccgggtggaatgactggaattgttggtcccaatggaagcggtaagagtaatattgccgaatcaatccgttgggtgatgggggaacaatctgccaaaaatctccgtgggtcgcggatgcctgatgttattttttcaggctccgccgatcgacggtctttaggcatggcctcggtaactttaaccttggacaactccgaccatttcattaagtcccccttcgatgagctcaagctttcccgcaaactctttcggaacggcgatagttcctattatttaaacgaaaaacagtgtcgtcttaaggacattaccgatttgttcatggataccggcatcggtcaagggtccttgtcgatcatttctcagggtaatgtggaacaaatcttcaacagtaaacctgaggagcgacgatcaattattgaaaatgtcgccggcgtctacaaatacaagcagcacaagaatactgcccaaaaagaaatcgatgagacttccgataatctcaatcgagtggaagacatcatttctgaacttcaaagccgaatggcaccgcttgaagagcaaagtagtctggcaacggattatctggatcaaaaaaagcgtttagatcagtttgaaaagcagcagttaattttggcaactcagaaattgatcgcagccagccagcagctcaaacacaccgttagtgaaaagtctgacttggttaataaaatttacgctcaagttcgccgggatgaaaatgaccgcgacaaactgaaagccaatttaactcaaaaccgggccaaaatcgaccaaatcaacgagcaaattctgacagcaactgaacaaattcagtcgctgaagagcaagcatcagttgtccgctcaagagaagtcttttaaggacgccgatttaaaccggatttcggaacaaatcaaactgactgacaagcaaattgacgattttcaggtcaaactcacccaatcggtggatgccggcaaacggctatcggaaaaaattgctgccaaacaagccgacttcgacaaactggcagaagcccaaaaagcgaatagcgtttcggtaattgaatctgaaatcgaccaattgcgtaaccaatatgtcgacttactgcagcaaaaaaccgacattaaaaatcaaattaccatgaaaactcatgatgaagcccaacttgagcagcaactggggtcacagcgacagcggattaataaagtgcgtgaggaccttggtcaaacccaggcagaattagctaacaaacaagctgctctggcttccagccaagctgaattgacggatgtttccaagcagctgggcgatttaactcaactaatgaatactcaccagcaggctgtcgacagttcccaggccaattggctggcagcactcaaaattgccgagcaggccaaagcaaaagctgagtctttgaaaaatcttcatgattcttatcgtggcttttaccggggcgtggcgaatcttctcaaacggaaaaaccaattaaccgggattttggggccagtcagtgactatttaacgattgatcaacgatatgtgaaagcgatcgagaccgcattaggatctcaagcccaacatgtcattgtcgaagataatcgggcagcttcctccgccattcgtttgctgaccaaagagcgtttggggcgggtaacgctgttaccaatttcaaccattaaaagtcgccggctaagttcgacgatcgttcatgagtcacaagaagttcttggattcattggtgtagcagccgatttggtatccatgccggataatctcaaccagattaaaggcttccttttggggaccacgattatcgccgacacgcttgaccacgcaattaacatttccaagcaaattaaccagcgcacgcgcattgtcactttggatggccaagtcgtcaatgccggcggctctctaaccggtggtgccagtcgtcatgataaccaaggggtgttggttcaaaaatccgagttggccgctctcaatcaatcgaccgctcagatggaccaaaagctgacggaaaatgaacgtcagcttcagcatgccaaggatgagctggctaaaatcaatgcgtcacatgagcgtggtcaacgaaaagcgttcgaaattcgccaacagaccgcaaccttggaggatcaatgccattcacttgaagaggctgttcaggaaaagcagcgtgaatttaagaccctccagctcgctttgaagaacgctgcccagtctgatggaacaactgacaccgaccagttggtcaaccgtcaggatgccatcgacaaacaattgcgggcagtcaatgatgacttggacaacaaacgggttcaactggcaaacgttaaacaatcggctcaaaaatttaccacggaaaagcaacaagtccgagaggcgattgtcgttgagcagcaaaagttgaatcagcttgaagttgatcaaacaggaatcaaaaagcagattgcgactcatcggcagaatcgggaccgcctgatccaacagcgagaccacttaaaggctgaactcagtcgtcaagtcgacgccgggacgttgaatgagcaaattaagaccgccgaagccaaccaacacgcacttaacctgacgcaaaacaagttgaaagccaccgttggtgaagcacaggatcatttggatcagttaaatcaaaagattcaagatgagcagattaacttgaataacgccaaatatgaacttaccagtgcccagacagctgctgctaaaaaccaccaggatctggataccaactttgcgactctggaaacgacttatcagatcgatcaacatgatttagcgaatcccgactggaattgggatgaaaagcaggttgccagccaaattaaaatgcttcgaaccgggattgacgaaattgggcctgtgaatatcggcgccatccaggaattcaaggaagtttccaagcgcttcgaatttttgaccagtcaaaaacaagacctcttggatgctaaggatcatttaactgccaccatgcgcgacatggatgacaccatcacgactaagttcgccatggcgttcaaacaagtcagccaagcgttttcgaaagtcttcgttgacatgtttggcggcggtgaagccaaactggtcttgaccgatcccaatgatatgttggatactggaattgagattatggttaagccgcctggaaagaactatcgcaacttaaatctcttgtccggtggcgagaaagccttaacagcgatcacattgctgtttgcgatcattaaggttcgaccggtgccattttgtatcttggatgaggccgaagccgcccttgatccgtttaacgcagaccgcttcgcaaaatacttaaagcgtttcggtgatgagacccagtttgtggtcatcactcaccgaaaagaaaccatgatttacgccgatcaactgtatggagtaacgatgcaggaatcaggcgtttcaaaagttgttactgttaatttagataatttaaaaacggaggtgagttgattgggactttttgatatatttaaacgtcgttccaaaaaagacgacgaaaaaaagccgactgaatcaactgaacaaaccgaacccaaaccagaagcacctgccaaagacgaccaaagcgccgccacttcaaatcaaacaaccacagatgttgaagagtccgccaaagccactaagagtccggctgatgaaccagctgaaaagaccgaaaaacaaccgacagaacagcctgaagaatcaaatggccaacaaaccacaaagcagccggacgatgctcaaaaaccaacaccaactgttagtgaaccaaattcatcggctgagcaggaatcttcgacagaagagtcggatatgccagctgagcctgaaaaatcagttgaaagtccagaaccggcagaatcagccacagattcaaatactcagcaatacgaaaaaggattggaaaagtcgcggtcctcgtttggtcaaaaactgaatgcccttttagcaaacttccgtcacgttgatgaatcattttttgacgacttggaagacatgctgattgaatccgacgtcggttttgaaacctcgatgcgaattgccgatgagttgcgcgatgaagtcaagctgcaaaatgccaagaagcccaaagatgttcaaaacgtaatcgttaaaaaattgattgacatgtacgatcaagccggcaatggtgaaaattcggccattaacatggcaaaatccggtccgacagttatcatgtttgtcggtgtcaacggggttggtaagacaaccacgattggtaaaatggctaagatgtataaagaccaaggcaaaaaggtcgttttagccgcggccgatacttttagagccggcgcaattgaacaactcaatgtttgggcagaacgagatggtgtggatatcgtcaaaggcaaagcgaaaagtgatccggcatctgtggtctacgatgcggttgttaaagccagaaaagaagactatgacatcttaatggttgatactgccggccggctgcagaataaggtcaacctcatgaacgaattaagtaaaatgaagaaaattctgactcgtgagattcccgaagccccacacgaagtcttgctggtacttgacgccaccactggccaaaatgcgatgacccaagccaaaatgtttaaggaaaccactgatgtttccggaattgttttgaccaagcttgacggcacagctcgtggcgggattgtcctcgccattcgcagtgaattacacctgccggtcaagtatgttggtttaggtgagcaggtcggcgatttgaagccgtttgatccaaacgactttgtttacggcttattcaaaggccttatttccgaatagtcaggtattttaacgttgactgacgttatataaatctgtacgctagatgacatattggccgtcaaaggagtttcaatatggaactggaaaaaaataactacatcaattctttgtttgaattttacgagccactgctcaccaaaaagcaggccaactatattgaactgtattatgctgacgactactcgctgggggaaattgccggtgaatataacgtcagtcggcaggccgtttatgataatattcgccgttccgagaagattcttcagcaatatgaagacaagctgaatttgtatcacagctttgttgaccggaacgacaaactagaccacattcaagcttatattcaaaaaaaatatccacacgatgacaaactgaattcaatgatcaaaaatttggaaacaaccgaagaacaataaggggtgaattaattggcttttgaaggattaaccgagcgtttacaaaacgccatgaaaactttacgtggcaagggaaaagtttcccagtccgatctgcgggcaaccatgcgggaaatcagactggctttactggaagccgatgttaatttccaagtcgtccgtgactttgtcaaaaccgttgaggagcgtgccaacggtgccaaggtgttggaagggttaaatccctctcaacaaattgtcaaaattgttgacgaagagttaactaaaacgatgggggaagaagccgttcccctgaataaagcagaaaaaatccccaccattatcatgatgtctggtctccaaggtgccggtaaaaccacaactgccgggaagttggctttaaaattaaagaatgagcagaacgcccgaccgttattaattgccgatgatatctaccggccggctgccattgatcagctgcagactgttggtcagcaaatcgacgtccccgtgttttcactgggaacggatgttgacccggtcgaaatcgccaaacggggtgtcgaacaggccaagcaagaccataatgactacgtgatcattgatacggccggtcgtctgcaaatcgacgaaaagttgatggacgaattaagtcatatcaaggatgccgttgaacccaacgaaattctgttggtcattgatgccatgactggtcaaaacgccgtggcgaccgccgaaggatttaataagaccttggacgtaaccggagttgtcttaaccaagttggatggtgacacccgtggtggtgccgcactttcaattcgtgccgtcactcaaaagccaatcaaattcgttggtcagggtgagaaaatgtctgatttggacgtcttctatcctgatcgaatggcttcgcgaattcttggaatgggtgatatgctttcactcattgagaagacccaaaaagagtatgatgaaaaacaggctcaggaattatccgagaaaatccaagagaatacctttgatttcaacgattttgttgaccagttaaatcaaattcaaaagatgggacccttggatgaaatcatgaaaatgattccggggatggcaaataatccccaattaaaaaacgccaacatggaccctaaagacatggaccacttgaaggcgattgtctattcaatgaccgatcaggaacggactgaccctgatgtattaaacccatcaagacgccggcgaattgcccgcggctccggtagaccaatccaagaagtcaatcgaatgattaaacaattcggccaaatgaaaaccatgatgaacaaggtttccaaaggcaacatgtctggcatggaaaatatgatgaacagtactggcatgggcggtaaaatgtccaaactggcaatgaaacagttcagccgtaaaatgaaaaagaataagaaacgccgtttgaagaaaaagaacaagaagcgccgttaattctgacaagttatcagcattgacacgccattaatttggtcagtttggccaaaacaagtcaatccatcagttcttttgatggtgtaaagaaaaaaacctttacaagcattcgaattactggtatattattaatcgttaaaacattacaggaggtaaaagcatgtcagttaagattcgtttaaagcgcatgggttcaaagaagcgcccatattaccgtatcgttgttgccgattcacgtagtcctcgtgatggtcgtttcatcgaaaacgttggtacttacagtccattaactcagcctgccaagattactcttgaagaagagtcaatcatgaactggctgaacaatggtgcccaaccatctgatactgttcgtaacatcttatcagatgccggtattatgaagaaatatcacgaagctaaatactcaaaaaagtaagtgagtgattatcatcatgacaagtattgatggtttaattaataagattatctcaccgttggtagactatcctaaggatatcgagatttcgcataatgaatccgatcgatttatggaatatcatctgaagttgaacgaagaagatattggcagaatcattggaaagcatggccatgtgattcagactatccggaccattgtttacagtgttccggttgagggtcaaaagaaagctcgtctgattgtcgacgatgggaaacaatagggttcttaagcgaaacgaaggttttgtttaggcccttttttctttattcaaaatgagattcattagagctggaggagtgagtgaatgaattattataatattggcaaaattgtcaatacccaaggcttgaaaggcgaagtcagagtgatttcgattactgattttccggaaaaacggttcaaagtcggcaacacggtttttgctaaattgcctaacaagcacgaacaagtggcgctgacaattgacggtgtccgcaaacacaaaggatttatcctattgcactttaagaatcatccctcgatcaatgacgtcgagtacttaaagccatcagaacttaaaattgatgagggaagcctctcaagtgatgatcttaagcctggtgagtattactaccaccaaatcatcggcctagacgttgttgatccaaatggtaacccaattggccaagtgaaggagatcctctcaccgggcgccaatgatgtttgggtggttgaacgcgatcagcacaaagatttactgctgccaaagatcgattctgtcattacgaatgttgaccttgatgccggtaagataaccgcagatgttccggagggcttggacgaatgagaatcgacgtactgagtttatttccagaaatgtttgcggtcccgatgcacgattcaattattggaaaagcaattgagaaccacattattgatttagatgtcaccaattttcgtgaatttaccaccgacaagcaccgtcacgtggatgattatccctttggcggtggtgcgggcatgctgctgcaggcgcaacccattttggatgcgtacgaccacaccaaacaaactgctgaagctgccggctatcctaagggcaaagtgattctcatggatccggccggaaagccattcaaacagcatgatgctgaagagttgtcacatgatgaccatttaacctttatctgtggtcattatgaagggtatgatgaacgcattcgttccatcgtgaccgatgagtattcattgggggactttgttctgactggcggggaattgccttcgatggtcatgatcgatgccattacccggttaattcccggcgttttgggcaatcatcaatccagtgttgaggaatccttttcaacgggtctcttggaagaaccccagtatacccggccggcagagttccgggggatgaaggtccctgaagttctcatgaacggcgaccacaaaaaaattgccttatggaatcaaaaagaggcattgagacgaacttacctccggcgacccgatctgatcgaccatcacaatttaaccagcacccaaaagaaattgttggctgacgttcggattgaggaagaagaaaagcaagccgcaaaagatactgacaagaaaaacacctttacagacgatgaataattgtgttacactaatttttggcgcaagccgcaaaacaacattccgctgtcagacaagataatgaatgttagtgaaaggaagatttgtttatgcgacaaaatcaattgattgacaagatcaacgcgaagcaactacgtaatgacattcctgatttccgtgccggagattctgtaagagtttacgttaaggttgttgaaggtaccagagaacgtattcagttgttcgaaggtgttgttatcaaacgcaagggttcaggcattcaagccacttataccgttcgtaaagtaagtaacggtgttggggttgaacgaattttcccacttcattcaccacgagttgataaaatcgaagtagtaagacaaggtcacgttcgtcgtgccaagctttactacctgcgtgacttacaaggtaaggctgctcgtattcgagcttcccttcgttcacgtggataatgaatcaattagactggatcgaattattcgattcagtttttttgtattctcattttcaggattcagcctacctcaatgcttaagttctggttaagactagcacaatccattgatgactgctaatcaggtcggtaaaatgacgcttattcgatgattatgatcggatttagttttggttaatttcatagcaaatcgggcacaaacggcgtttatttgctatcatagatattaggacatgaacacgattacatcgttgaaggtgatagttatggctgaatcagatgaagatcaaaaaaatattcaatggtttctgaagtatttacaaagtgaccgtcactattctactgataccatccaggcttatcagcaggccattgccgaattcacccgctttctggccgaaattcccagtgaacgcaaaccattgacccaggtggactcgtttgatgttgaagcatttttgagcgatctttatgagcgaaaatatgccagaaattccatcgcccaaaaggtatcggcattgaagtcgttctatgctttcctggtgaagaatactgtgatcgccaacaatccattcgaatatgtccacttgaagaccaatcatcggcgtttgcccagatttttgtatcaaaatgagatgcgggcgctttttcagggagccggacaaaatcccaatcaccaactgggattgcgcgatacggctgttctggaaaccttatatgcgactgggattcgggtcagcgagtgcgccggaattcagctcaatgacatcgatttggacaaccgaaccatcttagtcactgggaagggcaacaagcaaagatacgtgccctttggggaatatgctcaagaggcgattgaaacttatctcagcgacgccagaagcccaatcatggccaagtaccatcaagaccatccatttttatttgtgaatcattacggccgaccgctgacaagtcggggtatcgaatatctgatggatcaaatcgtcaaacaaagtagtctgacgacgaagattcatccccacatgctgcgacacacgtttgcgacagagatgctcaataatggtgccgatatgcggtcagttcaagagttgctgggacacagcagcctgtcgacaactcaaatctacacacacgttaccaaatcacatttaatgaatgattataaaaagtattttcctcgaaataatgattcattaaaatcaaactaataaaggggtatattatgccaatcaaatttgaagcaactactatcgtcgctgttcgccacaatggccatctcgcaatggctggagacggtcaggttaccatgggtgaaaaagtcattatgaagggaaccgcccacaaggttcgtcggatttatgacaaccaagtcgttgtcggctttgccggaagtgtcgctgacgcctttaacctcgaagaacgatttgagaagaaattaaaccagtttgacggtgacctgaaacgttccgccgttgaattggcccaggagtggcgtggcgaccaacagttacaaaagctcgaagctttgctaatcgtgatgaacgataaagatttattgctagtatccggccaaggtgaagtgatcgaaccagacgatgatattttagcgattggttccggcggtaactttgccttagctgcggcaactgccatgaaacatcacgctcaggacatgagcgccagagaaattgccgaagccgccattcacattgccggcaacattgatattttcacgaaccaaaacgtgatttctgaagaattataggaggaacttaaattgactgagtctactcaaacaccaaaagaaattgtttccgtgcttgaccaatatattgttggccaaaacgaggccaaaaaagcggttgctgtggccttgcggaaccgataccgcagaatgcagctgtcaaaagacatgcaggatgaaatttcaccaaaaaaccttttgatgatcggaccgaccggagttgggaaaactgaaattgctcgccgtttggccaaaatcgtcaacgcaccgtttgtgaaagttgaggctaccaaatttaccgaagtcggttacgtgggtggcgatgttgaatcaatggttcgtgacctggtcgaaaatgccatccaattggaacgggctgatcagtacaaacaggtccacgtcgaagcagaaaagcaggccaacaatcgcttggttaaacttttggcaccggcaaagaaaaaagagaaccgccaaaatgagatgcagaacctgatgaatatgtttactcagatgcaaaatggccagatgccgtctgaaaatcaggacgatcaagaagaagttacggatgatatccgtgaaaaacggatgtcgatcgcagaaaaactcaaggctggcttgctggagaacgaccaggttgaaattgaaatggatgatccatcccaacaacccgctggtcaaagcacgatgatgaaccaaatggggatcgatttgaatgataccttggccggactgatgcccaaaaagaaaatcaaacgcaccgttcctgtaagtgaagcgcgagaaattctaacccgccaggcttctgaagaactgatcaacaaggccgatctttaccataatgcgatcgttcgcgccgaaaataccgggatcatctttattgatgaaattgataaaattgccccgggaaagtctcaaaatagtggcgaagtttcccgtgaaggggttcaacgcgacattttaccaatcgttgaaggctctcaggtgaataccaaatacgggaccgtcaataccgatcacatgctgttcattggttcgggtgcctttgccgaaaacaagccttctgatttaattcccgaactccaaggacgtttcccaatcagagttgagttaaatgatttaaccaaagaagactttgtccgcattttgacggaaccaaccaactcactgaccaagcaatacattgctttgatcgggacggataatatcaaagtaactttcaccatcgaggcgattaatcggattgccgaaatcgccactgatgtcaaccacaatactgataatatcggtgcccgtcgtctgcacacgattcttgagaaattgcttgaagatatcctttacgaaggaccggatatgcagatgggcgatattacgatcactgaaaaatacgtcgatgataaagttggcaaactggctcaaaataaagatctttcacgttacattctgtaaaattgggaggaagagattaaatgattaccttgaaaaatcagtatttgaccgtgctcatcaacgagcagggtgccgaactcacctccgtgaaagatactgacggattagaatatatttggcaggcggatccagcattttggaagcggcatgcgccaattctgtttccaattgtcggtcgacttaaggacaaccaatacacctatgctggccagacttatgaaatgacccaacacgggtttgcccgcgacaatcagtttgaagttgaatcccaattaccaaccaaagtctcactggttttacggcccactgaggaaacgttggccaaatatccgtttaaattcgaactgcgaatcatttacgaactggttgatcatcaattgaatgtgagtctaaacgtcatcaatccaagtcaagacacactgttgttttcaattggagctcatcccggctttaacattcctttggtcaaaggagaaggtaacttcgaggattcctttattcgggtagcaccaaagaagtcatacgttcaaatcccattaaaaccgccgtatagcgatccaaacgatccccaggcaattgacctgaccaagccgctgccgttgaaccacgagctgtttaacagcgatgccatcgttttgagccttgatcgccaggaaacgactgtgatgctggccaatgcccaaaatgatcatggtgtttcactcacggttgagaatgcaccatatgtcggtatctggtcaccgtacccgaaaaaagccccgtttgcctgcattgaaccgtggtggggactggctgatacagtcaatgccgacggcaagctggaagataaatttgcgattaatcagttggctggccgccacgcctttgccggtcgatattcaattagtttcttctaactgatagtagctgtcgcatcaattgcccggccgattaaaattcaaactaaaaacgagtgattccttatttcagaaatcactcgtttttgattgggttattcattcggatctttacgttttcgcagccgattgccaaggccaaatggcaccatactttcggtgccgtttttaattcggttgatattggcccgatgccggtaaaaaatgaaaaaggtcaggatcaccgccatgacactcaataaaatgtcgtgggtaaagaaaattgcgatggtcgttaaggtaaaaccgatcatgctggcaagactgaccatgctggttaacaaaatcaccagaatccaaatcccggctgccaaaaagaagaaagccggcttgtatgccagcagcatccctgcactggttgccaccgccttgccgcctttgaatttatcaaagattgaaaaggtgtgccccaaaatcgccatgagtccaaagatcaacggactgatcgcggtgatatgaaaaaatgtcggcagtaatgtcgccaccgctcctttagaaatatccagcgccatgacaattgagccggcaatcggccctaaaacccggtaggtattggtggtcccgatattgccggagccgtgtcggcgaatatcaatgtgaaagaaaattttaccaatccagacaccgctgggaattgatcccagcaaataagctagcactaacagcattataatttgttcaatattagaattcatcttaaacctcacaatagtcgcaattaataaacttaatagcgtttctcattttagcatgtaatttgggttcagccaataaaatttcgtttccatcggcgtaaatttaggttattatgaagtagattgcaaaaaaaggagtcataacgaatggtaaagcaaaagcaaaaatatgatgattcctcgattcaaattcttgagggactcgacgcggttagaaagcgtcctggaatgtacatcggttccactgattcacgtggcctgcatcatttggtctacgaaattgttgataatgccgtggacgaagttttggccggttatggggacgaaattgacgtctcaattcataaggacaacagtatcacggtggtcgatcacggccgggggatgccaactggtatgcacgcttcagggaaaccaactcctgaagtgattttaacgatgcttcatgccggcggtaaattcggtcagggcggctacaaaacatccggtggactgcacggcgtcggcgccagcgttgtcaacgcactttctacttggctgaaagttgtgattgtccgtgacggttaccgttacgaagaagatttcaaaaacggcggccatccggtgggcacactgaaaaaattaggcaaaacccgcgctcatagtgggacaacggtaacctttaaaccggatccaactattttcaccagcacggtttacaatttctcagttctttccgagcgattacgggaatccgcctttctacttaaaggaaccaaaattaccctgactgacgaacgaaccgatcaggagcaggaagacgttttccattacgaagagggtattaaggaattcgttcaatatttgaatgaagataagcataccctgggcgacgtgatgtatttcgacggcaaaaaagacggcgtggaagtcgaagtggctgcgcagtataacgacggttattctgaaactatgctgtcatttgtcaacaacgttcgaaccaaggacggcggcacgcacgaggcgggtctgagaaacgcttggacgaaagcctttaatgactatgcccgaaaagtggggatgctcaaggaaaaggataagaaccttgaaggcagcgatgcccgcgaggggctgtccgtcgtattatcgttacgaattccagaagagattcttcagtttgaaggtcagaccaaagaaaaactaggcacccctgaagcccgctcaatcgttgataacgttgtcagtgagaagctgggctactatttgatggaaaacggtgaatttgcccagactttggttcataaagcgttgcgtgccagacaagctcgacaggcggcaagaaaagcccgggatgagacccgaaccggtaaacggcataaaaaacaagaacgcctgctgtcaggaaaattaaccccggctcaatcaaaggattacagccgaaatgagctgtttctggtcgaaggggattccgccggcggttctgccaaacagggccgagaccgaagatatcaggcaattttgccccttcgagggaaggtcttgaacaccgaacgggcaaaactcccggaaattatgaaaaacgaagaaatcaataccatgatttatacaattggtgccggcgttggcgccgattttaacattgatgatgccaactacgataagattattattatgactgatgccgatgatgacggtgctcatattcagattctcttattgaccttcttctacaaatacatgcggccaatgattgataatggcagagtcttcattgccttaccacccctttacaagctgcagaagggtgccggcaagaagttgaaagtccaatatgcttggaccaatgaagaattaaataaggtatcaaaggactttggcaagggctacagcctccagcggttcaaaggtttgggtgagatgaacgctgaccaactgtgggaaaccaccatgaatcctgataccagaactttgatccgggttcgaatcgatgatgccgccctcgctgaaaaacgggtgacgactttgatgggcgataaagttgaaccccgaagaaagtggattgaacataacgtcaaatttaatttagaagaagatggcagcatcttggataatacaagtgattagggggcgcgtttaaaaaatgagtaaaattgaaagtttgaccctcgaagatgtcatgggcgaacggttcagcagatattccaaatcaatcattcaggaacgggccttgcctgacattcgggatggtttaaagccggttcaacgacgaatcctttatgccatgaacaaagacggcaatacgtacgacaagccgtttcgtaagtcagcaaaatccgtgggaaatgtcatgggtaattttcatccccatggggacagttcgatttatgaagcattgaatcgaatgagccaggactggaaggttcgcgagccgctgattgaaatgcacggcaacaatggttcaatggacggtgatccgcctgccgcaatgcggtataccgaagcccgtttgagcaaaatcgccagcgaaatgctacgggatattgaaaaggacacggtcgactgggtcctcaattttgatgacaccgagtacgaaccaactgttttgccatcccgatttcccaacctgctcgtgaacggttctactggaatttctgccggctatgcgaccgatattccaccgcacaacctgggagaagtgattgacgcgattctttacctgcagaagcacccggatgcaactctggatgatttgatgcagtttgtgaaggggcccgatttcccaactggtgcaattgttcaaggaattgacggcatcaaaaaagcatacgaaaccggtcacggcaagattatcgtccgctcgaagacttccattgagccactgaaaggcaacaaatcacaaattgtcatcacagaaattccttacgaggttaataaggctcaactagtcaaacggattgatgaaattcgcttgaacaagaagatcgaaggcatttcggaggttcgtgatcaaagtgatcgtaacggactcagcattgtcgtcgaattaaagcgtgatgtcgactcaaaaggaattttgaactacctgttcaagaataccgacctgcaggtttcctacaatttcaatatggttgccatttcccatatgcggccggaacgtttgtcactgaaaaagatcttggtggcctatctcgaattccagcaagaagtcattgagaagcggaccaaatacaatttgaagaaggctcaggaccgtcagcatatcgttgagggactgattcatgccttatcaattttggacaaggtcatcaaaaccatccgagcaagtaagaaccgtaaagatgcccgtgacaatctggtcaaaacctacgatttttcagaaaaacaggctgatgccatcgttgccttgcaactgtatcgtttgaccaataccgacgtgacagagttggagaacgaacaccagcacctggccgacgaaattaccaaagacaacaaaattttgaatagtccaaaagaactcaatcgggttttggccaacgagttacgcgcattggcgaaaacttatcgcagcgctcggagaaccgagattcaagctgaggtttcagatatcaagattaatacagatgtcttgatccctgacgaggatgtgatcgtgatggtcagccatgacggctacatcaagcgaagcagcattcggtcatacaaagcttcgacaaccgacactggtttaaaagatgaagattatccaatctttatggccgaattaaatgcccgcgatcatctgtttatgttcaccaataaaggtaatctgatctatcggccagtctttgaattggcagatgtgaagtggaaggataccggtgagcatatttctcagaccatcgggttggatgctgacgaggaaatcattggcacctatgcttttgattcactcaagcaaccaggaaccttcttgattgcaactgaccaagggcatgtcaaacaaactggttttgcggatatgaagccgggacggacctacaagagccatgcctacacttatgagaagctcaaaactgctgatgagcgggtagtggccattcattatttgaagacgcccgcaactgctgggcaaatgcttcttatctctaataatggcttggcgttacgctacgggatcgatgaggtaccggttaatggcgccagaactaccggcgtaaaatccatggggcttcgaggtgttgataaagtcaccaacctccaactggtctctgaagacgatgtcttggcaattgtgacccaacgtggatctttcaagaaattagctgttaaagaaattcctgccacttcaagggctcgaaagggcgttatgatcctgcgggaacttaaaaataatccgcacagaattgtggacttttgtcgaattgaaagcgaagaccagccgcttgaagtgcggaccgatcatcgccgggttcacgatattttaccggcagattattcattgggtgggcgctattccaacggctcatttgtaattgatgttgacagtgaaggcaccccggtttcaatcagaccaaagtttgtcggcttatcaattgattaaatttttaccatattaattgattgtattaacaataagaattatcataatagcagtatcctgttaattatataatggtcgcacggaccgataaggagagtctgaatgaaaaccactcaggaaaatatttttgcatcaaagactttatcgtattttctccagttgtcagaaacgatgaactacacacaagctgcccagatcttgggaattacgcaaccagcgctgacccaacaaatcaagaagcttgaaaagacaatgggaactgaattattctactcggttggcaagaaattaaggctgaccgatgcaggtgtgatcatgttgaagacaacccggcaaatatacgatctgttaaatgatgccaacgaccagattcaacaagctaccagctcaacgactggtcaaattaatctgggaatcctcgcttccgttgaaaccaaagtctttgaagattttgccctggcactttaccaggaaaatccggatttggaagtcaatttccacatgctgaccagaaaagagatttgggaaagcttggagaacaaccgaatcgatttggcaatcatgtacctgccggatgaatcgattaagaactggaagccatacagctccaagaagattatctcggatgacttattgtttatccaccacaacccaagtttggccaaacgtaaacgggtccacttgaaagatgtcaacgacaggccatgggtgatgtatccacaagattattatctcaaccaaactttgcgggaatcctttaagaaccaaatggttgactggccaaaggtagcggcacgatataccatgcccgagcagattttgaagtttgccattaattcccacaccaacacggcattaccaaagtcatatatgctcaatatcgaccttaagaagttgactgacgatgacatttgggtcactgaattggatcctaaagtcaagtttgatctgaatttcgtctaccggaaccgcaagaacgaaatcccgcggattgaacgtttcttacagaagttcgatgagttccttgctaaagaagattatttagcccgtttagggaaataaattttgattatcaaaggagattatgtaaatgagtaaagaattagtttttggtcatcaaagtcctgatacagatgcaatcgttgctgcaaaagcctattcatatctgcagaacaaattagggtatgatactgaagccgttgctttgggtgaacctaattcagaaactgcatttgtgttgaattattttgacgaaccaactccacgaatcatcaaaactgctaaaaatgaagttgactccgtcatgttggttgaccacaatgaatttcaacaaagtgtcagtgacatcaaagatttaaccatcactcacgtggttgatcaccaccgaatttctaatttccagactgatcagccactatactaccgcgccgaaccagttggctgctgcagcacgattatcgttaagatgtttgacgaaaacaaagttgaaatccctgctcaattagccggcttaatgctttcagcaattatttcagatacgttgttactgaagtcaccaacgaccactgaagaagataaaattgctgtcaagactttagctgaaattgctgacatcgattacgaaaagtacggcattgagatgcttaaagctgggaccaacgtttcagcaaagacggaccaagaactcattgattctgatgccaagtcatttacaatgggcggtaagagtgttcggattgaccaaatcaacgtcgttgaattcagcgaaattgacaagcgtaaaaatgacattgagaatgccatgaaggctgaagctgctgataagggctacgacttgttcttagttctgattactaacgttttgaacagcgattcaaagatgattgttgtcggcgaaccagcatctgcagttgaaaaagcatttaacagcaaactcagtgacgacacaatgtcattaccaggtgttgtttcacgtaagaagcaagttgttccgccattaacagatgcattaagctaattcatcaactctttcaaacggtccggctaatctgaatggttagtttggccgtttttgtttactttgggttggttggccactataatgaatttagtttagttgtacacaacctaatttaatggagggttatcatggacaagcaggaactcaaaaacaaactaaccccggaacaatacgatgttacccaaaacaaagggactgaggcgccgtttagcggtcagtatgatgacttttaccaagccggtatttacgtggatgtcgtgagcggagaaccgctgttctcatcgaccgataaatatgatgccggctgtggttggccatcatttaccaaaccgattgacccagccaatattgataagcacttggacacttcttttggcatgattcgcgaagaagtcaaaagtaagcaggcgggttcacatcttgggcacgtgttcccagacggtcccaaagatgctggtggtcaccgattttgcattaattcagcagccttaaaatttattccggttgccgaattggacgcaaagggatacagtaaatacaaacaattatttgaataaatgaaattgaggtgcaatgcatggaagatacagcaatttttgcaggtggatgtttctggtgcatggtcaagccatttgacactattcccggtattaacaaggtcgtttccggctatactggcggccatgttcccaacccaacttatgaacaagttgccagccacaccactggccatactgaagcggtcaaaattttctttgatcctgaggtaatctcatatgataagttggtggaaatctattggcatcaaactgacccaaccgatgccatgggccaatttcaagatcgcggtgataattatcgtccggtaatttacgtgaaggatgagcagcaaagaaaaattgccgaagcttcaaagaaggccctcgccgagagtgaacaatttgacagtccaatcgtgacccaaattgaggatgccaaaccattctatccggcagaagaagaacatcaagaattctacaagaaaaatccgctccgttatcaaatggaagaaatgggcggacgcgaaaactttatcaagaagaactggcagaaaaattagttagccaaggatatttcagctattaatgaccattcacctaaagggctgtgacaaaacgcaaattttgccaacagccctttattattttgaattaaactgtaaggagaaatcgtcagatgatcaaatggtcaaataagacaatcaaagcatttcaggagacgctactagcctggtatgaccaaaataagcgggatttgccatggcggcaggatcaggatccttaccatgtgtgggtgtcagaaattatgcttcagcaaactcaggtggaaacagtcattccgtattatttacggtttatgaacgaatttccaacgattgaagatctggctgcagccccggaggacaagctgatgaaagcttgggaaggactgggctactattctcgggccagaaaccttcaaaaggcggctcaacagattgttttcgattatcagggccaatggccaacgactgcaaaagagcttcaggaattgagcggtatcgggccttatacggccggtgccattgccagtattgcttttggccaaccagtggcggcagtggatggaaatgcttttcgcgtttttgccaggctgttagaaatcgacgacgatgttgctaaaccacacactcgtcaggtatttgaaaaaataatcaacccaatcgttccaaagaatcgaccaggcgactttaatcaagcaattatggatttgggtgccagctacatgacagccaccaattatgataccagccaatcaccggtcaaagatttcaaccagtcatatttggatgggatcgaagaccattacccagtgaagaccaaaaagaagcgaccggttcgccacgattactttggagtggtcatccattccaaggcggggtacttatttgaaaaacgcccgagtcatggcatcctggccaatttttggatgtttcctttatttgaccgcaaaaatttaactgatgaccaaccggtgacagaatcaacgttaattgatataatcgaaacccgactgcagaccgattaccaactaagtgtcgcgttgcatccagtatctacgccaacggttgttcacacctttacccatcagcaatggaaaattaagttattggaaggccaaatagcggaaaatattgatttaagctattttccgggtaaatggatccactccagtgaatttgatcagatgacattttcgaaagttcaatcaaaaatgtggtctgcctatcagaaaactttaaaatcaactcaatcaattgatgagtcagctgtggatcagaaaacaaatcgatgaggaatgctgtggcaatctacccacgaattcttttagtgacgctgcttgtcacgatgaagttcatcaagggcttggcgttgcttggtgtcaatgatgtgcgtgtataagccagtcgcattggttgaactctggccaagctgagtggccaccaagtgctcattgttggtttccaaatagagcttcgaagccaatgtatgccgtaacttatggggtgtaatccgtacgtggttgaaagattgggagtatttcgccaccaatagttcaacagtcgcggtggaaattcttctgggttggcttgcccctttcgtcaaaaagagggcaggggtagtcttggtggccaaataccgttgcttacggacgtttaaataggttgccagatagggaagcacccaactggcaatgggcacggaatcgtacttgccgccttttcgccggacgacaattgccgctttgctcaaatttaaatcagagacatttgcattggtcagctcggacacccgaatgccagtaccaagcatcagcgcattgattgccacgtcacgttcacgatcgcgttgatataatgatagcgtccgtttattggtcagtgtcttgggatagtcattctggatgaattcaacgtatttcacatccgcgtcacccaacataagttgatccttgatgttgttggcacgggtttggtaggtttcgctgtcgggaaccaaggcaattttcttcatcacatttcggtaaaaataaggctcaccatcggcagtttcggtttcttccgataagtatcggaagaaggctgagagcgcgtttagcgaacgattgactgtccgatgagaaattggtgcttgcggatgggaagccgtttgcttgccacggttcagcaggtaagacttatacagttccatatcctgttttttgaagtgttccagcgcggagagtggaatttctttgacagttttcacgtcagtaatcccaacatcgatcatccaagtgaagaaacggtgaaactcgtttagatactgatatagcgtggcgggggataatggaaccgttgatttgtcgagataatattcattaatataagttggcagggtttgaaccagctgttgattttgttgaatatattgagatgattgcatttttaagctccttaattcagttaatcatatcccagcaaatcgcagtaaatttggtggggccgtttatttttttgcgtataacttaataaaatctgtattttattaagttaagtatatcataaatgagcatattaattgacccaatgttggaatcgattaatattaataagtgaacaatccaatttgaaagaggtttagatatgagatcggatttttgattaaggaggttctaaatatggttgatttaaaattaattcatcaagttcaactgggtattctggcaaatgtggcagcaatcaattctaaatatcatctggaatattttctaaccggtggttcagcaatcggtgccgtgcgtcatcacggctttattccatgggacgatgatattgacatcggtttgccgcgcactgattttgaaaagtttctgcaagtcgcaccggcagagttgtcacatcgaggatacttcgttgaagagaaccgcctcgatccacagtacgaatacgatttcgctaaagtgatggctgatggcacgcggatcttggaacatggccgtgagttgacaaaagctaagaatggcatttttattgatgtgtttccgttcgatcgaatgccaaataaacggccgcaacaggaaaaacagcaagcaaagttggcaatgctgttagaagagattcgaaagcgattttatcctgacctgtatcagcaaagtatcacacagtccaagtatgccgattataatttgagtgagctatacgatattcgactcagcacaatgacccaatataacggtcactcggaattaccgttgattaacatgtcatcaccgtatcagtacggaaaagaattaatcaagccgacagagatccatcatttaatcccaatggcctttgaaaatttacaggtgccagtcctagcagattatgatgcatacttaacgcgattgtacggtgactatatgaaattgccaccgttaaataaacgcattcagcgtcacgttttaaaagtacgagtggataattaccaaacgaacactcaagttgaatccggaaattctctggaagaagccgttagttaattgttcacgaaattaaagtaaagaaccagttaccattgccgagagtgttggctttggtagctggttctttttactttttgtctacttcgtataatatatattatgtaaagtagaatctgtatcaagaaaattgagtctgcaccccgcttctctgatacgtatctaaataattttattaaaacgaatcacgtcacttcgtttaacaaattttagctgctgccaaaatgattggcctgcaagattatctttcatgacattgacaaagattttatgaataccgacagcttggagctgttcaatcactttattgaccagttgagttcccaaaccttgattctgataacccggagcaactgccaaatgataaatcgtcccgcgccgaccatcagttgcacccagaatgctgccgatgatctgtttgtcagtcttggtctccgctacaaaacagaaattgggattgaatcgcaataatcggctgatttcttcaaaactatcgtcaaattcccgcagattcatgccgggaacttgttgccacaatgcataagcatttggataatcttctgcctgcatttttctggtgataatttgattgtccattgtgttgaaccttctttttaaatgattgtatatgccaataaccggttttgcctgagtcttttcttaatttgaatcatctatttgtatatagcaacaatcataatctctcattttaacgatcaaattagtgcaaaatatggttgaaactccgccggggcctcccgccttttcagctgaaatactggcagctcaggccgatatttggtatgtggttcaatcgaggagaaccagtagcgaaaatccaggtgttgatgagcaccctcgtctttttgcggattagctggaatatcaatgatgttgacatcgattaacgaatttggactagtttttaaaaccaaaccggtctcctcggtaaattctctgatggcacaatcaatcggcatttcgtgtggctcaacgtgaccggcaggcaataggattgtatgcaggtaaggatgccggataaagatccccttgcctccttcaaagaccatcgcacttgcggatagatgaaatggcgatttccggtcgcgaagtccttgagagtttgccctcagcaattcgatcgccgtttgcactttttgggtattcatccagggatacggctgactttttagcgttacgatttgggcgattaattgttcaactaagatggttgatcacttccttaatcacttaaaatgtccttgaagatctgatacgttttaattaattcttgggtttctttgacgttatggactcggataattcgcccaccaagttgggtcatgtaagcttcaaacagtaatgttgggatcagccgctcatctgagcctgcatcaaacagccgtttggcaaaacttttctgagaaattgcgatcatgatcggcgctccaaactggcgcatctgttttgtgtaacgcattttaatcaaatcaaattccagtgtattgcgatcagagaagccaaccccgggatcaataacaatgttctccctttgaagaccagcttgttctaaacggttaatcgagcctgtgaaaaatgaatgcatcgtgtcttcaagtgtcgttggttgttcgtcaaaattgcgaccattaaacatcgtgacgactgagggttgatattgttgaaccaaatccagtttggcttgagaattaaagccatcaatatcattaatgatctgaattccagattgcaacgcccgttcaatcactgagttggtattcgaatcgattgccaatacaatatttggaaaccgcttttgaatcgctttaagatagggttctacccgctgccactcttcatcgggactaatatcatcaaaatggggcttggacgatttgccacccagttcgaaggttttggcaccatagcccatttcagtttcgatgcggtccaaaacttgatcaatactggtattgaccccaccatcgtaaaatgaatccggggttaaattgagaatggaatagataatcggcgtttcagtcagattgaaatcaaaattcttccctttgaaatggacttcattagaattagtcatttgaattgctccttgtctttattaaataatctcgaattgggttgatgagataaaatgaacccaccaccaaaatcagctgatcggggtgattgcttgattccttgaggcttgccttaagggcagctatcgggtcggaaaaaaccgggtaaatcttgccagtaatgttttggaagaccgtttgaagacgacgttcgtccagcttgcgctctggattagcaggttgcgttaatttgaaggttgcattgggaatctgtgccagtaagcgcacattatcgacataatctttatccttcagaaacccggtaataatcaatttggattggctggaaaatgaatgtttcacggatccaacgaaagctgtgatcgcatcaacattatgagcaccatcgatgatgatcgtcggttgagcgtgaatggtttcaaaccgaccagggacatccagctttcccagcgcttgggttaataattgactgacatccagtgataagtgctgctttttttgaaaatcatccaaccacaacaacacggttcggacattttccaattggtaatcgcccggcagtccaaattgaaaatgaccagattgatgaccgacttgataaacgacattagttgctttagttaattgccgatcaatttgaactgcgtcggcatcaaggaaagtggcagctttgtggctcgcttcatctttcaagactgccaggacttccggccgttggttgggggccgcaatggttgtgttcccttgtcgaataatttttgacttggttgtcgcaatttcttcaatggtatttcccagaatgccaatatgatccatgccaattttagtaaagattgaatatatggttgttttcactgcattggttgcgtcgagctccccacccagaccgcattccaaaaccacatagtcaacttgttgatcagaaaagtactgcatggcggcaacaaacatggcctcaaattcagagagttcctgctgtccatcaccaaatgaagtcatcagctgcttgaggcgattcagatacttatcaaattgatcagttgggattgcctggcgattaatctgaatactattggtaatatcaccgataaacgggctggtaaataaaccaactcgttttcccatctgctggagtattgcggcaatcatcgttgccgttgaccccttgccgttggtaccgcagatatggatgattggatagtcagcatccgggttgcccaattggcgcagaacttgctttaacaaaccaatgcgatcaccttgattatataaaaattcggcaaagtgactggttaaatcatcgttcatatttgtcccacctggattgaattcaaaaactcacttctcagctcatcgttttgctggaagacaccggtaaatttagtggttcgggtcacggtgccggtttttttgacgccccgcatttcgatacacatatggcgggcatcgacaattaccgccacgcctttgggatggagaattttttccatttggctgagaacatcatccgtaattttttcctgcagacttaacttgtgtgatacaaaatcaaccagtcgcgggattttacttagaccaataattttaccgttatcaggaacataggcaacactgactttgccccaaaatggcatcatgtgatgctcacacatcgaataaaatggaatgcctttcaccataaccgtctttgagtcatctgactccggtgagtcaaacaatttatagtcttgaaaatcttccagtccgatagaatcaaagatgttggcatacattctggcaacccgatccggggtttcaataaggccctttctagtcgggtcgtcaccaattgctgccaatacgttagtgacgttactggtgatttcggtgtagaagttattagccggactgattttcttgattgattgatcatcttgctggagagacttaatggccgtagcaatcttttcagcgtctggaaattgttcatcaattaattcttgaatcggaatcaacacaaataatcgattaaacgcttcgggatgtggaaccgacagccctggttgatcaatttgttcattgccaaagaagataatatcaatatccacggtccttggaccccagtgaacctggcgagttcgatggaggccactttcgatttcatgaatcacctttaagagtgtcaggggttcataggtggtcccaatcttgacagctgtattgacaaatgcccgttgcttgacaccaccaaccggagatgtttcgtacagactggcctgcttttcaatcataatccgtgggtcactacccaatgcctcgatggcctgttccaaaaatgcctcgcggttcccaatattactgcctaaacttaaatatacatcttccatactaatgctccatttctatttcgacgtcgtccaaaacaccatcaatcggcgttccttgtttgcggatccggacattgacagtcataatccgcgaatcaatatttttaatagcggcaatcactgtctgggccaaggtctcaactaagtcaacctgattattgtcgatcaccttggcgatggttggatagaaatccgcgtatgacaccgtcgacttcaaatcatcatcagtcggatcggcatcgactttcacttttaaatcaatttgaatattttgaccaacgactttttcctcgggcaaaacaccaatatgactgtggaaccgcatgttgtgtaatgaaatgtaatacatcatgattcactcctttgtatacgacaaaaagcggcccgccgaccaatatgttggtgcggtgcgtcgcttctcattttatttaaacaacctgctctgaatattactcatcgtctgggaattcagcatatagtaaagaattgccatttgaatcggagtcatgaccaattcttttaacgctctaaccggtaaaaatgcccaaaatggcgtcttatataaaattgtcaaccaataggtattcaaaattgcgttgacgacaaccgcaatgattaattgggcaatgatcacgcgtttccatgtgatctctttgccatagaaaaaatagccataaatggcagcgcctaaaatcgcagagattgtaaacccaggaaaataaacactcccagacatcaatgtgccgatgatatccgttaatgcagcgattgtggatgaccacagtggcccatacagcatgctggcaatcgcagtgacaacgaagccgaaacttaaccgccaggactgaacaccgaccgtaaatcgaccgagaattaacaataacgacatgaaaattcccaagacaacaatatccacaacccgcagcttacgaaaacccaatgacaatgacttcatgatgcagcatctccttataaaggagctcaccattatttagagaactaaataacatagcgaatgcggaaacaacaccgcaaatggtcgacaagtcgaagccgatcatttttcgttcgaagttcacattccgttcctccgacacttaacgcattgaatcctaccccatatttattttatgtaactattaaagtttatcacatgcactaaaaaatgcaatcgcttagttcgtgttttactgaacaataagcgattgcatgttaaaatagttcattttaaatgttatcctgatcaaagtctcgaagccacgcaagagctaatgctttgtcgcctaaatgggtgccaatggttggaccaaaataactttgttcgattgtcatatcaggataaagttcgtgaattttatttgcccattcatttccggctttaggatcattgccgttaatgaccaatgcccgcaaaggataatcagctttttgtttggcagcagcaaagagttcctccactcgtttgagggcttttttacgcgaccggatcttttcaaaggcgacaatttcattacttttatcatcaaatgtcaataacggtttaattttaagaattccgccaatgaatgccgaggcatttgaaagtcggccaccgcgaaccaggttttgcagatcatcaacgacaaacagttcgtcaattgtctgccgaagcccatcaagatatgtaaggatctgatcgggcgtgcgcccaagtcgggccattttactggcttggatggccatatagcccattaacttaacggtgattttggaatcatatgggatgactttgatcccttcgatcgttggtgcaatttgagtcagggaactatagaagccagaaatcgtgctggcaagatgaatactaatcacggtgtcatagccttgtttagccaaagaattgtagagatcaatcatctcaccgattggcggctgagatgtactgggaaaggcctgagaattctttaacttatcgtagaattctgccgtcgtcaaatcgacaccttccttgtactcacggccatcgataatgacagggattggcacttcgataatgttgtatttcgcttgttcttccttggttaaatacgccgtgctatcagtcacgatcgcaattttcattaaattcacctgctcgtaattaaattctatccaaactcttttcaagacgattgatcaatatctttaaaagatttttctcttcatcagtccaatgattaaatacccggtcagtcagcttttgaatttcggcggcaacatattgactggcctgagttcccttgtcagtcaccttataaatcaattgtcgcttgtcccgaccaaccgcggtcttttcgatcatatctttttctaatagtcgcttcaactgccgcgacaaggttgaaatatccaatttggtactttcggacaataattcctgggtggtattgccggcaatgacttgatttaacaacttccattcagaaattgtcaggttcattgccttagtaatattgaatatttgagatcgatgatttttggcagcagaattaagtgccacaagaatatctttcatgatgaaaagacctccgaaaaattagtatacgctatttgataatgacatacaaataacatgtgccttccttagcatcagtcaagaaagtgcgctatactagtacatgctacttatacgaaagtgagtgataagatgtcatttgatggttcttttacccattctatgaaaaatgaattaaccgatctgctgcaaacgggtcggatcagcaaaattaatcaaccctatccgaatgaactcatattaacaatccgagctcacggaaagaatcaacagctgctgctgtctgccaacccgacgtatgcccgggtgcagattaccagggttccatatgtcaatcccagtgtgccgacaaactttacaatgattgtccgtaagcatctcagcggtggaattctcagtgagatttcccaacaggaaaatgatcgcgtgttgacgtttaccttcacggcgcgcaacgaactgggtgaccagacaaaattagatctggttgtcgaaattatggcccgtcatagtaacatcatcctggtcgaacaagccacggggaagattattgacgctattaaacacgtcggttctgacgttaaccgatatcgcctgttgctgcctggagcaacttatatcaaaccgccgaagcaggacttggaaaacccatttacgatgactgactttgaccgggtccgccaattgatcaaagattttccaaacgtggacgttttagctgaaaatctacggaaaacaattcaaggattgggcaacgacacatctttggcattagcaactagtttgcataaggacgagaaagttgagactaatttcaaggatttcttccaaaaattcgactcaccagagccaacctttagccatgttgcaggtaacaagattaattttaccgcatttccctatccgggtacaactaaaaatcaaactttctcaacattgagcgaattgctggatgccttttacgccagcaaagcccaaagagaccgggtcagagaacaaggcgcggtgctgattcaagtcgttaaaaaacagcttaaaaagaatcgcacgaagcttaagaaactccagcgggatatgaaagacaccgaaaatgcggatgattatcgggtcaagggcgagattttaacaacctatctcaacaaagttcaacgtggaatgaccagcattgaactgcccaactactatgatgaaaataaattgattaccattcagctttccgatcaacaatccccttcccaaaacgcccaacgatatttcaagaaataccaaaaattgaagaacgctgttaaatttgttggcgaacaaattcaactgaccaagcaggaggttgattacttcgaaaatattcaatcccaaattgaactggctgatccccaagacctggtcgacatcaagtacgaattggaacaaggtcattatctccgtgatcatgagcagaacaaaaagaagaaaaataagcgacaaaagattaacaaaccagaaaagtttgtcgcaagtgatgggacagaaattttagtcggtaagaataatctacagaatgaaaaattaactatgcataccgccgacaaacgtgatacctggctgcataccaaaaatattcctggatcacacgtcattatccgcagctttgacccgtctgagaaaaccctggcggaagctgccaatctagctgcctatttctcgaaagcgcgcggatccgccaaagtacaagtcgattatacgaaagtcaaaaatattcgcaaacccaatggtactaaaccggggtatgtcatttacgataatcaaacgacattgttcgtcacccctgatgaaagtctaattgatcagatgcgaaaataagcgggtgagtaatctgctttcaatttccggcatacaaagaatgcgcaccatatataaggagcgtcttcttaacattgtcagtggcagctgtttatcacactatttagcttgctaatatttagaatacacaaagggtcggggcaaaagttactattttgccccgacccttttgtcgtaatcttattcaaaattcttaaatgatagtgatgaaccgacttcttgcttagtggttccctcaatgcgactggattggagttctctgaaagggaaatgagcagtcataatcgatgcacgtttgtgctccgttggcttcaagtcttcccgcaaggcttccatatccaatgtgtgcaggtatttacggaccaaaacgttaatccaattaatcccggtcgttttggtgaggaaggcggtctcagtaattcgtacaggccgaatgccagtcatctcatatttagaatcaccagttgtattatacaagacttgaaccagcccctgccattcttttggatctaccttgttagtggcatcagcaatcaattttgcttcgtcagacttccagttatccatcggctctttatagtcgttaataaaccgcaggtcagtccgttgatctttccccacaaaagaaatggtcgtcacgggtaaaatttcatcgccttcgatgaacagatcgacagctgttgttgcatacttttgattgtatgtggcaactttttgatccggcggcaaaacgatgatattaagattttgaaattgttttaactgtttagacaagtagtgtcggttccctgggagaatgacgacatctggtttctccaaattaataatgttgagaatatttccgagttggatcggctcaatgtattgtttgtcacttaactgtggcgttagtgagacggcattcggatttgtgttcatgataattgttttatagcctgacttgtgaagcgccctgagaatctgtgaggtgtaataatccgctgccgaattggggccgagttggttcccaccccgaccaatcaccaaagcactcttttcttcaaatggccggctttcattttccaattcataactgctgtaaaaaatattggttgattccagcatctcaccggcgctcggctcaactgccttgtaagtgacgtgattctggtagttttcgttcaactgctgaatctttgaaatgttgacttgccataattcagccagcatgccgtcaccaaaaccgtatttgtgtccaatttcaatggattgcggtgacattgggttattgacaacaaaatcctgagctctcaataattgattcaacttgtagaaatagaaacgatcaatttgagtcagttcagatagctcatcaattgaaaagcctcgccgcaatgcttccattaaaattaatattcgactggccaatggatgaatgagttgattaatgacctcgtcatcattaaccgtcgacacgctgggcaaaatatcccgtggtgaaaactgggaactatgcatggatttaataattgcttcttctactgtccggccaattccaatggtagatccaaccgatttcattaaggtgttcaaatgctggtcaacgtccgtaatgtctctaaacggccataatggaatcttaacgaccacatgatccatggttggctccatgaacggcagaaacttgttatatttactcggtaacttgatttcagtcagattgtaccccatttcaagaaagcttgagacgtacgttaaggggtaccccgttgctttggcagccaagatggtgtttctggtaaagaacggactcaccttggtcacaaaatagttggcatcggttctggactgcgcgaattgaacatgacaagttcccgtcacattcagagcatccataatgcgaaaagttgctgacctgagcgcttgatattcttcattaatcaaagtctgcgttggagcaaaaatgattgaatccccagaatgaatcccaattggatccatatcttccattcccgaaaccagcagcttattgccgctttcatcgcgaataccgaccatttcaatttctttgtaacccacaatactctgttcaatcgagcagcgcttgatgtaggctcgcttgaaactcacgtccaaagcatcttctaattcgtcagtattattacaaataaaccgactggtatcatgacttgatgacatcggtttgacaatcactgggaaaccaacctcacggacaaagtccatggcttcgtcgtcatcggccacaattttcgaggcaatgactttttcgttaatttcggttaaagtatcacgaagtttctgattgtccatgaccttccgcaaatcagccggcttgatgcccaagagtgaaatattgttagaggccaaaatgccactttcagccagctgccaagcaatttgcatgccattaagcccgccagtggtcgccataatggcgtccggattttctttatcaataatgttgacgatattttgaaaattgacctcttgaacatacacattggctggttgaatttcttcggtggttaccgaaaatggattgttatccacgtaaataatcttcgcaccggtctttttgagcgccatcaagcgttcaaaagcggctgcatcaagttcattttcatggccaatgttggttgggccaccgccaagcaggaggaccttgttaatatctatcgtcattgctgtcccttcttcttgccatgatttccataaagtcgtcgaacaagccaacactgtctttgggccctggtgccccatctggagaaaattgaaccgaaaatgcggggtaatctctgtgccgtaatccctgaacagtgccattcaccaaatcgatgtgggtgataaacagtttggcatggtcaattgattttggatcaactgcatacccctgttcttgacctgagaaaaagatctcattggtgataatttcccgaatgggatgattactgccgtgatgctcaacggttagttgggaaactttagcgccattggcaagtgcaaacagttcatggcctaagcccatcgcaaacaatggcgcctgcgactgaacctctgtaatcatgtctaatacagattttggtaaattctccggcgaacctggaccggtcgataaaacaatgccatccggatccaaatccaaaatttgggcggcggaaaagttccaagggaccaccgtcacgttacagtcacgatgggataactcccttaaaatgccgctttttaagccaaaatcgactacgaccacgttggcgccttcatcagggttgggaaacggcttgggagttgccacttgagcaacttgttgatttgtcaaaaccgtcgcgtgcagctgatcaaaagcatgatcatccgcgacgtcgacaatgcttgctttcatattgccgcgcttctgtagatgatgtctgatttctcgggtgtcgacgtcataaattccggggattttgtgttgttttaaatatttatccaaagaaatccgcttaaagtggtcagtcgccagattttcgtactccctgacaatgacaccttttgcggacggcaaaatggactcgtacgcattctggtcgagtccggtattccctatagatgattgggtaaaaacgataatctgattatggtaaatctgatttgaaataatctcttgataaccgttcattgttgaattggcaacaatttcacccgtcgttgttgccagtgatccgaatgcctttccagcatacgcggatccatcttctaaaattaaatatctttccgtcatgctgactcctcgcaatgagaattatttgatgagttcaacagcatccttgtcatcaatttctgaaacataaaccttaatcttttccttttgagaacttgggatattcttgccgacaaaatcggcccgaattggtaattcgcggtgtccacggtcaaccaaaactgccagattgatactcttgggacgacccaagtccatgaccgcggaaagggcagcccgaacagttcggcccgtgtataaaacatcatctaccaaaataacccgtttaccttcgatagaaaagttaatcttgttattggacattttgacatcactgctcatggcatcgtgttcgatatcatcacggtagttggtaatatccaattcaccgacaggaatcgaaacattttccaattgttggagccgatcggcaattcggtttgccaaaaagattcctcgggtcttgataccaattaagactaaatcttcaacacccttgtttttttcaacgatttcatacgtaattctcgttaaggcccgctgcatagccattttatctagtattatctttcccattagtaaaagctccttaattgagtaacgtttgtacctgatgattgcataaaaatgctataccacttcagaatatgaaaacagcgccggattgtcaagatcctagagcgttgtttaatcgtaaattattaagtgtttgttcaaatattggtggcaggggcgccgaaaagatcatcaattgatgcgtccgggggtgttcaaatcccaactcctgggcgtgcagaaactgtccattgccacgaatggtttttcttggcccatataaaggatccccaacgatcggatgcccgatgtatttcatatgaactcgaatctggtgggttctaccggtttccagccggcaggcaaccaaagtgtagtcagcaaatcgctccaacacctcaaaatgcgtcacggcacttctgccgtccgaaacaactgcctgcttttttcgatcctttggtgaccggccaatgggcgcgttgacgactcctgaatcttccttaatgcgtccatggacgagagcaacatattttcgcaaatttttttgggctttcaactgctgtgacaaaaactgatgtgctttgtcatttttggcaaccatcaacaatcctgaagtatccttatcgattcggtgaacgatgcccggccgaaactcgccattaatcgttgacagtgggctatggtacaacagagcgtttaccaacgtgtggtccggatggcctggggaaggatgaaccaccatcccctgtggtttattgacaacaatcacatcatcatcttcataaacaatatcaagcggaatattctccggttcaagactgatcggagtcggttgcaccgaatcgacctgaattttatcccccgacttaacttgatactttggtttgactggctcaccattgaccttgagatgttgatcgtcaattaaattttttgcccgtgaccggctgattgaagaatcaagttccgagatgactttatccaaacgtccagtctggttggtaataatatactctttcaaaataattgttccccttaatcaactttcacggatgattgcaatggccaaaatcaaaattccaaacgtcaagtacatgtcagcacagttaaaaatcggaaaattgataaagtcgagttgaaacatgtcgaccacgtgattgttcatgatgcgatcaatgacgtttcccagcgtaccggctagcaaaagccccagaccaattcgatacggcatatttgaccagtacctcacaataaagtaagtcactaagattgccgctaaaatcgcgatgatcacgaaaataaattggtggccggataaaatgctccaagcagccccggtattgttaattctggtaatcgacaaaacaccgttgatcacagaaaatgaatcacctaatgccaaactggcaaccaccaagtgtttaacaatctgatcaatcgcaattaaggcaatgattccgataacataaagtactggcaaaataaacgctccctttagaacagcccggtaatccgaccctgttcatcaatatccatgtcgagtgctgcaggatgagtcggcagccctggcatggttaaaatttttccggttaaggcgacgatgaagccggcccccagttttagttgcagatctgaaacatggattttgaaattctcaggtgccccaagctgcttggcgtcatcagtaaatgaatactgggttttcgccatgcagacaggtaattgatcgtaacccaactttttaattcgctttaaagcagttttggctttatttgaaaattcaatcccatcacccccataaatttgggtgacgattttggccattttgtcctctattgaatcatcatcgttatataattcgtggaattcggctggccgttcacaagcttcaatgacatccttggcaaggtcgactgcccctttgccaccttcagcccagctgttgatgatcgtcccagtaaccttcaaatcattggtgacatagttttgtaaataagttaattcgtcttcggtatcagtggcaaacttattaattgcgacaaccactggtttgccgtactgctgcatcccttcaacgtgacgtttcaaattgacaacgccttttttaagagcctcaagattttctgtgttcaattcatgcttatcagcaccgccgttcagcttcaacgcacgaactgtggcaacgactacgacgcaatcaggactctgcttcagccggggtgtgacaatatccatgaacttctctgcgcccaaatcagacccgaaaccagcctcagtgatcgcataatcaccaaaatgcaaagccgcttgggtcgccaagatactgttacaaccatgcgcaatattggcaaatggaccgccgtggataaatgctggtgtatgttcgatggtttggaccaggttgggtttaatcgcgtctttaagcaataaagtgagtgccccttgaacgtgcaaatcagccacggtcactggttgccggtcgtaagtatagccaatcaacatccgactgatccgttgcttcaggtcaggcagactggttgccaggcataaaatggccatcaactcactggcaacagtaatatcaaaaccgtcttgacgcggcacaccggaggttctcccaccaagaccgatgacgacctggcgcaattcccgatcgttgacgtccatcacccgtttccaagtaatttggcgcggatcaatgtttaattgattgccgtgctgaatatggttgtcgattaaggcggctaatgtgttattggcctcagtcaaagcatcaaagtccccggtgaaatgcagattgatatcatccattgggacaacttgagcgtagccgccgccagttgcgccgcctttcatacccatgaccggtcccagtgatggttcccgcaatgccagaaccacctttttatgtaattcgttgaaagcatctcccaatccaaccgtcacggtggttttaccctcgccggcagcagttggattgatcgaagtaactaaaataagcttgccatttgccttttcagtggttgggtcaaaattgatttttgctttatactgaccatattgttcaatttgatcttcagcaatcccaattttttcagctatcttggtaattggttccataacagtttcttgagaaatttcaacatcgctcttcataatgattatgaccctcctaaataactatcgactgacaacggggcagcaattacttgttggaaatcaattctttgatctcaataacggagttggcgggtaaaatgaagctgtagatcttggtgttggcgacaaaggccagttggtatttcgaggtctgaacatgtgaaatctggtccagatcaacggttaaccagtgaggattcgtgatgcgactgacgaaaaatttgtgatcgtagacgtgaatactgcgaaaatgaatttccgcccagacgatcaccgcaaacaacacaaagaaaaataacgtaatccactgaaaatgagtaatttccagccagataatcacgccaatgaaaaagacgacaaaagtccaactccaacaaataatactgctcaatgggcttggttgataaaagaagtgacgcttttggcttatcataaataaactccttaaagaaagtgtagataacatgattaaactatatacagacgcagccgtcaatcagcatactggacacaccgccatcggcattctcattgtcaacaatggcaaacaaattcaacttaatcaagtgattacgccaacggacaatcatgatgcagagtttagcgcagcaattgccggattccaaaaattgatcgacttacaaattgatcccagtgaattgatttttttctatactgacagcaaaatcgtcattgacagtctcaataaacaatatgccaaacatttcgaaaaacatctcgacaaactactgggactgcaaaatcaattcgcaacggtggtcaacacctggattccagacaaacaaaacatgggcgcgcataccctggcacttcaagcactgcattcaatctagtcaatatactggctgaccggctttgtgtaatcctgccagtgatcgatttcccgttcaaacactgcctgagcaagaagatagccaatcatcggtccggtagttaaacctgaggaccccagaccgccaccaatcaagaagttgggcaatgtcgggactgctccaaagaatggcgcaaaatcttcggtgtaggctctggtgccgacccgcatgtcactcacttgggcgtccgttagcgttttgataaatactttggcattgttgagtaactgtcggcgagcagctggctgaggcgttaaatcgaatccctcatcattctcgtgagtcgcaccaatcaccaatttaccgccattgaacgggataacgtcactactgccctctggcatcataactggcatatttcgccatttatgcggcatcttgacagttaaatcgattaattgtcctttctgcggccggaccttcacgttcaaccccaatggctgaagtgattcgtgcatcctagcaccggtggcaataatcacgatatcaaaatgtttgggccccgctgtcgtgttaatggcgccattcgccgtcaaggaaacccgttcatttttgacatccaaattattggcagccgcccgttccagcagctcggaaacaaagtggccgccgtcaatccgtgcgccaccactgacaaaaacaccttccggagcatccgtgagcaatggcatccggcgttttacctctttggcgtccagcaattcgacccggcccatcgcagttgtatgctgctccttgatcttggcctcctgataaagcgccaataggtcatcgtggttcttgcgagtcacaatcgtacctgtctgctgataggcttggttgctcaactgagcgtcggaaacgagggatgggtacaattctgcccctcgttttgccaacgcgtaccagcgcttatttctgcgctttgagagccatggcgagatgataccggaggctgccttagtggcttgccccgtgtcgtcgtcaaatagtgtcacttgaatattgtcattgccttgtaggaaactcaaataaaatgcgtctgttgcaccaataattccgccgccgattatcgcgacttgtttaaccatttacccacttcttttcaccaagttgttcttattttagcatatattccgacttatttgctcttaatttggtctaatttacgcaaatctcgaactttctttccccagaactgaaaatagtccgtccttattgatccattgtagagctttcgtcgtttggttgctttttccccatagtacttttcaaagtcaaggtccgaggttaaaaagtattttgaccaactcgtgagcggattgaagactttccccatttgtttgtataactcatgggcatgttcttcatcactcattcgttgtccatagggtggattgccgacaatcacgccgttgaccttatcagttttgaaatcggcaaccgccaattgtttaaactgaatatcagccagcaggccggcctcttcggcatttcgtttggaaatttcgatcatattgccgtcaatatcgctggcagaaatatcaagttcaatgtcatagtcagctttggcgtcggcctcatcgcgaactttttgggccatatcatgatcaatccaaggccattgttcacaaatgaagtcacgattgaaacctggagcaatgttacgaccgatcatggctgcttcaattggaatcgtccccgaaccacaaaacggatccagaaatggcatgtcgggataccagctggttaacatcaccagggcggcagccatgttttccttaaggggagcagaccctttttcgattcgatagccacgtttgaagaggcttgaaccggtggtgtccatggtcagcatcacatgatccttattaattgccacttccagtggaaattcggcaccggtttctggtaaccgggtgtggcgatgataggcagtgctcaattcattgacaatcgcttttttgacaatcgcttgagaatcaggaacgctgtgcaattttgagtttcgcgaacggccctcaactggaaaggcggcatccattggcaacaacttgtcccaggcaattgcagtcgtttgttcaaacaattcatcaaacgtttgggcgtcaaattcatcaacaacaattttgatccgatctgccgttctcaaccacagattggttttaataatatcttcttcattaccggtgaatcggacccgaccattttcgacctggacgtcatatcccaagtcacgcatttctttgccaactaaggcttcgataccggcggcacaagtagccattaaattaaatttcattttatctatctcctgcattttctgggtaacaaaaaagtgggagcaagctcccactcaacctgtttggtgtaaatccctataagccatgttttgtgcttattatatcccaggacgacataacaagtagtaatcatctatctgagaaatatcgaaatacttctcccccacacttggttcatttaccgtgtgtgaagctcccctaccaaaagtttgggtttcccgctcgaggggtttaccgcgttccatcagtaccgtttccaatactgttcgtcactgtggcaccttagggaattaaagcatagcaagccttagctttaatatccgccgtaactcacaaagagtcccccggcttattttttcaccgagcacgaacactacgggcatcgcagcccgtgcgagaatggactttcctcagccgtaatgatacgaccgcaattactcaggatttacaccatattagttatatgcaagctttaaagcctgtgtgaatcattggtattattatcaagttgtgatccgaatactcgtctttcaaggttggaaaggcgctttaaaatgtccatattagtcgcacttgacattggctgactcggaacacttctggttggagcagtgccaccagctgatggcattggctgcgaaccggataccgcaatctgcttattcaattcatcgacttgaacttttaatcgctcattctcatcactgagggactggagttctttgttgaaagtttcataatccttgatgatgtcgtctaaaaagccgtcaacatcgttgggatcatagccacgcatcttttgcttgaattccttttgaagaatatccttcggagtataattaatgttttccatgtatgggttacacctcactatttgcaacaaaccaactaaaataatatcataaattagtcatcttgaacactattattcaagttttcctgatattcatccgcagcactctgtaaatcgtcgaaagtaattagcttatacggatatggatggttgtcggcaaacctttttatttgatcataatcatattgcgatttccctggattatctaaatcatatatcaataatgcctgatcggtatgactcagcatgaattcttggtaatttcttaactgttggggcgactgatacggcttttgagaaactgacgccgaaaaatcgacccgtgcctttagggtctgcagcttggtttgattgttttcgttccaattactgccgaagtcagcgaacggcagcatcattgacgtctgaaattcgcctggataggtctttttcaaattcagggccatttccaacgaccactgctcaattcccaactgtccgccggaaattaaccaatccatgccgtcaacaattgcctggtcaatttcattttttaagaccatatcaatgacttttcgttttggatcatcatctttaaaaattcctaattcatagcttcgatagccggttacccacaagcggctcatgatatcaccctaacgattaaatattttaaatgaagactctacttggtataataacattattgtggttattattaagttaaatgaagtacaatataactattcacaaaaaggaagctaacgttcaatgactatcagatacccgaatggaaaccagtttcatgagcagccgacttcttccggtacccacaatgattcgattaacttctcaaatcgaggaatgaccttagaggacgaaatcaacaagagcaatcagtattatcttcgtgcaggaattgcagttattcataagaagccgactccaattcagatcgtttctgttgactatcccaagagaagtgccgccagaattaaggaagcttattttcgtcgtgcttccactactgattataatggcgtatatcgcggaaaatacattgactttgatgccaaagagaccaagaataaacagtctttcccactcaaaaattttcatgaacatcaagttgaacatatgcgacaatgcctacaacagcaaggaatctgctttgcgattatcaaattcatttcggatcaggccgtgtatgttttgaaagccaccgacttgattacctattgggacgcccaaaaaagtggcggccgcaaatccattcccagaaaagtcattgaaaaggaaggctttttgattcaatacagaattaacccattactaccctatcttcgcgcggttgattctttcatcgaataagttacgaaggagaaggctatgtcacagaacaatccgaaaaattcacgcgctgaagttcggcgcggacgacagtttagcaatacccataaaaaaggcccctttcggcgaatcttcaaatgggctttaatcctggttggtgtcctatttctgtttggcgccggcctattcacgtactacgcttccagtgcaccacgaattacccggtctgcgctgaccagtgataactccactaaattctatgatgccaacggcacagtgatttcacgtctgggaagccagaatcgggactacgttaaatctaaaaatattccaagaaccctcaaacgggccgttgtttccattgaagatcgacgattctataaacaccatggcgttgaccccatccgaatcgccggagcagcgatctcgaatttgaccggatcttctttaggtcttcagggtggaagtaccctcactcagcagttagtcaaactgtcggtcttttcaacggctgccagtgatcgaacctttaagcgaaaggctcaggaagcttggctggcaatcaaagttgaaaatcgttacagtaagagtcaaattttggaattttacatcaacaaagtctatatgggcaacggcgtctacggcatgcagacggcggcagaatattattacgataaaacgcttaatcacttaacgttacctgagttcgctttattggcaggtatgccacaatcaccaacgctctacaacccttataagtatcctcagtatgcgaccaagcggcgaaatgaagtccttgatgcgatggtcaagaccaaagacattactgaatcgcaagcccaagctgccaaaaataccagtgtcaaagcccatctttcagcgacccacgcgaaggcgcgaacctctgaaaagacttctaaatacattgattcttatttaaagcagaccattgaggaactcgaggataaaggctacaaaccaaacagcggcctgaaagtttatacgaatttggacatgagtgcacaaaagaaactttatcaggtaagtaataacgatccgaccattgcctaccccaacaaccgtttccaagtcggtgcaaccattgtcgatgtcaataacggtaaagtcgttgccatgcagggcggccgcaaaaccaaagtggcgttcggtttgaacagggctgtccaaaccggcaggtcttctggatcaacagctaaacccattatggattatggtccagccattcaatatcttaaatacccgacctaccagccggtcaaagatacgccgtacgtttatcctggaaccgataaatcggtctatgactttgataacaaataccaaggcacgatcacgatgcgaaaagcactggttgagtcgcgaaatatcccggcaattcgaacacttgaaaatgttggggttcctaaagcaaccggctttttgaaaaacctggggatgtcgtttagcaaaccactcgagattcaaaatgggattgggctctacatttcctctgaacagctggccgcatcttacgcagcctttgccaatggcggaacctattacaaaccgtacttaatcaacaagattgttcaagttaacggtgtgacccacaagtatcaccagcaaggcaaacgcgccatgtcgccggcgaccgcatttatgatcactaatatgctcaagggcgtgatgacagattctgcaggttccgggactgcagccaaagtgtctggtctttatgaagccggtaaaactggtacgacacagtatcccgacgattatttgaacaaagtgccggcgatgtcgacgatggattcctggttctccggttataccaagaactattcattagccatctggactggatacgaccatcaattcaaagccaattcctatgtcacttcggcacaaacatcaatcgcccaggaaatctataaaaacgtgatgggctatatttctgaagataaacccaacaccgattggacccagccaagtgacgttgtcgcaaccaaccgtggcggcaccactgagtattacgtcgccggttatcctgggacagtcaccgataatagttcaaatcaaacgaccagtggctacacaactgaaggtggttcaagttccagctcggcagttgtcacgcaaccacgggaaaatgagagttccagcagtacagaaagttccaacgagtcatccgcatccacgccatctgagcaaaaaccgagtggcgatggtggtaacgatgattcaaacagtagttccgcatcatcgagttccactgacaatggcggtacgacgccagacaatggtggcggcaataccaatagcaatgacaataacggtggtactgacgaaacccaataaaatcagcacagtccatcagagactttcgacaaacacatcatttgtcgagggcctcttttcgtttaccaatattttctgcgggcttccttattacggttttctgaatgccagattgaagaactgattgtccctttgactatgtacgaaaaaatcggctaaaagtttagccgatttcctaattgtttatttatctgaattacctgacaagttgataaacggaatttccggaccgtcgtaaccagttgaaatatcatccgaatgtgaactattccgattctttttggcggcttcaacctgttgtggggtctttaaatttttcttgtaccaagtactaatgattcggtccatataatttaaattataaacctgacttaaaacggcttccttcaacgccagttgaatcaattccggtgaataatgatcaatatccaaccactgactgatagactccatctcaatcggcgacaaagttcgaccaaattcttgttcaatactttgaaagacagcttggcggtcgctgctgctaacagtcttgggcttttcgtttactgacgcctcaggagaggttcccgtgggcttgaccaatgccaatttttcatacatcggcgtgaaatcgtaagcatccacctgctgaccctcaatcactacttgcgtaattttggtcagcttcttttcaatcatttgatgaaataaattgaacagctgctgttcagaataattcgtctgtgcttgcagatctgccatttccggcattggaactaccaggtcatgattccccttaatcaataggtaaatgaaaagctcctgattggtaaccccaatctgatgataatgttttaacagatagttgctgacagtagtttgcccctcatttagtagattgcgtgcataatcgtccattcaattcacctcgaatccaccaaaccagtgtttaatttcaatttatgggtaaattcggttaagcagtcttgggaatggaattgcctcacgaacgtggtcttcacctgttaaccaggtcagagcccgttcaagtcccaaaccaaagccggaatgcggcacactgccgtatttacgtaaatccaagtaccatgagtattctttaggatccaaaccagccttgacaatttgatcatagagatagtcgtaatctgttgctctttccgaaccaccgataatttctccgtatccttcgggtgccaagagatcagcacaaattaccacgtcatcacgagttggatgtggcttcatatagaacggtttaattgctttagggtagttgatcacaaaaaccggttggttaaattgatcggcaaggtaggtttcttcaggagaaccaaagtcgactccccactccaaatcaaagccaccctttttgagcatcgtaatggcttcatcataactgattcgtggataaggtaaaacggtgtactttttgagaacttccgggtcgcgacccaatgtcttcagttccatttggcaattttcaagcactcgagtcaccaagtaagcaatatagcgttcttgaatttcgaggctttcttcttggtgcatgaatgccatttccggttcaatcatccaaaactcgatcaaatgacgacgggtctttgatttttcagctctaaaggtagggccaaatgagaacactttgccaaacgcttgggcaccggcttcttcatacaactgaccactttgagacaaataagcgtcgcgatcgaagtattccgtatggaaaagcgtcgttgtcccttcaggcgcacttccagtcaggatgggggcatcaattttgatgaaaccttcatcgttaaagaaatcataagtcgccttaatgacctcattacgaatccgcataacagcgtggggccggctggatctcagccaaagatgacgatgatccattaagaagtcaaccccatgttccttgggcgtaattggatagtcatgggtttcagaaaggacctcgatggtttcaatttcgatctcgtagccaaatttggaacgagcatcttcatgaatgatcccggttacccacatgctggtttcctgcttgacttccttcgccaactcgaaaacttccggggtaacattactcttcacgacgacgccttggaaaaatgccgttccgtcacgtaattgcagaaaggcgatcttaccacttgaacgtttgttggttaaccaaacaccaattttaactttttcgttaacgtacttaggtgcgtcaaccatgttaatttgtttcaattccgattcctccagatacttgtttttctaaaaactgattcataaattcagtgatccgctcaacggcggttaccaggtcttccaaactagtggcataactcaacctgaggtagccgggcatgccaaaagcagctccgtcaaccaccgcaacgtgggctttggccagcagctgatcgaccaattcccctgagtcattaagacctgccaggtcaacagccgcttcaacatttgggaataaataaaacgccccttgcggtttggctgccaacttaaaccccggaatttgttgcaccagcggataaatttgatttaaccgttgttcaaaggcctctcgcattgtctcaacggctgattggtccgactgaagggcagcaatcgcagcatattgacttaccgtggctggatttccggtcgaatgagatagaatcgaatttaccttgccgattaattccggcgccccggctaaatagccaattcgccaccccgtcatggaataggctttggaaacgccgttgaccaaaaccgttgaagcagcaacctcgtcactgatttgaaccaacgaaacaaactggttttgattataaaccaatttgccataaatatcgtcagcgattaaggtcacattatgcaagactgcccattgaccaattgccgccagttcatccctggaatacacggttccagtggggttttgcggtgaattgatcaccaataccttagcatttttagtcacagctgtatccaggctttgggtggtaatcttgaagtccgtccctgtctcaacaattaccggcttgccgcctgcaagattgacctgctggcggtaactgacccagcttggccggggcagcaagacttccgtgccgtcatcgaccaatacctgcattaacacgtacagcgccatcttggcaccgttggtcacactaatttgatcagctgggtagacaacgccgtagtcctgcttaatgcgctcggcgatggcttcttttaactggggtaaaccactggccggggtgtaaaaactggttttgcccgatcgaatagcgtcaattgctgcatcggcaatgatttttggggttggaaaatcgggctcaccgatgcccaaattaatgacatcgatgccctttctgatcatcgccttggcagtattggaaactttgacggttgctgaaggcgtgacctgcatcgcccgttttgaaaatttcattgaagtgtcctttcatttctagatgttttcaatcgatttgtaaatggtgccgtttttgaagctgattgtcgtaaagcacaaatgattcttggcgttcatatagctgaccacccaatatggctggttcttaatcatcgtcagcccaatcccgtttaattttgatgggtgtttttgccgttgaatcacatttttggcctgctgctcgctaataccgctgctgctattgataacgttgaccgtgccgccttttttagcgacgatgacgtaaacatttttgttcttgttatcaacaccggaaacggaataataagtcttccccaaattagaggtgtaaaacgagtcgactttcgttaacccggcgtactttttagcaatcgtttcggtctggccgcgggcaattgtcatcggccgctccgccgtgtgcaggataatgaagaacgaaaagcagagaatcaaaatgatcgagataacgatccaggaaattttaacgtatgattgttttttaactcttcgatgccgttgcatggtaacttcctctcaaatttcgttattcctaattatagcaaatatccgactgctcaaccgcagattaatttctgctttcaaaaaacttaaccatgtctaatacacattcatcaattgaaccgtgcacgacaggaatatcgttgcgcaaattggctagaatggtgctgccataccgcttagataataacctgggatccaaaataaaaatggttccgaagtcatctttggttctcaacaggcgtcccatgccctgacgcagcctgagagtcgctttggggagcgtaatactataaaatgggttcttacccttactgcgctcaatcgagtacagcgcgtgattataagggtctgagggcgtatcaaacggcagctgggcaacaatcaggttttccagtagatttctcgggaaatcgactccctgccagaaagtattggccccaagcaggatagcgggttcatgatggatgaactgcttgctgattttggcggctgttccgtgaacgccttgagccaaaacaaaatgggtcgctgtgaagccactttcctgaagcagccgatacgtccgttcaatcgcattgagtgagttaaacagtaccaaggtctgccgcggttcattcttataaatgacttcgatattgtcggcaaccttttgaagataattatcggaattggttgcgaattgccggtcgtcttgatcggtgaccaaatagagtcgggcttgatctttgggattgaagtcgcttttgagtcgtttaatcgaagaatcgtcgcgactaatccccaataagttgtaaatgaactgtgaacgtcgtgaagagaaaattgtcgccccggtaaaagttgccggttcaaaggcagaatagacatggtcacggagataatcttccgttttcaaaatcccccggttaagtgtcaggctattgacgtctttgacattattgacggtgacccacgtcacatgctgctcaattgactggtcgtcaacatcaacgattgctaacagcaagcgtaattgatgattaaactcattatagttttcaaaaaaagaataaatacttaagaaatcgtggttggtgtatgcaccggcattatggtcaatttgggcatttaaagtggccagcagtccgtccaagctgtcgtggagcgcgcggagacggttgatcggttcttgattggcagcggtggctgccttcatctcattaatcggaattaagcgctcgaagaactcggcattccggtggagccgtttgcccttgacgaccatttcaaagagggtcgtcgtgacggtcgagaccagggtcttggcctgtcggagtttgccgtcaagggcttcgatagcgtggtccaagatggcgtcgtcttccacaatttctttgatattatcttcgtgagtcccattaatatctgccaagattttgttaatcgccgttgtcagtgataacggattaatccgctcctgattgttacgaatggcagtttcagcaaactgctgggtttcgtcaatcagtaagtagggtttggtcggcagatccttgaaatactgccaatttttaattagataactgtgattgacaatcaaaaaatcagcattttgtgcctttttcaagttgtaacgcaaaaaatcgtcgtcataaaacggttcgtttggatccagccatttcacgccggtatgctgaattttccagacaaatggtgtttgatcgacgtttaagtgcagttcgtccaaatcacccgtagtggtaaccgtcagccagactaagatctgcgctttaataaacgcggtttgggttgagttgtcaggaacgtttaataagttgcggaacttgtagagatcgatgtagtgactggccccttttaaaatgacactattgactttgaaaggcagcccttcattgagcattggcaacgtctgattttgcagctgaaactgcagataagttgtcgaagtactgatgactgcaggcttgtgggccgacaccaaataactcaatggcagacaataccccaagctcttaccaatcccggttggggcctcaattaagagggtcttggctgcgtgatgctgttggtcggcataattgttatagatcaagttcatcattttattctgctcaagtcgcgactccaggttgtccggaagcagtttttgcttggccttttttgtttttggatagcgaagacgctgtttatcagactcatcagtcacgacgattgggtcctgttttcgcaaaaccagtcctgatgagattctcagctgatcaggcaatttggcagcgtgcacctgccttttgttggtttcatcggcatccaaaaaaacctgcatcgtgtcttgaggcagagacggattaacgctgatgatctgttccaaggtcattttcggcagcatcttaatttgtcgtagtaaaataagcaggagcttggcggttgccaaagcatcactatcggctgtatggggatggtcatgttcgatattgaaataactgctgagatcctgcagccgataactggataacgttggcagcaggatttggcttaaagtgacagtgtcaattgcttcaatttgtaattcggggtagccgacgcgttgaaattcagagttcagaaacggaaaatcaaaattcacattgtgggccacaaaaaccgtattattgagcaaggaatacagctgagcggcaacctggtcaaaagttttggccttttgcagccgttcgttggtgattccggttaactgcacaattcggttagggacttctcgttgtggattgatatcggtcacgaaggttttaataattttgttgttggaaaccaagcagcagctgaactgaattgtccgattatccgcagaaatatctgttccggtcgtttcaatatcaaccacggcaaaggtggtttttgaattcattgtcattcaccaatctgtttatgagctgacttttcttaaatattcactaactttaatcatactacaagcaagatgtgataatctaccatggaaagaagtagaattatttatgaatctctaaaaatatctttaaaacgttctcgaatcagtgaactatgataaaattggaatgtttgaaagtgagcggataaagttgaaagataaagcaactggaaaaagttacgcaaaaattatttggtttggtgagcatagtgtcgtttacgaaaagcccgccatcgccatcccaatctactccgttgatgtggttgcgaccattcaaagaattccaaccggccaacaaattcactgtcgttactttgacggcccaattagtgaaatggcggagaatctgcggggtgttaaaacattaatcactcatctcgttagtttgtttggcgctcaaaggcttgcttttgatctcgacatccaaagcaaactgcctgccgaacgcggaatgggatcctcagcggcaacggcaatcgcaattgtgcgggctttttttgatttttttgaggtcaatttgaccagaagccaattgctgaagttagcggatattgaagaaaagattacccacggcaatcccagcggcctggactctgcgaccgccagctccaacatgccgatttggtttatccgaaacaaaatcaacgagcagattgactttaatctgccaacctcatcattggtcattgccgatagtgggattaaaggaaaaaccagtgaggccgtttcgttggttcatgataacctggtcgacgaaccggaaagttctcaaccattaattgacgagcttggcaagattgccgaaacggctcgcaatgctttggcaaccaccgacgatgtgctactgggcaaactaatgacacaatcccaacgtgacctggcccaactcggcgtcagcaaccacactctggacacattctgtcaagttgcttgtgacaatcacgctttaggtgccaaactaaccggcagtggtttgggcggctgtgtcatcgccctagccaagaaccaacgggatgctcaacaaatttcgactgcccttcgaaaagccggtgccactcagacttggattcaatcatttaagaattatcaattttcaacaggagaagctcatgacaacctcgtcagataagaccgttacagcagttgctcacacgaatattgccttaattaaatattggggcaaacaaaatcctgaactcatcatcccctacactggcagtctctctttgacgctggatcaattttatactcaaaccagcgtgacatttaacgccaacctggataaagaccagattacaattgatggccagccggtaaccggaaaaagcggtcaacgggttcacaacttcttaagcattgtccgccaagaatctggaattgatttaaacgcccaagtcaaatcgactaatcatgtgccaacggcagctggcctggcatcctctgcctcggcgtttgctgcgttggccgccgctgccagcaaagccgccggcatgaatctgagtttaacggacttgtcccgattggcccgccggggatccggttcagcctgccggtcaatctttggcggctttgtggaatggcgaaaaggatcagacgataccaattcgtacgccattccagtcgaaacgactcatttgaacgacatccgcatcgttgcattaaccattgaaaagcatcaaaagcccatttccagtcgggaaggcatggccctttcagtcaccacctccccatactatccaacgtgggttaaggtcgtcgaagccgatctggagaatatcaaagccgccatccaagatgatgacttcacgcgttttggcacaattagtgagttaaatgccatgcggatgcacgccctaacactgagtgccgatccggattttctctacttcaacggcgacaccttgaccgccatgaacgaagttaaacggctcaggcattccgggattgaatgttactatacaatcgatgccggccccaatattaaagtcatttgtcaacaagccaatgttcaaaccatcaccgataccttctcaaacctgtttggcccaaccaaagtgaccgttgccaagcctggcccgggtgtcaaatatttataaactagaaaggaaatgatccgttgattaaggttaaagctccgggaaaattatatatcgccggtgaatacgcggtagtcgaaactggctacccttctattattgtggctttggaccaattcgtaactgtcgaaatttctcgaagcaagtcctatggcagtatcgtttcaaaacaataccgagaagattcggtctattggcgtcgtcgcggtgatcaaatgattctggataaccgtgacaatacttttaactacataatttcagccattcagctcactgaggaatatgcgcagtccctcggccggcagatggagctctatgatctgcggatcaatagtgatttggatagccccaacggaaaaaagtatggattgggttcttcagctgccgtgacggtggccaccgtcaaagctctctgtcagttctacaacttaccgctgaccaagagtaaactgttcaaactgtcggcaattgcccatttggacgtccaaggaaacggttctttgggagatatcgctgccagtgtatacggcggctggatcgcttaccgttcatttgaccgcagctggctcatggctgctcgaatgcaggaagacctgatttccttagtcaacaagccttggccgcatttaaaaattacgcaattaacgccacctgacgggttgaagctgattatcggctggaccggttctccggcctcaacttcgcatttggttgacaaggttgccgttcaaaagagcaatcagcatgagacttacacccattttctggccgaaagcaaagcctgcctggacgaattgattgacggtttcaaaaatggcagcctgtcggtcatcaaagagggaatcgcccgtaaccgggaaatccttcaacatttggctgcttttaccaaagtgccgattgaaaccccaattctcaagaagatgtgcgacattgccgtcgaccatgctgcagctgccaaatcttccggagctggtggcggtgactgcgggatcgtggttgccgacaaagataccgatgttgattcgatgatcgcccattggcaggaaaatggcatccagcagctggcccttaaagtccatcccgtcatcgatcttgacaaggagtagcttatgacttcacaacattcccatcgtaaagatgaacatgtgtccctggctgaaaagttctaccaacctgtcgacagctcgtttgccggcgttcgatttgtgaatgccagtctgcccaaatatcggttagatgatattgatttaaccacccagcttggccccctgtcgctgacgacccctttctatattgaagcgatgtctggtggcagcccccgcaccaaagagatcaaccggcgacttgctgtggtggcaaaagcctgtggattggcgatggcggtcggctctcaaagcgttgggttaagtgatcctgaggtgcgcgattccttcagtattgtccgtcaaaccaatccaaacggaattgtcttggcaaatatcggtgccaaccacagcgttgaggatgcccaaaaagccgtcgagatgatcgccgccgatgctttggagttgcacatcaacgtcgcccaagagctcgtcatgcctgaaggagatcgggagtttcactttattgacaatattcaagcaattgttgccaatgtcggtgtcccggtcattgtgaaagaagttggctttggcatgagccaagcaactatttcacaactggttgacctgggagtgaagtatgtcaacgtcggcgggcatggcgggaccaatttcgctgccatcgagaacttccgccgctcctcaaaagacatggcttatttgacggattggggactgagcaccgttgagtcgctattcgaagcccgcgccttttctgatcggttgggcatcattgctgccggtggtgtcaaatcaccgctggacgtggctaaatgcctcacactgggtgcctcagcagttggcgtggcaggttactggcttcatgagatcatccataaaagcgataatgaaattattaacgatgtcaaagaatggcagtacggactaaaagcaatcatgttaatgttgaactgccgaaccattgctgacttacaacggcaacggttgatccttgatccacaattgttgagctatttaaaacaaaggaaattagcctattaaaaaagagttaaatcaaaaatcagaagccacaatcttctgatggtgatttaactctttttacatcgcaaatctcagccccttggggaagaaattcttggccgtaccattcacaactttggcaaagccaactggctgctgctggcaaaccaggaggtaccacccctttttcagatctggtgagacttggaatgtatcgccatgcacgtacttttgccaatccgccaagtctatagtgattttttgactgacttgatcgggatgcagtgccaaggctaagccataactaggttcaaagcggttctttttgaaagtccccatctccaaaccaagtcggacaattttaatgccagacaagttcggcgtattttccggtactgagtaaagatgatctttgaaaaccaccaatttgtcaaagtgaacgttctttaaggttgctttggcaaactggttgaacaattgattctgatatttggagggcatttcaatatttcgactgatgccgcggaagcgacgcggtcctttgctaacttccgggtctgccggctttttcaatttggcaataaaatggccttctccgttaaaatgatgtggaaagatacgcacacagttggttaaatcctgattgccatcagcccaatctggttgaccgtcatccattccggcaaattttttaatcggttgaatgtcaaatccataggtgtcgaccagccaggcaatgatctgctcatcctcttcaggggcaaaggtacaggtggagtaaatcaattccccgccaggctttagattcttaaccgcctgggccaaaattgtccgctgacgggccgcacattcaattgggtaatcgacagaccagtattggacggcgtccgggtcttttcgaaacatcccttctcccgaacacggtgcatccaccaaaatccgatcgaagaattccggtaattgggctgctaaatggtccggatccgtgttggtgacaatcgtattggtcatgccaaatcgctcaacgttttcaaccaacgctttggcacgcttgctgtcaatctcgttggcgattagcaggccggtgttttgcagatagctgccaagatgggtggttttaccaccaggcgccgcacacaaatccaataccctttctcccaggttggggtgggcaacttcacccacatacatcgcactgggttcctgactgtaaaccgccccactttgatgatcgatggttttgccgctgacctgaccatgatagccaaatcggcagtgttccgtgggctcactcaggtccaaatcagttggttgactggctttcaatggattaagccgaaaacccggggttgtcggttcgtcaaagctggcaatgaactggtcggcttctgatttgcccattaattgctgatacttattcacaaaatcagttggtaagttcattctaatctccctttttggtactaataattgacgtgataggtgtttttggatattataaatggatatgttagtaaggagtgatcacaattacaaagaaattaatcgccctcgacttggacggcacaaccctaaataacgatagtctaatcagcgccaaaactgcccaaacaattcgggcagctgcgaagcaaggatacatagtcagtatcgtaaccggccgtcccaatagactctctgaaactttttatgacgatttaaagctaacgacgccaatgattaatttcaatggcaaccttggcattttaccacatcaacagtggaatcgtgaataccagtacacaattgataaagaaattgtgactgaattactggcaaaaagcaaaccgctcggcttgtcattgattgccgttgaaggccggaatatgtttttggccaaccagggattaagcagtggtttcggcttcttccccagcaccttggccaccaatcaggtactgagtcgcaaaagcctaaaagaaaacccgatcagcattactgttcaagtggaacccgaactcaagcaggggttgattgacttcgtcgaacatcaatttggcgacgaggttgaagtctccccttggggcggcccaaatccgattgtggaaatcgccacgaaaggtgtccataaatccaccggccttaaatttttggccgattactatggcatcctgcaaaaagacattattgcctttggtgatgaaggcaacgatttgaccatgatgcaatacgcaggcaccggtgtcgcgatgaaaaacgccattgataaaatcaagggccaggccgacgaggtcacggaattcaccaatgatgaagatggtgttgcccattatcttcaagatcgactggacattgctgttggtgcttaaccgatagcaaaaactaaccctcgggacgaacagcgatttaatcccatagtttaatgcagaaacgcagtcattccaaatgttggagtgactgcgtttctttgttaatggccagtttgccacacaagtaatgccagttgtcgtaagtttgagcaatcaaaagtggtcattgaactcacaacgaaaaaatgataaatgattagttttcgtcgggatgatactgaatcgttgcctggacggccttttgccaaccggtatacagttttgtgcgtgtctgctcgtccatttgcggttcaaaagcatcccgtgatttaacggtccggcgaatttcttcgatagaatcccaaaagccgactgccaagcctgctaggtaggctgcacccagcgcggtggtttctgaaattgaggcccgctgaattggcgttcccaaaatatcagcttggaattgcatgagataattgttattagctgcccctccgtcaactgccagcgacttcaaatcgattccggtttcagctgccatggtgtcaacaacatccctggtttgataagctaatgactcaagcgtagctcgaacaaactgatttttggtcgtgccacgagtcaggccaaagaccgcccctctggcatcctgatcccagtagggcgcacccaacccggtaaaggctggtacgacgtagacgccatcggtacttttagcatcaatcgccatttgttccgagtcaggggatgacttaaccatttccattccgtctcgaagccattgaatggcagaaccagcgacgaaaatacttccttccaaggcataattaactttgccattgattccataagcaatggtcgtcaacagcccccgtttggaaagtgtcggctcctcaccagtattcatgacgataaaggcaccggttccgtaagtgtttttgatcatcccgcgctgcagagccatttgaccaaacaaagctgcttgttggtcaccggcaattccagcaatcggaacctgaacacccgagaaggaataaccagctgtataaccataaatttctgacgaggaacggacttccggcagcatgctttcaggaatgtgcagcaggtccaaaatatctttgtcccaagtcaacgtgtgaatgttaaacagcatcgtccgactggcattggtataatcggtcgcatgaaccttgccgccggtcagcttccaaaggacccaggtatcaatggttccaaacaataaatcgccattttcggccttttggcgagcgccgtctacatgatccaaaatccattgaatcttagttgcggaaaagtaggaatcaatgatcaagccggttttttcatggatcatatcatcataaccgtcgtgcttgagctgatcggctaaggcagcggtttgtttggactgccaaacaatggcatgataaatcggctcgccggtatttttatcccaaatgaccgtggtttcccgctggttggtcacaccaattccccgaaccttgtatggttggacatccgcattaatcaaggcttctgagatcactgattgaacggcattccaaatctcattggcatcgtgttcaacccaaccggattttggaaaatactggtggaactcccgttgtgctttaccaacgatatcaccatcattattaaacaatattgcccgggtacttgttgtcccctcatcaatggacattatgtattgctgatcattcatgtaaaggtctccattcctattattcgtgcgtttaaacgctttttctttgttaagtatacaataatatcgactggcaaaccaaccttgagataaactttatcaaagtaaaagaatttgatgattcatccccgaattaaacgcaaacaaaaagcccgcaacaattgtctggcggacttccaaattatttgcgactatttttcgtcactcttgagcacaccgccaacactgtaacggttcttttccatttcacttaaaatcacgtgaacatgttctgcgggagcaccggtatttttaacaacggctgcggtaacgtcttccaccaagcccttcagttgatcttgagaacggccggcaattaaatgaatatctacaattggcatattttgattcctccatttgtttcgaatggcaaaagtataccttaaattatttttgcctgcaatatcttgatggcactttggacgtgtcaggaccgtttatggagcaaagatgatacaataattggagtaacatttaactgcgaataggagattttaaaatgataccatacaaaaacttttccgcctgtaccagtatgattgttggcaagaaagccagcattgacgggtcaattatgattgcccgaaacgaggatagtaaatcctcttggccaaagaattatgtcatccacgagcatcaagaatttagtgaaaccccggttttctcatccaaagacaacggcttcaagttaaccctgccgaaagtgcgctttcaatattctgccacccctgaatggactgacaagttcggcctgtttgaagaaaatggctttaatgagttcggggttgccatgagtgctaccgaaagcacctataccaatcagctggctttgggggccgatccgctcaacgaagatggcattggagaagaagcaatgattacggttgtcctcccctacgttaaaaccgcgcgtgaaggaattgctcgattgggccaaattgtggaatacttcggaacatcggaatccaacggcattttgtttgccgataagaatgaggcttggtatatggaaaccggcggcggccacaactgggttgcccaacgcattccagacgacggttacgcggtgattgccaatcaaagcgccattcaagacgttgattttaacgaccccgacaacttcatgtggtcacccaagattcgccggtttgtctccgaaaatcacttgaacccggacccgtccgggaaaaccttcaacttccgtaaaatctttggtaccgctgacttgtcagacacagtttataacaccccccgcgtatggtacggcttgaaaatgttctcaccagaattgaattttgagccaaccagccaggaaatgccgtttatcaatcaggccaaccgcaaactaagcttgtttgacgttgaagatttcttaagctcccattatcaaggcacaccgtttgaccccattggcgagggctctgagcacgataagcacctctatcgaccaattagtctcgccaagacgcaagaggcccacatcctccaaattcggccaaatatgcccactcctgctgcagggattcaatggttggcaatgggcgtcgctgctcaaagttcttttgtgccgttttatgccggcgcaaacaccacgccaaaatcctatcagaatgcttcaggcagctatgcccccaatcaagcctattggacttacaagcttgccggtgtcttagttgacccgcattacgtcaaattcgggcccaaattaaatgacaccaaggccaaactgcgagtgaatttccaacaagcagtcaaacaagctgatgcttcattccaaggtttgtccaatgtcgaactcgccaattatctgaccaaagtcaactttgccaatgccaagatgggcctggatgcttacaaccaattgattagtgacatcatcaccaattcaacagacctctcaccaatcaattttacccaggacacgaacctataatgactcgtctccaacattaagataatctgtcttaaaaattgaataacaaaacgaagccggccacaaattcaattttgtgagccggcttcgtttggttatgatgactgatttagtttagtaatgttctcgggtaaatgagcctggcagatcctggctggccttgacaaccaattttgtcagcagatcctcggtcgctttcatgacgtgatcagcggtccgggcattggcttggccaagggctcgaacaacgtgtgagccggaagcctctttttcggccatctgctgatcaacttgggcaattcgttcgtgggcataacccatttctttaagctgatagtcttcaatgtcttgcatcaaggcctgataatgatcagcagcaatcaatgaaatcaggcgatttgcccaataggcgttgtggctgtccagcgtctcggtggtatcacggtagcagtccggtgtattgacgacgttggtaaagaatggtgtcaacgtgttgaacggattggaggcgaatgtcagccactgaattgctgaataagctgaaggaattcctggacgtaactgcaagattgacagctcttggttgcggttgatgccaattggtcgatatggaacggtcttataatcagctcccggcgcaaacggatcgtaaggcgtgtcttgataatgggagctcagaacgaatttgatatcttcaatcgtaatcttgcggttggcgtggcagataaacggcaaatcattgctcattggcgtcttatccttcactgattccggatcgaaatatcgttgaccataccaagcacgtggtgtgttgtagtgacggtccagctgggtatctgagccaaagaccttcctgaagttaaagtgactggttgggttgagatggtgttcctgggcaaatttacgcaagtcttttgagaacataaagctgtcaggatcatcgaaatcgatctcttggatgcctgtctggttgggcgcgatgacataggcatcatctggaatccgttgggctacccagtgatggccaccggcagtttccatgtaccaaatttcgttgacatctgaaaacaggattccgttggactcgtatgtgccatatttctcaagcagtttacccactcgttgaaccccttctcgggcagaattgatatatggcagggtaattgttaacagatcttcttcgccaaggccgtctttttcaaatgggtcggcaccgatcacccgagaattggtggtaatcgtctctgtggcactcattgccacattatgggcattgatgcccgcctcgccccaaacacccttgtcagggacagcatcgggcactgaggtatatctcaatggattgtctggcagtttaacactaaacttggttaattttgactgataattgcgtggttggtcttctggttcaacaaccacaaacttctttggattaacggcatctccggcatcctcatttctggcgatgatggttgacccgtcatagctggccttcttgccgactagaatagttgtacaactactgtgttttgatgaaaacattttgaagcctccccttgtctttctatcaccttgattttacacccttttgtgcattgtggaacaaaagaccgttgaatgcaaaaatggggattgcggggtggtggctttttgtcaaaggaatcaattccatggaattgattctggtggcagttggatgctttttaacgattaggcttcccgttctgctatacaaatgaggggcaccaacgatgaacaaaattcgtgattcggaattcattcaggattgcttttacagggttagagcgatcagtttattccgtgctcccttgggcctttgagttcagctccgacgccccaggaccctactgcacaaacaaaaacaaccagcgatgaacaaaagacgttcatcaggactcattcaagattgcttttacagggatacagcagttggtttattccgtgcttccttcggcctttgagttcagctccgacgcccctgacccctaccacataagtgaggagcaccaacgatgaacaaaattcgtaccccgagattcattcaggattgcttttacagggctagagcgatcagtttacttcgtgctcccttcggcctttgagttcagctccgacgcccctgacccctactgcataagtgaggagcaccaacaatgaacaaaattcgtaccccggaatttattcaggattgcttttacagggatacagcagttagtttacttcgtgctcccttcggcctttgagttcagctccgacgcccctgacccctactgcacaaacaaaaacaaccagcgatgaacaaaaaacgttcatcactggttgtttctgcttgtgctccggggtcaacccagggctcgtcgcatgctttttatttttgtgccggttcctcatagtcgccgtttggacaaaccacttgcgtgccgcccttgacccgtttttcaactaagaagtgaccatcctttggacaatctctgccgattggcttgtcccaagaaacgaaatcacaatccgggtatcttgagcaaccatagaaaatccggttctttcttgattttcgctcaatgacctgccctttgtgacacttaggacaaatcacaccgatctccttaacaattgccttggtattgcgacaatccgggaatcttgaacaggcatagaatttaccgtaacggcccattttgatcaccattggggcgccacaaatttcacagttaatgcctgccggttcatctttaatttggaccttttccatatttttggttgcggcatcaacctcatcggaaaatggtttatagaacgtatcgactaatttgatccagttctctttaccttcttcaacctgatccagtttgccttctaaatttgcagtgaagtcaatgtttaccacgtctgggaagtattcaacaataatcttattgacaatttcccctaattcagtcggctcaaatcgacggccaacttccttaacgtaataccggcgctgaatcgtatcaatggttggtgagtacgttgatggccggccaacacccttttcttcaagggctttaatcagcgttgcttcactgtatcgtgccggtggctgagtaaaatgctggtccggattattcttaaccaacttaacaacatcgccactctccaaatcgggtaacaagttgtccttttctttactgtcaccataaaccttcaagaacccatcaaacttcatcttggaaccattggctttaaaaatcacgttattttgttcaattgtcactgccatggtatccatgattgccggagtcatttggctggccacaaatcttgaccaaaccatttgatagagtctaaattggtcgcgggtcagatattgtttcaaactggcaggcgttctgaaaacggaagtcggacgaatggcctcatgggcatcttgagcaccctcaggcaatttacctttaatcggtttcgttgccgcatattcggcgccgtatttctcatgtagaaattgggacgcttcgtgtttggcaatgactgaaattcgggttgaatcggtccgcatataggtaatcagaccttgactaccctctttaccaatattgattccttcatacagctgttgggcagccatcatcgtctttcgcgttctgaagttgagctttcggttggcttcctgctgcattgtactggtggtaaatggcggctgcggttggcgcttccgttcgcgacgggtcaccttggtaatatcaaagtcacctttgggatccaactgctgcagaaccttttgaaccgcctcgttatttggcagttcctttttcttaccgtttaagccataaaaggcagctttgaacttactgcggcccttcttaaattcagaatcaattgaccagtactcttctggggtaaagtctttgatggccttttcgcgttgaataatcagccagagggcgatcgattgaacccgcccggcactgagccctttcttaaccttttgccagagaagcggtgaaattgaatatcccaccaaccggtctaaaatccgccgagcctgttgagcatcaacgagattcatatcgatatttcggggatgtttgaatgattctttgacggcatccttggtgatttcattaaataccactcggttatcttcgttgggatctaaatccaaaatgtgctgaagatgccaggcaatcgattccccttcacgatccggatcggctgccagatacacttttttggcctttttagcggctgaccgtaattctttaatcgtgtcacccttaccccgaatggaaatgtagtgtggttcataatcatggtcgatatcaacgcccatcttactcttgggcaaatcccgcacgtgtcctttactggcgaccaccttatatgaacggccaagatatttttctatggtcttggctttggcaggtgactccacaatgaccagattttttttaggcgattttcgcttagtttttgattttgctttggcttttggtttcgtttttgtagaagttgccatattttctcccctcaaaactgcttatttttagttatattattgtaggaatttttattacaaatctaccacatcatattgcaggaattttaaagtgtcaactcactgcccttaaatccgcgtctgaaagtagtcctccaagatgtctaattcacgtaaaaccggttttgcgccggcagcgattaattcattggtaccaacggacagcggcatcataattgaccccgggactgctaagacattgcgattattttgcagggctaaattggccgtgatcaaactaccggaatgttttttggcttcagtgaccagaacactttgaaccaatccggcaatgatgcggttacgttccggaaagtgatttcgatagcccttggtatgattgggatattcactgattaacagatggtcggcggcaatcgttgcttgtagttcctgattggtatatggataacacacgtccaaccctgtcccaatcacggcaatggttttaccgtggttggcgatgacacattggtgggccaacgtatcaacccctttagccagccccgacacaatagccattgtattggaaactcttccaggaatcaaattttttaggatttcgactgaatatgaggtgcagtcccgcgccccaacgattcctaaaagcggctgggataaaagcgacaaatctccgcgataaaacagcactaacggcggcgcaaacgattctcgcagttgaagtggatattcagcatctgcaatgctcagccactgttcaccatcgaccagctggtccacccggtcttcgtttcgcattaactgttgataactggttttgaagttagccgtgttcttaacgtttagttgagcgacggcagccaagaatcctgaggtcggcagttgatcatcccgccagtcgacctgatttacccaagtataaatttttgacttaccaattatgccgattcctttacataaatgtattcttaacaaaaaatctcttaaaagcattgtcatcatccttttaagagttatctacgtaaaacatatttattttttgctaaactttttcactggggcaaaactcattcgatgaatcggcgttggtcccagttccttgagagctgctaaatgcttggccgttccatagccggcgttgtgtggaaaatcgtattccgggtactgcttggcgtactcgtccatcaaatggtcccgatagactttggcgacaatgctggctgcagaaacactgatgctcttggcatcacctttgatcagtctggtttgccgaatcggaacgggaatctgcatggcatcaacaatgatttcatccggctgtggggttaaagattccacagcttgtttcatggcaacacgagtggcttggtaaatgtttaactcatcgatcccatgattatccaccgatccaatccccacgctcagggcttcagctgaaatcagcggggccaactctgcgcgttgggccggtgtcagctgcttggaatcattgacggaaaccagatcaaagtcgtgcggcagaatcactgcagcagccaccactggccccgccagaggacctctgccgacttcatccacaccggcaacatattgcagcccctgatgccaaaaagaccgttcatatttaaaccgctgttcaaattcagcgagggctctggcctgcttttgcaggcggttttctgttgactgaattgccaattgaaccccttttcgcgggtcagcctttaactcaatcaaccgcggatcagcgagatcagacatctgggataaaacctgtttaacgtctttaattgttagcttggtcatcgtcactcaccgtttcaggatcatccaaagtaaaacgaccaattttgccggcacggaaatcttgaataatccgattggagccacgttcataatcatcgcgcatgccgactttcttagtaatttgtaacagcaggtcaacgtcggacaaatccaaatcgtcgtcagttaaatgataacggtctttgaggccttccgggtgaagctgtctgatctgctttaagccaaacaaggcaatgtcgtcactggcataaacactctctttgattgcaccggtcaatgccagcttatccgcaacctcttgactggaaaattttggccacagaattcccggcgtatccagtaattccaacttatcattagatttaagccactgttgccccttggttaagccgggacggttgccaacctgagcggctcgacggttgaccaatcggttcaaaacagttgatttcccgacattcggtaccccaacgctaatggctcggatcggtcgtttcttcatgcctttatcctgttcccgctgcaatttgtcacgcaaaatgggtgaaatcaccgaaatcacattattaatgccaaatttggttttggcatcaatggcgattgccggttggttgtgttcagcaaaatactgcagccaggcattggttaattgaggatcagccaaatcacgctttgtcatgatataaagatgcggcttatcggcactgattcgtcgaatttcagggttttgagaagtcagcggaattctggcgtcaatcacttcaaataccacgtcaactaaagaaagattttcttcaaactgacgaattgccttggccatgtgtcctggaaaccattgaattgttactgccattgtttcacttcctaaaagctttcttgatattccttccacacggaatcaaaaatttccatggtcggaaggtatgaagcattttcttctaaatacttggataacgcgtcaaactcatcttcttgtttgggaaatgactgatcataaaatgcgttgttggcaaattcagcctctggatcagtacttccggggttgcgtttggtcattaaatattggtagaacgttttgtgcatattagtcctccttgtcagtggtcggcaaaagaatctcaaaggcaaattttccttggcctttcaaatcgatggtccgggcccgataattaatcccattcttaccgttcatgtgaattatatcaagtttgatggttttatctttaggaatcagttggacccactttggcagtttatagttttgtttgacatacattaaaacaaaactgattggcaccggaaacttccccagtgccagcttattagcgtgaagttcaatattaccattgggcatcactttcgggtcgaaggtcagtgaataatcgacgttggaacctaataaagtcagcgagccatagacaatcccttcgttggcgacttcaaagtgatattgcgaaggtcggcccttctgcagcttatctaaataataattggatagttgattgagttgagctttattgatagtggcggaaattggctccgattggttggtcgacttttgattcaccaatttcgtcgtagatgacgataaagaaaccgccaaaaacatgccggcaactaaaacaaccaggaggccgattaacgatatgaaagcgattttccaaggattgcgggatttcgtctgcttggaggcttttctcattttggatcactcctttaaccaggatatgtgcttgaccatttgggaatacaagcgattggtcataatttgataccccttcaaattcgggtggaaatggtcatcatttgagagatatttatttgcttgggcaggttggccactcaataactgttcaatatcggcaggcgaatcatgattctcggcgataatgctggcagcggccttttcttccaaagtttttctggatttggcagtggtaaactgaccgtctgtaagtggtttgttaatcgaaacaaagtacatcctgtgctgttggtggatcactttattggtaatctggttggtatgggccacggtgtcgttgatatagttgacctgggggaagtaaacgtagacaggattgtaaatgccaaaaacgaaaatcggcgcccgacggtttaagtggcggatatttcggaatagccgggtaaccctggtttgatatgtttgacaataaccggtcaatttctggttcaactgatgtttgttcaagccaacaacgttcgccttcaaaaacttcagtaaatcgtttccaccagtggtaatcgtgatcacatcggcttctcgtatgctgtgctgcagccgttttgaataaaccacccgatgattaatttggttggtggtttcccctgaaatgccatagttggcagtggacaggtgaacattgggatttttttgaatcactttttggcgaatcaagtgggtatagccacctttgttggtcggatcgccaaccccttgagtcagtgaatccccaacagccgtcaatttaacttctcttggcagggtttctttggccgagttgaaataatggtagccgaaaaatgcgactgccccaatcacgatcaggccgatcaatccgataatccaacgaaaatgatgctgtgtctgtttaacatgtttattttgactcacaaaaacaacctctcaaatggtgatcaaatctaaaaggggtgacaacaaaacagccgctttgcctcgcccctttaagcaatatttcagatctgcaattactcgggatcactgtaataaatcaacgcaaaagcccctttaccggtatgcgtggaaatggtcggtgacgtcacccgttcaagaaatgatgcatcgggaaagtcagccttaagcttttgaacagtgtcctttaatacttcagtttcagtgacgtatgaaacgccaatcgacttaacagcggcggtgtttttcatttcatcaataataccattgaaaaactttttaagcgatttatcgccgcgacctttagaaataattttaagtttgccgtcagtgacttgaagccccaacttaatgtttaaaaagttggtgattgccccggcaatcggatgcaatcgaccgcccttgacaatattatccagagtcatgacacataaataaagcttggtgttaatacgaacctgattgactctggctaaaatggtgtccatgtcggcaccttgctgagccagcttagccgcttcaagcacttgaaagcccaggccgcggtcggtactttgactgtcaaccacggtcacatcggatttgctgattgtggctgcttgttcggctgcgtgaaccgtgccgctgatggcagccaacatattcaaacagagaatttggctgccgtcttcacccaaccggtcaaatgcttcaacaaatttaccaactggtggttgactggtctttggcagatcatgagccgccaacatttgaggaacaaaggtttcattggtgatcgtatcacgatcaacgtagaccgtatcatcaatcatcactgttaatggaacaattgtaatgccgtattgtttgagttcttcatctgtcaactgggcagatgagtccgtcacaatttttacttttgccatttacgccactcgtttctttacaaaattaataattaattgatagtccaacgacaattatatcaaagttctgccaaagattcataagcatttatgccggcgttattttctatcgaaaacttcaaaagtgtgggggtacttatttttgccgtcaacaacaccaacgaccgatttgctcaattcaaataaagaatagtcaatggctggcatataggtgtcaccggaaaattcagcttcaatcttcgtgcgataaagccggtcgacttttgaacgtaattgggcaaatagattggcacctccggtcacaatatattgtttatcgggattttgagcaatcaagtcacacagttgttcaatcgaagggataactttgacgcccgttggaaaatcagtttggtgtgaaaccacaatattctcacgacccggcagtggccgattataactgcggaaggttttcgatccggaaataatcgtattgcccatcgtggtttctttgaagtaatgcatatcgtccggcagatgccaaggaagttggccattggcaccaattaagccgttggcgtcttcagcccagataaaagctagcatcgacttcctcctaaactgcaaccggcgctttaatgactgggtatgggtcgtaatttttgaccttgatatcagccatttcgaattcatccaaatgtttcttttcaggattcagccacaattcgggtgcctgacgaggtttacgggaaaggagttcctcgacttggtcaatatggttcaggtaaatgtgggcatccccaaaggtgtgcacgaaatcgccaacttccaagccacactctctggcgatcatggaggtcaataaggcgtaactggcgatattataaggcacgccgaggaaaatatctcctgaacgttgatacaattggcagcttaacttgccatcgttgacatagaattggaataaggtgtggcaaggcggcaaggccattgttggcacatcctctggattccatgcggaaacgatcatccgtcttgaatcagggtgagttttaattaaatcaatcacattttgaatttggtcgatcgttccaccagtggaagtcttccaggcccgccattggctgccgtaaaccagacctaagtcgccatactttttggcgaaatcatcgtcgttgacaattcgatcacagaattgcttcttttgctcctgataaactttgttgaattcgggatctttttgtgcccgatgagaaaagtcagtcatatccgggccggtatagtcatttgaagcgacaaacttttcaaaagcccactcgtcccagatgtgattcttatgcttcaataaaaattggatgttggtgtcacccttcaagaaccataagagttcacttttgattaatccaaacggcactttcttagtggttaataaaggaaatcccttggataaatcgaatcgcatctgatagccaaacgtactgatggttccggtatgggttcgatcagcttttttgtggccattttccaaaacataacgtgcaagatctaaataggcgtcttctaacatggcaattctcctttttatcagaacgtgactgtttttaattattcagcgtattcgcttaaatattcccagcgtttcatttttttgtcggcctcggcagacaactggtccttttgtgcttgaagatccgccagcttatcataatctgagccattgttttgcatctgcttatcaatgtcttcaacttgtgattcgagcttttcaatgtcatcttcgatgtgatcatattcgatcttttcagaatatgtcaattttttcttggttttagcatttgaagcgggtgcgtcttgacttgagcttgccgaatccgattgagaagttgactgcccgctgtctgacttggcagacgatttcggcgccttcttcaatgaggccaggtaatcggtgaaccgaccgcggtgttcttcaatcacaccgttgcctttaaagatcagcaatcgatcggcaactttgtccaagaagtaacggtcatgggaaacggtaatgacggtcccttggaatttggaaatgtaatcttccaaaacggtcaaggtcgcaatatccaagtcgttggtcggctcatccaagagtaaaacatttggttgctgcatcaataatttcaacagatacaggcgtcgtttttcaccaccggaaagtttacggattaacgtgccgtgcatgaaacggggaaacagaaattcttcaagcaattcggcaacactaatcttgttgccggtattatcggtgacctgttggccaatctcactcaaataactaatgacccgcttatcttcaggaatcggctcggtcagttgcgtatagtaggcgattttgacagtttcgccgactttgataattccagaatccaatttcagtcgaccggcaatgacgttgagcaggctggtcttaccggcaccgttctcgccactgattccgatccgttcattcggctggacgagaatattgaaatccttgagaattgttttgccgtcaatggttaaattggcgtctttcatcttaagaacttccttgcccaatcgggtctggccaagggaaatgttgacatcctgatcaagctgtaaggtaccgacgttttcctttaagtcattaaaccgattaatgcgggcctgctgcttggttgaacgggccttcgcaccggtcttcatccacgccaattcctgtttgtagagctgttgagtcttatgctcggcttgaatttcaccttgaactcgggtcgctttttgctggacatagtcctgataattgccgtcatactggtacagtttgccaaatgacagttcccagattttgttggcaacgtgatcgagaaaataccggtcatgagtgacaacgatcaacgagcccttgtaggcagccagataattctccagccaatcaatggaatcaaaatccaagtggttggtcggctcatccaacaacagtaagttgggcgcttgaatcagaacttgtgccaaccccactcgtcgtctttgaccaccggacaactcggaaatcttctggttataatcggtaatcttcaactgggtcaaaatcgttttaacgtcactttgcgcgttccaggcgtcttcttcattcattcgggcttcagccttggtatatcgtttggctgcttctgggtcctctggatgcgttgaataatctttcaaagcagcttcgtaatggcgaattgtccgatagacagtttgcgatccggaaaaaacggcatccataattgacagactctcgtccagttctggatcctgctttaaataaccgatggtgtaagatttcgaggtaataatgtcacctgtcgagtcatggtcaatgccggcaatggcattcaataacgacgtctttccagtcccattagtcccaattaagccaattcggtcgtgttcattaataataaaattcagcttatcaaaaagcgtcttttcaccgtatgtttttgctaagttctcaacgcgcattgtttccattcaattatcagtcctcatttaaaaagttgatagctgcctgaacaagatcttcaggttcattgttgatcttatcggcaaccacattttgttcaagataattcaaaacctggccaagctgtggactgggttttaagacccctcttttaattaattcgccaccggttatcttcaactggtgcttatttttaatggcaagtcggttgtaacgttcagatagtccagtagttttcgactggtccgcaaatactgcgattgcgttgtcgacgttttcacttccggcatgataaagggttaaattagtcacttgaccacgttgaattgcgaaaagtaattcaaccgtaagtataacatcattaattattttattggcagtcttccacctttttaaaaagcgggtaatttgttggctgttgaatccgaatttaaaagccagaagggcccaaacctgaacttcattagtaagggtgaaatcagtgtcggcaatttgtctgagttgatctaaatgctcacccagtattgggacgtgttgatacaaattagtctgaatcatgatcttgaggccgtggttggcatctgatcccagcatcattttgacaaactcggtgtgggagcgttccacggcaatttttgccaataactggctatggagggcaatgccagctagtgtggcatcctcaatcttgaagtccaattggctggcaaaccggaccgcccgcatcattcgcaaggcatcttcattgaatcgctcattgggatcgccaaccgcgcgaataatgtgttttcgcatgtcgctaaggccgccaaacaaatcagtgacctgtccgttctcagccaatgccaaagcgttaatcgtgaaatcccgccgcttgagatcctctttcagggagcgcacaaacgtcacgtgatccggtctccggtaatcttggtagccggactcagtccgaaaagtggtgacttcatacccagtcccgtgatcaagaatcatgacggtgccgtgctcaattcctgtgtcaaccgtccgtttaaacaacgccttgacctcactgggataagcgctggtcgcaatgtcgacatcgtgaatcggccgctttaaaatcgtatctcgaaccgaaccgccgacaaaataggcttcatagcccgctgattcaatcttttgtaaaattggtaatgcttcgtggaattcttttggaatttctaccatccgcacaataatcgccatccatttaatatttatcctgttgtaattttaacagaatttccgcttgaaacaaaaagttcggtgaaatgattgccaattgtcaattagaattgctatgatgagttgtcagatcattcagggaggaaaaacgatggcacaaaagcaaagtcgcttcaaattagatatttcgttaattgatttactggtaatcgcggctggaaccgccatttattcatttggaatcgtcttctttaacatttacaatcatttagccgatggtggcgtgaccggtatcacactgattctccgggccctgtttcacattgacccggcctattcgaccatcctggtcaacgtgcccctgttcgcgatcggttatcgctacttaggaaagaaagatatgttttataccttatacggaacaattgccctggcgatctttttatggatttggcagcgggtcccaatcgtgattaatatcgatcacgacctgttgttgtcggcaattggtgccggcttatttggcggctttggctgtggaattgtttaccgctttggtgggacaaccggtggtgttgatattgtcgcccgcttattcgagcggtttaagggcgttcaaatgggccaaacgctgctcacaattgatgtcttggttttactgtcatcactcatttatttaaatgtccgccagatggcatatacgttgatctacgtctggattttttcaatgatcgtcaactttacccaacgcggcgcttacacggctcgggggattttgatcattagtaacgagtcagaaaaaatttccaatgccatccaagacgagctcaatcgtggcgtcacttttttgaatgccgagggaggctattcccaccgttccaaacagattgtctactgtgtggtctccccaagcgaactgcacactttaaaaaagctggtcgaatcgatcgatgaagaagcctttatttcaattattgaagttaacgaggcgatcggtgaaggcttcacttataagcggccaaagcgatttaaactgctatagaaccagaaggctatatgtatgataaaaggtcacccatttgggctatcccgccatggtttactttaactttagcgagatccctaactggtgacctttttctgatgtttagttgcggattgtgaatcacatttcatcccacaattcttccatttccatgtcatcgggaaccaaatccaagtattttttcaaggactgtttttcgagatccggtttgccgatttcgcggtaaaacagcgtggcgtgtttaagaaaatcgggattatcggaaagttcatcggcggccaattcgtaattgttggcggcttttttgatatcaccggtattttgataagacagtgccaaattataagcaagatgggcatcgacgacgtggtcttcaaaaaccccttctaaaagcttcagattatcgctgtagcgttcgtgagcaacgtaccagtctgatagtaaggtcaagatttccatgtcgtcaggggcgatctcatggcccttttggaaataggtcaaggctaaatcgtcttcgttcgccatttccgcaatttggccggccttctgccagattttttcgttaaattggtcaatggaaattccttcttggatcgcctttaacgcttcatcaacccgtttgaggttaacataggcatccgccaagtacgggtatagggagctgtactggggatctgaatcacgcaaatcctcgaaggctttaattgccttttgatactctttcaaattaaagtaggtgaatgccagttcaaatttaacgtcggcgttcatattaatcggcttgatttgttccagatagcccatcgcttgttcaaacttaccaatttcggcgtaggaaacacccagacgttcaaccaggttgactgaggacatttccaacgtaccagaggtgatcagcgctaaatataaattaatcgccttgcggtagtttctagtcgtgaaataaaattctgccagagcaaacttgatcacatcctcatcaggagccaatttttgggcttctaagagcttttgttcactaatctcgaacattccctgggtttggtacagatcggccgcaaccatcaaggaacggacgtattcgtccgactgcggcgaaacctgtgacagataattgagagctttgtcgtcttgatcatcatcaatggcaagttcggcgagattgatttttagaccgtcatcgttgggatattttttaaataatttttcgtaaatagtatttgagtaatttgaaaagccgagtgaatacagctcttcggccaatgagtacagcaaatcatccgaatcgtgatccaaagcttgctgaaatgatttcttaaaatcatcaatttggccgccttcaagttggtctaaagcagtttttgaatagctcatatttgtcctccaaagtgtataaaaaaagccagcccgacaaatgccgttctggcttaacagatgaatactatttaacagcatccttgagcgccttaccaggtttgaaagctggtaccttgcttgcaggaatttgaatttcttgacctgtttgtgggttacggcccttacgagcggcacgttgacgtacttcaaagttaccgaaaccgattaattgaaccttgtcaccttttgctaaactagcttggattgattcaaatactgcatccacagctgatgtagcgtctttcttagtcaaaccagttgctgctgcaacattggttactaattctgctttatttgccatgagtgtattcacctccctcaaagataggtatgtaaaccattgcaagtcgaattctcacaaatccggaatgctgaaataacgccgtttgccaacatcatttctttttcaaagatagcataagaatgccgtcattgcaatggttttgcccaatttagtgtcgataaacgccgaaaaatcaagattttgttaagaattgctgatttttgggctattttcggctgcgtttgatgattctgattggtgttccggtgaagtcaaaattatcacgaatttggttttcaaggaaccggacataagaaaaatgcatcaagtccggattattcacaaacaccacaaatgttggtggcccggttacgacttgggtcgcgtaataaattcgcagtcgtttgccattaaccgttggggttggatgaacagcgaccgcccccataatgacatcgttgagtgctgaggattgaacccgcttctcatgattgtcataaacctgtttgattaatgccggtagtttttcgattctttgcttagtaacggctgaaacgaaaatgatgggcgaatatgacatgtactggaattcatttctgatcagggtttcaaagtcctgttgcgtgtggttggtctttttgagcgtatcccacttattcaccaccgtgatgattgcttttccagcttcatgagcgtatccggcaactttcttatcctgctcacgaatgccctcttcggcgttcatgacgaataagatcacatcactttggtcaatggctttcatcgcccgcatgacactatatcgttcagtgttttcgtaaaccttcccgcgttttctgattccagccgtatcgaccatcgtgaacttgataccatccgcctcaaagcgggtatcgattgcgtctcgagtggttccggcaatatctgaaacaatgacccggtcttcacccaaaatggcgttaaccagtgacgacttgcccacattgggccggccaataatactgaaccgaatatcatcgttatccgtcttttcatcggtcttaggaaatttttcaacaaccttgtctagtagatctcccaatcccaggccatgcactccggaaatcggcattggatcgccaaatcccagtgaataaaactcatagatatcttcacggctctcaggattatcgaccttgttaaccgctaaaacaaccggtttatcacttcgataaagaattttggcgacttgttcatcttctgcggtaaccccttccttaccgctgacgataaagacaatcacgtccgcttcgtcgatggcaatttcggcctgactcttaatctgggttgcaaatggtgcatcactgatttgaattccaccagtatcgatcattgcaaatttagttgccagccattcaccatgagaataaatacggtcccgggtaacacctggggtatcttcaacgattgaaattcgatcaccggcaatgcggttaaagatagtcgatttccccacgtttgggcggccaataaaagccactgttggcaatgccatgtaaatccctcctttgcttggttaattcagaaagaaaggagctgggacaaaacttgcgttttgtttccagccccttttcatgattaaaataattgattatttgttatcatcgtcatcattgttgccggacttcttcaattcgtctccaatgatatcgcccaaagtaaagccggtttcttcttccggtgcattactgatggaacggtcgttagacttccgtgagcgtgatggtcggttgtttgacttctttggcttggcttcttcttcaggagcatcggtcaaagctttgattgataatgccaaacgctttcggtcagtgtcaacatcaagaaccttaaccttaatcttctcgccaaccttcaaaacatcagcaggtgtatcaatgtgctcatgggcaatttgggaaatgtgaactaatccctcaacacctgggaacacttcaacaaaggcaccgaaatcaaccaggcgcttaactgttccttcaagaacactgccaactggagctttttcttcgattccgtcccaaggttctggaagagtttgtttgattgaaagtgagattcggttacggtcgaagtcaacggataataccttaactttaactgtttggccaacctttaatacatctgaaggcttgtcaacacgttcgtaagcaatttgagaaacatgaaccaatccgtccatgccgccgagatctacgaaagcaccgaagttggtaagacgagcaacggttccttcaacaacgtcaccttcgtgaagagtttgcattaacttttcacgttcttcagctttttcagcttgaacaatagccttgtgagacaagatcaggcgattttcaactggatcaatttcaataatcttcaattcaagttcttgacccttgaattggtttaaatcatcaacgtaatggtcagaaatcattgaagctggcacgaatccacggacaccggcatcaacaaccaagccgcctttaacagcttggctgactttggcagtaatcgtttcatcattctttgacttttcagccaattcatcccaaactttgcgggtttccaaacgctttgaagaaagcaggaaactgccgccttccttgtcgctgccgattcgagaagtaacaaccaatttgagcttgtcaccctgcttgatatcgtcaacattttggtcagacgaaagttcacgtgggggaacaacgccttcaacaccggagccttcaatacccacgattaattgttgactgtcatctttggccaatacttcaccggtgacaacatcgccaacctttacttcattaacgctgtttaaagcgtttaataaatcatttttatcattatttgcattttcactcatcaaacaattcctccttgaaacaactctaatcataattttatcttaaattgaacaatattaccagtcaattgactaattagttgttatttcagtgttttatttatcacatctgcaatctttgaaaccacctgatcgatagaaagtgacgttgtatcaatttctacagcatcttttgctttggttagtggtgaaatctttctatgagaatctttataatctctggcctcaatttccaattgtagttcatccaaaggtgtattaatgcctttttgaatgttttctttgtatcggcgctgcgctcgttccgcaacactggcaatcaggaagattttaacttcggcgtcaggtaaaacggccgtcccaatatctcttccgtccatgacgatgccaccgtctttagcaatttcctgctgttgagcactgagttgctttcgaacttcgccaatggcagcgactgccgaaactgaattagtgacatcttcttgccgaatcgcctcggtgatttctttgccgtcaatgaagaccttttgtccgtcatcactgggctcaaaagtaatttttgaggcatggacaattttgccgatctcgtcaacgtcgtcaaaggagacgccctgacgaattgcctgcagtgtaattgcccgatacatggcaccggtatcgcagtagatatagtgaaattgctttgctacccgcttggcgacagtacttttaccagcagaggccggtccatcaattgctacttgtaatccattttttcgcattctaacattccttacctgacattatttttgagtgattctttaaagctaccgcacccgaagccgttgccccggatacagcttggaattggcattcagcccgttcatccgcatcagctgttcagtggtcaaaccgttattataagcaacccgaaacatcccctggccggccttgacagtggcgtattgatggccgctggcagcagtcgtcttgttagtcgttgaactgctggatgctgactgggcgttactagattgcacagtggaagcagacgatgtcgagctcgaggctttcggttgggttgaagcggctttactggccgactttggctgctctttctttacagctggcttggctttagttgaattcgatttggctttggccgctgaagaagattttttttttgcgttatcctgtcggacgaccctgacagacgaagacgcggcactctttgaatcattgcccatcgcactttggcgaaccaggccgtaaaccagcgcaaccaccgccacgataatgattaacgccgctaaaaccatcgtaatcagatggtggttttggctctgctttcgaagcttgactcgcgagagattaccgttttcatcacgatcctcagaaaatgtttgattccagggctgatcttcatcagtttttttatgttcatcattcgaattcatattgacccccctcttgatcaggatatagacaaacttattttatcattaattcacttaaatttaccttaattttttgataaaaacagctggtcgatgacttgctgccagcctttggtttcgttttgacctgatttttccggttgaatcaaatattgccggttaaaatcctgccagcgattccaaaaatcgacatcgtgatcgcagcaaaatgccgggtttcgttcgccatccgggactgtttcatcaaaatacttcagcagttcatcacgacggcatttttccgtgtagacgtattggaccatcgcccccagttccttcacccgccgagtacgagcaggatcaaagatcgatttggcctgctcaaacgagtcgccgctgtcgtggtaatatttgaccacccgaaactgatcatcggtggctaatgccttaggatgctgatacaaataacgcaataggctttcatccgggatcgtatgatcgatcagacccatttgtaagccgcggtcattgggttcatacatcaaaatcgccaaccccggctgctgatctctcccgcaacgaccaatttcttggacataactttgaatgttcgccggcaggtggtaatgaatgacaaagcggatgttatccttgtcaatgcccattccaaaggcactggtggcacagacaatgtccaaattccctgccaaaaactgctgttgaatgtgaaaccgcggctgactgtccatccccccatggtaggccatcacccggcgattggtttcattcgtcaacgtgttggcagcctgctcggctttactcttactggaaaaataaatgattccaggtccattgagctgcttgaccagttcaatcagagcagcgtctttatcatgttgattggcaaaaatttttgcacttaaaaatatattggcccgattgaccggcaagacaatttggtgaacgtcctcgaatcgaaaattcatatgccgaataatatctcgccgaaccggttgggtagcagtggctgtcatcattaacgtcagtggccgccccagcatctcccgcaccgtccctaatttgaggtaatccgggcgaaaatcgggcccccattcagaaatgcagtgggcttcgtcaacaacaaacaggccgatgctcagccgcttcaaccgttgttgaacctggtcatttgccagcatttccggagaaacataaataaactggtaacgattcaaatgatttaaaatcgccattttctcttgaaaatctaacgcggaagtcaacgcaaccacccgtttggatcccagaaattgcagtcgactgacctgatcctgcatcagagaaatcagcggtgacacaatcatgacccgttggcgggtgattgccccatacatctgataaagtaaagttttgccgccgcctgtcggcagaatcgccaaggtgtcctgatgggccaacagattctgtaagattttttcttggcccggccggaaggtgtcaaagccaaaatatttttttaattcacgtttgagatcaatgaccatctgtcgttttactcctgtatatctgaaaaagtcgaaattggaaaaatgccaattgattaaccacctgactggcatcttggaaagaccactcgcccacgtttgttggctgatgagctgctagttgattcatcaaatcttctgaaatcagggtcctatatggaaacttcgccaccggggtcaggatagctgcctccaagagatgttcataaaccgttgtcagcttgatgtgacgctgagttgcgatggcgtggggatttcgatccgcttgccggacaaacatcttaaaggtggtttgagcactgttggagataattggtttggccaatccggcagtcaatggtgcaaataaactcgtctttcctgcgcgcatgactttttccaggagcatcccatacaactgcagccactgcagttcgataattgtggtcggcacgtggcgtttgactgccacctgctcagctgtcaatcctgagaagtcatgtccaaccaggctttgaacgaagagatcagccagttcatcctggtggaggtcactcaaaaagctgtttaacaattggcggaaatgttccggtagatggtcctgcttatgatcaataaaccagcgttttaacagctgatcttcaaaataattaattgactggggatagtattgattgttaccgtagctgaattctgaaacaatctgggtggcaaaactgaaccgccgcatgaacttggccacatcatagcgcgacgaaactgccaggtgtttgagaggcagcagctgattcaaataagctcgctgctgttcgaccccctttgcagtcagttggattctgaagtcatcatcggcttgagccaacccgttggcagacaactgggtcaagactggctggtcctcaccaaagtcggcaccgtggagaacgtcgataaaatcaagcatcccatattccagtgcccagtataaattggaaacagtgcggcgcccccgtaaggtgtttttaatcgccttcacccgccgaaactgccgatcactaccaaaaattaacatgagaatgcctaagtccatgaactacctccgaaacaaaaagccagtccaaacccgcaagtttgtcccagcctctaagattactcactgttcaattatactatatcaaacaaattttgaatggatctatccacatttaccggagttttaagcgtggcaggaaactgttcttgattaggtagaaaacaccaccgacgacaattcccttgatgaagttaaacggtacaaccccagacaaaatgacggttgccagtggaaagcctaatttcatgccaatcaggttcatgtatagcggaataactcccagccagttggtcaatgacatgataattgtcaaggcaatcgccatggtcaaaattaccagtcctgctttcttccaccccttggtgaatgagaaaagccggtcagccaagtagtatgcccatatgagcaccaaagatgaaaccagggatgaacccacgccaatgaagttaatcacatcggcgccagtcgttacccagtaaagcaaggccttcaaaccagcaatcgtcatgccgccaaccggtccaaataagacggttcccagtaaaatcggcatgtctgccaaatccaagcgcatgtaaggcacgattggaataatcggcaccgacaaaaacatcaaaacatatgagagtccggcaaacacggacatctcaaccagacgcgttgttgcaaactgcgtatgcttaccactattttccattgaaaaaacctctcctccaatggtcaatcttcaaaataatgccctgacaaaaagaatttgtcagggcattacaaaaaatgtaaaatttaatcttctacataccagactttactgtcggcactggaatttcaccagctcagcacgatcactcgtgagtcgcggactatcaccgccggtcgggaatcacaccctgccctgaagataaaccaatttatttaattcaaatatagcagaaccaaggcaaatgtcaacgatttgtcttgcccgtcaattcctttaattcttcgacttcatgtggtttcaacggccgataatcccccggctgcaagcctttcaatgtcaaaaagccataggtttcccggcttaatttttcaactgggtgaccaattttttcaaacatgtttttgacttggtgattccgaccctcatgaatcgtcaattggacaatcgacgagtccttgttggtgcgaatcagcttggtcttggccttggccgtttttcgatgctcaattacgacgccagtccgcaagtgtttgaggtcgtcattggtcacaattcccttgaccttggcgacataggttttttcaacctcgtactttgggtgggttaatttgttgtccaggtcgccatcgttggtcaataataacaggccagacgtgtcatagtccaagcggccgaccggataaattcgttcggggacctcttctaaaatatcaaccacggtctttcggtgcttgtcatcggtcaccgcggtgatgacccctctgggcttgtaaagcaggtaatagactggggcttcttttgaaatcggcacttcgtcgactttcacctcatcgtttggggtgactttggttcccagttctttaactacctcgccattgaccttaacgtgtcctttggcaatcaattcttcagccttccgtcgggacgcaactcccgcgtgtgcaatcactttttgtaaacgttcttcattcatacatccacctcctaattttctttatcaatttctttgttaaaacgggttaatagtgaatcactggtgtcatcatccaagacttcatcctttggcaatggcggcaagtctttcaacgacttcaacccaaaataatccaggccaaaattggtgatcccgtattgcttggggttgccgacctcttctttgaccccagtcacttcgatcaaatcctggttgaccagccggtggagaatcgccgaactattgacccctctgatctgatcaatttcaattctggtaatcggttggttatacatgataattgaaatggtttccaatgccgcttccgacagaacccgcggtttggcatcgttgacataatcgcccactaattcagacaattcttccttggttcccagccgatagacgttgtcgctgacaaacacctttaagccgctatcttgatcttggctatatttttggacaattttttccaacaattgccggcaggcggccaccgttaacgccgtccgctgggacatttgccgcaacgtgatgccttggtcaccagaggcgtaaagcagtgcttcaatttttgccagattactgatcaacgtatccaggcccctttcgaatttcaatggtcgactgtacggttgcttggttgagccggacttcgttatacttggccatttccaaaattgctagaaaatcggtaacgacctcttcggtttgagttgaattggcaaccaatttatcgaaggaaatccggttatcagtttggtttaacagctcgcgcacccgttgactctggccttcaatcgtaaaggaccactcgtgaattaccgtcgacatgggttgattatacttgaagtgtttcaaagcatccacgtagctggccatgatgtcgccgctgttgaacggagatggctgaatcagttcggccttggttggcgccacgctcaactcggagcgggtaaaactctcccgccgtttcatttcccgctttttcatactggcagccaccagtttgtaccgcttataattcagcaactgggacactaattcctcacgggggtcggcctgctgttcatccggttgatcgtcagtaatcgtcggcagcagcatctttgacttgatgaccatcagtttggcagccatcacaaagtattcgccgacaatttccaaatttaattgctgggcatcatagatatactgcatgtattgctcggtaattcttgaaatctgaatatcataaatatccatcttggattcctgaatcaaatgaaggaggacttccagtggcccgtcaaaatcattcaaatgtaattccggctgcttgacttcaggcatgattaatcgcattctcccatttttcccaggcggctcgattttcaaagccgaccacaatttgatattttggatataaatcctggaggtcgtcaaaaatccggttatagttcccctgactgacgctttgcggggttaacaccaattgatgaaccaacagctgatttccttgaagttcaatgccgactaaacccgaccaattattggatgggtcccgccacaaataaatcaatcggtcgtctttggcggcgtaccagctcatttcttgggcaaccaagtccatattctgcagctcggaaaccaacgaaaagaggcccatcgtgatcttttcataatcttttcggtattgatataacatttattcaacctctttcgttatgctcgcggatgatatttattataaacttccgttaaatgcttatgagaaacgtgggtgtagatttgagtcgtcgaaatatcggaatgccccaacagttcctgaacgattcttaagtcggccccgttttcaagcaggtgggtcgcaaatgaatgccgcagtgtatgtggtgtgacatggcgtttgatgccggcctggttgacatattttttaatcatctgccagattgcctggcgggtcagttggtgaccgtgggcatttaaaaataggaactcggagttgggccttcccgaaagtagttggactcgcgtcgattggatgtattgattcaaccagtcgattgccacgtcgctgatgggaatgatccgctctttgtcgcccttcccaattgtctgcagcaagttcatcggcaaatgcaggtcacccaacttcaagttaaccagttcactgacccgcaggccggtggcatacagcgtctctaggattgcgcgatcgcgcagacctaattttttatgagtatccggcatcgatagtaactgattaacttgggccacagttaaaacgtccggcagtgtctgggcctttttaggcgaatcaaccttgagcatcggatcgtcaacaatcacgtggaattgaaccaagtactggaagaaccgccgtaatgtcgagaccaccctgataaccgtgttccgggctttatgctgccgttgaagagtttctaaataatccaagatgacaaattggtcaatgtcggcaattgatttggcgtgtttgtcaaaaaaagcaccggcctcctgcagatcctgccgataacttttaatcgtattatctgaaaggccgcgttcgacccgtaaataatgaagatagtcctcaatttgttcgtgcatcataaaagcctactttttcaaggaaatgtggccatcagcttgttcgatcaggttttccttcagcagatgtcccaacgcccgtttgaatgcgcctttactgataccaaagtaatctttgatggaatccggcgtacttttatcactgaacgccagttgtttgtcgtcggtatgttcaatggccgccaaaatcatctgagcgtcttcaccaatttcttggtaagcccgtggcttggtggaaatattgacactgccatcccgaagcatgccaatcactctggcttcaacttcctgtcccaaacgtggctccatgagtcgttcgtcaggatgcagaaaagccaaattgtaatcctcggtcaacaaccgggttccagaaatcttaagacgataagcccgagccttaagatttttgttctgcagatcatccttggccggcttggcaattgccgcaaaaatttcttcgtcggctaagtgaccccaaattcggtttttgttatccaccgtcaaatcaatcagcagttgatcaccgtcttgcggccacaatgaccggaccgtcggcagttcatcaattgagacaacgacgtctttattgggtaagccaatgtcgacaaagacccctaaaccaaatttttccttcacaacggtcgcaaaaccgtaatgatcacgacggatatccggaatgtttctggttatttgcattttatgctgttcattttcatacgtaaaaccagtgaaagatgcaccgattcgcaagggtttcttgagctcagtcttatcaaggagaaatgtttctccttcaatctgaacgtaatagtccttgtcattttcatcgatgaccttaccggttacaacttgcgcaataatattattcatgcttatctccgatctaatcgagcttaatcttattttacacgtttttcagtgaaaattcgaccgcccttatcataacaggaaacaggtccgaacggattaaccgcccggacctgtcatgattaattgtgattactcacaagttaaatttagattgatgatgaagcaccatggtaaataacgccacgatgtgaatcaacggtaatcaattcaccgtcagaaatcttgctggtagcatcagctgcaccaacaacaacggggattcccattgaaataccaacaacagctgcgtgtgaagtcaagccgccggtttcaacaactacggcacttgccttttcaatagctggtaagtattctttgtcagttgacttagtaaccaagatactgccttcagttactttgctcttggcatcagcagcgtttttagcaacaaccgctttaccaataacagtcttgtcaccaactccttgaccttgaaccagctttgaaccgatcagttggattctcatcaagttggtggtaccactctcaccaacaggaactccggcagtgacgataatcaaatcgccttccttagctaaaccagtttcgagagccttctttgaagctagttcaaagatttcatcagtgctcttaacttcgtcaaccaagattgggtgaacaccccagttaaccatcaaaccgcgacgagtacgttcgtcaaaagtaatggccaggatgtcagcatctggatgatacttggagatcattcgtgcagtgtaaccagaacgggtagctgcaacgatgcagtgaacgcctaattctttggcaacacgggcaactgagtcaccaattgattcagtaacatcgcttgagtcaaattctggacgtggggtaccaaattcgctgaaagcattttcagccttaacgtcgatacgagccatcgtttgaactgattcaacagggtaatcaccattagcactttcaccagaaagcatggttgcatcagtaccatcaaagacggcgttggcaacatcggaagcttcggcacgagtaggacgtgggttttcctgcattgaatcaagcatttgagtagcggtaataaccggcttgccaagttggttacatttcttgatcaaagtcttttgaaccaacggaacgttttctgctggaatttcaacacccatatcaccacgggcaaccattaaaccatcagataccttgatgatatcgtcaaagttgttgataccttcttgcgattcaatcttagggaagatttgaacatgttccatgtgtttttcttcaagcagttcacggatgtccaaaacatcttgggctttacgaacgaatgaagcagaaatgaagtcaatgtcattgtccaaaccaaaacgaatatcatctgaatctttttcagtgataccaggcaggttgattgaaacgccgggtgcgttaacacctttacgggaaccaagggtgctgtcgttttgaacagtgacaactaattctttgttagcatcgtcttttttagtgacaacagtgtccaacaaaccatcatcgaaaagaacatggccgccttcgtgaacatcgtcaaagagtccagggtaagtaaccgcgatcttgtctttagtaccctcaagacttgcgtccattgaaatacggaaaacatcgccagtgtggaattcgatcttgccgtctttttgaacagttgtccgaatttcagcacctttggtatcaagcataattccaacagtcttgccagtcttcttttcagcttcgtgaaccttgttcatacgatcaagatgttcagggtggtcaccatgtgaaaagttaaatcggaaaacattagctccagcttcaatcagcttagtaattgtgtctacatcagtacttgctgggcctaatgtacttacgatcttagttttcttcataagtaaaatctctccttcggtttttgggcacgcaacaccttattaaaatgtcgcaaaacaatttaaataacgcatcggtatccttttagatttcaatcgtattttatcactttttaagcgggttgtcgcccaccttttgggggtaagcgggctttccagcaccgacttggaatggcaaaagttaggtctaccgcaaatgaaagcctttacgtaatgaacctgacttctgaaaaattattccaaaaatttacttataaaccacattattcctgccaaagattgtgattaattgctctttggtttcagaacttggatttagccacagcttgtcctcgagctgccaagtttttttggtttctgtttcaaaaacgatgaccgggacctggccgtgatattggctgctcaggtcggccagtttgtgaaacattgtatttttgtcatgatcgcgatcaattcgcaaataccatttagattgctgttttgatcgcttgaggttcatcagggcgttagccgccggctggatgtcattggcgaccacctgaagatcgttgactttctcgacgttgcctttgatcaaaatcaccaagtctttatgaagccatgactgggtcttggcaaataagttgggaaagacagtcaccgaagtctgccccacctgatcattaccgtctaaaaaggccatttgtttgccggttttggtccggataatcttaaccttggtaatgtagagaatcaagtaaatatttttcataccggcactcaacgtagcggttgtctcagcatttaatcgctgttccaagggggcaaatcgttctgtcggatgaccagacaaataggcccctaaataagcattttctttttccagcttgtccatcagaggcatctcaggcatctttggcattttgggttccaacgctttgaacaagctcatcgaattgccacttaattcaacggagctgataaattcaggggcggcagcgattaattcggaacggttaaatggaaaaacatccaatgcgccggcataaatcaaggcattgatcaattcaactttgcggtacttgccgggcaggcggcttaaaaagtccggaaacgacttaaatggcccgttttgttgtcgctcagccaataaatccactaccatgtcgtgacgcacgcctttgattgaatcaaggccaaacacaatttgttgatcttgaaaggtaaaccgggcttcactatgattaatatttgggccaacaaccttgacccccattgatttggcagcttggaggtattctttgaccttaaccgaattattgttgaccgaatttaacagcgcaacgtgaaattcgcccgggtaataaactttcaagtaggctaattcataagccatcttgctataggcgaccgcatgggatttgttgaagccgtaattggcaaaccgctcgatatagtcaaagaccttattggcgactgaatctgaatatccccgctgtttggcgccggtgatgaactgagccttcatttgttccatcacgccaagctttttcttactcatcgcccgccgtaaaatatctgcttgacccagagaaaaaccggccattttggaagctaccagcatcacttgctcctgatagacaattacgccataagtcggctggagaatatctttgagcgagtcgtcggggtaggttaacgcttcatgattggtttttcgcttaaccacctcatcaatgttctgcatgggtcccggtcgataaagcgcgttgaccagggcaatgtcttcgaaccgttcgggatgcaggcgcctaaggacatttcgaatgccgttggactcaaattggaaaatgccagtcgtgtcaccgttggcgaataactgaatcgtcttggcgtcatccaagggcacagcagaaatgtccagaacctttccggtggttagttgaacctgttgtagtgcatcagccaaaattgacagattccggagtcccagaaaatccattttcaacaaaccaaccgattcaacataatctttggaatattgagtcatcaacagcccttcgttgccattttgaagcggcactaaattcaccaggggatcgtcgcttaataccagtccggctgcgtgggtcgaatagtgtcttggcaagccttccagcgtctgggcggtttggtagagtgcttcattaagcggactgtcagccaccagattcttcagtcgctgggaattggccaaagcatccttgagggtcacgtgaaatgcgttgggaatggccttactccactgatcttgctgggcagtattcaagccaaacacccggccgacatctctgatcgattgcttcgctgccaaagtgccaaatgtgatgatttgggcaacccgtttgtgaccgtatttttgatggacatattggatgacttcatcgcgtttgtcgtctggaatatccaaatcaatatccggcatctgaacccgttcaggattcaagaaacgttcaaacagcaaatcatatttaattggatcgacgtcggtaatcgttaaggtatacgctactaatgatccagcggccgacccacgccccgggccggtaatgatgtgagtctggtgagcgaaattaatcacatcccaaacaatcaaaaagtaattatcaaagcccatcgaatgaatcactgataactcctgatccagccggcgatgataaggggtcgcatctttaatctgatttttctttaatcgatccgccaatcccgtttcgcaaagctggcgcaggtaagttccggaatcgataccgtttggtgtgtcgaattgcggcaatttgggctgctgtttcttaatctcgacattgcaatcagcgacaatttggtcgacttgcgtcagtgcgtcagcgaggtgaatctgacggtattgagcctcaatttgtgtggccggacgcagccaatagggccccacttgcttactgagttgggccacgttggcgattttttctcccgcgccgatattttttagaacctgcatggaaaaatagtcggtggcgtttaagtattcaactggcgaatccgccaccaaagcaacttgcttgtcagccgccagcttacttaacatgtcatttaagctgtcagaggaatggtagtcgacaccgattttaagggcattaggatcgacgccaagggatttgacctgatcaatcaaatcagcagcgtcatcagcccgcccttgtagaagcaggtcattcatttctgctgccggcggcaaaatcagaactaaatcacttaaatagtcacctaactgagaagctgtcaattcgggtatggtcatcttcaatgttgataatttgagaagattggcatatccttgctggtttttggcaatcagcacccacccatattctttatcggtcaaaatcaagccggtcagctgcaaagtcagaccgatcagcggcttaacgccagcctttaaacaagcgtcgtagaattccacggccccgtacatcacgttgaggtcagttaacgctaacgcctgataaccgcgatccttggcttcagcaatcaagtccgcaatgcgaatcggactctgcagtaaactgtatgaacttatgacttgcaacggaacataactcacaggattgcccttctttcttaattaaaattataccaaatatatcaagcccacattcaaattggcaaattaaataaatgatgatttttcacaaaatatatgctaaaatgctattgattgtgaggtggcattagacatgaaacttattagttcaaatattgtagctgttttgtgggcatacatctttggagaaatcattggttacataggttccgccctcgaagttcgaacatgggatccttcccaaatcggaattgctgccgcaattactgcatttattgccgtaaacggtatctatctgatcagcaaggattctgcaacatcaagtaaatcaaaagaatagtttttcgaaacgttaaaaggctatggcagattttgccatagcctttttgttgtctcaatcaactttactggtgtgtgtcaaagaactgcagcagacgttcaaaaacaacttcccgatgcgtttcttgaagaacctcatgcttcatatgcggctcttgaagactgactacatttcgatagccgatctcatgcagcgttgcaaccgtgtctgccaagcccttctgaccaccactgaacttatcttcactgccgaccaaactcagaattggcagttgtggattgtgacagtcaaatttttgaaggcgtttcagggaataatcgccctgccacagtgttaccaaacttttaaccggatattcatccatcattaacggatctgtactgacccggtgaatgtttgcctgattatagctcaaccaggaatgatcccccggagttagaccggaaattttagatagcaaggaccatttagcatcttcagaatggcatttcaaaaagacccaaccaatgaataagccaagcggcaccaccggaatatagttggtggtcccggttaacgcaaccgcattgacttcctggtcgtggtgctgtaaatacaatctcgccaagatagatccaaaagaatgaccaaacagactgactggcaaattgggataccgggctttgatggattgggtaaccaacagctgatcatggatcaattgcggcagactgcgcatcatcccccaagggtcatcgtcggaaactgattggccgtggccgcgattatctgagatcaccgcaacatagccatggtcactcaaaaaccggcaaaattcataataccgttccttatgctccaaggcgccatgaataagttggacaattccctttggatgatcagcgggaaaatacgccaccgctaattgagtttgattttcagttggaagctggtaattaatcggcacaccgaattcctccccaggtagcttggtttaaatctgttcgtcagcaggtaattgttcaggaacaaagcttaactgatcgttatcaaggttaatgtgaacaacgctgtgaggcttgatctgatcagccacgatcattcgtgccagcggagtttccacgacgttggtcacataacgctgaagcggtcgagccccatattgcggttcatagccgttattggcaatccagcgtttagcctcgtcagaaattgacaatttgatgtcttgagccttggtacggccagataactgattaatcagcttctggacaatctgttcaatatcggccttcgtcaacggtgtaaaggtgatcacatcatcgattcgattcagaaattccggtttgaacgaagcttttaataattggttaacctgctgttgggctttttgtgaaataaccccgttctcatcggtgccttcaagcaaaatgtctgaacctaagttagaagtcatgattaaaatggtgtttttaaaatcgatcgtccgtccctgactatccgtcaaacggccgtcatccaagacctgcagcaaaatattaaagacatccggatgtgccttttcaatttcgtcaaataagacaatcgtgtatggattgcgccgcacggcttcagttaactgaccgccttcttcatagccgacgtaccccggagcagcgccgaccagtcgggaaaccgattctttttccatgtactcagacatatcgattcgaaccatgtgattttccgaatcaaacaagtcttcggctaaagccttggctaactcggtcttcccgactccagtaggccccaggaacaagaatgaacccagtggcttgcttgggtcttgaaggccggcacgtgagcgaataacggcatctgagacagctgtgaccgccgcatcttggccaattacccgtttgtgcagattgtctgccaagtgcagcaatttctttcgttcaccctcaactaatttggtgaccggaatgccggtctctcggctcactaccgccgcaatttcattggctgtaaccgattcactgaccagccaatcggaatgctgatcgttatcttcaagcttcttcaaatcggcttccaactggggaatcgttccgtgctgcaacacggcagcctgattcaaatcataggtgttttccgcctgtttcaattcattcttggcctgatcgagttgtttctttttgtcggaaattttcttaatagcttctttttcctgcgaccaacgggcatttaactggttgactttttccttaatattggccagttcttcttcgacttctttaagccgcttcttggatgcttcatcggtttcctgcttgagagcagcttcttcgacttccaggcgcatcatctggcgcttggattggtcaagttcagttggactggaattcatttcgacccgaatttcagccgaggcttcgtcaaccaaatcaatagctttatccggcaaatagcgatcggtaatataacggtcggatagtttggcagcagccaccaacgcgttgtcatggattctgacgccgtggtgaatttccaaactttcggacaagccacgcagaattgtcaccgtatcttcaacggagggttcgtggaccatgacccgttggaaacgacgctcaagagccttgtctttttccatgtacttccggtattcgtcaatcgtggtggccccaattaaatgcaattcgccacgagctaacatcggctttaggatattgccggcatccatgctcccctcagctttaccagcaccgacgatgttatgaatctcatcgatgaacatgatgatttggccctcggcttttttgacctcttttaacaccgcctgcaatcgctcttcaaactcgccccggtacttggcgccggcgattaatgatcccatatccaattgaaaaatggttttgtttttcaggttttccggcacgtcattagaggcaattcgcattgccaagccttcaacgaccgccgttttgccgacaccgggagcgccgatcaggaccgggttattcttagtctttcgagaaagaatccgaatcacatcgagaatttcctcgtcccggccgataattggaccgagcttattgtcccgggcagcctgaactaaatcggtcccatatttttcaagtgattgataactgtcctcttgattcttggtcgtcaccttttggccgccacgaattttttccacaacgttgcgcaccttttgctcggtaataccctgttgagaaagataatcggcaaatttgtcaccgtgtaactgcatcacagcaatcgttaaagtgtcaacagcgatgtaggtatcgccaaattcatttttaatctgttcagcattctgcaacagttcgtacaaattggaagagagtgactgaccataattaatgttgctgccttcaaccgtcgcgatggcatcaatttcagcatccagttcatcattcagatcccccaaattcaatccgagttgagaataaatctctcgggccaactcgccgggttgaaccaagaatttgaataaatgggccacggtaatgttttgctgctttcgagtagccgcaatctgttgggcctgagaaattgcctgcgtgacggcttccgttaaattatcaggattcattaaattatcaccttattaatgtattttagttgacgattttttcaagaattcgttctaataaaaaggttcgaaacaaaaatcattcttttcattccaaaccactaacgctatactatcaaattttgaatgccctgaacaataatttgaccttttttgacctattacttttcagcgtataatttggcgatttccagtaccacgtcaaccgctttttccatggtttgctcagaaacatattcaaaacggccatgcatattctcaccgccagcgaaaatgttcggcgtcggcagtcccatgtaagaaatcttagacccgtccgttccgccacgaaccgggaaaacatgcggtgtaacgtcaacgtttttcatcgcctgttcagcaatttttaccggtgtcggatcctttttgataatttctcccatgttgtaatactggtccttgatggtcaccttaacccggtcttcaccaaagtcactgttcatttggttggcaatccccttgaagagtcgttttcgagcttcaaagcgatctcggtcatggtcacggatgatgtagcccatttcggtgtggtcgacggttccctggaaatcatacagatggaagaatccctcccgatcctgggtcttttcaggacggtcaaagtcaggtaaggcggcgtggaaatccattccaacttggatggcattgaccataatacccttggcctcagctggatgaacatcggttcctttgatcacgacttttgcatcggcagcattaaaggtttcgtaattcaaatccccaagtgggccgccatcgacggtgtaagcaacatccgcgccgaaatctttaacgtcaaaatggtcggcgccggtaccaatttcttcatccggaccaaaagcaatcttaatgtcaccatgtttgacttcgggatgggcttgtaaataggtgattgcagcaatgatctctgctacgccggctttgtcgtcagctcccaacaacgttgacccatccgtagtaatcagggtttggcctgcatacttcttcaaactgggaaagactttggggtccagcgtatattcacccttctcatcaagtttaatgacagaatggccatcataattctcaacaatttgtggttgaatattttcagcattaaaatcagccgtatcaatatgtgaaatgaagccaacggttggaacggatttgtcgacgtttccaggaagcgtggcaaagacataggcactttgctcgttggtgtgaacgtcttttaagcccattttagtcagacgatccttcagttgattcaaaaaccgtgtctctctatcagaggacggaatgctcgttgattgaggatcagaacgggtattaatctttacaaacgttaaaaagttgggaattaattcggcgtattttgccatgacagttatctccttttatctacataaatgtgaatggatcggtattgatagttgactgataaatagccagctgccagtgatactggtcggaccactgtttgaacagctcggccaatttgggaatacaaatactttcaatgtggtggccagggtcgaccaccgggaaatcggcagccagcatgtcgtggccggtatgataataaacatccccggtgacatatgcgtcggcgcccttctgctgagctaagtggaagaacttgccgccatcgccaccaagaatggcaactcgtttgatcggctgagccatgtcgtgagcgattacccgaaggccggaaacaccaaaggtctgcttacagtcttcagccagttcacggacagacatgctgtgcggcaaatcaccgattcgacccatcgtaaagtgatgctttttgtcttccaggcgaatcaaattgtaaagtggcttttccagcggatgaacatctgacaaagtcttcagaacctgatgaagatttctttcgggaacttcaaattccaagcgcgagtcttcgatttcatttggttcaccggcagtccccatagttggatcggcgccggccttgggaacatagtagactgtcccgtcaatttcgtaggtatatccactgtactgagcagcactggcctgcgcaccggcatcgacaagtgacattcgaacagccgtcgcatagactttaggcacctgcacggttaatcgaaagaccgattcatcataggctgggaccatcccacttagattggttaactgaagtgcttctgcgagccaatcgttcatcccaccgtcagcagcgtccaaattagtgtgggcagcgtaaaccgtgatgtggttggcaattattttagcgtacatcgcattttgcgggtcatcgagatcaagattatgagctggatgaaacatcaccgggtgatgagcaaaaataaagtcaacgtggttggcaatcgcctcatcgacgacttccgggcgaacatccaaagtggtcatgactttgtgaatttcctgattgagtgaaccgatttgtaagccgaccggatctttttccattgccaattttttgggggcaaattgctcaaatctttcaattaactgcttagctttcaaccttgatcacctcattgattagattaatttctgactgaatggccgtcatttttgccgtatcgggagtggtggcctgacgcatattcttaatcacccgctttagcaggccaatttcttcctgccatttttcaacgaacaccggcgatttttcttgtagcaaaaatggaccgaactgaagggccaattttgaataagcgacgggtttgtcagcttttttagccgtaataatttcatagatatggccgtcttcttttagaatctgctcagcaaagattcgatattgattggccatcagccagtttctgacgaccggttcgccgacgtttggctggagaatcaatttttcttttccggtcagtttagctttaccagcttccaaaatgtgggtaatcaggttgccccccatgccggcgatggtgatggcatcaatgtcgtcgccgggttcaatggctgccaagccatcggcaagtcggggatgaaggatatccaataaatggtccttggtaatttctgatgtcgcgttggcaagcggccctttggcaacctcgccgacaacgccatagtcgataacatgattttgagccaagtgaatcggcaggtaggcatgatctgagccaatatctgccagtcggctgccaggttcaacgtggtcactgacagtttgtagtcgtttcgataaatgcgtgctattcatattttgctcctcattttgtgtataaattcattataaattatcctaatggaaaatgacagattccgagaagcattttacttggaagggccattttagcggacaaaaaaagtcggaacaccgaaatgccccaactcaatgaatgatcatattaaattaatctaagaaatctttaagctgcttgcttcgtgatgggtgacgcagctttcttaatgccttggcttcaatctgacgaattcgttcgcgagtcacaccaaagactttacccacttcttcaagcgtgcgggtacgaccgtcgtcaagaccaaatcgcaaccgtaacacattttcctcacgatcggttaacgtatcaaggacgctctcgagctgttctttgagtaattcataagccgcatggtcagcaggagaagttgcatcctgatcttcaatgaaatcaccaaggtgactgtcgtcctcttcaccaattggtgtttcaagggaaaccggttcttgagcaatctttagaatttctcgaaccttttcagttggcatgtccatctcggcaccaatttcttcaggtaatggctcacggccaagatcctggagtaattgtcgttgaattcgaatcaacttgttaatcgtttcaaccatatgaaccggaattcgaattgtccgagcctgatcggcaatcgcacgggtgatggcctgtctaatccaccaagttgcgtaagtcgagaacttgaatcctttacggtaatcaaacttttcaacggccttcatcaagcccatgttaccttcctgaatcagatcaaggaattgcatccctcgaccaacataccgcttggcaattgaaaccaccaaccgtaagttggcttcggcaagttcctgcttggcttcttcgtcaccggcttcaattcgcttggccaatgaaatttcctggtcagcactcagaagtgaaactcgaccaatttctttcaggtacattcggacaggatcgttgattttcacaccagtaggcgcggaaacatcagaaagttccttcttggtcactttcttggcagcaccgatggctcgcggatccggatcgccgttttcatcaacgacactgatcccggagtcctcgatactctccaagaggccttccatatccttttcactcagagaataaggcttttcaatcttcttttccaattcgtcataggtaatatggccaattggcttattagccttaacaatggcgtcaaattccttcttgtatggcttgtcagcttttttggtcgtcttggccttagttgtcttcgctttggttgacttggccttggtactggtctttgatgcagtcgttttcttagctgcagttgccttcttagctgtggcagtctttgtttctgttactttatcgtcggtttttttagtagccatcaaaacgcctcctgaagttatacttgttgcttcattctcttctgttgttcaagcttaacaatctcaatcgttaacgcacgttgcttgtcaacatcaccaatcttaacggcttgcttgagttctgcccgctttttctttaacttttcttccaccggggctcgatgcattaaaatgtttaaatagctatcaatttcagcattggtcggattatccggaagctcgagcatgtcaatatcaactaatagactttgcagtgagtcttccgaaatcagattgctgaacgtggcaacattataatcatcgaatttggtaaaatacccctcggctaaaaggtacaacatttggtactgttcatcaacaaatgagaaccccgaaacattacttacctttaaccaaatatcatggtagtgcagcatacggttcatcagctgcatttcggctttctcaactaacgagaaatgcttttgctgtttaacgacctgaacctgcttgtggtatggatgcggttcagccgccggggcgggttgtctgatcaatggtgctaactgctgttgcagcaattgcttggccactgaaaattcatccgccaaccggttaaggtaaagatcccgtgaaatgccggaatccactctgctaatcagctttaaagcttcagcaatgtaattagtttggtcaatctcagaatccaaattgtattgttttttgagataattcaattcaaactcaactggagcctgagcatggtcaatcaactgtttaaaatcgtcggcaccttttttgcgaatgaactcatcaggatccattccatcaggtatcgagatgattttcatcaccaaattgctcttctgttcattgaatgaatcaatggcgcgtttgatcgccttttgtccaggcgtatcaccatcataggaaatcacaacttcgcgcgtaatccgtttgatgtcataaatctgctgctcggttaagctggttcccatcgaagcgattccggacttgatccctgcttgaaaggcagtaatgacatccatgaatccttcaaataagattgccggctcaccggtacgaatatttgacctggccaaatctagattgaataacacttttcgtttgttgaaaatgtcagtctcaggactgttcaggtacttcggcatgtcggaatcagtggttaacaatcgcccagaaaaagcaatcgtttgaccggatccatttcgaatcggatacatcacccggtcgacgaaacggtctcgcaaattgccatcctggtcttcagaaaacaggccagattttcgcagcagttgaaaatcaactttgcgctcgtcgaaaaatggcttcagcaaccgctgtgccggagcatatcccaactggtaagtggcaatcgtctggtcggtcacaccacgtttatgcagataatcgagcgctggctgccccatcttggtattggtcaaaatatgatgatacagcttgacgctttgctcgtgcagatcaattaatgctttttgttgtgtgttttcgggacttgattgggaattgccgctttcacggaaatacttctcatcaacagaaatattttccatctcagcgacctttttaactgcctcaggaaaggaaacattctgcagctccataatgaacttaaagacgttaccgcccctgccacagctaaaacaatgaaaaatctgtttatcttccgagacggaaaaagatggggtccgctcctcgtgaaacggacaaagaccaaataaattctttccggactgtttcaattgaacaaactgggagacaacgtcaacaatgttaacctgtgacctgatttcttcaatcacatcttctgggatcttcgccattacttcgcctcccatcttcaaaactgaatcaatgcctgtaaaaagccgcacccaaaagtgcgacttgttttactggcgatacgtatttaaatattatcataaaacattaattagtacaaatattagccctcaaaattagcctttgacaaccaatttatcgaggtcgccgagatacataatcatgttggcaatcatggtgagttggcgcaagtgattattcttcagcttttcatctttggccatgaccatcgtggcatcgaaataatcattaattttatctttgagctgagctaaacgaccaaagtcttcttcggcactttgatgagtgtaatccttggcggcagctgccacagcctgattcaaagccttctcggaatcattttcaaacaatgccggatcaaccgttaagtcatcagccttgaaggcgcccttcttggcaatccgctgaactcgggtcagcgattcgataatgtccttgaagtcggtatcgtctttatgatcctggagtgttttggcactggcaatgttgaacaggatattggtgtgggaaccagaggtcaccgcatcggcaatgtcgtaacgaactcccaggtcgtccaagtactgtttgatccggtctttgacgaagtcactgacggcaggaacttgggctttcatatccagttttggtgcaactgacgcttgatcttcacgatcaattaacagattcaaagtctgctccaaatcaaagtttaactgcttgtcagcgacaattcgaacgacgccggttgcttggcggcggagagcatacggatcgtttgagccacttgggatcatcccggcagcaaagaacgtcaaaatactgtccagtttgtcagcaatcgccaaaattgaaccgacgttggtctttggcagctcaccatttgccgaaattggcatgtaatgttcagaaatcgcggtggcaacagcttgatcttcaccctttaacaaggcatatttgtcgcccatcaccccttggagttccgcaaattcaccaaccattccggtaaccaaatcaaatttgtaaatcgaagcagcccgctcaaggtccttgagctcctgctcggataggccagcaaggttcccaaggtattttgaaatcacttggactcgttgcatcttctcatacattgttgaaatcttatcgtggaagctgactttcttcaaccgctcaacgtaatcggcaatcgacttcttttgatcttcttggtagaagaacattgcatcatcgagtctggcagtcaagactttttcgtttccggcaaccacattttgaatatcataatcattaccgttacgaactgagataaaatgcggcaaaagtttgccgtcttgatcagtcacgtagaagaagcgttgatgatccttcatggaagtgattaggacttcatcagggatggcaaggtatttttcatcaaagttgccaaagaacgcggttggccattcaaccaagttattaacctcttccaataaatcgggatccagattgatctgccaattgttgtcagcagcaatcttgataatctgcttggtaattaattccttgcgtttggcggcgtcggtgacgacatactgttcagtcagtttttcttcgtattcgtcggcattggcaagttcaatatccttgcctaagaaacggtgaccagatgtcatccgatccgtgtcgacatccaaaatcttgaagggaatcaccttatcgttcaacaaggccaccagccatttgattgggcggacatattcaaacgaatacgtcccccatttcatcatggttgggaaagtcatggcggtaatgacatccttcatccccggcaaaatttctttaagtgatttaccggcaatgtgtttttcaacgaagacgtactcaacgcccttaacatccttaaaggtgatgtcatcaggagttgcaccctgcccgcgtgagaagccaatcgccgctttggtccaattaccgtcactatcctgggcaatttttttggccgggcccttaacagatttgtcaatatcgggctgtttgtcagctaaatcagtaatgtaaagtgccaaacgacggggagtactgaacgttttaatctcagcaaatgaaatccgttgatccttcaagaaatcaccggcacgcttctttagttgctggatgcttggggtgaccacgtgcgccggaatttcttccaatccgatttctaataagaaattattagccattatttctcctccttgtcgtcttttaatagtgcttggcgtttcttttcgtctttaatgagtgggaagccgagtcgtttgcgtgcttccacaaactctttggcaaccgaacgggctaagttgcgaattctggacagatagccggctcgttcggtaactgaaacagcccctctggcgtccagtagattaaaggtatggctgcacttgaggatgtaatcataggccgggtgaaccaaatcttggtccaacaggcgtttggcctcgcgttcataatcattaaacagggtcaacaacatctcttggtcggaaacttcaaaactgtatttggaatgctcatattcaggctctttgaaaatatcaccgtatttaacatcgtcagaccagttcagatcaaagaccgaattaacgtcttgaacgtatgaagaaaggcgttccaatccgtaagtaatttctgaagcgaccggatccatttccagaccaccaacgatttggaaataggtgaactgagtgatttccattccgtccagccaaacttcccaaccaacaccggcacaacccatggatgggttttcccagttgtcttcaacaaatcgaatatcatgctctaagggattgattcccaattcttttaaactgttcagatataactcttggatgttttccggagacggcttcatgatcacctggaattgatgatgttgatacaaacggttggggttttcaccataacgaccgtcagccggccgacgagaaggttccacataagcggcattccacggttccggaccgattgcccgtaagaacgtataggggctcatggttccggcacccttttcggtatcgtaagcttgcattaacatacatccctgggctgaccagtattgctgcagccgcaggataatttcttgaactgataatttttcagtcataaattttcctcctaattattcaaacgcataaaaaaagtccctatgttcaacgacttatagactaagccactcaacatagggacgatgaaatcgcggttccaccctacttctggtattactaccagcacttaattgttcaactcgaaaagcgccattgacagtaccgacgataatcagctcccactatcctgatttcgctaccagggtccatcctgtcatttcttttgtcatcattgaattatttatttcaaaaataatcatagttgacaatcaaaatattgtcaacgccgttatcagttataacttgaattttcccaactgatcaataaaatgtttactttttggaacgacaccgacacttcttgaataaatctggtcgagaacttcccgcaaagcttttttggtccgatcgttaaccttgatatgggttagtttggataagtcaactaccgaaaacagtcgaagatagtaaattgtgcgggcatccaaatgcatccggtatggatctttgttccaatgattctgacacaacagcccaccgtaggcctcagagtaatcaaaaggcagatccgtccggtgacagatcgtgcaatccacccaatttggtgcgacgccgtaagcattcagcagttggacctcaaaaatatttgtgatgatttgctcatcaaagccctggtcaatcagttgcaggccggtcaacagcttgtcgtaccaagtggcaatcggctcaccgtcgggataggccaaatcaatcagtgacatgatataagtggcataagcattcttagtaatgtcttcactgatgttttgaaagtggacgagatgcttatcattgaggatatatgacaatcctgattccttaatgtcaccgccatatagcccgtaggtaaacggcaggattgctgaacgcatcttgaaccgtgggcgtttggcgcctctaaccaggaacatttttttgccgaattctctggtgagaaattttatcagcaggtcgtgttcccgataggcttttgtataaagcaaaatgccattaaaatccgttcgctgaccttttgacaaactgattcacctctaataattatctttgcggtaaccgtaagaattgagcaggttggccttatcgcgccagtgaggttcaactttgacccacagttcgagaaagactttgttgcccatcatattttcgatgtcttttctggcaagcgtcccaattttctttaacatcgagccgcctttaccaatgacaattcccttttggccatcacgttcgacgataattgtggcccgaattctcaaaaggctgtcctctgtcttgatactttcaatcactaccgcagttgaatgaggaatttcctgacgggttagttccagcactttttctcggatcaactctgaaatcacaaatcgttccggatgatcggttacctcatcagctggataatattgaggtccgttgggcaattctttgattaaggtgtcgatcaattcgggcacattattgccctggagcgccgaaattggataaacatccttgaattccaaagcgttcttgtattgctcaatgatcggcataatgtcatcgggagaaatctcatcaatcttgttgatcagtagataaattggcttatcaacatttttcagctggtcgataatgaaattatccccggcaccgcgatgttcagtggcgttgaccataaacagcacagcgtcaacctcttttaaagcagacaaagctgattccatcatgaaatcaccgagtttgttctgtggcttatgaataccgggggtgtcaataaagacaatttgagcttctttcgtcgtgtaaaccccttgaatcttatttctggtcgtttgcggcttgtcgctcataatcgcaatcttttgaccaatgacccggtttaaaaaggttgatttaccaacgtttggtcgaccaacaatggcaataaagcctgaatgaaaatctggattatccatttcttactcctcttaatttaataatgcaatgaatctcggaacaaagatcagcatcccgatgatcacagcaaacagtgctgatagtaacacaccaccagctgctacatccttggctcttttggccaaagcgtcaaagtggtgaccaacaatgaggtcaacaacgttttcaacaacggtgtttaaaacttccgacccaatcactgagaaaaaagccgcgaacagccagagccattcgttgatgctaatcttcatgacaatggcgaaagttaacacaatgattgccacaaccaagtcaatccgaaaatttcgctcttccaacagcagtcgtttaatgccttcaagagcgtggccgactgattgaagaaacgacttattcttatccaattgtggcttgcggttatcttttgagtccataagcatttaaaatctctttttgaagcggaaacatgacatccgcatcagctttcttcatatgatcgtaaccattcaggtgtaagaacccgtgaacacacaggaaccccaattcccgttcaaacgagtggccaagataatcggcctgttcggcaactttatcaacggaaacgaagatgtcaccaatattttcaggaattgactctttcaattcttcatccatcacaatggggaaatcatcgtcatcatcgtcatcttcaatggcgaaactaatgacgtcggttgcccgatcaaccccccgatacttcttgttgatttggtgaatctcatcgttattgaccagggtcacggacatttcggtattgtcggccaaatgaatgtaagatccggcaaattccaaaacatcccgaatcaatttttgatccttttccgaaacccctttttcagttttatcgtaaatttctaaatccattaatttagttcctcaagtctattcgagattaattgccacttttttcgtaagcggtaatgattttagcaacaactgggtgacggacgacatccttagccgtgaaggtcacaaattcaatttgatcaatatccttcaagatcttttgagcggtaatcaatccgctggtcgaatgctttggcaaatcaatttgtgaaatatcaccgttaacgatcatcttcgagccaaatcccaatcgggttaagaacatcttcatctgcatgttggtggtgttttgcgcctcatccaagatcacaaaggcattgtccaaagtccgaccacgcatgtaagccagcggcgcgatttcaatcgtcccccggtccatcaatcgttcagtgtgctcggcacccaaaatggcgtgcagggcatcgtaaattggacgcagataaggatcaaccttttctttcaggtcaccaggcaaaaagcccaaactttcaccagcttcaaccgctggtcgggtaaggacaattttgtcaacagtgcccttcttcaaagccgcgattgccatgacgacagccaagtaagttttcccggtaccggctgggccaatgccaaaagcgacatcatgatgcttgattgcttgaatatactgccgctgtccaaaggtcttaacgcggaccgccttgccctttgcgtctttgatgagcacttcattgtataaatctttaaagtactccagcgtgccgttttgagccatattcatcgcactgatgaagtcgctgctgttaatattaattcccttttgaattaaagagagaatattctccaaaatgtgtaaggtaatgctaacgggttcatcctgaccagtcactcgaagtgaattaccaaagacattgatggagacatccattccctcttcgataattgtaatgaactcgtcttgagtcccgacaatttgtaataattcgttggggtcggatacaataaactctcttgtaacttgttgagtatcagccaagtaagtgagctccttttttattagtcatattggttcagatattaccacaaagttgtggttatctaaagtatactagctttgcagctgctgcttaaccaatttgttgataacactgccgtcagcttgacctttaacctttggcatgatggcacccatcactttaccaaagtcggccattgattcagcaccaacctgtgaaatagtttcttgaacgattttttcaacttcagcttcggaaagctgttttggtgcatactcctcggcaatctttaatttggcttcctgttcttctgccaaatcttttcggtcagctttttggaattcttccaaggattccttttgctgcttaatttctttcataatgatatcgttaatttgatcttcagttaaatcatgattgccatcggcaactttggcattcatcacctgagccttaatgccccgaatgacacccaagcggaccttatcacgagccttcatggcgtccttcatgtcagaaagcaatttatcatatacactcatcaaagtaacctcttttcgcttaatacttaaattttaacattaaaaaagatcagagactaataaacattagctccgacctttagtcatcatttattaaaaacgacgtttcttcttgttgttacgcttacgtgctgcttcagactttaatttacgcttaacacttggtttttcataaaactctcgtttacgatattcctgtaatgtaccgcttttagaaactgtacgtttgaagcgtcgaagagcatcatcaagagactcgtttttacgaacgactgtctttgccatatgaaattccctccctccgagcttaaatgtaactgtttaatcaacactttaagtgccttctaaaacggttcgaagtaaattatacatattaatcaatacatcgtcaatgatttaagataaaattgatgtgtcatgttaatatttacttaacaaatataattttaggagttatttatcatgaaaactcaaaacatttttattatatcggattcaagcggcgccaccgcccagacaattgcccagacggctttgtcacaatttccagatgtgaaagccgaaattcgccggttcccatttattcaaaccgactcaattctcaaaggtatcttaaaaattgccctcaacaaacaggcgatgatttttcacacgctggtaagtacggagctcagccagatggttcaagatttctgccgccaaaatggcatttatgactttgactgcgtccaaacgccaatggcaatgctcagtcaggttactggccaacaaccggctcacgtgcctgggttgattcatgatttaaatcaaaattactttgaacggatctctgcgattgaatttgctgtagaaaatgacgacggcaaaaatcccaagggattgctggaagctgacattgtgttgcttggggtttccaggacgtcaaagacgccgctgtcgctttatttggccaaccaaaatcaacgggttgccaatctgccaatcgggccggacctgcaactccctgaagaagtcaacgacatcgataaggataaaatgtttggcctgctgaacacccctgagaaactgagcaaaatccgtaaacaacggatgatttcttacggcctggacgctgatacaccctactcggatccggcccatatcaaaactgaattggcgtacgcgaaaaaattatatcgtcaaattggctgtttaacaatcaacgtggccaacaagtccattgaggaaacggccaccattatcttggaaagcctcaatttaaataccaccgaattcgaagattgatttggcctgcctagtaaggttttctggctttcatatcttcaataatgttgggattaaactgctgttttttcagcattgcaacttcataaccatgaggattccacttaacgtttttattgtcaggatccttcaaaattggcgtttccataattttgggaacgctttttaattgtgcgtgatgggcaatatagttcagggtatcaaagccaattgtccccaacccaagaatttgatggcggtctttatggctgccctgtggatttttggaatcgttcaggtgaataactttgagccggtcaaggccgatgatgtggtcaaattgattcaagactccatcaaagtcatttttaatatcataaccggcatcgctggtatgacaggtgtcgaaggtcacggagagtttgtcattatcgctgaccttatcgataatttcagccaactgctcaaatgacgtcccaacttcggtacctttgccagccatggtttccaaagcaatttggacgtgttgattctcctcaatcacttcatttaagcccttggcaatttgatcgatcgctttttgcggaccggcaccaacgtgagcgccgggatgcagcacaatttctttagccccaatggcttgtgcacgttgaatttcctgccgcaaaaaatcaacaccaaaactgaagttttccggtttgaaagtgttccccaggttgatgatataaggcgcatggaccacaaccgctttgaggccatgatcggacatatactgcttgccggcatcggcattcaacttctcaatgggtttacgaaccgtattttgcggcgctccagtataaaccataaagacggtttcaccgtaggaagccgcctctttggcagacccgaggaacatgtccttgccgttcatactgacatgagaaccgattaaaaatggtgtttcactcatttgtatatcccccttgtaaaattaattgactgacttttttggaagcctgaccatcttcccaggcacagaatttttggttaaaacgggtcaaattgtcactgaaatcagtaaaagcgccagtttgacggtattcacttaacttttgataaaagtcagtttgattttcaaccattggtcccggcagattagcttgatcgtactgaaagtaaaagccccgcagctgatcacgataatgagccagatcataaggataaaacagcattggccgcttgaggttggcaaaatcaaacatcactgatgaataatcagtaatgagtagatctgttattaagtatagttggttaatgtcgacatcagcgagaattttgacccggtcttcaaacccgctaatatcaatattgtctttaaccaagtaatgtggccgaatgaccagtagcgtttgaggatcgacattttcaaaaaattgtgccagatcaaacggcagcgtgaattggtatttccctttctcggaaaaatcgtcatcccgccaggtgggtgcgtacatcatcacctgtttaggctgatagccaactagggtttgcttgatttttcgaatgtcatcagcgttattttcagtatataaaatatcgtttctgggatagccaatatctaagaatttacctgaatagccaaaagcggatttaaaaatatcgtgtgaatattgatttggcgcaattaaataatcccaccgggcagcctcatcaataaattcctgatggtattcagctgtctgactgccgggaatctcaacgttttcaatatcgattccgagcttctttaacggtgttccatgccaggtttgaatgaaagtggttcgcttatttttgcgccaccactttggcatccgtgaattcatcacccaataatcagccctggcaatgtatttcacccatcccggcgtgaaccgtttgacaaattgaatatttggatactgtttaaccagcctgccgtactcactgggtttgacactgaaatagcaccgctttcgggcagtcgggtcatcttgggttaattgattgtagatagcaaatggattgtcactgacatctttgccgttaaaactttcaaataacaccgtcccctttttgacgggcatacaaataaacccatcgttcatcacgatgagtacaatgcgggctatgagtttaataagattgatcattgaacgtttcaaaagctcaccctcaaaactagattaaatcaacaaatcgagaacggaatttgtaatgcagatgagaaccaaccaataagaagaagagaatcatgccccaaaagacaatcgtcaaagttggtttctgccagaaccaggcactgcccagcatcccgtcacggaaaccggaaacgacgtagaagaatggattcaactgcagaatatgaacaaacggtgctggaaaggcatccgtctggaaattgaagagaacgcccgacatataaaacagcatccgcatgagtgactgcaacaagatccgataatcgcgaaccaggacggaaattgttgaattaaaaataccaaaagcaatcagccaggcaatcatacaaatgaagtaataaatccactgaatccagtaaattgacggcgtcaccccatataagaagccaatcacaattgaaaagaccagcatggtccaaaaggcacttaagttgctgacaatcttaatggttggcaaaatactgacgggaaatttcattttagaaaccatcccaacccgttggtagatgctcttggaagcatccaggctggcccggttcataaagaaccaaggtgtaattccgataaccatccaaaccagataatcgacaccatgagtggaattaccgtgtttcaggccgataccgaaaaccagccaataaataccaatttgaatcaatggatataagtattcccaaatgaggcccagataatggctttgatactcggctttatcttcatactttgagattcggaagataatgccgatattttgaaattgttctttaattaaagtactgacttctttcaatttgaggcactccttaattagaccctaagaatttgacataacgcgcaatgactctgtcagtcgcctgaccgtcgttataggtgttccaatgggcgttaaatttgtcgaagttaacgcttgtccctgccaggatttcgtttctgagctgctcgaccttataaaccggctctaccggtagccagtcgagaaaatcatcctgaattcctggatcgcttcggtatcgatcaagatcaaacatgaagaagatgatcgatttggcatttggcaataagctaaaatcaaatgccaccgacgaataatcggtgaccagtgtgtcagccacagctaataaatcactggtctccaattcgtgataaaacttaatcttgggattaccaatgcggcgcatcggcacttctttatcccgcaaaaccgggtgtagtttgacaaccaccaaggcagttggatctgctgctaaagcactgccaaggcccttgggcagcttaaagtcctgatgctcccgataagttggggcatacaaaatgacccgatgatttttcagttcaggaactgatcgataaattcgctcacgggccttgtgctgccaatcttgactgagatactggtcggatctggggtatcccagcagctgcatcttgtcaaaattttcatgataactgtgcacaaacacctgtcccattgcttttgatgcgacaatgtattcatcaaagtgatcataaactttctgaaaacggcgcttatcagaacgactgcgtttgtcggtggtcggatcttcccagccaaacttcttaatcgccccgtcagcatgccatatctggacaattttgacgaacggcagcttaaccaggccacccaaaaaagcgtagtagttatcgcaaataatcagctttgctgacatcaaaagcgaaacatcgtccatcacgaatttaatgccatcgcgaaactgccgcgttttgataccaaaggctgctaaatccgtcgcagccgcttcggtattggctcgataaagaacatataaaacgtacttctgaggcagtcgttgtgccaattgcttaatgaagtcaacattatcatcaaagctcatcacataaacaactttgttctttggccgccaaatattcaggactgagaataatttgattaaccataagtaaacaactttcaaaattttcaccgtatttcaatattttgtgatcacacacaaaaaatattataacataatccacttggagaacttgtttcttaggaaatctttaaaaatgccctcagggtttcggctcgtaaaacctccccaaaatcttgaccgaatctgaaatgctggcaaacgcgttgggatcggactccaataaggcttcctccaactcccccatttcatatcgtgaaatgaccgtgaacaagattgttttggcatcgtgttgataagccccttcggcattatgaacgatcgtgattccccgacgaagatggttttgaacactatcgatcacggtgttggggcgggtggtaataatcatcacctgcattcgctgctgcctggtataggtcatgtccatgatgcgcgcattaacgattagactgaggacagagtaaaaggcgtatggccagccatacatgacggcagctgaaacgatgattaacgagttaaaggcaatgttaatcgtcccaatcgagttaccggttcggtgacgaataacaatgcccagaatgtccagcccaccagtggaaatcccgtttcgaagcgccaacccggtcccaaatccattgaccgccccaccaaagattgcacagataatcggatcatgggtgagcggaattggtttgagtaattgaatcataaaactggataaaaagacggtaataattgtgaaaatggtaaattcgtggccaattgcccgccacgacaagacaaataatggcaagttcagcaggaataaagccagcccagttgaaatttcaaacggaaacgcccgcgtactgatggtgttcaacagctgagcgaacccggtaatccccgatgaataaatatgtccaggtgtccagaaaaaattaaccgcaatcgacactaaaattgcgtaaataaatgaagttgaaattttggtgacgtaggtgtgcctacgcattaattttgaaacgtcatccataaaataaatccccttcgaaaactttttgaacgtcttgcctaatgataaacgtaaatgacaaaaattacattaaaaatcctgtaatcagtgactagattacaggattttattgaaatcagttaatttgaaactcgaaactacttttcaccatcaggtttggcaacaaacaagccaagatcttcaagctgtttggtagcaacaggttgtggtgcactggtcagtggctcaactgctttggagttcttagggaaggcaatcacatcacggatgttatcgcgatcagcaagtaagcggacaaagcgatccaggccaatggcgagaccaccatgaggcgggaaaccgtaatccaaagcgttcaggaagtaaccaaattgggcttcggcgctctctttggtaaatccaagtgcttcaaacattttttcttgaagtgcccgggtatggatacggattgatccaccgcctaattcaaggccgttcaaaataatgtcataactttgagcgtaggctttgtgtgggtcttcgccttcattcattaagtaatgaacatcgtcttcattgggcatcgtaaatggatgatgggcagccacgtaacgtttcaagtcgacatcccagtcgaataatggccagttaacaatccacaagaaggcaaatttggattcgtcaatcatgttctgttctttggcaatctcaactcgaagataggccagcgtgttggcaacaacccggctgttatctgcagcaaacagcaatagatcgccaggctttgcttcagccttggccaaaatcttttcacgcagatcggcatccttgaagaatttggcgatcgggccgttaaagccatcatcggtcaccttcaaccaggccaagcccttggctccgaaacgttcaacgtaatcggcaaatttgtccaaatcttttcgggaatacttctcagctccgccgggaacggcaattgccttgacttggccgccatctttgacagcaccggagaagaccttgaaatcaacatccttcataatgtctgaaagatcttttaattccatgccaaagcgaacatcgggttggtcagttccataacgagccattgactcgtcccaatccattcgtttgaatggcagctgaacgtcgatgcccatggcgtctttcatgaccttggcaatgaatccttcagtgacatcttcgatttcttcttgatcggcaaatgacatttccatatcaatttgggtaaattctggctgacgatcaccacgcaaatcctcatcacgataacaacgcgcaatttgatagtatttatcaaaaccggcacccatcaataactgcttaaattgttgaggtgactgtggcaatgcgtagaaggacccaggataaacccgtgaaggaaccaaataatctcgagccccttcaggcgttgacttcgtcagtgttggggtttcgatatcaatgaaatcattttggtcaaagtaactgtgaatcgactgaataatccggtttcgcaacaaaatgtttttttgcatctcagggcggcgaagatccaagtaacggtacttgagcttcaggtcctcggaaacgttaatgccgtcttggatataaaatggcggtgtcttagcggtggctaaaatcttggcatcggtgatgtcaacttcaatcttaccggttttcatcttagggttgatttctttaggatcccgggcaacaactttacccttggcttccacaacgtactcactgcgcagtttatcggcaaccgctaaagcatcttggccaaattcctcactgaatactaactgaacaattccttcacgatcacgcagttcaataaaaatcaagccgccaaggtcacgacgtttttggacccagccttttaagacaacttcttggccgatgagctgttcatcaacaaggccagcataagtagttctcttcatgtctaatcaatctcctcatcatctgtaaaatatttggtaatgatctcatcaaaatctttgaaaatctcagccagcggtactgaaacctcggtcccggtccgcatctgtttgacgttggcagtctttttttccagttcactttcaccaatggtaattgtgtactgagcattcagcttattggcagttttaaactgcgcttttggtttgcggtcaaggtaatcacggtcagctgcgaaaccgtctgcccgcaatgcttggacgatttgtaacgtcaagacgctggtctgttcgccaatcccgactacgtaagcatccaattgatcaagaaccgggaatttaaccccttgggcttccatcaaaagcatcagccgttccatcccaaggccaaaaccgattccgggcatttcagggccgccaagctgctcaaccaagccattgtatcgaccgccggcacaaatggttgtgtagccttcgcccagggccttggaatcaaccatgatttcaaaaatcgtgtggttgtagtaatccaggccccgaaccatatctgggtcaacgacatacggaatgttgagtgattccaaaaggtgtttgaccttatcaaagtgtttttgggaatcttcatttaagtagtccaaaattgatggcgcacctttgacgatttcctggtcgcgtttgtctttgctgtccaatacccgcaacgggttcttgtgcagacgaaccttggaatcatcactcaactcatcaaagtgcgggtcaagatagtcaatcaacgcttgacgatatgcgtcacgggaggctttatcacccagactattaatttccaaccggaggccagacaagccaaagtgtttcagcaaatccatccccatggcaatcacttcgacgtccaattcgggctcattactaccaaaagcttctaccccaatttggtgaaattcacgctggcggccggactgtggccgttcatagcgaaacatcgaccccatataaaagactttgactgggcggggatgttcaggtccgtaaagcttgttttcgacaaaggcccggacaacaccagcagtcccttcagggcgtaaactcatgtgacggtcgcccttatcattgaaatcatacatttcttttgtgacaacgtcggaagtatcaccagacgttctggaaaagacatcaaaattttcaaacattggtgtccgaatctcctgataacgataatcgtcaaacagcatccgggccgtctcttcgacatagttccatttttgagcttcacctggcaaaatatcggccgttccttttggtcgttgatatcgcataattgtttcctcccacttaaattccgaaaaaaaagacccctgtccatagacaagggtgcattcgcacggtaccaccttaattaattctcaaggataacgctcgcacgaatagcatttcgctattaaccatcataagcaaaaagtgtcacttcaaaataatcgacgcatccttccaccaaatgaatgctctctgtatgccgcttatttcgatagttctttttatcggttggatatttaactgtctataagactagtgtaccagccagaaaatgtcaagggaacatcggcgttatttccattcagactggcctctcaggcttatttcaactataatatgattatttgagtgagggaacgattgaactgtgaaaaaaatttgggaaaacaaaagctggattgttgccaccctgacgatcatcatcacatttttggtgttgatcgtctcgctggaatccaattcagtgactgttaaggtcaatcaattaaatattcgaagcgggccagacgttacctactcggtaaaagccaaagttcagcatggacagcgattgcaggtgattagtcgaaaaagtaactggatcaaggtcatctataagcatcgcacgattggctgggtagcgtcctggctggttcaaaacagcaacgttcaaaatgtcagcagcttatcggaagcgacaattgttttggatccgggccacggcggatcggatacgggggcactgtcaatgaccgggcaacccgaaaaacggtacactttggaagttgccaaacgagtcgaacgactgctccaggcgagaggtgcccgggtcgtcatgacgcgcagttccgataaaaccgtcccattagccgccaggccggaaattgccaattcatcatcggccaacctcttcgtcagtttccactttgactcttcggatgagaacaacgttgcgtctggctacacctgttacttctaccatagcggcgactccaaacatttggcagaatcagtcaaccagcagatgaaaaatctgccgttaagttcgcggggggtggaattcggtaacttcctggtaatccgagacaattcggttcccgctattttgattgagggtggctacatcaataccaaaaaagattttaaccaaattcaaaagccggcctatcaaaaaaagcttgcgaaagacgttgtcgacggcatcgcaaactattttaaaaacaatcattaattatttgttggtcaaccatgggacgagttcattgatttcggtgacccgaatctcgggattgccggaatcaacgattgtgccatcgggatcaaacagacacgaagcgatatttgcattgtgacccgcagcaacatccaacttgcggtcaccaatcatgatcgctttttttctgtctacctggttggtctcaattaaccagttaattgaatcaggctgtggtttccgcggaaaattctgatcagatgtgacaaagccgctgaaatcgtccagcagatcaaactttctcagcatgcttttagcctggtcatccctgtgtgtcagcaaaaagttgcgtcccttcattgatttagccaattccaaaacctctttaacaccgggaaacggcagggcatcttcaaccaatttggtttggtgggtgcgattcaattttcgaagctgtttttcatcaatcccgtaaaaggctgagaactttcgaatggctgtcccaacgtcgtgttggcgcatggtaacataaatctggtcttgatcgatttcaacatcgtcaatccctaaatcacccaatgcttgaacaaacgcggaaaccattttcgggtaggtatcgaacaacgtgccgtcaaaatcccaaaataattgattaatcatttcgttactccttaaaaaagccgaaccacacgattcgactttatttttatctgatcattttttatttgttatccgtatcaaagataatcgtcactggaccatcattttgaatattcaccagcatatcggctccaaaaacgcccgtttgaacttccaaaccggtctgccgcagacgttcattgagttgctcatacacccgatcagcgtgttgcggttcgcctgccttggtaaagctggggcgatttccctttttggtatctgcatataaggtgaactgcgaaatcgacaaaattgcgccattcacggcattgatgtccaaattgagtttaccggcatcatcttcaaatacccgcagtttactaatcttatgggttaaatagtcaacttctgcctcaccgtcggcatcgctgacaccaaccagcagaacgaatcccctgccaattttgccgtgaatctgaccgtcaatactgaccgacgcttccttgactcgttgcaaaaccactttcatccagcaaaactcctatctgaattttcgttcaactaaataaacatcgtgaacgttcttaattgccccaatcaaccgctccagctgctccaaattgcggacgccaactgaaagggagatggtggccatcttattattatcgacctgaccattaactgacgaaacgttcttggtgacactattaacggcagtcaagacattcgtcagcaggccggcccgattatatccttggacggccaaactggcatcataaatcgtccgttcctcaggattgtcagcccaggcgacctcaatcagccgctcaccgttttcttccgcagttttaatgttcgggcagtcaacccggtggattgacacgccgcggcccttggtgatgtagccgacaatttcatcgccgggaaccggggtacagcagtgactcaatcgcactaggagattatcgacgccttcgatcacgataccatttgaggacttgcgttttttctgcttcttagcgctgtcagaatcttcagaaatggtctggtggccttccaaaacttctcgttcagcttgatcctgacgctcttttttgagttgggcccgggcatcctctgtcaatcggttaaccaccccagtcggctgcaaatccccaaagccgaccgcagccaacaaatcatcagcgtgttggtaatgcatgttaacggctgccttggtcaatttatccggtaccatgatccggttgggctcaaacccggcttcccgtagtcttctggaaatcaggttcttaccgtcctcaatgtttttctcacggtcttcttgtctgaagtactgtttaatcttatttcgtgcccgcctggtgtgaaccagcttcagccaatcacgactcgggccggctgaaccagtggcagtaataatatcgacaatgtcaccatttttaacttggtgatccagagggacaatcttgccgttgacccgggcaccagtggtgtgattaccaacctcggtatgaatcatgtaggccatatcaagtggaccggctccttttggcagctcataaacgtcgcccttaggggtaaagacatagacgtggtcgccaaacaattcacctttgacactatccatgaaatcggcggcatcgtcagtatcttcctggagctcgataatttgcttaaaccagttgagtttattgttatcctgcgaggttttgaccccgtttgtgattccctctttgtaggcccagtgagcagcaataccaaattcagccacgcggtgcatctcttcggttcgaatctggacttccaagggcttgccttccgggccaataacggtcgtatgcagcgattgatacatgttggctttgggcattgcaatatagtctttaaaccggccaggcatgggtttccactctgaatggatggcgcctaatacggcgtaacagtctttaattgaatcgacaattacccgaatggccaacaggtcataaatttgactaaactgtttgtgcttttcaaccattttccggtaaacggaatagatgtgcttgggtcggccataaatctccgccttgacgcccaatgcagaaatcgcctttttgacctctttgatggctttttcaatataatccacccgttgatcacgacgtgagttcatcaagtgcacaatgcggtagtattgctggggattgagataccgaagtgaaatgtcttccagttcccatttgatggttccaatacctaaacgatcggcaattggtgcgtaaatctccaaagtttcactggcaatccgccgctgcttgtcaggccgcagtgattttaatgtccgcatgttatgcaggcggtcagccagcttgacaatcatcactctgatgtctttacacattgccagcaaaagcttacggtggttctcagccaatcgttcttcgctggatttatatttaatcttggacagtttggtaaccccatcgacaatcaaggcgatatcgtggccaaacagctcttggatgtcgcctaaggtagccccggtatcttcgactacatcatgaagaaaaccggctgagacggtctcaggatccatatgcaggtcagctaaaataccagccacctgagtcggatgggtaatatagggctcaccagactgccgtttttggtactggtgagcaatttttgcaaattggtaagcttttcgaatctcatcaacatgttccttgttcatatactcagaaaccttattaatgacatcgtccggtgtccaaattttagttgccattgtatcaactcttctctcatttgcccaaaggcatcatcaaatcatctttatcataataatatcattgttgtcaaagttattcagcaaactaaatcagttcggtcagcgttgaaacggcactgagaaagtacagtggtgctgtttcagtccgcataatccgtggcccaagaccagctaacacaaagtcgtgatcgactaattgggtaacttcagccggactaacgccgccttccggaccgaagacagccgccatggtgccgcctgaaggagtctgcttgacggccttgaccaaattggtttcctcgccttgcttggcggactcctcataagcgaccaattgggtatcaaaatctaattggaataaagcatctaatccgcttaaataagccactgttggcacgacgtttcgatgagactgctcagcagcgctcaacgcaacttcattcagccgggtaatttttttagttgctttttgatcccatttaacaatcgaccagtccatcggcaggaaaatcacgtgagccacaccaagttcagtagccttttgaacaatccattcgggcttgttgcccttggacagaccactgacaatcgtgacagcgaccggcaattcaacgttgtgatcaagtggcttgataatattggcggcaacttggtttccctccagtcgactaatttcagcttcgaacacctggtggtcatcgccaaccagttcaaaccggtcaccaacttcggcacgcaaaacccggcccaaatgatgagaaatagttttgggaagttcaatcgactgtcccacagttaaatgttgacttacaaaatagtgttgcattatttgtcctcgtcctttggcttttgggcgatgaccccataccaatctttcattctcaaggtttcaatgatctgaaatccttgtgaggtcatcgcattttcaacggtttcaaatttgtccttgataatcccggatgtgaggaaaaagccaccaggaacgagattatcccatgcttggggaaccagcggcacgataatttcggccaaaatgttggcaaccacgatatcagcttgagtatggattccggccagcagatcgtttgccgcaacgcggattcctttagcacctggattgagttgaatgttcttttctgcagattcaacagcgatgtcgtcaacatcgtacgcgtggatttcccccgcgcccatcaacttggcggcgatgcttaaaacaccggaaccagtgccgacatccagaattgattcgccgccctgcatgaccatttccaaagcctgaagtgatagtcgggtagttggatgggttccggttccaaaggccattccaggatccaagcggacaattttttcctgagtggattttggctgatagtcttcccaactgggaacaatggtgatgaatcgcgaaattgatactggatggtaatacttctcccaggcagtttgccaatcttgattcacgactggcgtcaggtgaacctctgctggtccgggattcaaatcaaacttcgccaaacctcggaccctggtggcaatttggtctgcttggtcatcaatatgctgattgttgggataataagctgatacaatcgccccttgcctaatgtgggtgagatctttaggatcgacaatttcaccatgatctccgtagcggccgggttttaatttctcaaaatctttggcatcttcgattgaaaccccggtcgccccgtatgccatcaaaatgttggcaacggcctcaaccgcttcacttgtcgtcataattgataattctgtccagtccatggaattctcctttgtcggttgattctaaaatgaaagctggcttcaccccacaatgaggcaaaaaccagctttgatttcgaatccatatcacttagatgcaccatctgatatttcatgttgtttttctttctcacgcgcacggacctttgcctcgtgcttcaataggtgtccttccaagtagttcaatagttcggattcgttctcgaaaatccggggatgcttttgcttatgcagccgtaaatcaatttcgttgattcgctgtctgccagtccacttatgactgtagcgaataataagccggttatccaagcggtcgcggccaaatctgaaaatataaatattatccggtgtcagtaagggccgaatatattcttttttatagaagtaaccgttttttcttaaatattgttttgttcgacttagaatcattaacacctcccagcttattaaattttaatttttcgaatcgaataaaaaaacaattaatatatataataattgaatgtgagaagaaacgcaaacattttctcataatgaatcaaagttgcactccttaacaagtttagcatatgatgtaggaaaggagctgagaataatggaattattccgcattcgatttatcaataagattcgacccgacacgattgagattcgctaccgggcagtgttggaatcacattcaagtgatacggtttttgagggccatcagttattcctaagaagttatttggataccaccattttgaaatcaggtgaagtcgcccttaaagcaatttataatattttttctgccactccaaaagacttggtcttggatcaagtagcttttgaacagtcgcatgaccgaagcctcctgcaggttccaaccaagcagttctttgatcaatacatcatcgataacggcatgttggatcgcgtcgttcaccaccaaggagaggacggcaagccggttatcgataccaaattagtcaccgaattgcggattggttagcagacacaccgctagtgagatagcgaaaaatttgacaattatatgtcacttgtcatatggtaaatgtgacaagaaatacatatgccgaagcaacctttttatcatcaaattctaaatttccgggggaatgaatatggatgcaagacaaaaggttcaagctgtcctcgacagtgaagacagtgcctatcagatccagaagttgaccggggtgaactcatcaattatcatccgactcagaaatcacacgcgactggtggataacttatcactggggacggttgaaaaactggaacggtattttgattaccatgtcaaacatgaaaacgatgacctgcctcattcggtacagttatcccattttcgtcatcgactcattaatctcctgcaggagttataccaaatgcaacaggccaaggctgaggccacaaatgccctgccggacgaaaaagctatgacagtggccattgaacagttattcaacgatgttatcgccaacaaactggagctggaacacttagagactatttacagccgcgcgttttctgatagtgagcaattaacgagtccaacaaaatagtttgaagacatctgatcgcaacgagttatttcgctgcggtcttttttgacgtcataaaggccgtttcaatagaaaaggcgcctagtaagacgtcttttaaataccaaaattaccttaatttagcgtcgcaaccattaaccaacgctcccgtttactcaaccgaagtgtcgttgctaacaagcattgcctgcctgaaacgaatcagtgatttgatttcctcaatatcactggctgttgcttgcttttttatgaaatttctggctggactacggttcttcaggtagcgggcatgtgcaagaattattgatctgaataaattatttcgttaagcccaatggcccagtaaaagtacctatttgtcgcctttttcttcctcatcagtctgcaaaacagccataaaggcctcttgggggatatccacttttccaacagccttcatccgctttttaccaaccttttgcttctccaagagtttcatccgcctggttcgatcaccaccatataacttggcggtcacatccttgcgataggccttaatattggttctggcaataattttggcgccaatggctgcttggacgggaatttcaaagttctgtcggggaataatgttcttgagtttaccaacgatgtctcgagctcttggtgcggcaaattgacggtgagaaatgaagcttaaagcatccaccttttcaccattcagcaaaatatcaattttgaccaggtcgctgggtttgtagtcttccaactcgtagtcaagggatgcatagcctttagtgctggattttaatttgtcaaagaaatcaaagataatttcggataaaggcatgtgataaatcacgttgacccgatactcatcaaggtattccattgtgtcaaattcaccccgtcgtctttgacaaagttccatgactgggccgacataatcattgggtaccataattgtcgctttgacgtatggctcagaaatttgcttgatagcagaaacatccggcatttcagatggattttcaacttctttggactcgccatcggttagcttgacctcataggttactgatggtgccgtggtgatcagttccagattaaattcccgttccaaacgttcctgaaccacgtccatatgcagcaggcccaagaatccgcaacgaaaaccaaatcccagcgccttggaaatttccggttcaaactccagtgctgcatcattcaacttcaatttttccaatgcctctcgtaaatcgtcaaacttggcattgtcagttggataaagtccggcataaaccatcggatgcatttcccgataacccgggagcgcttcatctgcaggatcaagggcattggtgacggtatcaccaactcgggtttgggtaatatctttgatgctggcggtgatgtaaccaacgtctccagacatcagatagtcgcgtttaacaggtttaggcgagttaacccccacttcagtgacttcatattcactgccgctgttcatcattttaatcttgtcgccgggtttaacagttccttcaaataaacggacactcaaaacgaccccacggtaatcatcgtaaaccgagtcaaagaccagggcctttaggggtccttcaacgtctccgtccggcgcgggaattttgtggacaatttgttccaacaattctgggacaccaattcccttttttgcgctggccagaacggcatcagaggcatccaagccaatcacgttttcgatttcttttcggaccttttccggttcagccgagggcaaatcaatcttattaatgactggcacaatttccaaattgtcatcaattgccagataaacattcgccagtgtctgagcttcgactccctgtgctgcatcgacaaccaggacggcaccctcacaggcagccagacttcgagaaacttcataggagaagtcaacgtgtcctggggtatcaatcaaatggaactcatagtcgtggccgtctttggcatgatacgtcaattccacggcgttcaatttgatcgtaatgccccgctcacgttcgaggtccatgttatccagtaattgatctttcatatcccgcttggcaacggtatccgtcatttccagaattcgatcggctaaggtcgatttcccatggtcgatgtgagcaacgatggaaaagtttcgaatatatttttggtgattcttcattttatctaaatccatgttgtattctcactttcatttgtttactgataataattataccagccattccagtttatccaaagttaaaccgaaccagcagggttgccttgacataaaaagaggtcaagcaacggcaaaacagccggctgacccctccacatgatcatgttatttatcaaaagcatctttcatcttgtcaaaaaaattactaccgcccttgccagcaatgttgtcaccactggccttggcgaatgcttccaaggcaatcttttgattcttattaagtgacttcggtgtgaccacattaaccgtcacccgctcgtcaccattaccgttaccacgaaggcggggcgcacccttacctttgagacggaaagttgtcccggtctgggttccggctggtacctttaactcaacatcaccatgaaccgttttgactttgattttgccgccaagtgctgctctggcaaaagtgatgggctggtcaacgtagattgttgacccatcacgcgtaaagtctttgctgggtttgactcggaagacaatgtataagtcaccgtaaggaccaccattgtccccggcttcaccttggccttgaagacgcatttgctgcccgtcatcaattccggctggtacgttgacttcaagttcgtgacgctcgtcggttttaccactaccaccacaggttgggcacttttccttgatctctttaccagtcccatgacaaaccgggcaaacttgacgggattgcattctgccaagtggggtgttggtctcagtggtaacgtaaccacggccgccacagttcgaacaggtgactggtgaagtaccaggcttggcacccgttccgccacaagtcttacactgggcttcacggttgtacttgatcacagtcttcttaccgaaaatggcctcttcaaattccagggtcatctggtattgaagatcacggccctgttggggtgcggacggatctgcccgctgttggccgccaccaaagaactgactgaaaatgtcatcaaaaccaaatccaccagcgctgccgccaaagttaccaaagcccccgccttggccaccgccgccaaagccggcaccggcaccatcggccgaaccatattggtcatagttggcgcgcttttgtgggtcgcttaacgtctcatatgcttcattgatttccttaaattttgcttcagcatccggcgctttattgatatctggatgccactttttagaaagcttacgataggcgtgtttgatttcgtcatcgctggcgtccttggaaactccaagaatgtcataataatctttttctgccattagaaactcccatcctcattcaattcattaaccatgataatataccatattttaacaaaaagccaaagccagccggccttgacttctcattacaatatctgattataaattactttttatcatcatcgtgaacttcgtggaagtcgccgtcaacggtgccatcgtcacccttgccgtcggatttgtcatcagttgaaccacccttggcaccttcgccggcagcagcaccgccgtctttaggagcttgttgttgatacaacttgacagccaaatcttgaacaatcttgttcaaatcgtccttcttagacttcatttcgtcaacgttgttgtcttccttagctttcttgagggcatcacgtgcatcttcagccttcttgatttcgtcatcggaaaccttacccttgacgtctttgagagtcttgtcagtctggaagatcaactggtcgacttcgttgttcaaatcagctgattccttacgttgcttatcagcctcttcgttttctttagcttccttcatcatcttttgaatctcttcatcggaaaggcctgatgaatctttgatggtgatcttctgctctttaccggttcccttatccttggcagaaacgttcacaatgccgtttttgtcaatatcaaacttaacttcgatttgaggaaccccacgaggagcagccggaatgtcagtcaactggaattgacccaacgtcttgtcgtcagcagccattggacgttcaccttgaagaacgtgaatgtctacggcaggttggttatcagcagctgttgagaagacttgtgacttgctggtaggaatggtcgtgttgcgatcgatcagcttggtgaagacaccacccatggtttcaatacccaatgacaatggggtaacatcaagcaaaacaacgtctttaacatcaccggtgatcacaccaccttgaacagcggcacccaaagcaacggcttcatcagggttgattgagtggtttgaatctttgccagtccatgatttgacggcttcttggacggcaggaattcgagttgaaccaccatttaagatcacttgatcaatgtctgaagtacttaatttggcatctttcaaggcattatcaaatggcaccttggtcttggcaaccaagtcggcagtcaattcgttaaacttggcacgagtcaaggttgtttgcagatgcaatggaccgttgtcaccggcagaaataaatggcaaactgatttctgattcagtaacaccagagagatccttcttagccttttcagcggcatccttcaaacgttgcaaagccatcttatctttggataagtcaacgccattatccttcttgaaaccgtcaaccaaccagtcaataattcgttggtcaaagtcatcaccaccaagatgtgtatcaccattggttgagagaacttggaagacaccgtcacccaattcaaggatggaaacatcaaacgtcccaccacctaaatcgtaaaccagaatcttttcatctttctcctgtttgtccaaaccatatgccaacgcagcggcagttggttcgttgatgattcgcttaacgtttaaaccggcaattttaccagcatctttagtcgcttgacgctgtgcatcattgaagtaggcaggaacagtgataacggcattttcaaccttgtcacctaaataatcttcagcaaagtccttgatgtactgtaaaatcattgcagaaatttgttgaggggtgtatttcttgccttcaatgtcaacagtgtaaccttgttcacccatgtgactcttgattgaacgaaccgtgttagggttggtgatttcttgtcgcttggcaacttcaccaacttgtggctgaccatctttaaatgcaacaacagatggtgtcgtacgggcaccttccgggtttggaataattttaggcgcgctgccttcaagaacagcaacggcagagttagtagttcctaaatcaataccaataattttattacttgccataaataatcctctttttcttttaaagttttattttgctacaacaaccattgctggtcgaagcactcggtccttcaaacgatatccgtcttggaggacctgaacaaccgtgtcagctggatgatcatcatctgccggcgccgtttgaacagcctgatcgaacttgggatcaaatggtttgttcaacgcatcaatcacctcaacgccattatcagacaaagccttggtaaaatgctcgtaaaccattgaaaccccctgcttaagttgcttgccgctttcgtcggtgacatcaactttaagcgctcgctgcaggttatcaacaatgggcaggatatcatgggccagctgctggccgtcatacttgattaaatcagcctgttccttcttggcatgggtttcaatatttcgcatatcggcttccgcacgaaggaacttatcttccattgtatcaagtttcttttgtaaatcgactaccgtttgtttcaactttttaatatcatttgcgtctgggctttgggcctgatcagcctttttttccggcttagctgcctttttggctgccttggctggttgagttgattggtcctgtgttggcccacttggattcttcttaaccgaatcatctttgttttctgccaaacaatcgcctccttaaattattgattatcgtcatcgtagtagccaagtaacttcttggtcaattcttcccgcaaagcaccaacaattccgatgacctttgagtaaggcattctggttggtccaatgactgcaatcacgccatgaccatactctttcaaatcataagttcctgtgataatactataatcttttaacaggtcgttgcgcagctcgccgccaattctgacctgaacatctttagagttgggatcaataatctttgaaaccgaatcctcggtgcccagtaaattgtagagtggcttaagccgatcaacattttgccgttctgcaaacttcaatagattcagttcaccatcaacgtgaactttgtctcggcccgcttcgtccagcatgtccccgaagatcttcaagaagccttccggggtctgaatatatttggtcatcaacattggaatatcaaactttaacttgtccatgacatccttgagcggcttgccgaccagttcgctgttaatgatattcacaatggtttcaagttgctcggacgagacgttggccagcctgaaaatcttatcaatgacgtgaccagtattggtaacgatgatggccattacctgacgatcatccaacttgaccaaccggaaaccgccaagtttcaggttatcgccagactctggattaaaagtcagcgccatgtaatttgtcaaatctgacaatactttggctgactcctggacaatctcgtcaatccgattgaactcactgttaaaagaagttttgattaagtcttccgcaccttcgtccagcgggtccggctgaacaagattatcaacatagtaacgataaccttcgatcgatggaacccgtccggaagaaaagtgagtcttcgtaattaagccctttgattcaagtgcagccatatcatttctgaccgtcgcggaactaacgtgggtcggaaactcctcagccaatgccttggaaccaactggcattcccgttcttgtgtaatcacgaatgattatttgaagaatatctttttgcctatccgttagcacccaaatcacctctttttagcactcaatataaccgagtgctaaggcacatttataatttaacaaaccgtctattataagtcaagggaatatagccttattttagcattattttgtgtagagtgctaatagtgctaattcaagatctcaggatgctgctctaagtactcacgggtcgcaactttgtctttatccaactgatcaattaaatcttcgggagtctgaaatttgatctcagctcttaagtatgaaagccagttcacgttgacgacttcaccatagatgttgcggtcaaaatccatcaaattgatttccaccgtcatcggatgaacatccgagaaggtcacattcttgccgattgaagccattcccaagtactttttgccggcaatttcgacggtgaccacgtagattccaatcgttggcagccattgatattctgagtgttcaacgttggcagttggatagcccaacagtcgcccccgctcctcgccgtggacaatgacgccacgggtttgaaatgggcgccccaacaatttagtaacactatcaacgtcgcctgaatccaattcaatccggatccgagtcgaactgacctttttatcattaatgtcgacagacggcactgtgatgacgtcaaaagcccctttaacaaatttggggaaattggccatcgtggccacttttttatcaccataggtgtgatcaaaaccagccacgactgccactgcattgaaccgctttagaaagttgttgatgaattcttccggagtttgactttgaaaatcatacgaataattcaccagaaagacttggtcaacaccaaaatctcttagcagctgcattttataatcattcagcgtcaaatatcgctgttcatggggcgacatttttcggtaaacaattgccggatgatgatcgtatgtcaacaccgccaacttggcaccgcgcttttcagcctcggtttttgcccgttgtaaaactgcttggtgacctttatgaaagccatcaaaaaatcccattgcaacgactgtcggaccatcgaccttaaagtcatcagacaacggatagtgtaatcttgaaatttgcattgttaaaaaccaccttcattaagctaaaaacattctaaacggtctgtattgaccgatttgttcgtccaaccggtataatgccttcacctgttgttgataatctaatcgaactaccggcgcgtgggtaggactgattgattggtccaagaaaccgccatgagaaacgattgaccagcggctgtcatccaattgataaccgggatattccgccagtgcttcagataacggatgaaggacgatactcaggtcttccgcagcaacggcttctttgacttgagccaaagtggatgtctgtgaaatatcaaaaccaccgcttttaattctggtcagatcagacatgacagacggcaagccaacccgttttccaaaatctactgccagcgttctaacgtaagtcccctttgaacagccgacttcaaaatagattgtctgcgtgtgggcagcgtcatcatacgttgctggtttaatttgcttaaaataatcaatacgaatccggcgtggatcccggtcaatggtgatccccttgcgcgcatattcatagagcttgtggccattgactttgacggccgaatacatcggcggcgtctgcagaatgtcaccggtcaattgagccagagcggcgttaatctgttcatccgtcaacggcgttttaaccggcacctgttcaatcaagtgaccgtccagatcctcactatcataagcgactcccagggtaatcgcaccgcgatatacttttccggactgcattaacagttcactgatcttggtcgcctggccgatacaaattggcagcaccccatcgacatttggatccaaggtgccggtatggccaacttttttggtgtgcaaaatttttcttaacttgctgatgcagtcgtgacttgtcatgccacgttctttatatagtgcaattacgccatccattcgaattctcctaattttttcatgtaagaaaattatatcacaaaaaaactgcccagccattcaggcgtggacagttgagatgattattcaccatcttgatttaatttattaattaatcggtcaatcttgtcaccatactgaactgatgtgtccagctcgaacttgatttccggtgttttataaatacttaaccgatgaccaagttcgccgcggattagtccgctggctttttccaatccctttgcagttgtttcttcgtcctcttttttatcggacaaaatactgtaataaatggtcgcctgctggagatcacctgtgacttcgacaccagttaaagtgacgccctgaactcgaggatcgcggacccgctttaacagaatgtcgttaacttctttttgaatttcctgttctaatcggccaacccgataatgagccatcaaaacacctccaaattacttgacaggcacttgtttcatgacatatgcctcaatcacatcgccgactttgatatcgttataatctttgatagttaaacctaattcaaagccttgtttaacttcattgacgtcatctttgaagcgcttcaaactgtttaattcgccggtatagacaacgactccgtcacgaatcaaacgaactttactattcttctgaacgacaccgtcaaccaccataccaccggcaatcgttccgactttagaagccttgaagatgtcgcgcacttcaacctcaccagtaacttgttcagtgtaggtcggagcaagcatccccttcattgctgattcaacttcatcaatggcgttgtaaataacttggtgaagacgaatgtcaacgtggtcgctgtcagcctgtgacttggcttgtggtgttggtcgaacgttaaaaccaatgataatggcgttgctggcttcggccaaggcaacatcactttcattaatcgcaccaaccccggaatgaatgatgttgaccttgacgccttcaacttcaatcttttgcagactgttagccaaagcctcaactgagccttgcacgtcagctttgattacgatgtcaacttccttcatttcgccttctttaagcgaatcaaacaagctgtccaaggtaacccgggtggtctttcgtcgttcctcaacttgagcttccttggcacgttcttcaccaacggcacgagcggtcttttcatcatcaaagacaacgtaacgatcgccagcttctggtacttcattcaaaccagtgattgacactgggcttgatggcgttgctttcttaacatcgcggccacgttcattggtcatggtccgcactcggccgaatgtatgaccaacaacgattgggtcaccgacgtgtaaagtgccttgttgaaccagtaaagtggcaaccggccccttaccttgatccaaacgagcttcaattaccgatccggcagcgggttgatccggatcagccttcaattccatcacttctgcttccaagatgatcatatcaagcaattcgtcaatattcttaccaaatttggctgaaatatcaacgaagatggtatcaccaccaagtttttcaggaaccagaccatactgcatcaattgatcagtaacatgctgtggattggcatccggtttatcaatcttgttgatagccacaatgattggcgtcttggcagctttggcatggttgatagcctcaatagtttgaggcattacgccatcgtcggcagcaaccaccaaaatcgtgatatcggtaatattggcaccacgagcacgcatttcagtaaaagcggcatgtccaggagtatccaagaaagtgatcaggttgtcaccgtgacgaacttgataagcaccgattgcttgagtaattccccctgcttcaccagcagtaatgtgtgaatgccgcaagtgatccagcaaagtggttttaccatggtcaacgtgtcccatgatcgtcacaactggtggtcgggataccaagtgctcagtattctccatttctttttcaaagatcttatccaaatcggacaaatcttcgtggactttttcttttgcttcaataccatagtcggctgccaaaatctcaatcgtatccttatcaagtgattggttttggttcaccatgacgccgagcataaataacttcttaacaatttctgctggctcacgatgcagcaatttacccaattcctgggcgttcataccatcttgatattcaagcacctttggtaatggacgattctttcgttccggtgcaccatggtgttcaacttcacgcaatcgttgattcttttgcttacgttgtttcttgttgcgcttcttgttggctttacgggagccgccacgattattattccggttcaagctgccgccaaaacgaccactgccggtattgtgatttgagaaattgttggaactacggtttgtattactgttattattcgaactggtatgattgcttgcagttgtactgctgccagttgaatgactgtttgtattacgggtcgacgtattggatgaattgtttgaagcttgatgattgcgtcgatcattattctggttggtccggtgattattggactggttcgaattgttggaatgattttgattattcgaatggttattattgttggaatgatttctttgagcagtattatttgtgttgcgagcaacactcgagtggccgttgttattacggttgctctctgcatttcggttagcctgctgtgtgtttcggcttaccggatgggacccgttgctgtcatggtgagcagccggtcgactctgtgcatgagcattggcatgttcttttggctttgagtttgccgaatgaacattgttggtgctgctcttatggcttgattgactatttccagtcgattgtttgccgcctttactaaacatcgcccgaatttgacgctcttggttagcgtcaacggttgacatgtgatttttgatatcgaagccctgtttattaccacggtcaacgatttgcttactggagacattcagttctttagctaattcgtaaattcgctttttccccatataatcactctcctttattgttatcggttaattcaaccaatttttttgccataccccgatcggaaatgccaataatggttcgtttcattccaattgcttcactaagcactgctttagtgtaactgttattcacgggtatatgatagtaatttgacttatcattaaacttcttttgagttgccttgccggtgtcttctgcgataaacaagaaaaaaatcttgccgctgcggatttgagacaaaagcatatcttgaccggagacaattttgcttgcccgccgtgccagacctaaaaaattcaaaattgcctgatcattgtccatcttcaaacaactcttttcgggcttgcttatggtcaacataggcaattagatcgtcataaaagttgtcatccaaagttgttgaaaagactttttcaaaagtgtgttccgctttagctttgcgggcaatctcaacgttaattgagatataggcaccacggccggacttctttccagtctcatcgattgaaacgtggccgtctgagtcacggacaattctgactaattcctttttcggcgccatttcaccagtaacgatatctttacgcattggaatttttcgttttttcaaaaaatcgcctcctaaaaattagtcttgagtgtcctcattcgactcatcgggattggtattaacatccgcaccgtctgtcggggcatcctcagttgaatcctccgtttgatcgccttggtcggaagcctcatcagcttctgtatcatcgctagcggcagcggctttattggcaagaatttccttggcttcagtttctgatttgatgtcaatcttgaagcccgttagcttagctgccaaccgagcattttgccccttcttaccaattgctaatgacaactggtagtcaggcacaatgaccgtgcaggcccgctcgttgtcatcatcaaagataacatcaatgacctcagcgggattcaaggagttggcgatataagatgcatcgtcttcatcccactcaacgatatccatattttcgccgtggagttcgttaacaatggtttgaacccgctgacctcttgggccaacggcggttccaaccgggtcaatgtcggagttgtttgagcgaacggcaactttggcccggtcgccggcctctctggcaattgagacaatttccacagttccatcataaatctcgggaacttcttgttcaaataaacgtttgagcatccctgtagccgttcggctgacaaacacctgaggacccttggtcgcattctcaactttggtgacatagaccttgatacgatcctgtggacgatagacttcgttgggcatctggtcttttgaacccatcacggcttcaactttccccagattaacgtaaacaaatcgggtgtcttgacgctcgacagttccagtcaccaattcatcttcatacttggaatattcatcaaaaacgttttcccgttcagcttcccgaacccgctgcatgattacctgcttagcggtttgagcagcaattcggccaaagttcttgggggtcacttcgaatttgatttcgtctcccagttcataacctttgttaatttcaagggcctcatcaagagatacctgaagctggtcgtcaacaacatcgtcgaccaccgttttaacggcgtaaacgtgcatctcgccttttttgtcgtcgaatgacacttcaacgttttgggcctgaccgtagtttcgtttgtatgccgaaaccaacgcggcttccaaggcttcaatgacaacctcttttttgatgcccttttcttcttccagagcagacagcgctcctaaaagttctttactcattattgtgtctcctttaactaaaattgaattgcaagccgtgctttggcaattaagttccgcggtacttccaacgtatcctgcttaccccacttatcattttgaagcaccagtttgtcgtcatccaacgacttcagggtgccttcaaatgttttattgccgttaagattttgatagagggaaacgtgaatatactcgccaattgcctgtttgagttcggcgtcgtttctaagtggtcgttcagcacccggagacgaaacttccaggaaataggcctgggggatcgggtcgggatccattgcatccagcttttcgcttaattcatcgctgaccaagacgcagtcatcaatggtaatgccgccttttttatcaatataaacccgtaaataccagcttttgttctcttttacaaactcaacatcgaataagtaaaatgagtgtttttccagaattggttcaacaacttgtttgaccgtttcaacaacattgctcaaaaataggcctcctaaaaattatccattaaaaagagcgagcatctctgctcactcccttacaagttatttagtaaattaactataacatatccgatgattcattacaaggctggcgcgttttaacgccaatgtgcaaatcaattatgctcgccttacatcaaatcaaacaagttcaactgattttcatccggcaatcccgccagcacattgttctcagtcatgaagtcaatcaaagttttggaaactttgccgcgtttggctaagtcttctttggaaataaacggcttgtcctctctggcagcaacaatttgcttagccacgttcaaccccaatcctggaactgaattaaatggggcaattaacgtatcaccatcgatcagccattgactcgcatcagacttgtccaaatccaccatttgaaagtgatacccgcgttcgagcatctcattggccagttccaaaactgtcagcaggttcttctctttggtcgaagcttccattcccttatcattaatcatccgcatggcgtttttgaccgcttctttacctctgcacatcgagacaatatcaaaatcatcggcacgaacggagaagtatgaagcatagtaaaccattgggaagtagactttgaaataggcaatccgaagggccatcaaaatgtaagcagccgcatgggcgcgggggaacatatacttaatcttcagacacgattgaatataccaatcaggtatcttggctttcttcatttcggcttgccagtcgtcaggaattccacgaccatgacgaacactttccataatctggaaagacaattcagagtccagtccccaattgattaagtcggtcatgatgttatcccgacatccaatcacattggcaatggttgccgttccattcttaatcagctcatcggcgttacccatccaaacatcagtcccatgggacaaaccggaaatctgaagcaactcggaatagttacttggatgtgtctgttcgagcattccacggacaaatcgagttccaaattccggaactcccagtgttccagtctttgattgaatctgatcttccgtaactcccaagatttttgggctggagaagatcgacatcacgccgggatcatccattggaatcgtttttggatcgatgcctgacaaatcttggagcatccggatcatcgttggatcatcatgacccaagatatcaatttttaaaatattatcatgaatcgagtggaaatcgaagtgggttgtttgccaagcggcatcctgatcgtcggctggatactggatcggcgtgaaatcatagatgtccatgtaatccgggacaacgatgattccagccggatgttggccagtggtccgtttgacgccggttgcgccctttgccagtcgatcttcctcggcttgtcggtagacttcacccttatcgcgttcgtaagccttaacgtacccataggcggtcttatcggccacggtaccaatcgttccggcacgaaaaacattcttttcgccaaacaaaactttggtgtagttatgggcaattggctgataatcacccgaaaagttcaaatcaatatcaggaaccttatttccggtgaagcctaagaaggtttcgaacggaatgttgtgaccgtcgccaatcatcatggtgccacattcaggacactttttgtgtggcaaatcatacccggagctgtattcacccttggtaaagaattcagtgtgttgacagttcggacaacgataatgtggcggcagtggattgacctcagtaattccggtgagggtcgcaaccaaactggaaccaaccgacccacgggaacctaccaagtatccgtccttgttacttttggcaaccagtcgttgcgcaatcaagtaaatcaccgagaacccgtttccgatgatactctttaattctttatccaaacgatcagaaacaatcttaggcagtggatcaccataccaagcgtgggcggtgtccatcgtccgtgacttaatctcgtcttcggccccttccattcttggggtgtacaacttatccttcaatggatggacatcttcaatttcatcagcaatttgattggtgttgtccacaacaatttcttcggccttttctgggcccaggaagttgaagtcactcaacatttcatcagttgtgaggaaatgaaggtctggtaattcttgacggttcaggggattggcgccaccttgggaattaatcaagatttttcgataaatgtaatcttgcggattgagatagtgaacgtccccggttgccacgaccggcttattcagttcatcgccaagtttgaccatattggttaagatttgctcaagattttcatcatcggcaatcaaaccggattcaatcagtggtgcgtaagcacgtttgggctgaacttcaagataatcataaaagccagctttttggcgggcctcatccaatcccttttgcatcatggctgtaaagacctcacccgatgagcaggcagaaccgacaatcaggccatcgcggtacttctccagttgcgtccgggggacccgtggaacccggtagaagtacttgacgtttgacaaggaaacgattttaaacatgtttttgaggccggcctgggttttggccaataaaatggcgtgagacggccgagcatggcggtacgcatcgttatcagtcatgtgatcattaagctgatcgtgatagacaatgccgtatcgatcttcagcatcctttaaaaatagatagtttaagtggccagtggtttcagcatcataaattgctcgatgatggtgttccaaactgacatcaaatttcttagccaaggtattgagtcgataaccacgtaaattaggatacaaaaatctggccaaagtcaaagtatcgatgattggattttgcatctcatgcatgccatgacgaacgtagccggtgttcatgaaccccatatcaaacgtcacgttatggccgacgacaatcgcatcgccacaaaattcccggaaaagtttgaagacttcttcctcagacttggagccgtgaaccatctcatcggtaattgacgtcagattcgtcgttcgttccgacaaatgaaaacccgggtcaataaattcttcaaattgatcaatcacgttactgttctgcattttaacggctgaaagctcgataacacggtcataaatggctgataagccggttgtttcagtatcaaaaacaacgtaagtcgcatcctttaacggaacgtgcttatcattgtaagtaatcggaacgccgtcatccaccaggttaatttcaacaccatagagcatcttgatgtcatttttttggccggcatgaaaggcgtctggaaatccttggacacccgcatgatcggtgattgccagcgctttttggccaaagtgcttggcctgcttggcaaagtcggcaatgttattagtggcatccatttggctcattgtggtgtgcaggtgcagttcaacccgtttcttatcatcatctgcagtatcttgacggctaaccgtcttaatggggttaatatcataggcattcaaagttagttcatgagagtagttatcctcttggacactaccacgaaccttcacccaatcgccttcgttaacgccttcaaagagcgcttcttcacctttattggaaaatttctttacttgaatggatgatgtatagtcagtaatcttcagcatcaaaagctggcggccggaacgcaatgcccggatttctttatcgaaaatgtagccagagacaaccacagagcgttcctcttctacaatttcttccatcttcatgacgggtaaatcatctttgattcgccgaccaatggttgacttgcccccaccgttaccactcttgggatgagcttgagcattctccttgatcgcttggttagccttcttaactaattccgcattggcagcatcgtttttcttcttgagggcttgaatgttttgctgagaagaactttcatcgacgatcgtgtgaattgtaaagtcgggaaaacctgcccgttgaaaggcatcttcaattggccccaaggcagtgttggtcataaagtccttgacgatgtcattttcagcgacaaactccacccgcgaatcgacaatggagggaaacttgtctgcacataattccttcattaacggtgaggtaaccccactatgtggaacgacccattgccagtattgccgaagcagttgttcagtaaaggtatcattttttgcagaaatattcagtgaaacatcagcaatttctttaaacgcagactgtagtctggcattaaaatcgttaaaaacctcaaatggcaggattcgtggaagtgaaatgtcaaattgccaccgctggctttgtttatgaacttccaggcgatcaattttagcatcctcaaaataaggcaattcatttgcctgtgtccattgaagctgttcaagcaacttttcaaataattgatttcgatccaaactcatcacaatacctcttctaaaaataacggtttaacaacaactggctggacacaaaacccaagttttggtccaaccagtttagaagtgacgaaaacatacgtctatattaattagttacgacatcattagtcaagattcttcaacatttttttgattgtgtcactcaattcggtgacgttaacctcaacggtttcgccagtttttcggattttgatttcaacaatcccctcttcagccttttttccgattgttactctcagtggaattcccatcaagtcagaatcggcaaatttaaccccggcccgttctttgcggtcatcgaccagaacctgtaattgatcagctgttaattgggcttcaatttgatgagctaaatccatttgaacggcttttttggcattaatggggatgatgtgaacatcaaatggggcaaccgctttgggccataccaacccattttcatcggcattttgttcagaaattgctgaaagtaggcggctgacaccaattccatacgatcccatgatgaccggcacagcgcgcccattttcatccaagacgttggctttgagactcttcgaatagcgcgtacccagcttgaagatatggccaatttcaatgccacgggtaaatttcagtgttcccttaccatcaggtgttttctcgccttctttgacaaccacaaaatcgtccacgtcatcaattcggaaatcacgatcagaattggcattgacataatgataaccatcttcatcggcaccaacaacggcattcttcatgttggcaacccgttgatcagcgacgattcgaacatcctcaccaacgccaacgggccctaaagaaccaaagtctgcccccaaataggtcttggcttgttcgtcagtggccaaatccagaaagtcagcacccagatagttctttaatttaacgtcattgacatcgtagtcaccgcggacaaggaccatcaccggcttctcatcggcaatgtacagcatcgatttgatggtttgcttatctgagacttttaggaaagcagccacctcggcaatggttttcgcgttgggcgtttcaaccttcttaaggtcttcttcaggttcagttgaaggctggtcgtcgacttttgatttggccatttccaagttggcaaaatagtcactttcatcggaataaacaattgtatcttcgccgacagcagccatagcggagaattctttggaatcagatccccccattgcaccgccatcgccgatgatcactttgtacttcaaaccaattcgatcaaaaatattacgataagcctgctccattgcattgtacgttttatccagatcctcatcgttagtggcaaatgagtaggcatccttcataataaattcacggcttcgcagtaatccataccgcggacgattttcatcccgatacttgttttgaatttgataaagaaccagtggcagctgtttgtatgatttaatggaatcgcgaattaacgccgtaaacgtctcttcgtgagttggtcccaaaataaaatcggtttcatggcgatttttaaatttgaatagttctgggccatatgtatcatagcgccctgactctttccaaagatcagccggcaaaatgtcgggcatcagcatttcatgagctgatgttttttccatttcctggcgaatgatggtttcaattttgtttaaaacgcgataggccaatggcaaatatgcgtacatacctgcagaaatctggcggatatagccaccacgaactaacatttgatgacttaaagcttcggcgcctttgggggtttcttttaacgttgggatcagcatctgtgattgtttcatttataaggttctccttcaaaattaacttgtttaatgtaaaaagtatctctcaatatcattccaagtaaccagaatcatcaacagcatcaagaacgcgaagccgatcaatgtgataacagtttccgttgtttgagaaaccggctttcttctgatagcttccaaaatgtttaaaatcagtttaccaccgtccaaaccaggaattggaatgaggttgataattgccaggttgagtgagagaaatgcgaggaagttcaagactcctgaaagtcccatcttggctgcttgggaagttgtcgcaaaaattgccaccggcccacccaaatcgttgagactaaagtggccgctaaccatgctccacagggcgccaaacagctgcttggcaactgtccaagtggtggtgaaacctgaaagaattttggctttaaaactggtatccattgtttgagtaatgccaatgaaccctgtcttttgaccgccggaagtctgggctttgggtttcatggttaagactttatcctgaccatcccgctgaaccttcacagaaatttgcttatcagcttttgatcggatctgaacagtaagatcctgccaatcagtggtcttgtgtccatcgacctcaacgattcggtcaccggatttgacaccggcagtccgggcgacagaatcggtgggcatgacattgactttattggtattggatgcaacaccaccttgaacaaagcctaaaattgtatataccaagatggcaagtaataagttattaaacacaccagcaacgtttgtcagcattcgattaggcaacgatgccgattgaaattgaacatctcgaggagcaatttgtaattcggtcccgtctttttcgatgatagttgcgtcatgatccaccggatacgacttaacttgggactcatcaccattttcatatcccttgacatacaaattatcgtcaagattagtatctgtgatggttaagggaatgccctggaaaagtgaatgcttattgctggtgttaattgatgttaccacaccactgtcattcaattgaagagtcaccggcgtcccgggctttaattcgtcctcaccgtcatcggcctcaccggccatccgaacataaccacccagcggcaataatcttagggtaaaagttgtactatttttccgataataaaatacttttggccccatcccgacagaaaactcccggacaagaatgcccgagcgtttagcagtaatataatggccaaactcatgaaagatcacaagaataccaaagacgataatgaaaacaataattgtagttatcaagtgacactttcctcctaaaaactaaataacagctaacaaatgaagcattggtaaaacaaaaagtaagctatcaaagcggtccaagattccaccatgtcctggcagaatcttccccgagtctttgacgccataataacgcttcaatgcagattcaatgaggtcgccaaattgaccagctatagagagaataatcgtgaagatgaacatttgcaagagggagtgtccggcaattgggtaaaatgcgataaatgcggtacataaaatggtggctgcaagtgaaccgccgatcgaaccctcccaagttttattggggctaattcttggtgccaacttgtgtttgccaaacattctaccaaaaatgtacgcgccgctgtcagttacccaaacgataaacaaagcatacagcaatactgtcagtccaactccccgggcggcaacgaagtagtgaaatcccataccgatatacagcatgcccaggacaattaccccggcatcgtcaaacgagaacaggtttcgactcagaaccgtttggagaagcagcatcaaaacaaacaaaaagaagacaaagttttgactgatgtgtccgggtaaaaagctcgtccatgcatctggcagaatgagtgaacagactcccaaataagcaataattgattcaggtgaaatcaataatttcttcttcatcactaatatttcagagatggctacaatcccaagtgccaaagcggcaatatccacccagattccacccattacgatgattggaataaagattaataaagctactacggctgttatcacacgttgtctcaatttgtttctcctctatttactagttttaattccgccaaaccgacggtcacgctgctgatattccatgatcatttgttcaaaaaccgttcgatcaaaatcaggccacaaaacatcagtaaaaacaagttcactgtatgcaatctgccacagcaagaaattggatatgcgttcttctccgctggtgcggatcagcagatcgggatcggctaaattgccgagaaatccggtcattaaatttgcatcgatggtttgatccgtgatctgctctggatccagttgaccgctggcgacctgacggccgatttgctgaactgccattctgatatccagacggctgccataattcagggcaaagttcaggatcatccctgtgcagtcagcggtgtctttaatagcgtcattaactgccttttgtgtttgaacgggcaattgatccttgatacccatcacacgaacttgaacattatttttaaccaagtccggcacgaaatcgttgaagaacttaaccggcaagcccattaaataactgacctcgtcgtgtggccgtttccaattttcggtcgaaaacgcgtataacgtcagaaccttaacaccaagatcactagcgactttggtaatcgttttaacggtttccatcccgcgtttatgaccggcaattcttggcaaatggcgtttctgtgcccatcgaccgttaccgtccataataatggcaacgtgtgccggaatgttgtctgttttgagttgcggggttgcttgttgattgtcttgtgtgttgttaaacattttacgctccttaaaaactgaatgttggcttggctgtcagattcaaaaacagcatgggatcctcgcgacatatcgttaaacaccaaatggctggaacaaaaccaaagttttttcccagccataaaatgctattcgtattagtcggattcgccgtctggacgttcaaccattcgccattcaccgcggtttgcctcagccaatgtgttgaaatacttcaacagcttattggcatcttccggactcttttggcccagcaggtttaagcctttgccggttgtatagggttctgaaaggtccgtgatttcatggtcgttttcaatagttgctgtagaaaaggcaattacccagtcgttttcaaccagttgcgaaacgatgaagaataagttaaagccgtcgtttacatatgcaggcattgcatataagccatcttggaccggctgcaagtggccgccgttataatccaagacgcccaaattgtcctcagtaacaggcgtattcagtttaaaaagcatcttgccaaattcatcggttccaggtacaaccgcaatttcatcgttatctgaattattattgttattatgattatctgccatcgtattgacctctttctagccgttcatgacttcttgttctttgtcggcgacaattccgtcgacacctttaattgcatcatcagtcaatttctgaacttgatcttcatagcgatgcagttcgtcgtcagtgatatcttcactcttattgctacgcttgagtgtgtccatggcctctcgacggacatttctgatggcaaccttacttttttcaccggttgccttgacttgcttggcaatttccttgcgccggtcttcagttaatgcgggaaccgccaatcgaattgccgttccatcattagccggactgatgcccaagtctgcttcataaatgcctttttcgatgccttccaaggcacttttatcgtaaggggtaatcaaaatcacccgtgcttctggaatggtaatcgaagcgatttggtttaagggcgttggcgcaccatagtaatccaccatgacgccactcaacaagctggcgttggcatgaccggcacggatactgcccatatcatgttccaacacctcacgggtattcttcattttttctttcgcttcagttaatactgattgtgcatctgccataaattatttctccttcacagttgttccgatattatcaccagtcacgaccttacggatattgccgggcttgttcaaattgaagaccaccaatggaatgtgattatccatcgacagagaactagccgtagagtccatcactttaaggcctttttccaaaatatccatatatgaaagggtatcaaatttaactgcatctttgtgagttcggggatcggatgaataaatgccatccacaccgtttttagccatcaagatggcgtcagcaccaatttcggcagctcgcaacgctgcagtggtatccgttgaaaaatacggattaccggtgccggcagcaaaaatcacgacccggcccttttccagatggcgaacagccttccgacgaatataaggctcggcaatttgccgcatttcaattgaagtttgaaccctggtcggaactcccaaatgttcaaggttgtcttgaagggccagcccgttcatcgttgttccaagcatgccaatatagtctgcttgagcacgttccatgcccatctcggcaccggcttcaccacgccacatattgccgccgccaacaacgattccgatctggacacccaggttaaagatatctttgatttcttgggcgacgtttttgataacaggtggattaataccaaagccgcggtctccggccaatgcttctccacttaattttaaaataattcggttgtattttacttcagacatccaagtgcctcccatagttaatcgttactaccaattttagcatattaacgttgcaatcaacaagaaaacagggatattcaagaattcttatcaaatattctcagccagttcacagagatgtttcagaaaacagggttgagtcattcatgatggtaaataaaaagagttaggaaaagcggaatgctctgtcctaacccctattatttggttacgtcgttatctttggaaaaacgatttgtaaactaaattctgtcagcttacttcaattgatcgcgaacttcatcttcgaagctttgggtcttcttttcgatgccttcaccgacttcgtaacgaacgaatttaacaattgaaccgcccttggaagcaacgtatttggaaaccgtgacgtctgggtctttgacgaagtcttgatcttccaggcaaatttcggccaagaatttgtgtaaacggccttcaaccattttttcaacgatcttttcaggcttgccttcatttaaagcttcttgagtcaaaacttccttctcatgagctaaacggtcagcaggaacttctgcttgattcaaatattccggattagttgcagcaacgtgcatggcaacatccttggcagtttcttcatcagcgccttttaattgaaccaaagcaccaatgagtccaccattgtgcaggtatgaaccaaagacttcgtcatcatttttttcgacaacttcaaaacgacgtaaagtaaccttttcaccagtcacctgagtcgtttcaattaaatcgtctttaacagtccctttgtcggtctgcaatgccatcgctgcatcaacgtctgcaggcttattggtaacgattgcgtcactaacacgtttaactaattctttgaatggatcacttgacgcaacaaagtcggtttcggagttgatttcaacgattgcagcggtattacccttaactgcgatggttgccaaaccattggcggcaacgcgatcactcttcttctcagctttggcaactcctttttcgcgcaaaacttcaattgctttgtcgaaatcgccttcagttgcaaccaaggccttcttagcgtccatcataccgacaccggtcttcttacgtaaatccattacttgagatgctgaaatttttgccatcttagtggcctccctttaattgtgactaaaaactgactccacaccaaggccaaattggtccaaagcggtagagtcagcccgagtgctaatatttatttgttagaatcgttgctgccttctacggcgtctgcaatgtcttcaattgaatcttcttttttgtctgctttggcgccatctttaccttcaaaggtcttttcgttaacgtcatcttcgccttggcgaccttcaatgattgcgtcagccatctttgaagtgatcaaacgaacggcacgaatagcatcatcgtttgatgggataacaacgtcgatttgatctgggtcagtgttggtatcaaccattgcaacgatcggaatgttcaatttcattgcttcgtgaacagcaatttgctctttacgaggatcaacgataaacataacgtctgggatcttaggcatgtcttcaataccgcccaagaatcgttccaatttctgttcctgcttgattaaaagagaaacttccttcttaggaagaatgtcaaaagtaccgtcagttgacatcttcttcaagtccttcaaacgcttaacacgtgattgaatggtttcccaattggttaaagtaccaccaagccaacgattgttgacgtagtattgaccggcacgggttgcttcttcagcaattgaatcctgagcctgcttcttagtaccaacaaacaagacaacggcgcccttggcagcttcgtccttcatgaagttgtaagcaacatcgattaacttaacagtcttctgtaagtcaatgatgtaaataccattacgttcagtaaagatatagtccttcatctttggattccaacgacgagtttggtgaccgaaatgtactccggcttccagtaattgtttcatagaaataacagccatgatgtagcctccatattgtttttttcctccccaacgatcatttgaattaagaaccatccctggcaactctcaacccattacgtcaggtgtgtatttaaaacacctttaaaagtatataagaaaagccgcggaagcgcaagcacaaatacccggaacagattatttttttgtcaaaattgttaaatttcgatgaatcatgttagaatgatatttcgtggcgaggaggaatttatacatgattaaagccatcgttttcgatatcgacgatactttgtatgatacaaagcccgcatttgtacaggctttcgaagaaacattcaatctaaatttaccagaagaacagatgaatcagatctttgccaactataacgagcaagaacagttggcaattgcagaatccaactcagactccgatttgaaattatctgacgaagaaatcaactatcattcattacaccatacatttaaaaagtatgatctgcccggactgacacaagagtccgcaaaagccttttcggaggcctttgaaacggccagcagctccattcatctatttgatggattgaccactgtctttaataccctgactaccaaattcaagttaggcatcatcaccaacggaagcaacgatgttcaactcgccaaaatcatgaagctcaaacttcatcattggtttagccgcgaacaaatcattacctcagaagatgcgaaggctaaaaaaccggacccgcttatttttaccttgatgaaccgaaaattcaatttacggggcaatgagatgatgtacatcggcagctcctattttgaagacatcgtgcccgcaaaaaaggccggctgggaaaccgtgtggtataacagccatcaaagtccaatcgcagatcctcaaatcattcccgaccagacagtcaaaacaccggaagaattaaaagacttactcatggatttggctgctcaaatggactagcctatttaaaataaaaaggtttcaatcagagattgtctgactgaaaccttttttgtatatcaagccggtcaaattaaagttcaaccaacttgtctgatttaccagtattaattaatgatttgtttgcgtccatggcgaagtagaccatgttacgagcggcccgttttgtgtagaaggcaatatgtggacttaccaaaacattttcacgtttcatcaagttcttgagtcgttcgtcagggatcttgtcaaagctgccaaagtcagtattgaaaataccaacttcgttttcataagtatcaagggcagcaccgccaattttacctgaatcaaggccgcgaattaaagcatcagtgtcaacaagggcaccacgagctgggttaaggatgaagacaccgtctttcatttgagcgattgtcttatcgttaatcatatgttcgttttccttagttgcaggcgcatgcaatgaaaggacatctgattgagcataaagttcttcaggagtatcaacataaaccccttctttttcaagctctggattatgataaatatcataagcaattactttggcaccaaagcccttgtaaatgcgcattgcagctcggccaatccgaccagttgcaaagacaccaacagtcatttggttcaattcgtcagcaatatctggtgcccaacgaaggtcaccatttgcttgtttacggtcgaatgtgttggtccgacgaagtaatctcattaactgagttacagtaaattcggcaattgcttctggagaatatgcaggaacattggtaacttgaataccgttacgcttggcagcgtcggcatcaatattatcaacacctacgttacgaagtgaaaggtacttgataccaaagctgcccagcttatctaatacagatgcagtgtaaggcttttgttggtatgtaaccacaccatcagcaccttttgcttggtcaacagttgagtcgtcaagtaattcaccggttgaagcaacttcaacgtcgggattttcttcactccacttgtctaaataaggtttctcatcgtcacgaatgccatatgcaataattttcacgaatattacctcctaacagaatacttaaagtataacactttttgataataattttcactacttttcgtagtttgttcaataattcactctaattttatccccgcttgagctaaatgggcaattttttgagcccgactcaattgtttaaaggcgtattcagcgctcaaagcagcgtgtttgctgtcaaattgttgcttgaacaaaattttgattggtcggtgagagcgggtgtacttggcacccaagcctttcacatgctgttgaaatcttctttcaacattcgtggaaaaaccggtgtacaaagtatcatcggcacataaaagcacgtacatataatacttatctgtttgttccataaagcatcttctttacttcatcagtatagtcatcgccgtcataagtaataatatcgcggttgactttgagaccgtttgacttgccgtctttaatcgcctcaaccaagaccatgttggcgtcctctttgattcggggtctgacaaattgaagccgttttggctccagtcggtgacttcgtaacgccacgatcaaatccgtcagccgatcgggccggtacaccatgaaaagtttggcgttcattttcaacagtccggccgctgagctgacaatttcatttaaattagtggtgatttcatgccgcgcgatggccaagtatcgattcggattcttttcgctggtcttgtagttgacgaaatacggcggattgcaggcaacaacgtcaacagaatcttttggaatatattggtcggcatttttgaggtcgtcgttgaccactgatatctgctgagccaagtcattgagttcaacactccgctgtgccatatctgccagccttgtctgaatctcgatcatggtgatgtgagcagccgttttttcacttaaaaacagtccgactgccccattgccagcgcacatgtcgacaatttgtttggttctgtgttgcgtggtccgaacaaagtcggccagcaaaaccgcgtccaatgaaaacgaaaaaacgtctttgctttgaataatttggatgcctttgctgtataattggtcaattcgttcgtcttcatgtaagtttacttgcatatcgttatgttccttcacaaattagtttgccaaacgcttctattttaagttaatataattctatcagatatgaaagaaggaaatgaattgttttattcattcatgagagtccttgtccgaatcctggtgtttattatcaatggcaatgcccgttatgagcacaaggagcgactgccaaaaggcaactatattttggttggcccccatcgcacctggtttgatccaatttactttgcacttgccggcagtccgaaaaagtttagtttcatggcgaaaaaagaactattcaaaaatccaattttgcgttggattttggttcatgccaatgctttttcggttgaccgtgataaccccggtccttctgccatcaagaaaccagtccgaattctcagaaaatcagatttgtctttgatcttattcccatcaggcacccggcattccagccaattaaaaagcggtgctgcctttattgcccagctgtcaggtgttccgctggtcccggccgtttatcaaggaccactgacattcaaacagctttttactcgaaaacgggtcacgattgcctttggagaacccattacaattgaccgtaaacaaaaattgacggacgattttcaaaaacaaattgaaacggagatgcaaagcgcgttcgacgccttggattatgctgttaatccgaattttaaatacgttgatgtatcaaaaaaagaagagtaagtgaaatgacaaaaagccctcaccaagttggtggggactttttgtcattgaaacattctaatttttaccagtttggttttgcatcgaatgcatcatttgatttaatttcttttgggaaggtttttgacccatttgtatcatcagttggcgcaattgatcttcgctgaatggtgggttttctttgaggtacttttccatatacttccgtgcaccgtaaaagccaccaaccaagcccaagatcaaggctaacacaacgattaatatccaaatccaagttgccaagacaaggcctcctttatcatatcactaagtaattctacacaattatgccatagaattaaagggctaatcaacaaaatcccgattcttaggggaaaactgccccctaatcgtcccgaagacctttgtgacgttggacttccctgacttttccgggcgtcacttccttgccattcttatcataaactttcatcatttcaatctgttttttgaagttttcacggaagtgagcaacgtattttttacgcaaatcagcctgttccaacttttcaacttcagataagccctcattttttgctttgtgggccagttcattaattcttgggatgagttctttgaaaacatcgtcaccgatttttgattgcaattcttttttctcttgttcgttcattaaaattcctccatatcgactataataacacaattattgatagatacgcgaacgtgtgttttgaaatgtgaccgcggttatgatatgatttaggtattaaacaaagacttatgaggtgtctaaaatgtcaaaaacgaccaatgatccccaaagtaaacaataccagatccttcacttcatctgggaacgggttaatgagcagggctatccgccaacggtcagagaaattggtgaagccgttcatctatcatcaacctccacggtacatggccatattgctcgacttgagcggaaaggctatatcgttaaagacccggccaaaccccgcgcgctggaagtcaccagtagtggcttggatgtcctgggtatgcagccacaacaaaaacagattccggttttaggaactgtgactgccggtgaaccgatcttagctgttcaggaggccaccgactacttcccgctcccgcctgctctggcacacagtgatcaaccattatttatgctgcaaattcggggcgaaagtatgattaacgccggcattctcgatggggactatgtggttgtccgcaaacaggaaagcgccgataacggtgacattgtcattgcgatgaccgatgaaaatgaagcaacctgcaaacggttcttcaaagaaagcgatcactaccgactgcagccagaaaacgataccatggcgcccattattttgaccaaggtcagcattttgggaaaagtggtcagtttgtaccgcagcgatatttcataattatttctagctaaggactgttctgctaacagtccttttcttttaccctgagttctggtccaggacttttcggcaatgcccaacgagcccttctaccatcaatattatgcctgttgatctcgataaaccagctggtcggcctgtctgccaagcaacacgaatcgactgtcatcatcagcagcatcaaatgtaacatctccaccggcgtttgacaatccatttgcatacatcgcttcatactcaggaacagacagcctcgttcggttggcaatcacttgttcaacctggccggcaaggctctgcggttggatttcaggggcaattgtaccactgtaaaattccccttgagctcccgatccataactaaacaaaccaattcgatcacctggctgaagcgttttggagttggccagtagtgataacaagcttaggtagagtgacccggtatagagattaccgacgagggcattatactttttggaatgatcaaattctttgaggagtttttgtgagtgagcaccatcatcgataaccgtccgaagcgcctttaggcccatcttggtgaatggcagatgaaaagccaccgcggaaaaatcactcagcgtccgttgatatttcgcagagtaatctttaaatgtttggttgaagaaatcgatataaatatccgttgagtaatgcccgtcgacaattgcatcccgacggtaaaacggtcgccaaaaatccataatattttctgagtgaaatgcactttgattgtccaaagctaaaatttgtggatcctgactcatcagcatggcaactgccccgccgccttgggtgacctcaccagctgttccaatcccatatcgggcaatgtctgctgccaagaccaacactttactttcaggatgcattgcaatatgatcgaaagccatctgaacgccggccgtaccaccataacaggcttgcttaatttcaaacgatctggcggagttggatattccaagcaacgactgaacatagatggccgctgacttggagttgtcaacaccggtttcagttccaaagatcaccatatcaattgcttgtttatcgtcatcgcttaaaatcttggcggcagcattggcagccattgtgaccacgtcttgtgttggcgggattaccgcctggtccttctgtccaatcccaatcaaatatttattaggatcttcaccgcgggcatttgccaaatctgccatatccaaatagtaatcagaagtaaagaagcccattttgtcgattccaattgtcataataatctcctttaagaaagaatgagaccgaatattttaggtgcaatatccagtctcattatgtatgccgctgattgttaatgattatttattcgtaaaatgaatttggtaggtgtcattgccgttcatcgactgaatcactaagccttccagtaatggacccgcatagacgaagccttcatgctgatggccggttgagataaaggtccattgaacaacttgattaccactcaaggctgagccgaaaactctggcaccagtcaacgtcccaaccgaattatcagaaagaacaacttgttggtttcctagatttccattgacattaatagttaacattaaaattctcctagttatttcctttatacaacataataatatagcataattgcaatgcaaatgcgaattggttatagtaagcttatacttaaattaaaatatggagatgatgattatgaaaattaatatccatcgttccgcaacgaacaaggtgcttgccggcgtcattggtggcttggctgagcactttcaatggaatcccactttggcacgggtcgtatttgtcattctggcatttaccccattcttcccgggaatcatcgcatacctactgctttggattttgatgaaagcaccagaataattagtgctgcttcagtgatctgcggccaagccagtagatgactgccaacccaccaaaaaataggacaaagaacagtagaaagcattccaagaagaacgtatctggcagcatgttaatcaccggatcggtgttcgggtcaaaaatccagtcctggtttctgaataatacttcatgaaatgccacaaatacctggtcaaaattaacaaacatcaacgcgacaatcactaacgaaactgtggtgacgaccttaattggcgtcatcaacagccaagttagtgattttttgttgagccgatgcagtaggtaggcaccagtcggcactaaaatcagcccaacaaaattgttgaacaggatcaaacctttaacgtcccgaaagtgctgaagtccctttgcagaactgaagaagtaatccagctttaaagaaggaatccacggcacctgtaagtaggcaataatcctgacataatcatgatgcatctggctagcagtgcgaccagtggccgcagctaatttgagcggattaatattgaggtcaaacagccaaacactattgacagtcaaaaagatggcgagggcaaggcaccccaatatgattaaagtgccataaccaatttgttttccaagcattttcacatttataaccgccaatcatcaagtgagtcaatctggtgagtcggctgaaccgattctttggcaacctgttgctttgtcgaaagcccggtgtaaaccaggagcgtatcgactccggcattaatcccagccttaatatcagtgttgtaattatccccgaccatcacgacgtcagactgttcaaggccaatttttttaatggcactttcaataattctggctttgggcttgccaatcatgatcggttcgacttgggtggcatactcgacaaacttcacaacagaaccggctccaggcatcattccgcgctctttgggaatgtttgtatcggggttggtaccaatgaacgtcgaaccgcttcgaatagctaagacggcctctgaaagcttttcataggttaggtctgaatcaagccccacgaccacgtaatcaggatgatcggcttccaaacgataatcgttggctaagataacttgtttcaagcccatttcaccaacgatgtaaacggatgaagcatccccactacgatgctcattcatgtaatcaaccgtcgccatccctgatgtatagacattttccggtttgacgtgaatatcatggttatcagccaggttcttcaccacgtctctggggagctgagtggaattattcgtcacaaataaaaatggaatattggccttctgcaggcgctcaataaatcgtttggcagccggaatgcgttttttaccggcatacacagtcccatcaagatcaataaaatagcccttatagtttgtcatcaagtcaatccttctaattaatttttactctcacgaataataaagtggtgcttttttgatttttcttcagtcttcacgaccatattatggcgcttttcaattggcttatgggcggtaaccttcttttcttcaaaggcgtggttccgatgattgcgatgattactccggttgcgggaattatgagaccggtttgatcgatggttaccatgattattccgggattttctgatcaccggtcgggcctcaagattatgaacgacaaaataagcggcaccgaagttgacatcttccaaaatccagtcattgagtgcggaaataaacgggccggaagtttcagttcggtcatcattaaaaaatcctcgtaaacgtaatttgccgtatccccagtcgccaacaatgtaatcatactgactaaaagccggattgtaccgacgaacaaattcgttaaaatcaaagccatccgtgtgattggtatccaattcatacttatgatcattgattaagaattctgtttcactgactcggttgattcgtgccaatggctttcgattctcgtcttgttttgcaacgagttcatctaaggtttttctgtccaaagtaaccctcctttcactgattaagtggataatgtttggcgagataatccccaaacacatcccttaaattttcatcgtataaaatttcgttgtggccgataatctccaatgtcgggaagaacggaataaacaaatagtggtccggcatggcaatctggtatgttttcgccggtgaaaccaactcttcatggaaaaagagctggccggcatcttgatcataccgcaatccgccataatgtagctgaccaaaatacttgccacgaaaacccatccctttttgtgggaatttggtcaaaaagttcttgttcttttccatttctttgatgaggcgccagagattataaccgtccaaagtgacccgcatgacatgcatcgcgtggggcaacatctgatgcaattgatttcgatcaacaatcccttgaggcaggtcggttaaaaataggcccgaacttaaaatggcagcgcgagtatcggctttttccattatcgcatgcaaaccttcgtttaccaagcgcgaatggccaatgagattagttgtcattggggctttgattctggcaagtttgttgcgtgccagcagtttttcaccatgttgttgatattcctgaatttctgcatcatcttcaggcttgctgggcaaatcagcggttttaatcactttggcttgactggacacaatccgatgggaatcatcgatggtcagtgtaatctcaccaatataatgaccccatttttcggcagctgccagtagtgaatgattcactttttcaccgtgaacgagtaagtgatgcgtatgcgagccgatgatcacgtccaattgaggaaactgacgtgccaatagacggtcggttggcagccccaaatgtgatagtaacacacagatatcatatttgccggcgttatcggcgagaattttaggcagaaccgtttccggtttgagaggctcccaccccaagatcggatatgtcagtaaataaggcgctgtcagcccaatcagaagcacgcgtgtatgttgcggggtggtaataattttgctgggatgagcccattttggaattgatttggtctgctgatccaaaaggtttcccaaaatgacgtcgaaattggcatcattgtacaactcgtccaattgttcatgactattggtcaagccctcgttattgccaattgtgacggcatcataatgaatttggttgagcaactccacattggccttgccgttggttacttcagtgagtgggtggacgcgatcaaccgcatcccccaagtcgacagtgataacggaagaatcggctcgctgaagttctgctcggcgcgtggtgataaattgacgaatgcgtggccaattttcgaaatgggagtgcagatcgtttgtgtgtaaaattgttagcttctcagtcatcaaaccatccaatcttttctaaattagtgccgcttggcaaagtcttcagcttttccggcgaccatttcttcaatttcagcttgggaaaatggcgttccaaacggtggcttctttttcaaataatcagtctcgggcgtatccacaccgacattgatattttctttaatcggaactgcataatgatgaatgtgtccatgtaaattaataatttgtttaacgatgcccatcatcatcggatagtgagtcatataatactgacgatgattcatcttgatgagaacaccaacatcgtgaaattcaaacttttgatgattgcccacgggatgattatgctgctgcagatatttgaataaagcacgggaatcgtgatttcccttgatcaaaaccaagcggccattcaattgatccagcacttcaaaaattttttccagtgccactttctcaggtcgggtatgcaaaatcgcaatgtcaccaagatgataaaccacatcgtttttgcccacccgacgattccaattgttaatgatggtttcattcatatcctcgacagtcagaaatggtcgtggtgcgaactcgctaacgccaagtaaacgttcatgaaagaaatgcgtatcagcagtaaaaaattgcatgaacaggtcctctttcgtacataagttataccattaatgataccacccagcagccgtttagtaatgaaaaagtattcaaacaaagctgataacaccaatgaaaaaagccaaggcgccgatgccttggccaatcatcatttttcaacttctttaaccttatctgtcagacttttgaaaataaacagtccaattagccaaaccaccgagccgattaaagcaatcaacgtatccgtcttcatggtcaaaacaactgccacaaaagccatgaaaatcagtacgaagtaatcgctgattggaaaaagcggcatcttaaatttgagcgatttctgactgccggtttttttaacctgctttcgatacttgatatgagccaacacaatcattccccagacaaataggaaacaagttgtggcaacactggaaatgaaagagaacacatcaccgggcatcataatactcaagagcacgataaccgcgatcaccaaggtcgaaaaaagaattgcgttaaacggaatttgacgggcagaaagacgaccgacttttcgactgaattttgatttaccattataagtcaatgaaaacagcattcgaccagtggtaaataacgaactgttacaagccgaaattgccgcagttaagacgacaaagttaataatcaaagctgcggactggatgcctacaccggcaaaaacctggacaaaaggactggaagttggcgaaacgtgctgccatgggaaaatgctcatgagtgccaacagcgacccaatataaaacaagagaacccgggttggcacttcgttgatactctttggaattgtcaccaaaggatcctgagtttcagaagccgtcatcccaatcatttcgattccggcgaaactaaagagcaccatttgaaaggacaaaacaaatcctttcgcaccgttggcaaagaaaccgccatccaccacattcatcaatgatgcgtgtccgtatggtgttttaaaatggattgccaccaggacgattccaatgacaatcagtgcaacaattgcgacgatttttacaattgccagccaaaactcggtttcaccgaatgccgacacagcgacgatattgatgataaataggatcaataagaggaccagacctgtcaaccaaattggaatgtccggaaaccaaaactggacgtataatccagaggctgtcacttcggccatcgcaatggcgatccaacacatccaataggtccagccgatcacgaagcccattttttcgcctaaatattttttgatgaagaaaacaaacgaattgctttcaacatcagataccaacagttcccccagggcccgcattaataggaaacaagccaggccggcaatcccataggccaggatgattgatggtcctgctaaatggatggactgaccggcaccaagaaacagcccggttccaatcgttccaccaagggcaatcaattgaacatgtcgattcttgaggccccgggatagttggttgtcgtcttcttgattttccacaatgtgcctccgtttctaaaaaatgacaatttggtttattaaacaataaggctgggacaaaagtgcaaaacccttttgtctcagcctcgtttgtaacccgcgacgtccgaattcaaatggggctcaacggattctatgcttgaaaaagcaacgatcttcgcccgtaatgattgggtattaatgacgaccgtccaaaaattacttctgtgttttgcgtaatctttcgatatcgcgaacaatcattaactcttcatcggttgggatcaacaatgtcttaactgttgaaccagcggctgacaggtcacgttcttcgccacgaatgttatttttttcaggatcaactttgataccgaagtagcccaacttatcggtaacttcctggcgaatcataatgtcgttttcaccaattccggcagtgaagaccaaggcatcaatcccacccatttcagcaatgtaactgccaatgtagcggatgatacgattcttaaagatttcgcgagcgagcattgcccggtgattagtcttcataaccccttcaatttcacgcatatctgcggaaacacctgataaaccgacgaggcctgatttgtggttcaaaatatcaaccatatcatccatgtttttaataccggctttttgcatcacatattgtaatgcagaaggatcaacgtcccccgaacgagttgccatcgtaatgccggcaacaggtgagaagcccattgaggtatcaaatgacttgccgtctttgattgcgtcgattgaagctccggcacctaagtgaaggacgattaatttcaggtctttcagaggcttacctaaaagggcagctgctctggcagagacataacgatagctggttccgtgggcaccatacttacgaacttgatacttttgataatactcgtaaggcaagctatacatgtagttgacttctgggagtgttgtatggaatgaagtatcaaagacggcaacactaatgatatctgggagaatcttcttaaaggctttgatgccaagcaacgcagccggctcatgaagtggtgcaaactctgttaatgactcgatctttttgatgacctcgtcgtcaatcacaactgaatccgggaagagttccccaccagcaacaattcgatggccaacaccggtaatttcactatagtctttgatgatgtccaaactcaacagtttatcaaggacgagttgaatagcctgttcatgattatcaatatcttgggtatctttgaacttcttgccgtcaccgtacttgattgagatatctgatgcgcccaatccaattcggtcaatagcaccgcttgaaagaacggtttcctcaggcatttggaacaacttgtactttaaggttgaactaccagcgttaattgcaattgattttcccataataaataatgctcctctgtattttttaaaaagcttgataaacaattttataataaatcagtttgttcccaatcatcaatctcggtcaagaacttggtaaaggcttgttggtccttaaatgatggaaattcccccaacattaccggatccacctgtttggcaccgtcgccggcattttgaagaattaaaattgccttttgagccgcggcgtttgcaaagagttcttttggtaaattaagtaatccctgcaggtaaaccttcccttgcatccatttaagaagctgcttggcttcgctggtttggaaaagctgacttggcaccaggaagaaaccaaacccacccggcaaaacatgcttcatgccaaattcaatcagcaaatggtgcacgtatgaatgacccgtgtctgaatgggtagcaaatcccttggcattagcatcgattggatagtagccaatcggcaaatcactaacaactacatcgaccacgggagctaaaacattttggatcgtatcctcgtggaaaagctcagcgtgaatcttttgcagctcgactgagtctgcagccaattcaaacattgcatcgtcattttcaattccagaaatggtcggtgtaacgccaatactagtttgaagctgatgataaattgctgttagtagattggcagttcccatcgccggatcaagaatacttaattctttgcggtcatggaaaattccagcaataatatagccaatgacgttggcaatggtatcaggcgtcagttggtagttagcctgaatcgtgtcaactcgaatcgccttgagcacagccatttgaattgctttccggaaagtttcggcagtgaaatcgtccggattaaagtctgcataaatattagtcagctttttggtatcggcttcagtcagttcgtcatcttcttcatcgtcactctggataaatcccagtgtttcgatgaaagaatcaagatacgattgatccttggctttttgaatcaattctgtcgaacgattcaagatatcaaaaagctgctcaattttcccttgagccagaactctcaacccctttattcaatagttgaacactattaaatactaccagataagctgtcaataattcaagttagattgttatttcacaaccacaaaaaggccactattcgtgaccacttgtgcgttttgggtgaacatcttttttgagtggcttttcaaggaattgccgtctcatttgccgttcatgctcggtgatacgattaattgatcccaactcctgcttataagcagccagttgaaacatcaagcatgacatcaaaataccgacaaaaatcacagccaccaccgttagggatccacgcttatatttatcaatccttgaacggtaattttgaataagctgaacacttttggccattatcgaaagtaacatcagttcttagacaccccctgctctttgtccagcgtacccattgaacatttgtcaacgacggtacgtgacccttgtaggcaccggccaatcgaaccatgttttcataccgttcaattcgataagtttttttcgtgaccggactgtacatcacgcacttagagggttgacactgcttgatttcaaaccgataacggtcagattcgattatactgagataagaatgaaaattgatcacgttttgctttttttcgtttcccgcatatacgatcatcgtcatgatcgtccaaatggcgaatacaccaatcaccaaggtgatcaggccctcaattaataagtagcccggccgagtatcaaccttactcacggacaatttctgcttcatatttttgcctctcaattgtcatcactttttctgcgttggtaattgtctcattcatttgatgggtggtttggatgtagaacaaactgaaggtgcagatgatggtcagcccgattaatgaatcgatcaccgtaaaagcccgcttatttgttcctttccacatgatagccactccatcccatttgaattttttgattgtatttgacgttaccatccgaatcaagccaaataatcttagttggtgatgcaaacccatcgtcatgggcaatcatgcttcgttgtgatctcacgtgaatggaaggcggaaccgaaattcgctcctcatttacctcgtcatagtgagttttcttcaccttcatcggaaagaaaataacatctttatcccgaatggagattcgataagaaatgttctcggcctttgcgtttaatgtcatgcgggtccaggcactctgaaatgaccgccaaaacaacgcctcacttggatttccagactggacgaccttgatcagcatcaaattaatcatcaagacacctaacaccacgcctaaatataccaccagctcaataacggtaaagccctccctatttttgcacttcattatgagtaatcttcaggccttcatccttggcttgtttaacctgcttggcggtgagatagccaccttttgtcaggtctggaaaactaactgatttggcggttgggtgctggctgaaataggcgtcaatttgtgcctgaacaacttcggtcattgccgatgaatgaacagactgggcgtgttttctttgattggatagatttggaataatgattaaaattaataatgaaataataaacaagacgatggtcatttcaattaacgtaaagccttctctcattttcttaacgcgctttttcatttcaatacattcctttcactgagttataaattggaattagcagttgaaaatatgtcgaaacaatcgtcacaccgatcaccacaaacatagccggctgaataaacccgatcagtttatcggtggtcaggatcatttcgtcaaacatcaaccgtgaataggccgtcatcgaattggccatttccggaatcgtgttgccggagctcataaatttgataatctcattgggaataaaattgtgccggtctaccaattttcttaaggaccctcccgaaagtaaagtggcatgaagcctttcacctaagagatgaatcagtgatccctccttgaactcggataacgtggcataaatttctttaacactcaaaccgtttttcagaagagtggccaaattgctggccagataataagcgatatattttcgaaacaatttgccgacgacgggaattttgacaatcatttgggcctgggttatggcatcctgtcgactccagtgaactgtgctgccaatgatgccgatcaaaattgggattggcgaaagtcgaatcagctgctgccagtacgtaaccggttgctgatgattggctgtgggcattaaatcctgaatctgtggcaaaacgtagactcgaatcatcaagatcaacgttcctaagatcaggcacaaaaataatgggtacaccaacatcgctttgatctttttgagttgtttgagccgcaatcgatcaaagttggccagttcgtttaaaatgtcactgagttgaccgtgcttctccgcgattaacagctggtgataagcttgagtttcaatcaggggtcgaacactttccgaaaattcccggccggactttaacgatccaatcaccacattaacgcctcgggacaattgtttgtcagtgtcggcgataaatttcaacgcttgagtcagtgagaatccaattgacaaaagattcgccaaagagtcaaaaaaattagcttggaaaaccaccggccatttcttaaccgaactcgaatcgttgtgcagtctccggcgtaaccagttttgctttaacagctgttttgagtccatcctgccattcaccccaatcgtatgtattcatattgaccaactctgaataatcatgtcccatcaacattgcccgctgtttgccgtcggtggttggaatcagccgctgataagcgacgccggttaatgcttgggcaataaattcgtcgctgattccgagctgtttgagccgatcaatgactccaaccggatcctgagcgtgaacggtggtgtagaccaaatggccactcagagccgctttaattgctgcttcggctgtcattgcatcacggatttcgccgacgataaagacgtcaggccgatgacgcaggcccaccttaatcaagtcggtgtagtccatccctgcatcgtggttaacctgaagttgtaaaaaacgtggttccctaatttcaatcgggtcttcgatcgtcatcacaaattggtcggaaaccatctggttcaccaaattataaatggtggttgttttcccagagccggttggcccggaaaagacaatgagtccgcgttttcgactcatttcggaaattagttgaacttgtttttcatcaaaaaatgccgcgtgcacatcatcaagctgatagataatccggatgaccagtgactccaaccccgtgaaattgccgaccgaggataatcgtaaaaaatattggttatcaccaaaatgccaatccatcgacccaatttgtggccgccgttgttcacttaatgccatatctgcgatgtacttgcaatagttcatcatccgtctcgcctgtagatagccgattttatcccaaacaacgacttcgtttgcattacgaattttgaccaagtattcgtctccttcaggcaaaaaataaagatcactggcttgtgttttaatggcttcattcaaaagaccattaacttgctgactaatttccatttcattcacctcacatgtaatacatacgaatgaaaagttgaattttatttatcaaagcacaaaaaaatggccgatcaaatgatcggccattgagacattgaaatcatattaaattattcttctggtaaagtagcggcttcgtaaacgtcttggacgtcgtcgttttctgcgagttcgtcaattaaaccagtgtattgagaaatcttgtcctctggaacttctgtcgtgttttcagggaaaagacgaacttcggcagtatccaagtcgtagcctttttcctgcaaagcgtcgcggacgtcgtccattgatttgggatcagtgaagatttcgaattcatcatcactggtcttcatatcatcggcaccggcatcaagcgcgtccatcaacattgtgtcttcgtcggtgtcaagaccatcacgcagaatcacaatataaccctttcgatcaaacatgtatgaaactgatccacttgttccaagggttccgccatgatgagtgaatgcagaacgaattgcggcagcagttcggttcttgttatcagtcaaagcagaaaccatgatggctgtaccaccgggaccataaccctcgtaagtaatttcttcgaacttagctccaccaataccggaagccttatcgatcgcacgttgaacgttatcctttggcatattggcagcccgtgctttttccatcactagacgcaactgaggattgttttctggatcaggatcaccttttttagcggcttgatacaagtcacgtgatattttttggaaaatttttccacgtttagcatcctgagcgtttttacgcccctgaatgttatgccattttgaatgtcctgacataataactcctcttttctaaaatttattagctggttacaaacatacgtcaatattctaccagatacgcccccctctttcaagaaagcgcggccaaatatgtggcggcttttcaaaccagtttccagaacaaaaagagcgaatcgccacggtccactcctttgatttgatacctgattatttggtagattcacgcttcatcaaaccgtatgggagcaacacatttttttcgtcaaccggttcgttgtgcatcaatttagtcaacagacgcatggcaacggcaccaatgtcgtacaatggctgggtaattgaagacatttttggtcgaaccatttcggttaacttggtatcgttactggtgataatttcaaagtcatcaggaactttaacatcggcatctgacataccgttcataatcccggcagccaactcgtcgtcggtaaccatcgcagcggtggcgttaactgccattaatgctggttgaagcaaggttccggtcttgtatgtatcatcagtttcaaagaccagcttctcgtcgtaagggattccagcgctctttagggcctgtttgtagcctttcagacggaatttgccgttaatcgcctgctccaaggggccacaaacgaaagcaacccgccgattaccacgatcaatcaggttcttaacctcttcttggacagcggcaacgtagtcgatgttgactctcgcgtagagatcttcttcatctactgatccggcaaacacgattggcgtcttggttcgcttgaattcttcacggagcttatcgttaatttcgttacccatgaaaataatgccgtcaacttgtttggagagcaaggtatttaacaccttaacttctttttcattgttggaatctgaattggtcaggataatattgtatttatacatggtcgcaacatcatcaatcccacgggccaatgaggcaaagtacatattagtcacatctgggacaatgacgccgacagtcgtggttttcttacttgctaaacctctggcaacggcgttgggcctgtaatccaatttttcgattacgtcgagcacttttttccgggttgccggctttacattggcatttccattgactactcgagaaacggttgccatcgacacgcttgcttctctggcaacgtcataaattgtaattgtttgtttatccataaagatagccctttctttctcgttagaatatgttttcatcgattttcaaaacatcatctaatataccaaataaaaaggttttcagcaaattgaaaacgttttcagtcaaatcataaactaagattgctgaaaattcaagtgaaaacggaactttacggcgataattgaaaagaattttgtatgatatactgtggataaaataacgaaggagtgatcctatgaacaagatagaacaaattcaacggtggctggctgataacggccaagacatcgcactgattaccgaccctaaaacaatccaatacctcaccggattttatagtgatccggttgaaagagtcttactgatggccatttttaaagatcaggaaccatttatctttggcccggcactggaatcagaagccattaaagacaccggcttttcatccccagtctatggctacctcgaccacgaagacccttgggtgatgattgccgatcaaattcatgccagaaatactgacgacagtcattttgcaattgaaaaatcccagctccaggtagaacgattggaagctctccaacaagttcttcccaacgcggatttctcagcgaacctgaccccactgatcgaacaaatgcggttaattaaatcggctgacgaaattgaaaaattgaagattgccggcaagtgggacgattttgcattacaaaccgggtttgaagccgtccaggttggtaaaacagaagaccaaattgccgctgatctccaatatgcactgatgaaaaacgggatcatggaactcagtttcccttcccttgtccaagccggcccccacgccgcagaaccccatggggcaaccagtgaaaataaagtccaaaataaccagctggtcttatttgatctcggaactgtctgggacggctacattagtgatgcttcgagaactatcgcagtcggtaaacccgatgaaaagtcaatggacatctaccaagtttgtctggaagcacagctggctgcccaagaagccgctaaaccgggaataaccgctgaagaactggataagattgctcgcgatgtcatcaccaaagccggctacggggaatacttcattcatcggttgggtcatgggatgggcatgagtgagcacgaattcccatctatcatggctggcaacaagatggaacttcaaccggggatgtgcttctcaattgagcctggcatttacattccaaacgttgctggtgtcagaattgaagattgtgttcacattactgaagatggctgcgaaccatttacgcaaaccaccaaggaattacgctacattgaacaataattaacagcatcaaaaaaacaacctcatttgtgccttatctcaacagctgaagtttgactttgactgtttggataaattgcacattgaggttgttttttatttgtgatcgttgttatcggagtcgtcagtgattggaatctcattatcgccgtcatcctggtcggattgtgaatccaaatcatcagcagccttgggaattccggtatcttggaaggcatctttagcatcaacaacaatatcatcctgattgtcgtcagcatcgtcatcatcagctgcttggtcggtaccaaacgattttgctttgtcagcgaattgcgttttggcatcattgacagtccctttggtattttgcatttcatcatgaatcacatcttttaagtcgctaacggcatcgttggcgtaaaacgcgtagtcaactgcccgatcccgcaactcatcagccttttgacgggcgtctcgtttgagttgggccttctttgcttcgtccaatttttggtaggctgcatatagaccggcacccaatgcaccagcgaataagccaaatgctaattttttacccattctaatcatcccttcgattgtttatttagttgtatcctttgaaccgtgtcgattgcggtacatgttccaggcactcttgccaaacttaccggcgagccctgctgaaacaccctttttaccggtatctttgacccgtttagtgaggttttgagtagcggtatttaaacttgacacactctcacccaaatcagcggcggcttgaaagaccggtgtgacaatgttcaatttgtcatcaacatccttcagtaaatcgttggatgttgccataatattatcagtttgtttggcaatgacgtccacattactagtcattgtcttaattgtgcggttcacttctgaaatagttctgcttaccttcattaagaataagccaatgaagattaccaaaagcaaaaatgcagttgcggcgataaggccggctatttgtccagcagtcattgatcttcctccttgtgcaacatttacttaagaatagcattccagcaatggtttgacaatgaaaatgaacgaagagtggtttcttttgtagaaccaatttgctaagatgatattatacacaaagcgaggaatcccaatgataaataccttaaaattcacagttttagccattaattggcaaaaatatctcaacatggttgactgggatcagctggccatgacgattctggaaaaagtcggattattaattttattcagtctgttatttttactctttcgtcggattggtaaaggactgattaatcattttttcaaacgctatcggcgcaaatatcaaaataccgtagcagaaaaacggatcaagacctttcacaccctgacgctgaacattttgaactactgcctatggttcttctggatttactccattctctcaacggttggggtgccagttggaaccctggtcgcctcagctgggatcttcagcttggcaattggccttggtgcccaaggatttgtgactgacattgtcagtggctttttcattcttcttgaaaaggaaattgaagttggcgaatacgtccaaattggaacaattagaggaactgtaactgcagtcggactgagaacaacgcaggttgtcggggacgacggcacgttgaatttcatccccaaccgaaccatcaccaccattgccaacatgtctcgaaacaatatgacggcgatgattcaagttggcattttcccacaaacgccagttgataaagtcacccaaattatccgccaggtcaatgaagaacagatcccccactatccggatattatcggagatcccaagattcttggcaccattagcctccccaacggcaaactggttgttcaggtaaatatcaccacaaaaaacggcagccagtacgaagttgcccataactttttggccttctatctagctgcaattaatgaggccgggattcaactgccggcgagcccaacaatggtgaatggacaagccaactgatgtttgaataaagtgaccaattattagaaaaacgagattgccggcaaattttgtcagtaatctcgttttttgacttaattcatttttgtaaccatcaacgatattcacccaatggattatcgattaatcagacccttggagccttgaatcttggcgtgcttggtttcgtttttggatttgtgattatacaccggcaaagcgatgtagtgtttattaaagttgtgagccaaataattaatttctttaaatagttcccgacgggtaatgattcctttaaagtgattttcagaatcaacgtagaccagaaagttttcatccaccaaatacctgagaatggcttccaggttatcccgctcgtaaatcgttgggacatccttttgcatgatttgcttaactttcactgactcaagcggtcgactggtaatgccggtatcctgcatcatgagttcagtaatcatgggtaaagaaaccagtcccatgaaatggttatcgttatctaacacgggaatttttgcgtatttaactttcgtcaaaaccatgaagacgtgttggagatcattgtcttgattgacagttgcgaccaaatcagcggggattaaaatatcccggtgactttcacgcatcacggtctcaattggtttatcgatcatgtaatcctagactcctttttggttagaacggaaaacgaagttccaaattcgccaccggttcaaattggcggttgtaatattgaacggtgtaattgcgttgatccatgctgataatggcataggtaccgcccaacccggcgtattgcccacgtggataggcaatgcttccaggattcacaaacagcatctgatcgtcaaaaacagctcctaattgatgagtgtgcccaaaaaggacgatatcggcggataagctccgggcatataattccaaattaagcatgccaccattcacgttttgatgatgcccatgcgtcaagaggattcgtttgccgctaatttcttgaaccaggtggtcgggaaattcggcaaagtccatattcccctggacaatccgcagttgagaaactaatggatcgtccgccggtaattcagaatcgccgcaatggaaaatggcatccacttgaccggcgtatttgttcaccaattcttggataatggcgcgatctccatgactatcactaacaacaacaattttcatgagtcccacaaccccaacaatttacggatcaggttgcggatggcattgccccgatggctaatcagatttttatcatgggtgctcatctcggcgagtgttcgctgctggctgggcacatagaataatggatcatagccaaaatcgttattcccacggcgttcacgtaaaatttcgccgtcgattcgaccgttggcaaccaccttgtcaccctcaggcgttaaatagaccagaacagattcaaagtaagccgtccgatccgttttgttttgcatttccttcaaaagcttatcgttgttggcgtcatcatcgtgatcacctgcataacgggctgagtggacaccaggttggccgttgagtgctttaaccaccaggccggaatcatcagcgatcaccgcttgatgcgtaaagttcatgatgccggtggccttgagggtggcattttcttcaaatgtggtgccggtttcagcgatcgtcggcacattttcaaaatgcttcagtgatttaattgtgataccggttggtttaaaagcatcctcaaattcaatgattttatgagcgttttgtgaggcaatcacaatcgattcgggtcttttcacgttatcaaactcctttaaatatctaacttaacggcactgatcggtgttcccagtaacttgtcggcaactttggcgaaatccgccgggttcccggtggtgtaaaatcttcgaacacgctgtttttgatcgggggcaaaaccatcatgagctgctaaatctgccttgacttgctgagcagtggcgactcccgggtcaatcaacgtgacggcgttgcccatcacattttgaatttcattttttaaaattggaaaatgggtgcagcccataaccaaggtatcaatcggtttatccataaaccaagccagtcggttgttcaccgcaacctgagcttcaacggttccggcaagcccctcttcgaccatcgtaacaaattccgggcagcctaaggatgacacaactgctgatcggttggcttgtttgatcaatcgctgataatctccggagcggacggtgccgttggtggcaatcacaccaatctggccggatttagaggctttaacggccatttgggcacccggttcgattacgccgataaccggaatcggtaaaactttctttaaatattcatatgccgcagcagtagctgtgttacaggcaattacaaacattttgatattttgttcaaccagatagtctgcaattctttttgtgagttttctgacggtttcagaactcttttgcccgtacggtaaattggcctgatcgccaataaagatgtacgattcattcgggaggattttggtgatttcctttaagacggtaagcccgccgacccccgagtccataacgccaatcggccgattatccaacagaattccttcttcctttgtctcaataacattattatcttgcaaaagaatctttacttcaacttacaaaacaagattaatgattttattgtataatttatttattacattttgcattgatggagattaaaaaatggataacgaagtatacaagcattttatgactgacgatacaatgagagacctactgggccaggaattaattcgcgattcactgattcctgagattttaggcaaagacgcccacgaaatttcctattgggccggcaagcatctggcaagaaatcatcgtctggcaacctatgaagatttggaaacctttttcaaacaatttaaatttggtgatctaaagctacttaaacgctctggtaaccagatcagctggaagctaagcggcaagatcgtcgcccagcgtctcaacgcatttgatgatcctgatttttatctggaatccggattcatcgctcaaagctgtcagtatattcttaaccaacaagccgaagctgagctcgaaaaggccaatgttaataagggatttgtgcttttaagcacctatttgagccctgacaagccaactgatggtcaagaagcttctgctatatttgaaatcgttcaacccgatcccgatgacaattccaagcctgatgattaactcattggaatcaaaaagcccaccacaaaacctgatttggttttgcggtgggctttttgactgtgaaccgcttgagacaccgaagtcattctaaagactagccggcatattgatcaagcacttttttaacttgggcctttggatgatacccaacgatggtatcaacaactttgccgtcttttttaaccaacaaggttgggatactcatgataccgaatttggataaagtttccgggtttttgtcggcgtccattttagtgaacttaacattatccatttcttctgccagctcttcgatgacaggtgtctgcatccgacaagggccacaccaagttgcccaaacatcggttaaggtgacaccttcggcagtgtctttttcaaaagtttgatccgtagtttctttaagcatattaaaacactccaatcctttaatagtttaatactaacaattttttagcaaaaagcaaacagattgcacacaatcatttttattttaacttcacaaccgttgaaccatccccaccagcattcggtgcagaatagccaaaactctttacccgtgggtttcgtttcaaatattcggtgacccctttacgaagcgccccggttcccttgccgtgaataatcgtcactgaagggtagccggcaagtagggccgaatcaatgtagcgatcgacttctgtcattgcttcttcgtatcggtgaccgcgcagatccaaggtcggtgacatcccagtcgacctggtccgggacacgtgggtctgatactgattcttatcttgtttggctggagttgccttttccaaatcagattcttcaatctgcatcttcaaaatgccgatttggacgtcccacgtatggttcttatccttcctcagcaacgtcccctgttgaccataagatttgaccaaaacatcgtcgccgggatggaaatcgtgcttggccttttcttttcttaaaaccttattctttgtcagacttggagcagattccaattgattgagcgcccctttggcatcaatcagctcgttttccttaacggcaactttgccgacctgggcctgcttttgatgcagatcatcaataattcggtcggccttcttcttagcttcttcgaccacttgattagcctgttgcttagcctgttcgacgagccgttccttctgactttcgtacttggtaaacttgtcttgcaggtcatgctgaagccgggttgattctttcagttgttgatctaattcatcagcttcatcgtgagcccgcttagtttgcgctgtcagctcttcaatcatattattgatgtcttggttctcggagtcggtaaacgcccgtgcctggtcaataatggcctctggcatcccaagtttgctggcaatgttcaaggcgttactttgaccgggaattcccagtaaaaatcgataagttggctggagtgtctcaacatcaaactccatggatgcattaataatcccctgccggttgtaagcaaacgcctttaattcaggataatgagtcgtggcaatcagttcaccgccaatttgatgaaaagcatcaataattgccattgccagtgcggccccttctttggggtcggtgccggcaccaagctcatccagcaagaccaaactatctttactggtctgttttagaatactaatgatattgtccatgtgcgatgaaaaggtactcagattggcttcaattgactgctcatcaccaatatcggcaaagacgttatcaaacacgccgatctgagagtcttcattggcagtgataaacaggcctgactgccccattaactgcaggaggccgactgttttaatggtaattgttttaccaccggtattcggcccggtcacaataatcgtattgtactgatcgccaagttcaatatcgttggcaacgacttgatctctgggaattaacggatggcgcgcctttctgagattaataacatttttcggtgacactttgggcatcacactaccagtcgcatgggcaaatttggctttggcgttcacaaagtccaattggccaaccaaatccatgttggccaacaactcgtcacgatgcgggcgaattaaattggttaactctgccaaaatccgccgaacttcagctctttcagcaagctgatcccgacgcaattgattgttcatttcgacaacgttgtttggttccacatacaacgtttggccagaggcactttgatcatgaatgatgccgccaaatcgctgcttatattcggccttgattggcaggacaaacctaccgtcacggacggtaataatcggctcagaaaggtatttggcatctgaacccttaatgaacttccccattttcgaacgaatattactttgagtggcagcaatggtccggcgaattgaacgtaattgcgaagaagcgccatccagaatgcggccgtcttcatcaaccgaagccaccattcgtttggtcacttcaggcatcaatgtgagccgatcgacaattgagggaacggattttaaagtcacttcttcagccgccaaacccctaaaaaattcagtgacgacctgcacagcgcgtagtaatttggtgatatgagacagctcagttccgcttaatgacgcattttcaatccgcaggcgtttcatatacggtgcaatatctgcgagttttggaatcggaatttctccctttaagcggacaatgtcagccccatcggccgtctgtgccaagcgttgagaaacggtttcaaaggaaggactgggtgtcaataaatcgacaatttgtcggccacggtcggtcgtcagatatttggccagctgctccttgatttttccatactctaatgtttctaaaactttttcgttcatacattaacctcactagaatgttgattccaaatctgaatcattttatctgagagaatcggtgtttttttcacaatccactgggaaacgtcggattgttggtactgttcttgaatgctctgatcagggaacatcagcagaaagttcagcaagatgaaaatgaacaaatacttgatgagaagatctgcggctgcacccagtagtgcgttcaattgatgtaataatggcaggcgggtgatcggagataatagatcactcagcaaacgaacaatccgccaaacaaacccaaaaaggaaggcaaagatcacccatttgataatcaactcagcagtttgattgccgccgtttttaaaaattgcctgattaataaagtcagcaattggactggttccaacgatactgacgattgttgccgccaaaaagccaatcagacttaggacttcattcacgaaacctcgatgaaggccacggaaaaagccaaatattaaaatcagaatgatcccaattgtaaaaatcatctaatgaacctctttactgtgtgcgctttcctcaacatcaaattgtttggagattgcattaaaggcaattaggattgcccgctgctcatcagtggcagttggcatagcctcatgaagttgcttgagctgctcatttaataaatcggacaccgcctgcatatgatcaaccgatcccttaccgacaagcacgtaatccttgccatcaatggttgttttgaagcgacgtttttcgttactagacattacatcacatcctaaattctttcaattaaaaaggactgagactcaacgatgcttcgcctcaatcctttcgcaatagggacaatctttaattattgattgtcgttgctgtcatcatcctgatcgtcgccatctttacccaagaaggtgttcaaaactgattcgatcatatcccattctttgtcagtttcaattgcttgaagttctccaccttgaggatcacttggatcatcaccctttggcagtgcataagcttgaatttcgacttcttcatcttcacctttgccatctggataaatcagaatgtacgaccgatcaaagtcctctgatttaaaagtgaataatacgtcgtataaagtttcatcgccgttttcgtcgactaatgtaatttgttgttgtactggttcttggtctgccataattgtttacctcgctatattttagttaatttaccattgctgtccaaataattctgaagtatcaagccagcggccagcttatcgatcacttttttgcgcttggccctggaaacatctgcttcttctgtcaacatccgctgagcctcaacagtcgttaatcgttcatcttcaaaatcaaccggcaagttaaacttatcttcaagtcgtttgccatactgttgtgaagcttcagcccgggggcctaaagaattgttcatgtttttgggaaggccgacgacaaatccatcaacttggtactttttaaccaactcggaaacccgatctaaaccaaattccttgttgtcctcgtcgattcgaattatttcaaccccttgtgaggtccagcccaactcgtcgctaacagcaaccccgacggtctttgaaccaacatctaaacccattaatctcatttttcaccttttttcgtttcggttggatgattatccaaatagaaacgaactaactcttcgattatttcatcacgttcatgtcggcggataagatttcgcgcatcaaggttacgtggaatgtatgctggatcgccagaaatcaagtacccaacaatctgattatatggattgtaacccttttcttccagtgctgcatacacagtcaacaatgtttcgcggacgtcttttggctgaccttcattaaaattaaaaaacatggttttatctaacgaactcatacaattcacctctatgacttaaggtcatttgtattaattttaactgattataagtgaaactacaatcaagtaagccaatgtaaccgacatgtaaccgtggtgtaataattatttatttgccaaccaatcaaccgctgcgctcatcgctttatcaaggccagcaggatctttgccaccagcctgagccatgtttggacgaccgccgccgccacctttaatattgcccgcgatcgatttgatcagatcaccagccttaatgcccgccttgatctgttcatctgccactgcgacaatcaagtttgctttgtcgccgctgccggttccaagaaccaagacgtcagacaaatgcttagagcgccaagtatcagctaattggcgcagctgatccattccggcatctttgatgattccggtgataatggaatacttaccggcagttttcttgtcggcgaaaacattttgagcctgttgcccagccaatttggcttccagtgactgttgtttttgggtaagatccttaatttcgcccagtagttggtcaacccgtttgggtgtgtctttaatttgggtgactttcaagtcgccggcaatttgtttcagttccttttcatgatcgttcaacaacttgaaagcatctttggctgtgaccgcttcaattcggcggacaccagccccaactccggattcagagacaatcttgaataagccaatgtcgcgggtattgttaacatgagttccgccacagaattcaactgagaagtcgccaatgctgacaacacgtactttatcgccatacttttcactaaataaggcaatggcacccatctttttaccagtcttaggatccgtgacaacggtgttgacatcgatttcattgaagatttgacggttaaccatatcttcaaccttctgtaagtcttcatccgtaacctggccaaagtggttaaaatcaaaccgcaaatagttaggttcaacgagtgaaccagcttgttgggtgtgtccacccaaaacatttcgcaatgattggtccaacaagtgggttgctgtgtgattcttctcaacgcgactgtggaataatttgtcaacaatcaagtgataggtcttgcccttttcgagtggttcctgagtttttaatgtgtgcaaattctgaccattgggtgcatgctggacgtcaacgacatcggcaaccttgtctccctcttcatcaaggacaactccccggtcagcaacttggccgcccatttctgcgtagaatggtgttctatcaaaaatcacttcaacagagccaccctttgaatgatcgaccagtttttcgttctcgacaatttccaaaagctcggcgtgatcgacatccaaggtatcgtagccaacgtactcgcttggatccttgatttcaattaagagatcacgttgaacacccattgacttggcaccacttctggcctttcgggcacgatctttttgtttttgcatttcaacctcaaagcctggcttgtcaacggataagccggcatcattggcctcttcttccgtcaactcaactgggaaaccatacgtatcgtagagtttgaaggcagttgggccatcgatggtcgtttgatgatttgctttggcgtcttttaccacttgattgaacagtttcaagccgtcagtcagcgtttcgttaaaccgatcttcttctgaacggacaactttggcaatataatccttttgcttaagaacatcaggataatatgattccaaagtctggccgacaactgggaccaatttgtataagaacgcttcgttgattccaagccgctgaccgttaacgattgctcttcggatcaagcgacggataacgtagccgcggccgacgttggaaggcaatgcgccatcgccgatagcaaccgtgattgcccgggcatgatcggcaataattctgaaggcttcgttatccttcttgttggtatcgtatttcttattgtcacttaattcttcagtcttgcgaatcatcggcaaaaagaggtcggtttcgaagttggttcgggcatgttggaaaattgaaaccactcgttcaaggcccattccggtatcaatgttttttcgaggaagtggttcgtaagtatcttggggggtgtgattaaattgtgaaaacacaatgttccaaacttccagccagcggtcattttcaccacccggataattttccgggtcatcaggagctaaattgtcaaagtccttgccgcgatcatagaagatttctgaatcggggccggatggtccctggccaatatcccagaagttatcctcaatttcaatgatatgatcaggcgcaacgcccactttttcccaatacattttggcatctttatctttcggataaaccgtcatataaagcttatcgggatcccagccaaaccatttgggtgaagttaacagttcataggcccaggtaatggcttcttttttgaaatagtcaccaactgaaaagttccctaacatttcaaataaggtatggtgccggggtgttttaccgacgttttcaatatcgttggttcgaatactcttttgtgaactggtcattcgtgggtttttcgggacaactgaaccgtcaaaatactttttcatagtggcaacacccgaattgatccaaagcaatgttgggtcgtcgactggaatgagtgaggcacttggttcaatggtatgacccttttcctggaaaaaatcgaggtacatctgtctgatttgaccactgcttaactgtttcatgttctcttctcctttgacaaaattaaaacaccgttgctcacagagacgcccattgacgcggtaccactctgattgcaacgatgtttatcgttaaccacttgatctctataacgcagagttgcgtttgataatttaacttttaagagagcaccgtttaattttcgtcgcttttctcaccaaccaaaacgtctctgaaacaaaaaattaaacggcatgttcttaacacatctcaaagtatacttttttgtgaatatggtgtcaatacagacctattgataccgtgaagaactattcttacgttgtttccgtttggcccgtgcttcctcacgtttagcaacccgacgatccatctcgtcctttcgggcaatggtatttttaattcgccgtttgtagcccggcttgatcttcttctttttcttcttgatcatgccgatcatcgttggatccagcttatcgtgtttctttcgatgagtctttcgacgatttcgatcataagaatccacaatttcgccgttcttaagggctttcggttggaaatgaatgcccatatcttcaagttcttcaacttctttttcctcatcgggagaatacaaggtaatcgaagtcccggacatcccgtttcggccggttctaccaacacgatggatgaagaattccaaatcctcggtgggaatatcatcattgataacatccgataccccttcaatatcaatccctcgagcagctaaatcagttgcgacaacgaattgaaattcgaggtttttgacccgcttcatgatttgcttacgttcacgaggcttgagaccgccatgaatcatggcgactttcaatccctggcccttcaaatattcggttaactcctcgactcgtttgcgggtattggcaaaaatcaggaccaaataaggttccccaatggtcagcaatttataaatgagttgatttttgtcctgccccttcgtcgaaatcaaccaattatcgatcgtcggactgataattgtcgacactggaatctcttcgataaaaggattaaccatatatttcttcaaaaagacgttgattttttgtgggatcgttgccgagaaaaccatcatctgaacatgtttcccgaaactggcagcaatgttatcaaccacatccaagaatcccatgtccagggtcatatctgcctcgtcgataactaactgagaagccgtgtgaacatccagtccaccgttttggatcagatcccaaattcgacccggagtgccgacaaccagttgaggctgctcatgttgaatctttttttcctgacgggccttgtcagttccaccaatgtaggcaccggtagaaattggttctggtgagtgcttagccaactgcttagcggcatcaatgatctgataggctaattcccggctgggggtggtgatcaccgcttgaacctcatcttttgcgggatcaagctggttaaaaatcggcagcagaaaagcatgggtcttaccactaccagtagcggattggcccacgacatctcttccctgcatgataacgggcatcaccttttcctggacgggtgtcgggtggctgaagttcagctccttaacagcatccaataagaatggctttaaattaaattctgaaaaattactcatataatctcctacttgtttttggcgactaaatcattcaaatcgctcacaaattccttgatgtgggcttcatcttcgacaacagcaccacttgcgagtggatggccaccgccgccatactgcttggccaattcgttgatttctggtcctttagagcgcaaccgaatccggaaggagccatctttttgttcgacgaaaattgcccaagaaaccacttgtttgatcttgccaggtaacggcacgacggcagaagtactttcgtcccctaacttgaagggctctaatactttattggacaaaaccagataagcggcaccgctatcaagaatattcaggttctcataaacataagcggacagccgtgccagtggaatgtcgatctcgtcttctattttgttgacttcactggttgagaactgatattcagcaagttttgaagcaactgccaaagtatgtggcgacgtggaaggatacatgaatctgccagtatcaccgacgatcccggcataaagcagtcgggcaccttcatcgggcaaagttaactgatcacgattggcatcataaaaatcataaatcagctcagatgtacttgatgaatcgggctcaacccacataatgtgaccaaactgatcgtcgtttgggtgatgatcaatcttaatcaattcttttcccgtcgtataacgttcgtcatccacacgcggctgattggcagtatcaacaacgatcaccaaagcatctttatattgctcgtcggcaatttcatcggtggttcccaaccaggcaaaactatcatattgtttaccagcacacaggactgtcttatcaggaaatgaccccttaattagttgagccagtcccatctgcgatccgatggcatctggatccggccgtttgtgacgatgaataataatggttttaaattttttgatttcacttaatatttgatcttgaattgacattttatttgctccataactttattgtcgaacacttaagtatacattactttgtgaataagataaaccgctggggtggtgaattaatcaaacaggtgaagaacaatgttctcgtaagttaaatcatccaggttggtaatggtgattcccaacaggcgcaccccttttgaaatatccggcatatcgaccagtaaatcgttggcaagtgtaaagtattcttcggggctatttttaagatagttatccatcgtgacccgcttggtaaacgttgaaaagtcggcataacggatcttaagaaccaatgttttaccgtgcttctttttgtcatccattgccttgaccaccatcgcagcaattcgctggagttcgtcatcgacttcggtttgtgtgtcaatcgccgggccaaatgtccgctccttgccaatcgattttcgaacccgctgatactcaactggccgatcgtcaatgcctcgagcgcgctgatagagaacgtaaccaaatttaccaaagtgcttgatcaaatccatctgcgaccactgaatcagatcctgaccgttattgatatttaattcatgcatcttgggaacggtctttttcccgacgccgcggaacttttcaattggcaaacggcttaaaaattctaatgcatctcgctgttcaatcactgtaatgcccactggtttggcgtaatcagaggcttctttggcgagaaacttattgtaagatactcccacggaacaggttaagtgggtggcatcccaaatttcattttggatcattcgggcaacttgaatcgggtctgtgagatgttttttattatgagtgacatccaaataagcctcatccaaggcaacgtactcaatcacttccgtgtactcgtgaaaaatctcgtggatttgattggaaactgagcggtaaagatcaaatccagagaaccgaaaaaccgcctgcggacaaagttccagcgctttcatgacactcattgcggaatgtaccccaaattgacgggccttatagttagccgttgcaaccactcccctgccgccggttttgcgcggatccttggcaacaatcaagggttgagacttgagagtggggtctttgcgttcctcaatcgacgcataaaaggcgtccatatccacatggatgatgtttctagccgatgttttcactgagatcaccccaatcaaacatatgttctttgccgggtaaaaaaatggtcgggattatagaaatcaacttcccaaccgacttggtcaaactatttgtcttccgactttgtttcatctttggtatcagaatcttcggtagcgtcctgatcgctctttgatgaagcagcgtcatctttgtgatcatcatttgcagtagtagttgtatcgttgtttgctgcaggcgcagcaacagcaggctgcttaaccgaagcaattgcgctcagatcaaataccaagtagataccatcacaatccaaagtcacggttttttcggcttcgttgatttcgtcaacgacaccatggagccggccaatcgtaatcacttggtcgccttccttgatctttgaaagttgatcccgacgcttttgttgttgctttctttgaggacggatcattaagaagtacatcaccgcaaacaagacaacaatcattaaaattgagtaataagattgattcaaaatttttcacccacactttccatagtaatactttaccaaataagccctgaatagtctacacctaaaagttttttggatttggtttgttatatccatactgttcaaaaacttctgcccgcaagtccaacagattatcgtcaacaatcgcctgttgaacccgtttcattaaatggattaaataataaaggttgtggtaactgcacaaccgcatcccaaacgattcgtcggtcttcatcagatgacggatgtatgcccgcgtgtagttacggcaggtgtaacagtcacactggtcatccaacggtgtgaagtcacgggcatacttggcatttttaacaaccagtcggccatgggacgtcatcaccgttccgttacgggcaattcgagtcggcagaacacaatcgaacatgtcaatgccccgaatcacaccgtcaatcagtgaatcggttgctccaacacccatcagataacgcggcttattctcaggtaaaagtggactggtggattccagaatacgattcatttcctgtttggattctcctactgacaatccgccaatcgagtaacccggaaaatccaggctgaccaaatcgcgggcggattgtttgcgaagatcttcaaaaccggccccttggacaatcccaaacaacccctgccagtcaggatttcggtgagctttcagtccacgttccgcccatcgactggttcgctcaactgactttttgacgtaatcatacgactcaaaaaatggtggacattcatcaaggctcatcatgatatcaggacccaaatcattttcaatctgaatcgccttttcgggagacagaaacatttttgaaccattaatttcatttttgaaggtcacgccttcttcggtaatatcacgattcttagccagcgaaaagacttgaaaaccaccggaatctgtcaaaattcccttgtgccaattcatgaatttgtgcagaccgccggcctctttgacgatgtcttctccgggtctcagccataaatgataggtgttcgccaaaataattgtcgaccccatttgctccaattcttccggagccagagttttcacagttgcctgagtcccaaccggcataaacatcggcgttttgaaagttccgtgaagcgtggtgatttctcccaggcgggcgccggtgtgcttctcctttttaatcaagcgataacttatcgctggttgcatataataatcctcctagtgaatgtacattgcatcgccaaaactaaagaagcgatatttctcgtcaattgcatgctgataagcgttcaggatgttttcccgtccggtaaacgatgccaccagcatcaccaaagttgatttaggcaaatggaaattggtgataaatgaatcaaccacccgccactggtatcccggtttgataaaaatatccgtccagccggagtcggggcgaatttgaccgtcaaacttggtcccgaccgtttccagcgttcgaattgacgtggttccggttgccacaatttttccgccattatcccggacagaattcaacgtggccgctgcctggtctgacaaacggtaaaattcactgtgcattttgtgatcttcaatattttcctcatcaaccggtcgaaatgtccccaagccgacatgaagggtcagataaactaaatgaacgcccttatcttcgacttttttaagtaaatctttggtccagtgtaaaccagccgtgggagcggcagccgagcccatttctttggcgtaaaccgtttgatagcgatcaggatcatctaatttttctttgatgtacggcggtaagggtgtctcaccgagccgctccagaatttcgataaaaatgccatcgtatttaaattcgatttcgcggcccccgtgatccaattccttggtcacaacagctttaagttggccatcaccaaaattgataaccgtgccgaccttggcttttttggctggcttcatcaaagtttcccagcggtcgccctcaatattatgaagcagcaacacttccatgtggccgccggtatcggctttgacaccgtatattcgagcgggcatgacctttgagtcattcatcaccagggcatccccgggattcaaataatcaatgatgttgtaaaaatgacggtcctgcatctcaccggtttctttatccaacaccagcagtcgtgattcatcgcgatctttaatcggcgtttgggcaatcaattcatgtggcagatcataatcaaagtcttcaagggtgtaatttgttttcaagattctaattcctttcgtcctgaggtggcattggataactcaaatgagcgtatcccttgggagtcacaattcttcctctggctgtccgtttgattaaaccgatctggagcagataaggctcatacatctcggcaatcgtgtcggtttcttcgccaatattggcggccagggtgtttaagccaactggtccaccatcataatacttgatcattgtcgtcaatagtttcaggtcagtggcatccaaccctaaatcgtcgacttttaactttgccaacgcgtatctgacaattgccaaatcgacttggtctttgtcggatacctgagcaaaatctcgaacccgttttaacaagcgattggcgactcgaggtgttcctcgggaccgcaaagcaatctcatgggcaccggagtcctcaatatcaatttgaaaaatatccgcagttcggcgaacaatatcctccaaatccgtcgcattgtaataattcatgtgctctacaattccaaaccgatcacgcagtggtgccgacagcattcctgcttgggtggtggcaccaatcagagtgaatggcggcagtggaaaatgaattgggtgggcgcctgaaccctgcccaacgataatatcgacaaaaaagtcctccatggctgaataaagcatttcttcaaccaccttgggcagtcgatgaatttcgtcgatgaacaagacatcgccaggctgaagttcattgagtaaagacaacagatccccaggcttatcaatggcaggaccgctggtcgttctaatattgacgcccatttcattggcaatcaccatcgccaaagttgtttttccaagcccaggaggtccgtaaagcagcacgtggtctaatgactcctcacgttgcttagcagccttgatatagactcttaactcgtttttaacatcatcctgcccaatgtactcacttaaaactcggggacgaagcgatttttcaatgctgttctcatcggcatccacattctctggtgaaaccaatcgatcatctttttcattggccaatggatcatctcctcatccctaatgcattaacagtttcaatcctaaacttaagtattcatcggttgacaaatcagcttgcttaactaaatccggctcgatggcggcaatctgtttggcaccataacccagcgcctccaatgccgataacgcatcggccaattcaggagacttttcgggactgccaagcggttgggccagcgaagcaccattagttgcaatgtcgtcgagctttccctgcatgtccaaaataatctggcgggcagttttcttaccaactccggggaacttcgtcaaaaacttgacgtcttcattattaattgcggtgatcaatccatcccggtcgttgccggccaaaattgccaaagcacttttggggccaatcccggaaaccgaaatcaacttttcaaagatctgcttgtcttcaatggtcgcaaagccaaacagcaagatagccgtatcgctcactgactgataaatatagactctgatgacttttttctcatcaacattaaaacggtacgggtctgcggtattgatcaaataaccaacgccgcccactaataaaacgatgtgggtgggtgtgatatcaacaaccgtcccttccaaaaattcaaacatcaacttctcctcttcactaaaacgtatgtttgccaataaattgtaccatatctcactcggtactgggcaacaatctagatgatttcttggtctgtatgatgggggtcttgaatccgtttgaacattttttcaatgtcctcgttagtaaatttcaccagaaccggccggccatgggggcagttatatggattctcacactccggcagccgcttcagtaaggcctttgcctggagctcatcaagatgatggttcgccttaatggctcgcttacagctcatcatgatagccgttttttcgcggaaagcggccacggaaattttatgatcggataaaatccagtcaatcatttctttaatggtgtcttcttcctgcccggctttaaaccacattgggtgctcacggacgatgaaactgttctgtccaaacggctccaaatgaattccaagtttgtccagcaggtccaaacggtcgctaatcatcaagaaatccgaggttgagtaatcgagcacaattggcaccaataatttctgttggtcatcggaaacttcgccaatttgcttacggtaaaactcatagttaatccgttcttgagctgcgtgttgatccaccagatacatattatcagctgtttcagccaccagataggtgccatgaatttgaccaatatagtcaaggtgcggaaaaccagtttcaactaccagttcagactgctcaggcttggtacttgactggtgattgtcaatcgtttttggctgggttccttcaaatgcaggcaagccactcggctcatttttaagaaagtcatcaaattgagcaacttgtgagctggcaaggtcgtctctggttttgaccaccaccggcgttacttcaggttgggaaattgaaggcgtcgttggtgtgtcgacggcaaacagcggtggattcgtttgagcctgggtggcagtcgaaacatcaaactgtcttggtgcagcttgaaccggctgtttgaaatccctggttgcatctggaatcagctgcttgtctcttagcatgtcgtaaatggcattggcaattaatttaccaatcatcggttcgtcactaatccgaacttcctgcttggttggatgaacattgacatcgatcaaagcgggatcggcgtcaattttgattacggcaatcggaaatcgtccgatcattaatttggaaccatagcccgcaatcaccgctttggttaacggaaagttgcgaataaagcgtccgtttaaaatcagtgaaatatagtttcgacttgaacgggtcaattccggtaaactcacatacccactgactttgatgtccaaatcatttcccttaattgccgccatctttgaaaccgtcttgacaccataaattgcgcccaaaacctggcgtaaatcaccacgtccggacgttcttaacaattcacggccgttactgataaatgaaaacgcaatctcaggatgactcaatgccaagcggttgacaatgtctgatatttttgaaagctctgtattcggtgagcttaaatacttcaaacgagccggcgtgttatagaacagtgatgccacttcaacagtggtccctttccgtgattcagaagccttttgagtgacaagcttgccgcctttgtattcaacttccgttccaatcgagccggttgacgttttcatccgaacgttagcgacggaactgatactggggagtgcctcgccacggaacccgagtgtccgaacgcggaacaaatcccgttgctcagaaattttgctggtggcatgtcgtaaaaaggccgtctgaacttgagagctgtcaattccgttgccgtcatcgacaactttgatcaacttcaagcccgaattttcaacggtgacatcgatttccgaactcttggcatctattgaattttcaactaattccttaaccactgatgccggtcgttcaacaacttcaccggcggcaatctggttggaaaggattgttggtagcttatgaatttcattcaaatcaatcaccttagtctccgtttatcttctgctgccatttgtaaacttgattcatcacttgcatgggagtctttcccatcaagtctaatttctttaattgtgacacaacttcggcttgtttatcatcaatttgctcaagtggaaataaagacgtctgctgctcaggcgcctgctgaggggcctgttttggtgccgaagctgtttgatgctctttgtcggcctgttgctcaaggttggttaaaatgtcgttagcgcgatgtaataacccttctggcaggcctgccaatttagccacatggattccgtatgatttatcagcagggcccggctgaatcttatgcaaaaaaaccagttcgccattggattcggtcgcgccgacatggacattttgcagtcgtttgagagattcatccaaaacagttaattcatggtaatgagttgaaaacagggttttagcaccaatgttgttatgaacatattcaataattgcttgagccaacgccatcccatcgtaggttgcagtcccccgaccaatttcatcgaacaaaatcaaactgttgggagtggcattctcaatggcatcgttggcttctttcatttcgaccatgaacgtactttggccggagatcaaatcatcagcggccccaattctggtgaaaattttgtcaaacaccggcagtttggcctgtttggcgggcacaaaacaccccatctgattcatgatgacgcatagtgccatttgacgcatataggtacttttaccagacatattgggaccggttatcagtaggatgctggtatcttcgcccagattaacgtcatttgggacgtattgctggtggcccaaaaccttttcgacaactgggtggcgaccatctttgacttcaaccacgtgatgcgtcgtaagcgttggtcgaacaaatcggtactcctcgctgacggcggcaaagctctgtaagacatcgattgacgctacggcatctgctaaatcctgaattcgtttgatggatttcttaatgtcgtcacggatcttaacgaatagcttgtattccaaagttttactttgttcctgggcctctaaaatcagcgcttctttttccttcagctccggcgtcgagaatcgctcggcgttggccaaagtttgtttgcgctgataacggtttgctggaatcttgtccaagttgaccttggtgacttcaatatagtaaccaaaaacgtgattaaaaccaacttttaagttattaatgccggtaattttacgttctttggcttccaattcagccaaccatttttgaccgttattggtagcgtcccggtaagtgtccagctgctgattgtagccatccttaatcacaccaccatcggtaactgaaattggcggttcctcgacgatcgcagaatcaatttcgtcaacgacatcatccaaaggaaccaggtttttgagcatagcctcaaaactcttgtcggcgatttgctccaaaatatatttaatcttcggaacctgcttgagcgaagccttgagttgaatcaaatcacggccattgacactgccgaaggaaatccgacctgccaatcgttccagatcgtaaaccttgattaactcgtcttggagttgatttcgttcgaaatagtgatccagtaacacggcaactgcatcatggcgttgattaatcagtttgcggttcaccaaaggccgctcaatccattgtttgagttttcggccgcccatcgcagttttggtttggtcaagcagccacaataaagtgccggcttttttacctgtgcgaatattgcggattaattccaaattgtattgagaattgtggtcgagttccaaaaaatctgagggttcataaatcactgcccgctttaaatgctgcaggcttcttttttgggttgcttggatataatccaacaggagtttgacgacccgtttcatcaagtcgtcatcaacgtcctggcttaagtaactgactgaggcattgaccggcagaaccgattgatgggaaatcaaaatccccaatttttgaatcgtatcttgaattgactccggtaaatcagtatcaacgacaatttccttagtctgcaaagaaaccaattcgttaacaaattcagcctgcgtggttaatttggcaactttaagttcaccggtggaaagatcggcgtatgagaaagcgaactcatgattcttttgatcatccaccaccgcagtcagatagttattggacttggcgttttcactgccaacatccacctgcgtccccggtgtcaccaattgaatgacttctcgtttgaccattcccttagccaatcgtggatcttccatttgttcacagattgcgactttgtatccctggtcgactagaatatcaatataattttgcaccgctttgtggggcacaccacacattggaaccggattggccgcattccggctccggttcgtcaaagttaattccaataactgtgaacccttgatggcatcctcattgaacatctcgtagaaatcaccgagacggtagaacaaaaaagcatccggatactggtccttgattttttgatattgcaccatcattggagttaattctttttttgccaactgaaagtccccttaaattctcactgaattcgatttcagtatcgtctaaactattataaaacacaattaaatttgatcatcagtcatcgacacggtttcaatatgggtcgcgtgaccggtcttatcgtcaatatcgacgaagcagccggaaatgattccgcgaccggtttccataactttaaatcgggctggtcgctgatctaagaagcgttgaatcacactgtccggctgcatgcccaacatgccgtcagccggcccggtcatcccggcatcggttaaaaaggccgtcttgccttggagaatccgtgcgtcattggtttgaacatgggtatgtgtccccaccaccgctgaaattcggccgtccaaataacgggcgattgctaatttttcgctggtggcttcggcatgaaaatccataaaaatgcaattggtcgtctttcgaatctcttcaaccagttcgtcagccagctcgaatggatcgtcaaggttgtccatgaagacgcgcccttgaaaattcaggacagccagctgtttgccgttgacattgaccatggtatacccttttccgggtgttgttcgtttgggaaaattgtacggccgaatcagccgtttagtatcatcgatgaagtcgagaatttcattattgctccaagcatggtttccaagcgtgaccacatccacaccatcactcatcaattgcttatagatactcaaagtgatgccgcgacccattgaagttgcattttcgccgttcactattgtgacctggggtttcagatcctgcttgagtcttggcagataattgccaatcattgaaacacccttgtcgccaaccacgtcaccgataaaaagaattcgcatgtatttttcctcgatactttctgaataatataaaataattctaacatttataaaagaaaaaagaccagagactctgatcttttatcttgcgtattcgactgaacgaacttccctgatcaccgttactttaatgtgtccaggatacttcatctcagtttcaatcttttgtttgatctgacgggcaagcacaattgcctgtgtgtccgttatatcttcgggctttgcaatcacacggatctctcgacctgcttgaattgcgtaactcttttgtacttcgttaaagctgtcagtgatcttctcaagactatcaagtcgatgaacaaagctttcaagtgattcactgtgtgcgcctggacgcgaaatcgcgatcttttccgcaacagcaaccaactcagaaataattgtttctggattgtggccttcttcataacctttgatagcatcaatgacaacgggactctcatgatacttcttggcgaaatcaacaccaacctgtacatgtgatccctcaacaccattattggcagctttaccgatatcgtgtaataatcctgcgcgtttagctaaagtaacatcctcacctaattctgctgcaaaagcacccgccaacttggcgacctcaattgaatgactcagcaagttctgcccatgatcaatcttaaagttgagttgtccaactaatttgatcatatctgggctcattgaatgaatcccaaggtcgaatagcgtctcttccccaatttcttggatacgctcgtcaagctctttacggctcttttcgaccatttcttcaattcgtgccggatgaatccgaccgtccttgattaacttttcaagtgtcattttggcaacttctctccgaatcggatcaaagccgctcagcacaactgcttgtggagtatcgtcaatgattaaatcaatgccggtcaacgtttcgaaagtccgaatgttacggccttcacggccaataattcgtcccttcatgtcttcgttaggaagactaacaacggaaacggttgtctctgagacaacgtccgctgaactctgttgaatagcttcaattatcagatttttggcattttcatcagcttctgtttgggcttggtaataactttcttttaccattcgagccttttcgtcagccaacttttcgctagtttctttcaaaatcaggtcccgggcttcttcttgcgttaaagcagcaactttctcaacttcggcctggcgttttgcgataagtgagtttgcttcttcttgttgtgtaactaaattctgttgttcacgattaatcttctgctcttttcggttcaacgaactttcacgacgttcgaaagccgtgtctttacgatcaagagcctcttctcgctgcagcaaacgatcctcttgtttttgaatctccgcacgccgcgtcttcagttctttttcaaccgatgaacggtaacggtggttcttctcctgagctgatagagttgcttctttcacaaccgtctcagccttcttctgggcctcggtcaaaatgttcttagccgacccattggcagagtcaagatctttctcatggatcttcttttgtgcagacttgccgattacaaagcttaaaataccaacaaaaccaacaacaattatagcgatgattgcgaggattatcccagccatggtcatggcttttcacctccaaatcatcaaaaaatgattatttgtaaaccaattagatgttatttgattattgacacaattcttattttaatgtttgttaacactagtgtcaatcatctttacgttgcggtttttggtatttgtatataacaagatttttgagtgaccatattttcttttaaaatgtttcacaaaagcccgctgtgccttgattaactcacaaaaaatgggcagctcctctgagtgcccattaacgaaatctatttgcatttggtagtgccaattacttgccaatatcaagatcgatgctatcagttttggtttcttttgaagaaccggttgccgattcctttttggaatcctttttgtcggcttttttatcggtcttcttatcggaactggctttgtcatcagaggtgtccgagtcagtttcatcaggaatgtcgtaggcagccctgactttcttcatcacctcgtcatacatatcttgatgttcttcaagataagtcttggcattctcacggccttgaccaattctttcttcaccatatgaataccatgagccggacttgttaataatgtctttttcaacagccatatcaaccaattcgccagattgagaaatacccttgccatacatgatatcaacttcagcacgtttaaatggcggtgcaaccttattcttaacgactttgatgcggacacggttaccaatgatgttggtaccgtccttaatctgttcagcccgacggatttcgagtcgaattgtcgcataaaacttcaaggcacgaccaccgggggtagtctccggattaccaaacatcacaccaactttttcacgaatctgattaatgaaaatggcaatcgtcttggtcttactgatcgttccagaaagtttccggagggcctgcgacatcagtcgagcctgcagaccaacgtgggcatcccccatttctccttcaatttcagctcgggggaccaatgcagcaactgaatcaatgacgacgatatcaattgccccactggtaaccaatgcgtcagtaatctgaagaccctgttcaccagtatctggttgtgaaagtaacagatcgtcaatattcacgcccaagtgggttgcataaaccggatccagggcgttttcggcatcaatgtaggcagccgtgccgccgcgcttttgaacttcggcaaccgcatgaagcgccacggtggtcttacctgaactttcaggtccataaatttcaacgattctgccccgtgggtatccccccactcccagtgcatcatcaagcgctaatgaaccagatggaattgtggaaatttgagtatcggctttgtcgcccattctcatgatggatcccttaccaaattctttttcaatattctttaaggctttatctaaagctacttttctttggtcagccattaaattcctcccactatccttaacggaaaagtttacttactaactatactaatgattatccaaaaaagcaatcaaaacgcgaacaaaagttcgattaatttaataacgatgaatcatgtccaacgccatctccaagccggccttgactgcagcagcccgaatctgatttcgatcccccgtgaaatgaaactgtttcgcataagtatgttgggtcccataggcaatgccaatccagaccgtgccagcaggatcgccttccaacgtgtccggcccggccactccggtaaaggatacgcccagatctttattcatgatgcttcgggcctgatttgccatccaaatggcagtcggttcactcacgacaccattttcatcaattacttcacttggtatctgcagtagttgttctttaacctgatttgagtatgtgacaaatcccccctcaaaaacttctgagacgccgggcacattaccgagagtgctctgaaattcaccggcagttaaactttcagccgctgtaattgtaatgtgtcgggataatagttcatttactaatgtctcttccaatgtcatcttagttgctccctctagttcataagtacgttaaatacttggtttttatctaacaagacacaaataccggaagactcattttcatgaaccctccggcagctgtgattaaaatgaatctgaaaatactgagcgattttttacaaagtaatcaattcctgagtaaatcgtgaagaataggcaaatgtataacagaattaagcccattggaatgttgactgcatcaaataagacgttgttcaagaacagtaaaatgatcgccagcatctgagtggttgtcttgatcttgcccggccaggccgcagcaatgacttggccttcgttctcgacaatgattagccgcagcccggttaccgccaattcacggcagacaataatcgcggcgacccatgccggaacatcccccaggccaaccaaaaacagaaatgccgtcattaccagcattttatctgccaagggatcggcgaactttccaaagttggttaccaaatgatttcgtctggcaatctgaccatctaagaaatcggttagagaggcgaccacaaaaataattgtcgcccacaatctggtcatactgatcgtggttcccgcccaaacaacgctgccggaaaagattgggaccgcgaggatcaggataaagaacggaatcaggatgattcgaaatagtgttaatttattcggtaaattcatgttaaacctccagctgactaatagccattggtggtaccggtattattattcgtaccagtgctgccagttgttgcattcgtgttgccggttgtgtcagtaccagtcgttgaggacgttccagtggtgccactcgtcccggttgtgctattggtagttgaggcacccgtcgtggcactacttgaactagagctggttgaagcagatgaacttgacttgccaaactgcaatgtgacaactctcacctgagttgaaccgccatttaacggtgccgccaacgtcaacttcttgccgcccacggtaatccgggtcgcttcagcgttgccagtattaatcgtaacggtattggtcgagcttggaagcgagattgtatgtgaattaccactggttaatgaagcttgccataaagaagtgccatctgcagaaaccgacgtccaggcactcccggaaccggttacggaaatcttcagtggcgttgtaccggaagttccggtgactcggtaagtcagattgctgccagaagcagtaaccttcttaaaggtaatccccttggccttcttagtcgtcttggctttcttcgaactggaagccttggaactggatgatttgtcgccggaaacggaaactttgctggtctcaatttgcgttttggcagtgtttcgggtacttctagccgcagccacccaaatagcaatcaaaatgattaaaacgacgacggacaccgaaataatcggaatatagcgccgcagtttatcattgcgttcttcaacctttcgttgagcagatctcgtctcagggttgtcatcattgacccgatccacatattccgggtcttcggtatcgggcaatttagtatcaaactggcttagcagctcacttccgtccagaccaaccgaatcggcatactgcttaacaaatgctcgaacataaaaatcacccggcaaggcgtcaaaatcattatcttcgatcgcaattagatagcgtttctgaatcttagtgttcttttgtaaatcatccagcgtgtaacctttggccactcgtgcgtcatgtagttttttcccaattgttaaattatctttttcgtcgctcatactcattctccattgaattttttgtattctccactaagtatatcataaggaaagccttgattattttaagtaattcataaactataatttatcaactatccctttggctggtcggaattttgaatcatcacttcttgaactgttgcttggtccaaaaaactgtgggccgcctcaaaaacatcctccaaggttaatgatttgagaatctcaacctcatcatatattgtaacaggttcaccgataaatccgtcaaactggccactgatcgcttcttcagaatccatcatttcgatgtagttgccgaataactcgtttttttgcaactgaaattcggtttggaggtgaccaatcttggttggaatatctgcaatgatttgtttgagccggttaatgagttccaatggcttatcagtatcgccgttaatcacggcaaaatgaaagccgcgttcattttcaaattcccatgaaaacgtgtcatcaatgatttcatcatgatacagtttatcatattccacggagttttcactcaaaaacagatcaaacatcacagagatggcgatttcgtactttagtccatcccggcctgttgggacttggtcgcttccccgtagccccagcgttattttaggcctggaaacatccattttcgtgtgaagaacggtttctttggatgcctcggggagcgtcagtcggcgttgcaggctaatgggtgccggtgtcgattttcgccgttgattatcctcaatccagttcataacttcgctgggatcgagtttgccggtgataaacagactcatattttccggccggtaaaaggttcgataagccaactcaacatcttccagggtaatcttatcaaccgtctgaatgtcgccggcaatatcgtttgccaacaccgagtttggatacaaactggcaatcgttttaaagtacgcctgattgtccggatcattttgatacatattgatttcttgatcaataattcccttttcacgttggactttagcttgggtaaaatatggaatctggacaaaatccaacaaaatatccaaattttctttcacggattcggcagttgagaagaggtaattcgtcttggtaaaacttgtgaaggcattcgaacgcgctccggttttattgaacagctcaaaaacgtcgtaatcctttttatcgaacatcttatgctccaaaaaatgggcaattcctgcaggttgaacaactttttcgccattgagcatgaactgactgtcaatggagccataattcacccccaaaacagcggtcgtcttattaaaccctgctttgggttggagataaacggtcaacccatttgagagggtctgaacaaataatttttcattgtagtttggatagtcaatcaattccattatgcatcccccctgctgttcaactgataaatggctcgtaaagtcaaccgcttggcaacttgggcaatctgcgaacgcgtcacagaagcgacctgttgctcccatttggtatcactcaaactaaagcccatcatctgctggagatactgcttctcgattaatgatccgaggtgatcggcttctgaacgatgttggttaatcaatgcctgtttgacaccgtcgagcaattcatcggaatattgcccgtcgctggtctgctgcaattgatcggcgaccatctgaataacgcgatcttcatccttaaaatcaatccccgcctgaacggttaccattccgactaatgaattatagccactatgaatgtcgtaggccaaactgttcttttcacgaacgtttgtaaatagcaacgatctgcttgacccaccaaataactgattaaaaatgacggcagcaaagtagtcgtcgtccccaaaatagattggtagttcgtaagccatgctgagaactgactgagaaccggcaatcactttggttccttgttggaccttcgatattggtgccggcacaactcttaattgatagtcttccggcattcgatcagtaaatgaggtaaattctttaaatcccgttactagttggtcgtcaactaaatcgccaccagccaggatggtaatcttcgctgagttaaggacccatcgataaaatgtgtacagctcttgagcagaaatttggctcatttcttgatgactgcccatcaggaagtgaccgtggtcaggatcatttgggtaatacaaacgttgaagctccaaggttgagaaaaactccttgttatcttggatcgaatccagataatgaaccatattcccttgatgaatttgaaaatatgcttggttgaactgatcgccttcaataaatggatcctcaatcatttcctttagaaatgccaatatttcactagttagctcactttttggcggtaggtacttgtcattgggaaacgtaatcgacacctgcagggtatgctgattgccataccgtaagacagtcacaccaaaactggccccgtacatttttgacagttggcgggaaaccaacaactcactgttgtattgggcagagcaattttccagcagttcagccaacagtgccaatttggcgtagttttgatgttgggccggaaaggtgaaattcatcaccaatttattatttttgaattttgtggtgggaattgtcgtcaagctaatcccttttgcaatctcgtatttcactgagtttcctcctcaattagtcacaaattttatcataaaataaaatcattaaaatctcaatataatctgccaataataaggaaaaatagagaattgatcggcaaaggattcgaatacaaaaatagtctgttgacaaatcacatttgccacagactactaatgatcaaaattatttagcattcttaatgagcggactgtcccgatcagttccaaaccacttcatgttgattttgtgaagctcgccgtttttggctaatcgattgagaccttgatcaattttccgcttcaagacagtatcactttttcgcatgccgacaccatattcttctttaggaaattcactgggaatcgacttaaaactggattgatttggttgatgttccaaataataaccggcataaatgctgtcaatcagcaatccctgaattcggttggcattcaaatcgatgaacgcatctgtaaaggtgtcgtataagattggctcgtggcccttgatcttatctttcagcaatttaggttggttatcaatatccatggcccctgccgacccactctggacgccggcgacttttcccttcatatctgcgaaactgttgatatgttgattctttttggaaaccaatacttgatcattaattagatagggttcgctgaaagtaatcttctttgctcgctggggattaatagagaacccattccagataagatcaatcgtgccgtttcgaagctcggtgacgttcatcgaccaatcaattggctgaaaatccactttgatgccgtattgcttaaacacggcacgggccagatcgacatcatagccgacaatcttgccgctcttggtctgaaagcccattgggacaaaactgtcatccagtccaaccacgattcttttttgcttggaaaccgtcgaccacgtatccggattttcctgtgagccttggcgactgacatagcgtaccccgcaaccggataacccaatggtcacgagtaggagactggtaatgagtaataatcgtttcaaagattttaacattttacccctcctactgaatttgtttgacctgctgaatttcatccgcaacgtttttagcaaaatccatatcatgagtgacgacgatctgggtcatttcctgcttcttaagatccaagataatttgggcaacttcatctcgtaaagcgggatcaagggccgacgttggctcatcgtaacataggatcttcggtcgcattgccagtgcccgaacgattgccacccgttgcttttggccgccggaaagctgataaggatataaattttctttgccttccaagcccaagcgactcaataattcccgcgcatattttttgacgtctgccatcgtttcttttttgaccatcgttggtgccaaagtaatgtttcccaggaccgttaagtttgggaataactgataatcttggaaaaccaccccgatgatcgtgtctttttgagtcgtgttggttggatcaaactgagtgccgttccagtaaaattccccggtattcaccgactccaaaccggtaatacaacgtaacagggtcgttttgccggcaccggaagggccaacaattgccataatttcattatctttaacggtcatcgacaagtcatcaataatggttcggctgccaaatcgtttggttaaattcttaatctctaacatcgtaatcccctcctaacgccaaacattttcacgtttctcaattaacttcaacacaatcgtacataccgcggttaatgccagatagataatcccgactaatatcagcggcaacagcgtaacatccctggccgttgcgacgtttccggctcgcagtaaatcgcccaacccgataacgtagaccaacgaggaatccttgaccaggttaatcacttcattgccaattgatggcagaacaattttgaaaacctggggaatcacgatctttcgaatcgtttgtccataactcaatcgcagcaccttggcactttcaaattggcccttgggaactgattggaaaccgcctcgaaagatttcaccgaaatatgcggtgtaattcaagatgaaagcaaacatggcagcatcgtaacgttggaacacaatgtgaacaatcggtaagccataaaagacaaaaattaattgcaatagcagtggtgtgccccgcataatccaaacgtaaaagttaagcagccaggtcagcggtttaaatttttggatgagtcctaatccgactaatgcccctaatggaattgaacaaatcaatgtccagaagaaaattgataaagtcattttggttccagataataacgccggtaaaatttcttgtatatattgaatcatttgacatccctccataaaaaaatccccttgagtacacattgactcaagaggacgatggttttcgcggttccacctcaattcgcaacagattcacacctgctgcctcgtgaagtttagtcttgttttaaaataaaaatcctcttaagccatgatgacttaagaggacgattattcgcggttccacctctgattcacctctcactcacatgaaaggcctcaatgggtttaatatgcaacatactaaacttcagcaataacgtgcttaccgctttttcctactcagcttcagaaaaatgactcccagatgtgacgattaatgctcaaatgcttaactcccaccttgataagctctctgtgatttgattcattaatcggttctgatcaacgtctttaaaaatctttaattaagttagatttataataatattaattctgcttcccgtcaaggacttttatcctttacggaaccaatgactcactttttgccagaatgaaggctgctgttcatctttgatttccatcaatggcacagattcaccgactagtcgtcgggcaatgtctcgatatccctgaccagcagggttttccgcttgaagaacaacgggttcgccgttattggaagtggtgataactgcatcatcatcaaagacaatccccaatagttcaacccctaaatgatgggtaatttcatcaacatccatcaccgaaccgtctttcatcatatgttgacgaattcggttaataatcagatgcggctgttcttgaagcggatgctgctccaagagaccaaccacccggtcagcatctcggaccgcagaaatctcaggagtcgtcacaataatggcactatcggcaccagcaattgcgttcatgaaaccctgttcaattccggcaggacaatcaattaggatgaaatcaaagtccggcttcaattcatcaacaatttcgcgaacctggtcttcatttagggccgtcttatcagtattttgagctgccggcaaaaggtaaagcaagtcatcaaaacgcttgtctttgaccagtgcttgactgagcttggctcgtccagccgcgacatcgacaatgtcgtacataatccgattgtcgagtcccaagacaacatccaagttacgcaatccaatatcaagatccaaaagaaccacttttttaccgagcatggccagtgcagtcccaatattagcagaagaagtggtcttaccgactcctcctttacctgatgttataacgtaagccttacccattgatgactcctcctatctgattgtaaaacttgggattaatctgcttaagattctcaactttaccataatccagtacatgcagatcgttcacataaatcactgtgccgctgtccatttcacgtttcatgtcagcaactatttcgaactgttcgccgatccggacttgttgtgcgttatgtacatccccaataatcatcttgtcctcaagatccggtgcgccggcttgaataattccctggacgttgcccagaacaaaaatgttaccgccgacaaacagtttgccgccctcatgaaccgtgccgagaaataagacgtcgccttggatgtgaacttcctgcccgtttctaatcacccgatcaacaatgtggacgctggactgttccaaaatccgattggattcctctttagtgatcacatctgacgtaatcttatgcactgaaaacgtcgaataatctgaaaagattttctcaagttcggaacggtcagcagctggccataaccgcattccggtataaatatcaaaagcaatggtttgcggattagttgaggccgtctgggttttcaaattatccagaagttttcgaagtgaggaaaaaatatcctttagattggcattctcatccagaatgatttcataaccatccttggtgccctttaatacagctgcatcttgcattgtctactccccttcttattgcctatgagtcctatagagtgcctcaaccggaaagtaaacaattgtcaataacaccagattgagagccagtgtaggtgccaatgtgttaactaagaactgagcaacggatgagtccgtctccccaataaagacattggccatgtatcctaggctaactaaaactgtgattcctaaaaaatacaccaaaaagccactcatgaaatttggtggcaaaatttggtaaaccaattggcataaataaacgactaatgggaaaataaacacgtataccccaagcaatccagtgtagtacatatcaaaaataaagccaatcacagcggaccaggtgtatagatgtaattttttgccattaccaaagaaggctgccaaaatcaaccagaggacggttaaatatggcaccatcgtgttgggatatttaaacaaaataccggacattgtctggctgatggaaccatcaagaaagaacgcaatgaattgaccaattacaaagtaaactgcaatgggaacttttcgtttcacttaattgtccctcccatcaatctctgattgcaactgaaacaacttcaatgtcgtttaagttggcagccggtttaatataaacttttttggcaaggccataatcgtcttgggtcacttttgaaacagtacctacgtaaatccccttgggaatgacgcccccaagcccactggttgtcacccgattgccaactgataatttggcgttcgaggtaatattccccatgataatccggttggcagccgaatcatacgaggtgataataccattaacaactttggaattatcaccaagcacttggatggcaaaccggttggagttttcggcggtgttggaaattaaaaccaccttgctgttggttttgttgacttcagcaactgtcccgatcagtccaggaccggcgatcacgggcatatccttcttaataccagaagcttgacccttattaatgatcacctgacttgcccatgatgatggtgttcgggtaatgacagctgcgttgattttttcatatccggtcaaagtgctgccgacgtttaattgacgtttcaattgtttattttctcgcgacaaaacctgatccttgacctgtgtttgggtcaattgatcaacttttgacttgagacgttggttttcctgataagtgttcaaaagattcttagttgaaacaaatccgtgatgaataccgttcattggggcggcaacaatccgatcagcaaaaccaacaatatcatttccaaattgttgtaccaacggcggtgtgctccgcttgtcccgaatggcaaccgacaacgacattaaaccaaaactgacgatcaaacagattacgacaatcacaagctttcgactggagaaaaatttttgcataattgcctccattcgttattcaataatgaatcgatataaacgattaattattgttttttcttcattacattaatgctcttcaatgattctccagtaccgatggcaacacaatcaagtggatccgatgcaatggaaaccggaacttgagtggcttccgcaatcacatcagtaatatttctgagtaatgcgccgccgcctgtcagaacaattccatgatcaataacatcggctgcaatttcaggcgatgtttcttcaagggtttccttaatcgtggcaatgatggccaacactgattcgttaattgctttgttgacgtccgttccactaatttcaactgtggttggcaaaccggttaccaaatcacggccacgaaccggaacggctttgatttctttagcttccttggcagaagcggaaccgatatcaattttaagctgttcggaagtccgttcaccaattaacaaattgtacttttgacgaacatattgagcaatcgcttcgttaagcttgtcgccagccattcgaactgaacggcttgaaacaatgccgcccaatgaaatggttgcaacgtcagtcgttccaccaccaatatcaacaaccatgctaccggttggatccatgactggaagtccagcaccgattgccgcagcgaatggttcttcaatgacataggcatctctggcaccggctacccgggtggcatcaatgacagcccgtttttccacggcagtaatgccagttggcacacaaaccatgacgtatggcttacctgatgagtgtcccaaggctttttgaatgaagtatttcatcatggcaacagtggtatcgtaatcggcaatgacaccgtctttcattggtcgaacagcttggatacttgctggtgtgcgcccaatcattgctcgcgcttctgcaccaacggcgattacctcgcctgttttagtgctcttggcaactactgaaggttcgcgaaggacaattcctttgccctcgacgtaaacgatcgtattagcggttccaagatcaattcctatgtttttttccccaaatccaaacacgttatccatcccttcgttgtctatcaacttaatttagttcgatttttatagattgatttattattgtttaacgaaacaagtatatcataacgcgtccaaaaataaataaaatcaagtgaaacgacgcccgatttaatagattatttgaaattgtgatcggcattcaacaagaactttcgagcatcggaaataaaatataacgatccggtaattaagagcatatcatccggcgccagtttccgtctcaattccctgattgcgtcttgccaatcatcaatagcggaaacattttccggttgggttttcagttgactttccaatttttctggattggctgcgagccgttttcctggtccggcgaactgggtcaagatgatcgatgcattttgaacggtggccatcttgtccaccattttatcagcctgcttgtctgccagaatgcccatcaaaatataaatgtggccctgaggaaaatcgttctgcagggtatcgacaatcaggctaactgccgagatattatgcgcaccatccaaaacgatggtcggtttggccgaaattttttcaaaccggcccgcccaccgtgttgctgcaattcccttttgaatgtttctgacatccacagagcgctttgtgagctggtggtagtcaatgtatgcctggatcgccaacgcagcgttgtgagtctgataatcaccaattaaggctgtttttaaatcatgcaattgaaagtcggcggaactaaagtcaaattgttgaacccaattgtgctcaccgcgatcattgaccttaaaattctgccccagaatctgaatcgggctttgcttttgctcagcaagatttacgatcaccttgagcggttcggggtcaactccgccgacgactacgggaacgcccggcttaataatccctgctttttggaaagcaattttgggcaaagtatcccctaaaatgtgcatgtggtcccagccaatcgacgtaataaccgagactttggggataatgacattggttgaatcatacagcccaccaaggccaacttcgatcaaaacaatatcagcgtgtccttcagcaaagtacttgaacatcatagctgtcacaatttcaaattcggttgggccgccttccggcaactcggcgtcaagtttggcaatcgtcggataaatttcctgagtgagtcttagaatttcatcgtcggaaatgccgacaccgtcaacactgattcgctcattaaatttaatcaaaaatggtgaggtgaagctgccgacggttttgccttccgcttgaaacaagttccgtaaaaatgccagggttgatcccttgccattagtgccggcaatgtggatggcattgacatgtttgtccggggcacccaattcgtctaagaatcgccgcatccgttttaaggttggaattttcttgaatttggtccgtccatgaatgaaagccaaggcttcatcatatgtgttaatcattattttctccttaaaaaacgtgggcaaaaatgcggcttatagcctggcatgtgccaggaaacagcatttagtcccacgtttttaaaaattaaagtcagttaaatcactttacatctcactggaaatttgttggagccggtctttggctgcatccaattttgattggtaatcagcctgcttggccttctcttcagcaaccactgcatccggcgcgttctccacaaaccgtttgttagccagtttcttatctgaacgggccacttcggcttcaaacttatcaacatctttttgaacccgggcctgctcatccttcaagtcaaccaattcagccaatggaacaaagacagtcgcatccgtaatcaccgcagacattgacagctttggcgcttcaatatctttgccaatttgcaattcctgggtgtggcagaaccggtcaatgtagtcgcggttggattcaaagattgatttgagggtctgattgtcagtttgaattaacatatcaattggtgaggacagcggtgcgttggcttcatttcgaatattccgcactgctgtaatcaaatcaatcagtgactgcatctgatgctcagaagttggatcgtcaaattctttgtggtccactgggtagtcggcggttaccagtgacttgccaacgtgtggcatcatctgccaaatatattcggtcacaaatggcatgatcggctgcagtaagcgcagggtttgatccaaaacgtaagccaaaatgttttgggtgttcttcttcaacttctcatcgtcactgttgagagcttccttactcatttcgatgtaccagtcacagaaatcattccagatgaagtcatacaaataacggtcggcttcaccaaaattgtacttctcgaataagtctgaaacgtggttcacagtagcgttcagtcgacttaaaatccatttgtcagataattgccactcggacttgtcgggtaattccggcttgtcaatcccatcaaggttcataataacgtaacgactggcattccaaatcttgttaatgaaattccaggcagagtccattttgtcataactgaacttcagatcttggccaggcgtcccaccgattgacaggaaccagcgaagggcatcggcaccgtatttatcaatgacatccatcggatcaataccgtttccaagagatttggacatcttgcgtccctgagaatcacggattaaaccatgaagtaagacatctttaaagggtcgttcatgagtgaattccaagctttggaaaatcattctggaaacccagaagaagatgatatcgtacccggtcaccaaggtgtcggttgggaaatagcgcttcatgtcttctgtttcatcgggccagcccatggttgaaaatggccacagggcagacgagaaccaggtatccaaaacatctggatcctgctcccagttttcggcgtctttaggcgcttccatcccaacgtaggtctcaccggtctgcttgttgtaccaagcaggaatttgatgaccccaccaaagttgacgggaaataacccagtcgtgaacgttttccatccactgttcaaaggttccttcaaaacggtctgggaaaaagttgaccttgtcgttggtatcctggttcttaatggcctgttcagccagcggcttcatcttaacgaaccactgagttgacaaacgggcttcaacttgaaccccagtccgttcagaatgtccaactgaatggacaattgggtcgattgagagcatcaagccttcatcctgcaaatccttgaccatagcttttctggcttcaaaacgatccatgcctttatacttaccggcattttcgttcattgaagcatcttcgttcatcgtattaatgcgttgtaagttgtgacgattaccaaccttaaagtcatttggatcatgggctggggtgatctttaccatccctgtcccaaagtcagggtcaacgtactgatcggctataatcggcacttcacgattaatcaatggaacgcggactttcttgccaacgatatccttataacgttcatcagaaggattaacggcaaccgcggtatcacccatcatcgtttcgggacgggtggtcgcaatttcgatgtaatctttgccgttgaaagtcgtcccgtcggtaaatgggtatttaacatggtaaaaggcacctttatcgtccttatggatcacttcaatgtctgacaaggcagttcttgcttgcggatcccagttgataatgtattcaccgcggtagatcaggcctttattgtaaagcgtaacaaagaccttacgaacagctttggacaatcctttatccaaggtgaatcgctcacgactgtagtccagggaaagacctaatttggcccactgttccttgatggttcgggcaaaatcatctttccattcccagaccttttcaacaaacttttctcggcccaaatcgtaccgggaaataccctgtttacgcagcttggcttcaactttagcttgggtagcgatcccggcatggtccattcctgggagccataaagtatcgtatccctgcattcgtttgcggcgaataatcatgtcttgaagggttgtatcccaggcatggcccaaatgcagctttccggtaacatttggcggcggcaacacaattgaaaatggtttggcctttttatccccactcggtgtaaataccccttcatcaagccattcatcatatctgcccttttcaacggcagttggatcatacttcgttgacatttcgtgcaatttgtctgacataacgtcactccttccaaaattcaaatcgtttttatgtaataaaaaaacaccccatcctgtaaattaggacgaagtgttcgcggtaccacctaaattgggctgaaaagccccacttaatatcataataacggtctgataataccgactcatcttcaattgaagataagcagctcacaagctaccttcactcaacgcccggtaaaaatctcacagcaatgattttctttctgaaaccgaaacgttggctactctcttgctcaacactttaatttaattttaatcttaactaaatatctgctaatcgtcaatacgctgagcaacttttttcaaagcatttagtgcatcatcgtaatcaggctcattcccaatttccggaacaatctgacggtaaataatcttaccggtggcgtcaataataaaaattgttcgcgccaacgcaccaaagtttggcagataaagtttcattgcgtatcccagcgagaggttttcgtcggacagcatctgcaaattggcaaccccttgagcagcgcaccaattcttctgctgttcaatcgtattgttggaaaccgttaagaactggacatcaggaaacttgtcggcttcctggttaaacttgcgggtttcaactgaacaaaccggggtatcaatatccggaaccgttgacagcagggtaattctgccaataatgtcagcagttttcaccttattgccatctgcatcctcaagtttaaactttggcagttgttcaccgacttcgggtggattgccaaacatactctcttctttaccattgatcgtgattttcataaaagcactcccttggtctaacgactttatacataatgtagcctaaacaaacggaatacgcaagtccccgatcattaaagcagctcagcgaagacgtcctggttttggtttaggaattcttcgccaggtttaatatcggtaatttcaatgttgtcgattgcttttttcatcaacccttcaacatcgatatactgttcaaacttacgtgacttggccaaatcaggccgagtctttggtgccggcggtgtaaaaatcgtacaacagtcctcaaatggcagaattgacaggtcgtaagtcttgatctgcttggaaatcttaataatctccgttttgtccattgagaccagcggccgaagaaccggcatcgtggtgacgtcgttaattgccatcatactctctaaagtctgtgaggcaacttgtcccagtgcttcgccggtaaagacgccggtacaatgacgattttgagtaatttgggcagcaatccgcagcatcattctccgctggatggtcatcaaataaccttcagggaccttttccttgatggtttcttgaatctcggtgaacggtacctgaatgaactgaatattacccgagtacttgcccaacactgaggttaactgtttggccttattcagggcttgctcgccggtatatggcggactgtaaaagtgaatcatatcaattttgacaccacgtttcattgccaaatacgtggcaaccggcgaatcaattccaccagacagcatcattgtggcccgaccaccggtaccaaccggcaacccgccggcaccatgaatcttttctgatgagagaaaggcaccattcattcgaatttctactcgaatggaaatatcggggtgtttgacatcaaccgtgattccgggaacattttcgagaatataatcgcctaactggttgttgatctgattggtatcgtattcaaaatgtttatcctgacgtcgggtgttgattttgaacgtcgctccgtcatgatactgttctttcaccatttcaagagcggtctgcttgatgattgccatatccttttcaagccgaacagaaggatagaaattttcgatcccaaaaacacccttcaggctttcgatcacctgctggtcatcctcaccgtttagagccacatgaagacgatcccgttgcggcttgacctcaagcttgggaaatgggtggagaacagcccgcacattcttgccaagctgcttaataaagtcttttttatttttgccctttgtggacagttcgccataacgaaccataatttctgtatagtgcatagttactcctaacttaatttgtcaaattcttcatacaactggtcaaatacttttacgaattgtttggcttcatcaagtgtgttgtgatctccaagtgaaattcgaacggcactggtagcaatatcatcgggaacctgcatggcattcaacgtgccggattcagtatgatcctttgatgagcaggcgctggttgttgaaatgtaaatcccctgcttttcaaaagcatgaacgatggtttctccgcgaacccccttgattgcaaaacaaagaatatgcggggcaaaagtatcatcattcttggaaaaaatggtgactttatcaaactgactgatgtgatccataattaactgcttaatctggcgctcagtatcaattgcactaggttctttttcaagcaccaatcggatcgctttggccatggcagcaattcccggcagattttcagtaccggaacgttgattcttttcctggccgccaccgttcattaacggtgcaattcgacggccacggcgaccatatataaagccggttccccgtggggcatggaatttatgcccagaaaatgctgcaaagtcagttcggtcattgaaaatctgatcctgaattcccttgccgaggccctgaacagcatcgacgtgaaaatgaattttcgggtagttcttcagcagttctcccgcttctttgatcggctgaatcgtcccaatttcattgttgaccgccataatcgataccagcgttgtatccggacgaattgccgctttcaaatcagcaatcgagatccgcccctcatcatcaaccggtaaataggtcacatcatatccgagctgtttaagttgctcaaaagagttgcgcactgctgcatgctcaactgaggtggtgatcagatgcttcccaaattcacgtttttcaattgcagtccctttgatgacccaattgtcaccctcagttccgccactcgtaaagtagatttcatctgggtgaacgtttaacaaatcagcaatctgttttctagactgttccaacagattaaacgcctgttcaccaaagttgtgtaagctcgacgggtttccccaaatctgctcactcactttgttataagtgtcaagaacttctggtaagacttttgtggtggcactattgtcaaaataaatcatttgaaaccttcttctctaaatttattggttcgactccaacaaatataactcccacgatgatacacccaaactgtgagtctcacaagcattgtcgctgggcaatcaatgatggaaaacaaaaggcgaagctgttggtaaacattcagcttcgtctcatacgtcatattatgattcatcttcatcggttttttctgtctttaaatgtttcttagcattgaaataatcatctttgatcttggcaaacatccccgacgattgtttttccaatgctttggaaataatattcaaactctgctcataatcatatttttggtcaaaatacatctgggccgttttgctggccgccgcaatttcagagttgctgccaataaaccgattggcatactgcattgtctgttcggccaaagtggcatcatcaatcaactggttggtcttttcatccaaagtgtccatatccgattgaataattgttaactgtttggaaatgtcatcgacatcaatctgcggctgattcatggcatcgtccaggtgattgatttctctaatgactgccgtaaaagcatcttgataatcgttggatagtccaggaagattgtgattgtcaattcgccgtttggtattgcgcattgccaaatcaaatttggccaatgcatttctggctgcctgctcttgctctggcaacttaactgttgcggagaacaaatccttttgttcagactcgatctgacccagctctttgatcatgtgagtttggtcggcgtcaatcgttgaataaacagccgtcccattttgcatggcgttgacttcatcctggtacttcttttcaatggtggcaatttgttgatcaaattgatgattattctcaatttcttgatggttcaaaatatagcttttattcagcgtttcaagccgcagctgcaagtcgctgttctgtttacggacatgttcgatatattggccgataatcttagtatttttctcgaccttggggcgggcttggaattctttttcgattgcatcatacaatttgtcgatccggtcggcaatatcttgagtggctttttccactgaatcaacttccaaagtctttagcttattggtgttgacttttatctgatctgaaatccccttaagcgtttcatcgaacttatcgttgggaaaattatactgttttcctttgagttccttgtaaccactggtgatttcgtcaacctgctcaacaaattcctttgaaagtagttgatatagtttgggaattcgccccatataggattccaatttgtcagtcgaattgttgagatcactcaacacttcttcggcgctgttgggatccccactctttgtgagttgtgtaaattcatcgaaagttccctcaatgtccgagagcattttttccaagctgtcgatactcgggccaaatgactcgttcttgttaaggatgtcctctcgcaagcgtttgtacttcttttcgagttcttccagcgctaatttgtgctgcttgtttaaatcatatagttgagcaaggccggcctgaatttcttttaaggtggcgtcagcgtcggcgattgcctgattggcactctgccagtcactcttggtctttaaaaagttaatgcccttaccgtcttctttgactgccgcaatcccctcatcaatattgggcagcatttggttcttgtagtgctgatacttattgtataattgatcatatttcttgtgagattcaccggttaagttcattttcttagccagcgcaaactcatcatccaacggaattttatttaagtcccgtttgttctcgtaaacatcggttgccatcttgattgttcttctttggtagaaaacaaaaccaagataacccgccccaaccaacacgataattccaatcaacaaagtaagcattcgatcccatccttcagaaataaagatatataattgaacattatggtagtaaaattgcccaaaacaatttaatatgtatgaataatcaattaatgtgctctaagttgaattatatcatagtaggtccttttcaccatattatttttgaagtgaggaaaacaattatgcaaaacgttactaatttagtgaatcaacagcttgattcacttttagaaaatgaaacagatttgatttcgaacatggctaacgccactgcattgctccaagtcagcctcgaagatatcaactgggtcggcttttatcgttatgtgcccgctaacgatgaactaatcctcggccccttccagggaaatgttgcctgcatgcatatcaaaaatggtgacggtgtctgcggaacggctctcaaacaaaagcattcactacgagtcgccgacgttcatcaatttgccggccacattgcttgtgatgccaattccaattctgaattggtcgtcccactgtttaaagacggcaaagcccttggtgtcttagatattgattcgccatcactcgatcgtttttcgagtgaagacgagcaggttcttaaccagtttgccgacatcttcgtcaaacatgttgacttacagtagaaatctttatacaatggtggttgtgtaaaataacgcagcagtagacggtaagctcgtcaacatgttgttgccattcaattggttctgcaagtaactcaatcggctgcttgagcgaaagagcaaagcaacatgcacgaatactaagtctgcaacggcttattttactccaaaaaaatattggaggattacttatgtcaagatatacaggtccaagttggagaatttcacgtcgtttgggtatctctttatcaggtactggtaaagaactctcacgtcgtccttatgctcctggtgatcacggtcaagaccgtcgttcaaaactttcagaatatggtttgcaattacacgaaaagcaaaagcttcgttacatgtacggactgactgaacgtcaattcagtaacttgttcgttcgtgccggcaagatccgtgaaggtaagcatggtgttaacttcatgatcttacttgaagagcgtttggataacatggtttatcgtttaggtttggctactacccgtcgtcaagctcgtcaattagtaaaccatggccacatcactgttgatggcaaacgtgttgatattccatcatatgaagttcaacctggtcaagtaatctctgttcgtgagaagtctaaagacctccaagttatcaaggatgctgttgaagctgttgtgggtcgtccacaatacgtcagcttcgatgcagacaagcttgaaggatcattggttcgtcttccacaacgtgaagaacttgatgctgatattgatgaatcactgattgttgaatactacaacaagttgggttaatcattcagcgagcgttttgcttatgcaaaacgctttttttgtgccctcacgatcatgttataatttataggatttgatttttaaccatcacaatttgagaggaggatgagtatgcaacaaccccttgcctatcgaatgcgaccgaccaagcttgaagaaattgtcggccagcaggatttagttggcccaggtaaaataatcgaccggatggtgcgtgccaagatgctgtcgtcaatgattttatatgggccgccgggaactgggaaaaccagcattgccagcgccattgccggctcaaccaaatatgcatttcgagttctcaacgctgctaccgacaccaaaaaagatttacaggttgtcgccgaggaagccaagatgagcggcacggtcgtcctgttgctcgatgaaattcatcgactcgataaaacgaaacaagattttctattgccattacttgaaagcggctcaattattttgattggggccaccactgagaacccctacattaacatcaatccggccattcgatcgcgaacccaaatttttgaggtacatcccctcacggcaaccgatattcaaaaagccctcaaccgcgctctaaacgacaaagaaaaaggtttgggcaattatccggtgtcgattaccaaagaagcgttgaactttttggcaactgccactaatggtgatttgcgctcatcgttaaatgccttggaacttgcagtgaagtcgacacccaaaaatgatcacggaaaaatcgccgtcacccaggcaatcgtcgaggaatgccttcagcgaaaagcactcaattccgataaaaatggtgatgcccattacgatgtcatttctgcttttcaaaaatcgattcgcggctcggatacggatgcagccctgcattatgcgggcagattgattgaatcaggcgacttggtttcgattatgcggcgtctattagtgattgcctatgaagacgtcggtctcgctaatcccagtgcctgccagcgaaccgtggctgctgttgatgctgcgcgtcaactggggcttcccgaagcacgaattccacttgctaacgcaatcattgagctttgtttaagtcccaagtccaattccgcgatggccgcaattgatggtgccttaagtgacattcgatccggtaactatggtgatgtcccactgcacctcaaagatgctcattatcaaggtgccaagaaactcggccgcggggtgacctacaaatacccccacgattttcccaacgactgggttagacaacagtacctgcctgataaaattaagaatgctcagtattaccacccgaaagaaaacggtcgaattgagaccgcgtttaaagaacaatatgccaagcttagaaaatctgccggtcataaatagtattggagtgtaatgatgataattaatattttagtagcccttgctgtgttaattgccctatatattggctactacttactttcccaccttcacaaaaccatgtttaatatttcagttcaagatgatccccgcctgaaaggagctgccaaaaacggcggcatcatgttcatcattttggcagccttgggcgttctggcattaatcattcaaaatgatattctcattttagtggttcttttgtggatgactgcacatggtttggttgttgaattcgcaattctcaacgtcattaaccataaacaacggtaatagatttattcctttgtattttgccgaaagtaaagtacaattaagttaaacagatagaaatgagggtgggcataatgttacaacaacaatataaacaaattttggtcccagttgatggttcctacgaggctgaattggcttttaaaaaaggtgtagcagttgcgatccgtaataatgcatctcttcacttagtccacgttgttgatacacgtgcatttcaaaatatttcaagttttgacacatcaatggtcgaacaagtgaccgatactgcaaaggaaactttggataaatacatcgaagatgcaaaaaaagcggggctcaacgatgttgattactcaattgaatatggtgcaccaaagaccgtgattgccagagatattcctcaaaacctcaacatcgacctcatcatgattggtgcaactggtttgaatgccgtcgaacgactcttaattggttcggttaccgaatatgttaccagaactgcggtttgcgatgtcctggtcgttagaactgatttagacaataagccggcagttaatccaagcaagcacgtttaatgcttccaatttcgatcatcaaattgattaaagcaagctaaaaaggcagttaaaacaaaagtcaaatccttttgttttaactgctttttgcggctaacatgccagccatcacttaacaaaggtcggatgcccctcactttttgcaagctcgtttttgaccatctcgacgatatgggactggttgcgcttaagaattttctcagctaattccgtgttgcctcgaagttcggcaataaacatcgctgcaaactgcttcatagtggcctggacgacctgtcctttggcatacaggcattttgattccaactccgccagcacgtccaccttataaatcaaatcctgctccgtcaattcgtgtaaaatttcatgaatgagcggcagcgcccgatcatatttacccaactcggcgtacgcggcaataatatccacatagaggtcaacaatcacgatcatatcgtgcttgccggcctttttgactttagccaaaattttggcgctggaatcaatgaacccttcggcgcgatccaatttccccagcttttgataagccagaccaatgcccaaattggaccaggcttggtaaaaggtgaattcatcagcggaatactgcgtcaattgaagattgaagttgaaaatggcctcatcaatatcatcattgatatacaattcaatgaatccccgatagcaatgatacttgcccaacatatatcgggtattcaactttttgcagtcaatccgaccaatttgtctattagcgtcggcatacaaatgattccgcatatcgtcttcaatgtaagagaagactttatcaccatatcgcgtattcttggcaacatcggtaatttttaaatccagtttttggcagaggttgaccagaatgtcaacactgctgcacgtattttgattttcgatggaactgatggttgcttgggtacaaatcccttcagcgagctgaacttgggacatccccttatcttttcttgcctttttgatcaaggccccagtaatcaccattgtcatacaacgactccctatagttaacatgcttaacatacaacctgagtatcatattatatttataatcgacaatcaagaagatttttcctcatttttggcgggtaattcctcatgaaaatcacaagtgatcagatgatcattcacaacgccaaccgcttgcaaatagctgtacacagtaattaagccaatccgttgaaggcccatatttttaaaggccttcacaaacttttcggtaaatttttgatacatttttgggtctggcgctgcttttagtaaatgatccagtgaaaccccattaactggtccccaggttgcttcaaccaacattttaggattcggttgaatgactttggcgttggcaattatcgcactgacctttgcatgattacggataattcgacgatcttggcaaaaccgttcgacatctgactggtcacacttggccaaataatccagggaaaagtggtgaaagacttcatccattcccgattcaaattttaaaatcgttgaaaaagataatcctgcctgcatcgtctcaagacacagggctttgaatagtttttgcggatccttttgtacccgcccccaaattgtatcgtgataaaccaatagttcagggctggtagttgcccaagggcatcttttaaccatcactacacctcctactataaacctacgaaaaagtcacaaataattctgcaacgagttcaaaagtagaatccaacggtccttttgatagttaacccgcaatttttgaagacgcagcgcttgatcggtgacctgcccggtgatgcccagcatttccattcgcatcattgataactgactatcatctgtccaggaatagacgggccgaccggttctgccaaccgaggaaatcaagaatggattggcggtcagatgctgcagcgtgtaaaaatcgaccttgtacttgccaatattaccaaaattaagcatagtcaccagaccaacattgatttgtggaatccgttgtttaatttgtcggagaaatggataaccaaccgaatgaacccggtgtggtaaaaccgtcaattgagaggcaaactgttgggcaaatcgagtccccatctgtgggtcactgctgttagttaccttcaattcaatgatcagcggctgctttaatcggttcgccgttcgcagataatcaccgaacatatcaacatgatggaatttggtaatttctgccagattgaggcggttaatctcctgatccccgtggcctggaattggcacatcgttatcatgggcacaaataaagtgatgatctttggtttcttgaatatccatctcaacaaatggaaagtgataatggctgttacgcttcaaagcagtaattgtgtttccctgagcgttatgattaatgaccccgcggtgaacaatgatcgtgggatggccaaccggtcggacggaaaaggcgggattgatcccggcaaacagcgctgagaagataatcagacatccgcccacaccagcaatcagcccctttcctgtcagccgggcaaactgaatccccagcaggcgaccaatcacaacgatttcaacaaatggagccaccacatcaatcgttccttgtgacaaaaagaataggaatgaattgggaagcaatctgttcaaccagcccagcccaacaatcaacaggcagatgccaaccagcatcaaaaataataagcacagcttttgggcatactttttcaacgtcattaatttaacagtctgtttcaaagcttgaatcggataatcgccatccgcagcaagcagatttagcgcaaaatgagaaaaataaatcccaaccagcaataaaccaaaatagccgacgatggcagtcagcgcaagcggatagcgattgactgtcagccaagtaaactgatccccagaaatcggcaccgaaaacttaatgaaatttgagaagccaaacaggcctaatggcaccagcagaacaaacaggtaaacaccgcttcccagcagcgccaatagtgaccacgttcggctcaaaattgtcttgtgaacggtttggacgatcccataataaaatagaccgaccaacagtaaaaacatcgttagtgagcaaaataccaccgttgcgaagctttggtaagtgtccagaaaacgtctcaacagtaaaataaggacgatcaatgcccccgttaaataatcataaagtttggtttcattattccccatcaaaaaacttccctacatgcaaaaaaaccggcagcagaattctgcgccagtttgattatgctatttgttaatattttgatcgcgtggtggcaatggcttaaagtcatataagatttttgactgacgttcaaactcatcaatggcaagttggatcaggcgatcgattaattcagaatatgaaatgccagaggcagcgaatagctgcggatacaaactgatgttggtaaatccgggcagcgtattaacctcactcatatatggcttgtcgtctttagaaaccagataatcgatccgagccatccccttgagtcccaatgcccgataagttgtcaggcccatttcagtgatctgttgggcaagttcttccgagatatccactggaacgtcaaatttaacctgactggcatcaacaaacttattgtcgtaagtataaaaggcgtcgtctttgggtacgcgaatggccccaatcttggatgcgattggatgatcattacccaggatagaaatttccagctcttccggcccctcaatcgcttcttcgatcaagactttgctgtcatatcggaaagcatcgcgaatcccttcggaatattcctcggcattttcaactttgtgaatcccaaccgaagatccctggtgagccggcttgatgaacaaagtctgtcccagttcatcactgagagattcgtagctgtactgctcggccgtcagcggggtaatcacttcatagcgggtggttggtactccagccagtttgacaatcttcttggtaatgtctttatcaaatgacatggctgaccctaagattgccgtccccacatatggtttgtgcaggaggcgtaatagtccctgaatcgttccgtcttcacccaaattaccgtgaataatcgggaagaaaacgtcaatatcggattcttcagccaggttgattatccgagccaaaggattcttgagatccaatttagctaattcctgcttggcaacttcgtcttccggttctccgtcgaaaacccgagaggaagcttcatgatccaggaagtagccgttcttggtcatcaaaaacaaactcacatcgtaacgctctttatccatcgcgtcataaatgttatgagcagagcgttttgagacatcatgttccgaagagttaccgccaaaaatgaggccaatgtgttgctttttgtgtttttccatgaattctcatccttttataaattcgtatagtttccagaaacttaagtatatcacggaacttcacagttgaaaacatttacaaacgcttctcatcacatttttaggctgaattcaccgatcacaattattcacgttttaattgtttcttactgaacaagtagcgggtgatcaacaacaagatcacagaaacgatcagcatgctcacaatcatcggaaatggatcgtaggcaccagtggcccgccagccgaggacaaatttggcaaaattggcaacccaggtcatctgaaaattgcgatccaaaatgacccgggacgcggtgtacatcacggtgatgtagccgatgaccggcgtggcgatcaaaatgatccgctggacaaatttagagaacaacgttagaaagttcccgataaccatcccgctcaaagcgccaacgattaacaacaatccgctaaaaataaagttgaacaaaaatgcgacaattggattattaaagtatccagcgtacgaggacatgtagatgttggtgtctctggcatgccccaatggcatcaagacagcgtactgatacactaagttaaaggtattgccgatcaggattaacaagccattgacaatgacttgcgcattgaaaaaagtttctcgggaaatcccattttggatcaaaaacttgaagttttcataggacagcgttgaaataacaaacatatacaggccaaacgccgccgtcacccaggacccctgcatctgattggtcaaggaataatcattcagagatcctgagaagctgtttagtatcttttaagaagtaacctgataaaagctaacgaaaccatcatgagactagtgttgagcttacgctcacagttacgccataaacggtgataatttcccaaccaactaaatgaacgttcaatgagccaccgttgggggataaccgaaaattggtgtaactcatttcttttaacgacgattaccttggctgacgttaaactgctaatctcattagcaaaattttggccggtataaccactatcaaccatcatggttcgaaccaatttaaactgctctaaattaagggtaacgagtgcaatcgccccgtcacgatcagtgatgttagcccgggtaatatggatcgcttgcgggaagccattgatgtcgacggctaaatgccgtttaattcccgagatcttcttaccaccatcgtaacccttattttcagcggtagcggtgttcttgatactttgggcatctaaaatgacgaacgaagttcgggctgatcgcccttgccttaatcgtcgatcagcgacaatttttttaaaacctgagttaataaagctggtttatcaggggtgggggctttcgaccaattcatccaatagtagtaaacagtggaccactttggaaaatcagccggcaaatcacgccaagtacaaccatttttaaggacatagagcatggcacagaagatatcataaggatcaatgtgttttggatgagttcgttttcttgaagcttccagatcctggcggatcaaatcgaattgttgccgagaaatatcgctttggtaatgatgactaaaatgttgcatatgatcaccaacttttttgacagtagtttatcaaattattgggtcaaaatcaaagatactaaacagcttctgagatggcggaaaacagaaacggcagtaccaaaaaggcggcaaacaagaacagatacatttccgctaagccgataatctgtcgtcgaaacaggaatttggtgactttatttgtcttcattcttggcactcccctcatattgattggttagaaaaataaacagtttctgcaagtcaaagttggacagctggactgtgtcgggcaggatgcggtcgtcaaggtcaccatagacgtagttagcccggatggtgcccatcatgtcgtggccaatgacgtttaagcccttggtatattgctcgacgtctttttctggtcccacgaccgaatgagtcttggccaagacgtcttcaaccggctggtttaaaatcacccgcccctgatccaagacgatcacgtcactgataatattggcaacctcttcgataaggtgggtggaaacgataaatgtccgcgggttatcggaataggattgaatcaattcactgtaaaagagttctcgatggttggcgtccaaccccagaaccggctcatccagcaagacgtatttgactggaaggcacaaggccaaaatgagtttaaaaatcgagttgtaaccggtggataatttaccaaatttttgattgatatccaagccaaattctttgatcaagtgatccgctaattcatggttgaatccgccatacaaggattcggaatccttgagaatttgggtcaacttccagccgtcagcgtaaagattggcctcgctcatcaaatacatcaaacccagctttgagtcgttatcgctgacatcctcagaatcaatcttaacttcgccgctgtcggcaaaaatccggtcggtaataatactgagcagtgtgcttttcccggcaccatttcgcccaagtaagccgtagattttgttgccgtcaaatgacaaattaatgtctgacaagacgtgcttagacccaaatgatttcgagacgtgactgacttccaatacgctcattgctggtaacctcttttcactaaattcaataactcatcttcagaaatatccagattctgggcttcccgaaccagattttcgacaaactcgtcaaaaaagccattccgcttttctgccaagattcgctgcctggcgcctgcttggacaaacatccccagcccccgccgtttttcgatcaaattcttagcagcaacgatgttcatcccttttaaaacggttgccgggttaatatgaaactccttggaaatttctgtcgtcgacggaatctggtcgccttcagcaaaccctcccgaagcaatcgcgtcctcaatttgttcggcaacctggcggtagatgggctctgaactattaaactcaaacttcatatttatcaacccattctataatttctttcatttaacgctccaccttcgtctttggaaccacaattcgggaataaatcaggacggtcaaggcaaagtaaatcaagtagaggaccaagaagccgactgtcgtcagtccaaaggtttggtaggcgccacccatcaatagaccactcttggcgaacatttgaagtccgaaggcaacgtcgacgattcccaaaattcccggcagtgcaaacaagcccagaatttgaacaacaattgagtgatttaagaccgatcggcgagttccaatcttattgagcatatcaaagcggatcttgtcactggctgccccactcaaaatcttaaacattaggcagctggcgagcatggccagaaaggcaattcctaagaagattcccataaactcaagactgccaaagacactcttcagggattgatacatcgtaaacgaaacgccgacctgttccccgtttcgatagccgtactgcgtggactgaatgttggtaattttggtgagtggcgttgcggcagcgtccatatcatttgcgcgaaccaacaataattgattggtcttggcattaatttgattgaatgcctgagaactgaccactttgatttggtaggctttaatcgttggtacctgcagtccccacagctcttggtatgccgatgaatcactccgtttgaactgggaaattttggcggtaaaagcctttgatgccagtgtctttcgactcacaaacgccgcgtacttcaagggttggcgctgaagctggtcactccggtaataaacccgcttggtcgtcggatcaactttttgttggtaagtgacagtggatttatcttgaatctggccaaccagtgaacgcatttcctgattggggttggtaatagcaactgaatagtagccatttccggaagctaatttgggtaccatgtgttgaaaaccggttcccacagtaattgcccctagtgacaacgcaaacagcagcgagacaactgaaaggattttggtataatcacgaattctaaatttaagctgggccaatgtgaaactgttcaggcccttggtgctcatattagaacgttgaaatgcctggagcagcatcacaaaaaatgagttgaagacaaagtaggtccctagaacaatcgtgatgagcgcgattggaatggacatgactttcagtttttgaatgtcatacatcgcataatatccaccggccaagagaacaactccaagaattgcttgaacgccaagtgtcaaggccttaggctgctgccaatcactttgctgtccggaacgcaaaagctgcagggcggaggtcttggtgaatgtcctggcatttaagaaaccagcaaccaggaacaaaatcgcaaacaggataatcgttgcaatgacagctggcatataaaatgccgagaaattagtcaatgacatgtgaatgaggctggccagaaaatggctgagcacttgggtaaagccaatgccaatgacaatcccgacaactgtggaaattaaaccgatcgcaatggtctcaaggatgatcaatttactgatgacccctgatttggcccccagcatcatgaagagtccataatcatgttcacgcatactcatcaagaaattattcgcgtaaaaaacatataccagtgtgatgattgccagtaagatggatccgaagatgaaaacgatcttggcattttgtcccaccgcactgctggtggtaaatttatcatttgttgaaattgcttcaaacatgtagaaaatggctgtggtaatgatcatcccggaaaacagaaccagataatctttccaacgagccttgattcctgagattgaaattttaaataacatcgctaagctcctttgattgattactgttcaaatgtaccgagtttttcgaggatttcctgatagaattcatttctcggcttatcgccggcgtctacctcatcgccaatttttccgtctttgataaataaaattcgtttacagaaactagcggagaacgggtcatgggtcactaagagaattgagaccccctgttgattgatgttcgttaaggtgtccagtaattcacgggcgttggttgagtcaagcgctccggttggttcatccccaaaaataattgacggatttgacactaaggctctggcagcggcgacccgttgcttttgcccaccggataattgcgttgggtacttactcagcaagtcatcaattcccaacttgctggcggcttccttgacagcagtttggatggtggccgccttggcattttgaagcgacaacggcaaagcaatattttcttgggcggttaaggtttccaataagttaaagtcttggaagatgaaacccaattttttagaacgaaaatctgccatctggttcgcagttaaatgagttacatcttggccgtcaatttcgaccgaaccgctggttggttgatcgagagttgccaaaatatttagcaaagtcgtctttccggaaccggacgcgcccatgattccgacaaattcgccctcgttaaccgacaagctgatccctttcagagcttcatatggttttgcgctgtctttatcgtaggttttgtgtaaatcttctgtttgaacgattttagttgtcataagtgttcctccgtgcgttagttaattacttatgtaactaactatatatgctaagaatccggatgtcaaccaaaaacaaaaaagcgtgggccaataagtggttagcttccagagtataaggggattacccgaatatccggaatttggatgtttgggtaatcccctcatacggccggaagctgcttattggcccacagttctgctagataacattcagcctcttaatcgtctaaaagcgttaattaatctagattatcagtattaatgacattctgggtccctcgttcagtgatgatggagactaagacgttattgatcattttcatccgctgttcatctgtaatcgatgatcccaaatccttttgcagctgggaaacggcatcctcggaaatcgccacggctccttgaacaataatttttcgggccgacaaaatggcggttgcttgttgtcgctgcagcatggcgttagcaatttcagttgcatatgccaaatgcgtcaaccgggtctcaatgatctgcagaccggccacatccaaacggtcctggagttctttttgcaacgccacggaaacttcggttgcgttcccccgcaaggtcaatttgtcggtactgtcgtcaaaactatcataaggatactggctggcaatatgtcgaatagcggactcactttgaatctcaacaaactgttcataatcttccacactaaaaattgctttggcagaatcaacaactttgtagacaatgacagcggcaatttcgactgggtttcctttggaatcgttcactttgataattgaactattaaaattgcgaacccgcagtgaaatcgtctgcttgctggtcaatggcacggtcatgaataatccggaagttcgaattgtcccaatatagcgaccaaagaatgtcaacactttggcttcgttaggctggataatcgttaatgaacttgcaaataacaaatccaaaacaatgatgattgtcccaaaaacgatcgagccaattgagctgccttcaccgccaatccaaagcagataaccgccaactcccagcaaaatcaaggcaataattaagcccacataaccattaacatgaaatacatttttctctttcaaaaaagccgccccctataaactcggattcgtaaacaattactaattcaagtatatagcggacggcttttaattgatattaattacttaacattcttctcgggtaaaacggcacctttatagtgatgcaagatccatttttgagtcttggttgattgaagaaccttgactaccttcttgatggctggcttgttctgatcacctttacgggtggcgatgatgttcacgtatggtgaattccgtttttcaatcgcaattgactgcttaattggattcaacccggcaccaacagcgtagttggcgttgatgacaactgcatctccttcaccattcttataaatggttggcagtaattttggttcatagctgtgcttgaatttcagatgacgtgggtttgaagcaatgtcactgaagttggcagaagtaatgtcaatgccctttttcagagtaattaagccggcgtctttgaagatctgaaggattcggccatagtcgggaacattgctgctgacgatgattgtggcccccttcttgaggtcttgaagcctcttaactttcttcgagaaaacagcgatcggttccaagtgaacgccaccggcattgactaatgtcccgtggttctgcttgttccaaagtttcaggaatgggacatgctggaagtaattggcatccagttcgccgttggccaaagccttgttaggcattgtgtagtcttggaaagtggtaatcttcagattgacgccttcttttttaagttctggggccacgtggcgcaaaatttgtgcatggggcacggctgaagcaccaatttttaaagtggtggtctttttgctggaattagacgatgatgaacaccccaccaacaaaaaggcggtaaagacaactgcgaataaactcaataatttcttcttcatttgaaaccctcccaaatattataatgtccgtttgtcggtaatcttgacaaagacatctccgacaaattggacgacaaatacaaataaacaaatgatgaccgttgcgactaaggtcactgtgttgttgcttgcctgaaacccatcttgataagccaagtttccaaggccaccggcaccaatggcacctgccatagcggtgtaaccaatcaacgaaatggtggtaacagtagctccggcgatcaatgccggcttgctttctggtaacaggaccttggtgataatttcccaggttgtggcacccatagattcggcagcttccaagaccccggaatcaacctcacggaagtaggactcaaccatccgagcgtaaaaaggtgccgccgaaataatcaaggatggtaacgcggcccgcggcccaatgatcgttccagccaacttcatggtaattggcagtaacaaaatgatcaggatgataaatggaattgaccggaagatgttaacgaacaacccgaccagccaattgagaattcgatagccaatgcccggcttgttgcgagtctcgtataagatcaaccccaaaataattcctaaaataacaattgcaaccattgataacaaggtcatccaaacggtttcccaagttgccgacatcatcgaaccccaatcgacgttatgaaactggaagtaagatttgaatccagttgaattagccatgatgaatcacctccgttccaacccgcatcttcttcaggtattccaaggcatcgttaatttgattgtcatcgccgacaaattgcagatccagcgaccccaacgcgccttcttgagtttgatgaatcgcccctgaaataatgctgatggttaattccgggaaccgtttgacaacatccgaaacaattggcagttccgcctgtggtccatggaaaatcagtcggatgatttgcccatcaggatatttcttaactaattcatcaagggtcatcgtgttgtcactttgttgtggtgtaaattcttcactgacaaactttttggtgatttcttgttgtggatgacggaaaacctcaaacactgatccggtttcaacaactttgccgctgtccataactgccacccgttcacaaaccttggcaatggcgtgcatctcatgggtgattaataaaatcgtgaggttcatttctttattaatcttcagtaataaatcgagaacttcattagttgtgtcaggatccaaggcactggttgcctcgtctgaaattaagattgttggctcgtttgccaaggctcttgcgatgccaacccgctgcttttgaccaccggataactcggaaggataggaatgctcacggccctccaaaccaactaacttaattaattcctctgcgcgttgctttcgtttggctttgggaactttggcaatctcaagcggtaaagcaatgttgtccagcaccgttcgtgaccacaataagttgaaatgctgaaagatcataccaattttttggcgttgctttcttaattggcttccgtggagcttggaaacatccgtgccgttgatgtcaatctcaccggttgatggcgcttcaagtccgtccagcattctcaccaaggtgcttttcccggcgcctgaatagccgacaatcccgaagatctcaccatcgttaatctcaatgttgacatcattgaccgcggttagaccgccatccttggtactgtactgtttggatacatctttaaatcgaatcaatcttttcaccccttattagacaaaaaaagcttttcatcctccataagtcttaattgacttatgaaaggacgaaaagcttcgcggtaccacctttattcgcgattgtctttcaacaatcgcctcatgagtatcttcatactcaacgaaataatggtcgttacccattatcggcttgcaattgctcaccgacacatttttaaccaagaccatcttcaataacgatgattgaccctttcccaccagccgggctctcttgacaatctctaattatctactcatcttgtaatttttctatcatcaaactatcagttagtgtacctaaaaaaggtcctagcgtcaagaacttttattttttaatcttagcaatccatgaagttgccttgtcagtcccgtttagtactgaagggtcattaacggcattactgttgacagcagtcactttcccggcaactggacttgggatatccgaaacggctttgtcagcttcaacgtttaataaagtatcgctggtggttaattgagcaccaacctttggaagggaaacaaaagtgatgttacccagttcgttcttacctgcttcggtcaagccaactgtgacttccccgttattttcttcagtccaataatattttgtatccatcattaattccaccttttctaaaaattatgagaattctttgtcttctccaaacatgtaactcttattatgatactgcattgacataattaagccaatcccaatcatgttcccaatcaacgccgatcccccggcactaacgaagggcaatggaataccggtcaatggcaacaggccaatactcatcccgacattttcaaaaacatgaaacagaatcatcataatcacgccagtggaaatgtaagcgtaaaaaacattcctcgtatcgaatgtaaccttaatcatttgataaatcaacaggaaatacaataaaatcaaaatacagctgccaataaatccaaagttctcgccaataaccgagaaaatcatatcagattctcgcaccggcacatacacatgtgactgattaaatccggttccaaaaatcccaccagatccgatggccttcatactctgccacaactgatacccctgattagaagtatcggctgacgggttgagccaagtgtcaactcgggcaaactggtaggcttgaaaaccaaacttctccaacagatgacgcccggactccggaataaccaaagccaagatggttccggcaaatccaaagatggtaatcaccgctggcagaataatccgccatgtcactcctgaaacgatgatcaagccacctaagatggcgaagaaaaccaacatcgttccaaaatcattttgcagctttaacaagacggctaccggaactgtccacagcaacattttcccaattaataggaaatcacttcgaacagtcctgattgggtaattatcgttatgttgaacaatcacccgccccatcatcaaaatataggccggtttcatcacttcagacggctgaaaggtcaacccaaatagggagaaccaacttttggcacccgtattaatgtaataggtccgactgtataacaccaggacactcgccagcagggcaatccccagccagtaagtaatcggggcaactttccataactgctcggaatcaaactgcataataatgacaacggcgataattccgatgacgtaccaaaccaattgcgaaaccacctgtctcatgacgctggtagagcttgaatcatgagtggctgcaacgtaaatcgatgccagcccaatcaacgccagcattaagacacagaaaataattccccagtcaattcgcgattggtcgtctttagaggttctgcgactgctatccaaattagaccctcctcgttttcgatcgccaaattaatggtgaagatgaaaatctttgattaattgtgtcacaccctcatcgaaggttttaacatgaaacgcttcgtcgtgagtgttgactgcttgaaatttagtttcgctcaactgcttaattgagccaatcaatttcttgccgataaataattcggagatcgattctccattttgatccgttcgatctttaatttcaacgttgatacttttatttgctttactcatcatattctccttgttcaaagatcatttcaggtgcatggatttccggtattcatcgcgtgcgtccttattccgaaaaatggtgaagtgatccggaaccggatcatagccacccttaacaaacggatggcaacgcagaatccgggcaatgcccataacggcccccttgaacgcaccatgctttttaagggcagttaccatataactgctgcaagttggataataacggcaggtaggcgggaataagggcgaaataaagcgctgataaccatgaacaagactaatcagaatgtttttcactttgactcctgttatttttgatcttttgccttcaacttagggttcttaatatagtgttccaaaaggataccggcacccttggcaacattatccaaaggattttcggaaataatcacgggaactgttagtgcatcggcaattacttgatcgatgtttcttaataaggcacccccaccggtcagcatgattccacggtcaacaatgtccgacgccaattcgggtggaatcacttcgagaacttctttggcaccactgatgatcaattgaacggtatcgttaattgcttcggcgatctcattgctatcaatcgtaactgcccgaggcatcccggaaacagcgtcccggccacgaacttccaatgttttgacgtctgaatcgtctttcttagcggttccaatttcaatcttaatcttttcggcagtatgctcaccaataatcaggttgtgcttttgcttgatatagctggcaatctcggtgttcatcttatcaccggcaactcgaatggacttgctggcaacaatatcgcccaatgaaatgatggcgatatcactggttccaccacccatatcgatgaccatgttaccacgaggctggaagatatccattccggcaccaacagcggccaccttaggttcttcttccagatagacttgtccgccgccagccttttcagcagcctgcatgatcgcattccgctcaatttccgtcacgttggttggtgcacagatcataatttttggcttggacataaatcctttaacgtccaatttgttaatgaagtatgtcagcatttcttcagtaatatcaaaatcagagataacgccgtcttttaatgggcggatcgcacgaatgttacttggcgtccgaccaaccatccgataggcttcggagccaactgccaagactttaccagtccgagtatcgactgcgacaactgatggttcgtttaatacaattcccttcccggcaacgtaaatgagtacgttggcagttcctaaatcaattccaatgtcttttgccatctgtgtaggttcctcctgaaaaactttaatctcaaaaaataattataccacataaagtttgcgtttctaataagtctccaaacaataaagggttgagatcaagtaacgatcccaaccccgaaaaattatgaacgattcttgagcgattgattcaagacgattgagtcgtcttcaacgttgactcttttaatttcagcacctaaattagcgagcttcttgtggaaatcgtggtaaccacgatccaagtactgtaagttggtaacggtggtatagccactagcggccaagccggcaatcaccaaggatgcggcggcccgcagatcggtggccgcaacttcggcaccattaaaatcagtagggccatccataatgactgttcgaccagagatcgtatattgagcattcatccgacgcagctcttccatgtgcatgaaacgattttcaaaaacggtttcagtcattgagctgctgccgttagcggtcaactgtaaaatggtcatttgcggctgcatgtcggttggaaagcctggatgcggcattgtcttaacgtcaaccggtttgagattgtcatggccgatgacttgaatgccatcatcgctttcgttgatggtaacgcccatctcgcgcattttgagaattagtggtttgttatgctcgggaatagcgccatcaatcatcacgttaccacgagtaaccgcagcagcgatcatgaacgttccggcttcaattcgatcttgaaccaccgcgtgatcagtcccatgaagttcaggcaccccttccacgcgaatctgttcggttccggcgccgacaactttggcccccatcttgtttaaaacgttggccaaatcaacaatttccggctcgcgggcagcattctgaatgactgttttgccctttgctaacgttgcagccatcataatgttttgagtggcaccaacgcttggaaaatccagatagatttcagctccggtaagtccatccggggcgtaagcttcaacgtagccgtcatgttgttcgatccgagcacctaaagcttcaaatccttttaaatgcagatcaatcggtcgtgacccaattgcacacccaccgggtaaagcaacctttgcgtgcccgagtcgagccaaaagcggccccatgacaacaattgaagcacgcatctttgagacatactcaaaaggtgcttcactggagatatcttttgaagcatcaaacgtaatttcgttattggcttcatcaaaatcaacctttacatttaagaaccgcaacactttattcatggtatacacatcagacaacaatggcacatttgagataaccgtctttccctcaccggctaaaatagttgcagcttggattggtaaaacggcattcttggccccatcaatatgtactgtccctcgaagtggcttaccaccatgtacaataattttttccacaagaacgcctcctacatcacttaattagatacatcaaattctgaatgttaaatattacagagaggaaaaatgaactgcatgcgtacccaatcgcaattgaaacgagcacgatcagtaatttccccggcattgccctcaatgggatataacgctcgatgtggatttcttgaactgtccaaaacgccatagcgataaacaaaatgtatgtaatcaatgtaatcagcgcttgaatgccaatcgtattcatttgagtcttcccccaattcacagacaactatatcataaagacgcgaacttgtcttaccttttcggtttcttttacaaaaatataagcagaattgctatctaatcggcacattcggataacaatgactgtatatgattccgacaaaacgggagaaaaacgcaaacataaatacatcattcacaaatcacgataaaggaattctaacctgattcaccggtaatttcaaggattaactccaaccaaccaaaaaagctgcaacccaaatgggcgcagcttttgaagtaccgtgttcagtttccggaaaccgcaatcagaaataacggttatttcccggcaacgttgattctgttaattgcacggcgaagagcaacttgagcacgatcaagagcagccttatcctgtcgttgacgggcttcggcaattctttgttgcgcgttcttctttgctttttcagcacgggcaatatcaatatcattttgagtttcggcactatcagccacaattgtcgcaacgttgtttgagaattcgataaagccaccgttgacagcaatatcatcttccttgtcgtcgtatttaactcgcgtttcatcaacgtcaagtgttgcaataatcggaacgtgattagccataattcctagttgtcccgactgagttgaaacaactatcatactagcagtatgctcgtaaacttttccatcgggagtaacgatactaacggtaataactgaattatcagccaattagaatccctccttagtttgcagcacgctgcttttcattgtctgattcctgtttcatagccttggctttttcaacaacatcttcgatagggccacagttacggaaggcatcttctggaatatcatcgtatttaccttcaaggatttccttaaagcctttaacagtatcctgaactgatacgtatttaccaggtaagccggtaaactgttcagcaactgagaaactttgagataagaagaattggatccgacgagcacggttaacaaccgtcttctcttcgtctgacaattcatccataccaagaattgaaatgatatcctgcagttcacgatatcgttgcaaaacatgttggacttcagtggcaacttcgtaatgttcttgaccaacaattgctggatccaaagctgatgatgttgaagccaaaggatcaacggcagggtaaataccttgttgagtcaatgaacgttccaagttggttgtggcatccaaatgggcaaatgtcgttgcaggagcagggtcggtataatcatcggcaggcacataaacagcctggattgatgtaatggcacccttcttggttgaagtaattcgttcctgcagttgacccatttcagtagccaacgttggctgataaccaacggctgatggaatacggccgagcaaggcggaaacttcagaaccagcctgagtgaatcggaagatattatcaatgaacaacagaacgtcttggccttcttcatcacggaagtattccgcaattgtcaaaccagtcagggcaacacgcatacgcgcaccaggaggctcattcatctgaccataaaccatggccgtcttctcgagaacccctgaccctttcatttcgtagtacatatcattaccttcacgagtccgttcaccaacaccggtaaacacagaaataccattgtgtccctgtgcaatgttgtgaattaactcctgaatcaagacggttttaccaactccggcaccaccgaacaatccaactttaccaccacgagtgtatggttccaataaatcaatcaccttaatccctgtttcaaggatttcagttgatgggtttaattgatcatacttaggagcatcgcggtgaattggccaacgctcagcgtcagggccaaattctgggccgccatcgattggatctccaagaacattgaatactcgaccaagagtatctttaccaaccggaacactgattgaagattcggtgttttcaacgtccataccgcgacgaagaccatcggttccatccatagcaattgtccgaacaacgccatcacccaaatcaagggcaacttcgacaatcaaattcttgtcttcgctgacgtgaattgctaaagcagtgttaatttctggtaatttatcgtccaaggagaattcaacatcaacaactggtccaataacttgtataactttaccagtagaactcatgttagttaattcctccattcaaatctttctagtgactaagagcctcttgaccaccagtaatttcagtaatttcagtggtgatggcagcctgtcgagcacggttatactgcaattccaatgaggaaatcaaatcgtcagcattatcagatgccgacttcattgcagtcgaacttgaagcatgttctgaagtcttggcatcaaggattgcaccataaaccaagctttcagaatactgtggtaatacaacatccaagacttctttttcagaaggctcaacatcgtattcagcactcatcggcttaacttcaatgtcctggctggcagctgacgcaatggcttcatcatcgattggcagcatcttctcagctctgaaacgggaaataagacggttaacgaaatgctcgtaacaaacgtacaattcatcgaattgacctttatcgtacattgatgtcaccatcttgacgatttgacgaacctcgttaaaggttggcacatcgctaacgccccggtattcataagaaacattgtcgccgcgtttcttataaaagtcggatccggttccaccaacagcgagaatttgataatcattcgatcccgaatgcttctcaataaactcattggcttcacggataacgttactattataactaccaaccatcccacgatcagaggtgataattaaatatgcgcttctcttagtcttagattgatcttgatcagctgaatgacctgaggatttgtttagcccatctaaaatgtgagattgggctaaatgcaatacaacagatttgatttggcttgcatattccgcataactaaccgtatgcttttggatctggttcagttttgcctgagaaaccatttccatggcattggtaatttgtcgcgtcttcttagtagaagtaatccgatgtttaacatcgtttagcgaagcacccatgtaatctcaccctccttaaaactagtcatttgaagcagctgattgatcatcgtttgattgttgatcatcgtgcttacttggttggaaagtttgttcaaagtctttaattgcagcatccattttacttgtatcaggcaattgaccggtcttagcgatatcttccaacaaatctttgtgattttgatcgaagtaatcgaagatctcggtttgatatctcaaaatatcatcaattgcaattttatccaagaatccatgggtcaagcagtaaagaatgacaacctgtttttcaacggaaattggcgaatgaagtggttgcttcaaaacttcaaccgttcgggcaccacgatttaatttgctttgagttgcttcatcaagatctgaaccaaattgtgcaaatgattccaattcatgatatgaagccaaatcaagacgcaaagtaccagaaactttcttcatagccttaacctgcgcatcaccaccaacacgagaaacagaagtaccagcgtcaacggctggacgaacaccagaatagaaactatcggcatccaagaagatctgtccatcggtaatggaaataacgttagttgggatataagctgaaacgtcccctgcttgagtctcaacaattggcatcgcggtcattgaaccgccacccaacttatcacttaacttagcagcccgttccaacaaacgtgagtgggtatagaaaatatcaccaggataagcttcacgacctggaggacgacgaagaataagtgacaactcacgataagcatcagcctgctttgataaatcatcgtagataatcaaaacgtgttgacccttgtgcatgaagtactcacccatcgttgcgccggcataaggtgcaatgtaaagcaatgatgcaggttcggatggcccagctgaaataacagttgtgtaatccatggcaccgtacttttcaagggtacttacggcagttcgaacagttgattgtttctgtccaattgcaacgtaaatacatttcatattctgacccttttggttcaaaatcgtatcaatggcaattgaagtcttaccagttttacggtctccaatgatcaactcacgctgacctctaccaattggaatcaatgaatcgatcgctttaataccagtttgtaatggttcgaaaacagattgacggtccataacacctggggccttatgttcaatcgctttgtgatcgtcggctttaattgggcctttaccatcgattggttcaccgagtgaattaacaactcgtccaatcatctcgtccccaacaggaacttccataattcggccggttctctttacagaatcaccttcacgaatattcgtgtcatcacctaaaatcatgataccaacatcattggtttccaggttttgtaccattccataaacgccgtggccgaagtcgagcaactctccagacaacgcattttcgagcccatgagcacgagcaataccatcaccaacatatgtaacgatacctgtttcttgaacgtcgagctcgttcttatagccttgtaattgttgcttaataagagcactgatttcctcagctttaatgctcataagtttcacctctttaaatagatatcgttaattcaacaataattctttaaccttattaatgcgagtttgaacacttccgtcgataatcacatcggatgatcgaatcacgatcccgccgatgagtgatttatcaactttggtatcaaaaatggctttaaccgcacctacccgcttctcaaatgctgttgccaaacgatcaagctgatcatcgtcaagcggcgttgccgaaacaacctgcgcccggacaatcttcttgtcatcttcgtaaaccttttggaactgatcaataatgctcagaacctgtgggaaacggcgatagctggcaacaacctttaaaaagttattaataaagtctgatgcattttgggtgataggagccagcagagactttttctcgtcatctgaaactcgaatatcatcgagaatttcaatcaaccttggattagcagcaaaaattttacgtaattcaagcaaatcagcgtaaccagattcaagttcattagaatcactcagaacttcaaacatggcttttgcgtatttttttgaagcgctcatatcatctaatgtcatttctgcttacccaacccttcaatataagagtcaacaagtcctttttgatcatcttcgtttaattcttttgaaataatcttggatgcaatttcaacagaaagacttgccacatcttttcgagaattagccaaagcttcttgtcgctcttgttcaatgtccttttcagcagaactcttaagattcgatgcttcatttctagcatcttcaacaatctgttcttgttgtctttgtccattctgtttggcagtgttaataatggtatttgcgtcatcacgcgttttgtctaattcagcctgacgtttttgagcaagttcagctgctttagtccgtgattccttggcagaatcaatatcattaacaatcttgtctgaacggtcttgcatcatcttcgtaattggcttccatgcaacgatcttgaccaaccacattaaaacaagaaatgtgatcatgacaaacagcatatcaccaacataaagctgagctccaactactgaatatgaaaacatcaattggcacctccttctttgtgtatttgactaaaccggttattacttgttcataaccagcaaagcaacaacgaaggcgatgataggcatagcttcaaccaaaccaacaccgatgaacatgttactacgcagttgtccggataattctggctgacgtgccattccttccaacatcttagaaattaaaataccatcaccaacagctccaccgatagcggcaccggccattgcaatacctgcagcaattgctcccataattaaaaatcctccttatagtctccaaaaatatttttgctaatcttcaagctcgagctttcgtgaaatgtatacggatgataatgtcacaaaaacataggcttggatacatccgataaagactgagaaacctgtccaggccaattcaagaatgaatgaaacgacccacataactgctccaccatgcgacatgccaaggattattccaagaagcatttcacctgaaaggatgttcccaaatagtcgcaatcccaacgttaagaaattagtaaactcttcgaataagttaattggcaggaaaaatacgaatggctttaaataattctgaaaatgtcccttgtaacctaactgccgaattccaaggaattgtgcaagcgttagagtcatcagagacagagtcatagtaacaaccggatcagaagttggacttttgacatatgttacaccagaaatgtcgatatgcaagaagagtccctgcaaattcgcaataatgatgaacataaacagagtaaagccccataaacctagtgttctacttgtttcaccggaaatcgagcttcggacaataccattggtaaagtccaccgcatattctaaaacgttttgtgccttgcccggtttgattgtcaagtgccttgataaagcatacaccagaacaaaaaccacacaagcagccagtaatatcgaaattaaattaccaacgttaaacgtcagtcctaagaattcaaaagtagaagcagctccttccacaaaatctcacctctttcctccacataatcacgcatgcaaatcaatctggttttggtccagaagacagtaataccaaagtgaaacattgcgatggtactgaacacagaaccgtgttcaaatacaattgaaatcataccaccatttattacaaaattcaaaacaatcttgacagggaaacttcgcgtgagcagtagtgttcaacggcatgcacaacgaatgtcacccaagggtctttgattagacttaattcgttggctatcaaagccagaatccttttgtaaataaaataaaaagctgacgacaaaattttcattttgtctcagcttcaatcaattatttggttccaaacaaacggtcaccagcgtcaccgagtccaggaacaatgtagcccttatcatttaatttttcatcaagtgcagcagtatagatatccacatcaggatgagccttttgaagtgccttgaccccttccggagcagctactaagcaaacgaacttgatgttggatgcgccgcgcttcttcaaggcatcaatcgccatgattgatgagcctccggtcgcaagcattggatcaacgacaaaaatctgccgctggccaatgtctgatggcagctttacaaaatattcgtgaggttcgagggtcttttcgtcacgatacataccgatatgaccaactttggctgctggaatcaaatcaagcatcccatcaaccattccgatacctgcccgtaagattggtacgatggcgacctttttaccggaaatctgcttggcatgcgcaataccctctggtgtctcaatatcaacatcttccaaaggcatatcccgcgaaacttcaaaagccattaaagtggcaatttcgttgacgatttcccgaaactctttagtcccgcaattcttgtccctaatcattgacagcttgtgttgaatcaacggatgatccataacttgaaacttacccattattttccaactcctttttgtattccgaaataattgtatcacatatacgcgatcggaaagtatacaaaaaggcttgaaaccacaattagtttcaagccagtcaaaattattgattaattgggtgagctgcagttaattgttcaactttggcagcgacatcctttaagttttggtcatcatttggtttgtcaatcacttgtaaaatcaaattggcaaccgctttggcatcgtcttccttgaagcctcgggtggtaatggctggcgttcccaaccgcaacccgctggtcttcgaaggtggcaatggatcatttggaatcgactctttattagtagtgatgtgaacagtatccagcaggttttgcagctctttaccattcaatgaggtctgcgttaaattaagcgtcattaaatgattgtcagttccaccggtaagaacggagactgacttggaattctggaatacgtcggccattgctttggcatttttaatgatctgctcgccgtattctttgaatgccggctgcaaatcttcgtagaaggccgccgcttttccggcaattacgtgttccaaaggaccaccctggctgccagggaaaacagctgagttcagcttcttggcatacttttctttggccaaaatcaatccaccacgaggtccccggagtgtcttatgcgtcgtcgtggtgacaacgtcagcaaccggaactgggcttggatgcaatccaaccgcaaccaaaccggcaatgtgggccatgtcaaccatcagataagccccaacagaatcggcaatgtcgcggaacttctgccagtcaatgattcgactgtatgcggaggctccggcaatgatcaattttggttgaacgatctgggcaattctggcaacttcatcataatcgatcaattgcgtctttggatcaagcccatacgagaaagagtcgtagagcttgcctgaaaagctgactttggcaccgtggctcaaatggccgccggcgtctaaccccatccctaaaatccgatcaccaggctttaggaatgcggcataaacctcttggttcgcttgtgaacctgagtgaggctgcacgttggcatattcggcaccaaacaattctttggcacggtcaatcgccaattgttcaacaacatcaatgtactcacagccgccataatatctccggcccgggtatccttcagcgtacttgttggtaagcacggaaccctgagcggcacgaacagcgtttgatacgatattttcagacgcgatcagttcgatattatgctcctgacggttctcttcgttggcaatggcatcccaaagttctggatcctgctgtttataatcgtagttcaactgcaacacctcactaatttatttggtacaaataaattataactgcttgaaatgcatttgcccagctgatttattcaaacgattcatgtaagcctcaccaattccctttggatcaattccttgggtaaaaataattttataggcagggtggttatcaaaatcccgtagttcggcaaacaaatcatgcgctgctgtgcgggcatcattgccaagtgaaatcacatcgacattatccggccaattaattgttttgatgacgtcatcaaaagccatcaccccaattggctgtgggtgctgcttgatccaggcgaccacatcgtgccaatcgtcgtcaggatcgacaatgtagacctgagcattgggagcatagtgcttgtacttcattccaggggctttaggggtttgtttggcgcccacatgatggagttcatcaatcaccggtcgatgaataacggcttcaatatcctctttggtcacagcacccgggcgcaaaatcgacggggttgccacagacatgtcaagaatcgtcgattcgacaccaaccgtggtcggtccatcatcgacaattgcagcaatcttgccatttaaatcatgataaacgtgttgtgcagtcgttggacttggcttaccggaagtattggctgatggaccgacaattggtacgccggcctttgaaatcaaatccagcgtggcttggtttttcgggaacctgaacgctgcggtgtccaaaccaccagtaaccgccttagataaagcgtttggcttcagcttaaaaatcatcgtcaaagaacccggccaaaatttggccatcaatgctttggcgtcgtcggaaaatggctgggtgtatttttcaaccatcgcgatgtcagatacggtaacgatcagcggattatcactgggacgtcccttagcggcataaactttcttgaccgccgtttcattggtcgcatcagcccccaatccatagacggtttcggtgggaaatgccaccagttcgccttgacggataaagtccgccgcttggtctagttgctgctgttttaaaattaaagtttccatattatatagccttcatttctttacttgaatcatccgttgatgaccggagacatcgtgtttggcaattactcgagcgttgggcatggctgcttggaagatctcggtcacagccgattgttgctgaaacccgatttccaagtacaacctgccctttgaagttaagtgactctccgcatcggcagcaatttgtttgtaaatagcaagtccctggtctttcgcatatagtgccaagtcaggttcgcttttgatcacgctggcatccatataggtctgctcatctttggcaatgtatggcggatttgacacgatgacgtcaaatgactcatcaattgctgcaaaaacatcactcgccataaaatgaattgccgtgtgattagcaatcgcattttgccgagccacttcaattgccggcagggaaatatcactggcaaatacctgccagtggggtctggaatgcttgagggcaatcgcaatcgccccactgccggtaccaatatccaagaccttcaactcagaatctgagttttcagccaatatccagtcaaccaactcctcggtttcaactcggggaatcagcacatctggtgtgaccttcaatgataaaccgtaaaaatctgcctcgccaacaatgtactgtggcggcacccctttcagcaattgaccgatcgcgtcttgaaatacttgccactgcttgtctggcatctgagtgtggtaatgaatcaacagatcggtagccgacatcttaaatagtttctctaacaaaaaatcgacgtcgtacatgtcaatgtcattagattccttaatacgaaaagaagcccactttcgggcttcaaagtaggtcacgttttcttgattattcattggtcaaattctcaagtttcttggcttgatcagaaacaatcaaggcatcaataatttcgtccaactcaccgttcatgatccggtctaacttgtttaaagtcaagccaatccgatgatcggtcacccgattttgcgggtaattgtaagttctgatccgctcggaccgatcaccggttccaatggccgatttacgttcagcgttgtattgatcctgttcttgttgggcatagtaatcataaacccgggcctttaaaatcttcatggccttctggcggttctgctgctgggatcgttcatcctgcatcgcaactacaatgccggttggcaagtgggtcattcggacagctgaggaagtcttgttaatatgctgaccgccggcaccagatgaacggtaaacatccacccggatatctttgggatcgatatcaatatcaacatcctcttcttcaggcatcacaccaaccgtcgccgtggaagtgtgcacccggccggcagattcggttaccggcacccgttgaactcggtgggcaccgttttcatacttgagctttgaatagaccttgtcaccggtaatcattaaaacgatttctttgaaaccgccaacttcagtttcgttcttatcgatgatttccactttccagccctgacgctcagcatatttggaatacatgctgaataaatcggcagcaaataagctgccttcatcaccaccggcggcgccgtggatttccataatgatgtttttatcatcattggggtcttttggcagcagcataaccttcatttggtcttcgagcttgtctttttcgtcggttaggctggtaatctcatctttgaccatcgcttcaagatcatcatcaatcttttctcgaagcatctctttgtcatcgtcgagctgcttgctgactttttggtacttcttaaaagcggccacagtgtctcgaaggtcggcttcttccttagatagtttcatgaatttttgagtatcggcaatcacttccggatcactgattaactcgtttaactcatcatatcgatcaacgaccgattgtaatttgtcgaaaatttcgtccatttaatattcctcacttttgttacttaataggtggattgtaataatgctttctgcagaccggataataggattcgttcccacccatttggatttgttcaccctcatacaccggctcgccgttgtgaaaacgcaggttcatgatagccttcttgccgcagaaccagcaaatggttttcatttcttctattttatctgcgtataacagaaggtatttggaaccctcaaacaagttgttttgaaagtcgttcttcaagccaaatgccatcaccggcacgttcagctcatcgacgatccgggccagttccatgacgtgctttttctttaagaattgtgcctcgtcaattaagatacaactggcatggggatttagttcctgtaccaaatcaaagacattggtatcctcgcgaatcggttcggcttttcgttccaaaccgatgcgcgattcaatcatgccctgcttttctcgggtgtccaacgcactggtcataatgataacacttttattttgctcttcataattatgagcaaccttgataatttcgattgttttgccgctattcattgcaccgtaccgataaaatagttgagccaaaatatccacctttttccttaagagcttctcttccattatacagaaaaagttttgaaaatcgataataatgagaaaattcgccagcaccctcattattatcgaccccttaaagaacgagcgtatatatgttcaaacagttgagcatatgctacacttaatgtttgattaggttcattatgtacttcattttaagggagtaaagtttatgtcattaaaaagttcaattgcgactgcggccggtaagtcgtcttactggtttctgcatacatttttcaagggcggcagttcgcttcccggtaaaatcaccaaacggctcgatccagaaattctggcaaccctgggccgtgactacgacgtgatcgtcatcaccggtaccaacggtaaaacgctgacgaccgctctgacggttcaagtgctcaaagaaaagtacgataacattttgaccaaccccaccggctcgaacatggagcaaggcatcattaccactttccttcatgcaccaaagtcaaagggcaagcggccattggcagtgttggaagtcgatgaagccaatgtcatcatggttaccaaatacatcaaaccaaaagcgtttgttttcaccaacattttccgagatcaaatggatcgttatggcgaaatctatacgacctataataaaattttgaatggggtcgccttagcgcccaacgcaaccattatcgctaatggtgacgcgccgattttccattcaaaacaactgccgaacccgatcgtctactacggcttcgacaatcaaaaagatggcgacatcaaggcgacgcccaacacggacggcgttctctgtccccaatgtcagcatgtcctgcactaccatttcatcagctattccaatctgggcaagtacttctgccccaactgtggttttgagcggcccgaattgaattttgcgctgaacaaaatcaacgacttgacccccaaatcatctacctttgaaatcgatggtgagccgattaaaattgggatcggtggggtttacaacatctacaatgccctggcagcttattcagttggccgattcatgggagtctcccctgctcagactaagaaagcctttgaaaaaggaaaacagatctttggccgccaagaagagatcaacgttgacggcaaactggtgacactgattctggttaaaaacccggtcggcctcaatcaggtgatcgacatgatttccactgacaaggacccgtttaccttcattgggcttctcaatgccaattacgcagatgggattgataccagctggatttgggatggcgattttgaacggctgcccaagatgaacatcaaacagttcattactggcggtgagcgatacaaagatatcacctaccgcctccaagttgccggagtcgacccaaagaaacatttggttgaaccggatttggacaaagttgtcgaaatgatccccaaggcaccaaccaaaaaggtttatatcctcgcaacttacacggctatgctacacttaaggaaagtatttgcagccaaaggctttatcaagggaggaatggattaatgacctattctttaaacgtctgtcacctttacggcgatctgatgaacacttacggtgacctagggaacattttggtcctcaagtatctggccaacaaaatgggcgttgacctgacgtctgaagttgtcagcttggatcaaccatttgatcctgacaaatatgacatcgtcgtcttcggcggtggccaagatttcgaacaatcaattatttctaaagatatccaaaccaaaaagcaggctttaaccgactttattgaagataatggctccgtggtcgcaatttgtggcggctaccaattgctgggtcactactatatcggggctaacggtgaaaagctgatgggcatcggtgcattggatcactataccgacaaacaaaaggaccaccgttttattggtaacgtcgtgattgaaaatgaagaaaccggcgaaaagtatcacggctttgaaaatcatcagggaattaccttcttgggtcgcggtgaacgcccactgggaaaggttctggagggtcacggcaataacggccaggataagactgaaggggcaatttacaaaaacgtctactgcacctatttccatggtccaattcttgccagaaacaatgatattgctaaacacgttttgatgaacgcgctgaagcgaaaatatcctgacgccgatttaacagcacaagagaatctgaaagttggcgcaacattttaatatagaaatagaggctgggacaaaactaaaaattttgttccagcctctatttgcgcctgaatgttatctagcagaactgtgcgccaataagcagcttccggccgtataaggggattacccaaacatccaagttctggatattcgggtaatccccttatactctggaagctaaccgcttattgtcccacgcttattttgtctgaaaattattggtgtgcaatctcgttttctttcacaaaggttcgaatcagttggctgcgatatggcaaaaacaactggttgcttggatccgggtggactcggttggacaaaaagaccaacgccttatgcgaatagcggtcgaccacgatcagggtgcccgtgtagcctgtgtggagaatgtatggatgaccattataatgacgcaggatccagccaaacgaacgattcttcatgtgtcccggcgtttggtcaacgaagagctggtcaacccagtctgccggcagaaagttgggatatctgatatcgcccaacaaccactttgaaaaatgaatcagatcgctgagcggcgcaaacaagccggcagagccacagtcaggaccaaggattcgcgctttggggtcgtgaacggtgccgcggatcaaccccttactgggaattaattcggtcgggacaacattattaacctgatccggggtgaatgtcgcttggtttagttccaacggtcttaacacaaactcactaatcagctgttgaacaggctcgcccatcacccttgaggcaatccagcctaaaaagataaaattgtagtcttgatagtgaacaactttgccgatatctgaaccgcttttcagggccaacaacgccggcatcagttccgacttgggcagttgattgcggttagggatatagccgacaatgtctgaggtatgcgtcagcaaatgtctgatggtgacctggggcgactgccattgaggaaaatacttggtcaaggaatcatctagtgagattttcccggaagccagtagtcgtaaaattaaattggtggtcccaatcactttggtcaaggaggccagatcgtacaattcaccactgtgaagcggcaatctttccggtaacagttcctgttgaccaaaaacgtctgtttgaaggccatcccgatcaataatcccgtaactcacgccggggacaattccggcatccacaaactgatgaattcttgtgaccgtgtttggataatccatggacagcatcctttcgcattgagatgcattcattgtaccgctaatccacaactggataaagaagcgcaccggcggttgcttgaaaacattttccccactctgctcagatttgttacaataggaacgtaggatttttaagatcggaggaagttcaagtggcaagtaactcagacacaatttatcacgtcttatcatacattaaggcccatccggataaagtattcaccaagccggacacctatgacaacgtcgtggaaatgtaccttgatgacaccgttaaattaggaaatccagagatttatttccctgaacaaaaactcgaggttaatcgaatgtcgtcagattttctgtcaatgtacagtgatttgctggactattttcatgagatgacccaggtcaaagacgccaattatcacgaattgtggatcaccacctcgcatttagtagaccaacacaaatacctggttgacctgtcatttgaataaccagccaaataaaggagaccttcactttgattagcacgatgtttgatgtcattaccaagctgtcgtcttatgcgatggtgatttttttcgccatgtttgtctactttaagaccaccggcaaacacggtaaatatccatacggcaagtatgcgctgatttcattggtgctgatggctgtgttcggcacgttgttttttaattcgcccaaaggaaaagaagtcatcaaaaaaggcaatgccgagcaggctgagcggaccgaaaagaccgtgaaaaagccggccagaaagtcgactcaaaatactgaaactgccgtcaagaaagaactgaacaccacccatacgcttctatttgatcatcaagtcaagctgcatgccagccagacggcactcacagtgaccgttaccgataaaagcgatacaaccgagtcctttcggttaaccacgattggtattttgaaggcgattaaaaagaccgactatgaccgttatgatcaattcaccattatcttcaatcgaaatgttggcaacggtcggaaacgaaccattgtcaaaaccatggttaccaaacagacgctgcggaagctggatctcaacaagcttgagactaatcagttaaaatctaaggccgatgattactatgaaattaaataaaccctcactaaaatgaggcatccctccaaggaacaatttaccttggcggatgcctcatttttgattattgagttaactgataactagcttcgattaggtcgtgaatttgctttggatccacctggttcaaccgaatggctaaccagttggttttgttcatatgataagctggcagaaaccccaaactagtttgtcgaaactcaacttctttgggatccaatttgacatccaggatgtcttccttaccctgcccatcaagtccaagttgcgacttttcaacctgcatgactaagccgaaccattttcggttctccttgtgacgcagaacggcaaagctcggatactttttccacaggtattcagggtgaacatgatatttttcaatcacatagttggtaacatcttggtatttcattcgtaacctctctgattaatcaaaggattccaagtcaaggatctggtagtcatagcccatttccttcacgaattttaaaacatccttggaagcaacaaaaattgttctggtgttgacattgggatggaaggtcattgtcttttcatctaaaatggcccgatcgaaataaacatgaatattcttctcttgattgttaatcaatccaaaaatcgagacgatccccggctccaaccccatttgttctttaagtgattccgctgaggccatcttgatctgtttagtgttggtcaagtcttgaaattcatgaaagtctagacgtttggcatcgtccatcaccaacagataaaactcggttttcttcttgttggtcataaacattgttttggtccgaacgccctctttgcccttaatgaactcatcggcttcctcagtagtgtgggcagcaggatgttcaacaatctcatagggaattcccatcttatccagcgtttctttgactaacgtaaattgatccatacatatcggctcctatctgcatgaatatgcgtgaatcattaaccatttaattctagattagcacactttgggtcactgtggtgtaagcaattccaatctgggacgagtaagaacgggtaacggttaaagatccccttctgcacaggatgatagtgggatttatggaatataaaaaggtctgttacattgtctctgattagagagaaacataacagaccttgcaaaagattgggtatactggggtcgaaccagtaaattacggattcagagtccgttgccttaccatttggcgaatacccaatgaatatcacaactaaatatattaaagatttttctgcgttttgtcaactttatatttcagtttcctttgttgacaaatctttctgatttagatacactattatagtgagtttgatagcattgcccgctggtcaaactggtttaagacgtcgccctctcaaggcggagttacgggttcgagccccgtgcgggtgattatttgagtgatatggaaaaacaggaatcccttcaatgctgatataaaggcatttaaagggattttgttttctctcaaaaacatagaaatacaaaacccttgccactgatttgccactatctgaattaaaatcataagaatggcaaattagtggcaaatttcatgcttttacataattgatgccttaagttataggaatgtacacttgaatggttgaaattccaaaattatcatatcggttatgattgtcgcaataacttaaatataatattttagacaaaacaaaaaagcccacccagaacttaatctgagtgggcccttttgcatactttatttaatttctttgattaagtctacgtaatccttgttggctgttacatagccaacttgcgttttgagggagtagatgtcaccatttttaactgcgactccatagaagcgactacccttagcgaaacgcacatagcgcttgttcttatctcccttaaggggcaacttgttatacgcatgcaccatatcagctttaacttcatacaggcctttagtagcatagtattctggtttgattggtgtgtctgatttaccgtttgactttaataatcctttgaaatcataactagcatcaagcgacattcctttaaaacgatcagtgtattgccagatatccacatgattaattccgggttgtgaagtgccgtaagccgctacccataacttagcatgcttggacaactttgcttgattaatccggccttcctgaaaccatgaagtggatccataaaccattaagttgtggtagccattggcatagagatagcctagaaatttattgatgccagcagtacatttttgcggtaaatctggggcttccacatcaagtgccagccacgttgatttgtccaagcccatttttttaactttatccaggaaatattgagcttcattagtaccataatgccaaaaatgataaacaccaacaacgccataggctttataagcattggcaatttgattggcagcctttggtgaagtatatttaacaccttcacttagcttaaccattgcaccagaaacaccatgagattttaagccgttaaaaaatgaaaaggaatcggattgatatgatgacgtgtcaacgataattgaataagccattatttctcaacctcaccttccaattttgcaatatcacttgcaccgtcactttctacagtatcggtgctatctgattttgaagtatctactgtggcattcgtgttatcggttgttggttgagcatcgacttcaggcttctcttcaacaacgtcagaactaggagtagtagcaacaggggcaatatctttgcctgaacgcttgtactcttgataaatgccttcaatgagtcctttaatcaagtctgacttagcccacgtgtaaccacgatcactagcaaaagttaatgctccgttaagcacagcatcaaaacggccttgcttacttaacgctgctacctgggcatttagggcaactagtccttcaatcgcggttaaaagcgatttctcttgggcggtcttagcgtgtgcttgagcaagtggcaaagcggctttccaaacggctagaataaaagcaattcctgcagccaaaacgccagttgattgtaaatagttaaaagtcttagttaaaattgcgaacattatttggccacctcctgggtatcattttttgcaaaaccattaccagaatctgttgaagctgctggtaaggttggttcacttgataattcatctgttttgagtaatacttgaacatccgctttaaatggtgtcggtacttcatcaatcgtccggccaccatcggcaacatttgcagcaaacaaaattgaaactgtaccatactttttagttaacatttttaaattcctcctaatgaataaagtgcattaactgttgtagaatcaaataaatcacggaactcgagccaatcgcaatggtaaccaccttccacaagttctgacgattgataacttccatctcgtctttatgattttcacttttctcgtctccacggatgaccgcttccaagatacggttgttttgttcccgcaaatatttgttgctttcatcaacactctttaaagtgtcagtcattttgttgttaagatcagtaatccgacgttcgtgatccgatagttctttaccatgtttcaataacatttgatgatcctgatcgcttaaaggcatggcctcacttcccttctattttggggtaaaagaaaagccatctattttcatagacggctaattgcatatacataattttattaatagaaatatgaaactaaaaaagccttgatcctgggtattgaatcaaagcctgctgagagaccgtgtaagttgaattgtcaatcatctttaccaaataagtcggtccctcaacatagccattataacattctttgaaagttttcgggcaaaacaaaagcacctatccgtagatagatgcattttcatatacttttgggggatatatgaaaagaaaatatagatattactgaaggcgtatattctgaggaaaacatacactcgaggggtatgaataacaacagtgaatgcgctgttatccacgtgagatattataacatactttacttctgtactacagataacctgtgaagtaaattaatatgcggtaatactgtcaatgtaaagataggcatcattataatttttatatccaataaaggttgaattgttcccttcatccgttgaattgaaatatacagttgaatcattgctcttaataagtcttatcgttaagccagactctgcatatatttgcccatttgaaaagcttttaggcaagtgaatatttccactataactattatcaaaaccaactccagcagaagaaatatatattgcttttgagaagttcactactattccattttggcatttactaattgcattggacaaagtaattttcttgtttacaagaaaattattattaaaatcatcataaccaccaccaaatggatcatttatagcaaatgctttgctacctgaccataaaattgttcctattggtaggccactggagtatatttttatcccattatgataaacagattcaattttcttgcctttgtgatacaagctaataattttgttgccattgtgataaattgccattagctttcctccgtgtaatagaacccactagcatcgtttgttgatgccgtctgggcatcggaatcactatcctcaataacccactgcgcttgagtaataactggactgctatttgattgtaagccgtttgtgaagttggccattttagcggtatcagccgtagtggctggaatcaagcttggtaagtcggccgcatgcacaacttgactgtcgtcagccggagtataagtcttcccgttgactacgatagatccatcgccattgtcagttacttttttatccagctgctgattaacatcaaccgtcttggcgtaaggttgcaatgcccctgctaagtcagtatctgaaacataaatgtcatttgaattagtaaaagtgatattacttgtattgctaatattgaccttgtatgaataagtaaccgcttgcggagttacaccatcatattctggcaagtaattaggattaggagatatcgtaagtccatataatatctcattacctgaatcatctttagcatacacagcataagttttaacataaacgccatcagttaatgcttcattattaccagttgctcgaattcgagtttcgccagtgttcttatcaagagtaacttctgggttattaactacaatttcttgtggtgtaattgcagttaaagcttttatctgatcatcagttaattgactattatccatactggaaaaaacaattttgctaaaagtaatttgagtttgaccagcattaacttgatcaattaaggccttaccggaattagttaaaattcctacatttggtgttgccaattaagccatctccttaacagtaatttgtggatagaattgggcatgaactcccatataaagttgattgttaaccgtcgttgcatactgcaaatcttttaataagtattccggtggtagcattgactgaatagcattagttaaaattttacgtttgacctctgctttgtcacccgaattaaagtcaaagggaatattggtcacttcgacttcttctggattatcagtaccgttaatatcgaatatatccgtgccaatgtttaaaactgttgcaatcaaggcttttaaatcattagttgtaatgcccatatggttttccaacaattgcaaacgaacttgaaatcgtaaaaaatcatcgtcatcatctagccgattaatgccatagtccagagcaatatctgttaatgtttgcccacttgcattatttaacaaaacctgatctgatatactgagcaaatcatttttgtgttcattaagaagatcagcaatcaaatttaataagttttgattatttgattcatcttcctgattcataatcgccggaaacattgaaactaaccagtttcgtaaggtactatcggataaatccgtttcagtttgatacatttgcacacctctttagttttcaatcacgttaatcgtaatattatcagaactgataaccgctaattgaaaatcactgacactaatatccgtttctgccaatgtatcagcatttgtgcctaatttaacagcaacatcagtcacaccagcaggcgaatatccgggtccaaatagttttgaataaagaactttatcccccatattgagagtatcaaaataatttaaaatgttagtcttaatggcttgtggcccattgtcagtatcaaaaaccgtactgttaacattcaaatctaattcaatataaatcggtaccgtatcagctcgatcaaacaaaacggtatattgacgaccacctacgtccgttgccataccaattacggagccaatagtattagtctgcgggggtaaaacatcaaagaacttttgagaaatttgactatcatcaccgccaattacataaagatgaactgattttgggggatttccatagctgtctgtactcattgtattattattgaccaaacgaacatcagttactccagttaaattcttaatggcagtttgaatgccattaggcgtactattctcagcacttttacggttagctaaaattcgttgccgtagcgcatcatcagtttctgcatccatgccacctgtagctgcttgcaggttagtaactgcataaaagccatcaattgaattaactggattaacaatagttgctggcataacatttgagcccgttccggtatccatagctaccgcctgaactgtttgccggcccaagggattaccatcatcatcaatcaatggttgtgtatttccaccactatcaacatatgttgcttgttgagtaatcgtaatgtctgccaaggttgaaaacagttgaccatctggggtagaaaattgagttccttctggaatgacagttggtgaatctggatctacataaccatcaatttgcaaatacacataagcattggttgccggtttacggtaaacactaatttcagcagccaaatcatccaaatttgctccggaactttttaaaacaaaaaaggagttataaactccctgagccagactttccaacttgtcatcaacctctgataaaattccagcaatcattcctggcgtttgctcatcatctagatcaataccatcgccaaaatatttgataaacatagcattgatattgtctcgtagatcatctagttcaggacgatcatatccattagctgttagtggcatcattttcatctccttgatcatcgacgctaacattactcgtgacagtttcaccagttgtaagggtgaccgttgcttccagtgaagtaattcgctgttgttgattagctttgaatttagtaatttcaactgagtcaaaagtatcaggccattgttcttgcagatagtcagataaaattgactgaataatcccttgatcatctgcattagcaagtaattcgttgtgatcaagaccaatatcttcattccaaagcaattcagcaacattaatgttcaatagtaaactgagtttctgagcaatttcatcatcattttcgaccatattaaaagcaccagtgtttgggttaaaatccaaatcaccagtgctgtctaatccaaatgcaatcatggtttaatcaccgcctcaatcaccgcatcttgtatcgaatgcattcttttggtatcgattttgtagttgcttttaccagaccaattgtccatctcacgatcacaaaagccaacccaaacaaccgagctaattgccattggcttataaccattaagattaacatttttattagtacaaattttttgaaagaaggtgtccatttgccaaactgatgcaggaacaacaacttcagttaaagccgctcgtttatcaccatctgattgaagtggcagcggttgaacatcacaacggtgatgagccttatcatatgaaattacccgtccaattgtatgacaattaatttctgacttaaaaaattccaaaaattcatttttcaaaaaattggattgcttatttttggcatcaatcgcgacttttcttttcttaggcataaactaccacttccattttataagaatcctggtcatgagtatgatcaacactttttactctttgaagaccagtaagattggtcgacttcacataaaccgctgatccggcacaaacccgtggatcatcaaagcattctaaagtccatgtcggcttaccgtcatcatcactgttataggttggttcttgtgtcaatccatggtacatcgtgagatatagatgctcattataggggttaggcttattgccatcatcgatatataaagcacctttacgataataaaccgtgctcccacaatcttttacaattgcttgaattgcagctaaaggcttagccgataatgtatatccttttttgaaaacatgatttttctttaaattaatttctgaaatttcaatccttgcttcacgtttaatccgatcaataatttggctggctttagttccctttttgaacgtaatgttaactttgctgatctttcgtttcttgtatgaaattgactttccatcactggctttaacggtgtgagttaccattttcgaaccattaaaattactgtaaaggcgcttatcttttgaataatcgcgcccttcttcaaaagttatctgagtttccttatccataccgctttgagtctctggagcaatttgtgtgatagtaccctcggttaattttccgtagagataagtcggcccactgtaaacaatgatgtggtcattttgattaatcttggccaaatgcgcttttgataaattaaatagggttaccgtgcaggtagcaggactaccaccatcatcagagggaatatcatagttgattggtacgcccttcttttctgagagtgttagcttgttaccattatggttaataactaaagtagttgaatatccccaatagtaacccttgtttgtagttttttctgccattaatcctcaccatccggaatatcatcaatacataactgcacagtatcgcctaagtttccaagatcaatctcatcttcatttcctgactcatccattggaataatcgtttcagttggaagtcctggagcatttataccgcgccataaaggttgatttaaagtgaccacttctccaagccagattggtgtgccatctagttgataaatatctactgtaagcgattgatcaatttcattccactggaatccaaataaatagtttcctgagtctaaatcaatctcttgctgataaggaatatcatctggtgataccggaatataatcatgtactggcattattcatacctcactttcgctccaactgggatcgaattagctggccacttatttaacttttctaactcagaaacttttactcccgttttttgcgaaattgaccaataggtcatccctgttttaacggttgtcgttttatgagtggttttcttggtgccactttttttagtgcttgacgacttagtttttttctttgatttctttttagcataatcgattttggacttcatggcatacgtaaaggttattgatagtgtcaacgagttcttgttacctgtcgtgttagctgttttaccaacagaagacaggtaagcgtgtgcccacttagaaaagccacgtactgtaacctcaacgccctttctagcccaaccttgtaaaatgctaaactctgaatctaaatcactagctttgccaaataaataatacgttcctgatagttgcttggagcttcgaacactgtaattagttcgagtttctgagctatctacagcattagtcggcacatcctgctcatcagtttcggttggatctgcttcacctaagatataaactcgactagtcattgcgtctgctcgctgaattgttgttagtccattaagatacacacctttgtgtatcttatattttttcttggcagcagcaatttcatcattgattttagaccgattttgagtttgtttcttcttagtttccgcctttttattagcaacataagcattgtgataagtctgataaaccttcttatctttcgtcttttttgcattaatatcgttaatctttttcttttcaacattaatagcatgattggcttttgtgcgagcttttaactgcttttgatattcagcagtattggtaagcttagtaattgattgatagacttcttttttctgtttagttaggtctttaatggttgactcaattgattttttcttagaagatttcttggttttactcaataatttattttgcttatcaatttcgtcttgtttagcgtcataggcatctttaagactgttatacccattttgcttttgtaaataatcatcgtaagtgtctaacttatccttagccttatcaatggtacttttagcattatcaatttggtcagcatctttgctgacagttgatttccattcggttgatttcttttgcaagtatgttaaagtcttgcctttaacagaatgcgttgctgattttttggtcataccggaagtcctccttcatcattaaagccaagttgttgacgaaatttggcaaccttttcatcattcgctttattaagcacttcataaagcttgttgatcgtactatcgctcatatttccgccaccttggatagtgacattagtgcgggcatcgatggtcgcagttttcttgccattaataattttttcagaagcctcatgtgggatcatcaggccgcccgtatcaggtttaaatagttcccatcctttttcgtttacaaccgaaagctcatctttgttaatacgaccgcctttagcgtgtcccttaattgctttatatgcggcttcggcgttgctaatacgagttcttccggttgcgtcttcgttaccgcctgactcccaaccagcgaagaactttctagcagcttctgctggattagtcatccttaatactgctttaaaggctccagattcgccaggttcatgaagtgcgtattccagttgacctttggcagaatcccaagcataaccgtgtttctttaaccagttacgtaatccagtttcacgagtaaatgtccattggcctaatccagtaccatgatcagcgctatcaattgctttaggacttaagcgtgattcttgcatccagttacctagaataccagcaattccggcatcagtagcagagggataagcttgcttaagggctttcgctatttctctagctcgttgactctcatccccagcaagaccaacggcacccatatcgccattatcgccaaacttatcagctaacttagacataaatttgaagaatccgctgccaacttgtttcttaatgagcgattgaatgctattagaagctgattttttaccttttgaagcagtcttccttgctagtcctttaacctcaccaaatagcgggctatatcctggtactgaaccagagattgaatggataccaatatctggatggccattaggtgcaaatgctgaccaatatttatttccaccagcaaagactccaacgtgtttaccagggccccagaaaaccaagtcacctggtttagcgtttgaacgactaatgtgcttcgttttaccgtattgagcaccagaaaagtggggataatcaatgccaaaggcatgttttagagcatacataacaagtccagaacaatcaaatgtgttaggacccgcagcgccccaaacatatcttttaccacggccatacttttcaacggcggccagtagtccggtagcatcaccgccactgcctccatccagattaaccattccccaaagagacttccaccaattagtagccgaggatttcaccttaccaaaaaagccattggcaaagtctgataaaacagttcccttgccagatggctttttaagcagtccagttaaatatttacttggatctttaacgattgacttaacggtatcaaatactttcttagtggccttaagaatgccaccagcgaagccaccaatcgctccgattcctttttcaacgccaccaacaaccgatgaaccaatgttcttagcaccactccataggttaccagtgactttcttgacgccattccatagtccaccagtagcaaaatgctgaattccattcagtgataaggcaaactttgtttcagaagcattcaaaatttcggctccgggttcaatcaatcgtttaacgtcagtgcctttaatcaactcactcataccattaggatgaatcagcatttcacgattaccggtttcgggtgagtcgtggccatcatttagcattgctaaagttggcttagtaatctcacggcgttgattcccaaacacacctgtaccattggcaaagtgaacgtagccaatcttgccgattgctgtacttgaaccaccaaacatgtggataactccatcaattaaaccaatgccatcatttagaacttttatgatgtcgttgataccattctgaacgtgcttaacaatccctttccaaagattactaaaccaatcatcaatcccattccagaaatctttccatcccttgccgatatctttccaagcatttttaaagaaactaattatatcgccaagcttacccccggttagtttattcacccaatcaaacccagtcttaaataaatctttaacatcgttccaaaagtttttggttagcttaccaatatctttaccaagtcgaccccatttaccagtaaacacgtcaacaattacttgaataaggctcttgatagtacgccaagcgtccttaattattttggccatatccttgaatagccaaccccaacgcttattgacatctttgaccaaataattaatatatttacgaacgccattggctagctttccaaaccatttagttacgccttcccaagctttcttagcccatgaaattaaaccgttgacaaatttgcgaaacttcttgttgtgcttatataattcatacaaggctgcaccaacggcaatagcacctgtgataattgcgatgaaaggattagcttttaagaagttaaacgccagcttgaatccttttccggttgcaatggcagccgtcttaatgactgataatcctttaactacacctttataagcaagcttagctgtccacttaagactcttgtcaattgctctacttgttgctttagtagctgcccacaatcctctggtagcggctttggcctctttccaaccaatacttgcagtccacttgaggcttttgccaattcctctagcagtacctcgaatcgcttttgcaaataacgttaactctttttcaccgctttttccattaactctaggtttaagaatcaagccgctcttttcgccaaaccctaaaaagttttttgttgcagagacccctttcatagctttcgatgtagcccaaattccagctaacaacttaccaatatcctctaaacctttcttatgggtagtaatactttttagtgcatctgaaaagttatgaatctttttgctgttaccagctagtttccctattggagtcacaatggcactcaatcctgaaactaggcccttagcaaaaccaacactaatatcctttataatcttaacggtatagtataaacttttaaagaactcaacaattgacttagcatggtgagcaattgtatcagaaacattggtaacacccttagcaatactattcatcacatcattagccaaatgagggctttctttaggattaaatactttagcaaaagattgcgtaatagtatttaatcctttagaagcatctgttccaactttagtaaattccttttcagtctttctgtcagaaacccacttagagattgcgccaaagattggattcttcgctttcataaaaggtttttcgagtgcaccaaataacgctgctcctcgagcagacataactcgttccatccctggaagagttttcatcatgttttcagaagcctcagcatattttttgcccaatgaattcataacattttcggcatctttggcactgatcttaccagcagtcatattctttcgcaattgactcattgtaagatgggaattatccattgccttacgttcataggctagtagctttgatccaaacattggcaactgatctgaaatcatgttgaagtcacctaactgcattttagatgaagccatcatgtgtgtgaagttgagccctaagcgctttgtattttcagcacccatgcctaaagtatcagccattgtcaaaacagacttggtcagacgatcagttgggccttgtttgtctaggacgtgatagaactgctggttcaactcattcactaatccagctgattgaccaaaggaaactgacatgctattaatagctttaaccatgcgattacctttaacagatgaatcagttaaagtgtcccatgtggcatgcataacttgttgctctttgtcatactcttcacccgctttaagtgcagaccctattcccgatttcaaagaataccaagtgttaattgccgcgttagaaataaagctggccgtcacaacatctctcaaaaaatgagtccccttatggacttcatcaaatgtttttttagctgaatcatgtaacttactaaatgaaccgttcgactcagaagatccactacgcaattttcgaaacatttcactaaatttattgcctgattggtcagccgattttgccaattttttaacttcttcagcactcttattaatatcgctattcagtcctgaattcagcttgatttttttggcggcatcactcgtatacttaaattcttgctgcattttatgaacattttcagtgacctggtttgtttcattctttgcagaatccatactgtgataaacgtcttggattgcatcacgagtctttctgacttcgtcactactcttaccaccaaagccactaaaattatttttgaatttatcagtaattcgtgaggcttctttcattgtctcgaggaaatcatccatcatgctgttagctcgtttgaaatcatccatgccattcatgttgagatcaaggccaatacccgcatgacgaacttcttttgcttcagccattactatttacctcctttctaattaatttgcttatgttgaactccttagtgggataattgggttattccaacgaagggtggtgataaaaatggcttttgtaaatccggattcgtttgctaacgcagttcttgcttcaagaaaggataaagtttctctggaagatgctttagaattctacgagcaagctgtcaaaattgctcaagtgcataacgcaaaagaaccaaagggcaattttgaagatgctgacttatcatttgaagagcaagatcagctattgcgcgataagggaattatcgattagtcattgtggaaaggagtgggacctaatcctgctcctttttgctctcaaaaagagttttggcactgtagttattgtctaggagcttgatactattcatgatatttctatctagaacactgttttcgtttccgtatacgtttattagaatcaataacctaagcagtcgattagtccgtttaagctccataattacatcatccttggcactcatttgctcaccttctttcagctacaatgtctatcgtcgaattctctaatgcatactcccacgaagctcgttcaaaatccttgttgactaacttcgggccctaaccagagcatcgtgcaacatattcttggtaatgacgttcatactcttgcttggaaacgggactgcctttgaatgttaacccagtaaaaatagacttatgtttgtgattttggaaatctttactttctggaatcgcatttttttgcacatcatactctgcctccttaaattcttgcctctgtcaaaactagattcaacaacaaacaataatctcggttaatcttcaaatacgatgctgtagcctttcttcagaattacatcgttgaatgaaacactggcgataagttcattgccatgaactttatcgacaatattaatgctggaacagtctttcccatccaaatgaattggctgctccatttttttgactttaaccatttattttcctttctttttcccaaacatttcatttaatattttagccatgccgtaatacacaccttgggcaataaccgattccttttcttgtcgaactaatttagctttagctcgattaaaaatatactcatcttgggtcatcaaattaatctgatcttcgctaattcctaattcagttgacataaccagaaaatctttattgatctcatcctctgccaaccgatcatcgattttaccaaattcattaacatatttggaattactttggtcgtaacgttgttgcaagaaagcgaaacgattccatcaaaatatttagcaggccgtttcgtgccaatagcgtcccaagatatgcttgtgcttcacttaaagcagtagcacccaagccagaaccatgttcaccaatattccaatacttcatcttaacaatttccggtgtggtttcatcagtacgcaaaacttccttgttaagagaaaccagggtgtcgtgcatattgagtgccccagaagggcggttagtcatcatgaagatctgtaaggctgttcgataatccggaaagaccatattaatctttacatcgtcaccattgctattttgcttaataacggttttcttagttaatttttctggcagttcatgattcaaaacgccataatccaaatgcggactaaccaagacgttttgcatcaacatctcaaatgccttaccgtaatcagaattatcgccaccgacattcattaaatccatgatttgagtagctactccaatacctggatcctgcaaagtgatctttgttgtgtgttttttatccttgtcgtctgtccattcaaccgttttatgaatctcattgcccatcaaggcttcgagctttttttcattattttccattttaatttactccttatgtagagggccaccgcagcggtagccccctgttccattttaatttaagaaaacattgaatcgtctggctggttaccagtgttttgatagtaaccaactaataccgtccaagccaatgaatatgctgcttcattgccttggttagctggcaaaccggcgagtcggcagccttctgcggtaatcttttctccagttgatgcattaacaatattcaacccgaacaaatcatcagcggtcattgggccatcttccattaagtcatgctgagcatgatacatatagaacagaatatctgtcgtagatgttcctgggtaggtgtttaaggtaatcgttccagtttcatcttctgtatcaaagaacataacattcgaatgaaaatcgccttgcatagtagtatcagcatttgttctctgtgagctaaatggttcaccgttttgaaaaccgccaagctctttagattgattcttccacagcaaataaatgtgaaggaaacgagccgaatataggttaacttctttaccattggataatgtaattgccattagttatttccctccctttacaaagtcaaatcaagtttggcattaattgtattaatgtcatcagcaatttgagtgttcaaactaaacccattatatttacgggcggcaacgtcactgtttaacacgttggctcgaggaacactattaacgacaatcgccgtgtacagcacacccatttgtaataggcttgtgctgacggcgttgatagtttgtgtcatctctttgattgttgcatcattgtaaattgggaaatttttacggttaagatatttctgcaagttagtttgcaatgtatcaatcactaactgagtatgaacaaattgatcaatgtaattgccagcgagtgctttaccatttaacagcatataatcgccagccttattaacgaccaaagtggcattcaagccagcaattgtatcataatcatcggttgttaaatcagcatctggttcaaactgtgaaagattaccaatatgctgaaaatcaactggtaagttagcagcggcgtacgctactgcctgagcagcagggtagcgatccgtagctgtttcaacaattgcagcagtgttgcctaactggttctttactgtttgatagccagcaacatgagttgctaacgtttgcagtgcggtaaccgagtttggttgagttaccaacataattctttggttgtcatatagaaaatcagaaagcgcttcgatctcagtctcggttgctccgtcaagtactaaatatttaaaaccatcaaatagatgctgggcaattccaacaacaattcccggtgttgtggtagccgtaaccgtaccaccggtagttgttccttgagattgaacccctgaaggtgtattggaatccacattcggacacgcaataacttcaacaggcccattaaagccattaacatcaaacatagctgctgcttgagcatagacacctgtgttttctgcataatctgccgataaactatctaagtcatcataaatgttgctcttggtagtggcatcggtattttttgtagcaattgctactgatggagcgctatttggattagttaaggcatgaatagcgacaatgaaatgtacatcagtggtttgtttaacaatatctgacactatgattcagctcctttttttatattaaattctggattaacactagcaatatttcctgtttgcgtctgatcagtgaagttgtcttgaactccaaacgtataatcagctcccgccgtgaattgccaatcaacatctaaatattgatcaactggtggaatagcatcacagtctttagccacaatgcctttttgaagcaaatcatattcaggctgctgtagaaaaaacaattttcgtaactgatgtcctaatgatttagcttccatttcatcatttgaaatagctttaaattgaacatgcaaatcaaacgtttcgttttccacatcgttaaacaatacccgatcatagtcatcgtatatcttataagtaatatagggatacgctggcgaagcattgttgacactttgcggacgtacgggaacattagggaaatattgcttaatctcgacaaccaaggcggccgagaaagcatgataaaaatcgttactcatcagtaccaacctcttttatctgatagtaagtcattccagcagatagatcgtccgcatgattgactacttcatacttagccccgctagctcgttgaacgagcgttcccttaggacaagctaccatatgagataaccaatataacgtaccaaccggtaattgtccgccatcttcttgactgtacgtcatgttaggattagtggtattagtgataacttcggaaacgtgatagacctcatctggtcccataattggtttcccaagatcatctgtttcaccggtatcttttccaataacagtaatcgttaggtcttcagctaactgatcattcataaaagcaaagttgttaaagttctgaaacgccatgattacttaccggtagttgcttgggtaccagttgcatctgaggcttgggcggtgctctgatcactcaagcttacgtccccaccgacagaagttggtgttacttgaacattaccgggggttgattcacctgcaacggtaaatcctggtacagcaataaattggcctaagaatttttgggtatccggatcataaaaggcagcatagtattttccatcgggaacactatcgccagcatcataaccaataatatgaaccacatagggagcagaagtgctaggcaaaaatgcaatattgtctgatgtttctgtgctacggtccggttttacataagctccgctattgtctttagcagcttctacaacaactaattctttactcataaaatcaaatcctttctgtaatccaatgaatagagtcgcgtaactcgcccttttcaatcaatggatcatcaaatcctttgtttgcaattgtcaacggtgcatttttgggtttactaaactcttttatagttcgcttaatatcttcaacaacggcatcgcctaaaacaggaaaaacgtcctgataatttatctctccaacaaatactttaaatgccaaatcagccgctagttcggtccaattatcaaggtagtggtcaaacgtgtaacgtaaaaaaggacgcggtggaatatgcacctcatcctttaatatgaacatcactcgcattccataaggttgcgatttatctggaaccgccaaaacatgattatgtggtggcttgggccgaaaaagattagcaatctctccaggcttacgccctttagcttctttagttggaatgattagatatgctttattcttaggcttaatactctgataagcatctgctatgctatcgtccgccccatattcattaaccaaagctatcatgtttaaacgactgttagtccagggcaccccaatggataatctgacactctgcaacttttccagctgttcaatgccgactggtaaattattaaagtcttctgtcattctgtccacacggctcccagattgtctgaaacaccataatcatcaactacttggtcatactcttgtaagtagggatcaacaccattgaagttaaccatagtttgggtattgccaaaagtaccagcagactgtacaccaccatagttcataaaccagtctgtatataataaatgacgcgtccaggcaataattcccctagctaacgcgtcatcactaacttgatcatgctgagcttttgcgattgcatcatcaattctttcggtaatatggtcatcactgaagttttgaaaaattttataatcgcttttaacatcagcaattgtaggtgtttcagccattgctaattacctcctatttaccagatccgctggttgatgagctagatgagctacctgatgctttagctttaggtgaattgatagttgggacaacataatcagttcctactttaaaaccatatttaactaattgaatgttacgtgggtcataggatacttggaataacggcttagttcctgctgccaagtcagctaaataagtgtcaggtttagtttgagtcaagtcaacatctgttccggcaacgtggcaagtaactactcgtttttgaataattgctaccatgccgcccttttgaaattcgtcacgttgaacaactaggccattagtcggagtagcagttgcataatcaatggctccagggccgaagatgagtgcataagtagttccatcagaagcaaccggaatgctatcatcttgaatgatgctcataccttgataagtggcaattggagtagctgcgccagcaggttgcagatattcaatcaattgttgttcacgcatttctgaataagctgctgagttaacaactaatgtcgataaggtgttatccattacatcacccatgcgggcgagcgccttaacgaaatctgaggcggataattctttttcagaacccacaccataagtcttggcagtcgcgatatcagtattgttaaaagtggctttcacagtttccagcaaaatctttgtatcttggcgagtccaccagttgccaaagcgattagcaatctgctgttgggtacttgcaccagaaattaaatctccccagtcagtattaccgaatgacttgctttgatacatcttaatgccgtattcaatagccgaatcaacaccattagtttgaatatcgttagtatcattccattcatctgcatcaccgcttaaatcattcattgcagggatctcaactgatcgtcctggttgaagcaatcggccacctaatactggatcgttttttagaacaccagattgaacaaagcgattagtttgagtattttgacgatagatccagtctaaaaagactgttggttcaattaaattactaaaattggtagggtttccgttaattacggtcattacctacacctcctatttaagtttgttgtacaaatctgggttttgacgataaaggttagtctgctcttctaagctcatctgtgcaaaatcttcgcgtgtcatagaagcgttaaattgttgaccgccattctgtggtgattgattacccgtaactttcttttcgacagcttcctgaactgctttgttaaataagtttgtaaacttatctaagttattgttacgaacatcttctttaacatcactaataaactccgcaaattcagctggaatgtgcttgtcagttagaacagttttagttgcagctaaagcattcttacgatcagcttcatctaatttctcttgaaggcgatcttgctgctccttcagagcttgtcgttgctcttctaaatcggcttgggccttctcactagcattcatgccggcgcgtttttcacctttttcaagccattcttgttccttttgcttaagctccttttcaaaatcatcctgcagattactttcaacttctttagctttagcagccatcatttttccgatatcatcctgtgtataggttttaccagatggcttgggatctttaggatcttgagcaggatcgttagttgttggctttggatcagttggttcagggtcattacttggatcagcaaagaattgcaaattagttttcattgtcaaaactccttttttaagtccatagactgaattgtttgtaagtgcaataactagatcgattattctttaacgcctgtaattgagaaaaaggcaatccaaaaattcctattttaaaagaacggcacaatcgaataacttgtatacaaatattcagttgcgtataatcagatttagaaggatgcaatttagataatggaggatttcatatgaaaagatttggactttggtcaaaaatatcaattatcatttctatatctcaacttctattagccatttttaaagaaattcaaaactataacgactctaaaaagcatccttcaaaaaataagaaaggatgatgttttatgcattggttatgggttttaattattggtgccatcattggtgccattgctggagcaattactagtaaaggaaagtcaatggggtggattgctaatattattgctgggttaattggttcttctattggagaagctatactaggatcttggggtcctcaattagccggaatggcaatcgttccttcaatcattggggcagtagttgttgttgccgtagtgtctttctttgtcggtaaatccaagagttaacttttatgttttggttgagacatttattaacaagtcagtacctcaatcaagttattatgagtgaattaaattactgatattcatggtccatatagtttaaaactatgtggacttttttattctttaaatacacgatcgagctcaccgggcaacacgtttccatcttcatcgcacttaactaactggcaacgacaattgagatgtgtgtcatcctgaggaattggtgcctgcccacggataaagatttgtttatccaggtctttacattggtcacaaactttataatcctcttttgttaaccaaataacatacttaacattttgttcatcataagccttatttttgccagagtttgtattttcgattccttgggaagttgttaaagtatgaattctggatagcattttgttcataggtgttgctagattgtcattaattcgatcaccactttgaggaatactgcgggtcattttattgatgtctgattttttcatgccgcgactcaatcccttgttcagggtttctttcattcgtgtcgtcatgacgtcgccatgcacccaaattcgttgagaatactcagcttggttggctactttagccggaaccgttgttaacttattagggctagagtcctcatatccgttgatgtactgctgcttaagttcattaacggcaaatgattcactgtttgctgtagcaatactcataccggcgccaatcatcgcacccaacatatcacgccgagaaatagatgcttgggcaaagattgcttgcaagcgtttagacaatttatcactaggactagcgttagctagcatttcatcaattgcttggtaaaagctctgaatatcccaggaattaacctgttgagacacttgattaagagttaaaccattatcatcagcatattcgttataaaactcttggagatgattaccaatgatacttaaggcctgctgataaaaaccgtcaatcgtctgattgttgcggttgtcccgttgaatcagtttgttgatcttcttgcgctcctgcttgatcgttgtcatcatcatcacccgatccgttgttcatcttagcttgtacattcgccattattgtggcggtccgatcatcttgctgagctccctcatcatcagatctttcttgttcctgaacagcagggatcccagtaatgggttcggctaattcacgcaatgtttgtgcagagaacttgccagtttgattcagaccttgaattaatgtcatggtttcttggttattcttcggtaagtttggtgtaaacgtaatggttacattgtcagctggattacagtcattcgtaactttgatacctgtgcttgaaacatagttccaataaatcgccaatagtcgtagccgtcttctcaaacctcgctgataaagagtttccgacattgacatttcctgatcagatccccacagtttataagccatagcaacgccagacgcattggctgcaaagttctgatctgttgtatctggtgtgttagtgtctttatgaatatcagataacaactgctgaatataaatctgccactcagcagcattcaatgatttggttaaatacgatgctgaagtattacttatggttggcgaaccgttaggattatcatgcatgtagggctttaggtaaagcacgttagcttttgtatccaaaactttctgaaccataactggcgcattaggtttgccatttgtcgttgattgatttgtataacctccactaacgttatcaagatataccggctgacctttaggatctaacatttgttcagtcttaccagaatgattagcaactttcccattaatcatcaacattgcgttactgaaatcttcctgtgagttagccatttcagatagcgcttgatcataggcatcaatttcatctaatttagtttcccacgcaccgacccgttcctcattcaatcgatattcagttaatgggacttgttggaaatagtgtccttcatcgctagttaatttccaatcagaatcaggattggcaccagcagtaaagtgatagatgtggttgtcggtgtatacctcaatttgataatacgtttcatcagcaacgttcacggcataataacgaacagcaaataactcaactggttcaacatctgtcgaccaaacaacaaacgcgctgttagggtcaatcgccgtaatcttaggttgcttagttccttcaggtacatacagtaattcatatgcccgcccaacatttgccaaatttttacccataatcttttcatgatatggttcatcattagtttgattaaaatcatcaacagcctgaataacattttcaccagtgtcgttttcatcatctttattttgataaccaaaagtcagcggtgttccaaactcataaccaacttggatgttggtaatatatcgtgctaaagcgcttgatatccgattatcagcccgattagaacgcttattagacaaccaatagtgaatgttattatcagctaaataataacgttccagctccaagattcggggcagttgattattaaagtgatcgctgacgtaccattgcactaacttttgaaatttactttgatcgtctttaattggcttccatgaagacgccggaatgttgtacgactgattagtttgaaatgcatatcgattaccataacgttggccgtttaataagttaatggagtttggctgtggattgattgaacgataatgtgctgataaatcatttgtttccgccactgtcatttaccttactttcatcgtttttgtgtaattcacaatatttatgagcaaatttaacggccaacaactttttggagtcattgaccggtttgtctttttcattaatattgtcattcactaattttgctaaactttcaaatattattttgacatccaaaccaattggaatggaataagttatgccacgatctttaaattcaagcggctttccattaagcatcggctcaaacacattcatatccattggtgccgtttgcttagttgttgcttgttttttccattcttccattgtcattaactttgacattttcatcactcctaaaataaatcatcgggataatcgatcaatcctttgtcagcgagcagttgatcttgctgatcataattatcgtgtggctgattatattcatgattccattgacgtgttgcaatcgcgtaacgaatagcatccatcacgtggtcatgttctttgactggttcacccgttttgtcattccaaacatactgataaacctcatctaagaactgctgtatgccttcttgaacggccataaacttatgctgcttgataagccctgcaacttgttcaatgccctttaaaactgatttatacgcatactgagcattaatgttattttctttgaacttgtcaatgtgttcaactcgggccgtatcacaataaaacggtatattgtagccataatcttgttgaacctgcttggcaatcttgacccagtgcataatctgctccaaatgaccagtatgctcttcaactaagtaagtattaccatcagtatcgtcagccaatacaacaattgacgtatcgtgttcgtatccccagtcaacaccgcagtaatatgttagctgctgatcagcagtccgtttatcaaactcggcacgggtaattatattctttgacttgtcaaagtcctgataaactaatccttcaccggcaacccacaaaccgagtatcttacggtcatagaacatgccagatggtgttgttgatttttggccagctacgtattccggatccaatgaggtgttatcgtccattataaagtgattactaatgatttcgttagaatgcttcggattatctatataatccgttttgagccaatgtgtgggcacatcagtgttagtatcacaaacaactcgtgcacctggtgtagaacatcgtgatcggatctcttcgaatacttctttattggcaagtgaggcttcattaatgtaggctccaaacgaagtcattccacgaatagcacccaatccagatatagagcctgtaaacgtctgcactattttgactgccggtaaaccagggaatcgaattttgaatgaattatgcttatcaaatttgaaagtcaacccaaatgtattggctatctcggtcaagatgttattggcaattgacttgcttgaaaccccagccagaatgtacattggatatttaactttcttagatcgtgcaatttcggcggcatgtttaacctcatagagaaaaacaaaattatcgacaaaggttttaccagcacgaacagcaccataattaatcatcaatttccagtgttgattattcagttcttgatttaaaacctgctgttgcttcttagtaaatagatcgtcaactgtcatctttgtcacccccttggcacgttcttagcaagtttgctcatcatgtcggttaatgcatccatctgatcgtctttatcatcttcaagatctgccaacttggtttcagcaatttcagcctcagcattagctttgcggatcttagcattcgttaactccccatcatcggctttgagcttaccggccatctgcaaaactagttgggccgctgctacctgatctttaaccgttggcggcccagtatatgttttgtcactagtcagtttctgctttaaatgatcataagtagtcaaacgatgctttgaggatataccagcagccgtttttaataagttagcaatcaccatatccgttgttatctcagtttctgcttcggccttaccagtcttcctgtgaatgaattgttgaattccaatattttccaataaaaattttgttgcattcctagcgtaagccttagagtagtctgcatttatagctgattgataagcattattagttttaatatattcgttagcaaatttgcgttgctttggtgttaatttacgtttagacattacatatcaccacacctccatttagttattctatgtattaaaaagcactgccgttaagcaatgttatcggttttattcctaagttttaactcattcaatcgtcgagctgctaaactcttacgtttgcgatctttaattttggactttttatggctctttgtatgcttgttgtgtttactcaatagtaaaaatcctccattcaaagcatcaaattgtttgcaattatttaattactttaagataatgtatgtgtaccataaaataactaaggagatgttatttatgagtttaaaagataaagcagacagtgctaaagataaggtaagcggtaaagctaaagaagttgaaggtaaagttaccggtgacaaagctagagaagctgaaggtaagggccaaggcattctcggcaaagccaaggataaattatccgatgccaaggaaaccgttaaggacacagttgatgacattaagaaaaaagcagataaggacaagtaatttatcaatttcaggcgagtcttctaaccaggcttgcctgtttttttgtgcaaattaaaagcgccctctttgcgaagacgcttctttaagtctttgtccagttgcttgtctatctgtatttcttccttagaagtgtagccatagctggtttgcttcatgggcgtatatggatgcttacgatcactcatcagtaccaccagcccctataacggccatattcagcaatcaccgctggcaacaacatgaccagaattaaaatcattaatgtggccacattgccacctccaatttatgtatcaaaaaagcccacgttttccgccgcaggcatcatgtaactcactacagttcaagttctagacaacacaacatacaagtttttgtttttgcgtgagctgcatgttcgttgactggacgggtactactcattaatttttaggaagaatttactttgatacaagtccaatcaacaacgtggctggcagggaatcgaaccctgcacggtaatctttccgccctcttcgtacgtatacgttacagtcacacatctaaggaaagagagtgaaactcttttaacaaattccacaataccaatatacctcataaatccgtataaatagtccgatcatagtccactttgagtctggtttgagtctgatttataaatatgtaaatcatccaaaagatacgcatcagcaaattggagtaatgcaccgggcttaatgtggtcaaagtagtgtgaacgagaatagccaatggacatgtagcacattgtatccgtataattatctaaatatcgcatactcaaaagctctttgccgacgttgttgcatctaccaattgcttcaaccgttcttttaacaatttgctgagcgtatgctcttcgaacaattgttgtatcagcattattcagtgtggttggtgattttggcattccatccatcgtcggagatttcaagtctgcaatcattgcgtcatagttggctgaagttagcccacttatccttagcattcttggaaatacactgcccaagaaatgcttacaattctcaaccgttttatctttatcaatttgtggaaacaagctatccatttggttatccaagcccgacaccccttctaataagccttagttgatgttataatgaagttgcctatttgttagcatcaccttggctcccggaaacgggagtttttttatttacgcttaatcaataattcaggaaccttgtcaaaatcatatttataacaaaccggctcactatatccattgaaatagacagcaattactgatccattatccacaactctttgaattgaatccgtattgacccattccatatctccaaaagttattccctgtaatttaatccaccgaactctattagtttcgctataattgtacatttcatttttcctccactctgtcataagtttcttcaaaaatatctggcttggatggataaatttcaccgtgtacaccttggatgatgtaatcaccacgattagcaatatgatccccttcgagagttttgataaccaacttaacgtttggcgttccttcatagatgaaagccgctattccattcttaagcgccttgataatccattctggatcttctaattgttcttgatctgctgtccatttaaatgcttcaattacaactggtttcttttgatatttcattttatttttcctccacatcctgaaatgccttaacaacgtaatcagtaaactctttgcgattagcagcaatgtttctatttaatctcgttggtctaatcaactcgttaccatcgccaagatcttcaatatcaataagagtatcgtcagctatttcacgtgcagtagtatatccatccatattttctggtaataagacatcttctatataatctttagtttcttgcagtaacatttagatcaccccatatagtatccttgcttaacggcatcttcccattcgcttctaatccaaatatcttggaatttattaatacttccgtagcaatccactttgccatttacatggatccaatccaatttagaatacttacccattgcttgcttttctttatctgataagggtgttactgtccatcctggttgaatgtaatgctctagtaaattcattcatctacctccaaattaacttgtgccaaccagtcattgactcttgccgtcgcttagccttctcaaaccgatcaagagactgctgtttcaaacgtgcttcaacatcttgcccaatcttatactttttagccttcaatcgtttctgatgcttaatccttttcaagtcccatctgctcatttatctgcctcccgagattcaagaaggcgtaacattccagtaatggcactcaaaccattcttggtaaaccgcatttgaatagccttatctttcttacgaggatacttttgattcataataaaggtaaaggtaccatctgaatttggctgaattccaaaagtgctttcaataatccctttttctgacattgcttcatattcaaactggctcatttctctacctccagtaactcgtcagaaatttcgtcatcagttaatttatgcactgaaatctgtttaacatcattttgaactgatcgtttaccccgatcgccaacataagtaaccacttcgtcaactcgataatactcaaaatttccgtcatcaattttaattttgatgttgccacccttggtaatatctggcaaatactgtttgttgatacggaattcatttattgaactaatcacaaagcttaaaccaagaagaacaaagaataataaacctagtcctgcaaacacataacccacattacttatcattttctacctccaataattccggatttttgtgaatgtctcctataacttcaagtattttgcctgctccaatagatccaaaataatagttaccaacaagaaaacatccagacttataattaattagcatctgttgtccttgttcattttgaacaatatcattttcgtaaatatctttaccattcttatcttttaaactggtgaattgttcaagaacaaagttattagtcatttttttatgataagcatcaacgttttgaatatcccctccatcatcccagctaatttcagttggccaatccataacttgatcctccttatcccacgctctaaatttaatttctctgctcatctttgccatcctcctcgtctaatttttcaaacaattttggcatttttgaatacatattcaatgatttttgataatcttcatcgctcattttttcatccaaatttacatgaaatcttgcagatgtctgaataccatatcgacgatagacttcatcaaataggtctcttttggttttcatttgtctgcctccttagtgtttcatcgcccacgctttaagcatgttcataaacttggtatattgctcaagtggcacatcaaccttatctctactgtcaccagcaaaatatatagcaaaagtatttcctgtagttttagttacaaagctaactttgctaagtaaaatagcttgttggccgttttcatcttcgtattcaaacatttaatcatcctccacaaattcaaagtgtggatcatttttatcaaactttggcaaccattctgggtatttctgttgaagtttatcgtattcggattgagtaaaaagggtacctgcctcatcgccaaatatggttatatcattcgattcatcatctaaatataaatagcaacctaaatacccagtactttcgggaaacatctttacccgaaacttaggctcatccgcgcgctcatcaatcggtgtccgggaatacttgtaggctagtttttgcaaggcaagcaagctatcaggctctaaatatgttgcgtcatcgtaataactcataagcccgcactggtaatttttgattaaaagtatccatccatgatcttttgtccctattatcgttgcattattgtctacataaacccgataacccaggtcttcaactttacttttcaattcactaaatttcattttttgttcctccattaattgctccgatacttgtgtagttccgttctcaattcggtttcgtgtttaacaaccttcttagactcaattcgtatgattatcatctcttcaggcaagaccggagtattggcaaccccgtgtttatcagtcaccttggcaggcttctgaaaagatgggtaatcatgctgaagctggcgtaataagtccgcccttgttggccccttggcatatgttttgtgactcttaatgccgattaatttgataattacatctccccgtcgatttcattcatccgttttctggtcataatgttaaggctaattaggtcatcttctgacaacctaaccggtttaatgtggtacttctcaataaagctcttagcacctaattgatgcctttccgtgtgatgcttacggcagagacattcaaaatacagctttcggtggtcaaccaatgcacgatttcggcggccaaccggcgtaaaatgatcaatatcgctgtgcggctggccacagatcacacattttcggtatcttaaacattggacagccaagtgataatcggtggggatctgatcccacgtttttgtcttaaacggaatatcattggcaaaacagaagtctaagatgaatgtcaggaacttatttgctgtgtccatactgcaatctgccattgagaaagcctctgagccagtttgggcatagtagtaatactttatccactgctccatatcacgtaacatcgcaaatatcttcttgcgttgatccggtgaaattttccggccatcatcaatgtctaagtacacggttggctgttgatggctggcaaaccggtttagccgatacatattcagttcatcatcaagtttaatcgtgacttcatcgcccttgattccttgcagcttgccaaacatataatcacctcagtcaaaatggcatatcttcatcggtaatctcaattgaatcattactgcttgcaaatggatcattgcttcgctggttgttcgaccgttctggctttgaacgatgtggtaaatcgaagtcgttcacgctcaactccaggctaaactgtggttcgccttgttgattcgtccattggttgattgaccactgaccggacaaagccacgttgtcaccttggtggaagtatttcatgatggtatcagaacgctttccaaagacggagcatcgcacccaatctactccgtaattaccatttcgatctggtcgtttctgccgaaccgccactgtgaaatcagctacttggttgtttcctacctgcctggcttgtggatctttgcccacgttgccagtgattgacataattcgcataataatctctccaatcatgccatatactcaggtgaatgatgagcttgctgttgctcatccagattctccagccggtatatcagcactagtttttttaaatccttcaaatcattgataaaatccacatcaccgtacttgtcgttcatggcgtcaagataacgtttcttgtcctcaatcaaccgacaatgctgttgcttttcgattgtagccacctcaattgctttgtagatgtacttcgctcgttcattctcacaatccgctaactgctgtgaatcctgaagcacgtgaatgcgcttggtatacaatgcagcctgtttgagtagaatggctaccgctttggtaatgtgcagatcctctttggtaaacaactcttttaattcttgattattcatgtactgcatgtgggctcacctcagcaatcttttgtaaatctttctggaaatagaacttcaacaaaccagtttcaccatcacgattcttcttgatcgataagttcaagttaggatcatccaggtcatcacttggccgccacaggaaaccaaccacgtttgcgtcttgctcaatggcaccggtttcccgcaagtcgcttaaatttggctcgttgctttggcgagattcaacccctcgattaagttgactgagcgcaataattggaatttgcaagttctgggtcaacaatttcaaccgccgggaaacttcttccagtgcttgacgggtatcttcacgtggattgctggtctccacaagcccaatgtgatcgacaatcgccaagtagcggctagttttgcatcggtgagcgtgctgtttaatcacactgctgatgtcgtcaatggtggccacccgatcgtttgaccagaagcgaatgccagcaatttgcttaatcgtattggcagcgacttccttttggctctcactcatccgcacagctggatttttccaaagattcaacggaattccagacgtggcggcatacacgcgccgcatattctgcttggaactcatctctagggagaataattcaactgtcaaacttggatcacccaggatggcgttggttgccaggttcaaagcaaaagctgttttcccaactgacggacgtgccccaattacaattagctcgttcggtaccaggccaccacccagatacttatcaagccctggataggttttgataaacgaagtattgggcgtattcaaatcccgcagagcctcttcaacctgcttgctggcgtcaatgtcagcatgagtatcggtttgctcagcctgcttacgaatatcaagcaaatgttcaaagttaaattcgctgggatctttagccacattgatagcggcgcctttcatcatgccaatgtaataagcctggcgtaattgtttgaaggtagcttctgggtctagtggccgatcgaccccttgaattgaccggaagatcctttgaacatccagcttcttgccaaacggggtatcaccaaaagctgccgctatctgttcagcattctcgtagcgggtgccccacaagttgacatagcttgcaagagtccggtaagcattgttggtaaaccatttctcgtcgaccgtgtttgattccaggacttgcggttggttaatcaggaaccacatcgccttacgctcaatctctggcatgtttctgttagtgcccatcatcaacacctcctgctgctaaatagagttctggatgcagtattcgctcggcctcggctttagtgacttgcgggtactcagcctggataattggcatcgcctcgtcaagatcatttccggtctcggaatacttgtagagaacgaatttgtcacggtctctcagccactttttatgctcatcctgctttttagaaacccgttgttcaggggttgaaccttgaccggcttgcattttgaggtaaagctgatcgtactgatcccttagcttcttggctgaaaggatattggtcgaccaaaaagaatcatgttggcaccacttgataaccaaagctacctggtgcttatcacgatggtccagttcaacaagcttacgcatatcgtcagcccaagtttgcaagtttggttgtttaaagtctggattgttcagcatgatttgcttttgcagataaacagccaatttcatgaaatcatttgcttggtcgtaaaccgttttttttcggtttcgacgagaagtctttttttgtttctgtttgtgtttatttaatgccacactattgtctacaccactgtctacaccgttgtctacaccactgtctacaccgttgcccacactatatgtagacaaattgccgtaaagcttggtaatactgtactttgctgactggtttcccttacgtgattcccatgtaatgaaaccttgttgggtgagtgcgttgcgtgctttgtaaaagttggaggatttggatgtgtcctttattccagatcgctggcataacaccgacgaggctaccgtaaatgtatttgaccatgcagctttattgtttatggacattaaggcgtgccataaggcaatttctgatgagttcaatggatttagttcgagccggtcatagaacgctttgatctgaagtagatagttcattttttcacctccattggatttgattagtggttaaacatttaggctgtcaaacaattcatccgatgatttctcatcgtcttttgattttttagaacgaaattccatcagctcagtgctgagttcatgatccaaagcattcaagtcttctttactcatctgaccccaacttgatactttggcgtgcttcatcgtcgcttcaagtaatggtttaggctccattgccatctctttggccagagaagcaaccttacccttgatggtgtctttatcttcagcggtagccattggcttgctaggtgtcttagctggagcctgacggccatacttgcgcttatgtggctgttcttttcgagcactcttagttgcttgattaccatcgtcgtcaacgtcagacgtaacaccaaacactgctgataaggtgtaacgacgtgcgtaggtctcagctgatccaaacgcctgggcctcattcttacccactggaacgttcaacggatcgaactggatgtactggccggattcgtgcatgagaaacgtggagacagaaatttgatttccatcactggtaacttcctgtgtgtaggcgaagcctttcgggagtgccttatcaatggcatctacaacgccttccagcattacgtatttggacttaaagaatgggttgttcgcattcttttctggctgcttgatattcttacgaacctcattgagtgccttcgcaatttcagatatattctcacttttcttcatatagaccactctccaatttattagggtgataactaacagattccttttcgatcacagtaattccaggtactttctcgccattttgatcaatggctaccccgtcataatcggtcagttgttttttgaagtctgcccatttaatgtctttttttagtaagtctggataattcttttctacaaacggaagaagcttgctgggttcacgttggtattgtttagcatgacgcaggctggtataaccagccggaactttaaccttgccatcaggttgcgtttggcgatactgttcaatcaactgttcaaagtaatcctggctttctttcaatggtttagtttcgctttcgtaccattccttggtttgttcgtcaaatccggctttttgttgcgctttgatatccagctcttgcttaacctcagctaatttacgaaatgcccagtttgctttgttatcgtcatcaataacaaatgtttgtttttccggtgcctctttaatttcatccatagctaatcctcctcgtagattccggtaacttcgtaatcatttagtttatctttttcttttctgagacaagtcagcaacgctcttttaacgatcgggttgctttcttggtcataagctcgttccaatccagtgactctcaagcgcgcatatttaatttttctcaacccatattccagtttattattcatatttccactcctccaatatccatctcgtcttcatgctggtcttcatattcggcatattccgcctccgccaactcttcttgtgttggctttggatcctcatattcatcagccatgttttcgtaatactcatcctcattcattcttaatacctcccaaaaatcgttgcaaaaatgttcgtgtcggtctatactcaatgaatagaatgttttgtagtataaacaatctctctttggttgcaccagacaatcctacatgtctggtgctttttttattatctaagctttgcatattgctcatcctttccttatttcgttgatgtcgattttaacctgctcaaaatactttttgaaccagggcacaatgttgattggaccatcaaaccatttattcatccaagcaactttatcctgttgataaacacggtactgataaccaacagtaataccagcaacgcctatgactgcccaccaaatccaatccggtaatactaaaaccatgttcacatctcccttgctcgtattttagaaatataattctgaatttgttcagatggaatcctccaaccgttgtgagtatgctcgtaatcgataaatccaccattagctatatccaaatcgttacggtgactatacaaaaagttctttgctctggtcacgcctctttggtgccaaacgttccaagagaattccttgagtgtccattcctcaatgctgattcgattcttccaagttaaaaagtcttgatagtcggtgtcatgaaccagcttgtaaccatcgggtgcctgatatttaacaataattgaatcaactggttcactcatgttctagcccccaaacttttgattatattcatcaaccaattctttaatctcgccatctgataacttggcaaaaatcatttttgcgtaagtgtatttcaattcggatccaatctcttcaaaagaatccttaaaatgcttaagcaagaagtctgactgtgcaggtgttcgctgacgcggatccatggcaataatgtaatctgcttcatcttcagatgattgccgctcatgttcttcctttttctgagaaacctcatcagcgtataaatcttgctgtaaaactggattgttcatcattgatggaataccaaactcacttcttgaagcactgaatgccagtggtaacgaccatagcctttggaccagtgctttcttaacatctcgtggtgcatttcttcgaccagctcgaatattgcttaactgactatcagaaatatgggcctgttcagcaatttcagttcggtcaaacgtcttttttaatttgtctaaatcaagtgttaattgtttagcaaattttgaatctttcacttttgatcatctccattttgaaaaaagattaatcgtccttttccatctgatttggtaaattggacttaaggagttaagaaaacagtaattgctcctcactatcacaaagtgattgatacatggctttgagaaaatcatcaccatgccggtcaatcatttctttaaccatttcaacgccatgtgctttggcagttgggctattgagaatttgttctatcatttctgcacgagtcatgggatcaccttctttcgttctttgaaaattgaatccaacatcatctttagtgggataattaagctattccattaaaggtggtgacataatgtgaaactttatgaacccggaactgataacgttccaactggtaaatatcttgaagtcggccctcaaggtggtaaacttcaaaatcctagacacgctacaattcgtgtgtctggtcatcgtcttccccctgtgagtcctgatactcacaataagtggaagcataccagtggacgaactgattaacgttcgtgatacgacatagtgctcaagaacttatcaatcgcatcggagttgtctttatccgggttcaaaacgaagctttttacggagtagcaccacactaagcctaaaaagttgagctgaatccaggactcaaagacaacttcattttttccattacgatattcggttaggtaatgatggatcattcccttgcctcctttctcggtggctttgcctctttagtgagataatgtatttatctcacaacatcagaggtggtaacaatggccattagtcaagatttagttaatcagtttttgacaaaagcgtcggaacttactgagggaaaagctatacgatattcattaaaaacttcggatatttcttatcgtgatttaaaggaaactgtcaggtttttaaattcgcgatatcccaaatacgcttttttctgctatgaaggatctggtgagttattctttatcgttaaaaagctcttcaatcaattttgaagcctctaaaaagttttcaagactgtgagattcaggtttcttttttagattcttttcactgtcaaattcaacatcaacgctgtcgccaacactatcaatcgttaaatcaatttcaagagtgccaattaaaatcgttacgtgtttaggaagaatgcctccagtcatgagacctctctcttttgatgataagattttaatgacgctcttatttgtgcttgattttcgactcattcgctcacctccttaggtgtttggctcccgtccggtcatttaatcacctctttgggttttaatagcttatttataaagtattgttgacccttgccagtaattagtggtgtaaatttattaatggaaccatgattagtgctaatcacggtttcgcgaaccgacatcactttcaaatccattgcatattgtgttggagtattccggcgctgaccagagcgaattaagtaaccgtgttctcgtagccactcaaagaatcgattttgaccaatgttgtagccattctgcttaagaattttggcaaaggttccaacacgaacggtatcatttgaggaactgactgcgttacctagcaaagccggaattcgaagttccttattctcagtttcaagctcctgtcgacgtttctcttcttcaatccacttggttgcccgcgtgactggatcagaaatctgataagagtccttgccgagttcctgaagtgaagcttccattttgttaaaagctcgaatgtactgcagtttgaagttcaatgcttccttgccggtaaatcccattgccaataatgtgaagccatcacgattcaagtagtatgcttttcgatcacgtccataagaatcaggaacgtttacttcaacaaacatctccccaaaattgggtagatcttttcgaaagtgttcaatgtcacgcaaaacgtggtcatgacgcttcccaaacgtttcagcgacttgcaaactgctagtgacagcctgcttattcttcatgattactaagttattcattcgctcacctcctttctcggtggcacgggtggtgtttgcatatatttagcggaatgggctttctgtaaatcaatgtgtacatttttggcaggaaaaaggtattcacttgtagttcctaattcctctgccaaacgattaccaatgtatacagacggagtttgtttaccacgctcaatattacttatatacggcctatttatacccgattttcttgcaagttctgcttgcgaaatatcaactgccaatcgggcctttcggacattatttgaaatatttctcgctcgcatttgatcatctcccttctcaatcaacaaatatattgtacttcatgatttacgatatgtaaacacctaaatacgatttttttatatattttttgtacacaatgaattacaataaagatggaggtgcttcaatgactaatgataagaatcaattggggaactatctgaaaaagcttcgaggcaacttatcatatagagaggttgctagacggtcaggtaataaaattagccacagtgctgttgcacaagctgaaaagggtataaatacacgtggaaaatcgtttgtcccatctccggatactcttaaggagctatcaaaagtttatcacgcaagttacgatgacttaatgataagggctggatatttgcctaccgcgactaatgccaaaactacgccaacttttgatggaatcgaggctgcggcaaccacaaaatgggaaacatcgcatgaaccattagacgtctatgggaaaattaccgctggtattcctacctttgccgatgaacatatcattggtcaaacaattatccccgatgatttgatacgcaggtttggacgtgacaatttatttgcattgcaagttaatggggattcgatgagtagggttattgctccagggtttattgccgtgtttgctaaggattgtgggatagataatggtgacatctgcgccgttctgatagatggagaaaatgccacactaaagaggttcaaggaaacctccaaagcagttatccttgaaccagaatcatttaatcctatttataagccgctgatctttcctaagaacattgaccaagattttaggatattaggtaaatatgtattcgcaacaagtttattacaatgattattgaggagatcttaaaatggggttatttaaatcaaaagaagaaaaagaacaaaaaagagagcaaaaagttaagcgttttttagcacaacacggcttggatgacttaaatccaaaatcttatcagcttgttaaaaacattatgagccaaaatggattaatagacgtgcttgcttataatttaggtgctcgtatacatggatccgatgccgaaaacatgattatcaataatctgcaaactatcgtggaacaaaattggctgatgatcaagcagaatgatacactgcaaaaacaaaacaatgagcttcttaaagcgactaataaaaaaacagcaaaataggcgttcagatctattactcacatacagttgggtttgtgtacagatttagatgtaaatctattgattaaggagattatgggctaagaattgcttggaaatttatgtagggaaaatattaaggagcgagttaaatgaaattatcaaaagtagcgtctttgttaagcgtagcagtgttaggggtaacactaagcgcatgtggaaacacgaaaagtagcaaagaaaatagctcatcaaaaactatgacttctaaagtcgcagcaaagaagccacaagtattacatgataaatttcatgttaaaaaaatatctagtaaaactatttatcctaaaaaaggagattggatgaagggcccagaaggacaaagagtaacttatcttacaagtttacaagatatccctaatcaaacagttcatgggatgaaattgtttaatacgcagtatgctgttatagctatggaaaatttatcatctgacaacgaatacaacagtatgcagcctgatgctaaaactgttttcccaaataatggtgactttccaaagagcttaacgggcaaaacaataattctgctgcatctagaaagtgattttcaaaataatactagcaaaccgttaaattacgacggattttctgggtacgctggtggaaattttgattggacaaccgataatggggttcagattgaccattcaagtttgcaagttaacgacgaaacaaatagtttaactgttcaacctcataaaactgttcaggataaatcaatggatgcaattttatgttatggcaatgacgttcaagacgcttacaaaaagattaatagcaaacaccttactattaaaactgctggggtttcaaccgaagaagaatcacaactcggtggtattagaacactaaaattaaatattaaatagtcttattataatttagaggagatcttagaattgaagaaatattttttgatttttttcgcaaccatcgcattaatttttggctttgcgtttacaacaaatcaaacaattacacgtgcctcgtcaaccattccatattcgatgcgtggtcattggtataattatgataataaaagccatatgaggattacagcacgttacgtaaaaatgtatacgaactggagacacgttaagtacgttagtaaatctggttcgtattacactgtccatttttcaaacgctaatccgattgttttatggcatggcggttctgatacccttcatcttgaatatggtatgagcatcctagaaacgtatcaccgaaaataaataattttgagaattgtaaaattatacttcaaaaattaataatgtcaaagtggactaactattggagagatacacatggacgtacaaaatagagggggcatattaatcaaaaacttaatacgttttctagcctttatttctgccgtgtcgactgcagttttagctggcattttggtatatgcgatcacgcaaaacaaattcaacatacgcattaattttgctatttttatttcgataagtctttctatcatattgtggttatgtacaaccatggctcatatgtctattgataatcaacaacttaaaaataaacttacagtcttaaatcaatcgaaggatgacctaaaaaagaagtatgacacactcaaaataaatagagatgctttgatatctgatcgaactcgcctaaaagctgataaggaaagcttacaaagagatttacgagaagacaatcgtggcatagttgttgaaagagcacggtcggatcaactattacaaatctttactaatttattaaacgaaggaggtaaaactgagaatgacacaaaaagaatacaaagtcctaaagataattgatggtacccatattattatcaacgctggtgacgataatgacataaaagagggagatcactttagaatcattggtaaaaaggttacaaacatcgtcgatccagatactaaagaagattatggcccgctacagcctattaaagcacatataatggcagaaactatctacaagaaatttactatttgtacctcaattccccatatttccgatattactgcggtttcttctttatttagaagaaaagaatatccagagttagatgttaaccccaaggatattagtggcggttcaattaacgacaacaatccaattgaagttggggatacggttcttgaagacctcggctggaatactgcaaatagctctaccttctagtgtgtatacccgttttaagcgtttcttcaattaaaaatttttttctcttctcatctccaaatattgcagttgcttctgaatagcaatcaggttctgaccagtgaggattattagcctttaaaatcatggttaataagtttacagtttcccaataatctagcgaattacaaaactttttaattttattttctctgatgtccataaaatatcctctttctaaaagaataactttgtatcattatagcatcaacgttcaatcaataattaatttacttccccactcggaaccagtacctgttcgactcaggcatggggattacagtccaaatactgatgacgttaaaagctgaaaaatttaagggagaaatttgtatgttaaaagaatttaaagagtttatttcacgtggtaatgtaatggacttagcagttggtgtcattattggagctgcctttacatctatcgttaagtcattagttgataacttaattaatccattaattggtatcttcttgggacaaattgatttttctgatcttgcctttaaagttggtagtgcaacattcaagtatggggcttttattaattccattatcaattttctaattattgcttttgttgtatttctgttagtaaaaggtatcaataaagttatgcctaaaaaagaagctcccactgccccaatctcaatggaagctcagtacctgcaagaaattgctgatattttgaaaaagaataattcccaaaaataggctttcttgaataaattcaatcacgtcaaccttgcacttgtttttaacttttccacatggatttaaaaatgaaagaagtaattttttgaattatatagatatttttaatattaagcatgaaaatgctagagttattaacacaaaaggtgatttcaatcgtatttttattattgaagataaaaatggtgttcgatatacatgtttaaaaccagatgcaaaaagaatgcccaaaacaagtagtcacttcaaaactcttaattccaaacttgctccaattaattatttaacaccatatttcactggtaaaagaaccaaataacttgattatcaattttgtagatttgctacttagttcaggtagagtacatctataaacgtagtccttaatgtagggggtgacaatcaatggcaattgccaggttagaaaatggcatgtggcaagctcgtgtaagttaccgagatggtgttcgttaccgtcgccgtagcaaaaactttaaacgaaaaactgaagctgaacactgggaaacagatatgcgggctaaaatcaactctggcgccgatttccgcaacgctaacatcacgtttgccgattactttgaccgttgggtatcaatctataaaactgatggtgtcgctaagcatacacacgatatgtatgaattgacagctcaacatcttcggcactacttccctgctcaaaagttaattgatattcaaaaggaagattatcagaaatttatgaatctgtttggcaacagccatggcattgccacctcacgaaaaaccaatcaacaaattcgatctgccattcaagatgcactagctgagaatctaattcagcgtgattttaccttcaaagttaaaattactggatcaagccctaaaccagtcgatgataaatttctggatttagatgattatgcaattttacgcgactatctaatcaagcatgccgactttgaacatataagttcagcaatgttactttttcagctagaaaccggaactcggtttgaagaagcagctggcatgacctgggatcacttagatcttaaaactggaaaagtaataattgaccgccaatggtacccagcagccaatacattcactaaaaccaaaggcaacgggcaggcggatggaactattaccattcctgaaaattattgccgagctcttaaaaagttcaaggaagaagccattgaattcttttccgaccaaaaattagattacgccaagctcaatccacgtggtttagtcttttttagcaaatttcgtaggatcattaccaatgattctgctaaccgtgcgctaagtcgaatttgcgctaaacttgaaataaagagggttacgacacatgccatgcgccacacacatgccagctacttaatccaaaatggtgctaatctgacttatgtacaacatcggttacggcataaaaagttgcaaaccacgattaatacttacattcactttgtagaaaaagagaacgggaagtcggacaaagaagctatgaaattgctgggaaaagggtttaacaattgacgttatagttgtatcagtttttctctttgccatttttttgtaattatagatgaacgattggaacattataagctgtcacatcaacgattactagctattcttttaactaatccgattaccgttcgggtgataatcgttgatttaacaaggatcagcaaggtgttagccatttttttggctaacaccttttttgttgcaaaatccgctagacagtttcaataaattgtctaacaaaaaatgccacaacaaaaatttcacactgatgcaatttctggtcgcagaaaaataatgaggttcggacattaattgctacggtggatttgattaccacttttgtattgatacaacgtgcagcgacggccggctgaaagcctgcctggcctacttggcgatcgactgatccccaaaaagcgagccactccaaaataggaatagcccgcttctttgcttaaattctgggatcaaaacgcctctcgtcgcactgtctaatgtaaattatcgaataattctgacatatttagagttaccggtgatatacccaccagccacacggtatcgcaaggcaccgtgcttttgtagattatggccacgggaataatcataattggatactttgatgatctggcccttcttaatcgtgtgaggccgtccgctcaagttcacgttttgataacgatgaatggttgtcttcgcccgaactttcttaacggtccgatgccgacccatgttaaccagctttcggttagcggtgacatacctgccattcgtcaagatataacgggtggtcagattgtgcttcacgatccctttaactttgaggatggttccctgttgataacttctgaccttaccagtcaagtctttgtgcttataggcattaacccctgccggagaaatgaccgtaatgtgtttgtgcagagtagcgtaataaattggacggacatatcgccaattgccggtgatgtagccggtcttgcccgccgtcttcgataagtggttgacatcacggactttgtaacgcatcttcccacttgtggaacgagcataccccgtcaccacaaacatcggccggtaaatgcgcggtttcttgatatatttggcaattcgctggcctttggtgaagttaaccgttcgatacaaatagacattgttaatggcagcgactgccgcgccctttgtccccgcgtaatcaggaagctttggattagttggttgagttggaaccgttggctgcgttggtgtgactggattgatggggttaggcgtcggtgatggttgcggatttggcacaggctgaggggttggcaatggagacggtgttggcgtcggctgggtaaccgtcaattgaacgtcctttgaagctgacccattactgtaatggattgtgtaaacgcctggcgttttatacagattactcaggtctgagatgatctttccagagctgtctttcgccgtcaccaaaatatctttaaaggctaggtcttttccactggcatctttggcattatcaaatgcatctgccggtttccatgcctgattgacggggattgtcagcttgccatacttgagattgagggtactgctgtcagtcacgttgatggtgagcttcccttccaggggctcgtgaccacttagcagctgattggtaacaatgtcgaccgtgtattgaccaacctttgatttgacgtcatcaagcgaaacagttttgccagttgcatctttgatggtgtaagtgtacggaagagcctggccatcggaattgaccgccaaaattttacttttcaacgcatcttcagtgaacgcctggtttaaataaagatcaatatccgtcgtcttcaagctggcctgatcggccttaattgttaaggtaaatggttgtttctgatcaccattctgataagtcagcgagtaggttccaggagccagtgctgcaatagttgcctgggtaaccggctgaccattagcatcagtaatcgtaacagcattcttatcatcggttccattgtgagtcgctaattgaatcacactggtcggatcccaattcttagcttgaaggccctcatatactgaagccgaactattagtcaggttcagcatatattgattaatgggcgtggtgtcttgctgccagacataggtttcgtcttcagcaggccgcttagccacaaagtcctcaagggttggatagagctcgccctgtggattgttgaccgttccattggcaccaactgcttgccatcctggaccggtggcgtccttcaagggatcaatggggatttcatcgcctttttgatgcggcgggagagtggccaaagctgaatttttaaaggttggccccagtttcagattcgatagtaacgtatcctcggaaaacatactgccaatagccgtgacattggtcatgtcaaagtctgaaaggtccaatgttttcaatgagtgattcccgtaaaacatatccagcatattatcaatcttagaagctttcgaatgaggaaaagtgatattcgttaatacataatcccccccaaacatgtgatccgtattttttaattgagaaaaatcaaaattagaaagatcgacttgttcaagcttccaatcaccaaaaaacaggccactcatcgtgatgacattgggtgtccgaaagctggagacatcaacggatgttaagttgccatcttgagcaaacatataattcagcgtttcggtctttgacgtatcaacgtttcttaagccggatatactttcaagattccccaacgcctcaaaaaattcataggcaccatcctgctcaaattcaagcgggccatcaatcttaagctttttaatgcggtcacggaccccatcctgttgccaaggaagtgaaaagttctcgtgaatttttttgatcgtgccgccatataaagtcagctggtcatccttaaccgtgtaggagacatcttcgacctttcccgataggtctggatttgcctgctcgtcttgtgaagggtcactcgtgggagaaaccacggcactattggaacttggggcggctttcaccacgttggtagacattcccactcctaaagagaggccgagaatggtgctatataaatatttctttgctagtttcataattagccttctcactatcctgatattttgatttgcgcaacttcggtttggtgaccagttgtggacatttaatgaaaacgctactaattttaaaatattgtatcactttaaccatttatgcggtgacaacttgctcatcgcaatggtctgtgctaataatccgaatctttaaaggctgaagtcagtgtcttatatcaccaaacaaaattcaccgcccgcacccgtcctggtggtatcataaatgcatcaagattaggaggcttcatcatggaattaacggcaacagactatgaaattttaaaggcaatttataccggccgggtatcatccggcaccccggtcaaccacttcgtcgattattgtgataacgtcattggcggcgatcccaagccactggtcgcagccggctacatcgtgaccgaccacaacgaaatcaatggtttaacagaaaagggcaccaaggcttacgaagcccatgcagcccaagaatcaaacagctaacaaaaagtcatcattttgcatccttgagactctctcaagcaaatgcaaaatgatgacttttaatttagtgattttcttgttctttttcggcagctgtcgcatccggaataatcacggtaaacgtcgtgccctcacccagtttggatgaaactgaaatcttgccgccatgggatttcaccaactggtgaacaatcgccaatcccagtcccgactcaccgtacttaccggttcttcgtgaggcatcggctttataataacgttcaaaaatatttttttgctgatcctcggacatgccaataccggtatcggcaaccttgatgatggtctcgttgtagccccgttcaccggtcacggtaatcgtcccttgatcagtaaactggatcgcattggtcacaatattgaagacaatctggacaaaccgatcataatctgcataaattgacaggtctttaggggcgttcaaaacgagcttgtcctgcgattcttctgctttgctgtccaactggtcgatgacgttttcaaggaccttagcggcgttaaaatgacgcttgtcaagctgaatagagttggagcgaatcttttcgtaatccaaattctcattcaccaaccgaatcagccgctgagtttcactactcatcaagtcaatgctcttggcccttgactcctggggaatcacatcgtacttgattccttccaaaatgcccgagattgttgtgagaggagttcgcatctcatgtgccgcattggccaagaattcctggcggcgttcttcctgccgttgaatttcattgttggcctgctgcaaggattgggtcatgtggttgaaatcgacgatcaattcgccaatttcatctttcccaccgggtttcaagcgaatcttgtaattgccgtttgaaacctgattggcggcacttcgcagtttgctaatccgtcgattcagccgtctggcgatgaagtaactaatgaacatcgaaatgagcaacgccacaaacagcgcctttaacaaatcgcggttaatccgcttgacgttggagttaacatccgaaataaaggcaccaaccgtcacggcggccactagttttttcttataatagtatggctttaaaacttcaatcattgccggccgggtcttgccattgctgagcttgaaattcttattattgaccttccgaacgatctgattgcgccgcaaatgctcccagtctttctgggtaattcggggggcaacgccgttattgggatagatcacctggtcttgtggactgaagacggtaaaatggaccgcttggttctccaacaaggcttcagagttcttcaacttctcttcgtcaaaggtcactttggccttattcttggagctaatcgtcagcgattgttgaatcaaactatccgaatacttttccaagttatgccaggtttggtcatatacaaacgttttcgacatgcggctaaatgaaaaacccagcaataaaattgtacagccaattaccaaaaagaacgccaataattgctgataaatcattttcatttcttcttgcccacttcactatcatcaaatttatagccaacgccccaaacggtttgaatcacttgggtgccaaccttctcaatcttttgacgcaactttttgacgtgcgcatcaacagttcgttcatcaccatagtactcataattccagaccgtttccaaaagctgctcacgggaaaatacctgacgtggcttttgggccaacgtctttaacagttcgaactctttgggagtcagatcagaaatccgcttgtcatccaaatacacttcccgagtactggagttcaatttaaagtgatcagtttgaacgtcaaagacatttttggccttctcgtcctcagatttctcttcagtttcagtgtgggcccgtcgctgtaaggctttgattctggccaccaaggtaattggggaaaacggcttggtgacgtaatcgtctgcgcccatctcaaatcccaagacctgatcactgtccgaatcgcgagcggtcaacataataatcgggaccgtttgtgacttggcccgaatttctttggcgacttccatgccgtcttttttaggtaaattaagatccagagtaatcatgtcccaactatcaggatcttcgttaaatttgtccattgcctcaatgccgtcataagcaaatgtgacatcccagccttctttttggaagaacatctgcatcatttccgacactgatttgttatcttcaatcatcaacaatttcattctaaaaccccaccttcaataactgattgcttccaagttcccgcgtttccaatgctttcttaaatgattttgagaaatcgactctagtttgccggtccacggatcgttgtagtagtaaagttttctgttaaaaccggtcaacaagatcaagctggactttaaattatcgaggccggcaactttgactaaaatcggtcttctgcgcaaaagctgcttatctaatttgcgaaaatcaacgccgttcagatcacgaattgagtgggttaacgaaataatcaagtcactcaaatccattagggttcccgattgcgcgtgccacttctcaactttgtctcggatatcgctgacgtcgacattaatgccggcgctgttaagcagcattaaaatcgccgtacactgattatcaatatcggattgcgtgggctgcttaatcggttcaacgtccaatcggcgaaatgtctttcgaatatttcgtttgggcagccagccttccagatctccacaagtgaagtggtaccagactaatttgttgaagaagctaatctcatcaatcaaaaaatcctgtgccttgatgctgtccggaactttaattttattttttggatttacatttttttcgttaccgtttgctaaataccaatgttcgccgggaattcttcttagtcgaacgaagaaacggctggtcttttcattcgcaatggttgttttttccaatcgtctcaccccatatataacccattttaccaataattagaagaacttgcttggaaagtcgcaatattgttatgatagtaaagtatatgattataaaattgataatgaaaaggatggcttatctatgtataaaggaattgcgttctttgaccttgaccatactttatttaatgaacacacgcgtgtcgacgacgaagtggctgatgcgatgcgccaattaaaagcaaatcaggttctcccagtgatttcgaccggcagaaatttatttgaaatccccaatacaatgcaaaagactgggattaacactgtggtttccgcaaacggcagttacgtcatttttgaaggccagccggtttacaaagctgtcctggaaaaatctgttgttaaggattttgtggcgtttgccaaatccaaccacgaagcaaccacggttatgaacagccagggtgccaagattaattttatcaatgacatcgtccgcggcaattataacttcattaactcccggatgccaaacttgggcgtagatgatttcattgagaatcaagaagtgatcatgatgttgattaacaccaaggggcctgacgaaagatacattgaccggttcgccgacaccctgacattcttcagaaataccccgtttagcatggatattgttcacaaaggcagttccaagaaaaaaggcatccaggagttgattgccaacgccaatctctccggcatcccaacttatgcgtttggcgacggcaacaacgacattccgatgttggatttcgttgatcaccccgtcgtgatggaaaatggactgccacaggtgaaaaagtatgccgagtttatcacgaccaagaataccgatcatggtatcgttaacggcctcaaatattttgacctgttgtaagacacaattcttctcagttcccgtgatttatgatatgatgtgtattgtatcggggtcgttatggattcgacgggtataggttgagtctggattgcgtttcgtgcagcgccacgttaaaccgcccagtttattataactgcaaaaaataataacaattcttacgctttagctgcctaataagcgcttaacgtagatcctcctaatctcgcccatgggttagatctgggtcctaaatttagtgggctcacgcagtttgctcccacctgaagtgaactgaagagactaatcaggttagcctgctgtgggtgccttgatttatggcgtttcagtaggtgaaattcaaataatagatctatgaacgtagatatctaggtggcaatatgctcggacgcgggttcaactcccgccgactccatcaatatactaaaaggtcagccatgacagtgcacaaagcattgtcatggctgacctttttatgattacattgatttggtcattcaaagtaacaacagaaaaattaataaaatggcgagaaatgtcgtcttgcaatcgttaatcaaaactctttcgtacccggttcaaaacgattagaatggccaaagccacaaccgtatagacagccccactgtatcccagtgattttaatcccaagtgattgaacaagaccccaccggttgcagatcctaccgcgattcctacgttattaaaaatcgaaatcaaggatgaggccaagaccatcgactgcggatagtctttttcagccacagccaggtagaaaatctgcattggcgagttcagcaagtacatcgtcaggcccatgataattaaggcggccagtgcagcccacggcaacccgaataacagcgaaatcgccaacatggtcaaagcttgaatcacaaacaccgtgaccattgattttaagccattccgattcgccaaccggccgctgtattgattactgaacaacgatgccagtccaaagacaaacagaaacggcgtcacaaaactggttggaaaatgcagtccagacgtcacaattggtcgaaggtaggtataaacaacgtagaccccgcctaagttaagaattggcagacaaatccccaagagaatgcggggatctttgaaaaggctgaattgttcacccaaactctttgctttcccttgccgcaaatctccaggcagcgacaacatgaacatgaccgtaatcatgactgagatgaggacaattaaccaaaatgcccagcgccagccgacctgatcactaatccaagtcccaatcggtactccgaaaaccgaggcgacactgtaccccgaaaagacccaagaaatcaaccaggcccgtttatctcgtggggcaatgactgccgcaaaggtaatcgcaattgaaacagttatcccggcaaccactgcattcagcactcgggacaaggacagaataaagaatgagttggccagagccgtcatgacattggagattgtgaagacactcaacaacagcaacatcacccgcttgagtcgatgctcgcccaccaagatggttaaaattggcgtcacaatggcatagacaatcgcaaacatcgtcaccaagaagccgacgttggaaatgcccacgtcaaaagaatcggccaaatcattgatgattccaacaataataaactcgctcatccctagaataaatccaattgaaatgagaatgaagctttgcactttaagtgatttcatgtgttcccccccgtcaaaaaaatttatcaaaaacgattatacattatctggcactgtggttatacctcaatcgagcaaacagttgcatttgtcgaaatcagagcccccgttcatagatttgcttgcatctgccaagtcagccatgctataatcgattttggtgccaaaccacggtaagtaagtaacgatcggcgcgtatgcgttcagaaggtcgaagctgcttgccatttttttgttttaaggaacttttaaattcgcatgcctggtttccttcccagattgaatcatgattaaaaatgttataatcgtatcgtaaattgtttgagggggattcaacatgcaaaatcaaacaccatcacgattgcagcagaagcaatccaaacaggaacagaaaaaaactaagcacaccaagttaattgtttggttaagcgtcttggtgattgtcctagtcggttttctttacgttggtcatcaggttcacgaattaaccgacgctcagcggcaaaccaatacaattttggataaacccattaagaatacggtcgtgaaggttgtggaacccaagctgccggaagaggtccgtccacaagttgtcaaaatcatccaggaagaaccgctctatcgcctgcagcaggcagccgacaacccaacgactttccagcagattgctgacaagtatcaggtgccggaaacctacgttgcccctgccaagcagtactggttcagtcagcagaacgacgcgttgagatcagacatctatcatgccaagctcatgcagattatgtctgaactacgagcgttagataattcaaatcagtaagcttttggagagatagccaattggcatcttctatttcgacaaacatcatcaagaagccgttgaccaatacccagggattgtcctcggaaaaccaatcaacaaataatcgcatcaaatcatccagcagcgtcattcatggcgttgctttttatctgccatcattttatccaacgtcaactttcctcattttgagtttctttattgaaaaaaacatgtaaaatattaataaatcatcattttcataaatacataagcattggagctcagaacatgaaaaaaatattcgcactcgcattgaccttaatcgccgtcatctccctctcagggtgtagcggtcagaataaaagttcttcagacacaccaagttttcggaagaactttcttcaagttaagaatttccagctgaaaattaccaaaaccgctgtgattccagctggtgagactggtaatgaatttggcaagaaacccatttttgccctttggtacaccattaaaaacacaggcattcataaagtttcaccagtgtctgccgcttccgtgctccgcgcctaccagcctgctaaatccaaaaagcagttggtcgccgccccacttccggatcaagatttagctcccaaatacaaggtggctatcaagaaaaatcaatcagccaaaggctcaatggcctggaatctgtatgataccaaatccccaatcaagatccacggcgtgaaagccggcaccaaccaaatcatcggagtacaaacctatagcattaaataaacagactttttagccaaatatccaaaaaacaggatccccaacatgcgagatgatagcgtgttgggggtcctgtttttcaatttgctttattgctgagcattaaacttcgtaaacagtttactgaagtcgacggttcccagaccagttgcttggttataaaccttgcccggctggccggtatagtacagattggtattctccatcgtcgcgtcatctaaaacatggaacggtgtgtcggattgaacagcaaacttatacagctgtgggttccagaatccggcagaagtctttaaaccactgttgataacagcactggcgccagccatttgtggggcaacaaagctggttccgcctgcattcatccagatgggaacctgggtattcccggctttataagtaatgtatacgccataaccagttttttcatcagcgttcccggaaatgtccggtacatttcgtccctgatgagtcccagaaatcatttcaggatctgggttgaccaagtaaccacccttggtatatttcaacatgttaaatgcgttgtaagtgttgacgcccggaacaccaagctgataagcaggggttggattgagagttgaaaaaccaccaccgccaccagggaagacagttggcttggtaaccgtaccttgtgaataggaatcaccccaggcgcgctcttttttaacttgaatcaattggccgccaataattttggtataaggcaacgtcgttccgcccacttgaacggcatattccgatgttgggaatggcaagttggtggacttatttgcgacttcatacggtccactgtcaccggcagcgttaaaaatggtcgttccttgaatggctgcctgttcaaaaaccaggttgatggcatcattgaattctgaagctgtttcacttagcccgccacgaccgaagccattcaattcattaccaaaggacgaactggtcgtcaattgtttgtcacggttatcaccaatcgcagtggcaaatgcgtccaaatattgaacatccggcgtggtgtctccgttgctggaaaccccgacataagcgtcaatttgtgcttgatcagcaactcctccagcttgttcaacatccaaactggcttcttcctgggaggtcacatcatcattgttctttggctttggcccaccagtattatcggtggtgtagatcttgtgaattctggaaacgtcgctgttgacccccatttgtttccagtagtcggcaacatcacttgggttgaagtcgtaagtcacaattaccccaatacgttggccggccccatgcagattctggtcgtacagcttgttaacgccatatcgatcggcaaatttagtcggaccatatttcttcgccagctgattttgactgctggcgacaattggcgtgtcgtcttcaattaagttgtgggtaaactttaacgccttcttatcggttttcgtcgaagtctttttattgtcaacaaacaatcccaggactgacgcgacttgactggacagcttaccaggcaatttagtgccggtcacgtcccagtccttgttggtcttggctggggtcgccttaaaggccttcaccagattcttttgagatccctggactttcatcacaaagttgccaggataagccgccgatttgaggtgatattgactgaagtacttgttaaaatcagaaatttcggcgttggttcggccaaaacggtcagccacctgttgtggtgttaagtattgatgataattagccgatgttggatctaccgtttggctaacataagtattcattgcattacggtcgcgaacattaaagacaacattcaccgtcaccggggtctgctttgccttggccgaagctgtcgttgaaaccgcccccaaagttacgaatccagtcagcactaagagtgcacttttccattttcccataatctttgactccccttatttatatacaattaattataattcaatggtatccggcttgcatgattgaggccttttaatcttttgtgaatgaaaacagtcatctccagcatatttaatcagtatcaaaatgacacacaaaagaggctaaaacatcaattgacactgatgctttagcctctcacttagctatagaacgatttatttaactccgtgttgtttcaagaaggcactcaacggaaccaagtcttctgcgtagtaacgtttcttgaagtcgtcaatcgtcttttgatcgaatttatccggatccaaagtcaatttttcaactggaatcggacgctcgttggtaatcttgacatcgatcagcaccggtttgccggccttggtctcttcaacggccttatcaaaagccggcttcatttgatcaacggatgtcaccgtgattccaagcatcccttgagcttcggcgaccttggcgaaatcggtctgcggcaaactaattccgaaccactcatgactgtcatcctcttgctcatcttcaatgaagcccagcgcttcgttagaaaagacgacgttgatcactggcagcttgtagccaacttgggtgctcaggtcctgcatcaccatagctgcggcaccatcaccggtcaggttgaatacttgacgatctgggtagctcaacttagcagcaattgaccccggtaagccaacgcccatagtggcaaataatccggaagtaatccaaggctgatggccgttggtctttaacaaacgaacagcgttttgggtgacatcaccaacatcaatggagaagatggcatctttttcagcgatccgattgatttctttaaatgctggttcgaaacgcagcttgccttccgtccggttcatcatatggtcattgtattcgtgccaatttgtgacgttatcaacgttggctgcgtaccaatctgatggctctttagtttgacccatatcgatgaatttctgtaatgtcttcttggcatctgcaagaatggcaacgtccgtcttgtgacgtttgccaagcacttgtggattgttatcaatttgaatgaatttaacgtccggtttgaacatcgcttcagcaaacggatagttggagccgacaaacagcatcaaatcagtttgctgtaacgcctcgttggctggcttggaagcaacccgggcagcggaacccagtaaggattcaaagtcataagggataatttccttgcccagtgcggtcgtgatcactggaatttggaacttcttggcaaattccattacctcatcggcagcgccgtaagttccctggccgacgtacaggactggctttttagcctgatcaatcaagtccaatgcttgttggacctgctcgtctgaaccggtacctagttctggtttggcaaaattggcagcggaactataatagccatctgctggaatttccttattggccaaatcatttggaatcgtgacgatggctggaccgtgttgcgcaaacgcccgacgaatggcttcgtctaagatgtggggcagactttgagcggtcatgacggttcgagcataaaccccggcatccttaaaccatgggttctcatcgaattcctggaagaagtcctggttcatcagagcttgtggattttgaccaacaatcaagagaaccggaactttgtcagccattgcgtcataagccccttgatacaagtgagtagcaccagggccggctgagccaaaggcaaccccgatgtgaccggttagtttcgaatcggcaacggcagccaaggcacccacttcttcatgacgaacgtgaacataagtgattttgtctttttcagcatctaatgcatacattaaattgttaatggttccgcctgggatcccgtagatgtgatcaacaccccagctctcaagtgtgtgtaatgcagcaatccccgaattaattgtttcagccataattaaaacctccctgtaaaataagtaaccaattactgattaacatcatattagttttgtgcaatcgaaaatacaattaaaacgactttttgattgaaaacggttaatcggctattataaaaggattcccaagagataagaatataactttccggctatcaaaccattaaataatcgtcaaaaaatagttgacgtgggtattgcggtttgggtatagttaaatggcactttcaacgaccagctgaatgcacttgaaaactcaggagcatccagtcatgctcctgagtcattttgtccaaaactgacgacgcaaaaagctgaatacatattttgggggattatcatgaatcaagaaacaaagttctgtttaagttgcggcaaagagattccatttgctgcatcgtattgtccatactgtggcaaaccacaagtcggtttagccagtcaatcacctatgccatcagacgcttcaaagcaacggactgatgtggccgaatcaaaaaggcagctttggtacaagaattggatgatttgggccattatcgtattgggggttggcctggtaacttgtattgccctgttgaacagcgcgaaaacaacggttgtcatgcggcctgcagcgagttcgaagaccgctaagaccaaagcgaaggctaagaaaaaggatccaaaccaagtctcttcaaaccctcttatccatctgtcaaaagttggtcagtggaaaaatagcgaagttctaggaaaaatttccatgaccggattaggaactaaaccggatacgacaatccaaaatgggccgctttctgttaaatttaaacacgctgagatcgacaaagttcatgcaaatacagaagatcagcttgatcaggcactgacttcgtttaacaaagatagtatgcctaaagactacacgcgaatgaaaattgagtatgttgttaccaatcattccacaacaacgattgactttggcggaatcaagcaaattgtattttccaacggttatcaaataaacttcgatgacgatgcgatggctgatacaggttctgaagaagagttggctcccaatgccaagcgggtggaatatgacttagtcttattatctgagtccactacgacactgaagcccaaaagtattaagatcattacagatgagtctgacgattcaaaatctttagatacagtttctgatggatcaagtttctcagaaagtatcagttatcaagcctgactcgtaataacaagcataatagtctttgtttgcacgtaaccttgaaacacaaaaaccagcaacgatgaaataatcatcattgctggttttatttattatttaagagtaaagtagcgcactattcttcaaatatcttccctgccttagggcctggatccaatgtccaaatcttttcaatggtaatcacaccggcaccctttggagctgggaacttaccttctgcccatttggcagcttgatcaaagtagtcaccgtccgtgtagagtttcgccgttccaccgaaccggaatccttttaatgccttggcgttggcaacggccacaattgctttgccgttattattgatgtttgcttgggtttggccgccggtcatttcgttataaatcagatgctcatcatccagaacccgcatcgaaatcttgggtccaacatctggattgccatctgcatcaacagttgaaatatacgataattctccggcaatcatgtctttcattgcctggttcaatttagccatcataacatctcccattaatttaaagtaagcttattttagtgcctcactcctgaaagggcaatcatttacccttttggtgtgaaaatgctgtaatcgcaaaatgactcaagagtcgctgaaagatcgtgtgcatcaagcctttcaaaatgagccagccgacgatcacgccaaacgtgttggtcaacacgtcgttaatatcgacccatctggacagcccgaccgacagatccaaaacaaactgcaggctttcaatggtcaagctgacacccaacccggtcaataagacttttcgcagattgaactttggcagcagcaatcccaaatacacgcccatcggcagcatcatcaccacattttgataaaaatcagcagtggtactccaaaatgggatcaaattaatgggtgccgaaccgatcatcatcggtgagacttgttggggtcccacgaacgcgtatgatgtcggcgccaaggtaagatagctcacaaccaaaatatagatgattgaagtgacaattgtgaacagttggcaccaggtcaattgcctcaagttccttgattgaatcttcaaccagaccaatacaccagtaatatttaataaatatggcaaccatttaatcatcgtctcccacctttcttcgagcaaattcgtgactaaatttcatttgttaaattcattctagaaaggcgtggttaactgaaacttaaaccttaagcgatcataatcggttttagaaaaacgtaatgatcatccccaggttgccattgccagttgtgaatgctatctttacaagtatcattattgacggaggctatcatggatattgttttagcagttgtctggattttactggccacagcggtgtttaccatcgtcgttggtgccttttatctcatctataaaaatgcccgcggccagccggcacctttcaaatggcgccaactcttcgtcgccctggcagtattaagtctacttttcactctttttggcggcttaatctcaattattacgaatctccaatacggcaatccttgaacccatgaggattgctttttttatcaaatcgccgaataagactttggatcctggatctgttataatagaagtaggttatataattaaatagttatacctaatataaaaaatgaaggagtgtcctacttatggcaactattatttctgtttcagatttggcgaagttacctgacttacaagcaccggtgattactttgaatcttaacttgcgtaagctgtcgtttgaccaaagtgaacaactccgagttaagaatatgctgaaaaaaatccaaaaagaagtcggagacgatattgcgccatttattgctgatgtcaatgacctgacccgtgagcagctgccttatgaaggcatgaccgtgattgccgatcaccttagcaaaaatgtttatcatttgatccgaaccagtgtcgatgagccggactatcgaattgaagatgcaattgacttcctgttattactcagtgaagcacctaatcaggattacacattgatcgaattaaaccgtgacaacagtaaactctatcaactttccaacaagcgagtcaccgcacttgatgtcaaagagtatccagccaatgttaaagaagccctcggtgaggaattgcgtggcggtgaactgaactttagtgcccgcggcggcaatgcccaatatcacggtcataacgaaaccacccaggaaaagaaaatcgaccaggaacgttactaccgggtcataatggatttcctgaagggaaacgtggaattggcacaacatcaattcgtcctgatgggcctatctcaaaatattaacctattcaagaaagtcaataatggcttacaactagccgacttcgaggtggatcaatccgttcaaaatgacaccactactgagattgccaaattggtaaacacggcgattgacacgtacaaccgtgaaaacacagctgaagccattaccaagatatttaaggaccaactattcaccgacttccagaatattgaaaatctcttaaagtccagagagattcgtcacctattcgtggcttcccgtaatgaaatcaaggctgcggatccaaaggtttatactaaaatcaaccagatgattaagcaggcattagcccaggatacccgtgtgactgtcgttaatgacgatccatcagttccattagtcagtgcggtttaaccaatttcaataacaataaagggaacggcaagatgccgttccctttattgttattgattagccgacagacgttctgaaatatctgccgcaattttttccagtcggccctcattttggacttgggcaattttatagccgacaaaatatggtgaggtcgcataacgtgggacaattttgcagtaaaatttatcggccatttcgtagaaaaataagttgtacgatgacagtcggccacccatgtaatcgttcaacaagtatttgacgatcacttggacagcatcggccaagtcgttaatatgaccgacctcttcgatggcaatattgatttcgacaaacccaataatcggctgcgtggataatgtgatttcacagcgctcatcatgaatcacttcaactccggtaaaattactgatatcaacattttgataaacatcataattatccaatccgacaatttgaaaatgtggatgtcgtaaactgccgccggataacgggccatagttcttgtacataatcgtgctttgatatttattggacacaatcatttggtgccaacatttaaatgcaaattcgaacacttgccgattctgctcaactgaataagtggagggtccgccaagatggtcactggattcgatcaccacagtctgaaaggtatcttcaagagtccgaaacttattgaccagccaaatgcgatcgtcgtcccgtgccaaaatgttggtcaaatgctcaacatcacaaaacgggcagtacccttccggatggcgaatattctccggcttgccttgagcagcttgataatcaaatactaacggttgatttgccaattgattcacctgtctttcattgagaactttgtatgttcattatattcgaaaactggccgcgacggttaaaaagtccacgactcgccgcccaaataagtatataatgttgtcaatccagccaacatttagaaccatcttgtcagggggaattttatgggaaaaccaattactgttacactcgcattaatgagcacgctgttgctatcagcgtgcggcacttcgaattcagccaaaaaacaggttaatcatcactttgacagtcaaaaaaccgccgctgaatacaagcacgaccgagaagctgaagggatcaatctggctaattttaatcggattaatattggcgacattaccgatgctgcctatggttcctcagaagaccaagtcctcaaactcttcgggactccttcccacgttgatacggtcaacgtcaacggcgtcaccaagaagacaacccagtatacctggaaggatgtttctgcgactttcccggttgccaaggtcaaagtacagtttctcaatcacaaagctgtcgggaaatcctatacgccagctgccaagcgcaagcagcgaatcactgccaaatcaaaaattaaccagttgggtcttggaactacatatcaagctgcgattaatgcgttgggcacaccaaacggccagtcgattatcggccagggaccgatgtcagccaaatacttactctatgtcactgacaaaaaagggacggcgtacgatctcacatttacggatgataaattgaacaataagttcaaaacttcgatatactaagggtgtacatgcccaaacatttgataggaggctgcaaagatgaaagttatcaacgttgaattgtcagttaaaccagggatgcaatcggactacgaagcatttattgatgaattggtcgatggctcccgtggcgaagcaggcaacgtcagctacgaccatttcaagaagctccatagtgacactgagtatgaaattattgaacattggcaggatgaaaaagctgttgaattccacaacaatacgccccatttccaaaaatttttagccggggttggcgactttttgactaaagatcctgtgatcattcgaatggattataacgaataacggctcaagaggctgggacaaaagtatacgcttttgccttggcctctttttttgtgatcccatattatttatcaaaaacgtgcgacgacggccagcatgcttgcctagcctacatggcaatcggctgatcccagaatttaagagcacagatcaatcattccaaaaccaagaataatcgatctgtgctcttaaattctgggatcaaaacgcctttagtcccactctttttttgataccaacctttttctttttaatttcattgaaagcgcttataatcaaggttaaagaaacgtaggaggtactgccagaatgcaagacgaaagatggaataacccgttgtatcaaaccgaagctgtgaatgatgaaggtctgaacggccatgcttatgtcccagacggcatcaaagtggaaaccagcagcccattaaattcaaagccgggtaccaacccggaacaacttttgggcatgtctttggccacctgtttggaagccacccttcaagccgttgaaagagaacatggtgtcccccacaccgccgaggtccacgtcaaagtggcttacattggtgagcgggctgaataccaattcttagttcacgctcagatcatggtcaaaggtgttgactttgaaaccgctgaccaatttgcacaagaagctgaaaaccgctgcccagtttcaaaattacttaagaacagcgggaactacaccgctgaaacagttacgagctttgattaacccaaagagattgggacgaaaggcgatttgatcccagaatttaacgaataaacgcagttattccggactttggaatgactgcgtttattcgttaaatggccgggatcagccgtttgttgcaagttttatctatataaaagtggtaatgaaggttgcaatgaaagccagcgtaacaattaatgtcccaacctctttgattgcgataatgttctcaatctcatctaaaaagctggtaatgttttcaaataagctgtaatatttagttgaaataattaattaactgtttaaattattcaataatattcgggtatttaattgttttatgaatttgcacaatttgctaatattattttcatgttcacattttttactgtataatcattctaaatgaacttaatcaaatctcaggaggctttcttttatggatagaaaaatccctaatattatgggtactcaacatccagataacgcaggagttccattcttcaagcacaacgataatgcatttgtatccgcatttcgtgaaattgatgaagcttaccaaaacttttccaagctcgatgccgatgagtatatgtgggactgggaaggcaaacacgccgatgcatccgtcattgaccgtttgtactccgagcactacgaatatttccaaaagcatccccttggcaaagataagtacctcactttccgtctgccaaacatttgggaagaaaagggctacagtttgatgcaggcaatgaccaccatcttgtccgctgaagactttgcttacgatttggggtttaaggaacgaccgttattcgaagctatcttgcccatgacccaatcagccgaccagctgatttccatggaagacaagttcgccagcctttcccactacaagtcaactgaatttaataccgggcacaaagattcagatactctgcaaatgattccattgtttgaaggattcgaatcccagttacacgccccacaaatcctgaaaaaataccttgaaatgtacaaagaccactttggccgtgaattaagctatatgcgggtcttcttggccggatccgattccgctctttcaaacggtttcttgaacagtatcattggtaacaaattagccttgaccggtttggccgaatttgaacaagaatccggcctgccaatctatccaattgccggaaccggaagcaccatcttccgtggcggcctatcaccaatgatgattgaccgttacctcgaagaattccccggtttgaagacggcaacgattcaatcggcattccgttacgattacccgctggatgtggttgaaccagcgatcatcaaactgcgcgacggccttcaaaagagcaaatttgaaattatcgatcacgacgaccaagacattctcttggaaatcgctaaaaaagccgctgcagaatatcacgaaactttggatccactcattaacgacttacagccggtatttgatgcctttccaaagcgtcgggaccgtcaccaacacgtcggaatcatcggttactcacgtgacgtcgatggctataagatgcctcgggcgatcacctttaccggtgccctgtactcagttggggttccgccagaatttcttggaactggccgcatcttgaacaagctaagcgacaaagaattgaacaccttaatgaaatactatccaaatatcaaacacgattatgcccacgttgccaaatacttcagcaaggacgccttggatgctcttcaagccaagaaccctgcctggaaagcggttgacgaagatattgaagcagttgaacgactattcggtattcaggccggcccacagacacctgaacaagagaagcatgcccaactagccgctgatctggttaagatttctgataaagaaaccaagaccaccttaatcagtcgtcaggcaatcttgcgtaagttcttaggctaatcactaaaattccagctagtcggctggaatttttttaaccagacttttatactaaaattagttgaattttgaaaggagattttttagatgtttaagaaaagtatcttgttggcggtaacagccctgggccttggtggtttcgtatctgtcactcaatcccccgtttcaagcgctgccagcatgcccggatccttgagttatcacaaagctaattttaatgccaaaatcggcaccaactacaaatcatttaagctcactaatcacgcccccaacagcagctataaaaacattaagaccacttcatggaagaagagcggcttaaaggctggcaccaaagtccacgttgatttgtacgccaaccagggattgcagttcaactggtaccggatcaccaaatactcaaccaagaaggccaccaaacacaccaaagttcaaaaatattggatttacggccaagcactggtacttcctaaatcaatcaccaaccaactggctttgagttactaaagtttccactgcaccaagcaccgcttccgaatcgaatcgatgtattaaattaagaaggaatgatttgattgaataaatttcaaacgacttccagctgtaccgcatttttagctggaaagaatgctacaactgacggatcgacgatgattgccagaaatgaagatgccggcggaggcgtgaatgccaagcgctttgtggtggtgaacccgacagatcaacccagcgaatacgttttgacttttaaccaatttcgggttaagctcccaaacaatccgctgcgctacaccgaaacacccaacgctgacgttagtgatggcctctggggcgaatccggcattaactccgacaacgttgccatgagctcaactgaaaccgaatttaccaacaccaccatgctgggattggacccgctggtggctgacggtatcggtgaagaggccatgctgacttgtgtcctcccttacatccacagcgctcgtgcaggcgttcaacgcttgggcgatttggtcaccaaatttggcacttgtgaaagcaacggcatcgccttttcagattcagatgaggtctggtacttcgaaacagtcggtgggcaccattgggctgccgaacgaattccggatgatgcctatgcggtcgcacctaatcaaaccggcattcaagaaatcaactttgatgatcctgaccacttcatgtacagcgacgatctgaaagcatttgccgataaatatcacttgaacaaggcccgttccggctttaacttccgtgatattttcggtgaggacgttcaagcggatcactactacaacaccccgcgggtttggtatggccaaaaaatgtttaacccggaaatccaccaggatccagaaagtcggacaatgccatttaccagagttgccgatcatttgatttcagttgaagacattgccttcttcttgagcagccactatcaaggcactgattttgatccttatgggaaaaccggtactgaagaatcacggttgcgctatcgaccaattggaatgaaccgcaaccaagagatgcatatcctgcaaattcgtcccgattttccagcagaacacgccgccattcattggctggctgaaggggtcaacgagttcaatgcgccggtgccattctttgccaactgcacggataccccggataactttaagcacacgccgctgcggaccacgacagaaagcttctattggctgaataagttggtcgccatgttggctgaccccttctttgccgaacacgatctcgaagcaatgactgcagtttctgaaagccgcaagtttggctttgccaacggccgggctgcagtggcgactgcagatgcagaatttaaaaacattgccaaggacaagttacctgagtggcataatcaggttaacgacaagatcgctcacgcaattactgagaacgtgaaggatttgctgcatcaattgctgttgctgcgagctgaaaagatggtaccaacctttgaaaaaggcggggaattataaccggtccacgacccgcaattcgtcagataaagaatccacattttaactgtcaaatcaaaaatggattagcacccaacaaatcgttgagagctaacccatttttttgaatatcatttcacagtatttgtcttaatccgatccaacggaatttcccgtggtgtgaatgtatcgttggtctggccaagggtcaaggcaaatgccggcttaaaaccatctggaacgactccgcttggaatggattccaaactggccatattatagttggcacctaatccctgatcttcagcggccaattccatgttgtgaacaatcgcaccggctgaaatctcatcggaggcactttcttccttaactgaaaccacaatcaccgttggggcttcataaatgccagtcatttttgacaaaacagttggatcttggatcaccgtcaatcgataatcatcatagcgccccatcccaaccggactggcgttggctgcaaccaaaatttcgtgcagctgatcatcggatacttggcccgaatactcacgaactgctttacgtgactgaatcattttcaatgtttccatcaactatcactcctccaattttgtttccacttctattgtaaacgcttttttaggaaaatgaaccaaacattttcacctggaaattttaggtttgtttggtacactcaaagtattaatcatcatcaggaggtctcatatgacaaaatataatttcctacaaccaacccaattaagaaacggtgtcaccatcaaaaatcgcatcgcaatgtcgccgatgaccgagatgtccagttttgaagacggttcgatcaccggagacgaaatcgactacttccgattgcgtgccggtggtcccggcatgattattaccggctgtgccaacgtcaatgatctgggcaaaggtttcgaaggcgagctcagcgtcgcacatgacaacatgctgcccgggttatcacggcttgccaacgccatcaaaatcaatcataccaaagcaattcttcaaatcttcagcgccggtcgaatgagtaactcgcgggtactgcgcggccatcaaaccgtctctgccagcgcggtcgctccacaacgtttgggtgccgaacccccccgggccctttccgctgaagaagttgagcagaccattcaggacttcgccaacgccactcaattggccattgacgccggttttgatggcgtcgaactccacggtgccaacacctatttgattcagcaattcttcagtccccattccaaccgcagaacagaccactggggcggctccttggaaaaacggatgaacttccctttggcggttgtagatgcatgcgcagccgttatcaaacattctgataacccgcagtttatcttgggctaccggatttcgcctgaggaactggaaaagcctggtatcagaatagccgacaccctggccttggtgaaagaactcaatcaaaagccaattgattatctccacatgtcattggcagatgcttggcagggatcgattgtcgatcgtgatgaccagcagccgctcttcgaaaaagtccaagcagtcctcgcagatgatttaccattgatggttgtcggccatttggcatcccctgcccaagtcgccaagttgattgacgccggcgtccaatttgccgccatgggccgtgagttgatccgtgagcccaaatgggttcaaaaagttgaagctggtgatgaaaaggcaattcgctataccttctcattgcgggatttggacgaattaaaggtgactccgcccctgcttaacttcttgcggactgcgtttaagaagggtttcccgatctcgacagatgagaagcaaattcgaatttaattttattgattattatgccaatgagccattatttgataactgcaaattccaacgattacaatgaatcccaaccaggtacaagcccgcaacacatgtggtaatgacacatagtaatcaatcaaaaacatggcgatcgacgcaataatgatggtgaaaatatagaccgtgcgcaattgcttcactcctattcaatgtattttataaattcattgtcctctaaaaatatgaataaattgtgaattagccaaataaactgtaacattttcccaatcccaagtctggcaattacttcagccctaagtttcagttgtttgaactgttcccccttgacgtttagaacatatgttcgtatattaaacgtatgggggtgttcaacatgattcgagacgttccacgtgaccaatggctctacaacgaccgcggcatggtgaagtggctgggttactttttgagtgaccatacccaggatatggctgacaaaaaagtcgacgaggtcccgactcatcgattgccggaacaggatccggaagtcatcgaccgcgttttgcaggacagttggcagaattccaaacaaattacacttcaattaaatgatgacggctacttaaacgtttataatataagtggcattgtaattggcactaatggtgatctaatctatcttcaaaccgacaagttggtgaccatcaatgtcaatgatattcgccacgcgaaactcaaagaaggaagtaaatcaatttgaaacagaccatgagcgttccctgcaccaacaatgaaatcaccattatggttgactcgatcaactaccagtacttggcattacgccgggcatccttagatgttgctccactggaacaagtcaacgtcacgttaaccgacgaggacgtcgacggtcacgcctactacgaagtggctggctttagcgtcgcccaaaaagcccaactggcatccgttgatctggttccgggagactacgtcgtctatcgggcagtccccggtagtgagccaagcatggtcattcaattggttaataaatttgaccaagcaaattaattggagatgacagtcatgaacaaaggcacgcagttaatcgtaacggcgattgcgtcacttggctttttgggagcagtaacgacatcaacacaagcggcaacctggcacaagggaacgccaacagcactccgtggtcactggaaagacaagacgattaacattggtaaatactttggcatgaagaagtttgatagctatgaatctgtccgagttcgtaaaagtagtgtgaatgcctatttaacgcagtcagcaggctggcacattaccgataccaaatggaaagcagacggtaaaaccgcctacaccatcgtcggcagaaacgaactgaacaaactgcaccaagcccgattcacgttcaaacgagttggtcacggatacgttcacgtgtattatgacggtagtaacattgcggcagaaacgccattttcaccgaacttttatcgggtatctaagaaagcttaataaaagcgtggaattgcatgattacaattccacgtttttatttattctgcgattagtgattaactatattcctattgcaattatccattattaaaattacactatttagagttgctatttttcaaaacttataaaatacatatttggaagtcctgttaatgtcaaagcaaaatcgctattctctcattattatgatcttcggtgccttcttcggcattctctgttcaacgctcatgaacgtcgctttgccaacctttatgaaggtgttcgccatttcgtccggtacggttcaatggattagcaacggctacaccctggtcaacgcgattatgattccggtcagtgcttatctgaccaagaagttcacatttcgttctctgtttatttttttcgtcagcgtctttttagttggaacgatttttggtgccttggcacctaatttcttcaccctcatcattggccgcatgatccaagcaatcggtgccggaatgatgatgccgctggtaaataccctggcaatccgctacgccaagcccggcaaaaagggtgccgtgatggggatcgtcggcttagcgtttaacttttcgccgatcattggcccaacactttccggggttattttgaactatttctcatggcgctacctattcattttggtgctgccgtttatcgtcattgatttggtaatggccacgattgccctgcccaagatccccactaaccaggaacctcaatttaacaccgaggggttgatgaccatcagctttggtttgctgggacttctatggagtttttcaaacgtgagccagttccctatcacatctctaacagtctggctgccattcgtggtcggcgttgtcttaatcacgatgtttgccgtcactcaaggaaaatccgaccatccgtttgttaatttggcggtcttcaaaaatagtcagttcaccactgccactttggtcaactcactgattgtctcgacgatgtatggcaatacgattctgttgccgctgttgattcaaacgattatgggtaaaagtgccatcatctccggtctctcattactgccgggagcgctattaactggttttatgtcaccaatcagtggccggctgttcgatcgctatccggtacggatcattgtgaccaccggtattctaatcgattgttttggtaccatgatgcaggcattcattgatgttaacgcttcggtgttgatgctgacaatgggacagacaattcgccagcttgggctggtcttgattctcattccaattcagacccaagcactatcctatctgcccaatgaattgattgccgacggtgttgccgccttcaacaccttgcggcaaatcgcggcatcgtttggaacggccattattgtggccaccatcaacattgccagtcacttttttgctggccacgccaattaccaacagatgggcattcaagccggctttacgatgtgtttagccttcttggtcgtcgcgctctttatgtccagaaaactttacaccaaacagtcaccaaaacttcaccggaagtctcagagtaacttatcacacgtctcgtaacggagatgacttgagaggaggatggtcatgactaatttcatattcgtgctcctgcccgccgttcttgccgggattgtccagggagttaccgggtttggctcagcaattgtcttgatggtctttttgccgacaatcttgcccatcccccaaagtgccggagtggcatccctcattatgtccgtttccaacatcatgttggcttggcgttaccggcacagcatcaaattcaaacgaatcatctggccgtttgtcgtctatgccagtgtggccttcatggcattacaactagtcaactcaatcaatgtccatttgctgaaatccatgctgggtggtctgttggttgccctctcactgtactttttattcgttaaatcagaaggccggaaacattatcccatttatattgccattatctttatgatcgtttccggcttcttcaatgggttgtttggaattggcgggccgttgacggcactttattttctgtccttggcggatacaaaagaggaatatctcgccagtattcaagctttcttcttgattgatcaattgtatataacaagtattcgtttctataacggtattttaggtttaaatgacgtccccctcattctattgggaatagtcggtggcgtcatcggaaccatgattgccaaccgcattacggtccatatgaatatctcgatgattcaaaaatgcgtgtttgtgttgattggggttagtggcgtcttttacctggttcaatgattcaatctttactgtatgtataatatagcggcttgcacttggttgagaccagtgcaggccgctattttgatgggatattgatgaaattccgaaaattgtctcacgtattgactacaatccacgtaatcttaaagactcttgaggtatcttttcctggcaaaattaacaaccctcattgagattttacaagatgtccgtcatcataagggatatcagctaaacagatatgggaaagaattgcgttagtcatctggcctagcctttccgcatccagtcatcaagctctggggatttgtccggatcataatgtccttcttgatcaagctcaacccgctcatctggaatattagccaatagtttcttccagtcggacacctccggtacttttgaaagaaccacgttattattttgatcaatttgaatggataactttgtaccagcggaaatattcagtttatgcctcaccggcgctggaataactaattgtccatttttcgaaattgtcgccgtatattttgtcatggaatcctcccttctcaattacaacgtctcacattgaatctcatgctgatacattatacgaaacgacacatcttctgtcagtcatccaggtgtttaaaaaagcaccaaataaaagaccaggcacaaaccgccgagaatgataaataaacccccgatggctttcttatgccgaccaaccgacttttgatcatcgtggaaaagattcccagcaaccatccttgaccattttcccttgctcaccattaagcctgcgacgatcaaaaacaggccaacgccacatgttagtatcccgccgatgatattggatggtgtcattgtgtctgcccccctgtgagtttgttggctttattatatgccgggatggcgtgggtgtgtcattttttctatttatcacatcggttaatattcgttgggatttcagatattttagtcatacataaaaagcatccacggacaaactttcttgtgcgtttgctgtgggtgccttttttcattggtaagtgataggttcactgttatttggataaaatgtgctccgatggcccaacccctaacgtataaaccaaaaggacgaatcaatgaacaagaatcgttcatcaatccgtcctttcggcttatacgccgcggttaaccgggcctagtcgcactctaaccttgcgccttctccggatgcccttgcaggtaaataacatgagtattcaagaattcttcgataccatgacgaccatcatcgccgccgatacctgattctttccagcctgagtgtgaaccattcatagcttcaaagttaaatcggttgatgtaagtttcaccgtcttcgagttcgttggcagcacgcattgcgttgtccaagttctcggtgtagattgatgaagtcagaccgaagtcagaatcattagccatttcaatggcatcgtccaaagtcttaaaggtcaatactggcagtactgggccaaagatttcgtcttgcacaatttctgaatcttgtttgacgttggtgataaccgttggttcgtagtagaagccattttcgatgttcaacttgtgaccaccggctgtgaccttaccgccagcttgaacagcccgatctaccattccggaaactttgtccaaagcttcttggttaatcaatggacccataccaacgttttcatctttcataacgttaccgacagtgatctttgacatcttgtcggataacttcttgatgaactcatcggcaacatcctcttgaacgtatacccgttcacagttgttgcagagttcaccattgttatcaacacgtgagtcaatgattgattgaactgccaaatcgatgtcagcatctttgcagacaatggctggtgctttaccacctaattccaatgaaactttagccatgtgggttgcagcacctgccatgacccgtttaccagaatcaacagaaccagtcaaactaatgatgccaatcttcttgttcttggtgagttcgtcaccaaccacagaaccacgaccggaaataatgttgacaacaccctttggaatcccaactttttcaacaatcttggcaaattcaagtcccaagtttggcgtgtctgaagatggcttcatcacgatcgtgttaccagttaccaaagctggacccattttacgggcaatcaggaagaatgggaagttccatggtaagatgccggcagcaacaccaattggctgcttagcaatcatgatattttcattcttgttgtctgattggagaatttcaccttcataagttcgcgcagcactgcccatgtaatcgaagtagtcggctgagaacataatttcagtggttgccaatgacttgattttaccttgctcttcttggagcatttcaaccaagtgatccttctcgttacgaatttcagtggcaacatcgtgtaaatattggccacgggtagcagctggaactttcttccatgatttttcagcttcgtatgcagcatcgatggcttctttagcttcttcacgagttgcagctggaactgtcgaaatcttttcaccagttgatgggtttaaaacggtaatttcgttacctgactttgaatccatgaattttccgttaatgtacatttgataatgttttaatgcaacagcattttgtgccataatagttgctccctttcaagatacctgtcgaaaacagtgtaattgaacgccatctggcaggaacaaatatttttagtttattaatgaaacttttggatgccttgatgtgagtttgtggaaacgtgttacttgcctggcttgtaatcttcgtcaataacgagtactggcttgatcgtcttgccactgacagaatcagcgttagcttggttaatatcatcgaacttgtagaacttctcagtcttgtcgaagtcaaacaatcccatcttgtagaacttgatcaaacgagggatatcgacttgaggaattgagtcacccatgttgacaccaacgactttgcggtcgctgacacagagatcgttccaagtatccagatcaacgtgttggtcggtaacggcgattgttgcagtcgtgccgccttgtgccaaggccttgattgatgcttccatgacagatttaacaccagtggtgtcaaccgcatagtcaacaccgtaaccgtcagtcaaatcttgaatggctttaaccggatcagtgtctttactgttaatggtatcagtcgcacctaattccttggccaacttcaagcggtcaggaacgatatctacggcaatgactttggtgcagccggaaattcggccggccatcattgcagctaagccaacggctccagtaccaaagacagcaatggttgaacctggttccggcttcaaagtgttgaagaccgtgccactacctgtaacatagccacagccaagaggtcctaattgacgcaaatccaagtccttatcaactttaaccgcgttacgttcacggacaacagtggtcgtcgtgaatgaggattggtcaaacatgtcggcaacttggtgaccattttcagtaaagtgggcactgccgtcaggacgaacccccgacaagttgtttgctgcgtaattcaagcattgggttggaattccctttaaacagttgatacagttgccacagccataaaatgacagaacaacgtgatcaccgggcttgaagtctttcacttcagggcccactttttcaacaattcctgatccttcgtggccaagaacgattgggtaaccaatttcggcagttccttttcgtaaagcttcgtctgaatggcagatcccactggcaaccatatgaacttgtaaatcgtcagcttgcatatctgctaattcgacgtcatccttcatttcgaagtctccgccttttttgttaacaacagctgctttaattcgcataatcacatctccaaatactatatttgttatttagtgagcaattgcaaacaacagaaaagcaaatgattatccagcgcttaaatgagtgcgaatatgtgaattaatcatttgcttttttcaactaacaaccgcttacaatgcttattataggcggctgaaaattaatttcaatacttcttttgctttttatttgtgaaacgagctcatcaaatcacgagacccatactcccactttcagtctcataatttcaaaaaagttcgaaggttgtgaaacacttactaaagtttactgccattctccctgggttgggttgttcaacaacctgacccgaatcatcccgtcaatctgattaagttcatttaacaaggtctgtgtttgttgctgcgtgatttccgccaaatcggtattcacgatggtatagccataaccgtccatggtgtttcccatcatttcttgaaccggcaagtcatagcgactcataataccggcaacatccacccagaaggtatctctggcgtggaagaaaaacgtcagccgctggttactcatgaacggcaaatcaacccggggaaagttgaccgagcttctgacggtgccatattccaaaaagtccagcaggttctgcaaaatcaagttcgcagaatgggtcagcgcctcaattgtgttgccgcctaaatgtggcagcagggtaatctttggatggtcctggagttccgttttcggaaagtcacacacgtaaccggcaaactcgttgtgattcaaggccgagaccaccgcttgattatcgacaatctcgccgcgaccaaaattcagcagataagcgctatccttcatcatttcaaattgcttggtagacaacagctggttggtttgatcagtcagcgggagtaaaatcaccacaaaatcggcctgctccaacacttcatcaatggtatccaattgctggacgtgacgtagattcttgaagctgcggttatagccgataatctgcatccccatgtggtagcaggcgtccgccaaccgctggccgatggttcccaagccaagaattccaagtgtccggccataaagttcctcaccaataaaatcgccccgtttggcttcggcagcggcctgcaaatcctcccccggggcaactttgagctgctgcatcatttgaacggcaccattcagtggacgcagacatctgaaaaggttttgaataatgagctctttgacggcgttggcgttaacccccggcgtgttgaaaacggcagtcccgttggcggttgccgcatcgacgttaatcgtgttcgtcccagtcccggaacgggcgatcagcagcaatcgcttggatatcaagctatcatcaaccttggaactccgcactaaaatggcatccggggtatcggtgttggaggtacgaaagacgtctccagcaaaatcggtcaggtcaaaccgatcaatagtctttacttcaaacatttgtaagctccttttaactaaatagtgtgaaaacatattataatagtttttagaaattattttgagaaagaggttggtcgtatgcatattgattttgtaaagttgtcaaaagataaaccaacgattggaaaaatgactcaaaccaagaatactacattcggggaatgggtggaaataggaagcagcaatttaatcgataatagttcaattggtgattatacttacaccggccaatattgttttattcaaaacagtgacttgaaaaagttcatcagtatggcagcgatgattcgaatcggaccgaccaatcatccctacgaccggcctgcccaacacatctttgcctataacggcggggcttacggtttcgaccatccagacaccgaattcttggaaaaaagaacccacctgcggacaaccatcggcaacgatgtctggattggccacggcgtgatcatccaagctggcgtaacagttggtgatggtgccgttattggctcaggcgccgtggtgaccaaagacgtggagccctacaccatcgtcggcggcatccctgccaaaccaattaaggatcgttttcttgacgaaattaaaaccgatatggaagaaattgcctggtggaattggtctagagaggatcttgagaaatattacctcgatttccgtctaccggtaaaagaattcatcgataaacacctgcctaattaacgataattttgcacttacctgttcccaccaagcaaatctttgctataattaattggtatattcgcaaaggtacatattggaggagcatgagaaatgtctgaagaaaagactaagtcctgtgtcatgtgtgggaaaaccatcccggcatactcaaacttttgtccatactgtggcgccaagcagccatggcttgaagaagatgaagttcagaataaagatgttgaacaatttatgaagtggtaccaaaaaccggttggcaagtttatctcactggttgctgccgcgctcgtcatttattttgtcggcagtctattcaccctacaggacggcccgggtcataaaacggtggctcgtgaactgaaccagtatctgttcaatgcccaagataagacgccctacggcaagaaaccatccgttgaagccgataagaacaagggcgtcaccatcaaggtcagtcagaatagccaagcagtcaaagaactcaaggccggtaatccggacaaatggaactacctggttaaccgctcgcgggatcgttcaaaagctttccataaggtttacgccaaccaggcctatgccaagttcaaggtgatcgacaagcataacaagaagaaagtcttgttgaaagttgatagtggtgatatcaaatacaatattgccgataagtatcacaaataagctcggaaccaaaattaaaggcggttgtcacatccccaagcaagggaatgtgacaaccgccttttgaatttatttagcaatgacaatctcaggattttcagcattcaattgttgaagctgaccaacaactccaaaatattctttgcagagacgttgaatttctctgatggcaacatctgagcgggccgactgatcctcattaatcgattcaatatcgatgatcggattggtggtgtcctcggtcaattcagtccgctgattttcgcgccagttaaagcaacgacaaactgcgcctttatcgtccatataacaaatctcgccgggtaaagccggcatatcttcggtctcaccgtatggcaggaaggattcgccacccttggcttctcccaggtgcatatccccagcaatggcgtcgacgttttcaccaccaacggagacgccgtacttcagcgattggctgttataaatatcgactaacggcgcaatcggtgaaaatcgttttccgtgactgacccgttttaataaggcctcaatcgttgaacgggcgcccttcttggtcttaaacttccggaatgcttcccgccactcggcaaccaccggattatcacggaatgggtcaacggtgataaattgttcggccgcctcggtgccctcatccaggagtttctggaaatacgggtcgtccttttcattcacgtgattatcgatgccatgtaaggtcatcacgtcaatatggatgtctggaaataattcgatggttttgggatctaaaatgaattttttcatgaatgccggctctctccttcaattgttcggctcataatgaggtcgcgttggcggctttcgcccagcgtgaagacatgatcgccggtttgtttgaaaccgaatttttgatataactgttgagcgacaagattgtactcccaaacgcccagccaaacggtcgaacggtgtttatcttttgccaccgccaatgcttgagccatcaatttcgatccgattccttgtcgcttgaaagctggcttaatatagatgcgttgaacttccaaggcatggttgcccatggcttctgtctgggcattgccgacgttgaccttcaaataaccggctacttggccatccgccaaggcgaaaaagaaatcggaatccggatcggtgagctcttgtttgagccggtcaagattatacgattcatccaaatactgattcacgttggcaggactattttccggaccaaacgtatcagcaaaagtctctctgctgatctgctgcagttctgaaagatctgccaaagtacattttctaatcacaattgtcacaagttcatcctcaatactttctaagattgccttttttaacataatgccagtcatcgtcaatgttggcactaactttatgcaaaaggcgttccagttggtcggcctcatcgtcggtgatggactttagcgccacttggttggaatactgattttcccgcaaaatattcggataggtcgcctgacctttttctgtcggaaacaagcgtcgaatcttttggttggtcaaatcaggccgtttaactacaaagtcctttgccgccagcttatcaattgctcgggcagccgtggttcggtcgaccttgatcattcctgccagctggtcttgaaaaatcccggggtgctcacaaatcctggccaaatataaatattggcctttggtaagatcaaaccgtttaaattcaacgttggcaattgaatccaaggctctggcaatcgcaccgatgggtcgtaaaatctctgccacttaatcagccctttcttgatagaattgattctaaactatttttgttgtaaatgcaacattattatcagactgaagtcttcgcccgtcgctttttaatctggcgaaccacatatttccgcagctcttcaatcaggaagatcggcaccggaatgcagaataagaagccccattctgtgacgtttagcggtccggtattgaagacgccctggagaaatggaacgtacatcaacagtgcgactaagacaacttccacgacgatccccaaaagaatgcggtgattgctaaataagccaattgaaaagactgatgaaatctgcgttcggcagttcatcgccgctgcaatctgggagaagacaatggccgccaaggtaatcgtcgtcgcttccgcgtacaccaaaccggatccggccaatggaacttgaggccagccattgacgtggttgacgaagaagtaggcaaacgtcgaaattgccgaagcaatcaagccgtaccaaccaaaggctttccagataatcgatcggttcaacaagtgactgttcaatggacggggcggctgatccatgatgcctggctcggctttctcggttcccagtcccaatgccggcagtaaatcagttcccaaatcaaccgtcaaaatttgcataaccgtcaacggtaatggcaccagtccacgggtcaacaagaagatgaccgatggagcggcttcggggacattactagtgagtatatatagaaggaacttttgcaagttgctgtaaacggtccgaccttcttcgatcgcgctgacaatcgaggcaaagttatcatcggtcaaaatcatatctgcagcgtcttttgcaacgtcggttccagtcactcccatcgcaatgccgatatccgcacgtttgagtgctggcgcgtcattgacgccatcgccggttgaagccaccacgtcaccatttttctggcacatggaaacaatcctaaatttatgttccggtgcaacccgggcaaaaatgacttcccctttgacggcttcctgcagctcggcatcagacatcttatccagttcggagccggaaatgactctgaccttgtccgaagtaatgccaatcttagtcgcaatacttttggcagtcgtcgggctatcaccggtaaccatgatgatccggatgttggcccgtcgacaattgcgaacagcatcaaatatctctggtcgtggcggatctgacatcatggccagcccaatgaagaccatctgcttctccgcactttcaatcgtacagctttcaagtgactgctgacttagtggatcattttcatccaccacccgatacgaaaatgccagcgttcttaagccttgtttggcgtaattttcatttacctgcataattttagcctgatcatcagccgttaaaggtcgaatatgaccattatctaaaatccggtcacaaacgtttaattcactgcctaacgcccctttggtattgatgaccaacttaccgtccgcatttttagtgatgaccgacatcaatttacggccggaatcaaacggcaattcttttaatctgggaaacttttggcgttcggcggcggcatcaatctcggctttgcgtgacaggatcactaatccggcctcggttggggttccgagaatttttgatttttcaccggctttaccttcagtaacctcggtatcattattgatggttgcattaatcaacagcttctcgaggtcaggctgtcctgctagatcaacctggtggccatttaactgaatctgcccgttagtgacgtacccggttccagtgacatcatattcttgacttggcagccacagatggttgatagtcatctgattttgggtcagcgtgccagtcttatcggagcagataaccgtcgtctgtcccaacgtttcgacactgctcaggtttttgagtagtgcatgttttttcgccattcgttgggttccctgcgccaacgataaagttaccgtcggcaaaagcccttctgggataaaggcgacaatcatccctaatgcaaaaatgaaagacttggtcaccggatatttaacgaagaaaattgccagcaggaaaaaggcaacgccaatcataatcgcaataatcgttagttgccgggttaaatgattgagctcccgttccaatggatagacggtctttttctgtgactcagttaacgtggcaatgcggccgaactcagtatccattccggttgccaagcagagagctgtcgcagtgccgctggtacaaatggtcccagcaaagacgatgttctgttgagcaaattcgccatcgccgtgctgataagcgtcatgcttttcaactggcaccgattcaccagtcaaagaagattcgtcaacttggaggttggcagcattaaacaccctggcgtcggcaggaattgaatcccccgcttgaatatcaaaaatatcgccaggcaccagctgttcaactttaatctgctgagacttgccatcccgccgaaccttaacataagatggcagcattttcttcaatgagtcggttgccttttgagcggcgtgctgctgccaatatgaaaagcaaccattgatgacgttaactgcccaaatagcaattccaagttccagcatgccggcaaacatggcgatcacaccggatacccacaaaagaatcgccatcaaagaggtaaagttttccaaaaagattaacacttcggactttcgtttgccctgtcgaatcgtatttggcccgtatttttctaaacgcttctcggcttctgcctgcgagagaccaccgttgctggtttgaaactggttcatcaaatcagtgggatcagccttggcatcatcgtcaatcagtgtcgatttgttctgtttcattgtcaaatcaccccaatttttcaaattgttgacctaaccaactcaattatatcgcgattggagatcgtggtgatgattctgttttggtcaaaaagaaaaagtcagccctcatcaggttgactttcggtgaaacgtggttaatttaaatttgaaccggcagcagacttttctttcttaactttgcgaacattcgtcaaaacttctggtgtgaagagattgtcgaccaatgaatccgggagcagctgcttttgtttgacgagtgctttgacggattgttgagtggctaatgcttccttaatcaacgcggtcgtcttttcatagcccagcagcggtgaaagcaccgtcgccgcgatcgatgagtgttcgacttcctttcggcaatatgctgcattgactttgatgccgctgacgcagttttcaaccagcgtctcaattgccttggtcaaatgctgctcactagtcaaaatactcttgaacatgattggttcaaatgcattcaactccaactgcccgctctcagcagccattgtaaccgtgacgtcgttgccgatggtttcaaatgccacctggttaacaacttcggggatgattgggttgactttcccgggcataattgaggaccctgcagccttctttggcagctccagttcgttcaggccggcttgagggccactggaaagtagccgcaagtcattgctgaatttggataaatcagcagctaatgacttcatggccgaagaaatcgtggtgaaagcatcactgttttgagtggcgtccaccaaatcagcggcttgatgcaatgaaagatgagaatatttgttgagaatgggaataatggctgattcgtattcagcggtcgcgttaattccggtaccaatcgcggttccgcccaggttcacttgagaaagaaccttttgagcgtgctttaatcttgagagatcgcgtttaaacattgaagcataagctgtaaaggtcctgccaaaggtcgttggcacagcatcctgcagctgagtccgaccaactttgattgctgacgaatattctgcggctttatcggttaaggcgtcaaccaaactggaaacagctgacgtcaatggcgccaaccgttttaacatcgccatcttgcctgccgtcggataggtatcattggtcgactgtgactggttaacatcatcgttgggcttgattaccaagggctcttttccaccctgggcgcttaattgcatggcaagctgggcgacgacctcgttcacgttcatattggttgacgttccggcaccaccctggatggctggcacgataaaggcactgtagtcatttgagaatagcaattggttgcaggcagccataatcaaagcacttttttctttatccaaagtgcccgcctgctcgttagccaaagcagcggccttcttgatctgcagatagctttgaatgatggccggatcaactttttcgttggtgattggaaagttgtgtttcgctcgcagtgagtgaatcccataaaggacgttatcaggtacaaacatttctccgatgcaatctctctcaattctcattctattccctcgtttcatgtaatgttttgtgacatttacttacggctattaatatatacccatttttcagaaagtcaacagtcttcgttaaaattcctcaaattacaggtataccaatacctcacatcttggtgacaccattatcagaattttgcagtaaaatgagcaaattttggtcgatgtgatgtttggtgacattaatagcgattaaaaaaggccgaaacattggttgctgtttcggcctttccaagttattcacttgctatcgattaatctgtcaatcgtctgaaagagtggtatctgacgccttcacgaatgcaattcggtgattaaattgaatctgataataatcatcagtgccatgaatgacgttcttcggtgagttggaattgaagtgtgaattgaagtaatcagaggtgactgtgccgccataaacgtatttttgacctggctgcagttgataaattggtgttggtttaatgccggtaactttattcttcttcaaaatactgtcgcttggataggcactgccgtacaccggcacggcttttgatcctttagccgctacgagcttcccagtggcatcagttgaattagcaccacccggattgtagaaccaggcatcttgaccgccataatcaatttctgtccaatccccctgctgatcgatcttactaaattgttggccgtaaacggctttatcgccccagtcatccttttcagtggtgccggcttgaccggaagaaaagtccttatcagcaatcaagtcagcactgaagctaggttgcttgtagaggtaaacaaaatttgatccggttagcggaaggctgaccccgtcatcagtcactttttgtcccgaatcggccgtcaaattcgttttgtcattaggcgtaatggtgataatgtgactatccgtgctgccgtcactttttgataaatcaacgcccatcaattcaaagtagtgattccagttccaataagtcccaggatcccagtgcatccctttttgagctgccggtgttaaaccgggcacgttgtcatggccgataatgtgctgacgatccagcggaatctggtacttatcagccagatatttcaccaaagcggctgaggacttgtacatgttttcggtgtaccagtagccgccaactgccgcataaccctcgtgctcaatgccaattgaatgagaattaatgtaccagttgccggcgtgccaagcaacattttgcggtcgaaccatttcagcgactgtcccttcgaccgaactgacaacgtagttcgccgtggtatacgtcggtgtcgagaagagtgtcagagcttcttgaaaactggtttcggtgttgtgaatcacaatataattaatcttttcgtcgttcggccggtcagccaggtcatagttcccatagtcgccttgatcatcaaaggttttgtataatgcgggaatccattcgattggcaggccggcaggtccatcggtttggcccgattcaccggtggtatcgattgcttcatctttcaatgcattcaccttctggggtgagattttggcgccgttatgattgacgccttttgccaaaattttatatacgttggcggcgaagaaatcagcagctgcctgaaaatccgactggctgtatttcttaacggctgcagaccaactaccaatatttgacgttagccctttgcccgaggatttctgataggctgctaataaagccgccccaccatcaatattggcagctgaattggtcttcagttgactaacactgtgaccggtcaatttggccgctttttgcagcgtatgcagagaagcggcatttggcactttaaccgctttggaatctgcgccgcttggcgttaagccagtggtatcagtcaaatgcatcacaccatagccgccggccacactgggcttaccattgtggctatcaaacgcactttcattataagccaccgctttaagcagatctaccggcacctggtacttggcagccgctcgttggaaatctgtttccagcgaactggcctttgcatccaccaattgtgtattcaggccgatcaccattccgacaaatgcgatcacaatgaacaaccagcgaacttgcgaaaataaccactcgtgtttttccatgtcgtcactccttgtatgaatatccactattgtaaataatatttacaactaggatacaacgaacggcctcaaaaatatacttaaaattaaaaatattctaatcagtaagctgttcaatgaatggagccagtgatatatatcaggtaactatgtatttttgtcaactgtcattcgaaaacgaactaatcattttttaatttaattgacttcgattgtatgattcgttttcaaatgggtgtatactttttgaataaagattgtgcttggagggatgaatttgaaaacaatcaccagcaaactcatattgggacttggcctgacacttgcgatcggcgcatttaccttaacgccaaccgacactgaggccaaatcaacgatgactgtaaccagcaaccaggcgctcgtggcggatggcaactcccgcaattacctgacaaccggagcagcaccactctattcaaaagtgccggtctataagagtacaaaagttgtcaccaaggcagccgttttaaagacccttggcacaactgcggatgccgggcaaacctacttcagaggttatcgggcggctcagacctcaaatggcgactggtatctgaaagttgtttccttcgataaaacctatcggggctggatatttgccggaacaaccgatccgacgaccaatcccagtgatgtttccggcggcttaaaggcaacgacgaccttccaggaatcaacggtcccaacttattttgccaacaccacaatgtactttacgacaccaaaagcgtccacgttaacctacgttgcccctgactatacccaatataaagtggggcgcaatctcaacgcaacggcagacttttacaaggatccactgaccgtgaccaaggtcggcaccaagcaaaacaatcgcgatggcaatgccacttactactatgtaacagacgctgcccacccccaagtcaatggctgggttaagcaaagtgatgtgactacttcaagatgagagtgtgaaagaggacgtttagcaactaaattttaagcccctccagacggaaaccgagtcaggtttttgggtggaggggcttaaaatttagttgctgtcctcttgaacacgtttaatccaaataacagtaagacacaaggaaaccgagtcaggttttcgggtggcggcgcttaaatttcaattactgtcctcttgcacacatttaagctaaataaccgtggaattcaggcgagtgcgatgcgaggcgttttgatcctggccatttatagtagtaattaaaccaggtcccaacattcatcctcggagtaatataaaagatccagttaaaactgaaattcaagcagttttaactggatctaattttggattgttttcatttgacacaatcattcactttattaaaactttaggccaattcgccacgatcaatcaagcgactgttcaaaaactgataacgtttgggatcccctattaatttggagaacgaatagggttctttttcctgaagcaaaatgagcttaattaggtaattacgcaggatccaaggttcttctttttggcaatttttcaagtttaaaacgtcctgaatatgttcaggcgtgcttttcaaatcaacggccgccatctgcaaagtgatccctgacaactcgaagttgccttggagttcctgcttagttgcagctgcttcatctgaagttaagaccattctgtcacttcctcatcattgaactgatttaagcattctttgggaacacttaaatagcatgctaacacatctcaacttaacgcacaaatgaaggccacttttgctataatagaggttgcttcgctcaatattttcatgaaaattcaattcacgaaaaggtcgttcatggtactatatagtcattgaatgattcatttgatgtgtcaattcagataaaatgttcaatattcaacaacttctccaaatattcatgagcctgctgtttgtcggcatcatgatgctttaaaaagatccattttaaaaccagcacaaccgtctgactgcaatgatcgacgatcaattcaaccggtaggcccgccttggaataatcaattgatttggtgaggatttcctgcagcttatttttaaagtaattaataaaactgttaaccagctgtccggaaaaatcattgtactgaagcacgttatcgagtaacgtctggttatttttgaacacgtcgtaaagtcgatcaaaataggtgatcaacgttcgatcagctttcaattcagtcgcctgatccacttcaatttcttgggcaattacataccagcaatacgctgccaagtcgaatttatcgtcaaagtagttataaaaagtcgctcggggaaaattactcaccgcacaaatctcgttgacactaattttttcgaacggctctttggagagaagcgcgatcatcgtcgtcgaaaatgattccaaggttcgttgcgcaccacgcgttggtttctttgttaagtcatatttcatgagccagcctctgtttgcatttatcgaattttgtctaaatttaaactaacgcagcaaaatgtcccttgcgtcagattcacgccgagtttatcattttaatattgcttatacaagtgtctaaatttgaacaagagaataattttatcactagggaatgagaggaagaattttaatgcagaaattcaaagagaagcatctgttatcactgattgtgtggattggcctaattttggtggcaatttttacgttgccaaatatttcccaactggtccatgacaaagggactgttcagctccctgcttcggtgcagagtgaagttgccaataagattgagaaaaaatatgagggcggcaaaaatgcccgaaccctcatcgccgttttcaataacaagcacggcaagttgagtgatgagcagaccttacagattcaagacgccaccaacgccgtcaagaacgacccggacctgcacattatctccgtcacagccccaagtgacaaccaagctgccaaacagcagctgcagtcaaaagacagtaccacccagatggtcatgattaccgtgccgaaaaaagacaaggttcgtggccagactgataaaatcttggataagattaaaaccccgggaatgagaacttacgtaaccggtagtgatgtcttaaatgaggatttttcaacggttactgagcagggacttcaaaagaccgaaatcattgcggcaatcttcatcttcatagtgctgatcatcgtctttcgttccttcttaattcctgtcatttcattactgacagttggtgtctcctacctgctgtcattggacgtggtcatgaatttggcccagcgctgggatttcccaatctccaactttacccaagtctttctggtggtagttctgtttggaattgggactgattacaacattttattgtatgaccgctttaaagaggaaatccgtaagggtcaaggcgcaaccgacgcggcaagaagtgcgcggcgacatgccggacgaaccattctgtatagtggttcatcggttttaattggttttgcggccttagcattggccaagttctccttctaccgttcaggcgttgcggtcgctgtcggagttgccattctattaatggttctgttgactctgaatatgttcttcatgtctaccttgggagaacgactcttttggccaagcaaaaacctggctgcccatgatcgaagtttcctgtggaatttcctctcaaagttcaccctctcacacagtttcattatggttgggattttaatcattgctgctttgccactgttgttcgttggcagtcagaaactcaattttaacagtgccgatgaattgcccaactcggttcagtcaaaagcgggttataacatcattcaggatcactaccctgctgggatgtccggcccgacgaccgtctatattcaaaacaagaaaccactggatacccaacaacatttagccgaaatcgaccaattaaccggctacctcaattctgaggccggggtcaagagtgttgcctcagttacccgtccaggtggaaccaagattgattcactttatctaagaagtcagctggaaagtctgacgaacggcttaaaccaagccaatcaaggtatcaagaaagttcaaaaaggtttaaagagtgccaacgaaaaattagccaactcaaacacttctgaaagcatcgcacaagttgagaaattagctgacggtgccagcaaactagaggccggtgcgcaacaactgagccaaggtgtcacctcatacactgccggtgtcagcaacttggccagcggttcgcaacaactcagctcaggcacctccagtcttcaatccggtgtcggtcgattgtcagctggtagtcaacgattgaacacggggatttctcaagtgagaagccaaaccgctaagctaaaggcgcttcgtgcccggatggccgcattgcagtccggatcaagacaattatcttccggtcttggccgcttgaattcacaagttgctccgttctcaaatggcctgaaccagattacaagtggcgctagtcgactgaattcaaacagttcatcactggtttccggggctcaaagtgtcgctagtggcagttctcaagttaattcgggtgttcaaacattgaattcgaaaatgaaagagctccagagtcagatgcaggaattacaaactggtttgacttctgccaattcaggattagatcaagtttccagtggaaccaccactgttaacaagtacttgaaggaaatgcaaaagtcatacttgggcaacaccttctatatgcctgccgcaagtatcaagagtgcgtcattcaccccttctcttgacgcatttatgtcaaaagaccgtaagattaccaagattactgtggttctgaattccgatccaagtaccaccaagtcggctaaccggattcggacaatcactcgcgatctgaatgccaaaatgaaggacaccagtttgaaaaatgctaaggtcgctatcggcggtcaaagttctcaaacttctgaccttcaaaagattgccaatggcgatttcttccgaacggttgtcatcatgctggtgggaatcggtttagccctgatggtggttacccgctcactggttcaagccattaccattattggcaccttaatcgtgacctatatgggatcactgcagattaccaaatggctttcgggatatctgctgttccagaacatgctgacttggaacacaccgttctttagttttatcatgttggtggcattaggagtcgattacagtattttcttgatgatgaggtaccgtggtgatgccggcgccattccggatgtccgtcgacgaattttaaattcggcaaccattattggaacggtcgtcatttccgctgccatcatcttgggtggaacttttgccgcgttgattccgtcaaacgttttgactttgattcaagttgcgatgaccgtgattgttgggttgatcattttggtattgaccttgccaattatcatgtcggccatggttaaatggacctatccatacgtcaacgataaaatgtatcaaaagtccgttgataaagaagaaaaagagcatccaatcagaagaagtaaagataaacaataattgcattggtgaggctcgttgaccaaagtcagcgggcctttttttctgcttatttgacaaagccacacttggtacgctatcattttttagtataatctaaagaattagccaactttgtcaaaataattctgtttttgatccggacacttttaggagaatttaaatgaataaattgttgaaggttgctgttatcacagctgccagtttcatttttaccattttcgtcaaccaccagcctgctcaagctgctgacacctattatcatgttggtgccattcacagttcgacgccgaccagctggcgcgggaattggtattcatacgtcaacgggaagttctgtttgacccagattaacaaatacgccgtcacccaaaaatacaacggcaagcagcataccctttataaatccacttggaagagctatcgaaaattagctgttgctaaaatttccggtacgaaccggtacacgtttaacgcctatgcgaccaaagcctatcagagtgaccgtggctggcggaagacccaccgaactgttgagggccaaaagatcagtgttctccgggattattccggtgggggtgcattcgtcgatcttttccgttcgccggtctacaaatcctattccaatcactaaggagttactcacatgtcgacaaatcgaattgttaatgctttatcctatctttcaattgtcttcgcaccgtttatttttccactgattgtttggatcgtcagcgataacaatccagatatgcacagcactgccagacacgcgcttattttgcatttaatcccccttgtgctgaccatcctgaccatcctggttgtcggtatcagtggtgtgatttccgaaaaggccgcctttgccggatttcttttcctggcgctaatcgcgttagttatcctggtggatctggccatgttcatttataatctgtatttaggaattaaaattttggtccaagattaacgttaaccatccaataaagggattgccgccaaagctcagactttggttgcaatccctttattgtatcggagacaccgttgaaatccaccaattcagttgggggaataaatatcgatgccattttcttgatcgctaatgtaatagtgcttcggtgaacttatcaccagccataaaagataaaaatcaccgacacaacctgccccatgcagggctgccaatggtaagaataattcgccaggcagccatcccaaaagaaatatcgcaatcaggacaagtgaaatgacgacaaatggagtcgccccaatccaaataaattgctgcttggtatagagggacttggggctggaaacggataacatgccacttttgaaaccaattttaattttcccatttggcttaaagactttataaagaatcccgtgcaaaacctcgtggatcgtcacaatcactaataatgccacgatcagccaaacgaagtagctttcagtgaagttgacagtcattgagccgacaatggcaccaaacagccacaggaagcctaaaaaggcaataacggcgaccacatttagaccataaaccaaattgcggttattgctaatatcaacgtgtttatataaatgcacgattgttcaccccattttgctatttatcatcagtttaacatatattaaatcaaaaaatgactgttggcaggcgattccctgccaacagtcatttgacttcttagtaataaataaatacgggttccaaagtgtgcgtgttcttccacacctcacccattcgtgacggtggattattcaaacagccatgagaatggtattgtgcacgagcacttggattaccatagaccgaggcgggctgccatggtgaatcgtgcatcccaacccctgaattggtcaatggttcccagtagctgactggtgatgcatactttgaaccatcactgttcttccctctcaaagttgcgtgacgctgcttgtacataatgtaaaaggcgccttgaggggttcggttaccaccggtcaacgttccagacatgattggaatattagccatcagcttaccgtttttataaacgtattcatggagacgctgcaggtcgatggcgacataggtcttaccagaccccttaacaccataaccggttccaaccgcatagtgcttcaggttcattgtgacggaatgtgaacgaccaagattcttcatgatatttttggttaaagccgattgattaactttccagccataggttccaccagcatgaacacgaaccctcttgccttgatgagtggtaatccaaaccgacttgccaagggtatcgactttattggcaaatttggccacccaattcttaatcttggttgaatcaaacttataggtcccgttagcagttgggtaaccattggcaacccagcgtttggcaacaaacttataggtcttgttgtaggtattcaacgtgacagtgttgtccaagatgttggctaactgtttcttctgtttggcaatttgagtgctattcggcttgacgtacgcatctttagtcattttaaccgaaatcaataaactcgattttgcctgcttcttaaagtctttgaccatcttggccttatccagagtgcttccctgctggccagcttgaacaacaattttgccattcttcaaaataacttttgaatcaatggtctgtttgcgaccggtattgatttgatcaacccggttttcaaacttcggcagtaacgtcttcaagcggtaattgagttgcttgttggttacatcagacttggcactcagcttggcagaagtcatcgcactcattgaactacggtgtttgaataatttcttaacatccttggaattcacattgatttttgaatcccgaaccactaaataattgccgtcttcatcgatatgtgaggtattcaacttcttggttgcctgagcgaccgtcaaaccggaaacatcaacgtcgttaatcttggtgaacttgaaatgattttgaaaatagaaatgagagcccacgaagccaccaaaaagaaccaacacaaatcccaccaggatccgtatccatatttttttcttaggctttttagcgaacttctctttacgtgacattactaatgccaaccccctttatctgtctctaagcatattttacgaagttttagcacttcaatctagcaaaagctctcgccaaatcaatacttaaacaaatcttcagttttctctcataattttggatcatagggtttcatgttaccattaatctgacaattaattaagtcccgatcaggattggcagcttgaaaaggtcattggtagctgttggaattcccattcccgtcagaactggagccacttttcagtcccagacaaatccttaactgctcattcatttttttcattctggaataatcaagatcttatttactattcttccgtgaacctgtatattagtcttaatctttatcagtcgggagtgatagatatgtcgtttgaaaaagtgaaacagtactttgacgaggttggcttagccgatcgcattaaagtcttggatgaatccagcgcaacggttatggaagctgctgaagcgttaaattgtgaaccggaacatattgccaaaacaatgtcgttcttgattgattcccatccactgctggttgtgttggccggtgatgccaaagtcgacaacaaaaagttcaaggccgaatttcacaagcgtgccagaatgatcccaagagatcaagttgaggaatatattggccatcaaccaggtggtgtttgcccatttgctctcaatcaaggcgttaaagtctatctggacgtttcccttcagcggtttgaattcatctaccctgcggcaggtgacacccacagtgcagtcaaattatctgtcgatgagctcagcaaatatgcaaacgccgaccgttgggttgatgtcggcaaagattggcctgccgatcctaaagtatcgccaatcagaggataaccagctcaatattaaagttcaagaagtctattttgaggagcctattatgaaattaatcgtggaaagttccaaaccagctcgtggggctgctgcttacattcgaatgtccgtttttgtattggagcggggaatcgcctttcgagatgaattcgatgacaaagattccgacagcatggtttatgcggtcttatttgatgacaaagtgccagtggcgacttgtcggtttgaaacttacaatgaccacacccttaaagtcggcagagtcgcaaccctaaaggaagcccgtggacatggctttggcagaaaggttgtcagtgcccttgaagacaaggccaaacaaatgggtttcactcattcactgattcatagtgaaatggacgccgtcaaattttatcaacgcctgggttatgagatcacgtccgatgtgttttatgaggatggcgtgccttgtgttgtggtggagaaggatttgtagtcttaacgacgggcaacgatgaacagaaaacgttcatcatgcgtgttcgattttctttggttttgtagcctacagggtttgtaacgctcattatatctacagctcccttcggcctttgagatacgctccgacgaccccgacccctaatatataagtcaaagacagccctgatgaacaaaaaacgttcatcaggggttgtcttttgtcctttagcctacaggggttgtaacgctcattatatctacagctcccttcaacctttgagatacgctccgacgaccccgacccctaacatataagctaaagacagcccctgatgaacaaagaccgttcatcaggggctgtctttagcttatataccggggtcaaccgggtctcgtcgcgctcttagtttttaaacgaatgaatcggtgccgggattcttcctcccctttgaacgaacttcgctgggctgttggtgtttaccggcattaccggcgcatagccgaatatcccgccgaagtcaatttgctctccgacttgcttgcccttcgccgggatcacccgcaccgccgttgtcttattgttaatcacaccgatagctgcttcatctgcgatcatcccactgattgtttcagccggcgtatctcccggaacagccaccatgtccaatcccaccgaacaaacagcagtcattgcttccaatttttccaaattcaaattaccatgctcgacagctttgatcatcccactgtcctctgacacggggataaaggcacctgacagcccgccaacatgttcacaagccatcacgccacccttcttgaccgcatcattcaacaatgccaaagcagccgtcgttcccggggcacccacgctttccaaaccgatttcttcaagaatttcggcaacggaatcaccttgacttggggttggcgccagcgacaaatcaacgattccaaatggcacgttcagagctttagcagccacattaccgacaaactggcccattcgcgtgaccttgaaagccgtttttttgatcgtttcggaaaccgtgtcaatcgattcccccttgacctgttcaagcgcccgcttaaccacgcccggaccactaatcccaacattaatgactttatcagcttcaccaacgccatgaaaggcgccggccatgaacggattgtcttcaaccgcgttggcaaagaccaccagactcatacagctgaccggatcgatttcagacaaatctttaaccacttggcccatttgtttgacggcatccatgttaatcccggctcttgtagaaccaacattaaccgagccacaaacccgttgcgtctcactcaaggcttccggcatcgaagtaatcaattttcgatcacctgattggtagcctttttgcaccaacgcggagaagccgccgatcaaatcaacccccagggtttcagctgccttttccattgtctgcgcataggcgacataattatcatcgtgacacgcggcagcaatcatggaaattggggtcacagaaatccgtttattcacaatgggaatgccatactctgattcaattcgatcagcaaccttcaccaaatctttggcactggtcgtcaatttatcataaattttttgccgggccttaacaccatcgctatcaatacagtcgaatagtgagattcccattgtgatggttcgaatatcaagtttttcttcagaaatcatctgaatggtctctaaaatttgtttggtttccattttggcgacctcctaaagcttttgaatcgcgtcgaataattcttgacgctgaatattaatcgataggccagtctcatttgccaaatcctgtaagccctgtttgacaacttcaaactgcacatcatcatcgtcccattcgcccatgagcatcatggtaaaatcaccatgcatcagcgtctgggaaatatcggtaatgttaactttcaaagttgccaaccgttgagaaacttttgccacaatgccaatttggtcatggccaatcactgtaataactgctttcattgtctgcatcctttcaaattccgtgagtttggttatctattattaattgcatttatcatacccgatattaagtcactcggcaatttctaatttatcctaataaattatgtgtaaagacaatttatacttacaaataatgatataatataaattaatttacaacaaaggatggaaaatcacatggcaactgaaaaggaaaaatttttagcgggtgaaccatacttggtgatggatcccgaattaaccaacgacgaaactaaagcccgccgcttatgtaagatgatgaatgaactggacgacactgccggtgcggaaaaagaggccctggtccgcaaactgtttggctcagtcggaaaagacccctgggttcaaccgaacttccgctgtgactttggctacaatattcacgttggcgataactttatttgtaactacgataacgtcatcttggatattgccccggtaacaattggtaatcactgtatgctggctccacacgtgcaaatttacgcggcttatcatccccttgatcccaaacaacgagccaactttgtaggactgggcaaaccggtgactttgggcgatgacgtttgggttggcggcggatcggtgattctccccggcgttacgcttggcaacaatgtcatcgttggtgctaattcaaccgttaccaaatcatttggagataacctcatcattgcaggcaatcctgcccgcgtgattcgagaaaatcccaacaaagaataattaatttcaaatttgctgttgacaatcaaaataacagggtgtaaattaatgacaatcattaaattcaaattaaaaagcgatgaagagaaacgtcattttccgttcgtaataagagagttgctggttggtgtgaagcaatttacgtccttagatgattatcatctccgagctatgtgatcaaagttttagtagattgcattgggtgcacccattattgtgtcagcgtatcgcgaaagctgtacgtgtgaggtaatgctagtaatagcactacaaattaaggtggtaccgcgcaataggcgtccttttaactatccatttccgggtagttgaaggatgcctttttatttgaatttaattaattatttaaggtggtgaggacttatggaatcggtgattagcagctccaatgaaaacccaggtcagattcagattttgcaaacacataatttcaaccgacatagtgccattgacataacaacacatatatttcacgtcactgagtggtcctcactgtacatacagttgaggatccacagattaaatacaatttatggaggaaacgcttatggatgaacaagcaacgatggaattaacaactaaggaaaatgaattagcaaacaaattatttaacgcttacgagacacacaagccattaaaagagtccgactatgatggtgtcgttaaggatgaaaagtcagcctatcgggttcaaagacgactaacccaactcaagcaggaagacgttggcggctacaaagtatcgcttaccagtaagcaaactcaagatatgtttgactccgactcaccactatatggcgcccaagttaagagccatttcctacaatccccagttacccttcaccgtggcgaactcatggaaccacttgctgaagttgaaatgctctttactgccaaagaagatctcagcagcaaagattctttagaagatctcatgagaaagaccaaggttgctccagccgtcgaagtacctgattcacgcttcagcgactggttcccaagcctatctaaatatatggtcatgtcagatgcagccgttggtggctacgtcgtttacggtgatgaaaaagataccaatctcctatttgacaacgtcgatgatctagccaacgttaaatgtgaactattccatgacggcaagaagctaaaggacggcgcttcatcagaagtattgggcaatccgttaaagtccctccactggttagttgaaaagttggaatcacaaggaatgcccctacaagctggccaacgcgtttcaagcggtactttcctactacctgaatcactcagcaatggcgactggaaagcaacctttgataagggacttggcgccgtgttcttgaaagttgcaggtgattaactcagatattttttaagcagcaaattagcgtctgattatttttgaaatattgatgaaattgatgataattgataaaaatgaaattgaagcggctcttctcaaggcggaaaacttgggaggggcgcttttttgtggagttactgatctttttggggttagttctacccagatacaattttccttatacataaatcaccttccttttcccatgttattttgggttagattccaccaagtttgttgcgcttattatatttactgctcccttcggccttgaaaatgcgctccgacgacccagggcccggccacataagtgaggaatgccaacgatgaacccagaccgttcatcattggcattcctcacttatgttctgggccctaaacgggtctcgtcgcgctctgttttcaaaatgcgctccccaagccagcttcctccgctttatccaatcacgagtattgatgcctaacccgcatcaacactcgtgattacataaatgctcagaagctaaccggcttggtccgcgctctgtttttcttgacacaccaaacaaatgttcgtattatatagatactcaataaaacttttccaatcgcaggtgatccttatgcaaacacctcttgataatcccagccttttgcccagccacgacattatgtgcattgactgcaagtcgtttttcgcctccactgaggccatcaagcgcggggagcatcccctttccgccaaaattgccgtcatgagccgcgaagaatcctccggtggactcattttagctgccagtccctacaccaagaaaaactttggcgtcaaactggggactcggcgatttgaagttaatgatcagatggatatcgaaatggtggaaccgcacatggccgattacgttgcccttaactaccgaatcaaccgcatctaccgtcaatttaccgatgatattcactggttcccctactccattgatgagagcttcatcgatgtcagccacagccacaaattatttggttccaatgcccaaattgccaaattgattcaagacaaagtttttaaagcaaccggcattgtcacgacgattggcatcggacaaaatcccctgctggccaaactggccttggataacgccgccaagaaaaaagaaccttggcaggcggaatgggactacgccgacgttcccgatactatttggcagattccagatcttgccgatatgtggggaattggcagccacacggccgtcaaactcaatcagttgggcatttataccattaaagaactggcccacgccgacgttaatctgttaaagaagaaatttggtgtcatgggcgaacagctttattaccacgcgtggggcattgactactccaaccttgagaagcgttatcttccccgttcagacaataaaggttacggcaattcacaggtattaatgcgcgactacacggaattgggtgatctaaaaactgttttcggtgaaattgccgatcaagtcgcgacccgcctgcgaaaaaacaacgtcgtcgctgaagtcgtcagtattttcatcgggatggccaccacagacaagcaggggcgaacccacttctcagcccaaatgcacgttgaacccaccaactcaaccaaaagcattgccaatgccgtccactatttattggaaagtaaatgggacggcagcgcagttcgtaacgtcggggttcgctgcaatcggctttcaaaaaagcgtgaaacccgcttcagcctgtttgaggatcctatcactaccttggataaggaaaaattggagcaaaccatcgacattatccgcaaaaaatacggttacaaagcactaatcagagcttcgtccaaaaccaaaggcggtaccgcaatcgaccgtgccggtttggttggcggccatcaagcttaacgatttatctcaaggaggtcttcaccatgctggcagaatcaagagaactaattgacaagtaccaccaatacttcaagcgacttcccaactaccaatactggttggtgatcgtcgacaaccattttaacgaccgttattacttcttcatttatagtcggaaattaaaaaccaagttggtccgctcacatgagttattagcattggttcacgatccccacaaatatcagcaggttctctccgaccttaaaaacatgagtcatctaagcatcgaatacagggatacgacccatctggtagaaccaatgccagagattaccactgataaaatccacggtcacaacttctgagaagcggccaaggccataagtagcaaattatcaatcggatatggtatattaatggaaacacttgcagctttgaggaggcacgttcaaatgaatcgggtcgtaaaaaaattaacgttgctggcagtcggactgctttcgtttgcattgatgattgatgttgccgcaacctcggctgatgcaaaaaccacagcggcaaaagttgtccgggtcactccccagaaaagcacagcctatcgagcagtcaaagggattatctatggggataaaacgctaacgcaaaaacttcacaacgctaaaaattatccggaaacgatcttctacgctactaaacgggtgaccgtcagaaagccgaatggtaaaacggcagtctactattatgttgccaataaaagcaaaacaataacggggtatatttggcacggctatttaaccaaaacgcaagtggcaatgtctcagaagtcgctgatgaaattgagtaatgcagccccagacatgaatccggatgaaactatcctaagtctgaaaccggtgaactatgaaacccatgaagctgtttttgacttggcatataacgtttttcatttttcgccaacctcaatgttcaaggatcatcaagcgttgatttacgtggccaatccagaattgaaccagcacgttcaaaacgccatgaacaaatggaatactgccttgggtgaaaccgtctttcagatgggaagccaaagccactataccttaaagatttcatttggcagtgggacaaaagaaggctgggatggtctttacgacggcaggcaaatttatattgataaagcccactatcacgatgccaaatatccgctggggtatatcaaacccagtctagctgccaaatttacgattgatcaatattgggatggtgtcctggcacatgaacttggccatacccttgggcttgaccacaccggctatcaggcagacttaatgtatgcagcgaccagtgccggcaatatgattgccaaatatgcatggcagaagccggtcgaaaaatccatcaatggattggatggcaccgaaatggccacgatcaccaatcgcgatttgaatcgagcaaaattgaccaaacttcttggttactggtaactatggaggcggccaaagatgcttggctttgagttccacgattatctaaaataaagctgcgcgatcggctgattttaacgatttaggcaaacgagcgtgggcaaataagcagttagcttccagagtataaggggattacccaaatatccagaacttggatgtttgggtaatccccttatacggccggaagctgcttattggcgcacagttctgctagataacatttaggcgcaaaacgaggttgctagtaaactctaatcaaataaatgcagcttggcaatccgctgacaagcttcggtaaatcgcggctcgtcaattaataagcccacccggacgaaaccttctccgccttggccaaaaccgttaccaggagcgacagccaccgctgctttgtccagcagtagatcggcgaatgattcgctggtatagccctcaggaaccggcatccaggcataaaacgaaccgccggatggatagggttcccagccaattgctcgagcagccttgaaaaattgattccggcgtttttcatagagggcaaccaactcatgaacggactgctgatcgctattcaaagccgtaatggcagctttctggatggctgggaagacactcacaaataaatgatcttgaatcagattgatggcttcaatcatatcggcgttcccggccgcaaacccaatccgccaaccagccatattataggatttagagaaagtgttcatttcaattccgacttctttggcacctggagtttgtaagaaactgaccggttttcggccgtcaaacccaatcgccccgtaggcaaaatcctgcaccacaccaatatggttggtcttagcaaagttaaccgtctgctgatagaattccggcgtggccacagctccggttggattgttaggatagttgagatacatcagcttagccgcatccacgacttcgggtttaatggtccgataatcaggcaaaaagtcgtcttgttcacgcagcgtcatcagctccagtttgacttgtgccagtgaaacgccggacaggtaatcgggatagccgggatctggcagcagcattgtgtcccccgggttcagcagtgccaacggtagttccaccaacccaatttttgaaccgccgagaatggcgatttccttatcaggatccaaagtgaccccatattcacgttgataaaagttggccgctgcctgttttagttccgggtcacctctgaattgcgaatacttatgattggcaggattggcggtttgctcctgcatggatctgacaataaaatcgggagtcggctgatccggattcccctgacccaagttaatgacatccgcaccggtggccactttagcattgaccttcttgaccagaccggcaaaaaattgtttcggcaactgctgtaaaacgttcgattcttcaaatttcaactgatttcctccaatgtggtatgtataaatgatcataaaaatgctaaatgaattttaatgattattatgataaactgccaaatcaatgtcaacacattttctaatttaaaattaataattctcagcgttttgcaatgtcgcagcaagcttggcaccgtttgcacaaattggttaatgctatacagattcacaaatttctggtattatgttctcattattatatgttatgttttattacatatgtctaggaggaataattcatgaagcgcaaagtgttaacggctttcggattgctggcagcttttgccacgatcttgttctgtctggcactaccaggcagcaaagcacaagctaagacgtaccaaatcgggacggatgttacttatcccccatttgaatttgccaacaaggaaaacaaatacgttggaatcgatattgacattatcaagtcaattgctaaagaggaaggctttaaagtcaatgttaagccggttggatttaacgcggcggtgcaatccgttcaatccggccagcttgacggaattattgccgggatgacgatcaccccggaacgaaaagataagtttgatttcggaacaccctactataagactggtgcggtcatggccgtcaaaaaaggcagtgacatcaccagtttcaaacaacttaagggtaaaaaagtggcgctcaaaaccggaacggccgctgcggactatgccaatagtttgaagaagaagtatgggtttaagaccgtgacattcgatgattcagataatatgtatcaagacgtcacgaccggcaactcggttgcttgtttcgacgaccaacccgttctccagtatggcattaaacacggtttaaagcttcaaattgccagcaagcccgctaaccaaggttggtatgggtttggtgttaaaaaaggcactcacaaggcattaattaagaaattcaatgccggcctgaaaaagattcaggcgaatggaacttacgacaaaattgtcggtaagtatctgggaaacgccaataattccaaagtaaaaggcaaaactttcgttattggaactgatgttacctttcccccatttgaatttgccaacaagaataacaaatacgtcggaattgacatggatttaatccgagctattgccaacgaacaaggctttaaagtcaaaattaaagccctgggatttaacgcggccgtccaagccgttgaatccggtcaagcggatggtgtgattgccggaatgtcaatcaccaacgaacggaaagcccagtttgacttttccaaaccgtacttcaattctggagttgtcatggctgttgctaagaacagcaagattcataaattgtcagagttgaaaggtaaacgggttgcggttaaaaccggaacctcgggtgccgattatgctaatagcatcaaaaagaaatacggctttaaagtggtcacattcgatgattccaataatatgtatcaagatgtctcaaccggcaattcagttgcctgttttgaagatcatccggttatgcaatacgcaatcaagcaaggaaccaagttgaagattgtcaccaagcctgcattgaacgcaccatatggctttgcggttaaaaaaggtcataaccaagcacttctgcaggcgtttaaccaaggactggcagatctgaaggccagcggcacatatgatagcattaaggccaaatatttgggtgctgatgagattaagacagctgccaagacatctggcaacagcgccgaagaccggacgtttatcggcttaattaagcaaaataaaggtgccctatggtcagggctgcaagaaaccctttggctgacagtggtatcaatcttctttgcaaccatcttcggtgttttggttggattgatgggcgtggtgcctaacaaattcagtcaaggaacttcgacaacgttgatttacctgtttagaggaatgcccctgctggttttggcactgttcatttatactggaattccgagtttgactgggcaaaaaattcctgcctttgtcgccggggtcgtgacgctgacctttaacgaaggtgcgtatatcgccgcgtttgtcaaaggcggcattcaagccgtcgatcccggacaaatggaagcctcgagaagtttgggactgccgtttggaaaagcgatgcgtaaagttatcctgccacaagggattcgaattatggtgccgtcgtttattaaccaattcattattactttgaaggatacgtcaatcctatcaattattggtttgcttgaattgacccagaccggtaaaattattattgcgagaaacttggaaggattcaaagtctggacaatcgttgccgcaatttatctgattattattactgtattaacttggttatcaaattgggtacaaaggagaactaaggtatgagcgaaaaagtaaaagtcacaaatttagtcaaaacctttggtgacaatgaagtcctcaagggcatcaatctaacggttcaaaagaatgaagtggtcgttatcatcggcccttcaggatctggaaagagtacccttctccgcaacctgaataagttggaggaaccaacttctggatcgatcgttattgacaatgtcgacattgccagaaatgatgttgatattaacgcggtacgggaaaatattggtatggtgttccagcatttcaatttgttcaaaaacttatccgttggtgaaaacattatgttggctcctgtcgaactcaaaaaggaaaccaaggaccaggcagctgttcaggctaaaaagttactgaaaaccgttggcttacaggagaagttcgatgcgacagttcaatcattgtccggtggtcagcagcaacgagtcgccattgcgcgggcattggcaatgaatccagacatcatgttgtttgatgaaccaacctcagcactggatcccgaaatggttggcgatgttctagcagttatgaaggacttagccaaacaaggaatgacaatggtcgtggttacccacgaaatgggatttgccaaggaagtagccgaccgggtcgtgtttgtagatgacggtcaaatccttgaagaaggtaccccagaacaaatttttgaacacccgcagaatgaacgattacaggatttcttgaataaaattttgaacgtctaatagattagatgattaaattgatcagcccgttacgaaatatttcgtgacgggcttttttatcgtcagttgacattttagtgtgtcgttcaatggcatacactacgaaaggatcgtcagacattttcggatcctcatatgggggtctctagaagcaagtcccccatcagtgctcaagtttcttgatccttattctagctttaaccaaatcgatcttccagttcgtctgttaacagatgagattcaactgtataataaaaatgaatagttgttcgcattttatcgtattacgacttatgcggccgattgatttggccaacgaaacattttttgagggggatcacaacgtgaaatcacatcaacatatcctgctaacagccgtcatattgattgccataactggcggcttggtgggttgcagcgatggcagtggcagtcatcaggccgccgatcatcacgcatcgcaggtggctacaaccagtagttctcatgcaacccaatcagcaaaaaaagttcatactcattcacaccacagttcaactgcgtcggcaagccaacagcaccaagccattttgaacaagctggtgagttataccaacaaggaatccgccgggccgactggtgattattattggacaactggaaaagctcattttagccattttgccgggctggcagctggtgactatcatttctcagctgatgcccaaggcagatctgcgactgcccgagcagtgctgacttattctgaatatcatctgtcccagggcggtcgtcaaggagatccactggaacctcctgcatggccggaaaacaagatggtgtcaattacctatggactgacggggcggacctaccatggctacctttacaaccggagccactcgattggtgacagtttgctgggggccaaatcatatacatcaaactacaatttcacaacgggtacccgaccgcaaaatgtgggcgccgatcaaaatggtggaatgcgcgccgcagaggaagcggcggaaaattactgggaagacaaccccaatactcaccacgttatttattaccaaacaactcccctgtataagggaagcgaaacgatgccccgtggatcaattgtcgatgtccgatcatcagataaatctttgaacacggaagttgtggttatcaatgacgctgaaggtatccgaattgattaccaagacggcagcaacaacgccaaacagtatcaccgacgcagctcgacgatggcttatacacatcatcgttcaactacttcgactgggagctccaattcacatcagagtgctacagccacaactacaaatggcggttggacaattgctggatccggaatggtgtttgtttctgatagtgacaagtattattctgaggtcaagaatcccaataattaccattacgagagtgtttttcaagcaaatgccagtggtgcaacccaagcatcgcgtggtaatcaatatgctagaccctagctgaatcaagacaactttggattgaagacgataatcttcaatctttttcttttaaaaattgtcgctgattatttatagatgacctatttaaactaaaaaacggtagtgaggcaatggtaatggaggctcactaattttcctaccctccctcacccaatacatccgactatcgttaatcagtcctgtattgattggtaatgactcgcattgagctctatgttaaaatgatcacgtagaatgctatcctaaattaacttatgaaggttggtgaacgtccgtgaaatttttaattgtatgtgcatccgccttaacgctgtgtacgggtgccgttggtgtcactcattattgtacaacgccgcatcaatcacagcctcgtgttgagcgtggttgtggtatgtatcggtaattgtggttttgttcttgattcaatttcaagtcaataaaaaaggaatcattgattgatattcaatgattccttttttattgatatttgttagtgataccggaggtggggttcgaacccacacgatctcaacgatcactggattttgagtccagcgcgtctgccaattccgccactccggcaaaataatatttgattggccaacacatggaaaaaggcggtaatcggattcgaaccgacgatgaaggttttgcagacctctgccttaccacttggctataccgccataactttggctaacccaactgggttagctggattcgaaccagcgcatgacagagtcaaagtctgttgccttaccacttggctataacccaatcaaaaggcggtatgtgggaatcgaacccacgcgtgtcggatccacaaaccgatgtgttaaccacttcaccaataccgccatagtattattaacagggatagtaggagttgaacccacaccgacggttttggagaccgtagttctaccattaaactatatccctataagatggaggggagtggattcgaaccaccgaacccgaaggagcggatttacagtccgccgcgtttagccagacttcgctacccctccatgaatggcgcgggacagaatcgaactgccgacacatgcagcttcaatgcattgctctaccgactgagctaccgagccattaaccatcttgagtataataatacctatgttgtgcattcaattttcaaatacataacaacggttcgtacgagactcgaactcgtgatctcctgcgtgacaggcaggcgtcctaaccagctagaccaacgaaccaatgttgctatggaaatggaggatacagggatcgaacctgtgacctcctgcttgtaaggcagatgctctcccagctgagctaatcctccataatgacccgtacgggatttgaacccatgttaccgccgtgaaagggcggtgtcttaaccacttgaccaacgggtcataaacttattattcggttacggagagtaagggattcgaacccttgaaacaggcttttacccgtttacatcatttccaatgatgctccttcggccagctcggacaactctccattaaaaataataactccggcaggcgggctcgaaccgtcgacaacctgattaacagtcaggtgctctaccaactgagctatgccggaataatcgcgtggcaacgtccta
